European Patent Application EP 4 678 733 A1 - sequence listing, part 2

SEQ ID NO: 4 - DNA, 5305463 bp, Variovorax sp. (residues 1,768,489-3,536,976 of 5,305,463)
  source 1..5305463: mol_type = genomic DNA
  gene 3283935..3288059: gene = rpoB; note = CDS of the gene; part of the gene of SEQ ID NO:3; note (original language) = CDS del gen; parte del gen de SEQ ID NO:3
  gene 2014365..2015895: note = From 2014425 to 2015865: Complementary fragment to SEQ ID NO:1; note (original language) = De 2014425 a 2015865: Fragmento complementario a SEQ ID NO:1; product = 16S ribosomal RNA; product (original language) = ARN ribosómico 16S
  misc_feature 1..5305463: note = Part of the genome (contig); note (original language) = Parte del genoma (cóntigo)
gctgccaccgcctccgcgaggcccggcagctcgaacacgccatggcgcgcaaaggtgttcaggttctgacgcaccatctgccacgatccgcgctgcgcgatctgcgcccaagcccgtgcgtccagctccagcgcagtcagcatctgaaacggcacgtcggctacttcgagcgaacggtagcgcttgtagcgttcgaaagcctgcgtcacaggaggcagcgcctccagcgtatacggacgatcgatcagccatgcgaaccacgcggcgcgccaggcttcggcgggcttggggtgaaccatcttcaccacgtcggccagcgacggcgtgttgcccacggacgcattcagcagctgcgcttcggtcgcttcgagcagccattgctgcacgagcttcttcggacgcgtaccgagcgacttgcggccgacggcgccggaacgcagcatctgcacgaagttgcgcagcatcttgccgttgtccaccacgcgggggaaaaccttggcgagcagcgccacgtcgcgcaccgccagcgtggcggccagcagcgccggcatgtccttcatgtggccggcgcggcgggcgtacacagccgtcttggccacgaacaccggatcgacttcgcgggccagggccagcacggcatcgagctggtcctgcgcttgtgcgtagaaggtgttgctcaggcaaccggtggccgcgagctgcgccagctggtgcttgggcgacagcgaataggccacgccgcccgcttcgttgagcgcgtcggccgcaggtagttgtgcgccgcggcgggtcttgaaaagctgaaggtttgccatggtgacttctcctcggggttctctttttttcgatttcgtatctgggtatgcactccttattgcaacgggtgtgccaagtaccggccaccggacgcagcgggcactcaactcattgatttcaaaagagattttttgattgagagcggatttcatcgagctctacgtgcagtttttatccatagttcttataatttcggatagtcttttatccaaaccaatgaagaaacccaccgtcgtcatcggcttcctcggcacgcagctcgatgccggacaaggcaccggccgctgggagaagtggcgccccaccgtctcgctggcccagcacgacgacatggtcgtctcgcgcatggagctgctctacacgctgaagcacaaggcgcttgccgaggtggtcagggccgacatcgccaccgtgtcacccgagacgcaggtcaacctcgttcccgtcgatctggaggacccctgggatttcggcgaggtctacacccgcctctacgactgggcgcgcgcctatcctttcgacaccgagcgcgagcagtactgggcgcacatcaccaccggcacgcacgtggcgcagatctgcatgttcctgctggccgaatcgcgcgtggttccgggcgtgcttgcgcagacctcgccgcccaagcggcagcgcgcgggcaatccgggcgagatcgcgctgatcgatctcgacctgtcgcgctacgacgccatcgcgcggcgcttcgatgccgagcagcgcgatgcggtcgccttcctgaagagcggcatcgccacgcgcaatgcgcgcttcaatgcgctcatcgacgagatcgagcgcgtggccgtgcgttcgcgcgcgccgatattgctggtgggtccgaccggcgcgggcaagtcgttcctggcgcggcgcatgttcgagctcaagcaggcgcgccaccagatgaccgggccgttcgtggaagtgaactgcgccacgctgcgcggcgacggtgccgcatccacgctgttcggccacaagaagggcgcgttcaccggcgcggcgggcgagcgcgcgggcctgctgcgcacggcgcaccagggcgcgctctttctcgacgagatcggcgaactcggcctggacgaacaggccatgctgctcaaggccatcgaggaaaagcgcttcttcccggtcggcgccgacaaggaagtggaaagcgacttccagctcattgccggcaccaaccgcgatctgcgcagcgacgtggcgggcgggcgttttcgcgaagacctgttcgcgcgcatcaacctctggacctacgacctgcccggcctcgcgcagcggcccgaagacatcgaaccgaacatcgaccacctgctggccatccacgcgagcgaaagccatcgcgtcgtgcgcttcaatgccgaagcgcgcgcggcctacctgcgctttgcgcagagcggcgaggcgctgtggtgcggcaattttcgcgacctctcggccagcgtgacgcggctggccacgctggcggacggcggccgcattccggtggcgctggtcgaggccgagattgcgcggctgcgctggctgtggaaccgcgaaggcccggcgaagcgtggcaaagacgccgccgatgtcgacctcgacgccctgctcggcaccgaacgcgctgccgcgctcgacctgttcgaccggctgcaactcgaagcggtggtgcacgtgtgccgcgaatcgcgcagcctgtcggacgcgggccgccagctcttccaggcctcccgcgcgcagcgcagcgtggtgaacgatgccgaccggctgcgaaagtacctggcgaaacacgggctcgaatggagccgcatcgccgcggactgactgagctatcctccgcccggatggccatctgcgcattcggccgcactctaggagaaaactcatgtcgctgacggtgctcctgcgatgccacgatctggccgcgacccgaaccttctacgccgatgccctcggcttcgcggccaccccatcggcggaaaagaccctgacggtcgagaaacagggcagcaagctcgtcttcacgcagcaggatctctggaagaccccgcccatctgctccggcactttgtatttcaccgtggcggatgcggccggctactacgcggccatcaaggacaaagtgcccatcgcgtggccgctgcagaacatgccatacggctccagcgaattcggagttgtcgattgcaacggctatcacctcgctttccagcaacaggcctgagcggtcgatctggaatgcgccccacgcagctgcgcttcttcttcagggaaaacaatcgatgatgaactggaagccggcgctgttcgccctgcccctgttcctcaccggctgcgtccagtcgatgttctattaccccgaccgcgtgcgctacgagacgcccggcgcgctcgggttgcgctacgaggcggtggagttccggagcaccgacggcacgcgcctcagcggctggttcattccagcgaagaatcgccagagcccgaaggaagccaagggcacggtggtgcatttccatggcaacgcgcagaacatgtcgtcgcactggcgcttcgtggcgtggctgccgacgcaggacttcaacgtgttcgtgttcgactaccgaggctacggccagtccgaaggcaagcctgagcccaagggtgtgtacgaagattccagcgccgcactgaaccatgtgcgatcccgtgccgacgtcgaccccgagcgcctcttcatcttcggccagagcctggggggcaccaacgccgtcgcggtggtgggctcgggcaaccgggccggcgtgaaggcggcggccatcgagtcgaccttctattcgtattcgtcgattgccaacgagaagctcccgggtgccgggctgctggtgagcgacgaatacgcggcgtcgaaattcatcggcgccatttcgcccatcccgctgcttctgatccacggcaccgacgatccggtgattccgcattcgcattcgcggcgcctgctggacgccgcaggcgagcccaagcgcctgctcgaagtggctggcgcggggcacctggagccgatgaccgagcgcttcggcaccacgtaccagcgcgcgctggtcgaatttttcgacgcctcgctgcgtccacggcaaccatgaagcacttcgacgaaaccgccacgcgcgagccgctggcctttgcacggctcgtgcccgcgctgcgcgccgccttcgcggccgaggcgcatgtgccgccgcgccatgtgcacagcatcgagacggccggcggcgacaagggcaccgtgctcatcatgccggcgtggagcgacgcggggtttctgggcatcaagaccatcaacgtcttcccgggcaacagcgcgcgcggcctgcccggcctgcatgccacctatgtgctgtacgacgcgcgcaccggcgttccgctggcgatgatggacggcaacgaactcacggcacgccgcacggccgccgcgtcggcgctgggcgcctcgttcctggcacggggcgatgcgcgccgcttgctggtgctgggcaccggccgcatcgcacggctgctgcccgccgcgcatgccagcgtgcgccccatcgacgaggtgcacgtgtggaaccatcggcccgaaagcgccgaggccctggcggcgcaatggcgcgcggaagggatcaatgcccaagccgccacccagctcgaagctgcggtgcgcgaggccgacatcgtgagctgcgccacgctggcgaccgcgccgctggtgcgcggtgaatggctcgcgccgggctcgcacctggacctgatcggcagcttcacacccgccatgcgcgaggccgatgcgcgctgcttcgagggtgcgcgcaccttcatcgacaccgccgaggcgctgcagaaggccggcgaactgctcgatgccatcgcagccggcacgctgcgcgccgatgcggtgcaaggcacgctggccgcactctgccggggcgaacgaaacggccgcacgggcagcgatgagcgcaccgtgttcaaggcggtgggcagcgcgctcgaagacctgacggccgccacgctggtctggcagcacgccggatcgccctctgcctaaggcttaaggactagaaagcggtcgccggccgtccggggagatagcctttggctgacacgcgcatacgtcatgcagctgatggcacggcttttgcgctgaagctaacctgatgctcataccaagagattcagaggccagccgcatgctcaccatttttcagaaagccaccatcctcagcaaagctggtttcgaagtgcccgcctgcccggccgtagacacgtcgacatcgccgaccagcgccgtttcccagaagatgcaggagtggggcaaagccatcgaaaccatgtatgtgacctacgtcgcagcccgtgcggccaagagcctgcgagatgccgaagagtcccgccagaccgacatgctgcgccggctttcgctgaacgccggggccgcctgaccccagccgaaccccttcgggctcagccgaaggtgaacgcataggcctgggcgccggcgtccagaaactcgatctcgaacaggcgctccttcgcgccagccgcctggcgtaccagctgatacagcttctgtgcctcgaccaccccgtggccctgcgcatcggtgtccgagccgtggtccgcaagcggcggctttccatcgacccgcaccctgaagcgcaccggcttgccattggccgcgggcccgagcaccagatgcaagtcgcgcgcctggaagcgataggcgatccgtccgccggcaccgttcagcacggcgcgctcggcctccaccgtccagtcgccggccagtgcccactggttggtgcgcagtgaggacgaagcaggctggtagaccttcgcatggtcccgcgcgatgccgccgggcgatgcaaagccgtgcgcacgctcgtggcccaggtaggtctcgccggacagggctggctccgtgccgggcgcggcctgggtgccctgccccagcggcgccaccaacccggtggcgatgcgggtcttctgccccgcctcggccagcagctgctggatgaccagctcggccttgtcgtaccggttctcgccgaactggtgatggcggatgcgcccctttgcatcgacgaagtagaacgcgggccaggcgcggttgtcgaagccgcgccagatggcgaagtcgttgtccatggccaccggaaagtcgatgcccaggtctttggttgccttgcgcacgttggccgagcgcttctcgaacgcgaactccggcgtgtgcacgccgatgaccaccaggccggcgtccctgtatttttcggcccatgcgcgaacgtaaggcagcgtgcgcaggcagttgatgcacgaataagtccagaagtcgaccagcaccaccttgccgcgcaacgcctcgggcgtcaggggcgcggtgttgatccattcggtggcgccggcaagcgaaggaaagttgccttcgaccttgagcgcgcgcatgggcaccgtggccgggcggtcttccttttccgacacgcgcacgaggcccgtgtcttcgcgcagcgcgaccggttcagccaacggctcgcgcgaaggctgcggcgggtctttcttgattttttccaccagcgcctgctccagcgccgacgtggtgcccaccgacaggcgtgcgagcagcccggtatccagccccagcgcaatggcacccacgcccaccagcacggcagcgcccgccacgcgccgcacccattcgccggtatgcagcgaacgcttcatggccgtgagcaaccgcccgccgaagagcagcgcggcggcgagcgacgtgcaggcaccggcggcgtaggcgagcagcagcagcgaggtaccgacgctcgcgccattgagcgccgcgccggtcaggatcaggccgaggatcgggcccgcgcatggcgcccacagcaggcccgtgcccacgcccagcaacagcggcgagaacgccgaggcggtgcccgcgcccgcatggccgtgcggctcggacatgcgcagccccagcgccaccagcggccgggtcatgcgatcggcgacggccgggaacagcagcgtcgcgccgaacagcgcgagcattgccagggcggcgtggcgcccgtactcgttgagcgtgacgatccagccgccgcccaccgcggccagcgtggccacggcggcaaaggccaacgccatgcccagcagcatgggcaggccgtgcgagcgaaacgggcggtcggcgcgcgcaaacacgaaaggcagcaccggcaggatgcaggggctcaggatggtgagcaccccgcccaggtaggcaacgaggagaatgagcatgatgtcggtcgtccgggacgggtggattcagcgagcgggcgcggtggccagcgcgagccgtgcctccagtccaccttcgggtcggttgtgcagcgtgagctcggcgcccatggccatggccagctggtgggcaatggccaggcccagcccggtaccgccggtgctgcggttgcgcgaactctcgacgcggtagaagggcttgagcaccgcctccagctcatcggggggaatgcccggcccgttgtcgagcacgctcagcaccaactggccgccttcggcatgtacgcggaggcgcacgtcgctgccgaacttcagcgcgttgtcgatcaggttcatcaagatcctgcgcagcgcgttgggtcggctcacgatgggcgcgccggccttgccttcgagccgaaccggctggcccacgtcttcgtagtcggccaccatgctttcgagcagcgcatcggcatcgatacgcagcggcggctcggtcgcgccgtggagcgtgcgcgcataggtcacgccttcgcgcaccagcgagtgcatggcgtcgaggtcctggcggaacttctcgcggtcgtgttcgttgtccatcaggtcggtgcgcagccgcatgcgcgtgatgggcgtctgcaggtcgtgcgaaatggccgccagaatctcgacccgctcggccatgtagcccgcaatgcgctgctgcatggcgttgaaggcgcgcgccgcatgcgccacttcggtcgggccttcttccgcgagcgcctgggccttcaggtcgggccccaggtcgtcggccgccgcggacagctgcgcgagcggacgcgtgaccagccgaaccgcataccaggcgcaaacggccagcaccagcagctgaacgaccagcacccacatgacccagcccgacaccggcatgcccacgcgcatggcatgaaccaccaccgaagacccgtcgctcaggcgcacctggatctgcaggccctcgggcggccaggccacctcgccgaccttgacgatttcgaacgggcgcatcgcatcggcgatggccgcggcaaactgccgcgaaggctgcgagccaggctcggtgccctctgcgctgccgcccagcacgaagcggtagttgcgccgctccagccggtcgagccagccggcgcgttccgccgcgggcaggcggtcgaggatggcgaccgagcttgcgatgtcgcgctcgatgccgatcatcatcagctcgcgaagcgccaggttccgctcgtagcggatggccgcgaaggtaagaagctgcgcgacggccaggcccaccacgatgatcagcgtcacgcgatagaacagcgaaccgggcagcatccggcgccagccccgggcggccatgcccccaccggcggcacttgcggcaccagacgggttcgcggaaggattcgcgggagtggacatgcgcacctcttgtttatgaataccgctggctcacaccaggtggatggcaacgtcgatgttgccccgggtggccttggagtatgggcaggtctgatgcgccgcgtccgtcagtgcttttgccacttcgcggtcgaggcccggcaggctcacgttgaggcgcgcctgcaaaaagtactcggtgcccgccgcgccgaggtcgacttcggcatcgacggccaggtcgggcggcagcgtgaccttcatcttgccggccgccttgcccatcgcgccgatgaagcaggccgaccagccggcggcaaacagctgctcgggattggtgccgctgcccgcactgccgggtgacgaaagcttgatgtcgagccggccgtcggagctgcgcgcttcgccgtcgcggccgcccgaagaggtgtgggtcttgccggtgtagagaactttttcgatgcgggacatggtgattccttgggagtggttggttgggaacggacggattgttgggccgcctctcccctgccaacgcacattgcgtatgcctgtgtatccgcgcgataaatccacacactacgtttcaccgcggcacggctgcggcacattggcggcatcgtgacgcccccgagcatcgcggtctgcaaggctttcatgcgtccgctttgtatgcctgtgtatctgcggccgcagaagtacacgggcatacaagaacacccttttctcgacacatggcaaatacatgccgcgaatccaatggcgcatcgattcatccgagcaaccaactaacgccaaggaaacgcacatgtcgaatgaagcagtcaaccgccaacgccgatttctcctcggaggcgccgttgccggcgtcgccgccgcggagctggcattcatgggcgcggcccacgcggccccaacgccggcgggcaagccgcagaagctcggccccatcaagcaggtcaaggccggcgaactcgacgtcggctactacgaggccggtcccgcagacggcattccggtgctgctgatgcatggctacccctatgacatccacagctacgccgaggtggcgccgctgcttgccgcgcgcggctgccgcgtgatcgtgccgcacctgcgcggccacggcagcacgcgctttctggacagcggcaacccgcgctcggcccagcaatcggcggtggcgctggaccagattgcgttgctcgacgcattgaacatcgaccgcgccgtgatggtcggctacgactggggcgcgcgcaccgcctgcatcattgcggcgctctagccggagcgctgcctgggcctgctctcggtgaacggctacatcatgaccaacctgccgggcaacaagctgccgctgcccgccaaggcggaacacggctggtggtaccagtactactttgcaaccgagcgcggccgcctcggcctggaggccaaccggcgcgacatcgcacgcatcctgtggactaccaattcacccaagtgggcctatgacgaggccaccttcgagcgcaccgccgcatcgttcgacaatccggactacgtgcagatcgtgattcacaactaccgctggcgcctgagcctcgcggacggctttcccaagtacgccgaactggagaagcgtcttgccaccttgccgaccatcggcgtgcccaccatcaccatggacggcgattccgacggcgtggtgcccgcaaccgatggcaaggcctatgccgccaagttcaccggcccgcgctcgcacctgatcgtgaacgccggccacaacgtgccgcaggaagcacccgaggcgtttgccgatgcggtgtggaagctggcatccgcgcggcactgagctccaaccataccgggcgtgcgcgcaacataatgtcgcgcgccccccatcttttccgctcgatgccatgacgccaaagacttcggaccacatcctcatcgtcgacgacgaccgggaaattcgcgagctgctcacgacctacctggtgaagaacggcttgcgcgtggtcgcggtgcccaccggccggcacatgcgcgcggcgctggaggagtcgggcccgttcgacctgatcattctcgacctgatgctgcccggcgaagacggactcacgctctgccgcgacctgcgcaccggcaaatacaaggcgacgcccatcctcatgctgaccgcgcgcagcgaagaggccgaccgcatcctgggccttgaaatgggcgccgacgattacctggccaagccgttttcagcgcgcgagctgctcgcgcgcattcgcgccgtgatgcgccgcacgcgcatgctgccgccgaacatgggcgccatcgagtccgcacagaaactggggttcggcgaatggcaggtcgacacggtggcgcgccacctgatcgacgacagcggcgtgatggtggcgctgagcggcgccgagtaccggctgctgcgcgtgtttctcgaccacccgcaaaaggtgctgagccgcgaccagctgctgagcctcacccaaggccgcgaagccgagctcttcgagcgctccatcgacctgctcgtgagccggctgcgccagcgcctgcgcgacgatgcgcgcgagccccgctacatcaagactgtgcgcagcgaaggctacgtcttcgcttcggcggtcgaggcgagagactgaccgacgcgacgcactggcagtgggtcgggttgcgcacctcgtgcgccacgccgcctgcaaagaacagcagggcgaaccagagcttcttcatttcgggccgctcggcgcattggcagcggttgcattcgaaggctccgcaagcagcgcctggatcttcttctcggtggtgccgtagctgccttcgccaaagtgcgaataggcgatgcgtccctgtttgtcgatcaggtacacggcgggccagtactggttgttgaaggccttccaggttccgtagctgttgtcttgcgccaccgcatgcttgatctgcaggcgctggatggcgtccttcacgttcttggtcgatttctcgaacgcgaactccggcgtgtgcacgcccaccacggtcaggcccttgtccttgtatttctcgtgccattccttcacgtgcggcaggtgattcaggcagttgatgcaggtgtaggtccagaagtcgaccagcaccacctggccgcgcagcgcttcgagcttgagcggcggcgagttgagccaggtgtcgatggcctggaactccggcgcagcgcgcgccacgcccgcgggcgcgtcaccgcccatcggcggcgcggcaaaagtcaatgcagccaccgacgcggcaatggccgcgccaatggcaatgcgggagagcttcatggtgatttcctcggtgcgatgcgcaacgcgcgctggtgaatgacgggcggattgttttccgcccgtcgagcccctggcacacattgcgtatgcctctgtgtcgaggctggaaatcgacacactacgttgcacgaggcgggtgtgcgcgccccgtctccatcgagccaatcggccgggcagcaggctgcgcccggcgcggctctcagacccgttccaggatcaccgcaatgccctgacccacgccgatgcacatggtgcacagcgcatagcggccgccgcccttgtgcagctggttcaccgcggtggttgcaaggcgcgcaccgctggcgcccagcggatggccgagcgcaatggcgccgccgttgatgttgacgcgcgcgtcgtcgtcctggaggcccagcaggcgcagcacggcgaggccttgcgccgcgaaggcttcgttgagttcgatcacgtcgatctggtcgatggtgaggccggtgagcgccagcaccttctgcgtggcgggcgcggggccgatgcccatcacgcgcggcgccacgccggcagtggccatgccgaccacgcgggcgcgcggcgtcaagccatgcttggccgcgctggcttcgtcggccagaatcagcgcgcaggcgccgtcgttcacgccgctggcgttgccggccgtcacggtgccatcggggcgcaccacgcccttcagcttggcgagcgactccatgctggtttcacgcggatgctcgtccttgttgacgatgatggcgtcgccctttttctgcggcacgctcacgggcacgatctccgcgtcgaagaagccggacttctgcgaggccacggcgcgcaactgcgagttgagcgccatcaggtcttgcgcttcgcgctcgatcttgtggtccgtggccacgttctcggccgtctcgggcatggagtcgacgccgtactgcgccttcatgagcttgttgacgaagcgccagccgatggtggtgtcgtacaccgcgttgttgcggctgaaggcgctctcggccttgggcatgacgaagggcgcgcggctcatgctttcgacgccaccggcgatcatgaggccggcttcaccggcgcggatggcacgggcggccgtgcccaccgcatcgaggccggagccgcacaggcggttgatggtggcaccgcccagttcgagcggcaggcccgccagcagcgccgacatgcgcgccacgttgcggttgtcttcgccggcctggttggcgcagccgtagagcacgtcgcccacggcctgccagtcgacgttcttgttgcgttccatcagcgccctgagcggcacggcgccgaggtcgtcggcgcgcacgctgctgagcgaaccgccgtagcggccgaagggggtgcggactgcgtcgcagatgaaggcttggttggtcatggtgtgtctcgttggaagtgaatcgaactctgaagcccgcttttatgcggcgatcggcaagcccacgagcttctcgagctcctcgcggctgagcccttcgaccagatcgacgagcttcaagccttcggccgtgcattcgagcgtggcgaggtcggagtacacgcgcttgacgcagcggatgccggtgagcggataggtgcattccttcaccagtttgctcgcgccctgcttggtgagcaagtccatcatcacccaggtctgcttggcaccgatggcaaggtccatggcaccgccgacggcgggaatggcgtctttctcgccggtgtgccagttggcaaggtcgcccgtggccgacacctggaacgcgccgagcacgcagatgtcgaggtgcccgccgcgcatcatcgcaaagctgtcggagtggtgaaagaacgagccgcccggcagcagcgtgacgggctgcttgccggcgttgatgaggtcgtagtcttcttcgcctgcctcgggcgcggggcccatgccgagaatgccgttctcgctctgcaggatgacttcgcggcccttcggcaggtggttggccaccagcgtgggctggccgatgccgaggttgacgacggcgccgtcgaagatgtcctgtgccacgcgggcggcgagctggtccttggtgcgacgtgtgtagttggtgctgctcatggtcatgctgccttcttgaaaccgccggcctgggtggcgacgcgttcgacgcgcaccacctggtgcacgaagatgcccggagtcacgatggtctcggggtcgagggtgccgagctcggcaatatcgtgcacggtggcaatggtcttcttggaggccatggccatcaccgggccgaagttgcgtgcggccttgcggtagaccaggttgccccagcggtcgccgcgctcggccttgatgagcgccacgtcgccattgatggggtactcgagcacgtactgcacgccatcgatctcgcgggtttcgcggttgcccgcgagctgcgtgccgtagcccgtggggcagtagaaggcgccgatgcccgcgcctgcggcgcgaatgcgctcggccaggttgccctggggcacgagttcgagttcgatcttgccgctgcggtagagcccgtcgaacacctggctgtcggcctggcgcggaaagctgcagatgatcttgcgcacacgcccggccttgagcagcgcggcaaggccggtttcgccgttgccggcgttgttgttgaccacggtgaggtccctggcgccctgctcgacgagaccgtcgatgagttcgccgggaatgccggcggtgccaaagccgccgatgagaaccgtggcgccgtcttggatgcccgcaagggcatcggcgaccgagcgcgcgatcttgttgatcatgaagcctgtctccgggagttgaaaaagaaatcgaaccctgcgaacaaaccgccaaacaatcgcccgattctgcgaaccgcaaaattgttcgtctaaagaacatttgttcgtataatgaattctaaagacgaatgctcgatatggcaacccacacgacacaacccgacacaccagcccccggcgacagctacgtgcagtcgtttgcacgcggactccaggtgatccgttctttcagcgcaagcgcgccgcggcagacgctgagcgaggtggcggccgccagcgggctcacgcgggccggcgcgcggcgcatcctgctcacgctgcagacgctgggctacgtggtgaccgacggcaagctcttcacgctcacgccgcgcatcctcgacctgggctttgcctatctctcgtcgatgccgatatggaaccgcgccgagccggtgatggaagcgctggtgcagcaggtgcaggagtcttgctcggccgccgtgctggatgcgaccgacatcgtctatgtgatgcgcgtgccgacgcagaagatcatgcgcatcagcctgggcgtgggctcgcggctgccggcctactgcacgtcgcttggccgcctgctgctggccgacctggacgacgacgaggtgcgcgcgcggctcgaagcctcggagcgcacagcgctcaccaagcacacggtgaccgacgtcgacgcgctgatggccaaggtggcgcaggcgcgcaaacagcagtggtgcctggtgaaccaggagctggaagaaggcctgatttcggtggccgcgcccatcgtgaaccgccagggccgcatggtggccgcgctcaacatcaccgggcaggccaaccgcaccaacgccaaggtgatgcaggagacgatgctgccggcgctgatggaggccgcaaagaagatctcacagctgctctaacgaaccaacggcccaatccagcgcacccgcggaaccgactttgccgggccgccgggtgcgccccccagtgggggctgagcgcccgcggctccaggcccgcctgtgcgggcttggacgggccgaagggtccgtgcctccggcatggacaccgggcgccgaaggcgcttcggggggcgtcaagtgctggagtggatgcccttcatgatgatcacgccacccagccgcgcggtgtcggcgcgcatgcgcttggccagcgcgtcgggcgtgcccggctgggcctgccagccggtcttcagcagcgcctcgctcacttcgggcgagcccatcgcctcgaccagcgcggcattgagcttggcaatggcggccggcttcatggccgcgggggccgccagcgcggtccagatctccaggtcggcgccgcgcacgtcggcgtcgcggatcgtgggcagttcgttggccagcgggctgcgctcgggcgacgtcacgccaatggccttgaccttgccggacttcacatgcggcatggccaggccgggcggcagcagcgccaattgaatctcgcccgccagcaggccggcgatcacctgaggattgcccgtgtacggcttgtgctgggccgtgatggcggcgcggctcttgatgagttccatgcccaggtggcccacggttcccacgccgggcgtgccgtacttgccgttgctgccgaggttgcgcgtccacagcagcaggtcggccgcggtcttgcccgtggcattgcccgagaccaccagcacaagcggcgcagtgccgatcaggccaaccggtgcaaagtctttttccgggtcgaagctgagcttggggttgagcagcttcgcaatggtgaggttgccgttgatcagtgcgccgatggtgtggtcgtcgttggccttggccacctggtcggccaccagattgccgctggcgccgggtttgttctcgaccgtgaccggctggcgcaggatcttcgacagcggctccgcgatggcacgggctgcgaggtcgggcgaggccccggcgggaaagcccaccaggatgcgaacgggcttggtcggccatgcggcgtcgccgccggcagcaccggcgccggtgcgctgtgcccatgagcccggtgcaaaaagcgatgcggcaattgccgcagcgccgccttcgagcaggcggcgtttggtgatcttcaagatgactccagagaggaaagaggaggacgttgtttttgttgtacttacatcacgttacatgatcgggctcgattgcgcaagtcgatgcgtattcatggatgtggtcatgcggccgttggcagcgcaacgcgtcgggatgcgacagccccgagtgaacgttgtgtccgaaggttaactgcccacttacaatccctgccgcatcacccttcccccatacgaggtctcgtccgcaatgcccaagagccccctgccgcgcgcccgtttcagcttttcccccaccgtgcgtgccctgctcgtggccactgcctgcggcttggcactgcccgcgcttgccgcggtggagcacgacgaggtcgatcggctcatgcaggctggcaagctcgacgaggccatgtcgcgcgccgacgctttcctgaaggacaagccgaaggatccgcagatgcgcttcctgaagggcgtgatccagctggataccggcaagcgcaccgaagccatcgccgccttcacgcagctgacgcaggacgcgcccgaactgcccgagccgtacaacaaccttgcggtgatctacgcgagccagaaccagttcgacaaggcacgcagcgcgctcgaaagcgcgattcgcaccaacccgagctatgccacggcgcaagagaacctgggcgacgtgtatgcgcggctggccagccaggcctacagcaaggcattgcaactcgaccagaacaacacggcggtgcaacccaagctggcggtgatccgcaccttgttcacgccggcaccggtgggcggcaaatccgcagccacggcggtggcggctgcgcctgccgcaaagacggccgcgcccgcgcccgcttctgcgcctgcgcccgtcgcgaaggcagccgctgccccaacgcccccgccagctcccgtgcctgcacccgcacctgcgcccgtcaaggcagcggcagcacccgcacccgtggcagcgccgacgcccgtgccaccggcaccgccgccggtggtggtggcgaaggcgcccgaggcttcgtcgacgccatccgcatctgcatccacgccggctgcggccgcggcaacagcaacgcccggctcgacggccgaggtggaatcggccgtgcgcggatgggccgccgcttgggcgtcgcaggacatggaccgctaccttggcgcctacggccccgagttcaatcccggcggcggacaaagccgcaagagctgggaagaagaacgccgcgcgcgaatcgtcggcaagtccagcatcagcgtgaatctcgagaacctggcgatcaacgtcaacggacaaaccgcaaccgccaagttccgccagatctatcgcgccgacaacctcaacatctcgagccgcaagacactggagctgcatcgctccggcaaccaatggcaaattcgcaaggaaagcgtcggggggtagtggcggacatcgtccggcgcggccggctcccgaagaacgctccgttccggcgcagcgggaacatgcttgcggcgctcgtggcggcgtcggtcctgttgctgacggcgcccggctcggccgatgcctccaccaagcccagcggcaccaccaccaagtcgaaggccaacggcagccgacccacaaaccaggccgccagggaagcgaaaccccgggcaaagaagacctccgccgcacaaaccgcaagcgcggcaagcagatccacgccgcgcaaggcggctgcatcttcagccgcccttcagcaagccaacggcgccgaggcccgcctgattgcggtctacgaactgttcggccgcggccagccgcggcccgcgctcgccaaggcccgcgacctggtgcgcgattaccccaactttcagctggcccagctggtctacgccgacctgctcgcaacccaggtaccaccggcgcacgccttctccgacgcctcgggcatcgcacgcctgcgcagcgatccggccatggccgaactgcgcgaagaatcgcagcggcgcctgcaggccctgcgcgacaggccgcctgccggcaccgtgccttcgcagttcctggcgctgtccacgcgcagccgctatgccattgcggtcgacgcttcgcgttcgcggctctacctgctcgagaactccgacaaggggctgcagctggtggccgattactacgtgtcggtcggcaagtcgggcatcggcaaggtcgcggaaggcgacgcgcgtacgccgctgggggtgtactacatcaccagcagcctcgatccgaagtcgctgcgcgacttctacggcgccggtgcgcttcccatcaattaccccaacccgtatgacgtgcggcgcggcaagaccggtggaggcatctggctgcacggcaccccgccccagcagtttgcgcgcgcgccgttggcaagcgacgggtgcgtcgtcatggccaaccccgacctgaagcagctcctgcgcaaggttcagatcggcgccacccccgtggtcacggcccgcagcctgcaatggatctcgccgccgcaggcccagaaagaggcccagtcattcaccagcgccatcgcagcctggaaagatgcacgggccaatggcaatgaagcgcaattgaagaaattctatttgcctgaattccagcgcaacaacaataaaaaatccatcgaaggattttccgtgctccacgacgaagtggaatatgcccaaggcaaacgtgtccagttcaaggacatgtcgtatctgcactggcgcgacggcgacgaaaccatggtcgccaccttcggagaagtcttcgaaggcgaaaagagcgggcgcacccggcgccaatactggctgcgccaaggcagcgagtggaagctctttcacgaagaaatcctgggctgaacccggctttcggccctcctgccaggggggtcatactcaaaatccgtgattttttgcgcaaatgccggcccgaacttggccgttacatttcggctcacggcacccgtgctacgtaacacgtaacgcatttgttcccgtaacgccggccctgtgcgcgttccgtccgcaccgtaacgacgtcccctgttcaggggatgggtacctctgttctcagagggaagaatggtcaccagactgtgaactaccctctgaaattcaaacgcgtcttggggacggcgcggggttggccgcgttcctgcttagacccttcgattaacacaggaaccctcccatctcatgggtaccccttgttgatacacagagttacgccgtataacattcacctgtcgtcactgttgttaacaattccttaaaggggaaatcatgcttcgctctattgctcgttttctgcgcgatgaagaaggtgctaccgcaattgaatatggaattattgcggggttgatttcggttgtgatgattacagccattactggcactggcgggataggcgagagcctgtcagccatctggactgacatcaaaaccaagctcgccgccgcttgaagtgcaatgcaagcaatgacatcggcgtatttgatgtggttgcttttcattgcggtgtatgacttcaggcaacgtcgcgtccccaattggcttgtgctcgcaggcgccctcctggctcttgcagcactgacattggggatggcgcccgttacgcacgactgggctgccgccctgctcggtgcaggcgtggcttttggctttctgctgcttttctacgctcttggagtcatgggagccggcgacgtgaaattcgctggagcgctcggactctgggtaggcttttcggcgctgctccccgtctggctcatcggcagcctcctcgccagccttcatgccgcgctttggctgattcttcggcgctggccagtcttcccccggttttcgctcgtgcttttcgggccctcgtcgccggcagatggcaacccatcaccgccccgggttcgctttattccttatgcggcctatctcgcgctggccgccgcggtgtggatggtttggggtcgacagagcgcctagtcgctccgccaccacgagctgttcatcgatagctctcgaattgctcctccttgacacgccgctcatgatcaatctcaccaaaatcatcgccgccgtcctcgtgctcctggccttcgcgctcggcggctatgcatggatgctcagccgcaagcccccaccgcccgtcgccgtcgccccctctgccgccgctcccggcaaggccgcccaggcgcaaaccttccccgtggtcgtggcggccaagccgctgccggcgggccagccgatcccggccgatgcacttcgcattgaacgcctgacgatcaatccggtgggcgcgttccaggacaccgcgccgctcgcggggcgcgtgcccgtgatcgatctgggcgaaggctcgccgcttctccaaggccagctcgtttcgggtcttgccctgcgcgtcgcagaaggcgaacgtgcggtcgccatcaaggccgacgagatcatgggtgtgggcaacaaggttcaacccggtgacttcgtcgacgtgttcctgatgctcaagtccgacggcaaggacatcgaccgaagccaggcgcgcctcttcctgtcgcgcaagcgcgtgctggcgtacggcagcgcctccgtcgatggtctgccttccaagatggacaagaacggtaccgcacagcaggcccagcgcgccgaggcggcccggactgccgtgctcgcagtgccggtggacgacgtcaaccggctcacgcttgccgagaacagcggccgcttgatcctggcgctgcgcaatcccaccgatatgtcggaacccgatccgaagctcttcgccgagttgccccccgccctgcaaccgcctccaccgaaaaccggcgaaccgcgccgcccgcaactcgaaggcttggaccgcgcacaggctggcatcaccacggcggatttcgtgaccggcggcaagccgggcagcgcctcacgcgtgccggctattgctgctgcgcggattccaacggctcgcactgacgactcccgcggtggactcaaggtcgaagtcattcgtggcgaccgtagcgaaaccatcaactactgatcagcaacaagcgccacccaggaaacgaactccatgacgatcgcccttctcgcgaaaacaaccggtccagcccgtccactgggtccagcactcgcggtgctgtgcctgctggcctcgggcgtctggcctggggtctccgcagccgcagatccggcagaggcgacgtctcttcgccccgcacttcaactgcggatcgacgcgggcacgcaaaaggaactgctgatcggcaagggtatcgagcgcatggccatcgccgacgagacggtggccggcgtcgcgctcacccgccaatcgcccaactcgccggccgcgcgcctcatcgtcaccggcaaggctgcggggcggaccacgctcatggtctgggaaaaaggccagtcgaccgccacggtctacgcgctcgaagtgcggcgccgcgcctccacgctctccggctcgctcaacagcatgactgcgcaccaggaagcgcgcgatgcggcgatggccgccggcggagaaaagtcggcactgatcgatcgctccgtcgtcaacgtacggagcaacaccgtgcaggtcgaagtcaagatcgtcgagttcaaccgcagcgtgctcaagcaggccggcctcaacatcttcagcacgcgcgccaactccaacggtttcagcttcggggtcttcgcgccctcatcgctgcgctcggtgtcgttcgctcccaacggggcagtcagcagtgaacacaacaatccgctcgcccaggccttcagcctcctgttcaattttggcaaggccggtatcggcctgaacgttggcttcctcgaaggcaacggcatggcccgcgtgcttgcggaaccgacgctggtggcgctgtcgggccagagcgcgagcttcctggccggcggcgaactgcccgtgcccgcgccccagggcctgggcaccacgagcatcgaatacaagccgttcggcatcggcctcacgctcacgcccaccgtgctgtcgaacgaccgcatcgtgctcaaggtggcacccgaagccagcgacctggactacaccaactcgctcagcattggcggtgtcgctgtgcccgccatcagcacgcgccgggccgacaccacggtcgaactcggcgacggcgagagcttcatcatcggcgggctggtgagccgcaccacgacttcgaacgccgacaaggttccattgctcggcgacatcccggtgctcggaaccttcttcaagcagaacaagtaccagatgagcgagaaggaactggtgatccttgtcacgccgcatctggtgaagcccattgcacgcggcacggatcttggtccgtacctgccgggtggtgccgagcaacgcgatggccccgtgtggcgcgcgcatctgctggggccagcttcaggcacgactgtgccggggttctcgcgttgacagaaacgagctacgcaaagcctgcggccgatgccatgaacgctccacgcgacagcctccccgagaccggtgcggagagctatctcttcgcatcgccgaacagcagccacatcacatggctgaccgatgcacttggccggctgggcgcggtggtggtccttccatccgaagccaagtcgatcgacgagcggatcgccatgctcggtcccgcggcggtctttctcgatttttcgggcgaccacgccactgcggcaagcgaacttcatcagcgcctcaagcgtgaatggccgacgctgccggtactggcaacgggcgtttcggccgagccggcttccatgctcgctgccctgcgcgcaggggtggacgattttgtcgacatgagcgcaccgccgaccgatgcgatcagtacgctgcgcaagctgctcgatcgtcaaagcagcctgcaaagccgcacccgcggatgcacgcttgcactgcttggcgctcgcccggggattggcgtgacaaccctcgcggcaagtctggcactgatgctcaacgaccagccgtcccaaacggccgcgccttctcatgctcgcaacacgcgccgcggagttgcgttgctcgatcttgggctgcccgcccgcgacggtcttctgtatctcgacacccaaagcggcttcagctttgtcgatggcgtacgcaacctgcgccgcctcgaccagaccctgctgcacaccgcggtggcccaccacacgagcggcgtcgctgtgctcccgctgccagcgagtctcgcgcaggtgcgcgagatctcgcatgcggactcggtggcactgatcaagcggctcggcgattttttcgatttccagatcgccgacctcggcggtttttcaaccctcgatttcgtcgcccagaccgcgaaggcagcccagcgcaactgggttgtgtgcgaccagagcatcggtgcgatcgtctccactgcaaacatgctcaaggagctgcgcacccgcggcgtcgacaccgatcggctgtcgctcgtggtcaacaagttcgacagccaagtcgggctgccggccaaggacattgcggaacggctcgaactgccgctccaccatgttgtgccggcgcgcgctacgcaactgctggcggccgcgagccgcggcgaaatgctggtgcgtaccgcgcgcaatgacgcgtattcgcaagccatagcaagcctcgcacgcggactgaaccaggaatacatgtccgatgcaggccagccgccggccaagcaatcgccttgggcgacgcgaatgtcgcaaattgccggattctggaaaagctctagccaaggttgaatcgcccctatgtccaacgatctcgaattcgccgacgacgaccaggcgttcatcaattcccaacatttccaggacatcaagagctggacgcatgaccatctgctgagccgcatcgaagagctcggtgcggagttcggccgctggtcgcgcgcctcgatccagcagttcgtcgaactggaggtcgacagcttcgtccggctgcgccgcgttccgatcaatgaccgcgagatgcagctcatctccgatgcactgaccaaggagcttgcaggcttcgggccgctggaagacttgctcaacgatcctgccgtcgaagatattctgatcaacggctaccagaacgtatacgtctcgcgtcacggcatgctggagcgagagacggtgcgctttgcagatgcggagcacgtgatgcgcatcgtgcgccgcatcctcgcgccgctcgggcgccggctcgacgaatccaacccgatggtcgacgcgcgcctgccggatggcggccgtatcaacgtgatcatcgagccactggcgatcgacgggctctcggtttcgattcgaaagttccgcaaggagccgctcacgccggccgatctggtgaagctcggcaccttcgacgctggcatggcgcagttgctggaaattgccgtgcgcgcgcgctgcaatatcctcgtcagcggcggcaccagctcgggaaaaacctcgctgctcaatgcgctcgcaaccttcattcccgcgcgcgagcgcgtcatcaccatcgaagacacggcggagctgtcgctcggcaccagccacgtcgttcggctcgaaagccgccccggcggcttcgacggcacgggcgtggtgtcgatccgcgacctgctgcgcaacagcttgcgcatgcggccggaccgcatcatcgtgggtgaagtgcgcggcgccgaagtcatcgagatgatgcaggcgatgaacacgggccacgaaggctcgatgggcaccatccacgccagctcgccgcgcgaatgcctgtaccgccttgaaatgctcgcaggctttgcgggctatcagggcagcgaagtgagcctgcgccggcagattgccaatgccatcgatttcatcgtgcagatcggccgcctttcgaacggccagcgccgcatcctctcgctgagcgaagtcacgggcgtcaacgacaacgtggtggccatgcaggagctctaccgctacgagcccatcacgtcgcccgacggcgaggagcgcgaccgctggatatcgctgggcattgcgccgcattcgcccaagatcacccgcttcaggcagtcgctgacacgcgcgcagcagggagacaacaaccgtgcgtgaaatgctgctcgcggtggcctgcctcgcgctgctgctcgcagccgcggggctgctgctgtggcaatgggccaagggccgccaggcacgccaggcggccgcacggcacctgaaccagcagatccaggcaagcacggccgccggcgcaccggcgccgatgccgatgcctttgcgggaccccgccaacgacaacctcatggcgggcgtgacctcggacccttggctcaacaccgacgcaggcaacacggccgccgcacccgccgggttgctcgaaaaggccctgcccgaatggctgataggcgtgatcgctccgcgcacggccgcactgggactggccgtcatcgtggcggcggccgcactcgccggcctgcttgccggctgggtgtcgggcctgagtgcactcgcgctgctggctgttctttcggccttcgcggtctggctgcggctgcagaagttccgccgcaagctcgtgagccagctgcccgcgtacatcgacgcgatggtgcggctgatcaccatcggcaactccacgcaggcggcgttccagcttgcgattgccaccaccgaggcgccgctgcgcggccaactggagcgctctgcatcgctggtgcgcgcgggcatggacctggatcgcgccctgcaccagacggccagcaatgtgcgcatcgaggaaatgttcctgctggcgtccatcctcggcctgggtgtgcgctacggcgggcgctccgacctgctgctggagcgcgtgggcaacttcatgcgcgatcgcgagcaagccgagcatgagctgctcgccctgtcgtccgaaacccggctttccgcctggattctcgggttgctgcctgtgagcgtgggcgccttcttcatcctcaccaatcccggctacttcatgggaatgtggaacgacgggaccggacgcgtcatggtcctttccgccgcgggctttcagctgttcggtgcggcacttctctaccggctggcgaaactcacatgaccttcaccaccaaccagctggcgatcatcagcctggcgctgctggccctgggcctgatggccggtgccggcgcgctgattgccgcggagttgcgccgcacgcgcagcggcaaggtcatcggccgcgccatccagcaggtcaccacggcgccgggcggatccgcggcgtccgtcgatgcggccgacgggttcaacgcctcggcaaagccggacatcgagttgccgtttcactggctcgattcgcggatcggccgcgcacttgtggccaacgaggaccggaacctcatcgatcaatgcggcttttcctcgaagcgggcccagctggttttcctggtgacccgcatcctcttcaccttcctgcttccctttgccgtctacgtgctgtggagcgcgggccggccgcagcgcaccgtcaccatcgtgctggcggtcgcgttcgtcatcggcttcatggcacccaagtgggtgctcggccgcatcgccgccaagcgccgcgagcgggtgaaccaggagctgccgctgttcatcgacctgctccgccttctgcaaggcgtcgggctgagcctggaccagagcctgcagatcatggccagcgacttctcgcacgtgctacgcgtgctcggctacgagctgacctttgccaacaaccagtacagccgcggccgcagccgcgagcattcgttgcagcgccttgcaaccttgcacaagaacgagaacctccgcgggctcgtttccttgctggtgcaggtcgacaaacacggcggcgccgtgcaggaaccactgcgcatcttcagcgaccggctgcgcgaacaccggcgttccgaaatgaaggaacgcatcggaaaaatcaccgtgaagatgaccgctgtgatggtgaccacgctgctgccggcgctggtcatcgtcacggcggggccggcctttcttgccatcttccgctcacttggagccgccgccgcaaaatgaaaaccacccaccttcgcaccagcccgcgccctgcttaccgcttgctggctttggcctgcgcggcggccacgacgctcgccctcaccggctgcgccggcctcaaggaccagtacgccgccagcaccgatgcgcagcagcgcatggccgccgaagccgcggcggacacgaaggccggggcggccgtggacacgcaggcaacctatctcaagctcgtcgagcagatgcagaaggaagacctgtggtttgcatcgctcgcgcacatcgacgctctggaacagcgttggggcgtgtcgcccgaatccacacgcacgcgcgctgaagcgctgcgccagaccgggcaggctgcgcccgccgaagccgcctacaagcgcctgctggccacgccgctggcgagcgcgggctaccgcggactgggcctcctggcaggtatgcgcggcaactatgccgaggcggtccagctgcttgcgcaagcgcagcgccgcaccccgaccgatgcgctgctgctgagcgatctcggctacgcgcacctgggcgccggccagatcgaagaagcgcggctgccgctgatgcaggctctgcagttgcgccccgacagcgcccaggcgcaagccaatctcgcactctatctggaagtgaccaaccagcccgaccgggcggcagcgctgatggatgcccaccgcatgccccagccgacacgcctggccgtgcgcgaagcggcactgcagatgcgcgcatcgggcaagctgcccgcacccgttgttgctgccgcagcggcgggagctcgcgtcgaacctgttctgacgccccttgcgctcaaaccgtcccgatggagcggcgcgggcggcatgagaaccgcgagccagacgaacccttcggcctcggtatctgaagcgccgctttcactgaactcgacctcgcgaggtaccccatgaaccaccagcttgccgagcggatcgcgttgacggccgcactcttcttcgtggcgaccaccgccttggcgcaagccgtgccgccggcaccgcagcctacggaagcgcaggaggccgaggccgaagagttcgaatcaccgccaccgctgctcatgggcgatgcaacgcagagcctgctcgcctggcaacgcagcggagaaatcgcttcgcgcacgccccggcccatcgccggcaacgtggccagccgcagctatgagcgctacatcaagagcttcgagcatccgatcccggagcagctgggctccacggtgacgaagtcgaagggcggcggcggcgcctcttccggaggacggtagtcaaagagccgactctcgccgcgcaaagaaaaccacgatggaaacacgcagccacgcaaagcccggacatgtccaacacggcgtgtacgcgatcgagtttgcgttcgtgttcctgatcgcctttgcgctgctgtacgcggtgatttgctacggtttcttgttgacgatgcgcatgagcctgcagaacgcggcggaagacggtgcccgtgcaggactgcgctatcaaagcagcctggaagccagaaaaaccaaagccaacgacattgccgtagagcgcagcaactggttgcccgcgggcctgaaagcgaaccggaatatcgaggcaagaatttgcctggctggaacggacgactgctcgcaggcgtcgcccccttgcggcccggaatggaacaaccggtgccaggtggtcgtgaccgtcgctgtcagcgggatcgatacgttgtttcccgcgttcccgagttttgcggtccccgaccgaattgcgggccaggccagcatgctgctcgacgggaggtcgttgtgaagtccgtccagctgaaactcgaacggcctgtggctcgccgccagcgaggcgtcgctgccatcgagtttgcgctcgtcttcggtgttctgttcctcggtatctatggcctcgtgacgttctgcggggttctgtacgtccagcaggttatctctcgcgcggccgaagacggcgcaagagccgctcagtcctttcgcagcgacacgccgatcgccgacctgcggacgaatgttcgaacggcggtgtaccggtcgctggcactctcgatgattacgccagcgtccgagggcgccgccccttcgtcaaaagaagactggctccgggacaagatggcgggcacccctcccgaagtgactgtttcgtcgggagaaatcgcggtgaaagtgacttatccctaccgcgccaatccgctgctgccggccgttccgctcaccggaagctggatgcccgagcacctgcttggcaaggccacggccgccagatcctcttcatagacagatgcgaacgatgcgggcattcaatcgaagaacagcacggcggcaaggcgggtcggtggtcatcaccgcgatcatcgcgttgagccttctggtcatcgtgcttgtcggtgttgaactgggctatatgttctttctgaaacgcgagcttcagaagacagccgatcttgctgcgctggcgggagcgcaggccttgctacccgcaagctgcggcgaggcaacaaccgcagcagttgcgaacggcgggcagaacatgccgcaactgatgacgccgatcacagcagcagaagtccaatgcggcaactgggacccgaccctgcgtccagcgccccttcactttggcacacccgagagcgggcagatcctcaatgccgtgcgggtaacactcaccaggaccgcgccaccgttgctgccgaatctgccgggcaatcagtcttccgccatcagcgtcgaagcactcgcggccaagaagcagccactcgcttcactgagtatccgcagcacgatcgcagctattgacacccagcgttcggtcattttgaacgcgctcttcggcggcatgctcggcggttctctcgacgtgtcggtcgccggctggcaaggtctgctcgacaccaacatcaagctgctcgattttctcgatcagctcaagctggatctcaacatcagtgcagccaactacgacgaagtgcttggcaccaatgtgaacgccggcatccttttgcaaagcatgatcacggtcatggaacgcgggggcagcagcgccagtattgcggtgcaaacgctgcagcaacttctggcagcgtcggccgggtcgcccgagccgcttaccgtcggcgaactcctgaacatcgccgcaggcacggatgccgccgggttgcagaccgacctgcagctctttcaactcgttcagggtgtggtgcagctcgcgaatggcaagaacgcacttgcagccgacataccggtcgatgttccggggattgccggcatcaccgccaaggtccgagcgatcgaggcgccgcaggtttcggcgatcggcaatcctttgctgatcgattcgaatctgggtgtgaacgatcccaacaagatttatgtgcggacggcgcagattcgcttgttgctgtcgctgaacttgagcgggttgggaacggcggtttccgacgtaatttcttccgtaacgacggtgctgtcgccgctcatcagttccctggcaagcgtagcgacgctggacattggaaatatcttgtccaacctcatcggcgtgatcgcctgcgcaggctcatcttgtccgataacacaggtcgtctatgtggagccattgcccgaacccattgaaatcagcatcagttccggcaatggagaagctcttgtcacaggccatacgtgcggcacagacgagagcaagacgctgaacgtccaggcctcgaccaacattgcccagctcaacattgggaaagtgtcgaatgcactctcctcctcactacccgccacggcagaggcggtgggaatcttgggaatcggctaccgcgaagccaggtttgactcctgcatcctctcgatttgctccggtccgaaatggaagactgccagtggcaccttcatcagcgacaagcaaaacgccaagaagaatgtcatctctgaatttaggctcgttattaactcgggagtcggaggcagcgcaagcaacgcactgacgtactcggcgcctttggctgttaacttgccagagatcgatgcggcaccttatgacggcaccgggtccgatccttcgttccagccggtcagcgcgcaatcacttgtccagggtttgagtcccgcgctggccgggatacagattcaacattacccgggcgatgccagcggcatgctcggtccccttgtcagcggtatcttgaacctcgtgagtggcctgctcaacaccgtgcagaccatcatcacgaatgcgctctcccctttgctcgaccccgcagtcaacctgcttctggactcgctcggcatcgacctcgcgaaagcagaggtcggggctcgactttcctgcaaccggggtgccgagcttgtctattgatatacgtattcccctgtcatgagcgctccccccaacttcgacgaactcgacctctttgtctgggaaggcaaggccgacatcctcgaccgcattgctcggtgcatggcgagcttcgacgtcgaggtgatccgggccgacggcatgccgcctcctcagcaggagcgcggcacggcgcttcggccttcggtcgcgatcatcagcgtcacggtcattgacggcgggggcctggcacacgcgaccgaactgctgcaaggcatgccggtgatctgggtggccgcggcttctcgcgaccgcgattcacgcacgtacccgcccgagtacctgcacgttcttccctacgacttcacctgtgccgagctgcgcacgatggtcgccaagctggtgcggcagctgcgggcgcgcgacgtggcgccgcaggcgcccgatgtgctggtggcgcactcggaggcgatgaaatcgctgctcgccgaagtgggcgcctttgccgactgcaaccacagtgtgctggtgcgcggcgaaacgggggtgggcaaggaacgcatcgcgcagcagctccatctcggccatcagcactacagcaagggcgcgttcgtggcggtgaactgcggcgcgattcccgacgggctgttcgagtcgctcttcttcggccacacgaagggctcgttcaccggcgccgtgcatgcgcaccgcggctacttcgagcaggcgacgggcggcactctgttcctcgacgagatcggcgatctgccgaagtaccagcaggtcaagctgctgcgcgtgctcgaggacaacgcggtcacgcggctgggcgccacggcgccggttcgcgtcgactttcggctggtggccgccaccaaccgcaacctgcgcgagatggtggcgagcggcgagtttcgcgccgatctgttctatcggctcgcggtgatcgagctgcatgtgcccagcctcgaagatcgcggcgagatcgacaagatcgcaatcttcaaggcgctgctggccaatgtgctgggcgacgaactggaggcgttgggcgaaacgccgcactggctcagcgacgcggtcgcggagacctactttccgggcaacgtgcggcagctgcgcaacctggccgagcgcgtgggcgtgatcgcgcggcaattgcacgcatgggaccagaacctcatccagcgggccattgcgctcacgcgcggcacgccgatgcccactgcaggctcggccgacagaaatgggcacaacggtggcggcaacggcatcgggctcgatggcaacggcgaccgcaagggttggaacggcagcgagcgtaaccgcatcatcgcggcgctggagatcaacgactggaagcgtcaggacaccgcgcagcatctgggcatcagccgcaaggtgctgtgggaaaagatgcgcaagtatcagatcctggacggcgaaccgggcatccccgaggacgcctgagcccaccccggcttactgacggatcgccaggcgatcggctcggcgcagcggcgggttcgatgcggtcgcggtggcgccgcggtcggtcacgggttcgctggcacagcttgtgttgctcgagatgcacagcgcggtgagcaggccgtcttcgctcagcgcggggcggcccggcggtccgaagatgcggtcgatccaggcattgctcgcatcgggatcgatccgcagctcacccgtggtgcgtgcaaggcgcagctcgctgatgcgaaggtcgaacacggcatcgacatagtcgaacagcaggttgtagtagtcgagctgcgcgtcgagcacggccggcagcgtctcgcgaccgaactccatcaggcggcgccggccgcggaaagcctgacccgaggtgctgacggcttccatcagctgccgttcgcgttcgcgtccggacaccgtgcgcgaccatgaggccgacgtgagttccagcaggttgagcttcacgccttcgagcttggcctcctggttggcgacttcggccagcgcggacttcaaccgcagttgccggtcgaaaccgttgccaaagttccagttgagctcgaaggcggcgcgcgtcgggtcctgcggcgacacgccgcgcgggtccttgctcttgacgaccaccgcatccaccgtcgggtagatgctggcttcctgctggtcgaccagggcctgggcccgcgccacgcggcccttggcctcggcgatctcggtgctgcgttcttccgcgcgccgcagggcttcgtcctgcgaggcgatgcgccagaacgcgggcgcagcgagcacgggcagcgaatcggtgttgggcgtgaacttgaaatacgtattgaacttggccagcgcctcgtcgcgctgggcctgaaagtcggactcgcgggcggccacgctggcacggcgcgcggccgccatgttcaggtcgttctcgccggccgcgccaagcgcaacgcggcgtgcttcggctttcgaaagctcggccaccacctcggtggacttgcgcgcgatctgcttcttcaggtcgaagcgctgcacttgcaggtaagcggtcagcgcgtcgagcaccaccttctgcgaagtggtcaccacggcctcgtcgtcggcctggtttcccgcttcggcggcgcgcaccgcggcgctcatggcgccgccgtcgactaggctcacgcgcgcctcggcggtcagcacggtgtagttctcgctcctggcattggccgcgccgctgttgtaggtgccggacgcagtgcccatcttgaagcgtgggtagcgggccttctttgcggcatccacgccaaagctgctggtgttggcggcggcctgcgcggtttgcacttcagggtagtcctgcgagagcgtgacgagtgcctgcttcacgcgctgggcatagctcgcggcaccgatcgagggcgcggagaggcgtcgtgcggccgtcagctgcgccggcacttcctgcagctcctgcgcgattgcgcccggaggaacggcgaagctcgcgcacagtgccgtgcacaggatgccgcggcccactcggcgccggcccgtcaagatgctcgccctcatggttcgcggaaggcttcgcgccgcagcttgagcacaggacgaaggatgtaccagatgaacggatcggtccccaccttcaggtcgacctcggactccatgccggcagtgatgcggttctccggctgtcccacgtaggcctgcccggtgctgatgaggatgcggtagtagggcgccgcattggcaatggccggatcgcggtcggcatcggcggccaccagcgtgaccttgccttcgaccgcgccgtagcgcaggtagtcgtaggccgtgaccttcacgcgcgccgcctggcccacctcgacaaagccgcggtcgttcgggttcaggcgcgcctcgatcatgacctcgtccttgtcgggcaccacttccatgatcgcctcaccaggcttgatgacccagcccgggctgccgctgcgcagccccttgacgatgccgtcggcgggcgccttcacgatcgtgcgcgagcgctgggtgcgtgcgcgcgccaggtcttcgctcaggcttgcgaactggcgctcgacggtcgcgagttcatccgatgcgcggcgccggaaccggccttcggcttcggccatcttggcctgcgcctcagcgatggccgcgctggccgagatggcaccctggcgcgccacggccagctcgcttcgcacgccctcgacctgcctgcgcttctcgagcacctcgacctgcccgaccagtttttcgctcagcagctgttcagagatttcgagttccttctgcatcagcgccagccggtcgttcagacctttcaccttggcctgctgctcaagctgcttgctgcgggcctgctccaggcccgacaccgcgccggccatcacgccgcgctgctcgagcgcgcgcgcttcatacgcgccggcttcgccttcgagcacgctcgcgtcgatgtcggtggcaaagctctcgcgcttgagcgcctggccgcggctctcggccatgagccggacgcgggtggccagcgtcgaggcatggcgtgcgctgagttcttcgaggttgaggccgctgccgccaaggtcgatctcgaccagcgactggccctgcttcacgcggtcgccttccttcaccagcacgttgctgacaatgccgccttccagatgctggatcgacttgacgcggtccgacggaatcacgcggcccggcgccaccaccacggtctccatgggaaagcccaggccgaccacggccagcaccgcgaccacgccgccgatcacccattggcggcgccggccctcgggcgatgcatgcgccgcgcgcttctggtcttcgtcctgcagtatctgcggaagatctgatttcaagtcgcggtccccattgctcttgtcttcaatcgatgggctcactcaagccatggaacggttcgcggcgttgccctgcggcagcgcctcggcgtcgtcgccgccggcagcggaatcgcccagcgccaccaaggccttcttgaccccgaacagcttcggcaccatgaccgccgccgttccctgttcgacgttgccctgccccgtcacgtgatagaccacggtggcggccgagacgatgcgcagcgagtgcgtgaccaccaccacggtgcgcaccttggccaccgcaagcagcgtggcaaggagcgtgcgttcgctctgaaagtcgaggtcgttgctaggctcgtcgagcaccagcaccgagggcttgcgcaggaagctcatggccagcgcgagcttgcgccgctcgcccaccgagaaaccggtgccgccttctccgaccaccgtgcggtagccgtcgggcaggcgcgagatgaagtcgtgcgcgcccgaaagcctgcaggccgccaccacctgctcgtcgctctggcccggcgccgtgcggcgcatggtgtcgatcagcggcccgccaaaccagtagacctcctgcgacagatagctgatccagcgcgagagctcttcgcgcccgaattgcgaaaggtcgtattcgccgatgctgatgacgccgcgcgtgggcgcgtacaggcccgagatcagcttgaccagcgtcgacttgccggcgccgttgcgcccgacgatcacgtgaaggccgcccggcccgatgtcgagatcgacgttctcgagcaccggcttctgcgcgccttccgtgaagctgaagctcacgtctttcagcatgacgcgaccgagcggttgcggcagcgtcatgcccgagggcggcttttcgaccggctcggagagcactttttcgagccgctttgccgcttccttcgcggcggccagcgagcgccagctcgacaccagcccggccaccggctgcagtgccttgagcgccagcatgttcgaggcgaccaggccgccgaccgtcatccattgctccatgacagacaccgcgcccacggtcaccacgatgaccgagaacaccgtcagcagcaccgtggtgccgtcgcgcgcggattcgatctggccgttcttgctgaagctttcgcccagccagtcgttataggtctggcgccacatctcgatggtcgggccgtcgtttgcctgcgtcttgagcgtctcgcgcgcgttgcagatttccgaggtcatgcggtcgagcccgcggccgcgctgcacttcctcgacgcggccggtgcgcacctcgtcggcccaccaccaggccaaaaaagccatgatggcaaggaacagcgccaccaccggcagcacgggcaaggccacgatgccgatcaccaccagcgcgaagatcgccatcggcaggtcgaagatcgattgcgcgaggccgcctgtgacggtgccgcgcaccgaggccacgtcgcgaaagtactggtgccagatcgaggccggacgcgcttcgagcgcgcgcagcgggcggttcagcatcgaatggagcagcgcccccgaaacaccgtggtcgatgatggcgcccgcgttgcgcagcaggcgcgagcgccgcgtgcgcatccagaactcgatgcacagaaaaaacaggatgccgctcaccagcgcggccagcgtcgagacgccgctgcgcgacagcacgcggtcgtacacctgcagcagaaagatcgaaggcagcaggccgaacaggctgatgggcagcgaacgccatgccgcgctcttcaccagcgggtaggcagcccggaacgcggtgtgcagcgcacccgcgtacggactggcacctggctcctcgggcagttcggccaccagctgactgggcaagagaaacttgatcatgggaagaggccgatccgttcggcaatgacgcctgcgtcattatcaactgttacccaactgttactaggcaaaatgtcacgttacgcacctccgcatcgcggtgttcgccccggcttctgcgggactgtctggccctcgcgcgcgccgggtcgcgcggtggcttccgcaggtgcgcaaccggacgcagttctcgcgtgcggcgcggcggcctcgtcctgcggccagcccttggtcaacaccagggcgacgttggcgcacagcagcatgcaaagcagccatgcgcaaagcagttgcagccagcccagccaccagcggcccgccggcacggccttgggttcgaaggacaaggacaggggcgcgttcaatttcatggcaatgctttcaatacacgggccagccgggacaggccgacgccggcggaactcttggccagcacccagtcgcccggctgcagcagccctccgagcgcggtcgacaggtcggatacatcgacgaaccagtgcgaccggaccttggtgcggatgcgcgcgtgcagcgcacgcatgagcgggccgcacagcagcacgcggtcgggctgcgatgcgagcagttccggctcaaggtcgaggtggtgccgctgcgcggccggaccgagctcctgcatgtcgccaagaatcgccacgcgccgcgccggctcgcagggcgcctgcgacaacagttcaagcgcggcacgcatcgagctcgggttggcgtcgtaggtctcgtcgatcagcttgaagctgccgccgccgatgtggatggtgtgcagcgcgccacgcccgcccggcggctcgaagcgcgcgaagggctccaccgcggcagacagcttcaggcgcattgcctgcaacgcggccagcgcggccacggcgctggcgcccatgtgccgccccggcgcattgaggcgaagctggaatggctcgccgagcaccagggcctgcacttcgccatgatcgaacgcgagcagccgcacatcggcgtccctgtgctcgccataggtcaggatctggagctgctgcgccatggcggcctcggcaaaggccgcaaactcgggaaggtcgcggttcagaacggcgctgtcgcccggcgccatgtcctcgaagatgcggctgtcctggcgcgcggcggcctccgaggggccgcgatgtttctgcgaagcggatgaaagccccgtcaccaccatcaccatcggccgcaccagttgcgtcgacgcgaggatgtgcggcgagcccatctccaacacccagtaggccgcgtgccgcggcatgcaggtcaggttccaggcaaggcccgagggaaggctgacgttgccctcgggccgtccgacttcgccccacacggccagggtctcggccagcatcgcggccacggtgctgctgccggcgccactgcccagcacgccgcagacacgcccgccaaactcggtgcgcgcatgcgcgcccagtgccagcacggcctgctgcacgttggcaacctggagcacgggcacccgcttgtccagatgcggtgcggcatcggcgcacagcacggcggccgcgggctgcaacacgcccttgagcgccacggcggccagcggcgccttggcgggccgcgtctggtgctcgaacaccacccgccctttgcgcaggaaggagcgttgcgcgacgccgccggcgcgccagccgtcgtcgggcctgaccacccattcgccgccggtcacgcgcgccatttcgctcgcggtccagacagcgccgtcgtctttcacgctgccggcaccgggcaaggcccgccgctccagcagatagcggtggtaggccacgaagccggacacatactgggccacgtcgtcgatgcgcacgcggaacgcgtgatgccggatgaagaacgcgccggcgatggtggatggccgcctgaagtacatcgccatctcgggccagaagaagccgttctgcaggtagtgggcgcggtattcgagcgcgcggtagaacttctcggtgtcgagctcgtcgagcaggtgccgcatcgcgggcatggcctcgagccgctggagcatctgctgtgccgccagcatgagttcgagcagcgtcggaaaggtggtcttgcggtcgagcacgaagtccaggtacccggcaacgttctgcaggccgaagcgaaagtacttttcctgcgggctccagcgcgtgagttcgttgacgcagcagctcagccaatggtcgtgcacctgccagtgctggctcgcaatgaaatggtcgaaggccttctcgaccagcgccagccatctggcatcgcgcgtgaggtcgtacaggcgcatgaggccgtaggccgcctggccgtcgtggcagacagcgtgcgaggcggcctgcttcagctgcaggtcggcggcatgaagcacgtggttgaaacggcccgtggccgtgtcctgcagccatgcgatgcccagcgccaggttttccagcaacggcaaccagtcgcgtgtgcccatcgcctcgcaatacttcaccagcgcgagcacgcaggcggcattgccgcccagcttgatctcttcgccggtatcgatgaggaaggcgagctgggtgccgtccgcgagcctgtagtggcgtatgaacgaattcgcgaggtggtcgagcgcgtggtcgatggccgcacgcagcttgtcgtcccgcgtgagctcccacgcctcgatcatggtgtggagcgcgcccgcgtggcgcgacgcgtcataggtgggaatgcggcggtcgaagcacggaaagtagccgtacgcaaacaacccgtcgccctgcacctggcgcgcaagataagccgagccgctgcgcacgagttcgagcaccgactgcgaattgagcgccggcgcctggcgccggcccgcatcgagccccgtgccgacgagcttgtgcacgacgccgtccgattggcagaagacacctgcggtcgcaagcaggtagaccggctggtccgccggcaagtcgagccggggcgcacgtgcgaagcgcgcctggccgtagacctcgaagttgcgcgcgttgaccacggcgtgcgcaatggtcgagtcgccgcacagcatcgcgttggcgttgagttcctgctcggtgaacgcggtctcgaagctcttgtcgaaagccaggccaaggcgaaagtagttgcgcttgacggcggcaagctgcgccttgaactgcgcccaatccatcgggcttgcgccctcgacccagtcgatgcgcagccatggcgagaccaggccgtattcgcgcacccggcgctccacggcctcggcgccttcgcgccaggccgtttcgaattcggccgcacgcgcgtgcaccacgtgcgcgcgctgcgatccatcgctcaccgagaagaaaagcgtgaaggccggatatggcgcaggaagcgccgcacacaccgagaccaggcgctcgtggcaggcctggagctggtcggagaaggacatcattcggccccgatcgaatacgggagcccggccgcggccgtcatctgctctcgctttgacgtcgcggaccggaagctcccctcgaaggcatcgcggttctccggatcagcggtagctgaattcggctctgcgattgagctgatagccctcctcggtgggttggggggatgcgggtttttccatgccccagctgacggcctcgatgcgctcgcccggcacgccaagctgcgtgagcgcacgctgcaccgattcggcacggcgttgggccagcgcgaggttgtattcgcggccaccgcgcgagtcggtgtggccttcgatcatcaccttgctcgcgggacggttccggagaatgttcgcgtgcgcttccaccacgttgcggtcctgcggcctgatgtcgtacttgtcgaaattgaagtacacgatcttcggcgcgtcgacgttgtcggccggcggcgcgggcggacgcggctccaccttcgcgaccggagtgcccttgttcgagtagtagtaggtcgcgtcttcgcgcccgctcttgatcgccgttccgcaggcggcaaggcttgccgcgagcgcgacgacggtcaatatccgatagctgctgctgttgttcatatccaaatcctttcaggggacaggccgacaccggcctgtccctggtgctgccgttcttcttctcctctgctgccctttttgttgcttagcccagcaggccgtgcaggatgttcgtcacgggggtgagaacgttgccggtccctgcggcctgatcgaccaggctcgtgatcggggtcaccacgtcggtcacgatcggcgccgcttccgccacggtgtcgagcacgccgtgaaccgtttcaatcgccggagtgagcgtcggggttgcgccagccaggatgtcggtcaccggttcggccacctcggacacggcggagaccacgggttccagaacctcgccgacagtgcctgcggtgtcgagcaccggatccaggatgttggccaccgggttgctgccccccagggcgccgccgagcaagccgtcgctgccaagcaggctgccgaccaggccgtcgtcaccgagaaggtcaccgccgaggaggtcaccgccaagcaggtcgccacccaggagatcgccgccgagcaggttgccaacgaggccatcctcgccgagcacgccacccagcaggtcaccgccaagcaggtcaccacccaggagatcgccaccgagcaggttgccaacgaggccgtcttcaccaagcacgccgcccagcaggtcaccgccaagcaagtcgccacccaggagatcgccgccgagcaggttgccgacgaggccatcttcgccaagcacgccgccaagcaggtcgccacccaggagatcgccaccgagcagattgccaacgaggccatcctcaccaagcacgccgcccagcaggtcaccgccaagcaagtcaccgcccaggagatcgccaccgagcagattgccaacgaggccatcctcaccaagcacgccgcccagcaggtcaccgccaagcaagtcgccacccaggagatcgccgccgagcaggccaccgacaacgccgtcttcgcccaccaggccaccaagcaacccgtcgccgccgagcaccccgcccaacacgccgccgtcacccagcaggttgtcgaccagaccgtcgtcgccgagaacaccgccgaggaggccgtcgctggcaaggaggctgccgaccgcgccgtcgctgccaagcaagccgtctgcgccgagcaggccgccggcgaggccttcgtcgccgagcacaccgcccagcaagccttcgtcgcccagcacaccgccggtcagaccaccgagcaggccgtcttcgccgccgagcaggccacccagcgggccgtcttcaatcaggccgcccaccacgccattcgcgccgagcaggttgtccaccacgccgtcctggcccagcaagctgcccgtgaggccttcgctgcccagcaggccggcggccgtgccttctccgccaagcaggccaccgaccaggccgtcgccgacgagcaggccgcccaccgggctgtcgccgctgagcaagccgcccagcaggccgtcttcacccaacgggccgccgagcaggccgcccagggcgccgccatcgcccagcaggccgccgacgaggccttcgtcgctcagcacgttgccaagcaggccgccgatggcgctgtcttcgccgatgaggttgcccacggcgccgtcgtcggcgaggagcccgcccaccaggccgtcttcgctcatcagggtactcacaaggctgtcctcgccgagcacgccttcgaccaggtcgccgaccacgccgccatcgccgacgaggccgtcaacaacgccgtccacaccgagcgcagtggtcacgccgctcaggatgccgtcgtcgcctacgaggttgtcgatgccgttctgaagcgcgtccgtgaggtggtcgacctggccgaccagcgcgccggtagcaccgtcgcccaggagggcgtcgacgatcgggctcgcggcgccgcccacgctgtcgacgatggtttcggcagcatcgtccaccggatcgaactggttcggatcgtcccgcgtgaaatgttcgccgaggaccggggagaccaggtcatcgaccaggtcggtggtgctgtcgacgacgcccggcaccggggtgagcgaaccgccgaggcccaggttgtcgtcggtcgagcccaccacgccgcccgtgaggacatcgcccggatcgagcaggtgatcgccgtctgcgtctgcgtctgcatcggcatcagcatcagcatcagcatcagcgtcagcgtcagcgtcagcgtcagcgtcagcgtcggcgtcggcgtcggcgtcggcgtcggcatcagcgtcagcgtcagcatcagcgtcagcgtcagcgtcagcatcggcatcagcgtcagcgtcagcatcggcatcggcatcggcatcggcatcggcatcggcatcggcatcagcgtcagcatcggcatcggcatcagcgtcagcatcggcatcggcatcggcatcggcatcggcatcagcatcagcgtcagcatcggcgtcagcgtcagcgtcagcatcggcgtcagcgtcagcgtcagcgtcagcatcggcgtcagcgtcagcgtcagcgtcagcatcggcgtcagcgtcagcgtcagcgtcagcgtcagcatcggcatccccgtcatcaccactgccaagaaggaacggcaccgttccaccgtcgccaccaccgccgccgcccagggcagcgccaagcccggcggcacccagtgcgccgagcgcgaattcgcccaggccgaggccgctgccggccgcgaccttcttggtgacggccagtgcggctgcctcggcatcgctgtccagtggggtcacttgcaggtcgcccgaggcgacgtcgacgttgacttgttcaaggccgccgggcagcttggtcgaaccgatggtggcatcggtgccgccggtgaagacgccggccagcggcgccttgttgctggccgagccgggaaagagaacgttggcctgtccgccttcgggaacgatcacgcggtcgcccgccatcaatgtctggttgccgtccacaggaatgcggacaccgtcccgcatcaccgccacgcccggcgtagcattggacaatgtgcctacgccggcgggcgccgtcgtggcaaccgcggcagcaggtgccggcgagccgagcatggtgggcgcccccagcggtgtgctggtggcttgagcgatgaccacaggagcgacgccactggcggcaaatccttcggtcgatggggtcggtgcttgtggtgcgttcatgacagcctctgtgacaaaagatgcatgtacaggggcaactagcgtgccgattcgttaccgcgcttcgatatcggcccagccaatgacgcaagctattgattcatatagatatttatttaaaacggggcgtgcttgccggcgctgaaaaagcctccggaacgagtcttttggcacttcgttacgtaacgatgtaacgtctcgctaccggaacatcggcctccatttctctcttcttcatacagatatgttcaacccctcccaggaagacgtgcgccgcttcttttgcgatgtgtacgccaagcaccgccagggcttgccgatggaagcgctcgagacaattgccgcgggatggatcgacgagcaccccgaataccacgacgacctggccgatgccgatgcggcggtggcacgcgtgtacgacggctcgaacggccgggagaatccgtttctccacctgtccatgcatctgtcgatcagcgagcaatgctcgatcgaccagccgcgcggcatccgccaggccgtggagctgctggcggcccgccgcggttcgctgctcgacgcgcatcacgaggccatggagtgcctgggccagatgatgtgggagagccagcgcgccggccggccgcccgacggcaacggctacgtggcctgcgtgcagcgacgggcaacaaaagactaggcgcatccgcagggctggatcgctactcctgcggctttctcctgggctgcgaaggcggcgcgccctgctgcttggcaccttcgcggagcagcgcggccatggccacacgcaaggccgagggctctgcatcgctgcgcagcagcaggcctacgggttcgtcggtgccggcggtttcgatgcgcagccggaccaggcgttcgtccgccagttcgccgcgggcggcgccaagcggcgtgatccagaccgcgtcggacaccgcgagcaggccgcgcgccaccgccacgtcgagcgtctgcagcgcgttggccggaagcaccaggccgcgcgccgacaaaaagctttccgtgttgtggcgcgggatggtgccctcgccgtacaccaccagcggatagtcgagcaccgcctgcaccgacaccgttcgggtggaccgggccaccagcggatggccggcgcgcacggcaaacaccagcggctcggtgtagagcaactcgaagctcaggccgcccatgagccgcggatcgctgatgcggccgaccaccatgtcgagctctccggcgcgcagctcatcgagcagcaccgggttggccgcgctcttcaccaccacctgcaccgaaggccaatgctcgcgaaagcgcgcgagcgccatggggagcagggccggccccacgctcggcagcgcgccgatgcgcagccgctcgatgcgctggcccgaggccggcgccaccgcctctgcgctggcgtcgagcgcctcgagcacgcgcagggcatgggccagcagttgctcgccggccggcgcgagcccctgcacgccgcgccgcccggccttgctgcgttcgaccaagcgcgcgccgacgatggcctcgagctcggagagggtcttggagaccgccggctggctcagcgaaagccgctcggcggcgcgcgccagatggcgctcctgcgccaccgcgaccaggcagcgcaggtgccgtagctgcacgctgcgcacgaagtcctggcgaatatcggcggaggttttcaattacctttggttattcaaaacagatcaatcttcaatttacatcatcggaccggacttctaaagttcagcttccaaaactcgattcgttccacgacaggagacaacgcatgttggacaagatcaaggcaccccccgccgtcctcaccccgcgcgactggcaagcccacccttcttacgtctatcccggctacaagtcgaccgtgaagcgcgggccgcagaagcccctggttccgctgaaggcctcgctgggtgaattgcagcagccggtctacggccacgacagcatcggcgcgctagaccacgacttgacgcgcaacgcacgcaagaacggcgagccgctgggcgaacgcatgatcctcaccggccaggtgctcgacgagcgccgccgcccggtggccaacacgctggtggagctctggcaggccaacgctgcaggccgctacgtgcacaaggtcgaccagcacgacgcgccgctcgaccccaactttctgggcgcaggccgctgcctgaccgacagcgagggccgctaccgcttcctcaccatcaagcccggcgcctacccgtggggcaaccacccgaacgcctggcgtccgcagcacattcacctgtcgcttttcggccagagctttgcgagccgcctggtcacgcagatgtatttccccggcgatccgctgatgcagtacgaccccatgatcaccggcacgcccgagcgctaccgcaaccggctgatcgccgatttcagcctcgacatcaccgaggaaggctacgcactgggctaccagttcgacatcgtgctgcgcggcgccgacgaaacgccgttcgagaaccgttgaaaaaatgaaactctcccccaagctccgcgcacttcgtgtcgcttcgccaaccccctcgccgggggcaacaccagcggcccggcaaagccggttccgcggtgttcctggccttggctgcgttggtgcgggcgtcgcgcgcggcgcggtcgcttgccggaaaacttaaaggaactcccatgtcactgatgaccgcacaggaagccgacttcggccagaccccctcccagacggtgggcccctacttcgcctacggccttacggccacgcaatacggctacgacttcaaccagcctttcgacgcggtcgtggcgctggacgccgccgcgggcgagcgcatccggctcgagggccgcgtgatcgacggcgatggcaatcccatcggcgatgcgctggtcgaaatcagccaggccgacggcgaaagccgctatccgcagacgccggccgaggcccgcgagatcggctttcgcgccttcggacgcgcgggcacgggcaccgatccgcagaaccgcttcgtcttccacaccgtgaagccgggcgcagaaacgccgggcgaagccccgcatatcaacgtgatcgtgctgatgcgcgggctcttgctgcatgcgttcacgcgcgtgtatttcagcgacgaggccgaagccaacgccaaggacgccgtgctggccagcgtgccggccgagcgccgccacacgctggttgccgagcgcgtggaacaaggcggcgcggtgagctaccgcttcgacatccgcatgcagggcacggacgaaacggtgttcttcgacgtctgaccggcatcgcccggacgcaaaaaagcccgcttcacgcgggctttttcatgggagcggggaatggcgctgcgcgggctgcgcctaccgccgtttgtgtttgttactgcgcgccgtggtggaggcgcgagtccggcaccgtcttgagttcgccgggcagcgagctgatgtagctggcgagcgtcttgagttcggcggtggtgaacttcttgggctcgacctgctgcgccatgaccgcattggaacggcccaggtgcgggttgttcttgacacggtacgacttgagcgccacgaagaggtagtcggcatgctggccggccagcttgggcaccgtgccgtcgttcggcgtgttgaagttggcgccgtggcacttggtgcagctgttgtccttgtcgcgcgccaccagggcctgcacgttctcaggcatgggcttggccagcgcggccggcggcgcctcgccttccttctggcccagttggctgtaataggcggccaggttggcgatgtcctcttccttgagggtgtcggcaatggcgcgcatggtggggtgcttgcggtcgccgttcttgtaggcggtgagtgcggcagcgatgtagctggcgctctggccggcaatcatcggcaccttgtggatttccggaaagctggcctggtagccgatgatgccgtggcagcccacgcacatcgcgacctgcttggcgcccttctgggcatcgcccttggcttgctgggcttgcgccgagaccgtcacgcaagcgacagcgaaggcaaacatcgtggtcaacaacttgttcattttgcgcgcacaatctcgtggagatacagtttttcgaatcaacattcgattatatgcaagggtcctccgggaacccccgccggccgcccaaaggccgcgcaaagcgaatcgagtgtgttcttttctccacccggcctcctccacctgcttgcgttccactcatgaaattcaagggctcagacaactacgtcgccactcaggacctgatgctggcggtcaatgccgccatcacgctcaaacgcccgctgctcgtcaagggcgaacctggcacgggcaagaccatgctggcggaagaagtggccgggtcgctcggcctgccgctcctgcagtggcacatcaagtcgaccaccaaggcgcagcagggcctgtatgaatacgacgccgtgagccgcctgcgcgactcgcagctcaaggacgtggacggcggcgagcgcgtcagggacatccagaactacatcgtcaagggcgtgctctggcaggccttcacggccgaccagccggtggcgctgctcatcgacgagatcgacaaggccgacatcgagtttccgaacgacctgctgcgcgaaatcgaccgcatggagttctattgctacgagacgcgtgagcttatccgcgccaagcaccggccggtggtgttcatcacctccaacaacgagaaggaactgcccgacgccttcctgcgccgctgcttcttccactacatcaagtttcccgatgccgagacgatgaagaacatcgtggcagtgcacttccccggcctgaagcaggagctgctcacgtccgcaatgaagaccttctacgacgtgcgcaacctgcccggcctgaagaagaagccttccacctccgagctgctcgactggctcaagctgctggtggccgaagacattcccattgaggccctgcagagcaaggacgacaaggttgccgtgccgccgctggtgggcgcgctgctcaagaacgaacaagacgtgacgctgttcgagaagctcgtcttcatgcagcggaacaaccgatgagtccccgcccggccgctccgaaggggactcgcaccgcagtgcgaagcacggaggtttccttgtgagccagccacaagcgccgcatccggtcggccaactgctcaaactgggcgtggcgcaggccgtgctgttcgtggccggtgcgctgcttggccgctggatcgggctccagctggggctggatgccttcgggcccaacggttacggcaaccgcgagatcttcggcatcctgctgatcggcgtgggcggtggcggcggcgtgcaattggcccgggcctggtacgaccgcaagtacggcaagccaagagactgaaaaacaatcgcgagaggtgttgaaaagatggcgttcgtcgaacctgtcacgctgaaggcccgcgacctggcgctggtgccgctttcgctcgatcatgaagagggccttcgcgctgccgcggccgacggcgaactctggaagctgcgcatcacctcggtgccggagccgcacgaaacccgcgcctacatcgaaaccgccctgcagggccgcgaagccggccaccgctttgcgtttgccgtgaccgaggccgaaagcggcaccgtgctcggcagcaccagctttcacgacatcctgccggcggtcgggcgcgtggaggtcggctacacctggtatgccaaacggtgccagcgcacgcacgtcaacaccacctgcaagctgctcatgctgacgcacgccttcgataccctcggctgcaacgtggtgggctggcgcaccgacaatttcaacttcgcttcgcagcaagccatcgagcggctcggcgcaagaaaagacggcgtcattcgcggccatgccatgcgccgcgacggcaccatccgcgacaccgtgatgtacagcctgcgctcgggcgagtggcccgaggtcaaggcccagttgctctacctgctcgacaagccgcgaagctgaagagaagccctaggaaagcccgaccatgctgatcgatttcttctacacgctgcgctcggccaagctgccggtctcggtcaaggaatacctcacgctgctcgaggcgctgcaggccgacgtggtggggcccaactccgacggcgccttcggcctggacgacttctactatctctcgcgcaccgcgctggtcaaggacgagaagcactacgacaagttcgaccgcgcctttgccgcctacttcaagggcgtggagatgctggccgacttcaccaaggaagtgccgctcgactggctgcgcaagacgctggagcgcgagttcacggccgaagaaaaagccaagatcgagaagatgggctgggacgagctcatggaaacgctcaagaagcgcttcgaggaacagaaggaacgccacgagggcggcagcaagtggatcggcaccggcggcacctcgcccttcggccacggcggctacaacccgcagggcgtgcgcatcggcggcgctggcaagaacaagagcgccgtgaaggtgtgggaccagcgcgcctacaaggactacgacgacagccaggagctgggcacgcgcaacatcaaggtggcgctgcggcggctgcgcaagtttgcgcgcgaaggccacgaagaagagctggacctggacgacaccatccactcgaccgcggccaatgccggctacctcgacatcaagatgcggcccgagcgccacaacaacgtcaaggtgctgctgctgatggacgtgggcggcaccatggacgagcacatccagcgcgtggaagaactgttctcggccgtgaagaccgagttcaagcacctggagttctattacttccacaactgcgtgtacgacttcatgtggaagaacaacaagcgccgcttctccgagaagttcgcgacctgggacatcctgcgcaagtacaacaaggactacaagctcatcttcgtcggcgacgcgaccatgagcccctacgagatcctgcagcccggcggcagcgtggaatacaacaatgaggaagccggcgccgagtgggtccagcgcctcacgcacgcctttcccaagttcgcctggatcaatcccgagccgcagggcgtgtggcaataccgccagagcattgccgtgatgcagcaactcatgtccaaccgcatgtacccgctcacgctgcggggcctcgaagacgcgatgcgaatgctttcgaagtaaggcggcgtgcggcatgcgcctctctgtttccggatgcttccggagccggcgcgccttgctgtcaaaatccgcccatgttcagggtggtcccagtctttgcgccggcgtggttgccggctttgctttttttcggcgtcctgcttctgcaaggatgcagcctgctgccgaaaaaagaagccgccacggacaccaccgccccggccctggtgcgcagcggcgacaccgccgccgatgaaaccggcaaggacggcgacaggggcccacggcgcgctgcattcaccgtcgacgtgcgcgggcccgacaacgtgcgcgaatacctcgcgctgcatctggacatccagcgctaccgcgagctcgacgacctgggcgccaccgagatctcgcggctcatggtggcggcggaaaccaacgcccgcgagctgctcggcacgctgggctacttcacgcccacgctgacactcgaactcaacgaaacaccggccagcaccaaggccccgcgcgagatcgtcatcacggtggaacccggcgagctcacccgcgtgagcaacgtgcagctcagcttcggcggcgcaattgcagacgaccccactgccgaggcccagcgcgattcgatccgcaccgcctgggcgctgcggcccggcctgcccttcacgcagcagggctgggacaacgccaagaccaccgccttgcgcagcctcacggccaagcgctttcccaccggcagcatcgaggtgagccgcgccgaggtcgatgccgaccggcaggaggcccggctcagcgccacctatcagtcgggccccgcctaccgcttcggtccgctggtactgcgcggcaccgatcgctacgacgccgacggcgcgcgccgcatcgcgcagctccccaccggcaccgactacgaccagcagaagctgctcgatgcccagcagcgcctggccagcagcggctactacgactcggtgtttctcacgctcgacaccgagagcggcacgccgctggcggcgcccgtgatcgcccagctgcgcgaagccccgatgcagaaggtggtgctgggcgccggcttcaccaccgacagcgggccgcgcctgtccgtcgaccacattcacaaccggctgccgctgctcggctggcgcgccgtctcgcgcctgtcggtcgacagcgacgtcaagtcgctctcgaccgaatggaatgccattcccgacgatcggggatggcgctggttcgcgggcgccgggctcaagagcgaaacctcgggcagctacgtggtcgacagcggccgcgtgcgcagcggccgcagcaagtcgagcggtcacatcgaccgcagctacttcctgcaatacgactacgcgcagaaccgcggcaccaacgccccgccctcggcttccgcggtcacggccaactggggctggaccggccgctatttcgacgacaacgcggtgcccacgcgcggcttcggcctcgcgctcgagctggccgcgggctatacgctgaccggcgagcagttgcccttcacgcgcacctatgcacgctggctcggcgtgctgccggtgggcttcgcacaggaccgggacgccgccacgctggcgcgccgcagccgcctccagctgcgggccgaagccggcgcggtgtccgccaaggacagcgcgcagatcccctccacgctgatgttcctgaccggcggggacacgacggtgcgcggctacagctaccgccagatcggcaccgtgcgcgacgacggccagatcgtggcgggccgctacctcggcgtcgtgagcgtcgaatggcagcggcccttcgtctacaaagacaagctcaccgagtgggagagcgtggtgttcgtcgacgccggcgccgtggccgacaagcccggcgaactcaagcccaaggtcggtgtcggcgtgggtgcgcgctggcgcagcccggtggggccggtacaggccgatcttgcctatggcgtggacacgaagaagttccgccttcacttccgcctcggcttcaccttctgactccatcgatgcagacagacgcccaactccagtcccacaaagccgctccgcgcgcacggcgttcgcgcacgcgccgcgcgctgcgtgcgctgggctggacggtcgggggcctgctggccctggtgctggttttgggcgcgggcgcatggtggtggctcggctccaaccagtctctggcctttgcgctggccagggtcgcgctctacctgcccgccggccattcgctcgaaagccgcgaagtcacgggctcgctgcgcacgggcgggcgcatcggctggctgcgctggcaaagcgagaaactggccgtcgaggtgcacaacgccgacatcggctggcagcttgcgccgttgttccagcgcaagctgcaactcggcgaggtgcatgcggcgcaactgctcatcgagcgccgcggcccgccgagcgacacgcccaccgagccgctcgaacaactcgcgctgcccatcgaggtcgatctgccgttccgcatcgacgaagtgcgctgggccggaccgccggcgctgcaggcgaatcagctcgcgggcagctaccgctacaccgccgcgcaccatcggctggaggtcaagggcgtcgacattgccgaaggccactacagcgcgcgtgtgaacttgcaaggccccgcgccgatggcgctggacgccacgctgaacggccgcgtgaaggcaccgctggccgaaggccgcagcatcgacgtgctggccgaagccgcgatcaagggcaagctcgcaggcaccgatgcgcggctgcagatagccgccgagctgaagccggtcgagcccgacgccgaagcgcccatggaagccaagctgcaagccaatgtcgcgccctggctgccgcagcccgtcatcgatgcgaaggccgaccttcgcaacgtcgatgcggccacgctctggcccggcgctccgaagacgcgcctgaccggcacggtcgaactgcagcctgatgcggctaccggccccgcctcctggcaggcctcggccagcatccgcaacgcggtgcccgggccgtgggacaagggcgcactgccgctcgaagaggtcgaggcgcgcgtgggcttcgacggcacgaactggacgattcccgaagccatgctgcgcgcaggcggcggccgcatcgaagcccagggccgctggagccccgcgcccgcaccctggcaggtgcgcgccaacgtgcgcggcgtgcgggccggcctgctgcacagcgagctttcgggcgcgccgatcagcggcacggccaccgcgcagcagcgcgaagacaccatcggcttcgaactggcgctgcgcgccggaggcggtgccggcagcagggccgtgcccggcttcggcctcgaccgcgtgctggcccagggccagtggaaaaaccaggtgctggacctgcgcaccctgcgcctggaggccgaaggcgccgccattcagggcaggctgcaggtgcgcgtggccgagcaggccgcgagcggcaagctcgacctggcgctgccgggcggcagcgcgcaactcgaaggccgcatcgcaccagcgcaagggggcggcgacatcaaggcgcgcatcgacgatgccgacgccgtgcagcgctggatcgagggcctgcccgagctgtcgaaggtgttcgcgggcaagagcgccaagggttccgcgcggctcgacgccacttggcagggcggctggcagaccattcagcgccggctcgagaaccccactgcaccggcccagcgcggcatcacggagcccagcctgaaggcatcgctcggcgtaccgcagctggagctgcgcatgccgcccaccaatggaaacggcaatgcagcggccgccaccacggtgcatttgaaagagctgcacgcggaactcgccggcagcctggcccaggccacgctcgcgctgcgaggcgaagccaccaccggcacgcagaagctcacggtcgatgcacgcgcgagcggcggcctcgcgggcgccaaccattggcgcgccgcgctcgccagcttgcgcctgcaggcccaggacagcgcgcgggccgccgcggctgccgcgccctggacactggagctcggccgcgaagtcaccgccaccatcaagaccagcggaagcggcgccgcgagccgcctcgatctcgaagcctccgcggccaccgccacgctgcgcggaccggcgcccggtaccgttcgcatcgaatggcagccgctgcgcttcgcccgcagcggcgtggcgcccaaccaggcgtttcgcgtgcagtcgaaaggcaagctgcagggccttccgatggcatgggccgaggctttcggcgccagcaccaccttcaatgaactgggcgtgagcggcgacctgatgttcgacggcgactgggacatcgatgccggcgacacgctgcgcgcccatgcgcggctcgcgcgccagagtggcgacatccgcgtgcaggccggcgaggccgcgctggtcacgcgcatcacgagccgcggcaccggcacggccagcgagcgcacgatgaactccgccaccgcggtcggggcggtcgcgcccaacacgccagccggcttgcgccaggccgaactgcggctcgatgcgcaaggcgacgcggtgcgcgccacgctggcctgggacagcgaacgcgcgggcaagatcgacgcagagctcaacacgcgcatgcagcagcgcgcggagggctggcagtgggcggccgacgcgccgctggccggcaacatcaaggccacgctgccgaacctcggcgtgtggtcgatgctcgcgccgcccggctggcgcattgcaggcacgctggatgccgatgccgcgctctcgggcaaccgcaccacgccgcgctggaacggcacgctgggcgccgacaagctcgcgctgcgcgcgcccgtcgaagggctggacctgcgcgatggccgcctgcgcgccacgctcaccggcacgcgcatcgacatcaccgatttcacgctcaagggcggcgccggcagcaacgtgcgcatcgcgggccagagcggcaaccgcagcaccgcggccagccaggccggcatcgatggcggctcgctctcggcgcgcggcgacatcggctggggcgcggccggcgcgtcgggatcgggcattcgaatggcgctgcaggccgatctgcgcgcgctgcgcgtgctggtgcgcaccgaccgccaggtcacgctctcgggcaacctgcaagcccggctcgacggcggccagttcaacgtgcgcggcaagctcaagaccgaccgcgctgtgatcatcctgcccgacgaaaccgcgccgagcctgggcaccgacgtggtcgtgcgctcggccgccaaggaccgcgaggcggccgagcaggcacagcgcgacgccgcgagccacgaagcgcgggccgcccggccggaaaccgcgaagccgcccgacatcgtggtgaacttcaacctcggcgacgacttcgcggtgcaggggcgcggcatcaccacgcggctcgagggcgacctcgagatccggagcaccaagctcaatgcgccgccgcgcatcaccggcgaagtcaagaccgtgaagggccagtaccgcgcctatggccagcagctcgacgtggaaaccggcctggcccgcttcaacggaccgttcgacaatcccgcactcgacatcctcgcgatacggcccaacatctcgcagcgtgccggtgtgcagatcacaggcaccgcgcagtcgccgcgcgtcaagctttactcggagcccgcgctgtccgatgcggagacgctctcgtgggtggtgctgggccgtgcctcggccaccagcggcggcgaatcggcgctgctgcagcaggcggcgctcgcgctgatcggccatgtcagcaaggccgggagcggcggcagcctggcgagccgcttcgggctcgacgagctcggcttcaagggccccggcaatggcggcgatctgcgcgagtcggccgtgacactcggcaagcggctgtcgaaggatttctacctcacctacgaacgcagcgtgggcggcaccttcggcacgatcttcatcttctacgatctgacgcaacggctcacgctgcgcgggcaggccggacagaccagcgggctcgacctcatctacacattgaagtacgactgaggtccgggtctgccgccttgaccgcggaaattcacgggataagaatcgtcgacgcccttctaacaaggaacgacgatgcacgatgatggagacaagggcgagtgttccccactggaccgtcagaagtacgaccctccggggtactcgcgaaccacgttcttgcgcaacgcactgcagtgcgtcattgcagtcatcgcagccggcgcggcggcggcctccgttccctactggggaggcgatgactttccgctgatgagcctgatcatctacgtcgccggcatggtgttcatcgccatgccgctgtgcctctactacgagtcgctgctccagtcgcatgaagagcgcgtggagcgcgcaaggcacatgctggccgcctgactgacggccaacacctgacaacctagccggccggcttggccttgacgacctgcctcaaaccctcgagcgcagggtcgacgatggctgtgtccgcgcccaccgcatacaccgcgtaggccgggtagagaaactccggcgtgttgggcacacggcgcagccggcccgactcgagatggctgcgcaccacgtcgtgccgaaagtagccggtgccgcccgccgccagcaggtactcgcggccgagcggccccagcccggcactcaccgcggcgttcgagagctccggatacgcaaggccatgctgcgccgcgaactccgggccccaatccacatacacgtagtccgccggccgcggcacgcgcgggcgctgcgcggtggtgaccatgacgagcttctcctcgatgagcagttccacgcgcaggccgggccgctgctgcggcgcataggcaatggcgatgtcgagcacgcccgcagccaccttgtcgagcaggtcgtgcggaaagcccacctcggtacgaatggccagctgcggcgcggcggtgcgcatccagagcagccattgcagcaacagcgggtcccacaggctgatctcgcatccgatggaaagcactgcgcggctgccgctcggcaccgccacctggtggcgggcccgctcccatacctgcaccagcgtggtggcgtgcggcagaaattgctccccggcggcagtcagcaccgcgcccgccttgttgcgaacgaaaagcggccggcccagcagttcttcgagcgttcgcacgcgcgcgctcaccgaggtctgcgtgacgtgcagccgctctgcggcacgctggaagctgcgcgtgtcgacgatctctagaaaggttcgagccaggttgatgtccatgctgcatccgtttttgaatgcaatatttttgcactcaactggcaattaatatcgttttacttgctgcgaacgcgggtcgaagatgaaggcattccatagcaaccaggagttgatcgatgcccacccttcgccagccattccatgccagcccatccgcgagctttgtggatgcgttcaaggcgctcgtcgacgaaaccctgatgctcgccgaggcgctgctgagcccgaacaagatcatcggcgaggtggagcagatgcgtgcgctgcaagtggcggcggacaacatcgaagccaccgatccacggcgtgccgaggtgctgcgctcgcgcgcctcgcgcatcggcctgcgctgaagcgcggcgggccgcaagcggcgcagggttcgcacatttccctgccgagtttttcaagccggagagtcgaagggcacgatctgcgaaatgagcgccggaccgtcggcgagcagaaagtccttgaaggcctgcgccaccggcggcagccgcttgttgcggcggtgcaccacgtaccagttgagcatcagcggaaaaccttccacgtcgagcacgcgcaggctgccggcgcgggtttcctggctgatggtgtgcgccgatacgaagctcacgcccatgcccgcgatcaccgcctgcttgatggtttcggtgctgcggatctccatggcgatgttgatgccgcgcaggtcgccgccaaagccctcctccatcgaatgccaggtgtccgaggccttctcgcgcaccacgaagggctcgcgcatcagccgcttcaacggaattctcggcacgcccaccagcggatggttgggcgccgcgacgatcacgtagggatgcggcgcaaagggctggttgatggtgtccaggtcggttggcggacgcaccatgatcgccaggtcggtgaggttctccgcgatgtgcgtcatgagcccttcgcggttgtgcaccgtgaagttcagcgtcacgccgcggtgccggcttgcaaactccaccaggaggcgcggaaagaaataatcgcccgcgctgatcacgcccacgttgagcttgccgcccgagacgccgttgaactgcagcatcgcgttctcggccgcctcgaactgctggatgatggcgcggctgatctgcagcagctcggtgcccgcgggggtgaggtagatcttcttgccgaactgctcgaacagcgcgttgcccgcgtgctcttcgagcttgcgcacctgcgtggacacggccggctgcgtgaggtgaagctcttccgccgcgcgcgagaagctcagcaagcgcgccaccgcttcgaagactttcaactggcgcagggtcgcgtgcttcattcggaaaaaggttgctgcaatcgagcgggcatcgtactgcgcaccaggccccgcccaagcgcagcctagggtatgcgcgcgacgtgcagcaggttcgtcgtccccgaaagcccgaacggaaggccggccaccaccaccacgtcgttgcccgcgctggcgaaaccttcggtacaggcgacgcggcaggcgcactcgatcatctcggccacgtcgtgcacgtcgtcgaccagcaccgcatgcacgccccacaccatcgccatgcggcgcgcggtggccacgtcgggcgtgaggctcaggatgggcacggccggccgctcccgcgcggcgcgcaggctggtgaagcccgaagaggtgtaggtgacggtggcggcgggcgccagcagcgcggccacctggcgcatcgaagcgcacacggcatcggcggttgtggacagagatgcctcgtgcgtggcgtcgatgccgatccggtacgacgcatcggcttccacgcgcgagatgatgcggtccatcatggccaccgcttcgagcggatactttcccgaggccgattcggcggacagcatgaccgcgtccacgccgtcgtagatggcggttgcgacgtcggacacctcggcgcgcgtgggcacgggcgcggcaatcatcgattcgagcatctgcgtggccacaaccaccggcttgccgcgcttgcggcaggcgcgcacgatgaggcgctgcagttcgggcacgcgctcgggcggcaattccacgccgaggtcgccgcgcgccaccatgacgccgtcgcacagatcgacgatcgcatcgaggtggtcgatggccgcgggcttctcgagcttggccatgatccacgcacgcgtaccgatgatggcgcgcgcttcttcgatatcttcagggcgctgcacgaaagagagcgccacccagtccacgcccatggccaggccgcaggccaggtcgtcgaggtccttgggcgtgagcggcgagatcggcagcagcacgctcggcacgttgacgcccttgcggtcggagatcgggccaccgaccagcacggtggtctcggcaaagtcggcgctgtagctgtccacgcgcagccgcagcttgccgtcgtcgagcagcagctcggtgccgacctccagcgccgcaaaaatctcgggatgcagcagcggcgcgcggcgtgcattgccgctcgtcttgtccatgtcgaggcggaagtgcgaccccgcatcgagttgcgcgcgcccgccctcgaaagtgccgagccgcagcttcggtccctgcaggtcgagcagcacgccgatgggccggccgaactctgtctcgagccgccggatcgtgtcgaggcggcgtgcatggtcgtgctgcgtgccgtggctgaagttgagccggaacacgtccaccccgcgctcgaacagggcgcgaatggccggctcgtcggtggtggcggggccgagggtggccacgatcttcgcgctgcgtgtacgtcgcatcatccgttccatttcatcgatcgatcacaacgcgcacacggcgcagtatgcgcagcctgaacaaggctagctcgccatctcgtgcaggcagacccggccgcgctgttcttccatcgtacgcgccagcagcttgacgagcgaatacacggtgtcgatgtgcggcgtcggggtttcggtgagccgggccaactcgaccacggcgcccaccaatgcatcgatctccggcgcgcggccggcttcgacgtcctgcagcatcgatgtcttgtgcttgccgaccttctcggcgccggcaatccgtttgtcgagcgtcacgcgaaactcgatgcccagcttgtgcgccaccgcctgcgcctcgcgcatcatcgccgcggccagctcgcgcgaaggcgggtactggcagatgtcgaccagcgtcgagtgcgagaggctgctgatcgggttgaaggtcaggttgccccagagcttgagccagatctcggcgcggatgttgtcgagcactggcgccttgaagccggcagcgcccaggcaggccgacactcggttcacgcgctcgctcgacgaaccgtcgagctcgccgaccgggaagcgatcgccctcgatgtgcttcaccacgcccggcgctgtcagctccgatgcggggtacaccacgcagccgatgacccgctcggcgggaatcttcgcggccaccagtccggtgggatcgacgctgcgcaccggcgtgcccgccagcgcgccgccgtggtcgtggaagtaccagaacgggatgccgttctgcatcgtgaccaccacggtctcgggcccgaacagcttgggaacgtcgttcgccacggcttcgacctggtgcgccttcatcgcaaggatgacgatgtcctgcggccccgcctggtcgtagcggtcggtggccttgacgttacgcgccacctgctccacgccgtcggccccgatgagcttgaagccgttggtggcaatggcgtcgagattctttccacgcacgatgaacgtcacgtcctcgccggccagggcgagctttgcgcccaccagtccgccgatcgcgcccgcgccgatgactgctatcttcatgtcgatccccaaggttgtagattcttttcgcgcgggcagggctcagccgaaacggttgccgagcctgccgatgccgccgatctcgacctcgacaaggctgccgggcttcatcgaaccgacgccgatggaagtgccgcacaggatcacgtcgccggggttcagcgtcatgtcgagggaaatcaggctcacgagttgctggaccgaaaagcgcatgtcgctgatcggatagttctgccgcacctcgccgttgagcagcgtggtcacggtcagcgttgcggggtcgaggccggtggccaccaccgggcccatcgggcagaaggtgtcgaagcccttggcccgcacccactgggtgaacgacgcgtcgcggttcagtatgtcggccacggtcacgtcgttggcgcaggtgtagccgaacacgtgggccagcgcctcggcctcgggcacggcggtgcaggtcttgccgatgacgatgccgagctcgccttcgaacaccaccttgccctcgcacaagggcttgcggatgtccgcgccgggcgcgaggtaggagttgggcgccttcagcaggtacagcggttctgccggcactgccagtttcagcttctcgccgagcgcatggaagttgttccacagcgcaatgaccttggtgggctcggtgggcgttagcagccgcacgccggccagcacgaacacgcggccggtcggctcggggcggtcgaacatgttgccgcggtgctcgtgcacggcatcgccttcgagcgtgccgaatccggtttcgccgccgtgttcgaaacggacccattgctgtgattgctgctgttgcatgtctcgccttccttggttctgttggagtggttttttctcagggctcagtcgaagggcaggtagtcggggatgaccagcgacgcgagaagctttcccatctcggcggggttgtcggtcacgtggatgccgcactccctcatgaccgccagcttttcgcgcgccgttcccttgccgccggagacgatggcgcctgcgtggcccatgcgcttgccgggcggcgcgctggcgccggcaatgaagccgaccacgggtttttgcatgtggtcgcgaatccagcgcgcgcaaatttcttcgtcgttgccgccgatttcgccgaccatgatcacggcgtcggtgcgcgggtcgtcgttgaacatcttcagcacgtcgacgtgccgcaacccgcccactgggtcgccgccaatgccgacgacggtcgattgcccgatgccatagttggcaagctggctcgcggcctcgtaggtcaacgtgcccgagcgcgacaccacgccgatgcggcccttctggtggatgtggcccggcatgatcccgatcttgatttcgtcgggcgtgatgaggccggggcaattgggaccgagcagcaaagtcttgctgccttccatgcgatggcgggtgcggatcatgtcgcgcaccggaatgccttcggtgatgcacacgacaagatcgagcccggcatccacggcttcgtcgatggccgcggccgcgaagggtggcggcacgtagatgaccgagacggtggcgcctgtttctgccttggcgtccttgacgctgccgaacacgggaatgccgtcgaacgacttgcctgccttcttcgggttcacgccagcgacgaagcacttctggccattgccgtagtcgcggcacatggcggtgtggaactggccggtcttgccggtgatgccctgggtgatgacgcgggtgtgcttgttgatgaggatcgacatgtcagctctccacctcttgttcggggcgcttgtgttcagagcggttgtgttgtgagcgctcttgttcagggcgcgtgcacaggccaccgggtactcccctccgcgaatgtcccccgccttcggctcctcctttatttcgctgcggggagcacccggcgccctgcgcacacagggcgctgtcgttgttcggctcgatcaacaaccgctctgaataacgatcccgtcgatggggtgccttgcgcagcgaaataaaggaggaacccgaagggcgggggacattcgcggagcaaggtaccccgtcggcgggagcgcgccctgaatgacggacaacacgacgcaaagaaacgcaagacttcatagtcctagcccccccgccgagccgcagccacgaccgtctgggccgcatcggccatgtcgttggcggagatgatcggaaggcccgactgtccgaggatggtttttcccaggctctcgttggtgcccttcatgcgcaccaccaacggaaccgacagttcgacctcgcgcgccgccgcgacgatgccgcgcgcgatcacgtcgcatttcatgatgccgccgaagatgttgaccaggatggcgcgcagattcgggttgcgcagcatcagcttgaaggcttcggtcaccttctcggccgtggcaccgccgcccacgtcgagaaagttggccggcgatccgccatagagcttgatcgcgtccatcgtcgccatggccaggcccgcgccgttcaccaggcagccgatgttgccgtcgagcgggatgtacgaaagatcgaacttcgaggcctggacctccgccgggtcttcctcgtcgaggtcgcgcatcgccgcgatctcgggctggcggaacagcgcgttcggatcgaagttgaacttcgcgtccaacgcgatgacgcggccgtcgcgcgtcagcgccagcgggttgatctcggccagcgaggcatcgcaggcgtcgaaggcctgatagaggttctgcaccagcgtgcgcacctgcagcagcgccttgcccgaaaagccgatgtcgcgcgcaatgccatcggcctcggccgccttcacgccggtggccgggtcgatgaacagcttgcggattctttccggcgtgcgggccgcaacgtcctcgatgtccattccgccttcgctcgaagccatcaaggccacgcgccgcgaatcgcggtcgaccgtcatgccgaggtagaactctttttcgatctcgacgctctcttcgaccagcagccgctttaccagccggccttcggggcccgtctggtgcgttcgaagcgtcatgcccagcagctcgtcggcgtggcgccgcacttcggccgccgaccaggcaagccggacaccgccgcccttgccgcggccgccggcatggatctgcgccttcaccacccaggccctgccgccgatccgcgtggcggcatcggccgcttcgtcgggcgaaaagcacgcatatccacgcggcgtgggcacgccgtatttgcgcaatacgtccttgccctggtattcgtggatcttcatggcaattcaggccccgagttctgcgccgcggctttcggcccagttgaaatagcgctttttcatggcgcccgtatccggctcgcgcttttgatgctcttgcttcttctgctcgatcacttcggccaggaatttggcgtcataggcgcgcagcagatgcggctgataggcattcaggtagtggctgacccgctcgatgccgtcctggctctggcgcagcagttggcaataggtttcgcggtcccagtgccagcggaaccccagctcgtagaacgcggcgttgtaggcgttgcgctcggtttcgctgctccagtattgaattggcaattcatcgatcatgaaatttctcctagaaattgaacgccgggcgacaaatgattcgtggatcggcatgatcaaaatgtaggttcgatgatcgataaataatagttaaactattttattgaatgtattcgcaataagttatacattcgaggcgaataatttccatcgccagcgcatccgccgcccgcgtctttattgcgctattaaaaaagccgcgccgcggctcagatcacgccctcggcgcgcagcgcctgcacatcgcccgcggtgtagcccagctgcatcagcacttcttcggtgtgctcgcccagcagcggcgagcgcgtgacctcggtcgggctgtcggacatcttgatggggttgcccaccgtcaggtatttgccccgcgtcgggtggtccacctcgacgatggtgccggtctcgcgcagggacgggtcggcggcgatttccttcatcgaaagaatcggcccgcagggaatgtcgtactggttgaggatgtccatggcctcgaacttgtccttggtcatggtccattgctcgatgcgcgcgaagatcggcttcaggtgcaacaggcgcgccgcgggcgtggcgtaggcctcatcggtgatccagccttcttcgccgatgaccttgcacaccgcgggccacacggccccttgcgtgatgaagtagatgtaggcgttgggatcggtctcccagcccttgcacttgagaatcgagcccggctggccgccgcccgaggcgttgccggcgcgcggcaccgcgtcgccgaacttgccgtccgggtactgcgggtactcgtgcatggtgccggtgcgctccagccgctgctggtcgcgcatcttcacgcggcagaggttgagcactgcgtcctgcatgggcgcgagcacctgctggccgcggcccgtgctgttgcgctggtagagcgccgccacgatgcccagcgccaggtgcaggccggtgccgctgtcgccgatctgcgcgcccgtgacgaccggtgggccgtcgtcgaagcctgtggtcgaggccgcgccgcccgcgcactgggccacgttctcgtacaccttgcaatgctcgtacttgccagggccgaagcccttgaccgaggccacgatcatgcgtgggttgagctcctggatgtgggcccaggtgatgcccatgcggtcgagcgcgccgggcgcgaagttctcgaccagcacgtcgcaggtcttgatcagcgtgtcgagcaccttcttgcccttgggcttcttggtgtcgagcgtgatcgagcgcttgttgtggttcagcatcgtgaagtagaggctgtccacgccgggaatgtcgcgcagctggccgcgcgtggcgtcgccctcaccggcgcgctccaccttgatcacgtcggcaccgaaccacgccagcaattgcgtgcacgtgggaccggactggacatgggtgaaatcgaggatgcgaacgccctcaagtgccttgctcatcagctgtctcctttgatcgtggtctctgcttcttgcagacgagcgcgcaatttacgctcctccgcaaagcgggctgtttcgtctcgcacgaaggcaacgatgcccgtgacttcacgattttccgagaacagcatcgacaccgtgaaggcgatcgacagcgtgtggccgtccttgtgcagcgccggcacgcgcagcagatcggcaccgtacttggtgatgccggtgtccatcgtcttgtgatagccgtcccagtgccgctggcgctgccgctggggaatgatcatgtcgagcgactggcccagggcctccgcctcggtgaaaccgaagatgcgctcggccgcgcgattccagagcgtgatcgctccttccgcattgcacaccatgatcgcgtcgccggcgccttcgacgatctgcttgaaatcaacgttcgcttgcatgtttacctctggcgcttcatgtcgtttcgcagctcgcccgcctgtcgtcgagcgggcgagctggggtgggtccgctagacggccttcgattctttcaggttgtcgatctgcgccttcgtgtagcccagttcggccagcacctcttcggtgtgctcgcccaagagcggcgaggccgtgacctcgggcttgaggtcagagaacttgatcgggctgccgatggtccagtagctgccgcgctccttgtgcggcacttcgacgatggagccgctcttgcgcagcgactcgtcgtgcagcagttctttcatcgacagcaccggggcgcaagggatgtcgtgcttgcggaagatgtcgaccgcctcgaacttggtcttgtccttgatgaagtcctcgatggtcgcgaagatctggtcgatgtgcggctggcgggccctgggggtcatgtagtccggatcggtcttccactcgggcttgccgagtgcgtcgcagatcgggtcccaggcgtggccctgcacggtgaagtagatgtacgcattggggtcggtctgccagcccttgcacttgagaatccagcccggctggccaccgccgccggcgttgccgccgcgcggcaccaccttgtccttgaacgcgtccatctcgtgcgggtactgtgggtactcctctaggtagcccacgctgtccaggcgctgctggtcgcgcatcttcacgcggcacaggttcagcacggcgtcctgcatcgagcaggccaccttctggcccttgccggtctgctggcggccgatgatggccgtcaggatgccgatggccaggtgcatgccggtgttcgagtcgcccagggcggccgccgagatcgtcggggccgagttttcgcccttccaccagccggtggtggaggcggcgccgccggcgcattgcgcaacgttctcgtataccttcaggtcttcatagtggtggccgtcgctgaagcccttgaccgacgcgacgatcatcttggggttcagctcctggatgcgttcccaggtaaagcccatgcggtccagcgcaccggggccgaagttttcgaccagcacgtcggattcgcggatcatcttttccagcacggccttgccttcgggcttcttcgtgtccagcgtgatcgagcgcttgttgctgttcagcatggtgaagtacagcgcgtcgacgttggggatgtcgcgcagctggctgcgggtgacgtcgccggcgcccgggcgctcgaccttgatcacgtcggcgccgaaccaggccagcatctgggtgcacgccggaccggcttgcacgtgcgtgaagtcgatgatcttgatgccgttgaggggtttgttgctcatggaaattaactcctgggttgccttggattactgctgctgctttttctttgccgtgctcggattcaggctggtgatccggccgctttccgttccggccgtctcgtcgatgacggcgttgatcagcgtcggacggcgcgaggcgacggcttcggccagcgccttctgcaattcatccgcggtggtggcgttgacgcccacgccgccgaacgcttccatcagcttgtcgtagcgtgcgttcttcacgaacacggtgggcgccacgtcgggcgtgccgctcgcgttcacgtcggtgccgcggtagacgccgttgttgttgaacacgacgatgcagatcggcaggttgtagcggcagatagtctccacctccatgccgctgaagccgaaggcgctgtcgccctcgatggcgatcaccggcttgtcggtcaccaccgcggccgccacggcaaagcccatgccgatgcccatgattccccaggtgcccacgtcgaggcgcttgcgcggctcgtacatatcgacgatgctgcgcgcaaagtcgagcgtgttggcgccttcgttcaccacgatggcgtcgggccgtgccttcacctggtcgcggatcacgctcagcgcgctgtggaaattcatcggcgaaggccgcgcggccagcgtcacggccatcttcgacaggttcttgtccttgcgctcggcaatggcaccggtccattcggccggaggcttggcccacttggcatcgacgcccgcgagcaacgccgccacgcaggagccgatgtcgccgatcaccggcgcggcaatggccacgttgctgtcgatctcggtgggtgcaatgtcgatctggatgaactgcttggcgcccttctcctggccccaggtcttgcccttgccgtgcgacagcagccagttgaggcgcgcgccgaccagcatcaccacgtcggcttcctgcagcacgtaggagcgcgcggccgcggccgactgcgcatgcgtgtcgggcaagaggcccttggccatcgacatcggcaggtagggaatgccggtcttctcgatcagcgcgcggatgtcggcgtcggcctgtgcgtaggcggcgcccttgcccagcaggatgagcggcttcttcgcgcccttgaggaggtcgagtgcgcgattcacggcatcgggcgccggaatctgacgcggtgccgggtcgatcaccttgatgagcgaccggcggccggcttcggcatccatggtctgcgcgaacagcttggccggcaggtcgaggtacacgccgcccggacggcccgacagcgccgagcggatcgcccgtgcaatgcccacgccgatgtcctcggcgtgcagcacgcggaaagcggccttgcacagcggcttggcgatggcgagctggtccatctcttcgtagtcgccctgctgcaggtcgacgatttcgcgctcgctcgatccgctgatgagaatcatcgggaagcaattggtggtggcattggccagcgccgtgagcccgttcaggaaaccgggcgccgacaccgtcaggcagatgccgggcttctgcgtgagaaagccggccgccgcggcggcgttgcccgcatgctgctcgtggcggaacgagatgacccgcaggccttcggcctgtgccatgcgcgtgaggtcggtgatcgggatccccggcaggccgaagatggtgtcgatgtcgttcagcttcagcgcatcgatgaccaggtggaagccgtcgatcgtcgcgtcgtgcgccggcgatgcctcctctgtggggtgtttgagggcgaccacgaccgcgtcgccttctgcggcccggttcttgggcttgagggcgtcgtccagggtcgtggatgcctctttgtccgttcttactgaagacatgtctctccttcttgcttgggtgaatggccgaggcccgagccgggactatgattcggaggcatgctttcgggcgttgacctcggtcaactttccggaaaacggcaccggccagatgaaccagatgttgttgttgcgaattcgagcaagacgggacccatgacgctgttggaaaaccacccggagaaaaacatcattcgcgcgcagctccggcagaacatccttctcaaggacctgagcgagagcgagcgcgccgaactggaaacccatctcgtcatcgtggacggcaacaagggcgactttctgctgcaccagggcgtgcgcgagatggagcagtacttcatcctcgacggcatcctcaagcgggtggtgagcaaccccgagggcaaggaaatgatcctgcgctttgccgatgcgcacgacatggaaaccagctatgcggcgctccgcctgggcacgcccacgccctacggcatcgtgtgcgtcaccaaggcgcgcgtggccagcctgccgctgaaggagtggatcgcgttcctcgaccgccaccccgagaccaaggagctgttcgaatactgcgtgatgcgcggcatgagcgaaatcatggcgcacaccatcacgcttcatctgctcgacgcgcccggccgcgtgcaccggttcatgcgcaagcacccggagctcgaagaccgcattccgagcaaggagcttgcgtcgtatctcaatctctcagcagaaaccctgagccgcctccgcaaacgcggaaaaatctaggcaggcgcgttactcaggtctgcttcgccgacgcgaagcggcgcggaacggtcatcaggcgcagcgcgttgtcgacgccgctcacgccgtcgaccttggaagccacgtcctgcgtgagcgcgcgctcctgtgcattgagcacgatgccgctcagcgtgaccttgccctggtcggcctcgacggtcacgcggatgtcgccggtcgcctcgttgcccttcagcgccgacttcacccgcgccgcgagcgccatgttggccaaaagcgcgcgcgaggccggcgtctcggcaaactccggccgttccaccagcgcgcggatctgcgccacgcagctgtccaccgagagtcggtccgtgttgagcaccaggtcgtagagcaccgggtcgccccatgtcacgccgaactgcgcatgcatgcgggccgcatgcgcgtcgtcgctgcgccggatctcggcctcggcaaactcggcatcgtcggtctccaggtgcgccattagccattcgacccgcttcttcatcgagcgcgtgatgcgcacgcacaccacgtgcggcaccggccgcagcaggcaggttgcgccccagccgcgcaacaccacgttgccgcggtctgccagtgcaaagagttcttcggccgtatagagcgcaaggctgcgcttgtcggcggtgagccgttcgacaaaacctgccttgccgtcgcgcaagcggccaatgaagctggtcggcacctgcatgcggtcggccacgcgctcgatcgtctcgtggcgcatgatctcgaggccgagctgctcggcgaggcgctgcgacacgtccttggcgagggaacccatctcctgagtgagtgcaatcactggcatgttgttgttctccgctcagtccacgggccgttcgacggcaaattcgtcgtgcttcttgggcttgaccagcgccagcgccttggagatcagtggccagagcagcagcacgagcgccagcgtggtgatgccgccgaccagcgggttcgagaacatgatcatcacgtcgccctgcgagaccagcatggcctggcggaacgagtcttccgccttgtcgccgagcaccagcgccaggaccagcggcgccagaggaaagtcgagcttcttgaacaaataccccaccacgccgaagccgagcatgaaccagatgtcgagcatcgcgttgtgcacggtgtaggcaccaatggcgcagatcacgatgatcaccggcgcaatgatcgagaacggaatgcgcaggatcgaagcgaacagcggcaccgtgctcagcaccacgatgaggccgacgatgttgcccaggtacatgctggcgatcagcccccagacgaagtccttctgctcgacgaacagcagcggtccgggctgcaggccccagatcaacaggccacccagcagcaccgcggcggtgggcgaacccggaatgccaagcgccagcatcggcagcagcgcactggtgccggcggcgtgggccgcggtctcgggcgccacgacgccttccatctggccggtgccgaacttggaaccgcgcttcgacatcttcttggccaggccgtaggccatgaacgaagccggcgtggcgccgcccggcgtgatgcccatccagatgccgatgagcgagctgcgcagcgacgtcacccagtattgcggcagctgcttccacgtttgcagcaccaccttcggatcgatcttcgcggtcttgcccgagaacttgaggccctcttccatcgacagcaggatttcgccgatgccgaacaggccgatgaccgcgatcaggaagtcgaagccgcgcatcagctccgactggccgaacgtgagccgcagctggcccgtgaccgtgtccatgcccacgctggccagcgcaaagcccagcgccatcgacgccaggatcttgaacggcgaccccttgcccatgcctacgaagctgcagaaggtcaggaggtacaccgcaaagaattcgggtgacccgaatttgagcgcgaacttggccaccagcggcgccaggaaggtgatcatgatcaccgccagcagcgcaccgacgaaggacgacgtgaacgccgtggtcagcgcggcgccggcgttgccctgctgcgccatcggatagccgtcgaaggtggtggccaccgaccatggttcgcccggaatgttgaacaggatggaggtgatggctccaccgaacaacgcgccccagtagatgcacgacagcatgatgatcgccgaggtgggcgacatcgtgaacgtgagcggcagcagaatcgccaccccgttggcgccacccagcccggggagcacgccgatcagcacccccaggatgatgccgacgaacatcaggccgatgttcatgggtgtgaggatcaccgagaagccctgcatcagggcactgatttcatccatttcgcatttgctccgtgagattcagtagccgagaaaacggaggggatcgagtgcgcccttgaacagcggcaccttgaaccacacctcgaacatgaagaagaacaccgtgttgaccaccaaggccgcaatgacgctcttcacccacgagtacttgcccaggaacaccatgaacagcgcgatgtagatcgccgaagccacgtacaggccgagcagtgaaatggccgccacatagaccgtggccggcaccagcaccgagagcacgcgcttgagctgtaccgtgtcgacgaagacctcggtcttcttgttcttgccgagcagcgcctggtacaggatgccggcacccgagatggtgatgatcacgccgatgtagaacgggaagtaccccgcgccggggccatcgctggtccagcccgagcccagcctctggctctcgtagatcaccaccaggcctatcgccaccaggaccagcgcaaccaccgcctctaccaggttggtcgccacgcccctgcgcggcgtgccatcggaaatctcgtcgtgttccatggagtccccatcgttcgtatgtatgtgccgtgaaaaaaacgagagtgcagcgccccgcccgccgcccggccggcggcagtctcttcaggcaggaagcgagtgctgcagggcgctcgattgctgctgctgctacttgttgctggccaggaagccggcttcggtcatcaacgtgcggtgcgtggcctccgcttcggtgagccacttggtgaacgcgtcgcccgtcatgaaggtcgggttgaaggcacccttctccatgtattccttccagtccggcgtggcggcgatcttggtcagcaggtcgacgtagaacgcgcgctgttcgggcgtcacgccggggggcatgaagatgccgcgcagcatcgtgtacttggtcggaacgccggcttccttgcaggtgggaatgtcgttccacgactgcgtgtcggtcaccttggccttgaacggcatgcgctcgtcgtcgaacacgcacagggcgcgcagcttgcccgcgcgccactgggccacggcctcgatcgggttgttgacggtggactgcacgtggccgcccaccagctgcaccgccacctcgccgccgcccttgaacggcacgtagatgaacttggtgccggtggctttctcgagcgccaccgtgatgatctggtcttcctgcttggagccggtgccggccatcttgaacttgctcgggcccgccgccttggccgccgcgatgtactccgaggcattcttgtacggctgctcggcattggtccacagcacgaactggtcgagcgccaacatcgcgaccggtgtcatgtccttccagttgaagggcacgccggtggccatgggcgtggtgaacaggttggacagcgagatgacgatcttgtgcggatcgcccttggcttccttcaccgccaggaagccctcggcgcccgcgccgccggacttgttgacgacgatcagcggctccttcatgagcttgtacttgatgacgatgccctgcagcagccggcccatctggtcggcgcctccgccggtgcccgcggggatcacgaactccaccggcttggtgggctcccatgcgaaggctggcgtggccaccgcgagtgccaacatggccgcggtgaagactttggcccgacaagcgcgagtgcgcgaaaagaagttcttcatcatgttgtctcctgtgtaaggtgcgctcttttttggtggatctgagccgagatgcgaacagggcagatggtgcgcgctgatagaacttcgcttgcttgaccatggtcaacttttgcgagattttgtcttggggttagcccgcgccgcgtgatacgcgagcaagcgggccaaggcgacccgatgagcctgcgcagcggggcggcgccacgcggagcggcacgcattgcgcggccttttttcgccgtgccgaggggaatccgggtaaaccctacaatggagggcaattcaacccatccacgaattccaggagttcctttatgcctacccttgaccgaacgtccggcgcgagcgcatttggtggcttggctggcgcgctcaaggcatttgccgaagaggcctgcgtgctcgttcaggccttgctgagccccggcaaggtcatcgaggaagtcgagcagatgcgcgcgctgcacgtgcgcgccaaccgcatcgaggcctccgacccattgcgcgccgacgtgctgcgctggcacgcctcgcgcatcggcctgcgctgagcagcagcaacaggccacgcggcggctcaggcagccgacgcgccggagccgccccgaactggtaaagtccgggccgccctccgtcttcgtagttcaatggatagaacggggtcctcctaagactcagatacaggttcgattcctgtcgaaggcaccaaggacccgtttcacggcgtctcatcccacatcagaaacccgcacgctccaaggcgtagcgggtttttctttgcctcggcctgtctcagccggtagcattccatcgcagcggaataccatcatttttgctggtagacaccggcaccgacaaactcgataccaacaacgcatcatggcgctcaccgatactttcgtccggcaggttaaacacaagggcgccgacaacggcgagaagtacggcgatggtggcgggatgtacctgcacgtcacggcgacaggcaaatactggcgcatgaactaccggttcgccggcaagcaaaagacgttagcgctcggcgtctacgccgacgtttcgctcgccaaggctcgcaagcgccgggacgaagctcgcgaacagctagcagacggcatcgatcccagcaccgcaaaaagggagcaaaagaatgctctgcgcgatgcagtcgcaaacacatttgaggcggtcgggcgggactggttggagaagaccacggctaaacgccagccagacacccaacaaaaagtgcggacatggttggaaaaggatgtgttccccttcattggccgcatgcctatttcagctatcgggccccgcgatgttttggacaaggtcatccgcaagttggaagcgcgaggtgctgtcgacaccgcccatcgcgtcaaacaactctgcgggcaggtattccggtttgccgttgtatctgggctggcagaacgggacgtgactgcagacctgagggaagcgctggccacgaaggtcattaagcatcatgctgccatcactgagccggcggccgtggggggattgatgcgcgccattcatacttacaccgggcatgcgaccaccgtggcagcgctcaagttgtccccgctggtgtttgttcgcccgggtgagctgcggaccgctgaatggtcggaattcaacttagaggccgccgaatggcgcatccccggctcgaagatgaagatgggcattgaccacatcgttccactgtccacccaagccttggagatcctgcgctcgctacgtcccatcacgggccacggccgctatgtgttccccagcatccgcaccggtgagcggcccatgagcgagaacacggtgaatgctgcgctccgagcgctgggatacagcagcgacatccatacggcccacggcttccgggcaaccgcgcggacgatcctagatgaagtattgggcgagcgagttgacttcatcgaacatcagctcgcacacacggtgaacgataccaacggccgcgcctacaaccgtacggcccatcttccagcgcgccgggaaatgatgcaacgatgggccaactacttggacaagttgcgaattggtgctgaggtcatcgtgcttgctcaagccgcctgaggcaagctactgctcaaaatttaagcatccaattgggccgagagaaaatattttctctcgacctaagctgttgatttcattagatttttacaggaaccctgcagctgaagcatgtgctgcgtcgattacggccgctcgctcctccctataaatagatcgcacaccttgtgcattgacctaaaccaacctggagcgccatgcagcaacacaccattctccgtttcaaggatctcgtaactcagctccgcctgagccgctcaaccatctatcggttgatcgccagtcctagcagcggcttccccaattccatcgagttgtccgcccattctgtcggcttcctcaagtcagaagttgatgcatggatcgagcaacgtcggcgcaacgccgttgaagggaaggggcaagcatgctgagcctggcacagatagccgccgcgcaaggctggggcaagtggccggtttcccgtcaagctcgcgaagaccgtcagcgctgggccgaagagcaggatcaattgaatggatggttcttcttttccggggaagtttccgacgagcaaatgcgagctgtttttcgcaaagaggcacatattgcgcgggacaagaacggcaactacatcgtgattgaaggagcgccagatgcagactaaccacataaacgcggagcaactggcagatctcctcaccgaggccgtcgtcttggacaccatcgaacacgagggccagcgcacctatgtgctggagtacaccgggcaggacatcctagccgtggacaccctcaacggcggcgcgacggtcatctacccgtgcagcagcttcgacgctgaaagcggcggatcgatccatgaccacgctcgctcccagcgcgaaggttgagagcgaacgtgcactagcctccctcgatagcgttcccgcagcattgctgcggccagagccgcacgcggcgctgttcaagtccataacgatgctggcggccgagaagcgccagcacgaaggctcggagcgcttctgcgaggccgtccgggggctgaccagcgccagcactcaaacgctcatcctgcggctttctatgggcacggatacgctgctcatgtgggcaatccatctagagcttgaccgcagaaacgtgccaccgtgcctgcgctggccgacgaacgacagcaccccgcagcacgagttcgtcacatggcttgcagacatgctctggttcaccaagcgcaacccgaggcacacgccccgattccggggctggaaagggctattcgacacccccccgtgctctgctaagtggcacgcgacagcagcccggcagtttgcatttgtcagtgctcgctatagcgtggcgcactggtgcacgacggggctcgggctatccgactcacagaggcgagacctgatgacattgccgacaagcgggatgcgagccgagcgcagacgacttgctccccagcagtggacgattgcatcagagcgcttgctgagccatgcaatgagacatcgtgaccgctccgggcgccacacccctgagaacgtcgctgctaggcgtgcagcgcttctgcgaacgttcgtgctgtctcaccgtagcccgactgccaccgctgagaactggcgactacttactgggggtcagctgtcccggcaggccgtctccaaactgattgagacaatcaccgacatcgtcgtaagtgagcatagttgatcattttcgactgttcctatgtgcctccccatttctacgaaatggggggtatgcacgcaaccactgaatcgctagcactgacgccacgtttaggggttgcgctcggcttcatctcaaggggttgcgctcgccggcttcagcgcaaccccttatcccgctagattcgtgcgccagcaaggccagcagcggcgtgtaagcgccgctcctacctataagcaaaccgcaccataccgaccccatccccatcgaaaaaacatcgcgcttttctcggggctcggggctctcgggcagcagcgaccggcgcgaccgtctgccgcagcccgcagaccttgacacccctgcggggcagctcatggcctcgaagcccctcgtgaagttttttccgggggtttagcgagactgcttatagggcgcaaaggaaatgcttgctaccgcaggcaaaattcgacgggcgaaagtgttgcccgtgtggcactgcacagcaacgatccatgggctgcaccataggcctcgcgcgaggcaaaatcctagctatgaagccctcagccccctccgtcttgatcgtggtcctgctcgtgctccttgtgtggttcgccgccgcattggccacagtggagaacgagcggtacgcccttcaggttggcctgtgcaccttcaacccaactgatccactggcgctgttcgattgcctcaagaaagccgagacgcgcaccggttggtggtggcacatcttttacgcgctgaagggttaggccatggctcagctgatcccccagccactcgtcgccgtaatcgctgaactcgtcgcgcacgcagagacccatgcgacgcttcacggcttgtttatgcatgcggaagcctccggcgacgcgcctgacggcaacaagctcgccaaagctcaagactggctccggaatacgaacaagcgacatccggagcctctagctgtagcgggcggaatcatctgcggttacatggaagacccggacatggacgccgaatactcgtatgcaggatttggcgacgaacccgagtttgtagttaaaaagcgggcgctggtccgaaaggttgaagcggtgctcgggcggtgcgggctcaattaccactccggcggagttatcacgaccggaggactcgcaccaagcaaggctctaggggaaatcattcgcggccgagacttacccgccatccatcgtgagttcgagcgtgccatggagtctgtcgagtcgaagccgcgtgatgcggtttctgctgctgccaacatcctcgaatcagtcttcaaaacctacatcgaggacaacggtctcacgatgcccgacaagcaggatttgcaaccggtcttcaaggtggttcgggcagacctcggacttgacccgggcagtattgaggacaatgacctccggacaatcatcagcggcttgttctccgtggtggacggcatcggcgccctacgcacacacgccagcagcgcccatagtgaaggtcgaaagggctacaagctggagccccgacatgcccgccttgcggtcaacgccgcgcacaccgttggagccttcgtcatggaaacgtgggacaagaaggcgaggacggcgtagcgtggtgttgtccacatgcagctagggcaggattcgggtcgccgtgtgttgcattggcaacatatcacctagcatcatgatttgatggtacttgcgttggttctttgcttttgacttttgcaattactgagcattcatgcgggttgcagccgagttttcgattcctgtcgaagcaccagcaagccgttgaatttcaacggcttttttgtttggtggaaaggccgatcttccagctccgttcattccggcctctggcaggctctttgtcgtgggcagcagcggagagggcatttgtctccccggaaaaaggtgcgtaccgctcatgcgcgcgtgcggcgcaatttctacagtgacttcacggcgaacgctttgttccaaccaggcaaacaatgcggcgccagttgtccatctcactggagaacgcacatggccaaacagttcgctcagctcttggtgtcttcgtatttgcttgtgttgctcgctttgtggttcgtcatctgaacgtgagcggccgacggtccgtcgagactacttcctgctgcgattggatgcggacggcgccgaagtcggcgaaggcgccattccgccgtccacgcccagccggccaccgccgccgaggccctggccgcgcacggtctgcgccttgtagttgcgcagcgagcgaaccatctggttgaagccgtccatgaacgccgcggcaatcaccttgccttgcgccgtgttggtatagccgccgagattgccgccggcgcgggcgccgaacaccgagccgaaggcgccgaagtcggtcttggaggcgctgccttccgaagccgcgacctgcacgcccgagcggttgtcgatgagcgtgagcagcgcactggcttccttggtctgcatgcttgcgcccagcttggcaatcgcgaggccccgtcccccgcccaccaggccacccagcgcaccgccgatgccgccggcatcgctgttgctgaacacgatctcgggcgagaggccgtagtcggaggccaccatctggccgcggccgaagttgctaccgccgcgcatttcacccgactgctgcagcgcgcgctcgcgcgtcatggcgttcatgccggccgcgccacgctcgaccaccacgaagcagttcgactgctgcaccaggaggcgcagcaggttggccgtgggcggcaggcggtattcgccggtgaggatggtgtaccagccggagttcacgttctcgatcagcgagacggtgccgagcggcgactcgcagcgctccagctggctgctttcgccggcggtggccgaacctgccgcgctgcccgtggccatggtcttggacgactggctgcccatttgcatgtcgagagcgggcatgttctgacaacccgcaagagccaagagcccggtcaccgccgcgactgtcggaaatctcatgtatgaccgttccatggccgagtttgaaagtgggcgctggtatgccgcacccgttgattttttcatgcgttcctccctgttggttggcaaagggccgagatccggccccgtgcgaatttaggcggaaagcaagacgccctgtaagtggctaaagtcacttgctgcgtgatgcaaggtcgtccccgccatggcctgccgggcgcgggcgaacgctacttcggcgtgtaggtcatcttgatccgctctgttgtgatctcgggccgggggcctccttctggacgcgtatggatcttgagcaactgaccccgatatgctccttcggcagcgacccatgtggtgaaggtcgtgacggaggacgtgtcacccgtacctgtggtttgcctgttcgtgaacttgcaagcgttgaaggcgcccatctccgtttgcaaagtttcgcggcccacataggtcaggtctcgcgacacggggtactcggtctcgatctttgacccatccgccgtactgacggcaacagtcttgatcttggtgctgccacttgccacttgtccgggctgcatgtccaccgggccgcccactggtggatcgaacgtcactgtgatgacttgggtcgcgacttgcgcaatcgacccgtaggagaccacgttgccattgaccaggtcgtggtagttctcggcggcaggcgatggattgccggcggtatcgtggggttggaccttgacggtcacaggcgtgacaccggcaaacgacttgcgttcgccaactgtttcgacggtgcggcccaccgtgggggattgcccggaaatcgtcgttcgttcttcgtagtcccgcgcagttccggcatggaaatccgcttcgttcgtacaaggggccgagctcgttgccgatgccggtgcaggggctggcgccggtggcggcgggggtggtgaagaggagggtgcgggctccggagcaggcgcggcgggcaggattggaaaaccgccgccaccattgcctcctcctcctccgcctccgcatgccgccattaccgccgcgatggacgcgatccccgctccaattgcccatggatttctgttcatacgatctccctgttgcttgtcaaaaaaggccgacatccggcccgatgcaaatctaggagaaggcagagatcaacctgcagtgtctaaagtcacttgttgcgctcagggcaaacgccgacggcctgcgggcgcgagttcagccatggcttgcaggagcgtcgcggcgctcacgggcttgaacagcacaggtacgcccgaggcgcgcacacgctgcagccgctcgggcgcagtttcgcccgtgatcagaagcagcggtgcatcgagccgaaagcgttcccgcaggcgcaggccgacatcgagtccgtccgctccgtcagccagccggaagtcgcacagcagcagtgcgaacggcttcgcctgtgcatcagaatgcgtcagcacctcggctgccgcggcttcgtcggccacggccaccacatcgagggagtaggcgcccagcagcgccgtcatggcttgcctgatttccaactcgtcgtcgatcaacaggatgcgtccgcgcagatccggtacggcgaagcgatggcgcacgggcgattcgagatcctggagcaagagatccgtgggcgattccgatgttgcctcggccctcggcaccagcaggcgaaagcgtgtaccgcggcctgggcgcgaacgcacttgcaccggatgagcaagcaactgggacaggcgctgcacgatcgacaacccgatgcccagacctcgggagcggtcacgtcccgggttgccgatttgatagaactcctcgaagatgcgttccagctgtccgggtgcaacaccgatgccggtgtctcgcacttcgatccacaccgaatcaccacgcacaagtgccgttacggtcacgccgccgtgtcgtgtgtacttcaacgcgttgtcgacaaggttcgaaagcatgcgatacagaagttgcgggtcgctgcgcacccacagcccgctggcgcgaatgcgcaactgcaaattcttatggtctgcttgcgccgagaaggtgtgattgagcgggcgaaacagcgcgtcgagttccagagcacatggctcgggcaccaccactcccgcatcgagacgggaaacgtcgagcatggtgttcagcgacgcacccagggtatcgactgcccgcatcaggcgctcggcgttttccccttcggggcggtcgtgcagggcgttttccagggcggcgccgaacaatgcgatggcgtgcattggctgacgcagatcgtggctggcggtggccaggaagcgggtcttttcggcgctggctcgttcggttgcagcgatttgctcgctcaagcgagcggccagggcctcgttctcgaagcgcaggatcagcgattcggtcaaccgcctgttctcctgcaagccggcgcgaagggtgagtatcaggttgacaattccgaatccggcgaggaaccagttcagggcgctgccatgccagaccagggccgcgataagacccgtcatcatgggaatgccatacccgaacatggccggcttcagaggccatcgtgcctgcacggcccgtgtccaactgccgatgatgacgaccgtgaacacggtggtcatgaccagatccgtcgtcgacacaaggaacaagggcgctggagccgtcgcgatgctgaccatggtgaccaggcgggcgtacttgcgcgcccaataggggctgtcggacatcggcgtggcaggggtccagcgcggtgccagcaacgcgtacaggtccacggcggcaagaacgagcagccagtacaacaaccatggatgggcgagacgcgagtagctgaagatggccagcgcggccgcaaaaccgaaatgggccagaaccgctgtgctgtgaccggcgtagaccgaagccacgtgctcgcgcaatatgcgcagcctcagcttggcatcgacggccagatgcttcgacacgatggcgctcatcgaattgcctccccgcaggagttgtctcccgcatgtatttgtatgttgcccgcgcgggctgggcttaccgcaagctactgatcaactgcgcgcgcgagcgcacaccaaacagcaagaagatggtcgacacgtagttcttcacggtgccttcggtaagactcgctgcctcggcgatctccttgttggtcttgccttccagcacccactgaagcacctgtatttgccgtggcgcaagcgcctgccaggcgcggccatgggagggtttcgcgggccggattgcggtcgacgaagggcaaggcaagccgtctaccgcgtcgctcccgagcagcccacaggcccggatgaaactcaccacctccttgaggttcgccgacttggaaatgaaagcgctggcgcccagagccagcgcgccctgggcgatcgtggactgcgcaatggaggtggtgccggaccccgaaatggcaacgatgcgagcggcaggatagcgggcgtgaaaatccgccaggccgctcaggccctgtgtatcgggcaaggcaagatccagtagcaccagggcgatgccatcctgggctctttcatacaacgccaaggcctcggcgaggttgccggcctccaggacttcaaccgtttcgccggatggagaggactgtgcctgcagcagtgcgcgcacccccaggcgtacgagatcgtgatcgtccaccaccagaatggcgcgcggccgccgcgcaggcgcgggaacgccatgcgggggagattgattcgactcgacggtactcaagcaactgaatctaggcggttctgggcggaaaggtaagtgacgaaagtcaggttgcgctgcatgcctcgcctcgccaggcaccaacgatagcgccctctcctctggggccaggcccctgtttgcgattcctgtcgaagccccgcgaggccgttaactcttcggcccaaacggcgtctgcacgtcctgcgacgcctgttgctggcgttgcggtggaccgaccagtgcggcgggtccggtctgctcgcccaggtctttgcgcccaaggcctctcacgaggcggcgcggtatgtggtgtgttctcagaaactgcgccagagcttcactgcgcgcgggttcggatgccggtagaaacatgtgcatcacgctcatggtgtcgtcccgtaaatgccagaaatgcaagatggctggctcgcttccagtagacccggagccttgggtttgacgcggctctggcgtgccgcaggcggattatgggcgtcggatttcgatgcggtggcacagccccttggcaagtagtgttgctggaacgcttagggcttaccgataggtgctcttctcgtaatttacttactttttactactgttcgctacgctcgccctggcgttccaggccaggcgtgtaccggccagacccttcagccgaagctgtaggcacccgcccacgcgcacgggctggtttctcccgcaagcgtgggccgcgagcgccgccaatgtagagccctatctactaaacggagacgccgatcatgaaaagcatcatcctctggctgtgcggagtgccgctggtcgtgatcatcggcctgaaggtcttcggcattctctgaatgaagaagtaagtaaagaacgacgaatcccggttcctcctcacggcgcaatactgcgtcgttaagcgctccctagtgagcgcttttttttgcagcctcgctcacgcggtgggcggggtcagtgggtttcgcggcgcagttgctgcacgtcttcatgcagagaccgggcccactcgcgacgttcgcggccgagcgattgctgcggctctccaaagcgcacgatggccaggagcgccggtgcgcgcagcgtgttccagagcgatgtcagcaggttgtcgtcgtcgatgtagcgtggcgcctggctggtttctcctgtggccgcatcggcaaagcgcagcgcggcgggcagcaccggtgcgccggaagaaatggcggcctgcaagaggttggcatgaaagggcagcagcccgtgaccgtcgctggtggtgccttcggggaacacgccgatgcggtcgccgctctgcagcgcctcggtcatgtggtgcaccacgcgcattgcgtcgcgccggcgctcgcgctcgatgtagagcgagcccgcgccggtggagagcgtgccgatcagcggccagtgcttcacgcccgacttggagacaaagcgcacgtggcacgcggcgtggatggcagtgatgtcgagccacgagaggtgattgcagatgagcagcaccggtccctccgcgggcggcgtgccctgcactttgagcgcgacgcccatgatctcgagcaggcgcagcgaccactgctgcacgcgcaggttgcgctcttgctgcgacaggcccggaaaggtgaagcggatggtccaccagccgccaagcgcgtgtcccaccgcatgcagcaggcgccagcaggccttcagcgaatgaaccatcgagatgtgagccctctttttattattcaaccatggaccacgcggcctgcgacgagggtgtggcgcgcccgcccctgcagcgggtagcccgcgaacggcgtgtgcttgccctggctcttgagcgcctcgggctgcacctgccactcgatggccgggtcgaagacgcacaggtcggccacgccgcccacggcgagccggccgatgccggtggccgcgtcggcggcggtgagcaatcgcgcgggtgcggagctgatgacctccagcgcgcgcgacatgccggcaccgctgcgctcgccccattgcagcgcgagcggcagcagcaattcgagcccggtggcgccgggttcggcttcggcaaagggcagcgtcttggcatcggcctcgaccggggtgtggtcggacaccagcgcgtcgatggtgccgtcggccagcgcgaccgagagcgcgtcgcggtcaccctgctggcgcagcggcggattgaggcgcgcgcggctgtcgaaaaagccgatgtcggtgtcgaccagatgcagcgagttgatgctgacgtcgcaggtgagcggcaggccctgggccttggccgcgcgcaccagcgccacgcccgcggcgctggagatgcggcacaggtgcacgcgcgcgccggtgctcttcatgagctcgacgatggtgaagatggcgatggtttccgccgacacgggcacgcccgagaggccgaggcgcgtggccagcgggccgctggcggccacgcccttgccaaggtcgcggtcttgcgggcgcagccacacggtgtagccgaaggtgctcgcgtagagcagcgcgcgctgcagcacctgggtgtcggcgagcggcacgtcggcctggctgaagccgatgcagccggcctcggtgagctcagccatctcggtgagcacgccgccggcaaggctgcgcgtgagcgcgccgagcggaaagaggcgcgcgcattgcagcttctcggcgcggaacttgagcatctcgaccaggccgggctcgtcgagcacggggtcggtgtcgggcgggcacacgaggctggtcacgccgcccgcaatggccgcggccatttcgctttcgagcatgccttcgtgttcgtagcccggctcgcgcaggcgcgccgccagatccacgaggccaggcgcgacgatgcagcctgcggcgtcgatggtgcggtcggccttgaagccggcaggcacgttgccgataccggcgatcttgccgtcggcaatggcgatgtcggctttcttgtcggtgcccgaggcggggtcgatgacgcggccgttggtgatcagtgtgttcatgcttcgttacctgcgacgatgctcatcacggccatgcggaccgcgatgccgaaggtgacctgcgggaggatcacgctctgcttgccgtccaccacggcggagtcgatttccacgccgcgattgatggggcccgggtgcatgacgatggcgtcgctcttggccagctgcagcttctccggcgtgaggccgtaggtcttgaagaactcttgcgacgaaggcagcagcgcgccgctcatgcgttcgttctgcaggcgcagcatgatgatgacgtcgcagtccttgatgccttcttcgagcgtgtggcacacgcgcacgcccatgccggccatgtcgctgggcacgagagtcttcgggccgaccacgcgcacttcggcgcagccgagcgtggtgagcgcgtgaatgtcggagcgcgccacgcgcgagtgcagaacgtcgccgacgattgccaccgtgaggttcgaaaaatccttcttgtagtggcggatcgtgtacatgtcgagcagcccctgcgtcgggtgcgcatggcggccgtccccggcgttcaccacgtgcacgtgcggcgcgacgtgctgcgcgatgaggtagggcgcgcccgactcgctgtggcgcaccacgaacaggtcggctgccatcgcgctcaggttggcgatggtgtcgagcagcgactcgcccttggtggccgaggagcgcgcgatgtccagattgatgacgtcggccgacaggcgcttggccgcgatctcgaaggtggtgcgggtgcgcgtgctgttctcgaagaacaggttgaacacgctcttgccgcgcagcagcggcaccttcttgacctcgcggtcgctcacgctggtgaagttggcggcggtgtcgagaatgtgcgtgacgatgtccttgggcaggccctcgatcgacagcagatggatcagttcgccgttcttgttgagctgcggatttcgcttgtagagcatcagcggttctcctcgaccttgaggctgaaggcaccgtcgttggcgcgtgcaagggcaagcagttgcgtggccggcagcgtgagcgtggtggcggcgaaatcggccgccacgggcagttcgcggccaccgcggtccaccagcaccgcgaggcgcacgcaggctgggcggccgaagtcgaacagctcgttgagcaccgcgcggatggtgcggccggtgtagagcacgtcgtcgagcagcagcacgtcggcgccgttcacgtcgaagggcagcgcggtctgcgcactggccgagaggccgcggcgcgcgaagtcgtcgcggtgcatagccgatgaaatgacgccgggggcgccactcaggcccaggtctttctgcaggcgctcgaccagccaggcgccgccggaggtgatgccgaccagtctggtttgggggcgcatcagcgctttcacgcctgccaacagatcgagatatagcaattcggcgtcaggaacgacagggctcacgatgatggctccaggacaaggcaagggggaaggcagatgcggggaacaccgtggaaccggctttgccgggccactggtgttgcccccggtgagggggagggagaagcgacacgaagtgcgcgaagcctgggggagagcttcattgttggaggctcctcaaaaattgttccaggatgatgcaggcggaggcggcatcggcatctcgggcacccgaggccagcgcctcggtggtgctgtagcgctcgtcgacctcgaacacctgcagattgaagcgcccgcgcagctggcgcgcgaacttcagtgcgcggcgggtgttctcgtgcggggcgccgtcggggtggtagggcacgccgaccaccagcgcgtcgggctgccattccttgatgcgggcctcgaccagcgcgaagcgggcatcgccctcggccttgatggtggcctggggggtggcggtgcccagcaggcggttgccgctcgcgacgccggtgcgcttcaggccgaagtcgaaggccaggaagctctggaagtgcgagggaacggcaacaggaacgggaacggtagaagaagcggagggttggggcgcgtcaggcatggcagcggccatcacgcgtgtcccgcttccggcgacagcgtccacgcttccaggcccagcagcagcagcgccctgtcgtagcgctgctcgaccggggtgtcgaagatgacggccgggtcggcactcacggtgagccagctgttttcagccagttcggactcgagctggccctcgccccaggccgaataacccagcgaaaccagcaccttgcgcggtccggcgccggtggccagcgcctccagcacgtccttggaggtggtcatttcgagcccgccgggaatggtcatggtcgaggcatagaccgattcctcgggcttttcggcatgggagaacaccggctcgtgcaggacgaagccgcgttcggtctgcaccggtccgccctggaagacgggcgaatcgccgagctcgggccgcacgaggtgaagttcgatcttctcgaacagctccttgaggttgatgtcgctgggcttgttgatgacgaggcccagcgcgccgcgctcgctgtgctcgcagaggtagacgacgctgcggttgaaagttttatcttccatccccggcatcgcgatcagaaagtgatgcgtgaggttcatcggggcagaatcggcagccatatgccgccgattttactggccgtcgacaagacctatcccaaaggactcatgtggtttcgccgcgaccttcgcgtggacgacaacgcggcgctctaccaggccctgcgggcctgccggcaggtggtgtgcgttttcgtgctcgaccgggcaattctggaccccctcccccgcgtcgaccgacgggtggaattcatccgggaatcgctggcggagctcgacgccgagctgcaggcgctcagcggcggcctgatcgtgcgccacgccgcagcggtcgacgaaattccggcgctggcgcacgaactggacgtgcaggccgtctttgccaaccgcgacgacgagcccgacgccctgtcgcgcgatgcccaggtgctcggcgccctggccaatgcgggggtggcctttcacacctacaaggattccaccgttttcgaccgcgacgagctgctgaccaagacgggccagccctacacggtgttcacgccctacaagcgggcctggctggccaaggtggactccttcttcctgaagtcctacccggttcgcacccacgccgaggcgctggcgccgccgcccgaggcctaccgggcgccggtgccgtcgctggaggagatcggtttccggaagagcaatctttccgagctggagattccgaccggcaccagcggcgcggcggcgctgttcgaagacttcttccagcgcatcgaccgctacgacgcggcgcgcaactttccggcggtgcggggaccgagctacctgggcgtgcacctgcgcttcggcacggtgtcgatccggcaactggcgggagtggcgcaccagctcgcgctgcagggcgacgcgggcgctgcgacctggctcagcgagctggtctggcgggagttctacttccagatcctggcgcactttccgcacgtgcattcgggcggcgaatcgaagagcttccggcccgagtacgacaagatccagtggcaccacggcaagcatgccgaccagctgttcgaggcctggtgccagggccgcaccggctaccccctggtggacgccgccatgctgcagatcaaccagagcggctacatgcacaatcgcctgcgcatggtggtggcgagctttctctgcaaggacctggggctggactggcggcgcggcgagcgctactttgcgctgcacctgaacgatttcgagctggcgtcgaacaacggcggctggcagtgggccagctccagcggctgcgacgcgcagccgtacttccgcatcttcaacccggtgacgcagagcgagcgcttcgaccccgaaggcaagttcatccggcgctacctgccgcagcttgcggggctgtcgaacgcggccatccacgcgccctggacagcctcgccggtggaattggaggcggcaggcatcaagctcggcgagacctatccccaccccgtggtggaccatgccgaggcgcgcgaaaaaacgctgcagcgctacggcgtggcgcgggccaaggcgctgcagaaataacaaaggggcccgagggcccctttgctttcttgatgaacgccggagggcgtcatgcagccgcggccagcgccggttcgctcgtgtacgcacgcaccaggcgcagcagttcctcttccgagtagggcttgccaaggtagtggttcacacccagcgtgcgggcgtagtcgcggtgcttttcggcgatgcgcgaggtgatcatgatgatcggcaggcccgccatggcgtcgtccgcgcggatgttgcgtgccaggtcgaagccgtccatgcgcggcatttcgatgtcggacagcaccacggccgggcgctcctgctggagccgttcgagcgcctgcaggccatcggccgcgagcgacacgcgatagccttcgcgctgcagcaggcgctgcgtcacgcggcgcaccgtgatggagtcgtccaccaccagcaccagcggaacctgcggcaccggcggagccagcaccggcaacggttcgtgcggcgcagcaccctcttcggccgagccgccatgcgcgggtgccaccagcgcggcagcctggcgcaggcgagcctgttcgccatgcaccgcggccagcgccaccgggttgtagatgagcgccaccgcgcccgaagccagcaccgagatgccagccaggcccggcaggcgcgcaagctgcggcccgaggttcttgaccacgacttcctggttgcccagcacttcgtccacgtgcaggcccacacgctgcgctgcgcttcgcacgatcacgacggtgttgttcttgctcgtggagtgttcgctgcgtgcagaggcctgcagcagtgcaccggcccagtagaacggcacctgttcgctgccgaacggatggctgttgtgcaggtaggcggcttcgagctcggtgctgctcacgcgctgcaccagctcgaccaggttggacggcacgccgatcgacacctcgccggcgcgcagcatcaccacgtgcgtcaccgcggtggtgagcggcagcaccagcttgaaggtggtgccctggccggccgtgctgtgcgtttcgatgcggccgccgagcgccgcgatctgcgcacgcaccacgtccatgccgataccgcggcctgccagctcggacacttgcccggcggtggagaagccgggcttgaagatcagctcggtggcttgctcgggcgacagttcctggtccgcttccagcaggccgagcgtgcgggcacgttcggcaatgcgcttgtggtccaggccggcgccgtcgtcgcggaagctcaccgagacgtcgttgccttcgtggtgcaggtcgatcacgatcaggccgttggcgtccttgccgaccttttcgcgtgcggccggctcttcgatgccgtgcgccacgcaattgcgcagcaggtgttcgaaggcaggcgtcatccggtcgagcacgccgcggtccatttcgatggagccgccgacgatgtccaggcgcacctgcttgccggtgtctttcgacgcctggcgcaccacgcggtagaggcgatcggaaatgccctcgaactccaccatgcgcgtacgcaggaggccgcgctgcagttcgcgcgtctggcgggcctgaacgctgaggtcgtcttccgtcgcctgcaccgtcttttgcagcgtgcgctgcacggtggccacgtcgttcaccgactcggccatcatgcgcgtgagttcctgcacgcgggtgaagcggtcgaactcgagcgggtcgaagctctgctgcgaatccttggcctgcgcgaggcgggactgcatctggctttcggcctgcacctcgatgtcgcgcaattgctggcgcaggcggtcgaggttgcccgtcaggtcggagagcgaaccgcgcagctggccgagttcggcttcgaggcgcgagcgcgtgatgatgacctcgccggtctgcgccaccaggcggtcgagcagttgggtgcggatgcgcacggcctgggtcgacaccgcgcgcaggggcgcaagcagcgcgggcgcggggcgcggcaggagcgatggcagggcggccgctcccgctgcggaggcggcgtcttcgctgtcgtcggcggaggccgctttttcgtcattggcggagacgccggattcggcgggaacctgcaccagctggacacccggcgaggtggccgctgccgttgccaccagctgggccacttcggcctgggtggcatcgtccgcggcacgcagcgcgtcgaaggtcgcctgcagcgcatcgaggcgcgtgagcagcttttcgatttcgacccggtcggcgccgccctgggtgcccagggcttcgatctcggattccatgcggtgcgcgcgctcgccaaggcgcatggcgccggccagccgggcgctgcccttgagcgtgtgcagcgtgcgcagcacggaggcgcgcggcgcgttgtcgtcggggtggtgcgcccactggcgcagcgcgtggcccagctggggcagcagttcctgcgcttcttcctcgaagatcgggaacaggtcgacgtcgaccgcgtccgccatgtcgatggcgtcttcggaatcgtccagcgccacgtcggccatgccgtcggaggccgccatatgctggtgcggccgggtctcgatgcgcgcagcagcttcggccggcatgggcgcggcagcgatgtcgcgcagcgcctggagcgtgccttcggaaggctcgcgcaggaagcccacggcaaactggtgcagcaggcggcgcagctcgtcggccgcggcaaccagcaccacgccctgttcgcgcgaaccgctgccctgcatttgcagatgctgcagcgcggcttcgagcaggcgggccatgcccgagaggctgtggaacccgaccgtggccgaactgccggccagcgaatgggccagcgcgacggtcgaatcggacagccgctcatgggattcgagcgcccactcgccgacttcggtggccagttgcctggaccattcgtcggcttcgttgaggtagacgttgtagagcgcgatgccgatgcgcagcggcccgatgaccttgacctggtcttcggcacccgacacggcagcggccacttcggtggcttccgtggtgtcggcggtttccgggacctcgggctgcgggacttcttcggccgccgtggcaacagccggctcgtcggccaaggccggtgcttcgcccgccgcgaccacggcaggctcttcgggctccagctgcaaagctggcgcttccacgatctcttcggccggcgttacttcgacggcaaggggcacgggctcttgagcgatgaccggtgccggctcgggcgcccaatcaaggtcaggcaggccgtccagcgccggcagctcgggcacgggctcaggcgacggttcggcagcggcttcggccaggaacgaagcggcggtttccggttccgccttggccggctccaggaagtcgaacttctcgccggcggcccagacaggctcgtcggccggggtcggcttggattcgaagtcgaggaagtcggtcgacgtgaagtcgtcttcgggttcgggctttgcggcctcctgcggtgcctctgcgggcagttcgaacgcggcaacgggtgccggctcgagcggtgccgccgtggggaacgacaggtcgggcagttccgggagttccggcatcggaagcggggcaaccgccggcggctcggcggcaatgtggcgcgcggccacggccagagcctccgcatcggcgacacgcgccggcatggtgggcacgggctcgcccgccagcagggcattcgccacgcggctgaagtgcgacgactgccagccatgctgcgagcccgaagcgatggcttcgacccattggctgaactcttcgagcgccttgcgggtgccgacgagcagatcgggcgtggcgtcgcgctggtcggccagccaggtgttgagcacctgctcgaaagaccaggcggcgtcgccgaagtcggtcaggccgaccatgcgcgaactgcccttcagcgtgtggaacgcacgccgcaggatggtgagttcctcggtgtcgtcggggtgactgccgagctcgtcgatggcggccaggccgttttgcaccacctcgcgggcctcgtcgaggaagatgttctgcaggtcgtcttcttcgagttcggtgacttcggtgtcaggcagcgcggcaggaccggtgatcttgttcgtccagctgtcggccttgcggctgaattcctcgatgggcgacaccttcgccttgcggttgggcgtggcgagcgcggcgagcttcgacgcaatctgggcgtcgacttcctcgatgctgagcacggcatcgccaccggtggcggcacccggtgccgcggcatccgccgtggcgctgtcggtggcctggcggcccatcagcggcttgagttcgccggcttcctggtcgaacacgaacaggcgcttggcgagcgtgggctggtagcccagcatgtcgatcaggaaacccagcgcgcccaggttgttgccgagcgcgtcgaagctctgcatctcttccactggcgacgcattgcccaccagcatctgctcgacatcgtcgcgcatgcgctggacggtgtgggcggcctgctcgagcccgagcaccgagaacacgccgcgcatctgcagcagctgggtcggaacggtgcgcagcaggcccttctcggccggccggcggaaatactggtcgagcgacttttcgagttcgctcaggtggctgcggagttcgtcgaccacggtacccatggtctggcgatcgctcacgcggcgatacaggtcctccatccagggctcgagcggctccgaatggccgccttcgcgcacgcgctcgatgcggcccgccagttgaagggtgcgggaggtgagttgcggatcgctcgggtcgaggtcttcgagcgcggcttccaggtagagcaccgaggtggcgacttccatcgcaagctcggtatccggcggctggccggaacgcacggaggcttcgaccgcatgcgtgagtgcgtccaccatcggcaggatcggcggatgcagcctctgcagcgactcgccgagctgtgcgaaggtgtcggccacctggcgcgtgcgggtgatgtcgccgcccgaaagcgccgaccacatttccttggcagtttcgatgcgcttgcgggcctgggcgagcaccagcggatcgaagcggccgaactgttcgacgctgtagtcgacacgcggctcgcccgcgacgccccaggcggcgcgcacggtgcgcagcgtggcggcttcgtcggagtcggcggcgggtacggcctgcgcgcagaagaacagcaggtcctggccgaggcggtcggaaaccgcgctgtcgccgcgcgccagcgtggcgtattgcagcagcacgcgcgaggcggcgcgcttgacgtaagaatcggcggggatcagctccagcgccagggcttcgaaaaagcccgcggcgagggtccagaaacttgcgacgcggggcagcagcgcaccgcgcccgagccccaggcacagcgcctgcagccggcgcgcggcctgcgggtcgccggtcttgaccagctgcagcacttcgcggtcgagccgcgagcgcacggccgggtcataggccagcgcggcctgggtcagcgcgggtcgcacttcgacccagcgccacgcaacgctccagagatcggccggatggacgcgctcgttgccgaccagttcgagcacgtcgcggtattgcggaaacagcgcgaccgacgacacggccttgccggccagcagcgcgtggagaaaatcgacgacggcaaagccggcgcgctcgatcttcaggaccgcgctgtcggtgcagcgctgcggttcggcaatgaagccctgcaccgcgaattcgatggagccgagcaccagcgcgggggcgttgttgcccaccatctgaagcgcaccgacggactggtgcagttgctggcgagccatttgcagcgggccgctctcgagatccgaggcactgcccacgtcgcgcacgaagcgccgcagcgacttgcccacaccatcgagggatttctgaatttctcccagcacccaggccagcggcccgaggtcttcggtggccggcacgttgccggcaatgggggccgtggcaggggtttgaatcgacacgttggatgctcgccgttcttatcttttgtcaggcaatcttgaatcgggcgaccgagcggcgcagttcttccgccatctgcgaaagctcgcgcacctgctgggccgtggtacgggtaccttctccggtctgctcggtcaccgcaaaaatgtgctggatgttggcagccaccacgttggcggaatcggcttcgcgggacgcggattgcgaaatctgctcgatgaggtctgcaaggcggcgcgacacgcggtcgatctcggtcagtgcggtacctgcattgtcggacagcttggccccttcgaccacaccctgcgtggagcgctccatggcgcccacggcatcctgcgtgtcggtctgaatggccttcaccagcgccgagatctggcgcgtggcgtctgcggagcgttcagccagccgctgcacttcttccgccaccaccgagaagccgcgaccggcttcaccggccgatgcggcctggatggcggcgttcagtgccagcacgttcgtctgttcggtaatgtccgagatcagctcggtgatttcaccgatctcctgcgaggattcgcccaggcgcttgatccgcttggaggtttcctggatctggtcgcggatggagttcataccgccgatggcgttctgcacggcctgcagacccgacgatgcggcttgcagcgactggcgcgccaccgtggcggactcttgcgcttgcgaggacacgccgttgattcgctcggccatggtcagcaccgactggccggtttcgcgaatttcgcgcagctgttcggtcgaagcggccagcagttcggtcgaggtgctttccacctgcgacgtggtttgcgccacgcgggtggccgtgttctgcacgttgcccaccagcaaacgcagttcttccaccgtgtagttcaccgagtcggcaatggcgccggtgatgtcctcggtcacggtggcttcctgcgtcaggtcgccttcggccactgtctgcagttcgttcatcagccgaagaatggcagcctggttggcgttgttgatgcggccggcctcgtcgctggcctgttcggcagcaagacgttcgcgttcggcgacggcggcacgttcgcggccttcgcgcacctgcacgaaaccgatggcgccggccagagccagggcggccagcgagagcacgaacagcatcacgatcgttccggcgcccaggccggtgcgggcggagagcttgtcctgcagttcgccgagcgatttacgcagcggttcgctgtcggtcaggatggaagcctgcgcttcgcgtgcggccaccagaccctgcaggttgcccagaatggcggacgcctgcgtgcgcatctgctcataggtcttgagaatggcttcgagctgctggcgggtctgcgggtccttcgagccggggaaacgctgctgcgcattgccgtcgagcaggccgcgcgtggtttcctggaaggtgttcaagtccttgccgagcaggaacacggcgtcggggttcacgccttcgaccgtgaagaattcgttggtcgacttgccgatgcgctgggtcagcatcacgagctggccggcggccgagatttcaggcaacgtggcgttctgctgcatcttgagcgatgccacggtttccgtcatttcgagcagcgcggacgactgctggttgatgtcgcgcaaggcggcacccacctgcgtcaggatctggcgctgggccagcacggccttggcgctggcgtcggcacgggcgaccagcgggttgatcttgcccatgtcctcgtcgtactggttgcccacgcgttcgaggcgcagggcatcgtcgccgttggtcaggccctgcacgcggcgcgtgaggtcgtcggcgctgtccttcacttcgacgaaagcgggcgcgctgccgacgagtgcctgcgagatcgactttgcaagccgctgcgactgcatcagcgactggccggtggcggccacctgctgcgcaaggcgctcggcgcgaagaatggcggagccggccaccagcaacagcagcagcaccacgaccgccagcatgatcgccaggatccgctgctggcgcgccgggttggagcccgttcgtcccgcggcagcctgcgcggcttcggcagatgcggcatcggcctcgttggcggcctcgccgaccagcgtggcaccgtcggcaaagccggtgggcaccggctcgctggaggtgcggccttgttttctggcgaggcggacggtcttttcgtccggcacctgaaccgtgtcgacgtcgtcgagcgatatggtggaaccggagccgtcgacgcgggccttgtcgttgccgctttgagcgggcagtaatttcttgaacttgtcggcgatcgagctcacggtcggtccttcaggtggttgtcttctggctgtgcggatgcactaggcgccaatactcaaaaactggggttgctgcgagagcgcctgcaggttgatttcctgccagcgctcacccgccgcatcggtgaaaagatgcccgagccaggcgggtgcatctgcgcctgggggttccgcgcccgtgaaggcctcggccccccgcaaccccgccagtcgatcgaccagcaaagcgcagttgacttcgagcagctcgttgagggcaacgagccgcgattgcatgcgggccgcctcggtggccgcaaggccatcggacgtgccggaggcgaatgccgacagctgcaccacgccatagaggccgccgcgcaggttggcaacgccgaggaaccagggttccgtgtagggcacgggctggggcggcgtccaggggaagatctcacccgcgtggcccagtggaaagaggtacttgccctcaccggcctcgaccgcgagccacgtggcggccacgccggtggtgcgagcagcctgcaggcggctcgcaagccgggactggaaggctcgaagagcgtcgcgatttgccatggactcggcagtcttccgttcaggccagcgcgctgatcttggacatcagctcggccgcgttgaccggcttcacgatgtagtcgcgggcgccctggcgcatgccccagacgcggtcggtttcctggttcttgctggtgcacaggatgatcggaatggcggcgtactgcgggtcgcggacgatggcgcgcgtgagctggaagccgttctggccgggcatgacgacgtccatgaggatcaggtcgggctggtcctcttcgagacggcgcatggcgtcttctgcgttttcggcggtcttgacggcaaagccgttcttctggagcaggtcggacaggaacagcagttccgtcttggagtcgtcgacgacgaggatttttcgaatgggcattactgcgcttcctgttgaacgatgccaaactgctgcacggcctgcagcaattggtctttggtgaaaggtttggtcaggtagtcttgcgatccgaccatgcggccgcgggccttgtcgaagacgccgtctttcgaggaaagcatcaccaccggaacattggagaactgagcgttgcgcttgatgatggcgcaggtctggtagccgtcgaggcgcggcatgaggatgtcgcagaaaatcagatgcggcttgtggtcgttgactttcgagagcgcgtcaaagccgtcctccgcaaggagaacttcatgtccgccctgcttcagaaatatttcggcactgcgccggatcgtattgctgtcatcgatgaccagcaccttgtaacctgatccattcggccccattgcacacactcctgctgagatgagacttggatgcccgccgcaccgtacatcggcgcagatcgcgtagccctatgccatgcttcagatttcaaccatttcgaagtcttccttgcgtgcaccgcactcaggacaggtccagttcatcgggacatcagcccaggccgtgcctgctgcgatcccatcttccggtacacccaccgcttcgtcatagatccacccacaaatcaggcacatccaagttttcgtattcatcggagcttaaagtccttgttcattaaatgcaacgagtgtatctatgcgtatctcactggcgggcggtaaacgtcgcgcctatgccaccattgaggcgatttcggccggcgtatgaccatttacttacattccgcagacaacacccgcaaaccgggcaatcttaacgaccctccgccggacgctgaagaagcggccgaacgggacctgaatccgccctgcgttctggtcttcaatgccagcgatccgagcggcgccggcgggctgggggccgacgccctggccatggcctcggtgggtgcgcacatgcttccggtggtcactggcgcctacgcccgcgacacggccgagatattcgaccatttcgccttcgaggaagaggccattgccgagcaggcgcgcgccatcctggaggacgtggaagtccagctcatcaaggtgggctttgtcggcagccccgacgcgctgagcaccatcgccgagaccgcatccgactatcccgaggtgccgctggtggcctacatgcccaacctttcgtggtgggacgagaacctgatcgagccctatctggatgcttttcgagagttacttcttccgcagaccacagtgttggtgggaaaccacagcaccctctggcgatggctgcttcccgactggagcggcgagcgtccgcccggtgcgcgggacattgccaaggccgccggcgagttcggcgtgccctacacgctggtgaccggcatggtgctgcccgaccagttcatcgacaacgtgctggcctcgccgcagtcagtgcttgccaacgaaaaatacgagcggctggaggccgtctttgccggcgccggcgacaccctgtcggccgcgttggccgccttgctcgcaagcggcaccgacctggtggccgccaccaccgaggccctggcctacatggaccgctgcctggacgccggattccggcccggcatgggccacgtgcttcccgaccgcctcttctgggccgagccggaagatgaagacgatgacgacgaagaccccgacgcagcccccgatttcgccctgccccctcacgacaccagacattgatgccaaacgctgaccaaaacgacattcttttcgagcgcgcccgcgccgtcattcccggcggcgtcaattcgccggtgcgcgccttcaaggccgtgggcggcacgccgcgcttcatccgccgtgccgagggcgcctatttctgggacgccaacgacaagcgctacatcgattacatcggctcctggggtccgatgatcctgggccatggccacccggccgtggtcgaggcggtgcagaaggccgtgctcgagggcttctcctacggtgcgcccaccgagcgcgagatcgagctggccgaggccatcctcgccctggtcccgtcgatggagatggtgcggctcgtgagttcgggcaccgaggccgccatgagcgcgctgcgcctcgcgcgcggcgccaccggccgcaagcacatcatcaagttcgagggctgctaccacggccatgccgacgcgctgctggtaaaggccggctccggcctcgccaccttcggccaccccacctcggccggcgtgccgcccgaggtcactcagcacacgctggtgctcgagtacaacaacatcgcgcagctcgaggaagcctttgcgctgcacggcaacgacatcgcctgcctcatgatcgaggcgattgccggcaacatgaacttcgtgcgcgccacgcccgaattcgccgcccgctgccgcgcgctttgcacgcagcatggcgcgctcttggtgttcgatgaagtgatgaccggctttcgcgtgggcctgcacggcgcacagggcgtgctgggcatcacgcccgacctcaccgtgctcggcaaggtcatcggcggcggcatgccgctcgcggccttcggcggcccgcgcgccatcatggaacagctcgcgccgctcgggccggtctaccaggccggcacgctgtcgggcaacccggtggccacggcctgcggccttgcaacgctgaaggaaattgcgcgccccggtttctacgaagcgctgtcgaagaagacgcgctcgctggtcgacggcctgaaggccgccgccgcggctgaagggcagcccttcaacgccgacagcgagggcggcatgttcggcttcttcctgatgaacgagttgccgcagaactacgccaaggtaatgaccaccgacaacgcgaagttcaacgcgctgttccacggcctcctggaccgcggcgtgtacatcgcgccggcgctctacgaagcaggcttcgtgagcgccgcgcacagcgacgaagacatcgctgccaccgtcgaggccgcacggcagatcttcaaggcctcgcagccccgttgatcgtgatcgcctgcgggcgcgaggtcagtggcggaagtggcgcacgcccgagatcaccatgaccacgccgcgctcgtcggcggcatcgatcacttcctggtcgcgcatcgagccacccggctgaatgacgcagctcgcgccggcatcgaccaccacgtcgagcccgtcgcggaacgggaagaaggcatcgctcgccaccgcggtgcccttgagcgacaggcccgcatgctcggccttgatgctcgcgatgcgcgccgaatccaggcggctcatctggcccgcgcccacgcccatggtcatgccgccggcgcagaacacgatggcgttgctcttgacgtacttggcgaccttccatgcgaacagcaggtcttgcagctgctcgggcgtgggttgcttcttcgataccaccttgaggtcgctcgccgaaagctcatggttgtcggcagtctgcatcaagaggcccgagccgacgcgcttgacgtcgatcgcattgcggccgttgtcccaatcggtggcgccacccttgggcagggcaatctcgagcacgcgcacgttgagcttggccttggtcgcctggaacacttccagcgcctcgggcgtgtagcccggcgccatcagcacttcgacgaactgcttggcaatggcctgcgcggtttcgccgtcgaccggacgattgaaggcgatgatgccgccgaaggccgaggtcgggtcggtcttgaaggccttgccgtaggcttcggccgcatccttgcccacggccacgccgcaggggttggcatgcttcacgatcacgcaggccggcacgtcgaagctcttcacgcattcccatgcggcgtcggcgtcggcgatgttgttgtagctcagttccttgccctgcagctgcctggcggagacgagcgagccgggcgccggatacaggtcgcggtagaacgcggcctgctggtgcgggttctcgccatagcgaaggtcttgcaccttcacgaagcggccgttgctttgcgccgggaacagcgagcgcgtgggcgcgggctgtccgatgctggcgtcgaagtcgatggccgagaggtagtcgctgatggcgccgtcgtagtcggcgatgcggttgaacgcggccaccgagaaagcgaacttggtcttgtcgctgagcttgccggcggcctggagctcggccagcgccacggggtattgcgaggcgtcggtcagcacgcccacgtccttccagttcttggccgcgctgcgcaccatggccgggccgccgatgtcgatgttctcgatggcgtcttccagcgtgcagccggccttggccaccgtggcttcgaacggatagagattgaccacgagcaggtcgatggtgtcgatgccatgttccttgatggccgccacgtgcgccggcagatcgcgccgcgcgagcaggccgccgtggatcttgggatgcagcgtcttcacgcggccgtcgagcatttcaggaaaaccggtgtggtcggccacttcggtcacgggcaggccggcatcggccagcagcttggcggtgccgccggtggacagcagcttgatgccaaggccgtgcagtgcttgcgcgaattcgaggatgccggttttgtcggagacggagatgagtgcggtctgggccatggaatatgccgtggagttatttcaaaagtttgtgttcaaccagcttcttgcgaagcgtgttgcgattcaggcccaaccattgcgcggccttcgactggttgccctcggcgcgcgtcatcacgacgtcgagcaggggcttctcgaccacccgcacgagcatttcgtacatgccgtcgggttcggtgccgcgcaaatcgcgaaagtagctgtccagactggtgcgcacgcagtcctcgatgtgtttcttgctcatgctttttcttctcttcttctctctcaatcagcggcgcaggccgcctcctcttcacctgacagctcttcggccgcctggtgcacgggcatgcggtccatgcggtccgccaacccgtcgaaataatcgccgaccgcgcgcagttgcgccgtcgagtcttcgatggtgttcatccgtgcgcgaaaggcttcgccgtccggcagcgtacgcacataccagccgatgtgcttgcgcgccgtgcgcacgccgctgaactcgccgtacagcgcgtagtgctccaccaggtggtcgagcagcaggcggcgaacctcggcaaccaagggcggtgcaaggtgcgtgccggtctccaggaaatgagagatctcgcgaaagatccagggccggccttgcgccgcgcggccgatcatcaccgcgtcggcaccggtggcggcgagcacgtcgcgcgccttctcgggcgagcggatgtcgccgttggccaccaccggcacgcgcaccgcggccttcacggcggcaatggtgtcgtactcggcgtcgcccttgtagccctgctcacgcgtgcggccgtgcacggtgagcatctgcacgccggccgattcgaaatcgcgcgcgagcttcaccgcgttgcggtgctcttcgctccagccggtgcgcatcttgagcgtgaccggcacgttgaaaggtcgggccgcatcgaccacggcgcgcacgatctcgagtgccaggggctcgtcgcgcatcagcgcggatccggcccacttgttgcagaccttcttggccgggcaacccatgttgatgtcgatgatctgcgcaccgcgctcgatgttgtagaccgtggcctcggccatcatggccgcatcggtgccggcgatctgcaccgcgatggggcccggctcgccgtcgtggttggcgcggcgcgatgtcttgagcgtgttccagagttccttgcgcgaggtgaccatctcactgaccgcgtagcccgcaccgagcgcgcggcacagcatgcggaagggccggtccgtcacgccggccatgggcgcgacgaacagccggttttccagcgtgtgggtgccgatctgcaaggtcatgagagggaaagtgtcgcgcgttcggctgctgaaaaatgaggcacgattgtagccacgcgccgtttcgtcgactgaaacgatttgcgcccggggtaccggcgcaaacacccttgtgcacggcgctttttccgactgcgatctgaaaacgcactgcctatactgcgtcgactcatttcaccctatgcaagcctggctcgacgctcttctcgcgctactcgcgcttccgcagtacggactctccacgctgttcattgcggctttcgtctcggcaacgctgttgccggtgggctcggagccgattcttttcggcctgctcaagctcaatcccgacatgttctggtccgccgttgcggtggcaacggtgggcaacacgctgggcggtgcggtcgactggggaataggctatggcgcgcacaaggtggccgacaaatactcgcactcgaaacatcatgtgcgcgtattgggctggctggaacggctcggcccgaaggcgtgccttttgagctggctgccgatcgtgggcgatccgctgtgcgcggtggcgggctggctcaagctgcccttctggccgtgcctgggctacatggcgattggaaaattcctgcgctacgtcaccatgacggtcgcgctgctctacgtgtttccgtcgtgatgccgccgctgcggcttcagctcaggaggccgtaggggccgccgcgttccagtgcccgctggtaggcggggcgcgcatggatgcgctgcaggtatgccatcagcctgggccgcttcgcatcgaggccgccgcgcgcctctgcggcttcgaccgggaagctcatctggatgtcggcacccgtgaattcgttgccggcaaaccactcgctcttgccgagctcggcttccatgaagttcaggtggctctcgatattcggcgtgacgatggccgccttggccttgcccgcaatcatcttggcaatcggcttcgcgaagaaaggcatcttgccgttctcgatcttgtcgaacaccagcttgagcagcagcggcgacatggccgagccttcagcgaaatgcagccagtagcggtagcgcacggcctccggcgtgcccggcacgggcgccagccggccattgccatggcgctcgatcagcgtctcgatcacggcgcccgattccgccagcacaagaccgtcgtccgtcgtcaccaccggcgacttgccaagcggatgaacggcccgcagcgaagcgggcgccaacatggtctgcggatcgcgctggtagtgaacgatttcgtagggcagcccgagttcttcgagaagccaaagcacgcgctgcgagcgcgagttgttgaggtgatggacggtgagcatacggcgacaggtgcttgaaagaaggggcgtgccttttcgcgaaacaccgcggaaccggcttcgccgggccgctggtgttgcccccggtgagggggttggcgtagcgacacgaagtgcgcgaagactgggggtgagccagttacgaactgaagaggaagttcatcacgtcgccatccttgacgacgtattccttgccttccgaacgcatcttgcccgcgtccttcgcgccctgctcgcccttgtaggcgatgtagtcctcgaaagcgatggtctgggcgcggatgtagcctttttcgaagtcgccgtggatcacgccggcggcctgggggccggtgtcgccgatgtggatggtccaggcgcgcacttccttcacgccggcggtgaagtaggtctgcaggcccaagagcttgaaggccgcacggatcaggcggttgaggcccggctcgtcctggccgatttcggcgaggaacatcttcttgtcctcgtcgtccatctcggccaggtcggcttcgatcttggcgcagatggcgaccacgggcgcgccttgcttggcggcgtattcgcgcaggcggtccaggtaggggttgttctcgaagccgtcttccgccacgttgccgacgaacatcgcgggcttggcggtgatgagcgtgaacgacttgaccagcggcagctcttccttcgtgaactcgagcgcgcgcaccggcgtgttctcgttcagcgcggcctggcagcgttcgagcaggccgacgagcttctgagcgtccttgtcgcccgagcgcgccaccttggtgtggcgatgcaatgccttctcgaccgtggccaggtcggccaggcagagttcggtctggatcacttcgatgtcggagatcgggtcgaccttgccggccacgtggatcacgttgtcgtcgtcgaagcagcgcacgacgttcaccgtggcgtcggtttcgcggatgtgcgcgagaaacttgttgcccaggccctcgcccgtgctggcgccggccaccaggccggcaatgtcgacgaactcgacgatggcgggcaccacgcgctcgggcttcacgatctcgctcagctgcgcgagccgcggatcgggcacttccaccacgcccacattgggctcgatggtgcagaacggatagttctccgccgcgatgccggccttggtcaacgcattgaaaagggtggatttaccgacgttgggcaggccgacgatgccgcattgcaaactcatggggggtcctcttgggtaaccggcgattttaagggacgcggttctgggacgcgggtcgcctggttccgcggggcattcgaagtaggaacaccatcagggtaaaaccggattagcaaacgtttgcgcaaacgttttcgttggttaatatcggcgtccccggcaagagaccggcgcaccgctcaacccccctcaggagacaacacccatgaagttcacccgccgtacgctgcaaagcgcagccgccctgacgctgctgggcgcccttgccgcctcgcccgccctcgcgcaggacaagcccaaggtcgcgctggtcatgaagtcgctggccaacgagttcttccgcaccatggaagacggcgccaaggcgcaccagaaagcgcacgcctcgcagtacaccctggtggccaacggcatcaaggacgagaccgacacggcggcccagatcaagatggtcgagcagatgatggcgcagaagatcaacgcgctggtcatcgcgccggccgattcgaaggcgctggtgccggtggtcaaggccgccatcgaccgcggcatcctggtggtcaacatcgacaaccagttcgacaccgccgcgctgaaggaaaaggccatccaggtgcctttcgtcggccccgacaaccgtgccggcgccaagctggtcggcgacgagctggccaagagcctgaaggccggcgacaaggtcggcatcatcgaaggcgtctcgaccaccttcaatgcgcagcagcgcaccctcggctaccaggacgcaatgaaggccgctggcgtgacggtggtgggcgtgcagtcgggccagtgggaaatcgacaagggcaacaccgtggccgccggcatgatgcgcgagcatcccgacctgaaggcgctgctcgcgggcaacgacagcatggcgctcggcgcagtcgctgcggtcaaggccgcgggcaagaccggcaaggtgctggtggtgggctacgacaacatcggcgccatcaagccgatgctgaatgacggccgcgttcttgccacggccgaccagttcgcagccaagcaggcggtgttcggcatcgagaccgcgctcaaggcgctggccgaaaagaagccccagtcgagcatgcccgccgaagtgaagaccgacgtggtgctggtcaccaagtcgtcgtcgaagtaaatgttgctcgcccccagtcttcgcgcacttcgtgtcgcttcgccaaccccctaccgggggcaacacctgaggcccggcgaagccggttcctcggtgtttctggaatgaggtggtcaccgtgactgacgcccatcgcagtacgccggtgctctcgctgggcgcgctcggcaaggactatgcggcgccggtgctcgacgacgtttctcttgtgctgaatgccggcgaggtgctcgcgctcacgggcgagaacggggccggcaagagcacgctgtcgaaaatcgtctgcggcctcgtgcaaccgacacgcggccagatgctgctcgacggcgtgccgttccagcccgcatcgcgccgcgatgccgaacgcctgggcgtgcgcatggtcatgcaggaactagggctggtcaccacgctgtcggtggccgagaacctgctgctcgaccggctgcccaaccagaccggctggatccgccgcggcaggttgcatgagctggccgcgcgccagctcgccaagatcggcatgcagaacatcgacccggccacgcccgtggcgcggctgggcatcggccagcagcagatggtcgagattgcgcgcaacttgcaggacgacacgcgcgtgctggtgctggacgaacccaccgccatgctcacgccgcgcgagacctcgcatctcttcgagcagatcgaactgctgaaggcgcgcggcgtggccatcgtctacgtgtcgcatcgtctcgaagagctgcagcgcatcgcggaccgcgtggcggtgctgcgcgatgggcgccttgtggacgtgcgcgccatggccggcgtgcgcgaatccgagctggtgcagcgcatggtgggccgcgcggtgcacgaacacgaagggcgcgaccgccgcgtggccggaccggtgctgctgagcgcgcgcggcatcggccgcgcacaggtcgtgcgcgatgtcgacatcgacctgcgcgcgggcgaagtcatgggcctcgcgggcctggtcggctccggccggaccgaactggtgcggctgctgttcggtgccgaccgcgccgaccgcggtgaaattcttctctacgacggcacatccaacccgcagccggtgcagagcgcccgcaagggctggcgctcgccgatgcaggccatccgcgcgggcatcggcctggtgaccgaagaccgcaaatcgcaagggctgctgctcacgcaatcgatccgcgtcaacgccacgctgagcgacctgggcgcgatctctcgcgcgggctggctgcagcgtgccagggagcgcggcattgcgcggcgcctggtggaactgctgcgcatccgctcacgcagcatcgagcaaccggtggccacgttgagcggcggcaaccagcagaaggtggtgttcgcgcgctggctgcaccgcgaatgcaaggtgctgctgctcgacgagcccacgcgcggcgtggacgtgggcgcgcgtgccgatctttatgccgaactcgaccgcatgaccgacgccggcaaggcgctcttgatggtgtcgagcgacctgcgtgagctgatggccatgtgcgaccgcatcggcgtgatgagcgccggccggctggtcgcggtgttcgagcgcggccaatggagcgagcaatcgctgctcgccgccgcattcaccgacgcggcaggacgcaacgccgccgcgacgaccccgacggcgggatccgccatttccgattcgaatccggcccaagcggccaccgccgagacaccatgaacgcagccgctgctacacccgccacgacatccgctccgccctccgctctcaagggccagctgggcacctatctcggcttgacagtggtgctcgtcggcatgatcgcgctcttcggcgcgctgagcgaatacttcttcacgcgcgaaaccttcatctccattgccaacgaaattcccgcgctcgcggtgatggctgtcggaatgaccttcgtgctgatcatcgcgggcatcgatctctcggtgggctcggtgttggcactcagcgcagcagtgacggccgccgccatccttcagtggaagctctcggtgccgatggctgccgcgctgggccttgccacggggctggtgtgcggcaccgtgacgggtgccgtgtcggtcgcgtggcggctgccgagcttcatcgtctcgctgggcatgctcgaagcggtgcgcggcggcgcctacctggtgaccgattcgcgcacgcagtacgtgggcgacgccatctcgggcctggcggctccatgggtcggcggcatctccgcagccttcgtgctcgcggtggtgctggtggccatcggccagctggtactcacgcgcacggtcttcggccgccacgtggtgggcatcggcaccaatgaggaagccatgcggctcgcgggcatcgacccgcggccgatccgcatcatcgtgtttgcggccacgggcctcctggccgggctggcggggctgatgcagtcggcgcggctcgaagcggccgaccccaatgccggcgtcggcatcgagctgcaggtgatcgcggccgtggtcatcggcggcaccagcctcatgggcgggcgcggctcggtgatcaacaccttcttcggcgtgctgatcatcgcggtgctcgaggccgggctcgcgcaggtgggtgccagcgagccgagcaaacgcatcatcaccggcgcggtcatcgtggttgcggtgatcatcgacaccttgcgccagcgccgtgccgaccgccgcctggcctgaagctgccaacaaggggaacacgccatggccaccatcaaggacgtcgcgctgcgcgcgggggtttcggttaccaccgtctcacatgtggtcaacgacacgcgccacgtgagcgccaagggccgcgagcgcgtggaagaggccatccgcgaactgggctacgtgcccaacgcgatggcgcgcagcctcaagagcaacaccacgtcgacgctcggcatgctgattccgaacagctcgaacccctacttcgccgagatcgtgcgcatcgtggaagaccgctgcttcggcgccggctacacgctggtgctgtgcaacaccgacgacgagccccaccgccagagcgtgtacctgcaggtgctggccgagcgccgcatcgacggattgatcgtggtgtcgaccggggccggcgatgacgactcgctggtcacgcaactgcacggcctgcgcattccgaccgtgctggtcgaccgcgagattgccgacccggcctgcgacctggtggaaacggcccacatgcagggcggcctgctcgcggtgcggcacctgctgtcgctcggccacaagcgtattgcctgcatcggcggaccggtgggcgtgatgccgagcgagcagcgcatcgagggctggcgcatggcgctggccgaaggcggcgcggcaccgaatgccgacgcgctgctgtggcgcggcggcttcacgagccagggcggctacgaggcgatgcacgccatcttgcgcaccgagcaggcgccctcggccgtgttcgtctgcaacgacctgatggccatcggcgccttgcgcgccgcgcatgaaagcggcgtgcacgtgcccgacgacctttcgatcgtcggcttcgacgacatcgaactttcggcctacaccagcccgccgctcaccaccgtggcgcagcccaaggaacgcatcggcgcgctggcggtcgacatgctgctggagcgcgtgggcggcaagcggcgcgacgcgcgcaaggtggtgctgcagcccgagttgcgcgtgcgcgcctcgaccgcgcggcatgcgagctttcgcgaagccgccgccccttctgcgccctcttcttcgccctcttcttcgtccgcgtcttcgtccccggaaaaccgaaagtcccgcgccccgtgagctcaacgcctcctccttcttcttccagcgccgccgagccgccgcgcatcgtggtgctcggcagcctgaacatggacatcgtgctgcgcgtgccgcatgcgccggccgcgggcgaaaccctgctgggccattcgatcagccacattccgggcggcaagggcgccaaccaggccgtgagctgcgcacgcgaaggcggccgcgtggccatgatcggctgcgtcggcaacgacgcgcatgggcaggcgctgcgcgaagcgctcacgcaggacggcatcgacaccgccgcgctgcgcaccgccagcgccgagcccacgggcacggcgctgatcctggtggaagacagcggccagaaccgcatcgtgatagtccccggcgccaacgcgcaggtcgagatcgacgaggccgcgctgcggcagcagctgcaggccgcggccttcctggtgacgcagttcgagacgccgatggaccaggtggcgcgcgccatctcggtggcacatgacgcaggctgcaaggtgctgctcaacccgtcgccggtgcagcccatcgccgagcccctgtggccgcgcatcgacacgctggtcgtcaacgagatcgaggcccacgcgctgtgcggccaggcggccgacagcccgcaggaggccgcgctcgcaggccaggccctgcgcgccaagggcattgcgcgcgtggtcgtcacgctgggcgcgcgcggcgccgtggccatcgacgccgatggggctcgccaccatcccgcgccgaaggtgcaggcggtcgataccactgcggccggcgacaccttcctgggcgcgctggcggttgcactcggcgaaggccagcctttcgacgaagcggtgcgtctgggcatccgcgcggctgcgctgtgcatccagcagcccggcgcccaaccctccattccgcagcgcgatgccgtgctgcaaagccccatgcctcccgactggatcgcgctgtgaaacgtaccgccctgctcaacgccgaactttcccaggtcatcgcctccatgggccatggcgacatgctggtgatcggcgatgccggcctgccgattcccgatggcccgcggcgcatcgacctggccgtgacgcgcggcgtgccgctgctcaccgacgtcttgcaggccgtgctgtccgagatgcaggtagagggcgtggtggtggccgacgaggcgctgaatggcgccaaggttctgcccgcctggtacccgcagtcgctcggcatcgcgccacagactgtctcgcacgaggagttcaagcggcgcagcgcgacggcgcgcgccatcgtgcgcacgggcgaatgcaccccctacgccaacatcatgctgattgccggtgtgagcttctgaggcgccgcgcctttcccgcctattcgaaccggtagttcgcgcccacggcctgccccaccttgagcatgtgctccacgccctgcagcacgatgcagttcatgccgaaggtgatgcgcccgtcgacgcgcgcatcggcgcggtaggtgcgcagcatgtcgccgacctctgggctgctgatggcggtggccggatcgatgtccggaaccggacagcgggtgcagggcttgaccggcttgagctcggcctcgccttcgttcgtcgcgatgtgcagcgcgtcgacccggtcttcatcgtgcgactcgatgccggccagcacgatgttcggccggaagcgctcgatgtcgaccgcgtcgtggcccgcggccgccagccgctcgttgagttcggccagcgagccctcgctggccaccagcaggggatagccgtcggagaactggttctccgcctccacgccgccagtccattgcaggctcgacaggcgcttgtgctcgggatcgaagcgcaccaggcgcagcgcctgcggctggcccggttcggacaggaagtcgctgaaccactgggcggcgatgtcgcccatgtcgtaggctgccacgtcgtctttccagacgcgcacgcgcaccggcttttcgacgcgatcgaaggccaggtgcagggccagcatgcccggcgcgcgcagcaccacttccgtgtgcttcatctgcggctggatgagcgccatgcgcggcagctgccgctgggtgacgaactcgcccttcgcgtcgaccaccatccaggcgcggtcgaactcgaggccggtttcggtcagcagcgcctcgggaagctccacccccgcgcacgatttgacggggtagacgaacaggcgcgcaatggtcgcttggaggtcgaaaactggctgtgacacgtggggttccttggaattcggcagcgattgtcccgcatcgtcctggcggtgggcatagttcttacaatggcccgatggccctttcccctgaagtttgcatacgcggcgccggcatcgtcggccgcacgctggccctgctgctggcgcgcgagcgcgtgcgcgtcgcgctggtggttccgcccgccgcggccgccaaggaagacatccgggcctatgcgctcaacaccgcctcccgcaccttgctggaatcgctgcgcgcctggcccgatgcggcccacgccacgcccgtgcgcgaaatgctcgtgaacggcgacgaaggcgggcgcgtgcatttcagcgccgtgcgccagaaggtcgatgcactggcctggatcgtcgacgtgccggcgctcgagcagcagttggccgatgccgtccgcttccagccccaggtcgaggtggtgtccgaacccgttgccgcgccgctcacggtggtgtgcgagggcaaggccagcgccacgcgcgacgcactcggcgtgagctacgccgtcacccgctatccccagcacgcgattgcggcgcggctcgaagcggcccagtcgcacgacggcgttgcgcaccagtggttcaacgaccacggcgaggtgctcgcgctgctgccgatgggcggcctgcagagccattcggtcgcgctggtgtggtcggtcgaccagcttcgcgcgcccgcgctgctggcgcagagtgccgatgaattcaacgccgccgtgagcgaggccagccacggcgtgctgggcccgcttcagctcacgagcgagcgggcggcctggccgctttcgcgcgccattgccgaccgctggacgggcaccatgccgcaggccaccggcgcatcacaggctcaagcgcaaacctgggcgctggccggcgatgccgcgcacacggtgcacccgctcgcgggccagggcctcaatctcggtctggccgatgcggccatgctggccgacgtgatcaagcagcgcgaatactggcgcagcgtgggcgacccgcgactgctgcgccgctacgagcgcgcccgccgcgccgacgtgctgcagatgagccttgcgaccgacggcctgcagcaacttttttcgcacagcatgggtccgctgcccgtgctgcgcaactggggcatgcgcggcttcgaccgcacgcgcctcctcaagcattggatcgccaaccaggcgatgggcttgaaggcatgaatccatcgaccggactttccatgaaactcgtacgcaaccttcttctcgccgcctgcacgctgggtgcggccgtcgcggcccttgccggcgaagccgagatccgcaagaaccttcccgcgcgcattccgcagttcccggccatcgacgaggtcaccaagtcgccgctgccgggcatctatgaagtgcgcgtgaacggcttccagatctactacaccgacgagcagggcaactacctgctgcagggcaatctcatcgacgtgaaggcacgcaagaacctcaccgaagaacgcgtcgaaaaactcagtgaagtctccttcgacaagctgcccgtgaacgacgccatcaagatcgtgcgcggcaacggcaagcgcaagctcgcggtgttcgaagacccgaactgcggctactgcaagcgcttcgaaaaagacatgaagacggtcgacaacgtgaccgtgtacctgttcctgtaccccgtgctcgggcccgattcggccgcgaagtcgcgcgacatctggtgcagcaaggacaagggcaaggcctggggcgactggatggaggccaacgccaagcccgccaccgcggccgccagctgcgacgtggccgcgctgcagcgcaacgtggagttcgggcgcaagtacaacatcaccggcacgcctacgctgatcttcagcgacggcacccgcgccccgggcgccattcccgcggagcaggtcgagaagcaactcaccgcttccaagaactgatggctgcgccagccgtctcgcggcgcgcactgcctgcgccggccgccgcagtgcgctatcgcgtcgaatgcgcggacctgcacgcgcacctgttcgccgtcaccctgaccatcgagtcgccttcggcgcagcagcgcgtggcgctgccggtgtggattccgggcagctacctggtgcgcgagttcgccaagaacctgcagggcctgcgcgccacgcaggggcgccgcaagcccgtgctgacgcaactcgacaaatgcagctggcagatcgattgcgtgccgggccagccgctggtgctccattaccaggtctgcgcctacgacaactcggtgcgcaccgcctggctcgacgccgagcgcggcttcttcaacggcacgagcctttgcctccgggttgaaggccagacggaagcgccgcacgcgctggagatcgtcgcgccttcgccttccgccgatggcacgcgctggtcgtgcgccaccgccctcgtcccctcgaagaccgacaagcacggcttcggccgctacctggccgccggctacgacgagctggccgacagcccggtcgagatgggcgccttctggagcgccgaattcgaagcctgcggcgtgccgcaccgcttcgtcatcgcaggggccgcggcctcgttcgacggcgagcgcctgatcgccgacacgcaggccatctgcgaagccgagatccgcttctggcacggcgacaaggcgggcaagcgcggcggacccaagctgccgatcgaccgctacgtattcatgctcaacgcggtggacgacggctacggcgggctcgagcaccggcactcgaccgcgctcatctgcaaccggcgcgacctgccgcagcacggcaccaagaagcagcccgagggctacaccacgctgatgggcctcatcagccacgagtacttccacacctggaacgtcaagcgcatgcggccctcggagtttgcgcactacgactacagccgcgagaactacacgcacatgctgtggttcttcgagggcttcaccagctactacgacgacctgctgctgcgccgtgccggacgcatcgacgacgcggcgtacctccgcctgctcaacaagaccatcaaccaggtgctgcagacgccgggccggctggtccagtcggtggccgacgcgagcttcgacgcgtgggtcaagtactaccggcaggacgagcaaacgcccaacagcaccgtcagctactacaccaagggcgcgctggtggcgctgtgcttcgacctcaccctgcgccgcgaaggcaagggcacgctcgacgacgtgatgcgccacctctggacgcagggcggcgctggcccgatcagcgaagccgacgtggcagccgcactcgaagccgtgggcggccgctcgtatgcggaagagctggcgcagtgggtgcattccaccgacgagttgcccctggcggaactgctgcgcgcccacggcgttgcggcgctcgaagacccttcgcaaccggcgcaggctttggggctgcgcgtggccgaggccaacggcagcgtccaggtcaaggtggtgctgcgcggcggagcggccgaaaaggcgggcttctcggcacacgacgaatggatcggcgtggagctgccggcggtcggcaagaaaggccagcagcggcccgcgcaggcctggcgcatcgccaagctcgacgacctggcgctgtatctcggcgacgccacgcgctgcaccgcgctggtggcgcgcgaccgcaagctgctccggctgccgctggtgcggccggagggcgccaccacgtggcggctgttcctgcacgacgctgcgaaagttgcgggctggctcatgcccggcgcgcggcgctgatcgcgcttccggcagcgcggcttgccgtggctgggtatagtgaaccgcgtttttttccttcccccggagacacccatgagctacgaaaacatcgaagtgcggaccgaagcaggcaaggtcggcatcgtcaccctcaaccgccccaaggcgctcaatgcgctgaacgatgcgctcatgaccgagctgggcaccgcgctcaaggccttcgatgccgacgacgccatcggctgcatcatcgtcacgggcagcgagcgcgcctttgcggccggcgccgacattgccgcgatggccaagtacagcttcatcgacacctacaagggcgactacatcacgcgcaactgggaaaccatccgctcgatccgcaagcccgtgatcgcggccgtgagcggcttcgccctgggcggcggctgcgagctcgcgatgatgtgcgacttcatcatcgcggccgacaacgccaagttcggccagcccgaaatcaagatcggcgtgatccccggcgccggcggcacgcagcgcctgccgcgcgcggtgggcaagagcaaggccatggacatggcgctcaccgcccgcatgatggatgcggccgaggccgagcgcgcgggcctcgtgagccgcgtggtgcccttcgaaaagctggccgacgaagcgctcggcgcggcgctggtcattgcgggctactcgcagattgcggtgatggcggccaaggagtcggtgaaccgcgccttcgagagcggcctctccgacggcgtgatgttcgagcgccggctgttccatgcgctgtttgccacggccgaccagaaggaaggcatggacgccttcctcaacaagcgccagccggatttcaagaacgcctgagccgcatcgcctgagagccggcgcagcgcgccggctcgtcgggcgctactggcgcgcgagcaccgcccgcaacgctgcgagggtcgatgccggcggcgtgccgaccgttgcgccgccacccgtccccgccgcctgtggtgtccaacgcacctggtcgccggcgacctcgagcaccgcgagcagcgtggcgccgcggtacagctccagccgcgcttcgacgggcgcggccagttcggcgcccggtgcggtggctgaacgtgccgccgcatttaccagcgcggccagcccttccgtatcgccccgtgcctggcgcacgccctgccctgcgcgcatcaggttcaaggaggtccaccggtccagcgcagaaaacgccgatgtgtcttccgcgctggccttggccgcggcggacgcgggcgcgcgggcagcgggagcctggcgcaaggcgccggaagcctcggtaccggagttggcgctggcgctgcgctgagcggctgacagggccggagaagcgctgctgtcggccgactcgcgaggcgacggcggagcggccggtgccatggccgcagccggcggcgcgcctgcggcaacggggcttcgctgacggttttccggctcgttttcttcgcgtcgctcctcggcgcgcgggaaggcccgtggcgcgggtgcggattgctctgccatcggtgctggcgatggcggcgctaccgcgggagccgacggaggcgtaggtggcggtgcagccgcaatgaccggtgcaggtgcggccggcttgtcggagggcgctggtgccggcgccgttcggcgcaccgggtcttctcttcgctggggcgaccctccgctgaccgcgtctcgcgccgcttcggtcgcaggctgcgccggcgccggcgccggtgctggcgcaggaggaacaggggccggcgccggagcagacgcggcagtaggcgcggaggcgaccccggcctctccgtcgagccgcgcatcgggcaccggctcacgatgccagagcacggtgatgaaagtggccaccagcacggtcgcaaaggcagcattccacggcatgcgggcatgcgtttcgccgccgccaccgaacagccggcgccaccacggcgcagccaccgcgggcggggtcgcaggcacggtcgcgaggttgtgcgccatcttccggatcgcgtcacgggtacgcgggtcgggcagcgcatcgtggtccggcgcatgatccagcgcgcggcgcaacatcgggtcgcgcagcgtgccgtcgtcgccgtcgccgtcgaactccggggtgttgtttttgccgccgccgttgctcatgcgcgctgctccagcaccgacagataacgttccatgcagccgcgcaatttctgcagcccgtagcgcaagcggctgcgcacggtctcgaagccgatccccaggctggccgcaagcgcctcgacggtcaacccgtcttcatggtgcagcaggaaggcggcgcgctgctcggccggcaattcgtcgaggcaggccagcaggcgccggccggcggcgcgccagaacgcaagctcttcggccgaaggatgcgcagcggcgtcgagggtcgcgccgcgcacgccgcggtcgagcgtggggaccaccgcgtcgtcgccctcgtcggaatgcgcgtcgagcgccacttcgcgcccgctcacacgcaatcggtccatggccaggttgtgcgcaatggtgaaggcccaggtgcgccaggcggcgccctgcggcgagaagctgtcgcgcgcggagatgatgcgcacccaggtgtcctggaacacctcgtcggcctgtgcggccagcctggcccccagcagccgcttgacgaagcggaacagcccgccctcgtggcgcgcgtaaagcacgtcgaacgccgcgccgtcgccctgcgcgtacgccagcatcagctgctcgtcgggcatggcgtcgcgctcggtggcagctttggcggaaggggcgcggggcagcgcagacatcggcggattttcacccgtgcttgtacggtcggcgggccgcttcggggttgggcgtcgcaaaaaagacaccgcatccgacacgccgggcttgattcggtgcccgcggcctgcgctataatcttgggctcggtgcaaaactgcccgaacggctctttagctcagtcggttagagcgatggaatcataatccacaggtccgcggttcgagtccgtgaagagccaccaacatcatcaaaaagccttgcaagtcaacgacttgcaaggcttttttgtttttccggcgtgccgttttcgggtcccttccacccgcttttttccgccgaaggacacggtgcccgttcagcaggcaatgtagtgcgaacccccgccgatgctggctttggcgacccgcgtcctcagacaacccacagagttgtgcacagaaaagcaggacaagtcatccgcctgacttgagcgaaatgtaggccgcccgactcaacctgccttgcggaaggtgaggttgatgcgccgccggcccagcagcgcatgcggcctgtcctcgagcggcagcacgccgtgatagcgcaacctgtccggaccgccccacaccacgacatcgccgtgcaccagcggaatgcgaacggccttgtcgctgcgcgcgagcccgccgaacagaaaagtggccggcatgcccagcgaaaccgaaacgataggggcgtggtagccgcgctcgtccttgtcctggtgcagcgacaggcgggtgccgggctcgtagcggttgacaaggcaggcatcgggctcgaagccttcgaaccccgcttcggcggctgatgcttgtgccaggcgctcgaacaccgcgggcatcgggggccacggccggccggtttcgggatcgaactcggcgtagcgatagccgcgccggtccgagatccaacccaggcggccgcagttggtcatcgccaccgacatggtgaggccgcccggggtcacgaggtgccggaaagcggcgcgctgttcgacctcatgcaacgcgggcagaagatcgttcacgaagggcagcgcgaaaccgcgcagcacgaaggcaccagggccgatcgcctcgttaccgcgcggcagttcggcatcggaaaaaagatcgagcgtcacgcaacgattttctcgcgcgccgggccatcggcggccgccgcggccaccaaacgccccaacgtctgcatcgccttttcggcgtgcccgtcccaagcatggccatagttcaggcgcaggcaatgggagaaaccgcgcgtggccgaaaagatcggtcccggcgccacgctgatgccgagctccagtgcttgggcgtggatgtcgagcgcattcacatgcgccggcaactcgacccacaagaagtacccgcccagcggccgcgtggcgcgcgtgcccgccggaaagtagtgccccaccgcctgcgcaaagctcgcctgctgcaccgccagcgcctggcgcagcttgcgcaggtgcttgtcgagcccgcccttctccaggtagcctgccagcgcgagttgcgcgggcaccgaggtgctgagcgtggtcgtcagcttcagccgcgccacggcgcgcgtgaagcgcccaggcgatgcccatccgatacggtagcccggcgccaggcacttggaaaatgaagaacagtgcagcacgagcccctgcgtgtcgaaggccttggccggcggcggccgccggtcgctgaagtagagctcggcatacacgtcgtcctcgatcagcggcagcgcatgccgcgcgagcagttccaccagggccttcttcttcgcatcgggcatgaggctgccgagcgggttctggaaggtggtcatcagccagcaggccttgggccgatgggccgcgatggcgaactccagcgcagccaggtcaatgccttcgccgggatgcgtcggtacttcgatcgcgcgcaggcccatgcgctccagtgcctgcagggccgcgtagaaggtgggcgactcgacgatcaccgaatcgcccgggcgcgtgaccgccgcgaggcacaggttgagcgcctccatcgcgccgttggtgatgacaatttcgtcggccggcacctgcatgccgtcgcccaggtagcgcagcgcgatctgccggcgcagtgccgcgctgccgggcgtgaggtcgtccacggtgctccacgggtcgagcgacttggcgctcgcggccatgaactggcccagccgcgcgagcggaaacagcagcgggctcggaaacgccgagccgaagggcaccaccttgcgcgacatgctggcctcgaggatgtcgaacacgtggtcgctcacgtcgagagacttcggcccgtccgccggacgcgaggtgaggttggcttcgggcggcgcatcgcgcagcgcaccgccggtgacgtagtagcccgagcggtcccgcgcgcgcaccaggccgcgggcttccagcaggtagtaggcctggaacaccgtggacgggctcacgccgcggctctcgccggtatgccgcaccgaaggcaggcggtcgccgggcttcagcgtgccgtggcggatcgacgcctcgatgtcggcggcaagggcttcgtagcgcttcatgtcaggacggcggtcattcgaggcgactttatctgctccggtgttttggttcggatctgcatctgttttttcggggccggttgcggcacagtcggtgcatgtccaatttcatgcgcgcggtacgcgcggttctctggagtttcatcgggcttggcggccgccgcgcggacgccgaccggcgcaccgagcaagtcggcctgttgccgctgatcggcatcgcgctggccacggtgctgctgctcattgcggggctgctggcactcgcgcatttcgcggccggcgcatgaggaaggcggcccaccggctcgccggaatcgcgctgatgctactgctgctcggccacggcatcgcggccttggcggcgacgcccgccacgccctccggcaacgacatcgagcggcgcgtggccgcctgcatcgcctgccacggccgcgaaggcgccaccaccaacgccggctactttccgcgcctgtccggcaagcccgcgggctacctgttcaaccagctgcggagctttcgcgatggccggcgtttcaacgccgacatgacctacatggtgcagcacctctccgatgcctacctgatggaaatggccgagtacttcgcgggcctggacctgccctacccgcctgtctcgcccgcgagcgacgcgccacccgcgcagctggcacgcggccgccagctggcgctcgaaggcgatgccgcgcgacgcattccggcctgcgtgcagtgccacggcgccgcgctcaccggcgtgcggccggccattccgggcctgctcggcctgccccggctctacgtgtcttcgcaactcggcgcctggctcaccaacgagcggcatgcgctcgctcccgactgcatggccgacatcggacgccgcatgaacaccgccgacatcaacgccgtggccagctggctcgcggtgcaaccgatgccggccgatccgaagcccgccgcctccctgcccgccccgctgccgatggcctgcggcggcatgccgaaatgaggcgcccatgaggaagatgcgatacctcggctggacgctgcctgcgctggtacttctgctgggcgcggcggcggccggcatcgtcgcgctcaatctgcgcggcgaagacccgctgcccgagcaggccgaagccttcaacgccacgccccagcaggtcgagcgcgggcgctacctcgcgctggccggcaactgcgccggttgccacaccacgcgcggcggccagccctatgcgggtggactgccgatcgaaacgcctttcggcaccgtctattcgagcaacctcacgcccgatgcgaaggccggcatcggcagctggagcagtgcgcatttctggcgcgcaatgcacaacggccgcagcaaggacggccgcctgctgtaccccgcgttcccctatccgaacttcacgcaggtgacgcgcgaagactcggatgccatctacgcctatctgcgcagcgtgccgcccgcgccagcgcccaacctgacgcaccggctgcggtttccctacgacacgcaggccgcgctggcggtgtggcgggccctctctttcaggcccgagcctttcgtggccaatgcgggcaagccggccgaatggaaccgcggcgcctacctggtcggcgggctgggccactgcatcgcctgccacggcagccgcgattcgctgggcgcgacgcaggcgaacctgggcctctcgggcggcttgatcgcggtgcagaactggtacgcgccatcgctcaccgatccgcacgaggccggcgtggccgactggccctccgcggaggtggttgcactgctcaagaccggcatcgcgccgcgcggctcggtcatggggccgatggccgaggtcgtgtttcgcagcacgcagcatttgaacgacgccgacctggccgcgatggccagctacctgaaagacctgcctggcgcagcggcgcaaccggcggcacgcaccggcaccgcgcccaaccgccgcgatgccggcaccatggtgcgcggccagaagatctacgaccagcgctgcgcctattgccacggcgaccaggggcagggcgtgccgggcgcctttccacccctggcgggcaaccgctccgtgaacatggcgcagacggcgaacctgacacaggtgattgcacatggcggctacctgccgtccacctcgggcaacccgcgcccctacggcatgcctcccttcggacaggtgctcgacgcggccgacgttgccgcggtgctcactttcgttcgcggctcatggggcaacgacagcccacccgtggcgctgctcgatacgatgcggcggtgatcggcgactactacggattccggtgatatcgcagtccgctggcagcccctagcatcagagtggtacagacccccgtcggagagccgcacagcagcagtgccgatcgaaccagcccgtcgagaatgccccaaagtaccgccagcccggacgccaccgagcctatcgccaggccatctctcaagcctctttatcaaatgctgcgggtggcctcgcacctgctggaccaggccgccatcgaagtgcgcgaaaacggcccggatccggccgccgagaacatcgagagaatcggccgcgcgctgttcgaagtgattcgggtgcagcacaagatcttcgcgctgcagcccgaactcgaaccgaggtcgctcgccgcttcgtcccgcgaagccgccgccaaccagcttttctcccaattcatgcacgaagcgctcgaactggaagacgtgggcaataccgccgccgccgtggagcggtacacccgtttcatcggcatctcgccgtcgtaccaccaccgcgagattgcacgggcggaaatccggcggctctcctagcggaagtgccccggtccgtcgtgcgacggggctcggggaaggccgcccgcagcctgctcaggctgcgacgggctcgcgctgcgcgccggccttcgcgggcaccggcatgtgctgcgcccagtcgatgatctccagcgtgccgtcggcatgctcggccagcgccgtgaggctctcgacccagtcgccgtcgttgcaatagaggatgccgtcgatgtcgcgcatttcggcgtggtggatgtggccgcagaccacgccctgcacgccgcgcttgcgggcctcgcgagccacggcgttctcgaaatcgcccacgtagctcacggcacgcttgaccttgcccttgaggtacttggagagcgaccagtacggcagccccatgcgcgcgcgcagcgagttgagatggcggttgagcttgagcgtgaattcatagagcgagtcgcccacgtgcgcgagccacttggcgcactggatcacgccgtcgaacaggtcgccgtgaatgatccagagcttgcggccgtcggcggtctcgtggatccactcctcggccacgtcgatgccgccgaaattgtgatgcaggtacttgcgcgcgaactcatcgtggttgcccgggatgaagatcacgcgggtgcccttgcgcgccttgcgcaacagcttctggatcacgtcgttgtgcgcctgcggccagtaccagtggcgcttgagctgccagccgtcgatgatgtcgccgaccaggaacagcgtctcgcactcggtgtgcttcaggaaatcgagcagcgcgcgggcctggcagccgggcgtgcccaggtgcaggtcggagatccagagggtgcgatagcgcagcggcgggcgcgcaagatcgtcgtcctccggctcgggagcccgggtcgcggtgtcgcgccatgcgcggaggaaagcatcgtcgcgttgcatggacgggtaggctcccacctatgcgtgacggcgcgatggcgttccagtgacattccggtgacgcgtggcccggaggcaacgcgctgcaactgactcaagaggcgcagcgctggatttccacggtcgagtggcgaatttcctcgtgcatggagaaacaggcgcgcacctcgtcggccgacagcgtgggggaatgcgtcaccaccgtgagggcgcaggcataggcctcgcggcccacgcgccacacgtgcaggtcggccacgcgggtttccgaatcggccagcgtggtctccacgccttcgcggatttcgaccgtgacggggtggtccatctcgcggtcgagcagcacgcggccggtttccttgagcaggcccttggcccacacggccaccagcaccgcgccgacgatgcccatggccgggtcgagccaggcccagccgaagaaccagccgccgagaagcgccgcgatcgcgagcaccgaggtggcggcatcggccaccacgtgcaggtaggcggaacgcaggttcaggtcgtggccgtgagcatgatcgtggccgtggtgcgcatggccgtggccatggtcgtgcccatgcccgtgatggtgcgccgaccccagcagccgcgcacagaccaggttgaccaccagcccaaggacggccaccgccacggcttcgcggtagtggatggccgagggcgagagaagccgttcgatggagcccaccaccatcagcgccgccacgccgagcagcatcagcgcgctcgcgaagccgcccagcacctcgatcttccaggtgccgaacgcgaaccgcggatcgcgtgcgtagcgcctcgcggccgcataggcgaaagcgctcaggccgatggccagcgcgtgcgaactcatgtgccagccgtcggccaagagcgccatcgagttgaaccaccagccggcgccgatctcgaccaccatcgcggcgatggtgatccacatcacgaggcgggtgctgcgctcggccgattcgttgcctgcgccaaagtggtggtcgtgctgccaggcacggaggtcatgggtgtgcatggtttcaggctccaaagaggtcttgaccgtccgagcggctcgagggcggtgccacgccgaggtggcggtaggccgccagggtcgcgatgcgtccgcgcggggtgcgctgcaggtagccctgctggatcaggtagggctcgatcacgtcttcgatggtgcccggctcctcgccgatgctggccgccacgttgtccagccccacggggccgccgtcgaagcgatggatcacggcctcgagcagcttgcggtccatcaggtcgaagccctgcggatcgacgtcgagcatggcgagcgccttgtgcgcgatctcttcgttgatgcggccgttgcctttcacatcggcatagtcgcgcacacggcgcagcaggcggttggcgatgcggggcgtgccgcgcgaacggcgcgcaatctcgaagccgccggccgtatcggtttccaccttgagcaggccggcgctgcgccgcacgatgagcgccagttcttccggcgtgtagaactccagccgcgccacgatgccgaagcggtcgcgcagcgggttggtgagcatgccggcgcgggtggtggcgcccaccagcgtgaagggctgcaggtcgagcttgatgctgcgcgccgccgggccctcgccgatcatgatgtcgatctggtaatcctccagcgcgggatagaggatttcctcgaccaccgggctcaggcggtggatctcgtcgatgaagagcacgtcgttcggctcgaggttggtcaagagcgccgccaggtccttgggcttctcgagcaccggcccggaggtctggcgcaggttcacgcccagctcggccgcgatgatgtgcgacagcgtggtcttgccgaggccgggcgggccgaagagcagcacgtggtcgagcgcttccttgcgcttgcgcgccgcgccaatgaagatctcgagctgctcgcgcaccttggcctgcccgacgtattcgtcgagcaacttggggcgcagcgcccgctctatcgcttcttcctggggcgaagcgggggcggcggacaccacgcgtgggggcgcgggcgcgaagtcgtcagtctgaatggtcatgggagagggttttgcgtttgtgagtttagtgcctgctcactggcagaatgcttcggccatataacaaacgaggggaagccaagggtgtcgatctacgaactgaagccccggttccaggcgctgctgcggccgctggtcggccgcctgcatgccatgggcatcaccgccaaccaggtcaccttggccgcttgcgcggtgtcggtcgcactcgggctctggctcttcttcgccgccccctcgctggccgctttcggcctcatcccggcctggatgttcgtgcgcatggctttcaacgccatcgacggcatgctggcacgcgagcatgggcagcaaagcaagctcggcgccttcctcaacgaactgaccgacgtggtctccgacgccgcgctgtacctgccgtttgcgctggtgcagccgttcagcccgttctgggtcggcacggtgatcgtgctcgcgggcctgagcgaattcgcgggcgcgctgggcccgacggtgggggcctcgcgccgctacgacgggccgctcggcaagagcgatcgcgccttcgttttcggcgcgctcggcctctatgtggcgctgggctggccgctgccgggctgggctgcgtggctgatgccccttcttgccgtgctcgtggcctggacagtggtcaaccgcatccggcgcgcgctggctgaagctgcatagacgtgaacacaacgaacaaaacaatagcgacagggatccgatgaccgacaccaacacacacaccaacccacgcattccgcaagagcgccagttccgcacgcacgacggcgaatcgctcttctaccggcactggccggccaccggcgaagcgcgccgcggcgccatcgtgctgttccaccgcggccacgagcacggcgcgcgcatggcgcacctggtcgacgaactcgacctgcccgacttcgacttcttcgcttgggacgcgcgcggccacggccgctcgccgggccagcgcggctacagcccgagctttgccacctcggtgcgcgacgtgcagaccttcgtccagcacatcggcagcgcgcacggcgtggcggagcacgacatccatgtgattgcgcagagcgtgggggccgtgctggtctccacctgggcgcacgactacgcgcccaaggtgcgcgggctcacgctggcatcgccggccttcaaggtcaagctctacgtgccttttgcgcgcgccgggctgggcctgatgcacaagctgcgcggcctgttcttcgtcaacagctatgtgaaggcgaagttcctcacgcacgacccggagcgcatcgcaagctacgagagcgacccgctgatctcgcgcccgattgccgtcaacatcctgctcggcctctacgaagcggccgaccgcgtggtggccgatgccaatgccatcaccttgccggtgcagctgctgatctcgggcgcggactgggtggtgcaccacaagccgcaacaccagttcttcgagcggctgggcagcgccgtcaagaccaagatggaactgccgggcttcttccacgacacactgggcgagaaagatcgcgcgccggcggtgcaagcgatccgcgaattcattcttcagctgttcgaccagcctccggcgccggtcgacctgcgcgcggcgcacctcggcggcaacaccgccgacgaatcccgcgcgctggcggagccgctggcgcccctctcggcgcgcggcgcctattgggccatgacgcgcgccggcctgcgcatcggcggcaagctgtcgagcggcatcgcgctcggccatgccaccggcttcgattcgggcagcacgctcgactatgtctaccgcaaccacccgaaaggcaagggcccgctgggccgctccgtcgacaacacctacctgaactcgatcggctggcgcggcatccggcagcgcaagatccacgtcgaggagctgatccgcatcgcgatggaacggctggccgagatgcaccgcgaggtgcgcgtgatggacatcgcggccggccatggccgctacgtgctcgacgcggtgctcgcgagccccgtcaaggccagctcgatcctgctgcgcgactacagcgacatcaacgtgcgcgacggccgcgcgctgattgccgaaaagggcctggaagacgtggcgcagttcgtgcaggccgacgccttcgaccgcatcagcctggccaccgtgacgccgcgccccacgctggcggtggtgtcgggcctctacgagctgttccccgacaacgagatggtgcggcgttcgctcgcgggcgtgggcgacgcggtggaagaccgcggctatctggtctacaccgggcagccctggcacccgcagctcgagatgattgcgcgcgcgctcaccagccaccgccagggcgaagcctgggtgatgcgccgccgcacgcaggccgagatggaccagctggtggaggaagcgggcttccgcaagatcgaccagcgcgtcgacgagtggggcatcttcaccgtctcgctcgcggtgcgggtggcatgacctcggggctgggcgcgaaatgaggcggtggctggcgcagcgcccctggaagcgggccgccgcgtggctggtgttcctggggccgctcttctatgcaacatacggccttgccaattggtgggccaccacgcgcgcgcacgtgccatcgatggccttcgaatgggagcggcagctgcccttctgggcctggaccatttttccgtactggacgatcaacgtcttctacgcgctctcgctcttccttgcgcgcagcaagcacacgctcgaccggcatgcgctgcgcctcgtgagcgcaacgctcatcgcctgcacctgcttcgtcctctggccgctgcatttcagcttcgggcagccggcggtagaaggcgcgccggcgttcctcttcaatgccttgcgcggcttcgaccagccttacaaccaggcgccttcgctgcacattgcactggccgtgatcctgtgggactggtaccggcagttcctgcgcgccacatgggcaagggtggtactgcacgtgtgggcctttgccatctgcgcatcggtgctcacgacctggcagcaccacttcatcgacattccaactggcgcactgctcggcctgttctgtatctggctgtggccgctcgcgcgtacggtgtcgatgccgagcgcctggcaatgcacgcgcgatgcgcagcgctggaagctcgcgggcttctattcgaccggtgcggccctgttccttgccgtcgcgctctacggtggcggcgtgctgctgtggcttgcgtggccggcggcctcgttggctctggtggcgctcaactacatcggctacggcgcccgcggcttccagatggatggccgcggccgcatgggctgggcggcgcgctggctccttgcgccctatcggctcggcgcggcagtcaacgcatggctctggacgcgcaagctgccggcttcggtcgaagtggtgccgggcctgcgtctgggacgcttgccgacggaggccgaatgggttgccgccggccggccgcggctcgtgagcctgtgcgccgagttgcagacgcccgccggtgtgccgcatgcgcactgcgtgccaatactcgacctgacggtgccgccgaccgtgcggctgcaacgcgcagcggcggtcatcgaaggccagcgactcaaggccgacggcgcgccggtatgggtgtgctgcgcgctgggtttttcgcgcagtgcggctgcaacgatcgcctggctgggccgctatggttcggcgggcagcctggtgcaggccgaaagcgcggtgcgcctcgcgcgtccgcagatcgtgctgcgacgcgaatggatgacgtcgctggaacccctgaacgccgtgccggagctaccgccccatgactgacaacgaacgcgccacctgcgcggcgctggccggactgctgcgtgccttcatggtgcttgccatctggggctttgcgctcacgtgcatctcggcactggtgctcgcgctgacgctgcgctcgctctcggtcacggccgccatgggcttcggcgcggtcgtggtcctcggcctgctcgaacgctatttcgccttccggctgcggctggacgaggcgttgttcgccgatctcgggcgccgcgccatcgcatcgctcgacacgctcgaccacgcgctttcatcccttggactgcgcgagacgccgccagagcaaaaaaccacccgccccctcgacgaacgcgtgcagggcacccgccagctcatgcagcgccatgccatcgtggtcgcctgccagagcgccatgtttctcctcgccttgatgacacaggacctctcttgaccgaagaagacaacaacaagaacggcgacaagcccgaaagcaccgtgctgcgccgcgcgtttgccgtggtcgcgggcaagctgatcatcggtgcggccggtttgctgacgggcgtgcgcgccatctggagcggcaccacgcccaaggccgagcagacgctgtactttgccaaccacacgagccacggcgacttcgtgctgctgtgggcgacgctgccgcccgacctgcgcgcgttgacgcggccggtggccgggcaggactactggatggcctccaaggtgcgccagttcatcggcgccgacgtgttcaacgcgctcatgatccggcgcgacggctcgggccaaggcggcaacccggtcgatcagatgaaagaggcgctggaaggcggcgactcgctcatcatgtttcccgagggcacgcgcaacaccggcgacgagatcctgctgccgctcaagagcggcctctatcacctggcgcgtgcctgccccaacgtgcggctggtgccggtgtggatcgagaacctgaagcgcgtgctgcccaagggcacgctggtgccgattccgctcgcctgcacggtccgcttcggcgcgcccatccagctggccgaaggcgaggacaagaccggtttcattgcccgcgcacgcgccgccatgctcgacctgcgccccgaatacgaccgcgtgccagaacaagaaaaagcagcaacgacgccatgaacatctcgccctccacccagaccacgctgcaattgttcggcggcgttgccggcgtgctgattcttgcctccaccattggcgcgctgctcaagtggcgcgtggcccaaggccagcccaattcggtgatcgacaacctcaacgcgcgcgtgaatgcatggtgggtgatggtggcggtgatcggcattgccttcgcgttcggcaagggcggcgtgatcgtgctgttctatctgatctcgttctatgcgctgcgcgagttcatcagcctggcctacacgcggcgcggcgaccatcatgcgattgcggcggcgttctacatcgggctgccggtgcagtacttcctggtgtggatcgactggtacgggctctattcgatcttcattccggtctacgcctttctcgtgctgccgattcttgccgccgtgggcggcgacacgcagcgctttctggaacgcacctcgaagatccagtggggcctgatgatctgcgtgttctgcatcagccacgtgcccgcgcttctcacgctgcagattcccggcttcgagggccgcaacctgctcctgatcgccttcctcgtgatcgtggtgcagggcagcgacgtgctgcagtacgtgtggggcaagcttttcggcaagcgcaaggtggcgcccgaactctcgccctccaagacctgggaaggcctggtcggcggcgtggccagcgccaccgcgctgggggcggcgctctattgggcgacgccgttcaacccctggcaggccgcgctgatggcactcaccatctgcctcatgggtttcttcggcgggctcgtgatgtcggcgatcaagcgcgaccgcggcgtgaaagactggggctcgatgatcgagggccacggcggcatgctcgaccggctcgattcggtgatctttgcagcgccgatctactttcatgcgctgcgctactggtgggtgccatgagcacgcgcgccaaggctgacaaggctgcccagcgcgtggcctaccagatgcccattgaatgcagcactgccgccgtatgggagcattggctcaggcaccagcatgcgagcgcggccggcgtatggattcgcatcgcgaagaaagacagcggcattgcgtcggtcacccacgcggaggcgctcgaagtcgcactgtgctacggctggatcgacggccagctcaaggcggaggacgacaagcactttctgcggcgcttcactccgcgcaccgcacgcagcatctggtcgaagatcaaccgcgacaaggcgctgaagctgatcgacgaaggccgcatgcagcccgccggcctggccgaagtcgaacgcgcacgcgccgacggccgctgggaggccgcttacgacgcccagagcaccgccatcgtgccgcccgacctgcaggccgcgctcgatgcgaatcgcaaggcgaaggacttcttcgccaagctcgattcgcgcaaccgctatgcggtgctcttccgcacgcagggcgcaaagaagcccgagacgcgcgcgctccgcatcgcacggttcgtggaaatgctcgccaagggcgagaagctctatccctgagtaccgccgcaggcgctacgtatccgttctctggagcgtgtactcgccgggcttgtacggccccatggccacgccgacgtcccacagcttcagcgcgcccggcaagacggcctggctgccaatcttggcaacaccgcgttttcggatttcgcggttgaggcgggacgagaaggacgtgatcctgccgaagtcccaggcctcgaccccgccgagaacgtccacagtgtccgaccacgcctgtgcgcgcttcatcgagttgtggttggtgtgcgagttttccagtcgcgcatcgcccgcggaggccgagcccaggtacagctgcaccaggccccagccatcggcgttgtagcggaatgtggcaccaccgcaagcctgcgggttcagcgtcacgcggcgcggtacgaaggcggggcccgcgccgcgcacatacagctgcagatgcacggcatgccacctcctgccgttgggatagctgcgatcgaactgcgccagcacttcggccgccgagcggaaacatctcagcggttgcccgaagtcggacgcgagttcgtagacgtcgcagctttcttcggcgaacagccaagagagcaggctgtcgtggtcttccttcgtggcgtagaagtcgcagttgggcatgccctcggtcccttgcctgttacggcctacttcgccagcgccttcagcgccagcttgatgccttcgctcacggtcgcatccttcggcagcgccttgagcgccagcgcggcttccttgtcgctgtaccccagcgcgatcagcgcctggaggatgtcggcctgcgcgtccgaagccgcatgggcgggcatgccgatgtcggcgcccagcttgcccttgagttcgagcagcagccgctcggcggtcttcttgccgatgcccgggatcttcaccagccggccgagctcctgcgtcgtgatcgcctgcgacagctcgcccacgctcatgcccgagagcaggccgagcgcggtgcgcgggcccacgccggtgatcttgatgagctggcgaaaagccgcacgctcctcggcggtgccgaaaccgtagagaatctgcgcgtcctcgcgcaccacgaagtgcgtgagcagcgaaacgcgctctccggtgccgggcaggttgtagaacgtgctcatcggcacatcgacctcgtagccgacgccgttgcagtccaccaccacctgcggcgggttgcgttcggccaatacgccggtgagtttgcctatcattggcccacccccgttgcttgctcacttcgtgtagccgcctcccccctcaagggggcaacaccggcggcccggcaaagccggttccgcggtgttccccgctttggattgcgttttttcgagcatggctggtcttgcatagggctgccaaaaaaatggaaatggataccgcgtgattctgcgacacacctttaccccactgaacaattcgcgcctcggccacctgtgcggacctctggacgcgcacctgcgccgcatcgaggaagcgctgggcgtgaagattgcgcaccgccacgagcagttcaaggtcgagggtcccaaggcccccgcgcagcgcgcgatggacgtgctgcaggcactgtacgaaattgcccagcgctccatcgaccccgccgtggtgcagctcaccctcgcaggcgacggcacgatgatcgacggcgacgaggatgcggcgatgctcgtcacgcgccgcgccgacctgcgcgcgcgcacgccgacgcaggcgctgtatctcgacaacatcgccaagcacgacatcactttcggcatcggcccggccggcaccggcaagacctatctggccgtggcctgcgcggtcgacgcactggagcgcgcctcggtgcagcgcatcgtgctcacgcggccggcggtggaagcgggcgagcggctcggcttcctgccgggcgacctgacgcagaaggtggacccttacctgcgcccgctgtacgacgcgctctacgacctgatgggctacgagaaagtgcagaaggccttcgagcgcaacgcgcttgaaattgcgccgctggccttcatgcgcgggcgcacgctgaacaatgccttcgtcatcctggacgaggcgcagaacaccacggtggagcagatgaagatgtttctcacccgcatcggcttcggcgccaaggcggtggtaacgggcgacgtgagccagatcgacctgcccaagcagcagttgagcgggctgatcgatgccgagcgcgtgctgcggcgcgtgaacggcatcgcgatcacgcatttcaccagcgccgacgtggtgcggcatccgctggtcgccaagatcgtcgatgcctacgacggccagcgcaaacgtgcgggggcgcactgacatggcactggcccagctttcgctctcgctgcagttcgcgccgcgcttcaagggcatcgaacggcaccgcgccgcgctgccgcgccacagcgtggcgcgctggatccgccatgcgctcgaattggacggcgagatcacggtgcgcatcgtcgatgccgaagaaggccagcgcctgaatcgtgaattccgtggcaaggactacgccaccaacgtgctgaccttcgactatgcgcaaagcccgatggtgatggccgacctggtgctctgcgcgccggtggtcgcgagcgaggccagggaacagcgcaagaccctggccgcgcactacgcgcacctgctggttcacggcacgctgcacgcgcagggctgggaccacgagaccggcgaagccgacgccgaggaaatggaagcgcgcgagatcgaaatcctggcggggctcggcatccgcaatccgtacggccggtaaatgacttcggccgcggcgcccggcacgagcaccgatccgtggctggagcgctggcttgcgctggtcaccgagcgcgcgggaccggacccggtgctcgaactgggctgcggcaccggccccgacagtgccgtgctggtcggcgcgggtttgcgcgtggtcggcatcgagctgtcgagcgaatccgtggcggccgcgcgggcgcgggtgccgcatggcgcggagtttcactgcggcgatttccgtgatgcgccctttccgctgcccgcgggggacgcggagggcagcgtgggggtggtgctcgcgagcctgtcgctgcactactttgcgtgggacgaaacgcttgccctggcccggcggatccacggcgtgctgcgcccgggcggcgtgctgctgtgccggttgaattcggtgaacgacatccaccatggcgccagcggcccgccgccggaaggaaaggattccttctatctggtggacggcgtgcccaagcgatttttcgaccgtgccgcggtggaacggctctttgccgacggctggcgcatgctgcatctggaggaactcacggtgcaccgctacgagcagccgaaggtgctctgggaagccgtgctcgagcgcagctgaaggcggcgctacgccagcatctgcagcggaatggtcacgggtccgtcgttgaccaggtgcacctgcatgtcggcaccgaactcgcccgtggccaccacggggtgcacgccacgggcctgcgccacgaagtactcgtagagccgccgcccttcgtcgggcgccgctgcctgcgtgaagctgggtcggttgccgccgctcacgtccgccgccagcgtgaactggctcactacgagcagcccaccgccgatgtcctgcacgctgcggttcatcttgccggcatcgtctgaaaagatgcgcagcttcaacagctttgcgagcatgcggtcggccagcgcatccacatcgccgcgctcggcgcagagcaggaccagcaggccggcgtcgatggctccgacggtctggccggcaatgtcgacacgcgcgctggccacgcgctggaccacggccttcatgcctgttcctccatctgggtagcgcgggcttccatgcccagcggcagcaactggatggtcacgcgtaatccgggcacggcatccatcaacgtctgctcgagttcgtcgcgcagggccgcggcgtgctgcagcgtccagtcgccgggcacatgcatgtgcaggtcggcaaagcgacgctggcccgcgcgccgcgtcaccatgtcgtcgaagcgcacgcgcgcgccttcgggcaggcgcgcggcaaactggtcgagcgtggtgcgcagcgtggcgatggtctcggggtcgagggcttcgtccatcagcccttgcgaggagcgccataccagcctgatgccttcgcgcacgatgttgagcgccacaccgatggccagcagcggatcgagccacagccatccgctgaagtacacggccacgatgccgaccacgacccccgccgaagtccatacgtcggtcatgagatgccgcgcatcggcttccagtgcaatcgaccgatgcgttcgcgccgcgcggaacagcgcgaaggcaagtgccgcattgaagcccgaactgaccaccgaaagccccagcccccagcccagttgctcgagcggttcgggggcaagcagccgctgcacggacacccagagaatggccgccgcggcacctacgatcaggatgccttcgaagcccgaggagaagtattcggccttgtggtggccgtaggggtggtcctcgtcggccggccgcgcggcaatggtcaccatggccagcgcgaacatggcgctggcaagattgacgaacgactccatggcgtccgagatcaatcccatcgaattggtcacgtagcccgccaatcccttgagcagaatcgtgacgagggcaacggcaacggaaacgcgaagcagtgtcttgggcgtaagggtcatgcgcggcgagaatcgtcaagcgataaagacagccaaagtgaggcaaaaggccgcatctggccattggattatctggggtacgctctatgcgtaccggcgcgttttaatatttgtctcaccgcgagacattcgcagagaggtgatgtgatgagaaagttcttgagcgtcctgggagggctcgccttgtgtggcgcagcgacgctcgcccaagcacagagctctgcgagcgcgccaactgccaccaagccaatcgccgagcctcaggcgggcttcgtcaaatcggtgcgcggcaacgtgcaattgctcagcgccgccggcacgagccgaacggccattgccggtgacgcgctggccgccgtcgaccgcatcgtgacaggtcccgattcatccgcctccgtggtccttcgcgatgacacgaccctggtggtcgggccgtcttcgcggctggacttgaaggaattccatttcaattccaccacgcatgaaggtggcgtgctcgtctcgttgttgcgcggctcgatgcgcatgatcaccggcctgatcggcaagacgaaccccgacgcgattcgcgtggaaacacaaaccgccaccatcggcatccgcggcaccgatttcatcgtgcaggccgacggccagccatgagtcggttgaaatcccgcgccctctccttccttgccgtgccgatcacggcgctacttgccgcctgctcgacgccgggcacccgcgtggtgctgctgccgcaggcggatggcaagccttctgccgtgacggttcgcatgaaggatggcgaagaaattctctccaagccctaccagcgtgccacggcctcggtcggcgcttccggcgctccggtggtcgaccaggccgatccggccaaggtacaagccgagcacaagttcctgttcgacatgcagccgcctccgccgcagcgctacacggtgtatttcgacgtgggcggcacccggctcacgccggcgtcgcagcaggtcatgaacgaagcgctggttgcggcgcagacccgcagcggcagcgacatcgtggtgaccgggcacaccgacaccaaaggcgctctcgagcagaacgacatgctctcgcagcgccgtgcgcaagaagtggcgcagctcttcgtggagcggcagtttccttccaagcgcatcgaggccgtcggccgcggcgaacgcgaactcgccgttcccaccgcggacgaggtggacgaaccgcgcaaccggcgcgtcaccatcgaagtccggtgaggttcgcggctcctgccgcgcctccttccgtcagctgagagtcacgcgcgcaaacttgcgcttgccgacctgcaccacatagcggcctgcgggcagcttgagcgccttgtcgccgatcaccacggagtcgacgcgcacgccgccaccgtcgatcagccggttgccctcggaagtcgagggtgccaggccggcttgcttgagcagttgcgcaatgcccagcggcgcgccctgcagcgacacctcgggaatatcgtcgggcacaccgcccttgctgcggttgatgaaatcctgctcggccgtctcggcagccgccgcactgtggaagcgcgcggtgatttccttggccagcgccaccttcgcgtccttgggattgcggccggcagcgatctccgccttcaacgcctcgatccgttccatcgactggaagctcagcagcgtgtaccagcgccacatcagctcgtcggagatcgacagcaccttggcgaacatggtgttggcgtcttcgctgatgccgatgtagttgttcttgctcttggacatcttctcgacgccgtcgagcccttccagcagaggcatagtgagtatgcactgcggctcttggccgtattcctgctggagatggcggccgacgagcaggttgaacttctggtcggttccgcccagttccaggtcgctcttcaaggccacggagtcgtagccctgcatcagcgggtagaggaattcgtgcaccgagatcgactggccggccttgaagcgcttgttgaagtcgtcgcgctccatcatccgggccaccgtgtacttggcggcgagctggatcatgccgcgggcgcccagcgggtcgctccactcggagttgtagcgaatttcggtcttttcggggtccagcaccaggctggcctgccggtagtaggtctgggcgttggcttcgatctgctcccggctcagcggcgggcgggtgctgttgcggcccgaagggtcgccgatggtggtcgtgaagtcgccgatcaggaaaatgacccggtgcccgagatcctgcagctgccgcatcttgttgaggacaaccgtatgaccgatgtggatatccggggccgtcggatcgagccccaatttgatgcgcagcggcgttccggtggcttccgagcgctgaagcttgcgcacccactcgtcctggggaagcagttcgtcggtgccccggagggatatttcgagcgctcgtcttacaccatttgacagagtagcggatgtaacagattcggcgttcataggctttttggctgattttcaggttgccgaagttatactcagcccgacctttcaagcgccggattctaagcggcgcttttttccgcaccgtcctgccgcccatccgccccgggctttgcagcgcggatttgcagaacctgagctggaattcaaagtttgatcaacggcattctcgccgccgaggagctactggcttctcgcgtggcctatacattccggacctatcccaagcagatcaccgccgtcatcgcggcggcactgctgagcgccggcaccctggcagtggcctctctcggccccgatgcatccgacctcccggtccaacaggtcctggaagcgaccgctccactgtctttcgcagaacagagccaatcgctcgagaacttcagcttcacgctgtttcgcaccgacatcacgcgctccagcgacacggccgaggccctgctgaagcgcctgggcatttccgaccctgccgccaccgcattcgtgcgcggaagcagcgaagcccgcaacgcgctgtttgcgcgcgccggacgcaccatcacggccgaagccacgcaggaaaaccagctcaagaagctgagcgcccgctggattcccgacggtgacggcggcttcaagcgctttgttgtcgaacgcacgccgggcggctttgtcgcccttaccgagcgcgacaccctgacgccgggctcgcgcctggccagcggcaccatccgcacttcgctgttcgcggccaccgacgacgcacgcattcccgacgccgtcgccagccagctggccgacatcttcgcgggcgacgtcgacgtgcgttcgctgcgcaagggcgaccgcttcgccgtggtgtacgaaactttcgaagccgacggccaggcgctgcgcagcggccgcgtgctctccgccgagttcgagagcggcggcaaggtgcaccaggccgtgtggttccagcccgccgccggccagaagggcagctactaccggccgaacggcgacagcctgcgcaaggcctacctgagctcgccggtcgagttctcgcgcgtgtcgagcggcttcgcgatgcgcatgcacccgattctcaacagctggcgccagcacaacggcatcgactttgcggcgcccacgggcaccgcagtgcgcagcgtcggcgacggcacggtcgatttcgccggcacgcagaacggctacggcaacatcgtcatcgtcaagcaccgcaataaccagcagacggcttacgcccacctgagccgggtcgacgtcaaggctggcgaaagcatcagccaaggccagacgatcggcgcggtcggttccaccggctgggccacgggcccccacctgcatttcgagttccgcgtgaacggcgaataccaggatccggcctcgatcgcccaggagggcggcgctccgatcaccgcggccatgcgaccggctttcgaacgcatcgccgtgggtgcccgcaccgaactggctgcggcgttctcggtcatccaggccagcgcggactgagttccggcggcgcagcggcaacagccagcacagcgcggcccgctcgctctcccatccagcgatggccgccgccgaactcttcatcggcctgatgtccggcacgtcgctcgacggggtcgacggcgtactggccgacttttcggacggccgcatcgctgtgcgggcctattccacggccccgttccccgatgcactgcgcgccgaactgctggcgctgaacacgcccgacgacaacgagctgcatcgtgccgccctggctggcaacggcctggcccgggtctatgccggcgtggtcggccagctcctggcggacagcaacacccccgccggcgatgtaacagctctcggcgcccacggccagacggtgcggcaccggcccatcgagttcgacggggtcggctatacgctccagatcaacaatccctcgctgctggccgagctgaccggcatcgacgtggtcgcggacttccgcagtcgcgacctggcggctggcggccagggcgccccgctggtgccggcttttcaccgcgcactcttcgcgcgggccggcgaatccgtggcggtactgaacatcggcggtatttccaacctgagcctgctgcccgcggcagatgcggcgggagatccgacggtgcttggcttcgattgcgggcccggcaatgccctcatggatcactggtgccagcttcataccggccagcccttcgaccgcgccggccaatgggcggccagcggacaggtgctgcccgagctgctcgcgcgcctgcgggccgaggcctattttgcgaagccgccgcccaaaagtacggggcgcgacctgttcaaccccgcctggctttccgcatgcctaggcacggccacggccgccgcgcccgccgatgtgcaggccaccctggccgaattcactgccagcgtctgtgcggccgattttttgcgctacggaaacgatagcaagctgctgattgtttgcggcggcggcgccttgaacggccacctgctcgcccgcctgcgcgcgctgctgccgggcgttgaagtggccgcctccaccaagcacggcctgccgccgcagcaggtcgaggctgcggcctttgcctggctggcgcgcagcacggtccggcgcgaggccggcaaccttgccagcgtcacgggagcgcgcggcgctcgcgtgctcggagcggtctatccggcgtgaccggagcggggggcgatgccccaaacaaaaagccgcccgaaggcggctctttcaaaaaacgcgacgaagagcgactcaagccgagaagctggatccgcagccgcaggtgctggtggcgttcgggttcttgatcacgaactgggcgccctgcaggtcttccttgtagtcgatctcggcgccgaccaggtactggtagctcatggcgtcgatcagcagcgagacaccgttcttggtcatggtggtgtcgtcttcgttcgtgatttcgtcgaaggtgaatccgtactggaagcccgagcacccgccgccctgcacgaacacgcgcagcttgaggtcgggattgccttcttccgcgatcaggtcggccaccttggcggctgcgctgtcggtgaagacaatcggttcgggcatctgggtctggacgttttcggcaacagcgctcatgtggggtaactccttgagggccggacatgcggccaatgaaccaatgctactgcaatgccgcattctcggctggccagcgtagcgtgcacccaatgcaagtggggtcgaacatacgccccccaaggtgcggcaatgaaaaagccgcccgaaggcggcttttgtccgtagcgaacagtatcagcgcttgctgaactgcttgcggcggcgtgcagagtgcagaccgaccttcttacgttcgacttcacgtgcatcgcgcgtgacgtagccggcctggctcagcaccggcttgaggcttgcgtcgtagtcgatcagcgcacgggtgatgccgtggcgcgttgcgccggcctggcccgattcaccgccgccggccacgttgaccatgacgtcgaaggtttcggtgttattggtcagcaccaggggttgcttcgcgatcatgatcgaggtttcgcggccgaagaactcttgaatgtccttgccgttgaccgtgatcttgcccgagccctttttcagaaacacacgggcgacgctcgatttgcgacggccggtgccattgttccattcaccaatcattctcaaggctccttacagttccagcactttgggctgttgggcggtatgcgggtgctcagcgccaccgtacaccttgagtttcttgatcatcgcgtagccgagcgggcccttgggcagcatgcccttgacagccttttccagggcgcggcctgggtgcttggattgcatgtcgcggaagttggtcgccgtgataccgccgggatagcccgagtgacggtagtacaccttgtcgatcgacttggcgccggtgacgcgcagttgcgcggcgttgatgatgacgatgaagtcaccggtatcgacgtgaggcgtataaatggccttgtgtttgccgcgcaaacggagagcaacttcgctggctactcgtccgaggaccttgtcggtcgcgtcaatcacaaaccactcgtgcgtcacgtcagcgggtttggcgctgaacgttttggtcatgagttttctcttgaaaagagggtttggcgagcccttttccacggtcggcgttcctctgacgggaatctcttaggtgggttcaaagtctccgccgcggggctacaaaaacgctgcgaagcccgcgattatatgaagaaatggccaaacagccaatttccgggcttcgggagccctcagcgctggatgcggaccagttccaggctctcgttcgtcacgctggcactggcgcgccggtgtgtggcctcgaacttgacgatccgcctcagttcggggctgtacagaacggcaacgttgaacggcgtgccaacgggcgaggcgcccgtgccatgggaggcgtagatccagccttcgtagctgatgcgcagcacgttgagctccacgccgtccacgcgcgtcgcgtgttcagcgcccaccgaggcgttgagttcatgccgcagccgatcgtcggtggtcgtcacatagtcgaggtgccagcgcatgccaggccggatctcgtccttcgctgcccagccgcccggcggcgacgcgctgtcgaacaggccgccgaccggcgacgtgatggacaccagctgcccgttggccttctcgatccggctgccggcgttgaacgacagctcgtcgccgttgacccggtccaccctatagatcaccggcgaccggttgccggtcagccggtcggtgcgcacgtattcgagcgcgtcgccgacgcgcagcggctcggtcagcggaatgcccgccgcgccggcgctgcggcgggcgccgccttcgggttcacgggcacgcgccgccagctgcgcctgggcgcgggccggcaactccgccagaaactcggccggaatcgcgaaattcaggctgccgccatcgcgggcggcgaaggtggtgatgcccagcaggcggccgtcgctgtcgaacagcccgccgccgctcgaccccggggcgacggcggccgtggtctgcagcagccgcgcctcgccgtcgccgccgcgaaggccggacaggaggccttcgctcagggtgttttccagcccgcgcggattgccaatggcgtacacgcgctgaccgacgcgcgcaccgccggcgggcgccagcgtcaccggcggcgccgtgaagttggcgaccttgatctggcacagatcgcgccccgggtccgggtattcgagcgtggcaccgtaggtgacgttgtctcgcttgaccacgaaattactggccttggccagcacgtggcagttggtgacgaggcgaccgggcgcaatcaccacggcgctgccggcgcgcaacggacgctcctgcgcgtcgaaggtgcgcaccgcccagacgctgtccgacaccttggcgaacaggacgtcgggctccagcgcggcggcgctgccggcggccgaggcgatcgccaggaaggcgaccgcggcgcgcagccaccgcgcggggttcatcaacgtcggcttcacggcttggcaggcagcaagccgcgcaggtcgtccatcgagacccgggcgtcgggcgcagcggacggcgatggcgcagcaggcgccggtcgcgccggaatggccggggccgctggcgcgaccgccacgggaggaggcaccgctgccggcgcaggcgcgggcaacggcacaaccgcgacggcggtcttcggcgccggcgcggtcgccatctcggtcgtcccgatcttcataccggccgtcgcctggtccccggtctgtgcgctgcggtcgaagctgcgcacctcgccgaagatcagctggatccagctcggatagttgaatcccgctccggtgctggcgtcgatcaccgcgccgagcacgccgccgatcatcacgttgccaaccatgccgacattggcgcgcgaaatcgcctggccgcgggcgggcggctggccagcctgggtgcattcgatgctcaggttctcgcccgagcgccgcaccggcagggtcaggccggagcgcacctccacatcattgcggtcgttcgagacccggcaccgggccccgtcgacgaccttgccggcgggcgacagggtctcgatcttcacgttctgcgtggtcccgtgcgttacggaggcgcagcccgtcaaaatagacaaaacgcccgcgccgacgcacaggccccaaaatcgccatccggctcctcgcattgctgcccctcgttgcttgtttgtaaatcaatgtagcgccgcgcgagtctagcgctcccctttccactctttcaggcctcattccatgttcagttaccgccacgcgttccatgccggcaaccacgccgacgtgctcaagcacacggtgttgattgccacgctcgaccacctgcttgaaaaagaagccgccctgaccgttgtcgacacccacgccggcgccggcctgtaccggctcgacggcgactacgccggcacaagcggcgaagcggccgaaggcgtgctgcgcctgctgtcggagaaaaaagcccctgcggcccctgcccctgccgcgaagtcagccgccaaaaaagcagcgccagaagccgaaacccccttggccgctgcgattgcacgctacctcagcgtgatccacgacttcaaccccaagggcggcgcccgcatctatcccggctcgcctttcatcgtgcagcacctgctgcgagaccacgacaagctcaagctgttcgaactgcacccgaccgatgcccgcacgctggacgccaacatcgcccagctcgaggcgggccggcagatcgcggtgctgcgcgaagacggtttcggcagcgccaccaagttcctgccgccgccctcgcgccgcgcgctggtgctgatggatccgagctacgagatcaagagcgactacggccgcgtgctcgacttcgcggccgaggcgctcaagcgctttgcaaccggtacctacgccatctggtaccccatcattccgcggcccgaggcacacgacctgccacggcggctcaagaccctggccaccaaggccggcaagccctggctgcacgccacgctcacggtcaagtcgagcaagctgatcaccaaggagacgggcgaaacccagcgcccggggctgccggccagcggcatgttcctgatcaatccaccctatacgctgaagccgctgctggccaccgccctgccccagctggtggagcggttggcccaagacaggcacgccgccttttcgctcgattcgggcggctaggcttcttcgccttcttccctgcgcggcttatcggcggcggcgcggcggcacgttggccttgcgcggtgcaggagcagccgctggcgtttgggcatcggccgcttcgaccccggagccaccgcaacgcatgccttcgcggtcgatgatggtcagcgcgacttgcttgatgccgagcccgatcagcccgatgcgctcggccgcggcgcggctcaggtcgatgatgcggccctgcgcataaggcccacggtccgtgatgcgcaccagcacctcgctgccgttgaccaggctgcgcacgcagacacgggtattgaacggcaaggtcttgtgggccgccgtcagggccgtcatgtcgaaacgctcgccgctcgcggtcttgcgctggtggaacggaatgccataccaggacgccccgccgcgctcgaagatctcgcgggggccatcgcccggcacgccgtcgtcgggccccaactcgccggtacccgacacggtcaggtcgtagcgcaccgaaggcacgttcgatcgggccggcgcacccgggggaacagccaactggcgcggcaggggcaggagcttggcgtccttgtctgcctgcccgccctcggtggcgggaggcatggcacagccggccagcgcgcaagctgccgccacgagcgcgacgcgaaacgccgcgcgcagcgaacaccctgctcctgcacgcacccccttcaaccgaggcgctccaataccgccagcgtcgccgtcgactggttcatcgtgtagaagtgcagcgccggtgcgccgccgtcgcagaggcgcgcgcaaaggtcggtcaccacgtcgaggccgaaggccttgatggatgccgtgtcgtcgccaaagccctgcagccgcaggcggatccagcgcgggatctcggcgccgcaggcatccgagaagcgcatgagctgcgtcgagctggtgatcggcatgatgccaggcacgatgggcgtgtcgaggccgagcttgcgggcctcgtcgacaaagcgaaagtaggcttcagggctgaagaagtactgcgtgatcgccgaatcggcgccggccttcatcttggcggcaaaggcttgcaggtcggcttcgggcgagcgcgcttgcggatgcacctcgggatagcacgccacctcgatgtggaaatcgcggccggtctcttcgcggatgaaggccacgaggtcgctcgcatacaggaactcgccgccgatgccgtagccgctcggcaggtcgccgcgcaacgccacaaggcgcttcacgcccatggccttgagctcggccagctgctcgcgcaccgtggcccgcgtggcgccgatgcacgagaagtggctcgcggcatccacgccttcggacaggatctcgcgcaccgcaccgaaagtgccctggtgcgtggagccgcccgcgccgtaggtgaccgagcagaactcgggcttgcgcgcatacagctgctggcgcaccgcgcgcagcttgaccgcgccttcgggcgtcttggtcggaaagaattcgaaactgagtggaaggcgcacctgcgtctcctcaagagccatccgcgccaacagcgcgcacggcgtgaatgaaaaactcacggttgccgtcgccaccggcaatggggctgtcgaaccattgcagcacacgcagatcgagcgcctcgcaggcatcgcgcaagcgcttttcgaccaccgcatacatcgacgcgtcgcgcacgatgccgcccttgccgacctgccccggctgcagttcgaactgcggcttgaccagcatcagcaggtggccgtcgtcggccaggaatggcaccacggccggcagcaccaacgtttgcgagatgaacgacagatcgccgacgatgaggtcgaagcgcagctcggaaggctcttcgccttcttcctgaaggtcgtccggcgacaaagctcgcgcattgacgccctcgatggcaaccacgcgttcgtcctcgcgcagccgcgcatgcagctgcccgtggcccacgtccacgcccaccaccttcgctgcgccgctttgcagcaggcagtcggtgaagccgccggtcgactggccgacgtccaggcacagcttgcccgctgcatccacaccgctggccgccagcgcgccttcgagcttgagtccgccgcgcgagacgtaccgcgcctcggccgcgtcgtcgagctcgagctcggcggactcgggcacctcgtcgcgattcttcacgaccgagcgccacgcgtctgcggtgcccgcatcgcgccaccgcatgccgccggcaatcagccgcacggcctgcgagcgcgacgcggcaaggccgcgttcgaccagcaattgatcggcgcgcatcagtaccggtacgtgtccgccttgtacggacccgctttgtcgacgccgatgtaggcggcctgctcgtcggtcagctcggtgagcatggcgccgaccttcttcaggtgcaggcgcgcaaccttctcgtcgaggtgcttgggcagcacgtagaccttgccggcctggtaggcgtcgggcttggtgaagagctcgatctgcgcgatggtctggttcgcgaaggacgaagacatcacgaagctcgggtggcccgtgccgcagcccaggttcacgaggcggcccttggccagcaggatgatcttcttgccgtcggggaacttgatgtggtcgacctgcggcttgatctcttcccactcgtacttttcgatcgacgccacgtcgatctcgttgtcgaagtggccgatgttgcagacgatggcctggtccttcatcttgaccatggtgtcatgcgtgatgacgtccttgttgccggtggtggtcacgaagatgtcggccttgtcggcagcgtattccatcgtcacgaccttgtagccttccatcgcggcctgcagggcgttgatcgggtcgatttcggtgacccagacttgtgccgacagtgcgcgcagggcctgggccgagcccttgcccacgtcgccgtagccggccacgcaggccaccttgccggcaatcatcacgtcggtggcgcgcttgatgccgtccaccagcgattcgcggcaaccgtacaggttgtcgaacttgctcttggtgaccgagtcgttcacgttgatggcgcggaacagcagcgtgcccttggcgctcatctcgttcaggcggtgcacgccggtcgtcgtttcttcggtcacgccgatgatctcggccgacttgcgggtgtaccaggtcgcatcgaccgccagcttggccttgatggccgcgtagaggatgcgttcttcctcgctggtcgggttggcgagcacgcccaggtctttttcggcgcgctggcccaggtgcatcagcagcgtcgcgtcgccgccgtcgtccaggatcatgttcgggccttcgcccgtcgaacccttggggccgaagtcgaagatggcgtgggtgtagtcccagtagtccttcagcgactcgcccttgatcgcgaacaccggcgtgccggcggcggcgatggcggcggcggcatggtcctgcgtggagaaaatattgcacgaagcccagcgcacggtggcgccgagcgcctgcagcgtctcgatcagcacggcggtctggatcgtcatgtgcagcgagcccgtgatgcgcgcgcccttcagcggctgcgccttcgagaactcttcgcggatggccatcaggccgggcatctcggtttccgcaatgcggatttccttgcggccccaggcggccagcgacaggtcggcaatcgcctggtcggcggtggaaacgggggtgggcttgagaacagcgctcatgagaactccaacaaagctagtttgaaaggtgccactgcgttcgggggaaaagactcaccgcgagaacagcgggtgagcgtggttgcgatgtggtccgagcctcacgcctgacggcgctgcaacgctcctcggaaccgcggattgtagacgggcgggcaaggcgagccaatcgccgggatatcccatatcccggaaagcgcgtttcgccaaccaagggaaatcccgcaggcaaattttcaggccgggcacctccgcaatgcccgcccggcgtatcgtggcagcggactttgccgtccggccggtccttgcatccctcaccgttcacacgacaccaggagataccgcaccatggccactgccaagaaagccgccgcgaagaaaaccactgacagcagcaacaacagcagcaccaagacggaggcccctggtgccgccgacatgctcaatccaatgaagaatctcaaggccatgaccgaccggctgcaggagctcaacctgaccggcggcgcgagcaagctgctcgagagcggccagaaggaccttcaggcactgatgcaggccaacgaaaagtcctaccagggcctgcagaccgtggtgcagcggcagaccgagatgatcaagagcgccatcgccgagtggcagacggccgccaaggagatgcccggcaaggaccccaaggccaacctcgccaagctcgacgagctcggccgccagtcgttccagcgcgccatcgacgacatcaaggaactcgccaacctcgccgccaagtcgcaggccgatgccttcgaactggtgcgccagcgcatccaggccaatgtggacgaagtgaccaagatgctgaagcgcaagtaaggcgttttcggcggctcgggcgggcggcccgggaccgcccttctaaaatcgggcattcccctgcagattgcccaccttgtcttttcttgccgaaacccgccgccgccgcacctttgcgatcatttcccaccctgacgccggcaagaccacgctgaccgaaaagctgctgcttttctccggcgcgatccagatcgccggctcggtgaaggcgcgcaaggcctcgcgccatgccacctccgactggatggaaatcgagaagcagcgcggcatctcggtggcctcgtcggtcatgcagatgctgtaccgcgaccacgtgatcaacctgctcgacacgcccggccacaaggacttttcggaagacacctaccgcgtgctcacggccgtcgactcggcgctgatggtgatcgacgccgccaacggcgtggaatcgcagacgcgccggctgatcgaggtttgccgccagcgcgacacgcccatcatcaccttcgtcaacaagatggaccgtgaggtgcgagagccgctcgacatcctggacgaggtggagcgcgaactcggcatgccctgcgtgcccatgacctggcccgtgggccagggcaagtcgttccgcggcatcatgaacctgcgcacgcaggcgatgacggtgttcgagtcgggcagcgagcggctgccgcacgacttcgagaccattccgctctcggagcgcgacacgctgaccaagcgcttcggcgccgatttcgaatccgccatggacagcatggagctggccaccggcgcctcgcccacctgggaccgcgaggccttcctggccggcaagcaaacgcccgtgttcttcggctccggcgtgaacaacttcggcgtgatggaagtgctcgatgcgctggtcgacctcgcgccctcgccgcagtcgcgcaccagcaccacgatggtcaaccgccaaccggtggtgaaggagatccagcccgaggacagggacttcgcgggcgtggtgttcaaggtgcaggccaacatggacgccaaccatcgcgaccgcatcgccttcgtgcgcatggcctcgggcaagtacacgccgggcatgaagctcaaggtgcagcgcacctcgaaggagctgcggcccaccagcgtggtcacgttcatgagccagcgccgcgaagcggtcgaagaggcttatgcgggcgacatcgtgggcttcaccacccacggcggcgtgcagctgggcgacaccatcaccgacggcgcgagcctgcagttcaccggcctgcccttcttcgcgccagagctgttcatgaccgtgattctgaagaatccgctgcgcaccaagcagctgcagcaggggctggcccagctcggcgaagaaggcgccatccaggtgttccgtcccgagatcggcggaccgatgctgctgggcgccgtcgggcagctgcagttcgaagtggtgcagcaccgcctgaaggccgagtacgacgccgacgtgcggctcgaaggctgccagtacaccggcgcgcgctggatcacggccgacacgccggccgagctgcgcgagttcgtcaacgcctatccgcagcgcatggcgaaggacgcagccgacacgctggctttcctgtgcacctcgccgtatgacgtgcgattggcgcaggagcgctttccgaagattcacttccatccgctgcgggagcatgcggggttggcgctgcagagtgccggctgagccaggcatgcgccagccgacctcgctgccccactcgccccatcatctgctgccgctggcgcagtgggcggcagctgcgcgcagcaatctgatcggcgtgttcaccgacatcgacgacaccctcaccaccgaaggcgccatcacgcccgatgcgctgaaggcgctgggcgatctgaaagcggccggccttcacgtcgtggccatcaccggccgccccgtgggctggagcgtgcccttcgtttccgcatggcccgtcgactccatcgtggcggagaacggcgccgtcgccctgctgcccgtgccaggcggcaagctgcaaaagcgctaccagcaggacgcggcaacccgcgccgccaacttcgatcgcatgcaggccgtgctggcgcgcatcgagcgcgagatccctggcgccggccgcgccaccgactcgccgggccgcgagaccgacatcgccatcgaccacagcgagttcgtgcagctgagcgaagagaccatcgcccaagtcgtggccctgatgcgcagcgaaggcatgcacgccacggtcagcagcatccacatcaacggctggtacggcgacaacgacaagctcgaaggcgcgcgctggatcgtgcgcgaactctggggccgcacgctcgacgacgagatcgggcgctgggcctatgtgggcgactccaccaacgaccagttgatgtttcgcaccttcgctcacagcatcggcgtggcgaacgtggcgcgcttcgtgccgcagctggagcatctgccacgctacgtgaccgagggcgagcgcggcgcggggttcgccgaagcggcgcgcgccattctctcggcccgcgctactcgctgaccggcaggctgcgcgcgttgcggcgcagcactgcccattggcgccagatgccgaaggccgcgatcagcagcagcaccgccgcataaccttccaccgtgttcagcaggccgagcggcttcaccaggaagcccgccagcatcgcgggcaggctgaacgcgaggtagcagaccacgaagatggcggcgaagagttcgccgcgctcgtgcgaatcggcgagcggcgccagcgtctgcaccagcgccgagaacgcgccgccgaagcccaggcccgcgatcgcggtgccgacgaagaacagcgcgagcgacttcgtcgcgagcgacgccagcagcaagaccagaccgaccgcgatgctggccgcgccgaagacgacggtccgcggtgcggggaaacggccgagcagcgtgggggcgagcgcgccgaagcccgagagcaccgccaccgtgaggccgttgaccacgccgttgtcgatgtggaacacgtgcagcatcagcgacggcgcgagcgacaggtacagcccgcccagcgcccacaccgcgatgaacaccggcaggccgcgcacgaagtcagcccgcgcccgcacgggaatcgacacgcgcggcaccagcgaggccagcgcgccggcgcgcggcgtgacggtctcgggcatccacagcaccacgaccgcgccgaccgcgaacaccacggccagcacaccgaacaccagcatcaccggctggacggtgaacctgacagccatgccggtcagcagcgcccccaccgcaaggcccgcgagcggcgacacgctggtgatcatcgcgcccaggcgcttgcgcgatgccggcgccgcctcgaccaccgccgcgctcagcgcgccgctcgcgacgcccgttgccacgccctggacgacgcgcgcgacgatcagcccggcgatgtcgtgcgccaccacgaagagcaccattgccaccgcctgcagcactagcgccgccagcaccaccggccgccggccgatgtggtccgacagcgagcccgccacgagcagcgagatcaacagcgcaatcgcgtagatcgcaaacgccaccgtgagcatcgacgccgagaagccccaggcgtgctggaacacgacgaacagcggtgtgggcgcggcggccgcgaagaagaaggcgaagagcacggcggccagcagcgggaaaccgaccgctgccggcaggcgccagggcttgggacgggcggcgatgtcggcggtggcgacggcgagttcagggcaggaggaaggcattggagatccttaacgcaacttttttagcttttgcgattctagacctgtagattcactaaagcaaacatctttgcgttaaagtcctcacatgaaccatgttgtccttcccaacaagcgtcccggcggccgcagcgcccaggtgcaggcgctggtgcgcactgccctcgaacaactggtggccgaacaggggcgcgagcgcgtcaccgtgccggccgtggccgagcgcgcgggagtcagcgcctccagcatctaccgccgatggggcgatctgtcgggtcttctggccgagacggccacgcaccggctcgacccgaaccggccgctgccgaacaccggcgcgctgcgcgcagacctgaccgcgtgggcgcaggaactcatcacgcacctggcgcagccctgcagcaagtccttgttgaaagccgcggccgcgctggccaccggcgacgcggagacggattgcctccgcaaccgccgcagggaagcgctgacgctggtcgaacaggcgcacgcccgcggcgagcatgcgcccgaagcgcagcaggtgatcgatcacctgatcgcgccgatcgtgtttcgtctcgtgttcggcgccgatcccgtgaagccggagttggcggagcggctggtgggggagttgtttgcgatcagttcgtcttcggttgttccttcgccaaccccagcttctcgataaccaccttctctttcaccaccgtgtcctgcgcaaacttggtgtacgtcgccgaactcatgtagttcggcagcatgtcgtagcgccccagcgaagccacatagctcggctcttccatcgcctgcttgaacgcgtcgtgcagcttcttcaccacctcgggcggcgtgcctttgggcgcgccgatgccgaagggcgagttctgcacgatgtcgtagcccagctctttcagcgtcggcgcatcggggaacttggccaggcgcttctcgccccaggtgttgagcacgcgcagcttgccggcctcgacctgcggcgcgaagccggtgctgtcggcggcggccatcagctggccgctgaccaccgcgagcatcaggtcggcgctgcccttgtagggcacgtgctgcaactcgatgccggccttctgcgcaatgatttccgtcgtgaggtgcggactggtcaggttgccggtcgagccgtaggtgagcttgccggggttggccttggcgtaggcgacgaagtcggcccaggtcttgaacgggctgtcggccggcaccacgatgccgaaggcatagcccgtgacgttgagcacgtagctgatgtccttgagcggatcccagttgatcttggtggtgtagccgaggcggaacacgccgagcggaatctgcgccagggtgtagccgtcgggctgcgaggtctgaagcgcctgggcgggcaaggtgccgccggcgccgggcttgttctcgatgatgacgggctggccgatgatcttgcttgcgttgtccgcaagctggcgcatggtgatgtcggtcgggccgcccgccgggaaggcaatgatcagcttgatgggcttggcgggaaaggcctgcgcgaacgccgccagcggcgaaaggagcccgcacgcggcaagcgttgcggcacagagaagggatcggcgggacatggctggctcctgaagcaggggaaaagggcgcattgggccctgcccttcccgccgcggcaatcggtgctcacccgactgctgtcacgtaggcggctcagcccgccgcctgctcgaaaccctccagcacgttgacggcgttgacacccacttccgccaccgcatagccgccttcgaaaacgaacaccgtgggcaagccggcgcgggcgaggtcttcgcccatgcgcaggtagtcgtcgctcttgaggcgaaagcccgcgaccgggtcgccctcgaacgtgtcgacgccgagcgacacgaccagcgcacccgcgcgcaccgcggcaatgccgtcgagcgccgtcttcagcgccgcgcgccaagtggcaaagtcggtgccgcgcgccagcggcaggttgtggttgaagccgagcccggcgcccgcgccgcgctcgtcggcgtggcccaggtagtacgggtagtcggtcatcgggtcgccatgcaggctcgcaaaatgaacgtcgctgcgctcgtagaagatggcctgcgtgccgttgccatggtggtagtccacgtcgagcaccgcaacccgttccacccccgcatcgcgcagcgcctctgcagccaccgcggcgttgttgatgaagcagtagccgccgaagaaatcggcgcccgcatggtggcccggcggccgcgtgagcgcaaaggcggcgcgctggccgccgatgacgcgctgcgccgcggtccaggcgcaggcggcaccgtggcgcgcggcagcccagctgccggccatcagcggcgtgcccgcatcgaacgcaaacagccccatgcgcgcaggaaagctcttgggcagcacatcggtgcgcatgccgcgcgtgggccagtacgaaggcagcgcatcgcgcgacgcgttggacggatcgagcgccacccactcgtcccacgcatgggcgatgaagtccaggtagcgcggcgcatgcacccgggccagcagggcctcgtcgaaggcgtcgggcagctgcagcgggcccagggcgcggcgctccagctcatgcttcacatggtcgacgcgggcgggcacctcgaagcacggcaccagctcgccgcggaacatttcgactttgccttgatgcagtgcgtgctggtcgttgtagatggtgagcatgccgccatcatgccgcacgccgcagcaccgcacggcgccggccggaggccgtcagcccgaacagatccttcgggtcgtcgagctcgggcaccagcgcaatctgctggccgatgccgcgctcgatggccagctgatggatgtagcgcagcgcggtgtagtcctccagcgcgaagccgaccgaatcgaacaccgtgacctggtccgcgttctcgcgtcccggcaccttgccgagcagcacctcccacagttcgtgcaccggaaagtcggccggcagctgctggatttcgccctcgacgcgggtctgcggttcgtactcgacgaacacgcgcgccaggcgcagcacgtcggggtgcagttcggtcttgccgggcgaatcgccgccgaccgcgttgatgtgcatgcccggctcgatcatctcgggcgcaagcacgaccgcgtggccctggtgcgccgtgaccgtggtgacgatgtccgcgccgcgcacggcctcggcaaccgaatgggcgcgcaccacctcgagcggcgtgcaggcggaaagatggcgcaccagtttttcggtggcgtgcgggtcgatgtcgaacacgcgcacttcctcgatgcccagcagcgcatggaaagccagggcctggaactcgctttgcgaaccgttgccgatcaacgccaggctgcgcgagccgggccgcgcaagggcctgcgccgccatggccgaggtggccgcggtgcgcagcgcggtggtgagcgtgagctccgacaacaacaccggatagccggtatcgacctcggccagcacgccaaaggccatcaccgtgggcagcccgaccgccgtgttgtgcgggtgcccgttcacgtatttgaaggcgtaggcgccatcgtcggccaccggcatcagctcgatcacgccaaggtgcgagtggctggccacgcgcgccttcttgtcgaactcgcgccagcgcatgaagtcgtcgcgcagcgcatcggccagggccttgaggaattccggaacgccggtttcgtccaccaggcgaaccaggctgtgaacatcgatgaagcgggtcatggcatggctccttgcgtagcccgggcacggcgcttcatcccctcacatgtttactccaccatggctgattcaggatgcgcctgcgccaagggttcaagccattctgcgcctgcctgcatcaccgcgccagtaccggcgccaaagcgacgccggtgtgggtagccaaacgcaccacctcttccggcggcgccgccgcaacgatgcgcccgccggcgttgccgccttcagggcccaggtcgatgatccagtcggcttcggcgatcaggtcgaggtcgtgctcgatcaccaccacgctgtggccgccgttcaccagccggtgcagcacgtggatcagcttttcgacgtcggccatgtgcaggcccacggtcggctcgtcgagcacgtagagcgtgtgcggcgccttctggccgcggcgcgtgatgtcgtcgcgcaccttgctgagttcggtcaccagcttgatgcgctgcgcctcgccgcccgagagcgtgggcgacggctggcccagcgtgaggtagcccaggcccacgtccttcagcaattgcagcggatggctgatgttgggcatggcggaaaagaactccaccgcctcgtccacttccatctgcagcacctcgccgatgctcttgccgcgccagctcacggccagcgtctcggggttgaaacgcgcgccgtggcacacctcgcagggcaccttcacgtcgggcaaaaagctcatctcgatggtgcgcacaccggcaccgtcgcagccgggacaacggccttcgccggtgttgaagctgaagcgcgccggtccgtagccgcgcgccttggcttccagcgtgtcggcaaacagcttgcggatggtgtcccagaagccgatgtaggtggccgggcagctgcgcggcgtcttgccgatgggcgtctggtcgacctcgagcacgcggtcgatggtctcgtagccctccacgcgatcgcagccggaccaggccgggcgcttgcccgcagcgtccgcgtcgcggccggccttggtcatgcgctggacgacgatggcatgcacgctggccagcagcacgtcgcgcgcgagggtggacttgcccgagccgctcacgccggtgaccaccaccaggcggtgcagcggcagcgtggcggtcacgtcctgcaggttgtgcaggtcggcgccatgcacggtgagccattggccaccgtcttccgccttcgggtcgggtgagggaacaagccgccgtgcgtgcagcggatgcttgatggcatcgcgcaggtatcggccggtctgcgagtcgcccgccgcctggatgtcggccaccgagccttcggccacgaggcgaccgccccgctttccggcgctggggccgatgtcgatgatgtggtcggcgcggcggatggtgtcctcgtcatgctccaccaccaccagcgtgttgcccttgtcgcccagcttgtgcagcgcgtcgagcaggatctggttgtcgcgcgcgtgcaggccgatggtcggctcgtcgagcacgtagcaaacgccctgcaggttgctgccgagctgcgccgcgagccggatgcgctgggcctcgccgccgctcagcgtgggcgccccgcggtcgagcgtgaggtagcccaggcccacctcttcgagaaactcgagccggctcctgatctcgggcaccaggtcgcgcgcgatctcggcctcgcgtcccgtgagcgccaggccttcgaaccactgccttacctcggtcacgctcatgcgcgcgagctcggtaatgccgatgccgctcatcccgtcggccggcgaggcgccgaagctcaccgcgcgcgccgtggcattgagccgcgtgccttcgcaggtcgggcatgccacgtcggccaggtcttccacctccggctcggcaaaggtctgctcccggcccttgctgtcgtcgtcgcggatggaatcgtcgaagaccttgcgctggtccttgctgagcttgacgccggtgcccacgcagtcggggcaccagccgtgcttgctgttgtagctgaacaggcgcggatcgagttcggcgtagctggtgctgcagaccgggcaggcgcgcagcgtggagaacacgttgacgcggccgatgccgtgagccgacacgccggccatcatcgcggccttgaggccatcgagctggctcagcacgtgcaccacgcccttgccgtgttcgagcgctttggtcagcgcctcgcgcagttcgttttccttcgaaggcagcacgtcgaggctggccaccggcagctcgatgctgtgttccttgaagcggtcgatgcgcgggaagcccgtggtcggaagaaagtcgccgtccacgcgcagatgcgtgaagccgcgtggccgtgcccagtcggccagctcggtgtacacacccttgcggttgctcaccagcggcgcgagcaggccgatgtgctggcccttgaagttgcgcatcagctgcgccgcgatactgtcgggggtctgtggctgcacggccgcgccgtcgtgcgtgcaatgctggatgcccagcttcacgtacaggagccgcaggaagtgccagacctcggtggtcgtgccgaccgtgctcttgcggccgccgcgcgacaagcgctgctcgatagccaccgtgggcggaatgccgtacaccgcatcgacctcgggccggcccgcgggctgcacgatgctgcgggcgtaagcattcagagattcgaggtaccgccgctggccctcgttgaacaggatgtcgaaggccagcgtcgatttgcccgaaccgctgacacccgtcaccacgctgaacttgccgcgcggaatgttcacgctgagattcttcaggttgtgctcgcgcgcattgacgatctcgatggcgttgctgccgggcgccgtcttggcgttggcaatgtagcgccgcgccgcgcgctcggccaccttgtaggcctcggggccgatggccagctcgtagtcggccagggctgcgccggtgagcgaggcgcggttctcgcgcagctgctcgggcgtgccctcggccaccaccatgccgccgccctcgccgccttcggggccgaggtcgatgcaccagtcgctcgcccggatcacgtcgaggttgtgctcgatgacgatcagcgaatggcccgcgtcgagcagcttgcgcagcgcgcgcatcagccgcgcgatgtcgtcgaaatgcagcccggtggtcggctcgtcgaacaggaacagcgtgcccctgcgcgccaccgactgcttgctcgccgtcgcgctcttcgcggcctccgccagaaagcccgcgagcttgaggcgctgcgcctcgccgccgctcagcgtgggcaccggctggccgagcttcacgtagtcgagccccacgtcggagatcggctgcagcacgcgcagcacgtcgcgatcggcttcgaacaccgccgccgcctccgccacggtgaggtcgagcacgtcggccacgttgtaggcgcgccccttgcgctcgaccttcacttcgagaatctcggggcggtagcgcttgccgtcgcaatcggggcagcgcaggtacacgtccgacagaaactgcatctccacgtgctcgaagcccgagccgccgcaggtcgggcagcggccgtcgccggagttgaagctgaacttgctcgcggtatagccgcgctggcgcgacagcgccgcggtggcaaagatctcgcggatcgcgtcccacgcacccacgtagcttgcgggattggagcgcgccgtcttgccgatgggcgactggtcgacgaagaccacgtcgccgaggtgatcggcgcccagcatgcggtcgtgcgcgcccggcgtttcggtggctttgccgaagtgccgcatgagcgcgggcgccagcacgtcctggatcagcgtcgacttgcccgagccgctgacgcccgtcacgcacaccaggcgcgcgagcggaaagtcgaccgtgatgctcttgaggttgtgctcgcgcacgccctccaggatgagccggtgcgtgttctcgctcacgagccgcttgaagcccatgccgatcttcttgcgcccgccaaggtactgcccggtgagcgtgtcggcatcgcgcagttggtcggtggtgccatcgaacacgatctgcccgccgcggatgccggggccgggacccatgtcgatcacgcgatcggccgcgagcatcacggccgggtcgtgttcgaccaccaccagcgtattgcccgcgtcgcgcaggcgcagcatggcctcggtgatgcggttcatgtcgcgtggatgcaggccgatgctgggctcgtcgagcacgaacagcgtgttgaccagcgaggtgcccagcgccgtcgtgagattgatgcgctgcacctcgccgcccgagagcgtgcggctctggcggtcgagcgtgaggtagccgatgccgacgtcgtgcaggtagcgcaggcgggtggtgatttcttcgaagagcagcttgagggcctggatttcgccctcaccccggccctctcccgcaagcgggagagggagtgaatcggaaccctccgccagctgaacggtcttgccccctctcccgcctgcgggagagggctggggtgagggctgctgcctgtcgaagaagcgccgcagccgctcgatcggcaacagcatcaaatcatgcaggcaaagccccggcaacgcctcgagctgtgcccgcgtccacttggcaccggtcggcatgaatcgcttggcgggctccagcaccgcatccgcatcttccttgctgccgatgcgccagagcaggctgtccagcttgagccgcgcgccgctgcatacggggcatggcgtgtagcttcggtatttggacaagagcacgcggatgtgcatcttgtaggccttgctctccaggtagccgaagaagcgccgcacgccataccactgcttgttccagttgccttccttgtagttgggcgtgccctcgatcacccagtgcttctgctcgtcggtgagcttgttccagggcgtgtcgcgcggaatgcccgctgcctcggcatggcgcatgaggtcgtcctgcgcctccttccaggcgggggtctggatggtcttgatcgcgccggcgcgcaaggtgagcttgtcgttcgggatcacgaggcccaggtcgaccccgatcacgcggccgaagccgcggcaggtgtcgcaggcgccgacggccgagttgaacgagaacatcgacgggatcgggtcggtgtagcggatgtcgctttcggggcagtgcaggccggtggagaacttccacacgtcggtgggggcattctcttcagcgcccgtggcgtgcacggtgacacgcccgctgccgcgcttgagcgcgacttcaatcgcctccaccacgcgtgaacgctcggcactcgagatacggaagcggtcggccaccacgtcgagcatcttgcgcggccccgtcggcgtggccacttcgcgctccgcctgcacgcgcgtgaagccgctggccgacagccattgcgtcacttcttcggccgacgtgccggctggcagttccaccggaaaggtgaccaccaatcgcggatcgcccgccgcaaccgcccgctctgcaatctccgcatagatgctgtccggcgaatcgtggcgcaccggcagtgcggtctcgcggtcgaacaactgggccgcgcgcgcatagagcagcttcaggtggtcgttcagctccgtcatcgtgccgaccgtggagcgcgatgagcgcaccgggttggtctggtcgatggcgatggcgggcggcacgccctccaccttgtccaccgcgggcttgtccatgcggtccaggaactggcgcgcataggcggagaaggtctccacatagcgccgctggccttcggcgtaaagggtgtcgaatacgaggctcgatttgcccgagccgctcggcccggtgaccacggtcatctcgccggtgcggatgtcgaggtcgaggttctggaggttgtgctggcgcgcgccgcgaatccggatggagccctgtgtcatgagtgccttggggggtggggcaaacattctagggagtggtaagtgacggattcgtgcactccgtcacatgatccacgcccgtgcaggggtttgtaccgattcagttttagacactttatgtaacaaatagcacctttgtttacgtttccatctgcattgggaagttatccatgaacaagctgcatgtgctttgcgccgccgtattggcactggccgcgacggccgcgcccgcccagatcctgatcggccagaccgcgggcctgaccggttcggtggccgcgggcgtgaatgaaaccatcaccggctcccagctggtgatcgatgccgtgaacgcgcaaggcggcctccacggcgaaaagatcgaagtcctgcgcatggacgacggcttcgacgtcaagcgcgcgagcgagaacgcgcgcgtgctgatcgaagagaagaaggtcgtagcgctcttcatgagccgcggcacgccgcactcgcaagccatcatcccctggctcgacaagcacgacgtggcgctggtcggcccttccaccggggccatggcgctgcacaagccggttcaaaagcacgtgttcaacgtgcgcgccacctaccagcgcgaagccgagaaggcaatccagcacctgctcaccaccggcatcgcgcgcatcgcggtagtgcacgtgaccgactccttcggacaggacgcgctcgagggcgccatgacgggtttctccaaagcccaggccaaaccggtggtcaccgtgcccgccgaccgcgaaaagcccgactacaagaccatcgtgccgaccatcaaggatgccaacgcgcaggccgtgctgtggatcggctccggcaccgccgtggtcgagggcatcaaggcgttgcgcgcctccggttcggccgcgcaggtggtcaccttgtcgaacaacgcctcgtcggggttcatcaagcaactgggcgatgcgagcaagggcgtcatcgtgacccaggtcttcccgaacgagcggtccatcagctaccccatggtcaaggaagcgctcgtgctgtcgcaggccaagggccaggccgaactctccccggccgccctcgagggctttgccgcggccaaggtgctggtcgaggcgctgcgccgcgccggccccaagcccacgcgcgccaaggtgcttgcggcgctcgaaagccttcgcgcctacgacctcggcggcctggaggtgagctattcgccgcaggaccattcgggcatcgatttcgccgacctggcgatcatcagcgacggtcggttcaagcgctaggccagcagcgctggccccccgcccgcgcggggtggcgcggccctggaaacgactttctctctacttgggggcggcagcaggcgcgggttcgtgcgttgcgtcgccgccgtgcttctcgcccgacatgtcgatcttgtcgccgcccttcgagatgacatagagagcaatggcggcaaagatgatgaagccgacaacgagtttccacatggatcttgtctcctgatgatgatgatgatgtgagggttcaagaaaaaggcctcatgccgacggcatgaagcccctttgttgaacggagggccggcttgcgccgccctccttctgaacctgcgttcagtcgttcgcgtagatgtcgacgtccttggtttcccggatgaacagcgtgccgatgaccagcgtcattgccgcgatgatgatcggataccagaggccgttgtacatgttgccggtggtcgccacgatcgcgaaggcggtggtcggcagcaggccgccgaaccagccgttgccgatgtggtacggcaggctcatcgaggtatagcgaatgcgcgtcgggaacagttcaaccagcatcgcggcaatggggccgtagaccatcgtgaccagcagcaccagccagaacagcagcgcgacgaccatcaccttgttcatcttcgcgggatcggccttggccggatagcccgccaccttcagttcctcggtcacgcccttcttgaaggcggcgatctctttggcggaggtttcgtcgaacttcaggttgaccacgttgcccaccggggcctcgatggtcttgctgccgatcttgatgatggctttggagccgggcgcaccttcgacgttgtcgtagctcaccgagttctgcaccaggtagcgcttggcaatgtcgcacgaactccggaagtcgatttcacgcgcaaccgggttgccctggaacgaacacgacttgggatccgccgtcaccgtgacgccggcggtggcttgcgccttcgccaggtcggggttggcatattccgtgatcatcttgaagaccgggaagtaggtcaccacggccagcaggcagccggccatgatgatcggcttgcggccgatcttgtccgacagcgtgccgaacaccacgaagaacggcgtgcccagcagcagcgaggcggcgatcatcaggttggcggtggtgccgtcgaccttcaattgctgcgtcaggaagaacagcgcgtagaactggcccgtgtaccagaccacggcctggccggcggtcaggccgatcagggccaggatcacgatcttgaggttcttccactggccgaacgattcggacagcggtgccttcgaggtcttgccctcggccttcatcttctggaaggcgggcgattcgctcagcgagaggcggatccacaccgagatgccgagcagcgcgatggagaccaggaacggaacgcgccagccccactcgccgaacgcctgttcgccgagccaggtgcgcacgcccaggatcaccagcaggctcaggaacagcccgagcgtggcggtggtctggatccacgaggtgtaggcaccgcgcttgccgtgcggcgagtgctcggccacatacgtggcggcaccgccgtactcgccgccgagcgcgaggccctgcagcatgcgcagcgcgatcaggatcaccggcgccgcaactccgatggtcgcgtagctgggcaacaggccgacgatgaaggtcgacaagcccatgatcaggatcgtgaccaggaaggtgtacttgcgcccgatcatgtcgccgagccggccgaacacgatggcgccgaacggccgcaccaggaaaccggcggcaaacgccagcagcgcaaagatgaaggccgcgcccgcatccaggccgctgaagaactgcttcgcgatgatcgcggccagcgaaccgtagaggtagaagtcgtaccactcgaacaccgtgccaagggaggaagcgaagatgaccttcttctcctccgcggacatgggccggggggccgggtgcggcatccccctcgaatccagtgttgctgccatttgcgtcgtctcctgtgtatgcgttcgttcggtcccggcattcggaaccgtgatgcattcttggaggcgcgactgacccgagcctttcgcgaaactgaaccgacgcttacgaattaaggtgaaacccgcgggcctcgtttcagcctgtaagaaatcggctggttactcagcttttgctgccgcgcagcaaggacggccgctggtcggcgccggcccattccgggccgtcgaaccacgcatcgtcggccaggtaggcgcgcagcatcgcaaggccgtcgaaaccccagaacaggcggccgtcgaccacataggccggcgtgccgaacacgccaagctgcagcgcctcgtcggtgttgcgcttgagcagcgccttgttctcgtcgctgttcatgtcgcgcttcggcttcagctgcgccgccagcgcagccaggcgcgtggcatcgcccgcctcctcgccgccgtgccacacgctgcggaagatggtttcggccgcaaggcggctgatgctgccgtcgtcggaggtcgagagcgcaagccgaaggtgcggaagcgggttgtaggggtgcgaggccggcatctcgatttggatgccgttcgcacggccgagccagagcacatggcggtaggtccagctgcgcttggcggggatctcggccgggccgagctgcccgtggtgcttgaggatcgcgccaagcagcaccggcttgtaggcgacgctgtagctcaggccttcgagggcctccggcagatgctcgaacgccaggtgcgcgtagggcgagatgaagtccaggtagaagtcgatgtgcttcatgcgtgcttgtctcctgattcttccgggatgcgccagatgccggcgcgtgcccgcaactctatcgcgcgccacacgccgcgccgcgcctcgtcttccatcttgctccagcccgcgatctcggggatggtgcgcaggcacccttcgcagaagccgctcaggcggtccatgcggcagaccgaggtacagggcgatggcgcgtcgtcggccgcgcgctgcacggcaacggcccgttcggccagggtttccgcagcatcgaaattcacaccacgtccgccacgggcgcaccggtgagtttctcgaggtcttgcgggcgcagctggaacaccgcgtgcggatggcccgcggccgcccagatctcctcgaagcggaacagctcgcggtcgatcagcaccacgggcttcgtcacatgtccaaccggcgacacgccgccgatggtgaagccggtgcgcgccttcacgaattcggcatcggcgcggccggtcttgccgaccagcgcatcgactttcttctcgtcgacccgcttgtcgcccgaggtgatgaccagcaccgccacctcgtcgctcttgcgccggaagatgatgctcttggcgatctgcccgaccaggatgccgagcgcgtcggccgcctgctgcgcggtgcggcaggcgtcgtcgagcatgcgcggcaaatgcggatggcccgcgtcctgcagcacgcgagaaacacgttgcacgccttcgggcagcgaatgaagttcagcgccgcacatcacagggctcccacggttttcggcgtgctcatcagccggccctcttcgtgcggatcgccttcgacgcccgcgaattcggctcgcgccccagcgcctcgctgatgtacacgcccgcgtcgatcagcttgtccaggtcgatgccggtctcgatgcccatgccgtgcagcatgtagaccacgtcctcggtcgccacgttgcccgtcgcgcccttggcatacgggcagccgccaaggccggcggaggacgactggaagttccagacccccagctccagcgaggccagcgtgttgaccagcgcctggccgtaggtgtcgtggaagtggcccgagatgtggtccacgtcgaaatgcgccagcgctgcctcgatggcggcctgaaccttgcgtggcgtgcccacgccgatggtgtcggccacgtcaacgcgctgcacgccgatgtccttcatcagcttcgccagcatgcccacacgttcgggtgcgatctcgccttcatacgggcaccccaccgtgcacgacatggcgccgcgcaccgcgatgcccttgtcgcgcgccgcggccaccacgggtgcgaagcgctcgatgctctcggtaatcgagcagttgatgttcttctggctgaaggcctcgctcgcggcgccgaacaccacgatctcgtcgggccattcttcgcgcggcgcggcaatggcggcctcgaagcccttcatgttgggcgtgagcaccgagtagcgcacgccggccttgcgtcggatgccgtgcatcacctcggcgttgtcggccatctgcggcacccacttgggcgacacgaagctggtgacctcgatctccttcaggccggcgtcctgcaggcggtgcacgaggccgatcttgacttcagccgagaccggctgcttttcattctgcagtccgtcgcgcgggccgacgtcgacgatcttgactttggtggggagcttcatgggatgtctctgggttcgcagggaaaagaaaaaatccgtccgtccattgtcggccgtctgcgtgcggcgtgctcggcggcgcggttcacgccgtttcacgctgcacgaaatccgatggcggctcggcgggcgcggggacctcagtcacctccagtgcactcacctgcgcgccgtccggcccgctgcgggcccacgcaatcagcgcctcgaccgccacggccggaccgaaggccagcgcctccacgctgccgtcgcgtcggttgcgcacccagccgcgcacgcccaggcgccgtgcggcctgcaccatcgaccagcgatagcccaccccctgcacgaggccgcggacgacgagatggcgggtgacggcgggtggattcatggcgttggcaacatcagtacgacctgggcagtccgggcgcgccgtcagtagccccgcgtgggatcgaccacgccgctgaccggcaggcccttttccatcgcgcggatttttccagcaatctgggcgatggattcctcgcgcagcgtgcgcgccgagccgtgcggcgtgacggtgatcttcgggtggcgccagaaggcgtggtcggcgggcagcggctcgacctggaacacgtcgagcgtggcgccggcaagctggccggcgtcgagcatcggaatcaggtcgtcttcgaccaggtgcgcgccgcgcgcgatgttgatgagatagccgcccggcagcagcttgccgagcgtcttgcggttgaggatgccgcgcgtggcctcggtcagcggcagcaggttgaccagcacgcgggtggacgacaggaactcgtcgaactgcgcctcgccgctgaataccttcgcgccgtcgatggttttgggcgagcggctccagcccagtaccggaaactcgaactgcgccacggctttcgcgacccgctccccgagcacgcccagccccatgatgccgaccgggaagtcgcgccgcagcttcggcttgcggtagctccagcggccttcgcgcgcgtcggcctcgtaggcatcgaactcgcggaagtggcggatcagcgcatggcatacgtactccgccatctgcaccgacatgcccgcatcgtcgagccgcacgatgcgcgtgtgcgccggcacgcgcagcttgagcagcgcatcgacgcccgcgccgatgttgaacagcccgcgcagtccgggttgctcatcgagcaactgctggggcggcacccacacgaccgcgtggtcggcctgggccgcccccggttgccagggctcgatctgcgcgccgggcaactcggccttgaggccttcgatccagggttcggggcggttgtcggtgagagagacgatgattttcatgaatcgaatcttattagggccgcggcttgtcgccctgtgttccttcttctatgctcgtgcgccagcatccaagaccaggcacaccaggagaccgaagcatgatcaaagtcagcgtgatgtacccctacaccgacggcgcaaggttcgaccacgcctactaccgcgacaagcacatgccgcttttgaaggcgcgcatgggcgatgcctgcaggtcgtacaccatcgacaaggggctggccggcggcgcacccggaaccccgccgacctatgtcggcatgtgccacgtgttctgcgactcggccgaggcgtttcaaagcgcgttcggcccgcatgccaaggagattctgggcgacatcaagaactacaccgacatcgcacccgtgatgcagatcagcgaagtggtggtgggctgacccagggcggaggtcaggccgccgcggccatccgcagcaattcatcgccttcggccacctgctcgccgggcgagaacatcagctcgtccaccgtgccgtcggccggcgcggcaatggtgtgctccatcttcatggcctccatcacggcaagcggctggccacggctgaccttgtcgccggccttgaccgcaaaggacacgaccttgccgggcattggcgccgtgagccggccgccttcggcatgggtgtcgcccgcgtgggccaggcggtcgatggcggtgatcttggtggcgcctttcgatgcgaagacatgcgcggtggcgccgtccagatgcacgtccacggtctgccgcgtgccggcaaactcgacctcgaactcgcccgacggaaattggcccacgaccagcgggccttccacgccgccggcttcgagccgcaggctgccgtcgcgcttgtaagtcagcaaggccgtctgctcggcgccacgaaactcgaagtcgaagtggcgccggtattcgccatgggagcgccagccgtcgcgccgctcgaacgggtcgggcacgccggtcggccgttcggtgatcagggtgcgcgtgatggcggcggcggcggccagcggcaggcccagcgcctcgcggtcgaacagcacggcgcgctcacgctcgatcagcgccgtatcgaggttggccttggagaacgactcggtcgcgagaatgccgcgcaggaactgcacattggtcgacacgcccacgatctgcacctgcgccagcgccgcatcgagccgcgccagcgcctcggcgcgcgtggtgccatgcacgatcagcttggcgatcatggagtcgtagaacggcgagatctcgccaccctcgcgcacgccgtcgtcaatgcgcacgcggctgcgctggaaggccgtggcttgcggcttgcggtacacgcgcagcgtgccggtggcgggcaagaagttgttgtcggggttctcggcgcagatgcgcgcctcgatcgcgtggccgtggatctgcagctcctgctgcttcgcgggcagcgtctcgcccgaggccacacgcagctgccattcgacgagatcgagtccagtgatggcttcagtcaccgggtgctccacctgcaaccgagtgttcatctccatgaagaagaagttcatctcgggttggcctgcccccacgctcggcactgacgtgtcctcgctgccccccggggggcgctcgcttgcttggggcggcccggcgcggcgctcggctcgcgctgctcgacgatgaactcgacagtgcccgcacccacgtagttcacggcgcgcgccgcagccacggcggcttcgcccatctgcttgcgcatcgcctcggtcatgccgggcgcgggcgcttcttccagcaccttctggtggcgcctctgcaccgagcagtcgcgctcgaacaggtagacgtagttgccgtgcgtgtcgccgaacacctggatctcgatgtggcgcgggcgctgcacgtacttctcgatcagcacggcgtcgtcgccgaagctgttgatcgcttcgcgctggcatgaggccagcgcggccgcgaagtcttccgcccggtcgaccgcgcgcatgcccttgccgccgccgcccgcgctggccttgatgagcaccgggtagccgatgcggtcggcctcgcgctgcagcagcgccgggttctggtcatggccgtggtagccgggcaccagcggcacgccggctttttccatcagctgcttcgattcggccttgaggcccatggccttgatggccgacggcggcgggccgatgaagaccagccccgcgtcggcgcaggcctgcgcgaactcttcgttctcgctcaggaagccgtagcccggatgcacggcctcggcgcccgtggccttggcggcttcgaggatcttttcccagcgcaggtagctgtccttcggcgcgctgccgcccaggtgcaccgactcgtcgcaggcgcgcacgtggttggcatgcgcgtcggcatcggaatagacagccacggtgcggatcgccatgcgtctcgcggttgcggcaacacggcaagcgatttcaccgcgattcgcaatcaggatctttttaaacattcggagtgtctcccggaggattctttttcagttgaaacgcaggcgtgacgcccggatcgggtcggccgctgaagatgcgtgccacgcgggtgaacagcgccttgagaaagcgccagctcttgcggatgagccacacgctgagcgccagcacgaggacgaacagcgcgaggaagaccagcggatgcgccaccgcgagccacaagcccgcgggcaccatgctgtcttcgaccagcgatgcgcccacgttggaaaacggctcgggcgaggtgttgatggctgcgcgcgtcgtggccttggccgcatgcgcggtggccgcgaagccgccgcccagcagtgcggccacgacggccatcacgccatggtcggcgccgaacacgctggccgcgagcgccgcaccggcgggaatgcggatggcggtgtgcaccacgtcccacagcgaatcgaggccggggatcttgtcggcgaaaaactcgatgaacaccatgaacccactggccgcgatgaccaccggatgcgcgagcagctgcaggccgctcggcaacggcacccagccgaagtagccggcgagccccgtcagcagcacgacgaggtacaaccgcacgccgctggcccagccgatggccgcggccagggcgagcagttgggtcatgtcgagcgcattcatggcatgcgctcagtggcccagccaggacggcttgcgtttctgcaggaaagcctggacgccttcgcggccttcatcgctgacgcgtatgtccgcgatgccctccacggtcctggcgatcagcgcgtcatcgatctcgcggccgtccacgtcggcgatcagttgcttgcaggcacgcacggcggccggactggcaccggtgagcgccttcaccagctcgtcgagcttggcgtcgagcgcgtcggcagcgacgacttcatgcacgaatccgatgcggtgcgcctcggcggcggtgaagcgctcggccgtgagaaagtagcgctgcgaagcgcgggtgcccatggcgcgcagcacatacgggctgatggtcgcgggcacgaggccgatcttgacttcgctgaggcaataccatgccgtgtccacgctcaccgccatgtcgcaggccgcgaccagccccatgccgcccgcgtacacatcgccctgcacgcgcgcgatggtgggcttggggcactcggcaatggcgcgcagcatctcggccagcttgcccgcgtcggcgacgttctcgtcgcgcgtgtagtcggccatgcggcgcatccagttgaggtttgctcctgcgcagaaggccggtccgttggcgccgagcacgatggccttcacctgcggcgcggcgccggcttcggtgaaggcctgcgtcagctcggcgatcacgacgtcgtcgaaggcattgcgcgcatcgggctggtcgagccagatgcgtgcgatggcgccttcgatcgtgaggttcagcttggtgaaagtgctcatgccgcgtcccttctgtcacatgcggaagatgccgaacttcggctctggaatgggtgcgttgcgcgcagccgccaggcccagcgccagaacacgccgtgtatccgccggatcgatgatgccgtcgtcccacagccgcgccgtcgcgtagtacggatggccctggtcttcgtactgctggcggatcggcgccttgaaggcttcttcctcttccttgctccagctaccgcccttgagctcgatgccgtcgcgcttcaccgtggccagcacgctcgcggcctgctcgccgcccatcacgctgatgcgcgcgttgggccacatccagagaaagcgcggactgtaggcgcgaccgcacatgccgtagttgccggcgccgaagctgccgccgatgatgatggtgaacttgggcacgttggcggtggccaccgccgtcaccatcttggcgccgtggcgcgcgatgccttcgttctcgtacttgcggcccaccatgaagccggtgatgttctgcaggaacaccagcggaatcttgcgctggcagcacagctcgatgaagtgcgcgcccttctgcgccgactcgctgaacaggatgccgttgttggcgatgatgcccacgggcatgccttcgatctcggcaaagccgcagaccagcgtggcgccgaagcgctgcttgaactcgtggaactcgctgccgtcgacgatgcgcgcgatgatctcgcgcacgtcgaagggcttgcgggtgtcggtcgggatcacgccgtagagttcttcgcgagggaatgcaggctcgcgcatctcggtcttcgcagtggcttgcgcggctgccactgcattgagattggccaccgccgaacgcgcgagcgccagcgcatgcaggtcgttctgcgccaggtggtccaccacgcccgaaagccgcgtgtgcacgtctccgccgcccaggtcttcggccgtgaccacctcgccggtggccgccttcacgagcggcgggccgcccaggaagatggtgccctggttcttcacgatgatcgactcgtcgctcatcgccggcacgtaggcgccgcctgccgtgcacgagcccatgaccaccgcgatctgcggaatgccctgggcgctcatgttggcctggttgtagaagatgcggccgaagtggtcgcggtcgggaaacacctcgtcctggttcggcagattggcgccgcccgagtcgaccaggtagatgcagggcaggcggttctgctcggcgatctcctgcgcgcgcaggtgcttcttgacggtcatcgggtagtaggtgccgcccttcaccgtcgcgtcgttgcagacgatcatgcagtcgacgccgttcacgcggccgatgccggcgatgaggcctgcaccaggtgccgattcagcccccttcgcgtcgaggtacatcgcatgcgcggccagcggcgcgatctccaggaacggcgtgccggggtcgagcagctcggccacgcggtcgcgcggcagcagcttgccgcgtgccgtgtgcttggcacgcgcggcttcgccaccgccctgctccactttcgcgaactgctggtaaaggtcgtcgaccagcgcgcgcattgcggcggcgttggcctggaagtccgccgatcgcgcgttgagtttggtttcgagtttgctcatgctgtcttttcttgttcgaggccgagttgttccgccatcgcttcgcggatcttgaatttctggatcttgccggtcaccgtcatcggaaacgcggtgacgaactggatgtacttcggcaccttgtagtgcgcgatctggcccttgcagaaatcgcggatctcgtcttcggtcgcggcctggcccggcttcacgatgatccaggcgcacagctcttcgccgtacttcttgtcgggcaggccgaccacctgcacgtcctgcaccttgggatggcgatacaggaactcttcgatctcacgcgggtagatgttctcgccgccgcggatcaccaggtccttgatgcggccgacgatgttgacgtagccctcggcgtccatggtggcgaggtcgccggtgtgcatccagtgctcggcgtcgatggcttcgcgggttttttcttcgtcttgccagtagccgtgcatcaccgagtagccgcgcgtgcagaactcgccggaggttccgcgcggcacgatggcgccggtttcgggatcgatgatcttcacctcgaggtgcggctgcaccgtgcccaccgtggacacgcgcttgtccagcggcgtgtcggtgctgctctggcagctgacagggctggtctcggtcatgccgtacgcaatggtgatttcgctcaggtgcatctcgttcaccacgcgcttcatcacctcgatggggcacggcgagccggccatgatgccggtgcgcagcgtggagaggtcgaactccttgaagcgcggatggtcgagctcggcgatgaacatcgtgggcacgccatgcagcccggtgcacttctcggcctgcacggtctccagcacggtgagcgggtcgaacccatcgttcgggtacacgatggccgcgccgtgcgtgaggcaggccaggttgccgagcaccatgccgaagcagtgatacagcggcaccggaatgcacagcttgtcggccggcgagagcttcatgcactcgccgatgaagaagccgttgttcaggatgttgcggtgcgtgagcgttgcgcccttcggaaagcccgtggtgccgctggtgaactggatgttgatcgggtcggtggccttgagcgtcttctgcacctgcgccacgcgcgggtcggccgcatccccgctcgcaagcaattggctgaagcggcgcatgccgggctcttcgacatctgccgcggccttgccgtcgatccagaaggtgtgctgcagctgcggcaggcgcttcgggcccagttcgcgcagcatgccgaggtagtcgctggtcttgaattgcgccatcgtcaccagcaccttgcagccgaccttgttgagcgcgtattcgagctcggaggtgcggtaggccgggttgatgttgacgaggaccaggccggccttggctgtggcgatctgcatcagcacccagggtgcgttgttgtgcgaccagatgcccacgcggtcacccggctcgaggcccaggttcagcaatgcgctggcgagcttgttggactcggcctgcagctcgcggtaggtgtagcgcttgccttcatggcggctgatgagggcctcacgatcggggtgcttttcgaccatgtcgtcgaagaagtcgccgatggtttgctcgatgagggggacgttggtggcgcctcgggccatgctctgtgtcagtggcatcgtcttgtctcctggtcttgctccctctcccctgggggagagggttggggtgagggcgccggccctcgatgaagcgcggcgctcgactcgatcgctgctgccctcaccccagccctctcccagagggagagggagcaagaggggacagcgcgattcatcctaggcagtttccgagaacagctcgcgaccgatcagcatccgccggatctcgctcgtccccgcaccaatctcatacagcttcgcatcacgccacagccgctccaccggaaagtccttggtgtagcccacaccgcccagcgcctggatcgcctcgccggccatccacgtcgccttctcggccgaatagagaatcgcgcccgccgcgtccttgcggaaggtgcgcgcatggtcgttgcggtcgcaggccttgcccacggcgtacacgtaggcgcgcgtggcctgccaggtcgaatacatgtccgccagcttgccctgcatgagctggaattcgccaatgctctggccgaactgcttgcgctcgtggatgaagggcagcaccgcgtccatgcaggcggccatgatgcccagcgggccacccgagagcaccgcgcgctcgtagtcgaggccgctcatcagcaccttggcgcccatgccctcgccgccaagcacgttttcttcgggcacttcgcagttgtcgaagaacagtgggtaggtgttggagccgcgcatgccgagcttgtcgagcttggtgccggccgagaagcccttgaagctcttctcgacgatgaaggccgtcatgccgcgtgcgcccatttcgggttcggtcttggcgtagatcaccagcgtgtcggcatcgccgccgttggtgatccacatcttgccgccgttgagcacgtagtagccgttcttcttctcggccttgagtttcatgctcaccacgtcagagccggcgttgggctcgctcatcgccagcgcgcccacatgctcgccgctcaccagcttgggcaggtactttttcctttgcgcctcgctgccgttgcgatggatctggttcacgcacaggttggagtgcgcgccgtacgagagacccaccgacgccgaagcgcgcgagacttcttccatggccacgatgtgcgccagatagcccagctcggtgccgccaaattcttccttcaccgtcatgccgtgcaggccgagctcgccgagcttctgccacaggtcgtgcggaaacaggttgtcgcggtcgatgtccgcggcgcgcggagcgatttcgttcgcggcaaagtcctggatggcgctgcgcagcgagtcgatggtgtcgcccaggtcgaagttcaggccgggatcgtgcatgtgtcttgtctcctctgagggggtcggcgcgcaggctgtcccacgcggattggcgcttggaagaaacgcagcttacgcctcgccgcgccgcaattggcgccacaatggttgcaaattgcgccacgcctgatccaccgatccatgacttcgcccgctttcctccgatctgcccgcgccgccacgccgatggccttcgtgagagccatcgtccagggctacgagcactacggcgccgatccggcgggagccctgcaggcggcacagatcacgccgcgtgaactggcccgaccggatgcgcgggtgacggccgcgcagttcgaggcgctgtcgggccacgcgatgcaggaactcgacgacgaggccctgggctggttctcccggcggctgccctggggcagctacggcatgctgtgccgcgcctcgctgacctcgcccgacctgggcgtggccatcaagcgctggtgccgccaccaccgcctgctgaccgacgacatcgcgctggcgctggaagtgtccggcggcatcgctacgctgcgcatcaccgagaaccgccccctggacgaggcgtttcgcgagttctgcctggtgaccaccctgcgcttcctgcacggatacgtctgctgggccatcgactcgcgcatttcgctgcgcgacgccgcgtttccgttcgcggcgccgcagcaccgcgacgcctacccgctgatgttcacggccgacgtgcgcttcgatgcgcccgaggccagcttcagcttcgacgagcggtacctcgcgctgccgctgcagcgcgacgaacgcgcgctgcgcaccatgctcaagcgggcgctgccgctcacggtgctccagtaccggcgcgaccggctgctggggcagcgcgtgcgcgagctgctgcgttcacgcgcgagcgaggccaccaccgcggaggccttggccacgctgctcaacgtgtcgagccgcacgctgcaccgccagctgcatgaggaaggcacgtcgatgcagatgctgaagaacgaggtgcgccacgagatggcggtggacttgttgcgccggaccacgcgccccatcaagcaggtggcgctgtcggtcggcttcaggaacgaaaagagtttttcgcgcgccttcctgcaatggaccggacacgcgccgcgcgatttccggcagcagggaaagtagcgctcaggccgccggcgcgtcgatgagtgcgagcgcgtcggcgatggattggctgtcttccggccgcaccagcttggcgacctgccgtccgtcgcgcatgaacaccagcgtaggccaaagccgcacgttgaacgaacggcccagcggacgcccgctgccgtcctcgaccttgatgcgcttgatgtgggggtacttggcaaaggcctcggcgatgttcggctgcgcggccttgcagatgccgcaccagttggtgccgaactcgaccacggcggggcccgcgagcgcatcgatctcggcgcggtcgggctgctcggtcttgtactcggaagtcatgcgatctggctccttgtggacttactttgccgccattgcagcagaaacccggcgggcttgcctgcgacaggggcttggttcttcggcctgtaattttcagaccggttgcaagccgtgcgcggccaacagcgcgggcagttccttcatgtcgctgaacacctgcagcgcgccgacgctgcgcagcgcctcggggccgctgtggcccgattcgcccgtgctgtagccgaacaccgtggcgccggcggcgacaccggccatcgcgccggtgaccgtgtcctcgaccaccgcgcagcgtttcggatcgacgccaagggcggcggccgcggccaggtacacatcggggtgaggtttggagcgcggcatttcgtgcccgctgaagatacggccttcgaagcaatcgagcaggccgaccttcgccagttgcagctcgaccttgtggcgatcggcgcccgaggcgcaggcaatgcggccatcgagcttcgcgtgtatttcgcggatggccgcgggagcatggggaatcgccgtcaggtcgcgttcgagcgcatcgttgcggcgggccctgaatgctttaagccactcttcggtgatccggacgcccgtcttggattcgatgagcgcggtttcgtccttcacggccttgccggtgaaggtgttcatcgactcttcggtggtgaggtgccagccgagttcgcctagcatttcggcgaggatgcggttggtgatgggttcggaatctactaggacgccgtcgcagtcgaagaggactgcggcgaaggggaatgagggcatctttgtttggctttgttcggatttggggacgatggtagcaattgggcttgtttgcttcccgaggccgggatatccgcccggcggcggactcactttcttttgcttcgccaaaagaaagtaagcaaagaaaggcgacccctactgtctgcgtccctccgctgcgctgcgggcaacctgcggtgctcgactccggcggggtccgcagaactcgcttcgctcaaacagctgcggccctgatcccgcctccatctgcgctcctcggcgcatacagaaggggtggggacgagacaggccttcgcttcgctcggccgggagcaacctccaataccaaacagccaataccaaccaccgcaggcgcgcagcgcctgcggtggttggtggccgagcgaagcaaaggcccgttcggtctccaagcccctctgtatgcgccgaggagcgcagggtttcgcggatcagggctcgcagctgtttgagcgaagcgagttctgcgagaccccgcgaaacccgagcaccgcaggttgcccgcagcgaagcgaagggtcgcagacagtggggtcgcctttcttttgcctacgtttctttggcgaagcaaagaaaagtaggtcgcccgccggggcgagtcccggcctcggaactcaaaagaaaacaccgatcaacgcgcgtgcgtcacccctccatccaccaccaacgtagaccccatcacatagtcccccgcccgcgaagccagatagatggccgccccagccatatcctcaggcgtcccgatgcgccccgcaggaatccgttccttcacctcatcgccatgatcacgcgccagcttgttcatgtccgatgcaaacgcacccggcgcaatcgcgctcaccacgatgcggtcttgcgcaagccgcagcgccatgcgccgcgtgagctggatcaaaccggccttgctcgcggcgtaggagtaggtctcctgcgggttcaccgagatgccgtcgatcgatgcgatgttgatcaccttcgacagatggtcggtcgccgccttcttgagcatcggcgtcagcgcctgggtcaagaagaacggtgtcttcaggttcaggtccaccaccttgtcccagccgctctcaggaaactcgtcgtacggcgcgccccaggccgcgccggcgttgttgaccaggatgtcgagcgagtcttcatgcttcgcataggcgtcgaccagcgcctgcgcgccttccagcgtggacacatcggccggcagcgacacgcagtggccgaaggccgaaagctccttggcggtctggtcgcaggccgcggccttgcgggccgagatgtacacgcgcgcgccctgcgccaggaagccttcggcgatcatgcggccgatgccgcgcgagccgccggtgatcagggcgctgcggcccttcagcgagaagagttgggtggtgtccatggtgccggtgtctcctgaatgaattgacgaaaaattccaggaaacgagcttagtgcgccgcacgccggcgcagcgtcaccttggcggcagcgacaggcttcgcgggctggtgaagctgcgcagctcgccgctcaccgggtcctggaacgccaccgacttggccagcagctccagcggcttgtcgaagtcgtcgctgccctgcggcagcagcgtcgggtagatcggatcgttcacgatcggcatgcccagcgccatgcagtgcacccgcagctggtgcttgcggccggtgaccggcgaaagatcgagcagggcatggccgccctcggcccgtttcaccacgatgcgcgtttcggagttgggctcgccctcctcttccttcacgcgcatgaaatgttcgtcgtccaccagccggctgcggtaggtgccaggcaccgacgacacgcccggcggccatggcaccacggcttcgtagtgcttggcgatgcggcgctccgggaacatggcctggtaggcgctgcgcgtttcgggccgcaccgagaacagcaccagccccgccgtgctgcggtcgatgcggtgcagcggcaccaggtcgtcgagcttcagcttgcgtttgagccgcaccagcaggctttcctgcaagtacttgccggtcggcgtcacgggcaggaacggcggcttgtcgaccaccaccagttggtcgtcctggaacagcacctgctcgtcgaagggaatgcgcacctcggcatcgagcgtgcggtagtagtacacgcgcagcggcgcctggtagcggcgctgcgcggtcacgggcacgccgtgttcgtcgatcacgtcgttggcctcgatgcgcgccatccacgcttcgcgcgtgatcgcgggaaagcgcgccatcaagaactcggcaatggtgggccacgagccttgcggcaggccgacgcagctcggaccgacgccgtcgcgcgtgggcagcggcaagcgagggctcgtcattgcgagagctcgttctgcagcagcgacagcgcctcgctgaacaagggccgcgccgccacgtcggcttgcatgcagcggtctttgagggcagccatggcttccggcggcgcatcgctgcaatgcgcgaggagttcttcgagcaggcagccgaaggcgcgcatctccagccgttgcagcgcctcggcttgtgccgggtcgagcgcgccggtcatccaggccgctccaaagtcgccgagcaacccgccgccctgcgcgctccagaggatgttgtgcgcgtagaggtcgccgtgcaggatgcctcgcgcatgcaggtgccgcatggcggaggcgatgtcgcgcgcgatgcgcagcgccacgccggaggtccattgcgcgtcggccggatagacgtcgcgcgtgcaagaggcaaggctcggcggcccggcgagcgtgcggaacgatgggtccaccagtgccatgaccaggccttcggcaccgtccggatgcccgtcgatcctgctctgcgcggcaacgagggtcgggtgtgcaccggctgcgatgctggcggccatttcactgtgcggccagccgtcgctcgtcaccgcacccttgaagagcttgacagccaccggccgcatcgccgagcccagcgttgcctggtggataacccccgaagccccctcgccgagcttcgggcccagcgccagttcgcgccagtcgacgtgcggcaccgacagcgcggcgatggccgcatcttcggcttgtgcatcgaaaggattgcccgcacccgcgagccacgagaggcgcggcagcgagagcagccatggaggcagcgcctcgaaacggttggcggaaatgcgcagcagttcgagttggctgcagcccgccagcgaatccggcagcgcacgcagttggttgccggcgagcatgagcttctgcatcgcgccgcattgacccagcgcctcgggcaagctctcgatcaagttgtccgtgaggatcagccagcgcagcaacggcagccgcagcgccgcggcgggcacggcaccgatgtggttggccttgaacccgaccatttccagcgtctggcactggccgatcgagtcgggcaaccgggtgaagcggttgtcggagcagaacagcacgcgcaggcgatgcagccggtgcagatcatcgggcagcgaatcgagcgcattgcccgagaggttcaggatttcgagcgaatcggccaggtcgaagatctcgcgcggaaactcggtgagtccgcacgagagatcgattcgttttgcgcctgccagccggcccgcgcgcagctcagcaagcgtgtccatccaccgagtctaaagtgcctgcgccgcggcggctccggcaccgaagcggtagatgccgtcggcgcccagctcgcgcctgacctgccccgcgaaccacagcaggtgcaggtgcgccaccgtctcgcccatcgcaaaggtcatctggtgcaggtcgagttcgcgcttgaagaggatgggcaggccctcggccgcggtcagcggacgtgcggtgcaggcttcgagcagttcggccaggcggtcgcggtggtgctcctgcagctggtcgacgcggcggtgaatgcccgtgaacggcttgccgtgcgatggcaggcccagcgtatcggccggcagcgccttgaacttgtcgatgctgtccaggaagagccgcagcgagttggcttcgggctcgcccgcgtgcacgctcacgttggtcgagatgcgcggcagcatcatgtcgccgcccagcagcagcttcagctcgtcgcagtacaacgcgatgtgctcgggcgcgtggccatagccgctgatgcagcgccaggcgtggccgttgatggccacggtgtcgccgtccagcatgcgcgtgaagcggtcgggcaccgagggcaccatgttggcgtagtagttggtgcgcgcgcggatcttggcgacggccgcgggatccgtcaggccgtgcgaggcaaagaagctcgccgcggcatcgccgcccgccagcgtgtcgccgttggtgctcagcacgcgggccacgtggtagtcggtcgagctgatccacagcggcgcattccagcgcgtgcacagccactcggccaggccgatgtggtcggggtgcatgtgggtgacgatcacgcgcaggatcggcaggccctgcagctgggtctcgaagatctgctcccactgcgcgcgggcttcgtcatgcgcgatgcagcagtcgaccaccgtccagccctcgacgccgtcgatgctgtcgcgcagcagccagaggttgatgtggtcgagcgcaaacggcagccgcatgcggatccatcgcacgcccggcgcgacttccagtgcttcgccgggggcgggcagggtgtcgcccagggggtagtggagttcgcgttcgaggaggttcatgtaagattgacgtttacgtaaacgtcatgtgttaagggcaccattgtagggagcgcggggcaaacctgctgtcgcgcccgcaacgcccccacagacggcttccagacagaccgcagccatatgtccgcgcagactttcaccatcagccagctcgcgaaggagttcgacctcacgacgcgcgccatccgcttctatgaagacatggggctgctgacgccggagcgctccggcatgcagcgcatctacagcgcgcgcgaccgggcgcggctcacgctcacgctgcgtgccaagcgcctgggcctgagcctgaccgaggccagggaaatcctcgacatgtacgacagcccgcgcgacaccgtgccgcagctcgagaagtttctcggcgtgctcggcgcgcaccgcgcccagctcgaagcccaactggccgagctgcaggccaacctggcggaagtgcgcgagcacgagaagaagggccgcgcgaccctggccaaggcgcagaaggcggccaggacggcctgatataccgcacccaatcacgactcatcgacaatcacgcccatgtccgacactcttgatgacctgtttgcccacaaccgtgcctggtccgcacagatggaacgcgaccggcctggcttcttcaccagcctggtgaagcagcagacgccgcgctacatgtggatcggctgctccgacagccgcgtgcccgccaaccagatcaccggcctggagccgggcgaggtgttcgtgcaccgcaacgtcgccaacatcgtggtgcactccgacctcaacgcgctctcggccattcaattcgcggtcgagcacctgaaggtcgaacacatcatggtggtgggccactatggctgcgccggcgtcaaggcggcgctcagcggcaagcgcatcggcctggccgacaactggatccgccacatccaggacgtgcgcgaccgccacgccgtgatgctcgaaaccctgcccgaagacgtgcgcgtcgacgcgctgtgcgaactcaacgtggccgagcaggtggtcaacgtggccgtcagcaccgtcatggtcgatgcctggggccgcggccagaaggtcaagatccacggctggacctttggcgtgcacgatgggctgctgcaagacctggggctgaatgtcgacggcgccaagccgctcgacgcggtgtacaaggccgcggtgcagcgcatccgctacaagtggagcaagccgctgggtatctcgccgtccgcgcaggccgggtccgacggcaccgaggtcatcgaagtcattccggctggcgaggccaacacccccgtcggcgaaggcaccgaagcgaaacccggctgaagccatgttcccgcagcgtctcgattcaccgctggcctacgacatcgccaaggcgatgatcgatggattcaatcgccattacagcctgttccgcgctgaatcggcacgcgccaagcaccgattcgaaacggcggactggcacggccagcagcgcgcgcagcgggaacgcatcgagttctatgacctgcgcgtgaacgaggccgtggcccgcctcgaaaaagagttcaaggctggcgaccagccgatggaggtgtggcaccaggtcaagctgcacttcatcggcttgctggtggaccaccaccagcccgaactggccgagagcttcttcaactcggtgaccacgaagatcctgcaccgcgcctacttccagaacgacttcatcttcgttcgcccggccatcagcaccgagtacatcgagccgcgcggcgcgcccacctaccggccctactacccctcgcacgacacgctggccgacaccatcgagcagatgctcgacgactacgccctgcagggcggctttgccaacaagcggcgcgatgccgagcgcgtggcgcacgccatcatggggcgctttcaccaggtgaagctgcgcgccaatttccagctgcaggtgctctcaggcctgttctatcgcaacaagggcgcctacgtggtcggcaagatcatgaacggctttgtcgagctcccgttctcgctgcccatcctgcatgacagccatggcaagttctacgtggatgcggcgctcttcggcgaagacgacctgcagatgctcttcagttttgcacgcgcctatttcatggtcgacatggaagtgccgtcggcctgcgtgcagttcctgcgctcgctcatgccgcgcaagccgcgcgcggaaatctacaacgcgctgggcctggccaagcagggcaagacgctgttctatcgcgactttctttcgcacctgaactactcgagcgaccgcttccgcatcgcgcccggcatcaagggcatggtcatgctcgtgttcgacctgccgtcgttcccgttcgtgttcaaggtcatcaaggacttctatccgccgcagaaggacaccacgcgcgagcagatcaagagcaagtacatgctcgtgaagcagcacgaccgcgtgggccgcatggccgacacgctggagtacagcgacgtgggttttccgctcgaccgcttcgagcccgagctgatcgaggagatccggaagttcgcgcccagccagctagagatcggcgaccgcgacggcaacggggagatggagctggtgctcaagcacgtctacatcgagcgccgcatgatcccgctcaacatcttcctgcaggaagccttcgacacgctggcccaccccgaaagcccggcccatgccaagcgagcgaaggagcagctggagcatgcggtgatcgaatacggcaacgcgatcaaggacatggtcgccgccaacatcttcccgggcgacatgctgtggaagaacttcggcgtcacgcgcggcggcaaggtcgtgttctacgactacgacgagatcgaatacgttaccgactgcaagttccgcaaggtgcctacgccgcgcaacgaggaagacgagatgagcggcgaggtctggtattcggtcggtccgaaagacgtgtttccagaaaccttcgaacccttcctgctcggcaacagcgacgtgcgcgcggccttcatggcgcaccatgccgacctgctcgacgctgccttctggcagcaccacaaggaacgcatcgaggccggccagatgctcgacgtgttcccgtacgaagaatcgcagcgcttccagcatgaaggccatgcgacccatttctgattgagtccccggtccacgacgaccactttcaactttccgaaggagaccaccatgcctgaatccatcgtcatcgtcggcgccgcccgcacccccatggggggcttccagggcgacttttcttccctctcggcgcacgacctcggcggcgccgccatcaaggccgccgtcgagcgcgcgggcattgcgcccgacagcgtgggcgaagtgctgttcggcaactgcctgatggccggccagggccaggcgccggcgcgccaggcggcctacaagggcggcctgcccgacagcgcgggcgcggtcacgctcagcaagatgtgcggctcggccatgaaggccgccatgctcgcgcacgacctgctgctggccggcacgcacgacgtgatcgtcgcgggcggcatggaaagcatgaccaacgcgccctacctcatgctcaagggccgcggcggctaccgcatgggccacgaccgcatcttcgaccacatgatgctcgacggcctggaagacgcctaccagccgggccgctcgatgggcaccttcggcgaagactgcgccgccaagtacaagttcacgcgcgagcagcaggacgccttcgccattgccagcgtgcagcgcgccaaggcggccaccgagtccggcgcgttcaaggaagagatcacgcccgtcaccgtgaagggccgcggcggcgacacagtcatttccatcgacgaaggcccgggcaaggtcaagctcgacaagatcgccacgctcaagcccgcgttcaagaaagagaacggcaccatcaccgccgcatcgagctcgtcgatcaacgacggcgccgccgcgctggtgatgatgaccgagtcgcatgcgaagaagatcggcgccaagcccatcgcgcgcctggtcggccatgccacgcatgcgcagcagcccgagtggttctccaccgccccggtcggcgccgtggccaagctgttcaagaagacgggctggaccgtcaaggacgtcgatctctgggaagtgaacgaggctttcgcggtggtgccgatggcgctgatgcacgagctcgacgtgtcgcacgacatcgtcaatgtgaacggcggcgcctgtgcgctgggccacccgatcggcgccagcggcgcgcgcatcatggtcacgctgatccatgcgctgaaggcacgcggcaagaagcgcggcgtggccacgctgtgcattggcggcggcgaaggcacggccgtggcgctcgaattaatttaaattgacatttattgttgatttttcacattcattgtcgtttgattaattaatgacaattgttaattatcggaagcgcgaagttatttctttactcctgattccctgataccatctgcgcgcagcctttgccacagaatgacagaggctgcgcgcagcgtgaattcagggaaaagaatgaacaagaagagaggggcggagcgtgcgtcgacctattgggcggcttcgggaaaattcttgcgtcgattgcccggcgtcttgaaaatacttcccttggttgtggcagcaattctgatattgcttgctgcgctaccgagatctcgcgttgatcttgcagtcgccgacgccgatgagttgctcttgaggctggcagcgctaggccgcgaaggtgcagccgtcttatgcaatcctgaaggcatcgaaaaatacctcgccgttcgcattgataaagaaaatccaaataaaaaggaaggcgacagctcccctgttgccgtgaatacaccaagtcaatccgttttcggaagttattggaaacttcaagcgagtacgggcactgtgtgcagactccaattgcaagtcgcaggtcgtcgattctgtgacacggattccgcgcgcacacaacgcttgatcggccgccgtgttcaaactcgactggccgtgccgggtggagccgacttctacgatcatgggtacgagctggcgcgcgattccacggagagatcggttatcggatggcggggacctagtcgggcgtgtcctgccgacgttgaaatcgctgtggcaatccgttgaatggcagcgcgtgagcgtcgctcgctgccgtggcccgcgctgcttgcgggaatcgttttttttgccgcgagcgccatgctgctgtacgaatcgacgcgcgaatactttcctcgcagagatttgcacgcgttcgacactcaacatgctgaactattaagcgccgaacggcgggccgcttacgagcgggaactgttcagcgagttgtcccaatggaatcgccccagccgtcgctacccgagcgaggctggtatcggtcaacgcgaaaagcgatggagacagctggctggcgaagggctcgagctggcgcacctcgccttgcaggtgcttcagcccgacggcggcttcgtctacccgctcgagaagccgatgaatcggttgctagccctcgcagagcgaggcgactccggtgcaatgtgtctgatgaccgggcttgtcagccaagtcaagcgctcacgtttgtcggccgaacactccgaaatggcaaggaaatggttgattcagggtgccgaacgcgggcacgcggagtgccagttgcagctaggacgtcgtctgatcctaggtatcgacgggatgaccaaggatgcgaagcgcggactggccctggaacttgcggctcgccgagatggatacgctcacgacgtcgacgggctcgtatcgtattttcaacagcgatggtcaaccgattctgccgatctcacaagactgtactgctggctgtcgatccatgcccagtcacgcgtgactgatgggccacagaacatgctgagactcctgcgtgccgaggcgcgacgcatcgattccgaggggctggtgcatctcgcaaaccagctcgagaactcgcggttttccttgcaggcatgtgttgacttgagcggagtctgaggtcatccctggcggccaggacgatgcctagaatgccagcttcgtgcacatctggggacctcgttcatgtattcggccaatctccgcaacaccgtcgccgctttggctgccttggttttcctggcgcccgcccccagctgggcgcaaaagcgcgacaacgtgctgttccaggcagccaccgacgcgcagcctgcggtgctcaagacgttggagcagctggtcaacatcgaaaccggcacagaagacgccgaaggcattgcagccgccggcaacttcctggaaggcgagctcaagaacctgggcttcaccgtcacgcgcagcaagtccaccagtctcgtcgtgggcgacaacatcgtcggcaagctcaaggggcgcggcggcaagaacctgctgctgatgtcgcacatggacaccgtgtacccgaaaggcacactcgcgaaggcgccgttccgcatcgagggcaccaaggcctacggcccgggcattgccgatgacaagggtggcaacgccgtcatcctgcacacgctgaagctgctcaaggactacggcgtgcgcgactacggcaccatcaccgtgctcttcaacaccgatgaggaaaaaggctccttcggctcgcgcgacctgatccaggaagaagccaagcaggccgattacgtgctgtctttcgaacccacgagcgcgggcgacgagaagctttcgcttggcacttcgggcattgcctatgtgcaagtcaacatcaccggcaaggcttcgcatgcgggcgcggcgcccgagctgggcgtgaacgcgctggtcgaagcttccgacctggtgctgcgcaccatgagcatcgacgacaaggcgaagcacctgcgcttcaactggaccattgccaaggcgggcaacgtgtcgaacatcattcccgccagtgcgacgttgaacgccgacgtgcgctacgcgcgcaacgaagacttcgacgccgccatgaagactctcgaagaaaaagcgcagcagaagaagctgcccgaatccgacgtgaaggtggtggtcacgcgcggccgaccggcgttcaatgccggcgaaggcggcaagaagctggtcgaaaaggccgtggcctactacaaggaagccggcggcacgctgggcgtagaagagcgcaccggcggcggcaccgacgccgcctacgcggcgctttccggcaaaccggtgatcgagagcctgggccttccgggcttcggttatcacagcgacaaggccgagtacgtcgacatcagcgccattccgcgccggctgtacatggccgcacgcatgatcatggatctgggctcgggcaagtaagccgcaaacaaaagaagaaagacaggagacaccccatgctgctcagtgccgaccaggaagccatccgcgacgcggtacgcgatttctcgcaggccgaactctggcccaacgccccccgatgggaccgcgagcacagctttccgaaggaagcgcaccagggcctggcggcgctcggcgcctacggcatctgcgtgcccgaggaacacggcggcgcgggcctggactacctcacgcttgcgctggtgctggaagaaatcgccgccggcgacggcggcaccagtacggccatcagtgtgaccaactgccccgtcaacgcgatcctcatgcgctatggcaacgcgcagcagaagaagcagtggctcgaacccctcgcgcaggggcagatgctcggcgccttctgcctgaccgaaccgcaggccggcagcgatgcatcgagcctgcgcaccacggcgcgcaaggacggcgatgcctacgtgatcgatggcgtgaagcagttcatcaccagcggcaaaaacgggcaggtggccatcgtcatcgccgtcaccgacaagggcgcgggcaagcgcggcatgagcgccttcatcgtgcccaccgatgcgaccggctacagcgtggcgcggctggaggacaagctgggccagcacagcagcgacaccgcgcagatcaatttcgacggttgccgcatcccggcggagaacctcatcggcgccgaaggcgagggctacaagatcgcgctcggcgcgctcgaaggcggccgcattggcatcgccgcgcagagcgtcggcatggcacgcagcgccttcgacgtggcactggcctacgccaaggagcgccaggccttcggcggttcgatcttcgagcagcaggccgtcgggttccgcctggccgaatgcgccacgcagctcgaggccgcgcgccagctgatctggcatgccgcgagtctgcgcgatgcgggccggccgtgcctcaaggaggccgccatggccaagctgttcgcgagcgagatggccgagcgcgtctgcagcgcggccatccagacgctgggcggctacggctacgtgaacgactttccgctggagcgcatctaccgcgacgtgcgggtgtgccagatctacgaaggcacttcggacatccagaaactgctgatccagcgcgcgctggcgtgagcatgcgccgcgggcgcttcggtgtcatcggtttggatgacagacagcaacgcgccggcggcgcagcatggcggcctcttcgtcggaggtctttgccatgtccaatttcaaacccgttcccctcgccctggcccttctgtgcctcggtgccatgggctcgtccgcgcaagcccaacctgccgccccggacctcgccacgctgaccgctagcgacgcggtgcggcagctctgcgcaggcacggtgagcagcgagcagctggtgtcggcctacgttgcgcaggccaatgcaagaacgaacctcaatgccttcgtcacgctcgacgaagccggcgcgctgaaggccgcgcgcgccgccgatgcacagcgcaagcgcggcggcgcctgcaagccgctggccggcctgccggtgaccgtcaaggacaacatccaggtgcggggcctgcctgccacggccggctcgcctgcgctgaagggcttcgttcccaaggcggacgcccccgtggtcgccaggcttcgggcggcgggcgcggtcatcctcggcaagacgaacatgcacgagctggccttcggcgtcacgggctacaaccccgcattccagagcggccccgaggtcggtgtgcgcaacgcctacgacccgagccgcattgcgggcgggtcgtcgtcgggcaatggcgcggcgctcggcgcgcgcatggcgccggccgcgctgggcaccgacaccggcggctcggtgcgcattccgtgcgcgttcaatggctgcgcatcgctgcgtccgaccatggggcgctattcgcagcaaggcatcgcgccgatctcgcacacgcgcgacaccgcgggcccgatggcgcagtcgatggccgacgtcgcgctgctcgaccgtgtgatcgcgggcggcacgccgctcaggccggccgacttgaagcgggtgcggctcggcgtggtgccggccttctacacgaacctcgacgcggacacgcgcgccgccaccgatgccgctcttgccaagttgcgtgcggccggcgtcacgctggtggacgtggagatgcccaggctcatggaactcaacggtgccatcggctttccgctcgcactctacgaggcgcacgacgacatggtggcctaccttgcgaagtaccgcaccggcatcgacatcgcgcagctcaccgccggtatcgcgagccccgacgtcaagggcaccttcgaggctttcgtgatcccgcgcaagctccccgcgccgaacggcacggtcgatgcgaagccggcctacgacaacgcgatgcgcgtcgcgcgccccgcgttgcagaagctctaccgcgacaccttcgcgaagaacaagctcgatgcgctcgtgttccccacggtgccgcgcgtggccctggcggccgggcccgaggccagcagccccgagaacttcggcgcgctgatccagaacaccgaccccggcagcaacgccggcattccgggcgtgcagctgccctcgggcctgggtgcggccagcggcttgccggtggggcttgaactcgacggaccggccggtagcgaccgcaggctgctggccgtggggctcgcggtggaaggcgtgctgggccgcctgccggcgcccaaggcgaaatagcgccttcttgaccgatcagcgcttcgccaggccggccagcgccgaccggcgttcgatgccgagcttgtcgaaggtgcgacgcaggtaggtgcgcaccgtcggcacgctcacggccatgcggcgcgcgatctccttgtcggtgaggccttcgcacacggcccgcgcgacctcccgttcgcgcgcgctcaattcgcgccaggcggtttcggcaggcagcggcatggcagccggcgtgcgctgcgcacgctgcagcgcaccgatgaacgccggctcgatcaggtcgagcagcgccttctcgtgatcgccaaaatcaccgcggcccttgcgccgccagatgcgcagatcgcccagcgcccggttgccttcgaacgcatgcaggttcatgccccagtgcagcccgtcgcgcgagagaaagtcggtgaagaactccgtgcgcatcagttcacgctgcggcatcacgtcggtcacccgcgtggcgtggcggtgcgactgcagcacgaaggtgatcgggtcgtgatgctggtgccattcgccgtagcggtcgaggttggcggggtccatgttcagcgccacgcggccctcgaagcggccggtttcagcatgccacacgaaggaggcgaactggtccgcatgcagcaggtcgagcagcgcccagcccatgcgctcgcggatgtcgctttcgcctcggtcttgcgcgagcagcgtgaaaacgccgcgcagcgcctgctgttcggagcctgtcaggtacatcgccgcctcgctctgtgggtatgcccgaagaaggctagcgtttagcaagcactgcgccaagggagtatctccggaggcggccgcagggcttgccccatcggagggagggccttgaggtgttccaataggggcttcatgagtgccaccgatcccaccaccggaccctgcccctgcggccgcacggaccgccgagacaagcccatcggcttcgccctgtgctgcggccgctacctcgacgatttcgagggcacgcccgcgcccgacgccgaatcgctgatgcgttcccgctatacggccttcgtgctggagcgcggcccctacctgctcgccacctggcacccgtcgaagcgcccggcctcgatcgagttcgaacccggcgtgaaatggctcggactcgacatccgctcgcgctcggtgctggacgccgaccatgccgaggtcgagttcgtcgcccgccagcgcagcagcaccggcaccgccacgcgcctgcacgagcgcagccgcttcgtgcgcgagggggaccgctggttctacctcgaaggcgacctgcagacccccggttgacgcgccgggcctcggcccgcacaataggccccgctccggggtgcacgcatgtggcgtgctgagatggcaaagtgccgacccgcgaacttgatccgggtcataccggcgtaagaagagctgcactccctgactccggtcccgccacccaccccgcgtggcggcccaaagtccaccgagcgattgcggagcaccctttccctcaacaaggagtgccccgcatgaatgcccccgacaagttcacctccctgctttcgctcacgcgcgagccgtttcccgcttcgcacaagtgcctgattccgggcagccggcccgacctgaacgtgccggtgcgcgacgtgctgctgaccaacggcgagaccgtgtcgctctacgacacttccgggccttacaccgatgccaagatcgacatcgacgtgcgccgcggcctgcccgacgtgcgcggcgcctggatcgtcgagcgcaacgacaccgaaagctacgaaggccgctcgcaccaggcgctcgacgagggcctcaagcacgcccacgaccacgacgcgcagcgcctggccgaactgcgtgcgggcgcctctgcgctgcagcgcacgccgcgccgcgcgaagtcgggcgccaacgtcacgcagatgcactacgcacgccgcggcatcgtcacccccgagatggaatacgtggcgctgcgcgagaacggcaaacgcgaatggatggccgaatacctcgccaacgaggagcgcgcgaagcgcgtggccggcaacccgatgggcgcaagcattccgcgcatcatcacgcccgagttcgtgcgcgacgaggtggcgcgcggccgcgcgatcattccggccaacatcaaccaccccgaagtcgagccgatggccatcggccgcaacttcaaggtaaagatcaacgccaacatcggcaactcggccgtcacctcgagcatcgaggaagaggttgaaaagctggtgtgggcgatccgatggggcgccgacaacgtgatggacctgtcgaccggcaagaacatccacaccacgcgcgactggatcgtgcgcaactcgccggtgcccattggcacggtgccgatctaccaggcgctggagaaggtgggcggcgtggccgaagacctcacctgggagatcttccgcgacacgctgatcgagcaggccgagcagggcatcgactacttcaccatccacgcgggcgtgcgcctgccgttcatccacctgaccgcggaccgcatgacgggcatcgtctcgcgcggcggttcgatcatggccaagtggtgcatcgcgcaccacaaggagagctttctctacgagcgcttcgaggacatctgcgacatcatgaaggcgtacgacgtgagcttttcgctcggcgacggcctgcgtccgggctcgggcgccgatgccaacgacgaagcccagtttgccgaactgcgcacgcttggcgaactcacgcagatcgcgtggaagcacgacgtgcagaccatgatcgaaggccccggccacgtgccgatgcacatgatccaggccaacatggacgagcagctcaagcactgccacgaggcgccgttctacacgctcgggccgctgaccatcgacatcgcgccgggctacgaccacatctccagcgccatcggcgccgcgatgatcggctgggccggcaccgccatgctctgctacgtgacgcccaaggagcacctgggcctgcccgaccgcgacgacgtgaagcaggggatcattgcctacaagatcgccgcgcacgcggcggacgtggcgaagggccaccccggggcccgttcgcgcgacgacgcgctgagcaaggcgcgcttcgagttccgctggcaggaccagttcaacctcgggctcgacccggacaccgcacgcgaattccatgacgagaccttgccgaaggattcgagcaaggtggcgcacttctgttcgatgtgcggacccaagttctgctcgatgaagatcacgcaggaagtgcgggagtacgcggcgaagaagggcgtggcggaggcggaggccatggcggccggcatggccgagaagtcgcaggagttcgcggcggctggcggggagatgtatatcccgatccgggcggtgtcctagggtttgattccggggccgggcctcgccccggcctcggacctcaagaccatcgaggcacagcctcgtccttgagctgctgccggagcaggtcgtagtccggcaccacgctctccaccgtctcccagaaccggtgcgagtggtccatcacgcgcagatgggcgagctcgtgcgcgaccacatagtcgatcaccggcaggcgaaagtggatcaggcgccagttcagccggatcgatccatcggcgctcgcactgccccaccgcgtggcggcattcgacagcgacagcttctgccagcgcacgccgagccgtggcgcgaagtggtcgagccgttcgatgaaaagacgccgcgcctggcgcatgagccaggcctgggccgcgtcgcggatctgcgaagcctcggcgttctgcgccacggccagccgcagaacgcgcggacctttgccgtcgtcatcgcccgcgtcgagcgtgccgccgacgcttgcgaagccgtgcttcggatcgaggcggatcacgaccgtttcgcccatgaacggaaattgcgcgccgtctttccaatcgatgcgcgtggcctcgacgcgcgcgtggcgctgctgggtttcgagcagcttgcgcaggatccagtcggacttttccttgatggcggcatccacgtcgcgcagcgtgacccagcgcggcgcgcgcaccgacagcccttcggcaccgaccacgaatccgatggtcttgcgcttgccgcgcttgaactcgtaggccacgcgcgccgagcccagcaccgcttcgcgcgtggcctgcgggtgcacgaagctcgcgagcgccagcgtgtcgcgaagcggaatggcgggcagcgcggggccggcgtcgtcgaccgaaggcggcgccacgggcggcgcggccttcttcttgacctttcgggtccgcggcagaggcggcttggccggcgcaatctcgttgcccagcccttcgaacaggtccatcgtgaactgaagcagtccccgcatgtcgggctcttttctttcctcttcagcccgcttcttgcggcacctgcagcggcgggctgtcgcggtaggcctcggggtcgagccggcgcatctcggattcgatccaggcctcgacttcgcgcatcagctcgtcgggcttgcggccgatgctgggaatggccgggccgatcgacacgtcgaccacgccgggacgcttgatgaaggccttgcgcggccagaccttggcggacgtgacggcaacgggaatcaccggcacgccggtttcgcacgcgagccgcgtgccgccgctcttgtaggtgcccttctggccgcgcggaatgcgggtgccttcgggaaacatgatgatccagatgccctgcgcaagcagcttgcggccctggttcacgaccttgttgaaggcctgcgcgcgctggctgcggtcgatgtggatcatgtcgagccgggccatggcccagccgaagaagggcacgtagatcagttccttcttgaacacgaaagccagcggatgcggcatcaacgtgggcatcaggaaagtctcgaaggttgactggtgcttgaccagcaggaccgcgccggcgagcttgtcggcgggcaggttttccatgccggtcacgcgggtgcggatgcccagcagcacgcgcgcgccgccgatggcccagctgagccattgcaccgccatccagtagagcggaatgccgcgcttccagagcgaactgacgcacatgatgatgccccagggcaccacggtgacgagcatccaaagggcatggagcacggaacggataaacgccatcagacagccacctgcagtgcggcctgcgcttcgcgcgcaagcaaaaaatcgacaaaggcggccaggttctcgtgaaccatggtgttcgccgggtattcggggggcagcggattgacgccgcggcagaccgcgcccatgccggtgagcagcaggtgcggctcgcagccggccgccgccccggcctgcagatcgcgcaggctgtcgcccgcggtgggcacgtctttcaggtcgatgccgtagcggtcgccgatctggcggaacaggcccggcgcgggcttgcggcaatcgcagccttcgtcggggctgtgcgggcaatagaagaccgcatcgacccgcccgcccacggctgcgagcatcttgtgcatcttggcgtgcatggcgttgagcgacgccatgtcgaacaggccgcgtcccaggcccgactggttggacgcgaccaccacgtgccagcccgcatggttgagcttggccacggcctcgagcgcgccgggcaagggcgtccactcgatgtcgctcttgacgaaatcttcacggtgcacgttgatcgtgccgttgcggtcgaggatgacgagtttcatggcgctggcaataagccctcgtttcaaagctcaggccgccagccgctcgagctgcgccacgcggttcatcgccacgtgcagcgacatcagcagccccagccggttgaggcgcaggtcggcctgttcggcattgaccatcacgccgtcgaagaaggcatcgaccggttcgcgcagcgcagccaatgtctgcagcgaagcggtgtagtcgccggcatcgaactgcgcattggcggcgggcacgacctcggccatggcggcgtgcagcgccttctcggctggctcgtgcagcagcagttcgctcacgtgcgcatcggcttcgggcgctttcttgaggatgttgccgatgcgcttgttggcggcggccagcgcggccgcggcgggcagcgcggcaaaggcccgcacggctgccagcagcttgggcacttcgcccaggcgctgcggtcgcggcgcgagcacggcgtcgacttcttgcgcgctggcgccctgctcgcgcaggctgccggccagccggtcgagaatgaagtcctgcagcagggccgtggccttgccggcgtcgaagccgtcgatgtccttgaactgcgcggcggcgtcctgcagcagcgcatcgagcttcagcggcaggtttttctcgatcagcatgcggatcacgccgagtgcgtggcggcgcagcgcgaacgggtcgcggtcgccggtcggcaggttgccgatgccgaacatgccgaccagggtttcgagcttgtcggccagcgcgaccaccaggcccacgttgttgcgcggcagttcatcgccggcaaagcgcggtttgtagtggtcttcgatcgcgtcggccacttcggcggacaagccgtcgtgcagcgcgtagtagcggcccatggtgccctgcagctccggaaactcgccgaccatgtcggtcaccagatcggccttggccagctgcgccgcctgcaccgcatgcgcggtgagcgtggcgttccccagcggcgccgcaatggcgcgcgcaatgcgcatcacgcgctcgacgcgctcgccctgggtgccgagcttgttgtgatagaccaccttgcccagcgattcgacacgcgaggccagcgacttcttgcggtcctggtcgaagaagaacttggcatcggccaggcgcgggcgcaccacgcgctcgttgccgccgaccaccgcgctcgcatcctcggggctgatgttgctgacgaccaggaacttgttggtgagcttgttcgatgcgtcgagcagcggaaagtatttctggttggccttcatcgtgaggatgaggcactcctgcggcacttcgagaaactcgcgctcgaagctgcagaccagcacgttgggccgctcgaccagcgccgtcacttcgtcgagcagcgcgtcgtcgtcaatcggcacggtgccgccgccgacccgcacggccgcggctgcgagctggcgcgcgatctcggtgcggcgggcctggaagctcgcgatgaccgcaccgtcgtcctgcatctgcagcgcatagctgttggcgtcgcgcagcaccaccgggtcgacggccgcttcaaaacggtggccgtgggtttcgcggcccgcatgaagacccagcgcctcgaccggcaccacggcatcgccgtgcagcgcgaccaggccgtgcgcggggcgcacgaagctcacgctgctccagcccggcagttcgcagccggtttcgagctggtagctcatcaccttgggaatcggcagcttggcgatcgcttcggccagcgccttttggaggccttcggccagggtcgcgcccttggcggtgctttcgtggaacagggcttcggccttgccgtccggcgcgcgcttgaggcctggcacggccgaggcgtcagcgcccagcgcggccaggcgcttgagcagcgcgggcgtgggctggcccgaggcatcgagccccacggccacgggcatgagcttttgcgacacggccttgtcggcggcgcgctcggccacgtgcgtgaggtgcgcggccaggcggcgcggcgatgcgtaggcagtgagcacggcccccgcctcggcgagcccctgcgccacgagctggtcgcgcagcacgccggcaaaggcgtcaccgagcttcttcaaagccttgggtggcaattcctcgacaaacagttcgacaagaaggctggcagacgacatggctcagagggataggacgaaaactgcgccgcgggcggcgccggtcacgggcacgcagcgatgcggcaccgtggaagggaaggaaaagaagcaggcgcggctcatgcggcaacggcaccattgtggcggcgctccatcgtgcggcgcgccatcagcgcgagcaccgcggccaccagcagcggtgcccagacagtgaacacctcgttgatcagcacctgcgcgccgcgtggcgagaagaagcgcttgagcgcgatcggcgacacctcgatgggccgccacgggctgaagtagcgcacgtcgctgaacggccagaagaaggcgatgccgatgccgccgttggtcagcatgtccaacagcggatgcgacacggtgcacagcgaaatccaggcccagccgatcgcccggcgcatgccccagcgcggcgcgagccaccagccggcaaggccgagcaccagcgcgaacagcaaggtgtgcgtgaagccgcggtggccgcccatgccgccataggcgatgccgagcttgaaggccaggccgtcgaagtcgggcacgatggacgcgagcatgcccgcaagcagcgccgcgaccggcacgcgccgcgtgcccagcccgatggctgcgcagacgggaacggcgacgtgggtgaagacggtgggcatggggcagtttcggcaatggcctgaccggtcaggctgccttcttcggcggcatctgcgcgacccattcgcgcggcgccatcgggaagcccagccgctcacggctctcgtagtagctctgcgccacgctgcgcgcgaggttgcggatgcggccgatgtaggccgcgcgctcggtcacgctgatggcgccgcgcgcgtccagcaaattgaagctgtgtgcggccttgagcacctgctcgtaggccggcagcgcgagctgctcggtcatgaggtgcttggcctgcttctcgtgcgcggcaaaggcggtgaacaggaactcggcgtcgctgtgctcgaagttgtaggtcgactgctcgacctcgttctgcttgtagacgtcgccgtagctcaggccttcggtccacgtgaggttgtagacgttgtccacgccctgcaggtacatcgccaggcgctcgaggccgtaggtgatctcgccggtgatgggcttgcagtcgatgccgcccacctgctggaagtaggtgaactgcgtcacctccatgccgttgagccagacctcccagcccaggccccaggcgccgagcgtcggattttcccagtcgtcctcgacgaagcggatgtcgttcttcttcaggtcgaagcccagcgcctccaggctgccgaggtacagctccaggatgttgctgggcgccggcttgagcaccacctggtactggtagtagtgctgcaggcggttggggttctcgccatagcggccgtccttggggcggcggctgggctgcacgtaggcggccttccagggctcggggccgagcgcgcgcaggaaggtggcggtgtgcgaggtgcccgcgcccacttccatgtcgtacggttgcagcagcgcacagcccttgtcggcccagtacgactgcagtttgagaatgatttgctggaaggtcaacatgaagcgggccggcgtgaccgggcgttggacggtagcgcggcggttcaccgcgaaagcagacgattttacggtcggagggcaactctcccacagccggccgggatgccggccgccggcgcggcgccgcgggccgtgcgataactccgagccggttgcgcgcgatctcctctcgatcgcctcgcaattgcctttttcaagtctttccgagcttctccgagcccctaccccggtctcccgccctcgccccgcagtcttgcacgagcccgcgggacccgctccttttccgtttcatccagacatgccagcgccctgcatcggtccgagttccccgttattcatcgtcctcaatgccggctccggcagcgcggacgccgcccaaatccgccggatcgtcgaggagggctgcgccgcggcgggccgccggcaccgcatcttcgtcgtcggcgaacgcgcgacggtgcaggcgctggcgcgcgaggccgtcgaacgcgcccgcgccgtgggtggggtggtggtggccgcgggcggcgacggcaccgtcaacgcggtggcgcaggccacgctcggcagcgggctggcctttggcgtgctgccgcagggcaccttcaactacttcagccgcacccacggcattccgcgcgacacggcagaggcgctgcaggtgctgctgaccgggcagccccgaccggcgcaggtggggctggtcaacgaccgcgtctttctggtgaatgccagcatgggcctgtacgccgagctgctggaagaccgcgaaagctacaaggcgcgctacggccgcagccgctggatcgcgttcttcgccggcctcctgaccgtgatgcgcggccaccggcactggaacctgcgcatggcctggcgcggccaggagcgcgacctgcgcacgccgacgctgttcgtgggcaacaacccgttgcagttgctgcaggtcggcatcgaacacgccgatgcgcctgaaaacggccagctggctgccgtggcgctgaaacccatgggggttcttgcgatgccgggcctcctggtgcgcggcgccctgggccggctcggcggcgccgacgaggtattgagctttccgttcgaatcgatgacagtgaaagcaggccgctcgcacggcgcgcgccgcgtgaaggtggcaaccgacggcgaggtcgcatgggccgagatgccgctgctgttccgcgtctcccccgagccgctgtggctgctgcggcccgacatcgcgcccgaactggaagccgccaaggaatgagctgcctgcttcagatctccgacacgcatttcggcaccgaacggcccgaggtgatggaagcgctcgaacggcttgcgcatgccttgtcgccgcaggtggtggtgctctcgggcgacatcacgcagcgtgccacgcgcgcccagttcgcgacggcgcgcgccttcgtcgacaggctggccgcgccggccgtgattgccattccgggcaaccacgacattccgctttttcagttgggggcacggctgttcgcgccttatgaaaggtacgccggcgcattcggcaccgacctggagccggtgttcgaatccgccgaatggctggtggtctcggtcaacaccacgcgctggtaccggcacgcggacggcgaggtttcatccgcgcagatcgagcgggtggcggcccggctggcgggcgcttcgcccgagcagctgcgcgtggtggtcacgcaccagccggtgatggtgacgcggcaggaagacatgcggaaccgactgcacgggcgcgaagccgccgtggcgcgctggtgcgcggccggcgccgacctgatcctcggcgggcacatccacctgccgttcgtgcgttcgctgcacgacgcctatgccggctgtccgcgcacgacgtgggcggtgcaggccggcacggcggtgtcgtcgcgcatgcgtgcggggcaccccaattcggtgaacgtgctgcggctgggcgacgcggaagacggccgcgcctgccaagcggagcgctgggaccattcggccgcggacaaggccttcgtgtgcgccaaagtattgcagctcccgcttgccagcgccgcggcacccgcttagggtgcgcggcatgttgacggaagcccctgccctcgttctgcttgcgcgccagctcggcgagcattcccttgcatggttcgcatgcgttctcgccctttcggtgttcggcgccgccgtggcctgccgggcatggcggcagcgccgggcccggaccctgccgaccggggaaccggaagaaccgcggctcgcggccgcgctggcgacgggcttcctggtgatcctcggggcagcgagcctggtggcgtacatcgcgtcgaagctcggcgacggacgcctgctcggcctggccgaccaggcgctggccgatgccatcggcgaccatgtgccctgggccgccctcgtcgctttcagctggctcacgcacctgggcgacgccgaactgctcgcgccggtgtgcctggcagtggcctggctgctgtggcgcaaggcacatcatggcctggcgctgggctgggtgatggcgctcgggggcatcgtgctgctgaaccccgccctcaagcgcatcttcgcgcgggcgcggccgctgcacgaccatgggctggcactggaaacgagcttcagctttccgagcggccacagcgcgggcgccatcgtgagctacgggatgctgacgtacttggcgctgcgcctgttgccggcgcgctggcatgtgccggcggccatggcggccgcggctgccatcgtcaccatcgcgtgcagccgcgtcttcctgcaggtgcatttcgcaagcgacgtggcggccggcctgctgaccggcctcgcctggctgctcgtgtgcgtgagcagcctcgaatacgcgcggcaccgcaagcggcgtgccgcgcgctgagcgggatcaatactcccagaagatgcgctggagttctttcgtgtcgctggtcttggtgagggccaccatcgcgaggatgcgcgccttctgcgggcgcaggtcgtgcgccaccacccagtcgtacttgtcgtcgggctgctcggcattgcggatcacgaagccgtcggccacgcgcgagctgcggatgatgatcgcgccgtcggtgcgcgccttctgcaggttcggcacgatgcggttggccaccgagccgttgcccgtgccgccatggatgatcgctttcacgccgctcttggcgaacgcgtcgatggcgatggacgaaacgccctcgtagcccatggcgatctcgaccggcggcagcgcgttgatggcgtcgatgtcgaattccgaagccatggtgtggcgcttgaccggcgcgcggaaccagtagttcttgccttcgaccaccatgccgagcgggccccactggctcgagaaggcgctggtcttgacattgacgttcttgctcacgtcgcggccgctgtcgatgttgtcgttcatcgtcacgagcacgcccttgcccgccgcatccttgctgccggccacgctgaccgcgtcgtacaggttgagcgcgccgtcggccgaaagggccgtgcccgggcgcatcgaaccgaccacgacgatcggcttgctggtgcgcacggtgagcgtcaggaagtaagctgtttcttccagcgtgtcggtgccgtgggtgatgacgatgccgtccacgtcggcctgcttggacagcgcggaaacgcgcttggccagcgtcagcaggttgtcgttggtgaggctttcggaagcgacctggaacacctgctcgccgcgcacgttggcgatcttggagagttcaggcaggccggcaatcagcttgtccacgccgaccttggcggccacgtaggtggcgctgttgacggccgaggcgcctgcgcccgcaatggtgccgccggtggccaggatcaccacattgggcaacgcctgctgggcttgcgccagggcgctggccgcaagcagtgcggcgccggccgcgaaggccctgaaacggggagaaaggtacatgaaggaactcctttgtcttgaacgaatttctggaagcggcgagaagatacatgaaccatgcccgcatgccccgcgcttccatgccggcatggcatgcggccatgcggattaccatcgccgggcgcaccgccgcaaatccatgccaatgaacgccgatcccaccgcccttcccccgaccgccgcccaggaaatgcccgccccggacggaccgctgtcgcgcgcccgccccgggcgcgagcgcatcatggcggccatccgctcggcggcggtcaccgagttcagcctgcacggcctgaagggcacctcgacacaggccattgccgcccgcgccggtctcaccaagccccagctgcactactacatcgccggcaaggaagagctctacgaggagctgctgatgcaggtgctgcatgcctggaaggtggtgttctcgttcgaggacgccagcgacccggccacggtgctgggcgactacatccgcaagaagctcgaccacgccttcgacaacccggagatctcgcgcatcttcacgcgcgaggtgctcgacggcggccgcaatctcgaccgctactggcccaatgccagggcctggacgcagaaaaaggtcgacgtcatcaacggctggatcgcgcgcgggcaaatgcgcccgctcgacgcgcgcctgctcctgatgcacatctgggccatgacccagagctacgccgactacgcgatacagacgcgcgtgatgctcggcctgccgcccgacgcacccatcgaccgcgagccgattgcacgcgagctggtggctttcgtgctgggcggctgcgggatcgacaggccgtagccgaccgccgcgaggcaggtcagacgaggttcacgcggccggttgccagatcgtagatgccgccgacgacccggaccgcgccgctctcggccataccgccgaggatgggggccgaggtggccaggcgtgccacgctctggcgcacgttctgctcggtggcggcttccagcaaggacgccgggttgcgccgcgtcgcggcctccacggccggccggatcgaggcgaccaatccgggcaggtgccccggcagcacggcgttttcctgcagcaccttgatggtcgcggcaatggcgccgcagttgctgtggccgagcaccatgatgagaggcacgtcgaggaacttggccgcgtattccatgctggcgatggcgtcgtcattgacgaagttgccggccagccgcaccacgaagagatcgcccgggccttggtcgaaggccagttccggcgccacgcgcgaatccgcgcaactgagaatcgccgcgaacggcttctggcccgtggtgcgcgccacgcggccgacgctgaagtcgcgctgcgtcggcttgccctgtgcgtagcgcaagttgccttgcaccagtcgccggagcgcggcctcgccgccgatgcggttgtcgggcagcggcgtatctgccgcgaacgcattggcgccggaggccaaggcagcgaaagcggcggcaccactcagcaaccggcggcgcgacgttgccggcaatgtggcggaaggaaggcaatcacacatgaggaactccgttcttggtgaatagtgagctcgccggttgcccggcagggaaggccggggggctttcgcaccggcgtgcgaattgttacgctctgtatcgcaaataacaaagtccaaaaattgcatggattcgatgccgccgccggatctggcgctttccatctctcatgaggcccgctgcaaggcggtcgcgctctattgcgacgcgatcgtgcgcatgcactggggcgagaggctcatcaacaagatcttcggccgcgtcatgcagtcgcacgccgccgggcggctggtcgtgcagcactaccgctggaaagaagaaggcgccgaacgccccacgctggcgctgctgcagcgaaacgcgagccacggtacgcgcacgctggccagcttcgtcaccgtcctgcggctcacgggcatggtggcggcggaggccgacccccgtgaccgtcgcgtgcggtacctggtgccacaggagcggctcatcggcgggctgcgcgcatggattgcccaccatctgcgctgctgcgaggcgctgggcctgctcgatgccggccacgcggcgaggctcacggacgatgccgccttcttcgatgcctttgtctgccgggccggcagcatcctggaccgggtcgtgtcgcaccgcggccgcttcggcggctggagctggttcgacgaccgcgacggcggcgggcgcgtcgcgatgctgctgttacgcgatcatttcaaggccaaccccgaggctcggtcgcccttgctggcgtttccgctgcgcgcccacgaactcgccgacgggctgggactgtcgcactcgcacgtgcgcggcatgttgaaggaggcgatagaggcgggccatcttgctcacgatgcggggcgcgcgcaggtgcggctcacgcctcgcttccttgatgaaacgatgagctggctactgcacttcctgtcgtggtttgccgaggtcgcgcatgcggcccggcgggcctgctgaaaacgccgcacggcgtggggcggtgcggcttcaggcggtcgcggaaatgacttcgtcgatgcgcgcatcgttcgtggcttcgggccggctgcgcgtcctgctgcgctgcccgtcgatggccacggcggcttcgccatgcaccgtcacgcgccgcaccaggcgcggctggttgccgtagtcgttgatcgcaaagtgctgcgtggcgcggttgtcccagatcgccacgtcgtcctgctgccagctccagcgcaccgtgttctccaggcgggtcacgcggttctgcaacagctcgaagatgcgcgccgactcgccgctcgacaaccccaccagcttcttcacgaaatgcccgagcagcagcgcgcgctcgcccgagaccgggtgcacgtgcaccaccggatgctcggcttcgtacaccgccgagacgaacacgttgcggtggtggcgcaggcgttcttcttccacctgcacgcggtcggcgccgtagtcgtagtcgttgctgtgcacggcccagagctgatcggccagttgcttcagttgcgcgggaaggcgctcgtaggccagggcggtgttggcccacaccgtgtcgccgccataggcaggaatcttgacgccgcgcaggatggatatcttgggaaaggcatcgacgaaggtcacgtcggtatgccacgaatctgcgcgcccgccgcccttggaggcgtcgagctcgaacagcttggtgcccgtgggcgacggcaccgtgggatgcgccaccgtgcggccaaagcgcgcgccgaacgcctggtgcgcggcgtcgtcgagatgatcctgcccgcggaagaacaacaccttgtgcttcaccagcgctgcgtcgagctgctcgatcgcttcccgcggcaggtcggcggacagcttcaggttctgcacctcgccgccgatgtggcccgcgacgcggcggatgcgcagctcgccgaagctcgtatcgaagggcgtagtgagggcgtgatcgctcatctggggaatctcctgttcatgcagctggaaacccggcaaggccggaggccgccgattctctgcgtgcatgtggctgcgcccaacgaacgagtctgcgtttcgacatgcgcgaatcttctaagcaggaaggcgcgtggaaccgctccgcattggccgatccccagtccggtgcatccggactggcacgtcgcttgcataacctgaccacttgctctgattaatcggtcaaacaccatgcgcgtgctcgtcgtctactgtcatccggtcgaaaccagcttccacgcggccctccaccaggaggtgctgaagaacctgcgcgcggccggccacgaggtggacgattgcgatctgtacgccgagggcttcgatccggtgctctcgcgcgaggagcgtctcggataccacgacgtgccgggcaaccagttgccgctcaagccttacgtggaacggctgcagtgggccgagggcatcgtgttctgttttccgacctggtgcttcggcctgcccgcgatgctgaaggggtacttcgaccggctcttcatgccgggcgtggccttcgacatcagcgacccggccgacgtgaagccgatgctcacgcacatcaagcgcatcagcgccgtggtcacctatggccggccgcgctggatggcctggtacatgggcgacccgccgcgcaagatcgtcacgcgctacatgctgcggctcacgggccggcgcgccaaggtggactaccacgcccactatcacatgaacgtggcgaccgagccccaactcaagcgcttcatggcacgggtgggcaccgcgatggcgcgcttcgcatgaacgccgcgccttcgctgctcgacaacgcgcgcctcccgcgttggctgctgccttcggactggccccagcgcgatggcgtgccggtactggcacgccttgcgctggaagccggccgcgtgcagtcggtgcggcccgcgtccactgacgacgccgcgcgctccgccgaaagctgggacctcgcgggtacgctcgcgctgccgggcttcgtcgacgcccacacgcacctcgacaaggccttcacgctgccgcgcatgaaagcggtgcagccgggcctgctcggcgccatcgacgcgatgctgaacgaccgcgtgcactggagcgccggcgacgtgcacgagcgcgcctcgcgcgggctgcagtgggcctgggagtgcggcaccacgcacgtgcgcacccacgtcgactggtgggagcccgatgcggtgccgctggcctggcccgtgatggccgagttggcggaggaatgggcgggccgggtgcggctggagcaggtcagcctcatcaagctgccgttgttcgaagacgcggcgcgggccatgcggctcgcaaggcaggtgaaggccacagggccgcatgcgctgctcggcggcttcgtgcactccaccaactggagcgagaacgcgctgcgcaacctgctggtgtcggcgcaggcctgcgatctggacgtcgacctgcacgtggacgaagaactgaattcagcggcggtcggcttgcagaccaccgcccgcatcctgcgcgagatcggcttcgaaggccgcgtggtctgtggccacatctgcgcgctggccgcgcagcccgaggcccaggcctttgccacgctcgatgcggtggcgcgcgcaccgatcactgtggtgtcgctgccggccaccaacctgctgctgcaggacgcggtgacgggccgcaccccgcgcctgcgcggcatcacgctggtgaaggaagcgcgcgagcgcggcattccgctgctgtttgcgagcgacaacgtgcaagacccgttctgccggctcggcagcttcgatcccgtcgaggcgctgagtaccgccgcgctggtggcgcagctcgaggagcccttcgacaactggtcgcaggcgctgtgccgcggcgactggctgcagcgtgggcccgccacgacggcgcccacgctggtcggtgccaaggccgatctggtgctgttcacgcaggccgaccgccacggctggccctcgcgctcggccactcgcgcggtgctgcgcgaaggccgcgtcacgcacggcgatgcgacgccctttcttccccgctaacgcacaaggacaccccatgctccacggctacattccgccccatcgcttcctgccctacctgagctggaccgaaatcgccgccctgcccgaccgcgagaacaccgtcatcgtgctgccctgcggcgccatcgagcagcacggcccgcacctgccctgctcggtcgacagcgtgatttcatcgggcgtgatgggcaaggcgctcgagaagctgccggccgaagtgcgcgccttcgcgctgccgaccatcacctatggcaagtcggaagagcacctgcactttcccggcaccatgacgctgaccggcaccacgctcttgtcgaccgtgacagagatcggcgaatcggtctaccgcgcgggctttcgcaagctgctctttgccaatggccacggcggccagccgcaggtgctggagatggcggcacgcgaactgcgcctcaggcatggtgacttcgtggtggtgccgcatggcgtgtcgcgcctgccgaacgcatcgagcaagcagatcagcgagcaggaaaagcgcctctcgatgcacgccggccattccgagaccgcgttgatgctggcgctcgcgcccgacacggtgcacatggagcgcgcggccgccaactttccgccgcccttcccgatcaagctgctgtcggccgacggccgcccggcctgcgcatggaccgcgcgcgacttcggccccagcggcgtgatcggcgacccgaccagcgccacgcgcgagcagggcgaagaaatcctggacacgctttccgacagctgggtgcaggcgctgaccgagctgcatgcgctgcgctgggttgtgcgcgaggaagccacctgggagcgcggccaccagcaaggcttcatccagcagtcgttcgagcccgcctgaggcgcgctacttgcatcggtccaccggttttttcaactgttcttccaccagacccgagaggttcccaccatgcgttctttcgctctttccatggccggcgccgccgcgctcgcactgctgaccgccgccgcaccggcccaggcacaggacaagttcacctacatgaccaactggtatgcgcaggccgagcacggcggcttctaccaggcggtggcgcaaggcatctacaagaagtacgggctcgacgtgaccatcaagatgggcggtccccaggtcaacatcacgcagatgatggccgcgggccaggccgactgcatcatgggttcgagcgacattcagatgatgcaggtgcgcgaaggcggcgtgccagtggtcaacgtggcggccttcttccagaaggatccgcaggttctgatcgcgcacgacgacgtgaagaagttcgaagacctgaagggcaagacgctcctgatcggcgcgcaggcgcagcgcggctactggccgtggctcaaggccaagttcggccttaccgatgaacagacgcggccctacaccttcaacatccagcccttcgtggccgacaagaacacggcgcagcaaggctacctgacctcggagccctacgccatccagaaggccggcgtaaagagcaccgtgctgatgttcagcgaccacggcttcccggcgtatgccaccacggtgtcgtgcatggaaaagacggtgaaggagcgcagcaagcaggtggaagccttcgtcaaggcttcggccgagggctggaagagctacctcgccgatccggcgcccgccaatgcgctgatcaagaaggacaaccccaacatgaccgacgaccagctggcctacagcgtcgccaagctgaaggaaatgggcatgatcaccggcggcgacgcggccaagctcggcatcggcgtgatcaccgatgcacgctccaaggcgagctacgacttcctcgtcgccgccaagctgctcgacccggcgaaggtggaactcgccaagacctacaccaccgagttcgtgaaggacgccaaggttctgccttgagccctgtgccatgaatcgcatcgagccccacaccctcgcgccgcccgcggtgccagccgtgcccgcggtggaagttctctcggccgagaagacctatcccaacggcacgcaggcgctgctgccggtggacctgtcgatcgccgagggcgagttcgtcaccctgctcgggccctcgggctgcggcaagagcacgctgctgaagatggtggcgggcatgctcgagcccagcgacgggcggctcctggtgtggcgcaagccggtcgccgagattcacagctgcccgcacaagctgtccttcgtgttccagtcggccacgctgatgccgtgggcgagcgtgcgcaccaacgtgcggcttccgctcgacctggccggcgtgccgcgcaaggaggccgacgcgcgcgtgacggaatcgcttgcactggtcggcctggagaagtttgccgacgccctgccgcgcgcgctctcggggggcatgcagatgcgcgtgtcgatcgcgcgcgggctggtcacccagcccgacctgctgctgatggacgagccctttggcgccctcgacgagatcacgcgccacaagctcgatgccgacctgctcgacctgtggcgcaagaagaagctcacggtgatcttcgtcacgcactcgatccatgaggcggtgttcctctcgacccgcgtggtgatgatggcagcgcggccgggccgcgtggtggaacaattccacatcgacgagccctacctgcgcacacccgacttcatggtgacgccggaattcgcgcgccatgccaagcgcctgcaggacagcctgctgcgcgcgagccaaggcgacgaggagcacgcgcgatgaagaagagcccgccccttctgagccaaccgcgtgtgcagcgcgtgctctaccccgtgctcatcggcgtggtgctggtggcgctgtggcagtggatggtggttgccatggagctgccgccgtacctggtgccttcgcccttcctcatggtgcagacgctcgtcaccgactgggtgccgctcggcaatgcgctcctggtcacgctcaagatcacgctgctgtcgttcgcgctggccacggtcgcgggggtgttgatctcgttcctgttcgtgcagagcaagcgcatcgagaccgcgctctttccgtatgcggtactgctgcaggtcacgcccatcgtcgcggtggcgccgctcatcatcatctgggtgaagaacccggtggcggcgatgacggtgtgcgccgcgctggtggcgctgtttccgatcatcagcaacaccacgctcgggctgcgcagcatcgaccccgacctgcagagctacttcaagctcaaccgcgccacgcgctggcagcaactggtgcggctgcgcattcccagcgcgctgccgtacttcttcggcgggctgcgcatctcgagcggcctggcgctgatcggcgcggtggtggccgagttcgtggccggcaccggcggctcgggcgcggggctggcctaccagattctccaggccggctttcaactgaacattccgcgcatgttcgccgcgctgctgctaatttcgctgaccggcgtcgcgctgttcgtgctgatggcctggctcaccaagctggcgctgggctcatggcacgcgagcgaactttcccaggattgaaaaccttgaccatgaacgcttccatttccatcatcgaacagctgctgttcgacctgcccgacctcgactggatcaccgacgaaagccgtgtcgcgcggctgtcgcaagacttctcgtggttcagcccggtgctgaaccgccagttgaaagacaagcgcgccgacgtggtcgtgcgtccgcgcaccgaggaagagattcgcgccgtggtcggcgcctgcgcgcggcacaacgtgccgatcaccattcgcggcagcggcaccggcaactatggccagaccacgccgctggcgggcggcgtggtgctcgacatgacaggctacaacgcctttctgtgggtgaagcccggcgtggcgcgcgcgcaggccggcattcgcctgggtgagctcgagaagcaaaccaaaccttcgggacaggagatgcgctgcctgccctcgacttaccgcagcgccacgctgggcggactgttcggcggcggcttcggcggcgtgggctccatcaactatgggccgctcggcgcaccgggcaatgtgctcggcatccgcgcgatgaccatcgaggcggagccgcagatgatcgagctgcgcgggccggaggccatgcgcatgcatcacctctggggcaccaacggactggtgctggaactcgagattgcattggcgccggcgcacccctggctcgagacgctggtgaccttcgacggttttgcagacgcgctgcacttcgccgacaagctggcgaacgcgccgggcatcgtgaagcgggagatcgcattcttcggcgcgccgattgcggaccacctcgcgcagcttgccgcgcacctgcccaagggctgccacacggtgctgtcgctgatggccgaatcatgcgaggccgcattgctgcagctggccgaagcgcatggcggcacggtgggctaccgcaagacggcagccgaggtgcagaagagcaaccgcacgctgatggagttcacctggaaccacacgacgctgcatgcgctcaaggtggacccgacgctcacgtacctgcagagcggcttcgtgccgggccggcatgtcgagcagatcatcgagatggaacaactgctcggtggcgaggtgctgatgcatgtcgagttcctgcgcaacgtggcggggctcatgacctgcagcggattgcagctggtgcgtttcagcaccgaggagcggctcgcggagatcatcgacattcaccgtgcgcacggcgtgcacatcaacaacccacacgtgaacatcgtggaagacggcaaggcaggcgggccgctgccgccggaggtcatcgagacgaagaagcgcttcgatccgatgggcctgctgaatccgggcaagctgcgcgactggccggtgaaaacggcgccggccgccggctgaccagggcgcgggcgctcaggcccgccgacggcgcagcccgaaggcggccgccacgatcgcgaacgccgtgatccagagcggccacaggccgaacggcgccacccagcgcgcaaagggcgtgagccccgtgcggccttcgaccgatgcctcgagcacgccgcgcgtgagccgcggcagctcgtgcgtgacacggcctgcggcatcgatgaccacggttgcgccggtgttggtggcccgcaccatcggccgcgcgaattcgagcgagcgcatgcgcgagatggcgaggtgctggtcgatggccacggagttgccgaaccaggcgatgttgctcacgttgagcaggatggtcggggccgtggcctcgttcttgaagttggcgccgatctcgtcgccgaacaggtcttcgtagcagatgttgggcgcaacgcgctggccctgccaggcgaaaggcgcctgcgccaggccgccgcgggcgaagtcgccgagcggaatgttcatcatccggatgaaccagcgaaagcccggcggaatgaattcgccgaacggaacgaggtggtgcttgctatagctgtagggccgcgcggcgccgggctggaagccgagcaccgcgttgctgtaggtcccctggccgcccatcggcaggccgacgatggcggcctgcgtgccatggctgtagcgcgcctggatggcttccagatagccggcgggcagttgctgcggcagcagcggcagcgcggtttccggcgtgacgaccagcgaggccttggcatcgcgcagctgttcgccgtaccagcgcagcgcaaggtcgatgccgccgccgggaatgaatttttcgtcttgggggatgttgccctgcagcagtgccatctgcaggtggccgctcgagcccttgtcaccctgcgcgctggcgggcaacgggttgaccaggtgcggcgccgcaaacgcagcaatgacgaggaccacggcctgtgccagccccagtgtgcgggcgggccgtgtcagtgcaacgagtgccgccacgagcgcggcgaccgcgccgatgccgtacacgccgatccagggtgcccaggcggccagaggcccctcgacgtgcgcatagccgccggcaccccaggggaagccggtgaaccagctgccgcgcacgagctcggccagcgtccagagcgctgcgaagaccagcgcgccgctcaccggcccctgcgggcctcgggcgacgaaccaggcacaggcggcggcgtaatagagcccgagcgccgccgcgagcgagagcaccgcaatggccgcgagcggcgccggaaggccgccgtaggtgtgcatcgagatgaaaagccaccagaagctgccggtgagccaggcggtcgagaaaagccagccgtgcaagccggcgcggcgccagcccgcgccttcggcgcgcagccagtcgagcaggccgacgagggccgccagcgaaacgagctgcagccaccacagcgggcggccgttcgcgggccaggcgatggcggcggcctgcgcgagcccggccagcgcgaagccgagaaggcgcagcaggcccacggcggaaaaggtctgctgggtgcggagcgttgccgctgcgggcagcggcatcagtcggccgcgtcgctgccgcgggccggggacaccttgaaccagcgcacggccccgcccttggtgtgcagcaccacgaagtcgaagccgccgatggcgtgatgctcgccgcgcttgggaacgtggcccatctcgtgcgcgatgaggccgccgatggtgtcgaagtcttcgctcagctgttcttcgtcgaaggtgatgccgaaggcttcggccacgcggtcgatgggcgtgtcgcccgagacgcggtaggtgtggtcggccaagccgaagatgtcgccttcgtcttcggcaatgtcgaattcgtcttcgatctcgccgacgatctgctcgagcacgtcctcgatggtgatgaggccggccacgcggccgaactcgtcgatcacgatggccaggtggtttcggttgccacggaactcgcgcagcaggtcgttcaggcccttgctctcgggaacgaaggtggcggggcgcagcagagcccggatgttgagccctggcgcgcgctgcagcttgagcaggtctttcgccagcaggatgccgatgatgttttctttttcgccttcgtacaccgggaaacgcgagtgcgcggtgtcgatgatcagatgcagcagcgcgtcgaacggcgcgtcgatgttcaccaggtccatgcgcggggcggcaaccatgacgtcgccggccgtcatgtcggccatgcgcagtacgccctcgagcatcacgcgcgactccgcgccgatcacctcgttgtcctcggcgtcggcgagggtttcgatcagctcgtcgcgcgagtcgggaccggggtggatgaattcggccagcttctggagaaagccgcgcttgtcttcccgttcgacgggagcgcgttcagagtgaggttcggccactgcgggaggcgtagttgaagagctgcaaggataccggatgcgcgtgacaggctctaccgcacggccctcatggccctttctcgaggacgctcagggggcagatttgcttcgcgcgtctctcatgccgctgcgcacttcctgcaggctggcaagaaaggcccagaactgcttggcgcgggtcttgagctggtaatcgaccgccgcgtagtgctcgagcgcgatctcgctcatgcggctgtcgaaggtggcgctcggcagctgcagatgcgcctcggactcggaaccgctgcgcaccacggtggcaccggcgttgcgggcgatcttcagcatggcggcgttttcgctcagcgcatggatgaagagcatgcccacgccttcgttgcgcgccacgaccacagcacgctcgaacagccgggcgccgtagccgcggccgcgcgcgtgggcggacaccgagacgccgaattcggcgcagtcgctgtgctggtcgtccggcgcgaacgccaggtgggccatggcaatgaggtcgagccggcggttgtagatgccaaacagctcgtcgcggtcgaagtcgagcccgtcgacgtagcgctgcacttgctcgtcggccgcggcatagccgaagcgcaggtagcggtcgtgcgggctcaacgccagcaggtgttgcgcgatgcgctcgcgttcgcgcgggccgatcgaacggatcggcaccatgacgggtgagggcgcggagctcgcgcgtggttgcgcctcaaccatgggcgctttcaggaaagagccgaggccgagagacgccttcagaagggtcttggcggtaagcatggctcaaatataagggttttcccttaatcaacaagcctgcatgggtactttcgagcttcataggtgacgaggtaccaaagcgcgtgtcgttcccgcaaccgtttcgtggctaaaccggcacagctgttgtggccttgacacggtcgagcacgaagctggtcttgcagtcctcgacgctggggtgcttgagcagggtgtccatgatgaagcggctgtagtgccccatgtcggcgaccaccacgcgcagcaggtagtccatgtcgcccgtgagggccgcgcactcgacgacttcgggccaggtctgcacgctcgcccggaacaggtccatcgggttgcgcttgtggctttcggtgtgcttttcgagccggacgttcagataggcggtgaggccgaggccgatgacctcggggcggacgagcgcaacatagcggtcgatgacgccgctttcttccagccgcttgacccgccggagcacggcgctgggcgacaggctcacctgttcggcgatctggtcgtaggtggcccgcccgtctgcttgcagcgtgcgcagaatcaacctatcaatcttgtctagtgcttccatatccgcattttcgcagttttattgcgtcatggccattttcaacgcccattaacgctgaaaacgtgagggggatccgctctacagtgcatcactggtcgttctcgccctttcgctgactgttttcattccttcgaacccacttctggagaccccacatgagccacgccgacgccccccctttcacgccctgggagaacccgatggggaccgatggcttcgaattcatcgagtacgcggcgccggatccggtggccatgggcaaggtgttcgagcgcatgggcttcacggcggtggccaagcatcgccacaagaacgtgctgctgtaccgccagggcacgatcaatttcatcgtgaatgccgagcccgactcgttcgcccagcgctttgcgcgcgaacacggcccgagcgtctgcgccatcgcattccgggtgcaggacgccaagcaggcttacgagcgcgccatctcgctgggcgcctggggttttgccgacaaggcaggccccggcgagctgaacatccctgccatcaagggcgtcggcgacagcctgatctacctggtcgaccgctggcccggcaagaacggcgccaagccgggagacatcggcaacatcggcttctacgacgtggacttcgaaccgctgccgggcgtggcctcgcaagatgcgctggcgcccaagggcaacggcctgacctacatcgaccacctgacgcacaacgtgtaccgcggccgcatgaacgtctgggccgccttctacgagaagctcttcaacttccgcgagatcaagtacttcgatatcgaaggccagctcacgggcgtgaagagcaaggccatgaccagcccctgcggcaagatccgcatcccgatcaacgaagaaggcaaggagcaggccggccagatccaggagtacctggacacgtaccgcggcgaaggcatccagcacattgcgatgggctcggacaacctgtatgaaaccgtcgacgcgctgcgcgccaacggcgtcaccctgctcgacaccatcgacacgtactacgaactggtcgacagccgcattccaggccatggcgaaaacgtcgccgagctccagaagcgcaagatcctgatcgacggcaagaaagacgcactgctgctgcagatcttcagcgagaaccagctcgggccgatcttcttcgagttcatccagcgcaagggcgacgacggcttcggcaacggcaacttcaaggcgctgttcgagagcatcgagctcgaccagatgcgccgcggcgtgctgtcggccgcaaaataatcatttctttcactggccaggagcctccatgcgcagcacgttttcgatcggcttgactctcatcgcggccgcggccgttctttcgggttgcgccatggcgccggccacgccggcggccggctcctcgcggctggacgtggtgcagaaggccgcggcgctgcgcgtctgcacgcctggcgactacaagccgttcagcttccagaaggccgacggttcgttcgaaggcatcgacgtggacctgatggcgggcttcagcaccagcctcggcgccaagccggagtgggtgaagaccacctgggccaacctgctgcccgacctcaccgccggcaagtgcgacatggctgttggcggcgtgtccgtgacgaccgaccggcagaagcgcgccttcttcagcgcgccctacatggtgaacggcaaggcgccgatcgcgcgctgcgccgacgttgccaagtaccggaccgtggccgacatcgacaagccttcgacgcgggtcatcttcaatccgggcggcagcaacgagcgctttgcgcgcgccaacttcaagcaggccaagctcacgatgcatggcgagaacgtgacgatcttcgacgaaatccttgcgaaccgcgccgacgtgttcgtgaccgaatccgccgaagccatcacgcagcagaagctcaagcccgggctctgcgccatcaaccccgacaagccgctgcagtacggcgagatggcgtggatgctgccgcgcgacgacgtggcgttcaaggcctatgtcgaccaatggctgcacctgcagcaagccggcggcgacttccagcgcgtgatggaccgctggctcaagtaacaaccaaacaacgctttcccatggacactcccgccgccgctgcccctgccgccgtcacgcccgtcgtttacggcgcttccgatcgcccgccgcgcggcgactattcgcgcggcggcgtggtgcaggccgactacacctgtccgcaggactgggccagctatacgccggccgatcacgacacctacaagcggctctacgaacggcaggcggcgcagctgccgggcctggcctgcgatgcgttcatcaacgcgctgccattgctgggcgtgaaggaccgcattccccgcttcgaggaaatcaacgagcggctgcatcgcgccaccggctgggagatcgtcgcggtgccggggttgattcccgagttgccgtttttcaccctgctggcgaaccgcaagtttccggtgaccgactggatccgcaagccggaggagttcaactacatcgtcgagcccgatgtattccacgacctgttcggccatgtaccgatgctgttcgacccgacctttgccgactacgtgcagcgctatggcgagggcggcatcaaggcgcacgaactgggtgccggcgagaagctggcgcggctgtactggtacacggtggagttcggcctcatccgccagcccgccggcctgcgcgcatacggcgccggcattctgagttcggtgggcgagttgcagcatgcggtgcgcagcgacgaaccgcaccggctgccgctcgatctgctgcgcgccatgcgcacgctctacaagatcgacacgtaccaggccaactatttcgtgatcgacagcttcgcgcagctgttcgagctcacggcgcccgacttcacgccgctctaccgcgcgctcgaggtcgagtccgacattcccgccggggtgctgctgccgggcgagaccggcaaggcctgaagaagacgcgcttctcggttcgattgcggcactctcgcgcactgtgcggtgccgcgcagctatcgcctgcgcgacagcgcccgccccgctcctaggacaagcccgctggcggctggctgcctctggctcccacaatccgcgcaaaaggagcttgcatgcagacatccgcgcgacaaaactatccggccgacgtgccgcacgagatccatccggaacagtaccggtccctgcctcacatgttcgacgaagccttcgggcgctacgccgaacggccgttctcggtctgcatggaacgttggatgtcgtacggcgagctcgacacgttgtcgaaggcgctgggcgcatggctccagtcgctcggcctcgagccgggcgcgcgggtggccatcatgctacccaacgtgccgcaattcgccgtcacgatgtgcggtgtgctccgggccggctatacctgcgtcaacgtcaacccgctctatacggcgcgcgaactcgagcatcagctcaaggactcgggcgccacggccatcgtcatcctggagaacttcgcggcgacgctcgaacaggtgatcgagcgcaccccggtcaagcacgtggtcgtcaccgcgatgggcgatctgctgggcggcctttatggcgcctggatcacggtcgcggttcgccacctggcgaagatggttccaccctacaagctgcccctgggcaacggccgcaccgtgacgccgtttccgaaggtcatcgaagaggggcgcggacgcacgctggcggcggaccagagcacgctcgattcgatcgccttcctgcaatacaccggcggcaccacgggtttgtccaagggcgcggtgctgacccatcgcaacatcgtcgcggccaccttgcaggcggaggcgtggttcacgcccgcgctttcgaaggcgggtgacctggcgaaggtcaacagcattgccgcgctgccgctgtatcacatcttcgcgctcacgctctgcctcctggtcatccgccagggatcgcacatgacgctgatcccgaatccgcgcgatttcaacaagttcatcgcggtgctcaagaagcgcccgttccacatgctgcccgcggtgaacacgctgttcaatgcgctgttgatgcatcccgaattcaagtcgatcgatttctcgacgctgttcgtgtcgcaggcgggcggaatggccgcttccgagggcacggccaggcggtggttcgaggccacgggctgcccgatgatcgaaggctggggcatgagcgagacctgcgccatcggcaccaacaatcccgtgtcgaataccgagttcacgggcaccatcggcttgccgctgccgagcatcgagatcgccatcaaggacgacgaaggcaactccctgccggtcggatcgccaggcgagctctgcatcaagggccccaatgtgatgaggggctactacaaccagccggccgaaacggctgccgccttcacggccgacggattcatgcgcaccggcgacatcgccgtcatgcaagaggacggctacagccggatcgtcgaccgcaagaaagacatgatcctggtcagcggcttcaatgtttttccgaacgagctggagaacgtgatctcgctgtgccccggtgtggtcgaatgcgccgccgtcggggtgccggacgaaaagcagggcgaggcgatcaaggtttttgtggtgcgcagggacccgacacttaccgaagacgccgtgctgcaatactgcaatggacaactcaccggttacaagcggcccaagcacatcgagttccgggattcgttgccgaagaccaatgtcgggaagatcctgcggcgggagttgcgccccagcgcgggcgcctgaatgagccaccaggctgcggccgggctgccggcgaacattgtcgtcttcgagcgcggctggctttcgtcgaacaacatcctgttcatcggggccgaggagaccgcgctggtcgacaccggctatgccacgcatgccgagcagacgctggcgctggtcgaatcgaccttgggaacacggctgctcgaccggattctgaatacgcacctgcacagcgaccactgcggcggcaatgccgccttgcagcaacgctacccgtcgcttcgaacggacattccaccaggcgaggcgacattggtggagcggtgggacgaagagcgcttgagcttccgtgcgacagggcagatctgcccgcggtttcagttctccggcttgctgcagccgggaaaggaatgcatcctgggcgacaggccgtggcaggtgcatagcgcgcccggccacgatcctcattcgatcatcctgttcgatccggtctcgcagacgctgatctcggcggacgccttgtgggaaaacgggtttggcattgcctttccggagcttgctggcgaaccgtcattcgacgacgtggcggccacgctggatcggatcgagacgctggcgccgctacaggtgatccctgggcacggccgcgtcttcgacgacgtcggcaacgccctggccacagctcgccgccggctcgaaggccttcagcgcgaccctgtgaagcatgcgcggcatgccatcaaggtgctgatgaagttcaagctgctggaagtgcagtccattgctctggacgattgggaagcctggcttcgcggcgcaacgtatctgggtgtgattcgctcgcgcttctttgccgatatggagttgcgtcaattgaccgacgacattctggtcgaattggtctacgcgggcgccgccgaaatggacgcgtcttgcgttcgtaatatctagctctgctgcggcaataaaaaaagcgcgtcacctgatgatgacgcgcttttttgaagcaccaaaagaaaaagcccaacacgctgtgttgggcttttccaggctgtaagagcctgacgatgacctactttcacacgggaacccgcactatcatcggcgctgacgcgtttcactgtcctgttcgggatgggaaggagtggtaccacgtcgctatggtcatcaggcataacttgttgtctgactgatcacgtgatcaatcaaacgaattcatagagtttggaatcagcacgcagtatctgcgctgtttgaatgtattttgaatgcgtcaacttggcataacaccttgatcggattgatcaaagttatagggtcaagccgcacgagcaattagtatcagttagcttaacgcattactgcgcttccacacctgacctatcaacgtcctggtcttgaacgactctttagggggctcaaggccccggcagatctcatcttgaaacgagtttcccgcttagatgctttcagcggttatctcttccacacttagctactcggcaatgccactggcgtgacaaccgatacaccagaggtgtgtccactccggtcctctcgtactaggagcaggcttcctcaaatctgcagcgcccacggaagatagggaccaaactgtctcacgacgttttaaacccagctcacgtacctctttaaatggcgaacagccatacccttgggaccggctacagccccaggatgagatgagccgacatcgaggtgccaaacaccgccgtcgatatgaactcttgggcggtatcagcctgttatccccagagtaccttttatccgttgagcgatggcccttccatacagaaccaccggatcactatgtcctgctttcgcatctgctcgacttgtcagtctcgcagttaagcacgcttatgccattgcactatcgtcacgatgtccgaccgtaactagcgtaccttcgaactcctccgttacgctttgggaggagaccgccccagtcaaactgcctaccatgcactgtccccgatccagataatggacctaggttagaacctcaaacacaccagggtggtatttcaacgttggctccacaagatctagcgaccctgcttcaaagcctcccacctatcctacacagatctgttcaaagtccaatacaaagctacagtaaaggttcatggggtctttccgtctttccgcggggagattgcatcatcacaaacatttcaacttcgctgagtctcaggaggagacagtgtggccatcgttacgccattcgtgcaggtcggaacttacccgacaaggaatttcgctaccttaggaccgttatagttacggccgccgtttactgggacttcaatcaagagcttgcaccccatcatttaatcttccagcaccgggcaggcgtcacaccctatacgtccactttcgtgtttgcagagtgctgtgtttttaataaacagtcgcagccaccgattttttgcaacccattcatgcttcgttgttcactacacactaatagggcacaccttcttccgaagttacggtgtcaatttgccgagttccttctcctgagttctctcaagcgccttagaatactcatctcgcgcaccagtgtcggtttgcggtacggtcgtatatagctgaagcttagtggcttttcctggaacctcgttcagtcacttcacggacaagtccgctcgatcgttggcctcggtatatgtgcaccggatttgcctaatgcacgcctacatccaactaaaccagaataatccaataactggatgacctattaagatccgtccccacatcgcactatatatcggtacaggaatattgacctgtttcccatcagctacgcatctctgcctcgccttaggggccgactcactctacgccgatgaacgttgcgtagaaaaccttgcgcttacggcgagggggcttttcaccccctttaacgctactcatgtcagcattcgcacttctgatacctccagcacgctttacaacgcaccttcacaggcttacagaacgctctcctaccacttgcaataaattgcaaatccgcagcttcggtaactggcttagccccgttacatcttccgcgcaggacgactcgatcagtgagctattacgctttctttaaatgatggctgcttctaagccaacatcctgactgttttagccttcccacttcgtttcccacttagccaattttagggaccttagctggcggtctgggttgtttccctcttgagtccggacgttagcacccggtgctctgtctcccaagctgtactcatcggtattcggagtttgccttggtttggtaagtcgccatgaccccctagccaaaacagtgctctacccccgatggtaatacttgaggcactacctaaatagttttcggagagaaccagctatttccaagtttgtttagcctttcacccctatccacagctcatccgctagttttgcaacactagtcggttcggacctccagtacctgttacggcaccttcatcctggccatggatagatcacttggtttcgggtctacacccagcgactgatcgccctattcggactcgatttctctacggcttccctattcggttaaccttgccactgaatgtaagtcgctgacccattatacaaaaggtacgcagtcaccccttacgaggctcctactttttgtaagcacgcggtttcaggatctatttcactcccctcccggggttcttttcgcctttccctcacggtactagttcactatcggtcgatgatgagtatttagccttggaggatggtccccccatattcagacaggatttctcgtgtcccgccctacttgtcgttagctcagtaccacacaggtcatttcacgtacggggctatcacccgctatggccagtctttccaaactgttccgttatgtcttgtgctatcactaacaggcttctccgatttcgctcgccactactttcggaatctcggttgatgtcttttcctcgagctactgagatgtttcagttcacccggttcgcctcgcatgactatgtattcatcatgcgatacctttcggtgggtttccccattcggaaatctccggatcaaagctaatttgccagctccccgaagcttatcgcaggctatcacgtccttcgtcgcctatcatcgccaaggcatccaccacgtgctcttattcacttgaccctataactttgacgtttctttcgaaactacaaaatcatcacaaggaatatgtcaggtctttcacctgacgcgttatgccgttacattcaaaattcgatttgactcgaaattgaagtttcttttgacgcaatcaaaaattctatgttgctgatggcacggtctgcactaaacctttacgaatgtgcagtttccatcagcaacgctgattcgactctatgaatttttaaagaacagccgattgatcaagagatctcgatcaacaacaaagaagcctcatgcctgagcaagaagccgctttggtgttgaatttaagtatcgatttattggtggaggatgacgggatcgaaccgacgaccccctgcttgcaaagcaggtgctctcccagctgagctaatcccccaaaactctcacacgagaaatcagaagatttggtgggtctagttgggctcgaaccaacgacccccgccttatcaagacggtgctctaaccagctgagctacagacccaatcgagaatcaatgaagatttcgacttcttccaacaaccgataagtgtgggcgtttaaattaaattgcttgtttccagaaaggaggtgatccagccgcaccttccgatacggctaccttgttacgacttcaccccagtcacgaaccctgccgtggtaatcgccctccttgcggttaggctaactacttctggcagaacccgctcccatggtgtgacgggcggtgtgtacaagacccgggaacgtattcaccgtgacattctgatccacgattactagcgattccgacttcacgcagtcgagttgcagactgcgatccggactacgactggttttatgggattagctccccctcgcgggttggcaaccctttgtaccagccattgtatgacgtgtgtagccccacctataagggccatgaggacttgacgtcatccccaccttcctccggtttgtcaccggcagtctcattagagtgcccaactaaatgtagcaactaatgacaagggttgcgctcgttgcgggacttaacccaacatctcacgacacgagctgacgacagccatgcagcacctgtgttacggttctctttcgagcactaagccatctctggcgaattccgtacatgtcaaaggtgggtaaggtttttcgcgttgcatcgaattaaaccacatcatccaccgcttgtgcgggtccccgtcaattcctttgagtttcaaccttgcggccgtactccccaggcggtcaacttcacgcgttagcttcgttactgagtcagtgaagacccaacaaccagttgacatcgtttagggcgtggactaccagggtatctaatcctgtttgctccccacgctttcgtgcatgagcgtcagtacaggtccaggggattgccttcgccatcggtgttcctccgcatatctacgcatttcactgctacacgcggaattccatccccctctaccgtactccagcaatgcagtcacagatgcagttcccaggttgagcccggggatttcacaactgtcttacattaccgcctgcgcacgctttacgcccagtaattccgattaacgcttgcaccctacgtattaccgcggctgctggcacgtagttagccggtgcttattcttacggtaccgtcattagccctctttattagaaagagccgtttcgttccgtacaaaagcagtttacaacccgaaggccttcatcctgcacgcggcatggctggatcaggctttcgcccattgtccaaaattccccactgctgcctcccgtaggagtctgggccgtgtctcagtcccagtgtggctggtcgtcctctcagaccagctacagatcgaaggcttggtgagcctttacctcaccaactacctaatctgccatcggccgctccattcgcgcaaggtcttgcgatcccctgctttcatccgtagatcgtatgcggtattagcacagctttcgctgcgttatcccccacgattgggcacgttccgatgtattactcacccgttcgccactcgccgccaggattgctcccgcgctgccgttcgacttgcatgtgtaaggcatgccgccagcgttcaatctgagccaggatcaaactctatagttcgatcttgatttttgcgccccatctcgcgatgaggcaaaactcataaaaaaagaattaaagtgaacttcacttctatctcatgagcgtttttaagtcttgcgacttgttccgaagaacttacgcaattaccttcaaacgcccacgcttatcggctgtaaatttttaacgaaccccgaagcaactttcgtctacttcgtcttgctttgctgcgatcagcgaagccttgtagtctatcacggttttttaagtaccgtcaaacttttttcgctttcaacatcttcttttcgcaccccgcaaccttcgctgcgagacgctgaagctgtttcagcggagccttcgattatgcactgttttttcaaaccgcgtcaacttcgaaggaagttttttcgactttcatcttcttgctgcagcccctttggggctactgcttgaagcgccttgagagcgttgtcagccgagcccacgagtatatgccaaatcctgggcactgcaagactgcagagaacaaaatcaacgtcggagcctttgcatccgggggcagcgcttcgcgctgcccccggatgcaaaggagcctcctccgataatcggagccacatggcactcatcacactcctcgacgcccaactcgcgttcggtcacgtcccgctgctcgatcatgcggacttctctcttcttgaatcggaacgcattggcctgatcggtcgcaatggcgctggcaagtcttcgctgctcaagatactggggagtctggagaagacagacgacggcaccctgcagatgcagcagaacctgcgggtggcctatgttgcgcaagagcctgtgctcgatatggatgcggatgtattcaccgcagccagcgaaggcctgggaagcgtcattgccgtgcgggacctttatctctccggtgcggaggggctggatctggacgcccttcaatcgcagatcgaagctttcgatgcctggaactgggagcagcgcgtcgaagagacgctgcatcgcctccacctggaccgcaatgcccgcgtcggctctctctctggcggtacccgcaagcgtgtggcgctggcccaggccctggtggccgcccccgacgtccttctattagacgagcccaccaatcacctggacctggattccatcgaatggctggagcagctgctgatcgacttcaaggggagcgtggtcactgtcacccatgaccgcagcttcttgaatcgcgtcgccacccgtatcgtggagctggaccgcggcaagctgggttcctaccccggcaacttcgagcagtacctcttgcagaaggaagagcagctcgcccaggaagccgtcatcagcgccaaggccgacaagctccttgcccaggaagaaatctggattcgcaagggcgtggaagcgcgccgcacgcgcagccagagccgcatcagccggctcgaaaccctgcgggcgagccgcacggcgcgccgggaagtgcaaggcagcgtcaacatggacgtggcttcgggccagtcgagcggcaagatcgtggccgaactggcgggcgccaccaagtccttcggcgaaaagaccgtcatccgcaacttcactgggaccatcctgcgcggcgacaaggtcggcctgctgggccccaacggtgcgggcaagaccacgctgctcaagctcatcctgggcgaactcgaaccggacagcggcaagatccgccgcggcaccaacctgcaggtggcgtatttcgaccagatgcgcgacaagctcgacctggacgccacgctggaagacttcatcagccccggtagcgaatggatcgagatcggcagccagcgcaagcacgtgaagagctatctctccgactttctcttttcccccgcgcgcgccaattctccggtgcgctcgctcagcggcggcgaacgcaaccggctgctgctggcccgcctgttcgcccgtccggccaacgtgctggtgctggacgaaccgaccaacgacctggatatcgacaccctcgagctgctggaaggcctgctgcaggactacgacggaacggttttcctggtcagccacgaccggaccttcctggacaacgtggtgaccagcacgatcgcgttcgaaggcgatggccattggcgcgaatatgaaggcagcgtgcaggactggctgatccagtcgaagcgcgcgcgcgagatcgcggaacaacggcaagccgccagccctcccccgtcgccagcgccggctccgacacctgccgcggccgaacccgcagccgccgcccgtcccgcggccgcgcgcaagaagctcagctacaaggaacagcgcgagctcgaggcgcttccggcgcagatcgaggcactggaagccgagcagaagcgcatcaccgaaatgctcgagctcgacggcggggcgatctatgccaccgacgcctcacgcgcggccgaactgagccagcgccacgcccagatcgacgacgaattgctggccgcgctggagcgccaggaggaattgtccgccgggcgttagtgcattagttctgcagcggactctcccgccgtcccacgtgcggacagcgccgactaggctatatatgcggcttcaaagctccgggaacgccgcatgccttccatctacgcgctcttcggccggtccgttgcactcctggccattgttctgcagggcgcttgcgcgcaattgcccgagcaggtcgaccgcccggtatcggtcgcaattccgtcgcccaacggcaccgccctggaggccttggtccagcagcgccgcaaggccgatggggcgcgattcgaatccggcttcctgctgctcggcgggcctcccgccgcctacggcagccggctcgcattgatcgaaggcgcccagaagacgctggacctgcagtactacgcgatccacgccgacgccagtaccggccggctgttgcgggggatccgggcggcggccgggcgcggcgtgcgcgtgcggatcctgctcgacgattttcacagcaccggccgcgatgcgctggtgctgggcctcgcgttcgtacccaacatcgagatgcgcctgttcaacccgcttgccggcgcgcgtgggtcttcgttggcacgactcttcaactcgatcggcgatgcctcgcggatccagcagcggatgcacaacaagctcttcctcgccgacaacgtgctgggcgtgaccggcggccgcaacctgggcgacgcctacttcggcaatgcgctgaagggcaatttcatcgatctggacatcctggcggccggcccgatcgtgcaggacctgtcgcgcagtttcgacagctactggaacaacgagcgcgcctaccccgtgcagtcgctggtcaagcgcgaagagctgcaggccatccgcgaacgtgcggaacgggtcgaccgggaactggccgatgaatcggcccggtccttgaacgcgccaccaccgacaccccagacgccgacgcccacggaaggcgaccccaagcccggcgccgccccaacggcggcgcagttgacccgggcatgggacgaaaagcccctggatctgcgcaccgcccgcttcgtctgggcgcccgcggtgatgctcgccgaccagcccggcaagattcccgccgacaaggggccgaaccaggagaaggcaccgggcctggtggtgagccaacccaacgacagggccaacccgtcacgccgggccgcatcgctcgaggccagctccgacctcgccgccggcagcgacacggtggtggaaggcctgttgcaactgatcggacaggcgaacagcgacctgctcgtcatctcgccctatttcgtgcccggcccggacatgaagcaagcctttgcggcggcccggggccggggggttcgcatccgcgtgctgaccaactcgctggcgtcgaacgacgcgccggtggcgcatgtcggctattcgcgccaccgccaggatctgctcaagatcggcgtcgaactctacgaactgcgcagcgaacaggccagtgtcagcaacgccttcggctcatcgggcgacggcagcatcggcgcatcgcgctccatgctgcactcgaaggtgctggtgatggacggccggctgctggtggtcggctcgatgaacctcgacctgcgttcgcaactgcagaacaccgaaatcgccctgctcgtgcgaagcgccgaactctcccgctcggcgtccgagcagatcgagcgcggcatgcgcgaaggctcgtggcgcgtcgagctgaacgacggctcgctggtctggcgagcgcccgaaggcagcggcttgaaagacacctccacggagcccgacgccagcctgaccctgcgcctgatgctcaagctgttcggcccgctggcgccggaccagctgctgtagcgcgcgagaggccgaatcccgctgcttgggggcggcaggtcagtgcttgtgctgatgggcagccggcgcggccgcgtcggctccttccggcgcgcccaccggcagcttcaggtcgagcgaggttttctggcccttcgcgtcctcgaaccggagcgtcatcggcacggtcgaacccttggccagcgcctgcttcaggtccatcatcatcacgtggtagccacccggcttgagctcgacggtctggcccgcgggcaactccaacccggccggcaactcgcgcatcttcatggtgtcgccttccatcttcatctcgtgcacttcggccacgccggcggccggcgtcgagatgccgaccagcttggtgccggtgggtgcggtgagcttcatgaaggcgccggtgccgctctggcccgggaccgactggcgcacccaggcatcgcgcacgtcgaccgtggccacgccctgcgccaccacgtcgagcctggcggcaggggtcttgagccccgcagtcgaggtgcccgacgccggcacctcggcccagtcgatgcggcccacgtcgcaggtctgcagcaccttgaaccacagcggccccggcgtgccgggcaccttgccgcgcaacacgaattcggcgcgttcgctggcaggcagcgccgtttgcgggctttccgcggtccagcgaacttcgccgtcgccggcattcttctgcacgtcgagcttccagcccttgcgcgcctgcgcgtcgctcaggatgaagcccttgggcaggcgaacggccaggccggtggtggccttggcgccttcgcaggcatggcccacgcggaaggcggcgtcgtagtcactgccgacggtgacgccgccgcgcggcagggtgacgtgggcgaacgcggttgcggtgcccgccagcatggcgcatgcggcaacggtcttgagggtgatgcgcgggtggttcatctggaactccttggagaaagcggtgaaaagagagaaagaaggtcagaggtcgaacttgagttcggccacgtaggtgcgttgcgtgtagggatggaaggcccagtacttgttgttgttcaggttgtcgatgcccacggccgcgctccattgccggtcgatgcgatagcgtatgcgcgcatcgaccacgaagaacttcgaaaagcccatatacgcggcgccgttcgtgtcgctgttgtccagcgtgccgtattgcttgccgctgtagcgtgcgccgaccgtgtagctccatctggcgtccggccgataggtggcgagcagcgtggcccgcaccttgggcacgcgcggctgttcgtggcccacgctggcgggaaagccgctgttggcggcgatcttcgatcgcgtcagcgtgaggctgccgctcaagtccaaccccttcgcgcccacatcgaccgcgttcaacgccacctccagcccccgcgtgcggatggcatcgacgttctgcaccgtgctcgccaggttggtgagtgcctggctgtagagcgcgtccttggtgttttcgaagaagagcgtggtgcggaggacgccgtcgagcccccatgttttcagatcgcgctcggcgctgagttccgtggtccacgaacgctccggccgcaaattcggattcgtgttgacgatgcggctgccgtcgatcgagccctggtagagctcgctcacggtcggcatgcgcaccgcgcggccggtcgaggccttgaacaaccaatcctgcgtagcctgccaggcgatggcggccttcggcgagtcgtagctgttcttgcgcggcgcaaaatccagcagcctggtcgcgttgccgagctggccgccataggcttcccatcgctcgtggcgcaggcccagcgtggtcttccagttcctggcaaaacgccaggtgtcctgcacgtagagcgactggagccgcgtgttgccattgaaggcggagaacggcgtcacggccggtccgccgatccaatcgagcgtgttgccgacgctggtgcgcaggcgcgccgtgtcctgctggaaaccgaagtcgaccacgtgtgcgcccacgccctcggccgagccggtgggccgccacgtgcctgccgccttgaaggtgtgccagcccgagccgctcatgtcggtggtgcgcccggggccgccgttgaaggcgccgggcaagggcgtggtcggcgtgcgcgaggtgtctctcgaatagtcgaacaggctcgcggccacctcccagtcgaacacgccgccggtgtggctcttcaccgagaggccatgcatatagtgcgtgagcgccgtctccgtcggcgccagcgcggcgctcggcgaatccaggttgtaggtgcgcccggcgatattcacccgccccgaatacacgggccggccgaggccgtcgcgcaggtaggtgtcgacgctgccatgcgtggtgttgttccaggcgcccagcgtgtaggtggcgcgaacggtggacgaaaagtcgtaggccaccttcagcttggcctgctcctgcgtggtgtcgtagatggtggagccgcccaccagccaccagggttggttcgacgggttcagccccagcaccgcaccggtgaccggcgtgcccgcattgcccaaggtgccgacgctcaccagccggttgccgaacaccagcgcctgccccttgctgtgggtgcgcgaggcactgagccaccatgaccagtcgccgctgcggctgcccagtgacaggtcgagctgctggcccgcgggcgacgagtggctgttgtacaggtcgaagttcgaggcaaagccgctgagcttgacgtgcgcttcgagcttggtgggcatgcgcgtcacgtagtcgaccacggcgccgaccgagttgcccgggtaggcggccgaaaacggaccgtagagcacgtcgacccgttcgatttcttcgggcgacaccatgccccagcgcggcgcgtaggtggcgccgttgcccagcgggttcgacagcatgatgccgtcggcgtacaccatcgagcgggcactgttgcccgtgcccgaggcgcgcgtggcaagcacggcgtggttgaaatcgccgatgtagcgcttgcgcaccacaaggctcggcaggtacttgagcgcgtcttcgctgtcggtcgcattgaccgtttcgacgatctgctcgtgcgtcacgccctcgatggtggtcgggatctgcgtcggcagcgaggtcgggcggccgtcactgacggtgacggtgctcaaggtgcgcgggccgccgccgtcctccgacgggtcaggcgcgttttgcgcccacacgggcgcgccaaggggaaatgccatggcgatcgccaaggcgcgggaatgctttttcattgggaacctgctccacgaacttcaagccggacaggccgcagcgcccctcggatcggggcacgtgcggctacggttttggcagtttcaggagaaggccgggggtccgcgcgcaggcagcggcgcggcggtggccgcggcaagtcgcgcggcgggaatcgactggagcacgcggcccagcggcaagggcagatcgaaggccgcggcggccggcgacggaggcggtgcgccggtcagcaggcacagcggacagtccatgtgcgaggcgcccacttcctgcacgccgtcatcggtctgcaccaccgccttgatcgaaccggcgctcgagcacaccagttccatggcctgcggatgcacgatgggcgatgccaccgccacgccaagcgagagcatgaaccacagcagcgcccatcggccgacgaggccgaggaagcgggggtggtttcgcagcaggtgcatggcaaatgagattatcggcgctgtttgctcttgggtgtcggcgtcgtgctgcgctgcgccggcttggcattgcccgccgtcctggcaccgctccttgcggtggaacccttggcattgcggccgccccgcgcggccgccttgggcgcaggcgccgtcggcaccgcgaccggcggctgcgcggcgagcggcaccgccgagacggtgaatccacgcgccgccagcagcgcgggcagtccctccggcccgaccatgtgcaaggcacccacggcggcaaagacgcgcttgccgcccgcgtgcatgcgttcgatgccgtccgccagccccggattgcggtcgtcgagcaggcgcttcatcagccgccgctcggccggcgtgttgaggcagttgcaccactcggggtagcgggcgagcttgtcggcgtcgccgcgggcccagacgtcggccagctctttcatctgcgtgcgcagctggcccgactccagttcgtcgagggcggcgtcgatctgctccgcctcctcggcttcggaatcgccggtcagcatcttcagttgcgccgcagcactttccagcgcgaacaccggcttgccgttgttgcgcgcggagacggccagcgcctcgtccgcgccgaactccggatacaggccgtcgacgcgggccaccaggccggtcagcgccatcacctgcaggatgggttgcagcccggccgtggtctcgggcgacacgcaggccgcctctctctggcgggccaggcgctgcgcgcgctcgccgctgagcaaccgcgccaccacggccggatccgccggctgggtcagggcgcgcatcgcggcctggtcgcgcgtgtcgagttcgagcgccagcgcgtcgctctgctccagcgccttctgcacggtgggaccgggccgtacccattcggcgcggccgagatgaatggttccatagagccaggcggtccggccgtccctttcggcgcgccacagcaggccgcgatcggcggcgttccattggcccactgccgcacccggctttccaagactggcaatggccgacggcgggcaggcggcatgcgctgccagggcaaaaacagaacagacgccggccagcgcaaggcgcggcaggcgtgaaaaaagcgaggggcgcataggcgccttcaaatcgatattgcgccacggcgcaatcagggcccggagtatccgcaaggcttgctccacgatgaaagaaagtccggcattctcacagcaccgctgcccataatccggaaccatgcagagcatcttccatcttgcctttcacgtccgcgatctcgacgtggcccgccgcttctatggcggcgtcctcggctgcgccgaaggccgcagtaccgatacctgggtcgatttcgacttcttcggccaccagatctcgctgcatctgggcgaaccgttcgccaccacgcgcaccggccgggtcggcgacgcaatggtgcccatgcctcatttcggcatcgtgctcgcactccctgactgggaagcactcgcccagcggctgaaggctgccaacacggacttcgtgcttgccccgcaagtgcgcttcgaaggccagccgggcgagcaatggaccatgttcttctgcgaccctttcggcaaccccatcgaggtcaagggctttcgctcccttgcggcgatctacgacaaatgaaccctctgcgccgggccgcctccagccggctcgcagcttctgcgcgagctcgcgtcgtcgtgcctcgcattgcaactgccgcgctctgttttcttgcggccggcgttgctcacgccgcgctcgactgcgagctcaacggccgcagcgtcaatccgacagacgccagcagcgtcgggggcaagacggggctcatgcgctgcaaggaacgcggcaccggcgaactccagcgcgagcagcaactgcagaacggcgtcttcatgggcttggcccgcttttatgaaaaaggcaagctggccaaggagcacacgctcaatgccaagggcaacatccacggcctcgcacgtgagttcgcgcccaacgggcaggtcgtgcgcgaggccgtctacgacgacggccgcgagcgcgggctggtgcgcagcttctaccccggcggccggctgcgccgcgtcaccttctatcccgatgtcggaaccgaccgtgccttcgtcgagttcaccgagcgcggccagatgtcggcgctgcgctgcggcgaaaagccgatgctcgcgccggtggcagacgacgcggggctgtgcgggttcactggcgggccttcgcaagtcgagcttttcgacgagcgcggcatcctgcgctcgcggctctcgtacctggcgggcaagcgcgtgcggtcgcagaacttctacgacaacggcaagccctcggtgcaggacgagatcgtcggcaaccagcgcaccgagcgccagttttcatccgagggcgtgaagcgccgcgaaacggtgtggcggctggtcgagcgcactgcggtgcggcaacgcgagcaggagttctccgaaaagggcgcgctcatccgcgaccagcgctggaaccccgcgggcgaacccatcagcgacgacagctatcacctcaacggccagcttcgcagcaagtccgtctaccgcggttcgggcgattcgcgcacggtcgagatcaccgagttttacgacagcggccagcgcgccgcctatggccgcttcctggtcgtgggccgcggccggcaaatgcccattggcaagcaccagcgcttcagcgagaaaggaacgctgctggccgagtcgatcttcgataccaagggccgcgtaacccgcgagcgcagctgggacgagaacggtgtgctggagcgcgacgaccaggtcttcgacgagaagaaatagctcgccgctccccggcctcgcgcaacttcagtccagcttgacgccggcctgcttgatgatggggccccagcgctgcgactcggcgcgcgacagcgccgcgaactgggccggcgtgccgggcattgcttccatgccgaaatcgtcgaagcgcttctgcacggccggcgtgccgaaagcgcggttcaggtcggcgttgagcttggttaccaccgcaggcgggaggccggccgggccgagcacgccctggaacgcgaacacctcggtattgggtacccccacttccgccagcgtgggcacgttgggcagcagcttgctgcgggcgcccgagccgatggcgagcacgcggaccttgttggcctgcatgatcgacaggcccgaggccaggtcgaggaacatgcacggcacctggccgcccatgacgtcggccatcgcgggcgccgcgcctcggtacggaatgtgggtgatgaaggtgccggtgcgcaccttgaacatttccatggccaggtgatgcggcgagccgttgcccggcgaggcatagttgaccttgccgggattggccttcacgtaggccaggaactccttgaagttcttggccgggaaatccgggtggaccaccagcgcgagcggaaacttgccgatggcgccgatgtaggtgaagtctttctcggggttgaacggcagcttgccgaacaggtgctcgttgaaggccagcacggcgttgtcggccgacatcacggtgtagccgtcgggcttgctcttggcgaccaggtcggcgccgatgttggtggaagcgccgggccggttgtccacgacgatctgctggcccagcgtctggcgcatggcctcggccagcgtgcgcgcgatcacgtcggtgccgccgcccgcgggatacggcaccacccacttgatgatctgcgagggatagtcctgcgcgcgtgcgaagggcgtggcggccacggcggcgcccgaagcgagcgtggcaagaagtgtgcggcggtccatgtcgatcagtctccggtttgtagtatttctgctgcggacagcgatggtacgggcagcgcatgcagcgcgtcggccagagcgcggcggcagcgcgcctcgtcgccgacctgctcgaaaagcagcagcgcgagccgcgcgaggaacagcgattcgcgctctgcgccggcttcgctgatggcgcgcgcgcactcggcatacagacggtctcgcgcgtcggggtgaagcgatgtcgtcatgcggcaatctccttggtcgcaacggcggcgcgcgccagcgcatccgacaacgcgccacgcggcagaaggcgctgccagcgcgcggccacgtgtccatccgggcgcagcagatagacggccccatcggttgcgcccagcgcctcgaacacagacgggccggcatgcgcatccgcaccctcgacgcccgggcttgcaatggtgcgaaccgcgaatggcagggcgccgccgcacgcttgcgccacctcgccgtccggcagcgggacggcatcggctccgggctgcagcaccagcaacgtaaagaccgggccgatccagtcgctcaggtggccgcgctcgagctgctgctcggccacgacctcgccgggcagcggccccgacggcagtgcatcgccttcgctggacagcgccgaatcctcgtagcgcacggcctgcgtctggcggggattgatcagttgcgcaatgccgcgatgcgattccgacaacgaaagcgcggcctcgcgcagcagatcgaagccacgcgaaggcggcgacatgaactcggtgctgcgcatcgcgttctcggcattcacgtgaaaggccgcgatgcgctcttgcgagtacgaatcgagcagcgccgcatccgacaggccgcgcgccacgaaggccagcttccaggccaggttgtccgcatcgtcgaagcccgaattgaggccgcgcacgccgaagatcggcatcgcgtgggccgcattgccggcgaagagaacgcggccatgccggtaactcccgagcgtcatcgcgcccgcgcggtagaccgaggtccacaccgtcttccagggcaggtggccttcgccgatggcgtcgagatggcgctgcacgaactcggccaccgcggccggctgcagcgcttcctcggtgctttggccggcgcgcaactggtagtcgatgcgccagatgtcgtcgggctggcggtgcatcagcacggtcgagccggggttccacggcggatcgaaccacgcgcggcgctcggtcgggtgcgtgctgtgcagctcgatgtcgatgatcacgtagcggccttcgtagcccgtgccctcgagcgcgagccccagcgccttgcgcacgaagctctggccgccgtcgcaggccgcgagccactggccctgcagccgataggcgccctcggggttgcgcacgtcgagcgtcacgccgtcttcatcctgcacgatgccggtgagttcggtaccccagcggatgtcgatgagccccggcgccttttcgttgcggcggaagatctcttccagcaggtactgctcgatgtagtactgctcgaggttgatcatcggcggcagcttctggcgctcatcgtgcggcatctcgaaccgaaaaacctcggacgtcttgtagaagctgcgaccgccggtccacggcagccccttggccatgaaggccggcagcacgtccagccgttccatgatctcgaggctgcggcgcgagatgcaggccgcgcggctgcccacgcacaccgtgtcgtcggcttcgagcaccacgcagcgcacgccgtggtttgcgagccccagcgcgagcgccatcccgacgggtccgccgcccgcgatcaccacggggtggcggccgggctccacgccgtcgtgctccagcggcggcgtccacggcttgtagcgcgtgtactgaaaggcgccgacggagggcggcagttcgctggcgctggccattggcggcacggggcctgtcgcggcatcggcggcgcgcgtgccgggtgccgccgcggcgaccgcaatggtgaggttcgtcatgcagcgggattgtcccgatgtgcggtgccggccactgtcataacttcgtacgaagtaattacccttggcttatctgctcccatgagacgctggcgcattcaacccaccgcgggcaccgtgttgtccgcggccatcgtcggcgacgtgctggcaggtgtcgccacgccgcatctggcggccagctgcctcgcggccatgcaccgcgtgatgcccgtgaccttctgcaccgtgttcgcggtcgatgccaccggccgcatcgaggcggtgtcggccgccagcagctacggcaccacggccgaacgcacgaccgagcgctacgtggcgcagcgcttcgacctgctcgatcccaacatgacatggctcgcatcgcgcaagctgcccaagcgctcgcaactctggctgggccaccagcgcgccgacgaagtggccgaccccgcctaccgggccgcctgctatggggacgtgggcatccgggaacgtgcgtcggtgctgctgttgacgccggccggccaacgcgtggccgtgagcttctaccgcagcctcgcgcagcccgaattcgatgccgccgaattcgcggcgatcgaaggccatgccacgctgctggccgatgccaccctggcccatggccgcagcgcggtgggcacgcgcgaagcggtggcgcccgccctcgcctcgggcctcttgaccctgagcctgcgcgaacgcgaggtcatcggccacctgctggccggcaagaccgccaagcaggtggcgcgcgacgtgggcatcgagctaaccacggtgcgcacccaccagtaccgggcgttccgccggctcggaatacgcacgcagaaggaactgctgctgcgcgtgacacaggaagcgccgtagcgcttcgccttacttggcagcgtccaggcgcttctgcatgcgggccgaacgctcggccgatggcggatgcgagctcatgagcgagctgccggtggcgccgccactgagcttggccagcttgtcgaacgcgctgaccagccccttgcgctcgagcttgcgttcggtgagcaggtcgaaggaatagttgtcggccgcgctttcgttcgcttgcgagaactgcgcgttgacgaacttttcgcccaggtcgccggcttgcgactgcgacagctgggccaccacgccgccggcggcgccggccagaccgcgaacagccgaggcggcgtaggccgtctgcatgcgcgacttggaatggcccagcgccacgtggccgatctcgtggccgatgacgccgcgcagctcgtcgtcgttcatcaggtccatgaggccgctgtacacgcggatgcagccattggccatggcccaggcattcacgtccttggtcacgtagaccttgtagttggcggtcttgccgttcacggtggtgggcatctgcttgatgacctggttcaggcgcgtggcgtagcggctgctggccggcgcgatctggttcttctggtccatggcggcgcacgactggtcggacatcgtggcgatctcgccgtcgctcagcgacatggccttgaaggccgagccgcctgcctgggtgagtgcgccggtgtcggcgttcttcatggtttcgcagccgacgagggcggagaccgcaacgacggcggcggcaataggcaaataacgcattgaaaactcccgtttttcttgatttgaatggcgactgcggaagcagccgccgaacgcactgccgctcgcgaatgattccgagtcgcggcagcgggaggatcatagccatggcgggcgcgatgcccgcgaagcgcggaggcttcagtcttcgccggcgtcctcggccggtgccttcaccagcgacaccggcgccaccttcggccgcccgctcgtcgacacgatctcctggtcgatcgcgccgaacagcgaacggccgtccaggcccttcatctcgatgcggatcgtgtcgccgaacttcatgaattcagtgaccggctcgccgccctggatggtctcgatgcagcgcttctcggcaatgcacgagtagcccttgggccagtccatctggccgttcctttccacgcccttgttgctcacggtgccgctgccgacgatgctgccggcacgcacgttgcgcgtcttggcgatgtgggcaatgagctggccgaagtgaaaggtcatctcgggcccggcgtcgcacatgccgaccttgcggccgttccagctgctttgcagcgtaaggtggacgcggccgtcctgccaggcttcgccgatctcgtcgagcgtcacggccacggggctgaaggcggtggccggcttgctctggaagaagccgaagcccttggccagttcggccggaatcaggttgcgcaggctcacgtcgttggccagcatcaccaggcggatgccgtccagcgcctggtcgggcgtggcgcccatcttcacgtcgccggtgatcaccgcgatctcggcctcgaagtcgatgcccatggcttcactgggcacgaccacgtcgtcggtcgggccgagaaagtcgtcgctgccgccctggtacatcagcgggtcggtgtagaagctctcgggcacctcggcgttgcgcgccttgcgcaccagctcgacgtggttcaggtaggccgagccgtcggcccactggtaggcgcgcggcaggggcgccatgcacatcgaggggtcgaacgggaaggaatggcgcgcgcggcccgtgttgacggcgtcgtacaggtcctgcagctgcgggcccatgaagccccagtcgtccagcacctgctgcagccggctcgcgatgccggtggcgtagtgggcgagcgtgaggtcgcgcgagacgacgacgagctggccgtcgcgcgagccgtccttcagggtggcgagtttcatgatggcaaatgcgtgagaaaggacacggcgcgaaaacgagagccggcgccgcgcccactaaactggttgaacgggcggcagtgtaccgaggtgctcttggtgaacctccgcgctggcgcccactccaccaccccatgccgacgctcgtcgcccctctgccgccgtccaccgtccctctcggccgcccctcgtggcgggtgctggccgggctgacgctggcggtggcgctggttcatgtgctgctgctggggctggcgccggccgccatgggacctgagccctcgccgctcgcgaacaagttcactacccggaccatcgtgatcgcgccgccggctgcggaaatgccggctgcgcctgctgccgcggcgcccgccgcccaagccaagccaccgccgcccgcaaaaccgcggcgaccgcgcgagccgtccccgcccaagccggcaccggcaccggcaccggcgccccaggtttcggaacagaacccgccgcaaacgcccgatctcatggcacagaacgctgccgattcaggggcaaccgcccctgaaccggcggcaagcgctccggcaggcgctgcactgggcggcgcaggcagcacggccaacaccggcatggagaacggcacgcccggcgagtccgcgggcgccgcttccgccacggcgggcaacgtcgtgggagctgaagcactgcgcattccgggttccgtgaaattggccttcgcggtcaccggccagcagggcgcctcgccgatgcagggcgttttcggcgacctggtctggctgcaggacggcagcagctacgacgcccggctgtcgctcaaattcctgttcaagaccattcgcagccagcacagcaccggccagatcggggccaccggcatcgaaccggcgcgcttctccgagagccgcaagggcgaggtggcctcgcacttcctgcgcgaccagggacaggtgatgttcagtaacaacgcgccgagcgtgccgctgcttccgggcgcgcaagaccggctcagcgtggtgatgcagctgggcggcatgctggccggcgatccggcccgctatccggccggcagccgcatttccgtccagacagtcgggccgcgcgaagcgggggtgtgggtgttcaacatcgaaggcgaagagcagatgacggtgccggccggtgattacgcggtgcgcaagctcacccgcaacccgcggcgcgagttcgacgacaaggtcgaaatctggctcgcgccggcaatggggtacctaccggtacggatgaaactgacacagcccaacggcgatttcgccgacatgcagttgcgcgaaacccttcccgcgggcccggccagctgagcgtacaaatcgagtaaagaaataccgttgtgactgcaatgcgacaacccttcttgaatctggcgcgttgattgctatctaagccacatgaacgctatcgacatactcacaggccccgcaatgaacatgctctatgactcggagtccttcgtcgtcgtgcacgtgcagccgaacgaaagtgatacaccggcgcaacccaatgtgccggttctggaacgccacggcttcgaaatcgtcgacaagcgctccggcaaggaggtctacctcgacggttcctgggccgaactgttccagcagcagattgccgcctggcagctcaacacgcccacgcaggaagaggtcgaagacacgctcgagggctatgccgagctggcccacacgcccgtgctcgtgcactgaaatacgccccgccgactgcaaaaagcgcccaatgggcgctttttttgcgtctttttcaggcccagccgttcatttgtgcccgtagatccaccggtacatcggccctaccagcagcagcaccgccaccagccggcacacctgaaaagccgtcaccaccggcacgccgagctgaagcaccttggcggtgatcgacatttccgcaatgccgccgggcgaggtggccaggatcatcgtggcgggatgcaggtccgtggcccacgccagcagccaggcggcgcctgcgcacagcaccagcatggcggcggtgcccagcgccaccgaccccagccagcgcggcgccgtgtgcagaaactcgcggctgaagcgcacgcccaggctcacggcaatcacgagctgcgcggcgttcgacatccaggtgggcacggccgaaagcggctggcccgcaatggtgaagcccatcgccaccaccagtggtcccatgaaccaggggttggtgcggcccagcgcccgcatcgcgaggccgccgatgcccgtggccagcgccagcagcaggagcccggccgcattcacctcgcgcaccatgggcgggttgatttcgagcccgtgcaggccgctccactgcatggcgaacgggatcgcgatggtcaccaccaccaggcgcaggctgtgcgccgcggccaccagatcggtgcgtgcaccggccgattcggacagcagcgtcatctccgacgcaccgccaatggcaccggcaaagtaagtcgtcgctctcatggagcgtgccggcacatgcggcatgcgcctggcgtgcagcccgtgcagccagcgcccgaagccccagccgagcagcaaggcccaggcaatggcaagcgcaatggcccaccagacgccggccaccagcgcaaccacctgcggcgtgaagtagaggcccagcgcggtgccgatggtccactggcccgcattgcgcagcggcgtgaagctggcggtgggcgcacctgcgatcgaggccagcgaaaccgcaagcagcgggccgatcatccatggcagcggcgtgcgcagggcgaggcaaagctccgccgcggcgagtgccagcaacagcgtggccagcacgcgaaccaaaaaacggaaagacaccacaggaaaaagcggaaatggacggcacggcgtgcgagcgccaacgcatagtatggcgcgatgcgatgccaaccctcccccgcgcaggccgcccgtttgccgttgttgcccctgttcgcggtcgttgccgcagccattgccattgcgtcgctggcgggttgctccgccttcttcgacggccccaatgcgccggtggcgcgccgcgccgcggcgttgctgcccgcggacgcactgatcctcggcgagcagcacgacgccgccgagcaccacgcgatcgaacgcgaaaccgtcgaagcgctggcaggccagggcaagctggccgcgctgctgctcgaaatggccgaggaaggcaacagcaccgcccgcctcgacaccgcagccaccgatgcgcaggcgcaggccgcgctcggctggaacgacaaggcctggccctggcaaagctacggtccggtggtgatggccgcggtgcgcgccggcgtaccggtcatcggagccaacctgccacgcgcgcgaatgaagaacgccatggccgacgtctcgctcgacgtgcaactcaacggcgaggcctacaccgcgcagcaggacgccgtgcgggagggccactgcaagctcttgcccgagccccagatcgtgccgatgacgcgcatccaggtggggcgcgaccgcgccatggcgcaagccatcgtcaaggcgcgccagccgggcaagacggtgctgctgatcagcggcgcgggccacgccaccaaggtgctgggcgtgccgcagcacctgcccacggatgtgtccgtgaaagccgtacggctgcaggccggcgaatcaccggacgatgaagaagaaaacaagggcgcctacgacgccgtctggcgcacgcccccgctgccgccgaaggactactgcgcgagcatgcgcaccaaatagcctcctgcgcagcggctcaggcgagcttcttgatcgaatccgccagcgtgttgaccagcgtgtcgatgtgctgcttctccacgatgtagggcggcgcaatcaccagcacgtcgcccgcgggccgcaccagcgcgcccttgtggaagcaatccagaaagatgtcgtaggcgcgcttgcccggcgtgcccgcaatgggcgcgagctccaccgccgcggcaaggcccaggctgcgaatgctgatcacgttcggcaggcccttgaaggtactgtggaaggcatcgcccagcaccttgcccatttcgcccgcgcgagcgaacaggttctcctgcttgaaaaggtcgagcgtggcaatggccgcggcgcaggccaccgggtggcccgaataggtgtagccatggaagaactcgaccacgtgctcgggcgcgtcggtcttcatcatcgcgtcgtacagcttgtcgcggcagatcacgccgccgagcggaatcacgccgttggtcacgcacttggcaaagttcagcatgtcgggcaccacgccgtagtagtccgatgcaaagttggtgcccatgcggccgaaaccggtaatgacctcgtcgaagatcaacaggatgccgtgcttgtcgcagatggcgcgcagcttctgcaggtagcccttgggcggcaggtaccagccggccgaaccggccaccggctcgacgatgatcgcggcgatgttgctcgggtcgtgcagcggcaggatgcgggtctcgagctcgaccagcgggtcttcggcccacaccggctcctcgttgtggacgtaggcgtggttcaccggatcgtggatgaagcgcatgtggtccacgcgcggcaaaaaggccgagccgaacaccttgcggttgcccggaatgccgcccaccgacatgccgccgaagcccaccccgtggtagcccttctcgcgcccgatgaacacgttgcgatggccctccccgcgtgcgcggtggtaggccagcgccaccttcatcgaggtgtcggccgcttccgaacccgaattgcagaacagcaccttgttgaggtcgcccggcgccatcgacgcgatcatctccgccgccttgaacgccttgtcgttgctgacctggaaggcggtggcgtagtcgagcgtgtcgagctgcttcttgatcgcctcgttgatcggcttgcggttgtggcccgcccccacgcaccagagcgacgagatgccgtcgatcaccttcttgccgtcgtgcgtggtgaactccatgccgtcggccgccacgaagacgcgcgggtctttctggaagtggcggttgggggtgaagggcaaccactggttgcccatgttgaagtcctgataagccatgatttctcctgcttaacgcgcaccaaaaaacggcattctggcacccctgcgacaatcatgcccctgatgacgaccactacgcccgcctacatcctgaccctctcctgccccgaccggacgggcatcgtgcatgccgtttcgggtttcctgctcgaacgcggcggcaacatcgaggaagccgcccagtacaacgaccacgacaccggcctgttcttcatgcgcgtgcgcttcgcctgcagcgaccacccggaggcggcgctgcgcgagcagctcgccacctttggcgccggcttcggcatgagcctgcaactgcacgcggcggccgaaccgatgaagaccgtgatcctggtcagcaaggaaggccactgcctcaacgacctgctgttccgctggaagagcggcctgctcgccatcgacgtgcgcgccatcatctcgaaccaccgcgacttctaccagttggcggccagctacaacgtgcccttccaccacattcccgtgacggcggccaccaaggcgcaggccgaggccaggcaactggaaatcgtcgaggccgagggcgccgagctcgtggtgctggcgcgctacatgcagatcctgagcaacgacctgtgcaagagcctggccggacgggcgatcaacatccatcactcgttcctgcccagcttcaagggcgccaagccctactaccaggcccatgaccgcggcgtgaagctgatcggcgccaccgcccactacgtgacggccgacctcgacgaaggcccgatcatcgaacaggacgtggcgcgcgccgaccacaccgacacggtcgaagacctcacggcccgcggccgcgacaccgagagccaggttctcgcacgcgcggtgaagtggcacagcgagcaccgcgtgctgctgaacgggcaccgcacggtcgtgttccgatagcgcggcgcccccggggggtcagttgcggttggggttgtccggacggcgatcgtagcgattcggcactccgtcgcggtcacggtcccattcgccgcggcggtattcccaacggccgtcgcgttcgcgccattccggcggacggtaggcatagccccgacgggcacgcacccacgagccccggacccacacgtgttctccgttgcgccattcgtagtgccccggggcccacacgtagccacggcgcgggggcggcatgcgctccgaacgcggcggcggcggcggcgtctcgacgatcactgggcgctgcgcatgcgcggtggtcggcagggtgagtgcgcctcccacggaaagcagcgaagctgcgccgatggccaaagtgattgcgactgttttcatgggtgtcccctcatgagtggttggagccttcatgctgccggcgccatgtgaagcgcctgtaagcactcgacgggactttgtgtagaggtgtttcgcaggaatgaatacctttgttggcactcactcttgcaattcacgaagatcgacggccgcggccatggcggcatggcccgccttgttggggtgcaggtggtcgccgttgtcgtacaggggattcagcgtcatcggatcggcggggttgcgcaggatggcatcgaaatcgatcacgccgtccacgtcctggcggctgcggatccagcggttgacctcgccgcgcatggcctcggaagtttccgcccaatagggtgtgttcttgaacggcggcacggtgccgatcagaatcttcacgcccttggcacgggcctgcttgatcaactgctgcaggccatcggtgatgcgctccgcggtcgccacctcgtgctcgggcgttggccgccccggcaggccgacgaacacgctgcggccgatgtcgttggtgccgagcagcacgatcacgtgcgtcacgcccgtctgccccagcgcatcgcgcgcaaagcgcgaaaggccattggggccgatcccgtcgaccagcagccggttgccgccgatgcccgcgttgagcaccgacaccggctgcgctgccgcgggactgttgcgcagccgcgttgcaagcaggtcggggtacgacccgtcgcctccctcgccgccgcccgcggtgatcgagtcgccgaacgcgaccactgcgcgcgtgagctgcgaggtcatcacgtcgaggcccgtcacgatgtgattcagcggcaagggcgccgcatccggcagcgtggccgcggcaacggcgttgccgctggccacccagctcgcgtcgggcgcctgcaggtgaatggtcgcaaaaggcacggcgcgatcgaaaaaggcgctcgcaaccaccgcctgcccggcctcgactttcagatcgacaccatcgctgaagatttccgcgcccggtgcgacgaccacgctgccacgcccgccgaagcgcagcacccgcaccgtggacggcgagatggcgccaccgcccgtgctgcgcgccacgctcgccgcggcaatgcgcaagggcgtcttgccgaaccgattggagaaacggatgcgaacgcgctcgccactcagcgcgggctcgaactgctgccgcaccgtctgcccgcgaaaggcgtcaccgccgggccggggagccgctgccgtaaagagcggatttgcactcagctcgcggaagtccagcggagcggcagcccatccggccacccattgcgcctcggcgggctggcgcggacgcgccgtgggctgaacggcctgcacggccaccgcagcggccagcagcaagaaaccgaccgcggccactccgtgccgcagtaccccttggcgaagaacggaaagccaatgcgaacccagtttcatgcgcaaagcgactcagtttacggagcctccttgccctggcatgtgacgaggtctagtgcatcgttaccaagtgtctacataaggcaagggcgcctgcattggacgcactgcggatgcgagtccgcgcaccagccaggtgcgcgtttcggcaggatcgatcaccgcatcgatctccagcgtctgcgccatgtggatggcctcgccgttggcgtattgctgtgccacgagcttcttgaacaacgcatcgcgctcggcaccttcggccaccgcggcaagctccttgcgatagcccagccgcaccgcgccttcgagccccatggcaccgaattcgcccgagggccaggccaccgtgaagaccggcgcatcgaagccgccggccgtcatggcctgcgcccccaggccatagcccttgcgcagcaccacggcgaagaagggcacgcgcagatgggaagccaccatgaacatgcggcacacgtgtcgaacctgggcctgtgcctcgatctccggccccaccatgaatccgggcgtgtcgcacagcgagacgatcggcaagccgtgcgcgttgcacagctgcatgaagcgcgcggacttgtccgcggcatccacgtcgatggcgccgccgaggtgatgcgggttgttggccatcagccccaccggcttgccctcgatgcgcgcaagcgcggtgacgatgcccgcaccgaagccggcacgcagttcgagcagcgagcccgtgtcggccacgccgcgcatcgcggcgcgcacgtcgtacacgcgcagccggttctcgggcaccacgtggcgcagcatgcgcggatcggcgcattgccagtcgctggtcgccccctggaagtacgagaggtattgtcttgcggcagccaccgccgcagcttcgtcttcgacgaggatgtcgatcacgccgttgcgcgactgcacgctgctcggcccgatctgctccggcgcaaagctgccgagaccgccgccctcgatcatcgcggggccgctcatgccgatgttgctgcccttggtggcgatgatcacgtcggcgcagcccaaaagcgccgcgttgcccgcgaagcagcggccatgcacgatgcccaccaccggcaccttgcccgacagcgccgcgaactggctgaaggtgtggttgttgaggcccgcgacgatgggcatgtcggtgtcgcccggccgcccgccgccaccctcggcaaacagcaccaccggcagcttgagctgatgcgccaccgccagcagccggtcggtcttgtggtggttgcgcatgccctgcgtgccggccagcaccgtgtagtcgtaagccagcaccgcgcagcgcgacacctcggggccgaactgcttcgcgttgatgctgccgaggcccgtcaccatgccgtcggccggcgtgttggcgatcaggtcttcgagcgtgcggcgccgcgtctgcgcggcaatggcgagcgcgccgtactcgatgaagttgccggggtccgagccggtgtcgcacaggtcggcgatgttctcgcgcgcggttcgcccgccttgcgcgtgccgcttggccacggccgcgccgcggttggcatcgagcgtgtaggcatggcggtcgatcaccttctgcagatcgggacggatgacgtccaggtcgtgctcggcgcgggcctcggcttcaatcgcctctgcatcgacgggctccagccgcaccagcgactggccctcgacgaggtagtcgccgggctcggccagcaacgcaaccacccggccggcggtgggcgcatgcagcaggtgctccatcttcatcgcctcgagcacgccgagctgcgcaccggctggcagcacgtcgcccaccgacacctcgaactgcaccagccttgcgggcatgggcgccttgacggtcaggctgtcgaggtcttcggaaacgtcgctcgcccgtgcgcttgcggcatcgggaacgggtgcgatcttcttcggccgcttctcttccaatgccgccgccgaggccagcagatcgcccagatgcgcctccacgaatcgggtgtgcaccgcctggttcgcaaactcgggccgcgtcgcaatggcacgcagcaacgcaaggttggtggcaatcccgtcgatgtggcattcgtccagcgcgcgcagcgagcggcgcagtgcatcggcgaactgcggcgatggcgaatgcacgatcaacttggcgagcaaggtgtcgtagtgcggcgaaggcgcaagccccgcatagccatgcgtgtcgacgcgcacgcccggccccgccggcagatcgaagcgccccagtgcgccacccgaaggccgcgcattgccctctgtatcgagcgtctcggcattgatgcgccactgcaccgcgaagccgcgctgcgatgcagtgcggtccgcgtccacgccgagcgcacggagcggctggccggcggccaccgcgatctgcagctgcaccaggtcgagcccggtcacggcttcggtcaccgtgtgttcgacctgcagccgcgggttggcctcgatgaagacgaagggaagcgtgggcgacccggcatcgaccaggaattcgaaagtacccaggccgcgatagcccacggcctttgccatgcgcagcgcggcctgtgtgacctgcgcgcgcagcgcatcgggcagcgaagggctgggcgcgatttccaccagtttctggaagcgccgctgcaaggtgcactcgcgctcgccgaggctggccacggcctgcccatcgcccagcacctgcacttcgatatggcgcgcgttgcgcatcaggcgttcgacatacacgccttcgacgccgaaggccgccttggcttcggacatgcagcgcgcatgcgcttcgggcaactcgcccgcctggagcaccgcgcgcatgccgcgcccgccgccgccgccaatcgccttgatcatcacgcccgcgccctcggcatgctgttcggcaaagaaggcctgcgcctctgcgagcgtcactgcgccggcgctgccgggcatcacgggaacgtcgcattgcgtggcgagtgcgcgtgcgcgcgccttgtcgccgaacagcgccagctgatcgggggtcgggccgatgaacaccaggccggcctcggcacaggcccctgcgaagtcggcgcgttcgctcaaaaaaccgtagccgggatgcaccgcatcgcagccctgcgcgcgcgcaatggcgatcaaggccgcaatgtcgagataggccgacgggcccgttgcatcgagcgccaccacggcatcggccagctgcacgtgcagcgcggaggcgtcgtcgcgcgcatgcaccgccacgctggcaatgcccaggtcgcgcagcgcgcgcaccagccgcacggcaatctcgccgcggttggcaatcaggatcttggagaacaagagagcgcctttcaggtcttgtctttcagcagccggcgcagcaccttgccggcgccggtggtcggcaatgcgtcgatgaagctcacggcacgcggcgccttgtagctcgccatgttgtcgcgcgaccaggcgatgagcgtgtcggcgtcgagcgcggcgccgggcttgcgcacgatgaaggccttgaccacctcgcccttctcggcgtcgggctgcgcgatgacggccgcctgcgccacggcgggatgcttgatgagaatggtctcgacctcttcggggaacacgctgtagcccgagaccttgatcatctccttgatacggccgatgaaggtgaggtagccgtccgcatcgagcttgcccatgtcgccggtatgcacccagccattgcgcagcgtcgccgccgtggcttcgggcttgttccagtagcctttgaagcagccggggctggtcagcacgatctcgccgacctcgcccgtgggcaggtcggcctgcgtctcggtgtcgacgatgcggatggtcacgcccggcaccgcaatgccctgggtgccccagcgcggcgaatgatgcggcgtgtaggtgtcgcaggtgtgggtttcgctgagcccgtacgcggcttcgaacgacgtgcagttgggcgcatgcgagcgccactgcgcggccagcgcttcagtgaaggtgatgccgaagctggtgaccggattgcgccggaggctggagagatcgaagctcgcgatgtcgggcacctgcatgcaggccacgttcatcggcgcgatgctgtaccaccagttcaccttgtactgcgcaatggcctgcagcacggcgcgcggatcgaagcgatgcagcagcaccgacgccgcgccgctgagcacgggcacgttcacgcccatcagcatgccggcgatgtgatagagcggtggaatcgacagcagcacgtcgctgcttgccacgctgttgcagtcggacgccgcacgtgtcttgaagagcgcgttgccatagctcagcatggcccccttcggaagccccgtggtgcccgaggtgtaggtcatgagcgccacgtcgtcgagatcgatggccacgggctgcggcacggcgccgctttgcatcacggccaggaaatcttcgcagtccgcaggcacgctgcgcgcggcatcgcgctcggccagcagttcggcgggcaggtcgagcgcagcttggtcgggcaacaagtcggcgtagtgcaccacgaacacatgctcgagtgcgctctccggctgcaccttgcgcaccaccggcagcagcggcgcggcggcaacgatcgcgcgcgcaccgaggtcgttcacctggtaggccagctcgtgctccttgttgagcggactgcacggacagacgatggcgccgatcttctggatgccgaaatgcgccgccaggtactgcgggcagttgttgagaaacagcaccaccggctcgcccttcttcacgccgatggcctgcagccgcgccgcgaaggcgtcgctcgcgcggtcgagctgggcccacgtcatggcacggccgtaccagatgcaggcagcgcggtcgccgcgctctcgcgcatgggtgcgcaggtattcgtgcaggggctgttgcgggcgatcgggcaatgtctccatggcgtcacttcctcagggttatcgatagccgcctgcgcggggcaggcgcttgccaatgagtgcatggtgcaccaacaatcctacccatgggtataacttcggcgacacggcacaaaccctctggcaacgccagaacctcggcgggcgccgccgcacaggcgcacctgccccagggcacgggccgacagcgcgcggccacgcagagcaccgacctgcagcgcgagcgcatcctgcaggctgcggcgcagctctttgccgcgcagggctacgccaacaccaccatggcgcagatcgttcgcgcgctgggcgtgaccaagcccttcgtgtactactactttcgcgacaagcaggagatcttcgaaacgctttcgtggcgccccgcggtcgactgcttcaccgcgctcgacttcgccgcgggcgatccgcgccgcgcgagcgagaaggtgctcgaaggcatcgagcggctgattcgcgccaccatcgcgcaccacccctgcgccttctttccgtaccgcgagccgcaggtttaccggcccgaatacgtcgccgcgcagaagaagctcgcgcaccacttctacgacctgctctgcccgctgctcgaagaagcgcgccgcgatggcgacctggatttcaccgagaccaagatcaccgcgctcgctgcctgcagcctgccgggttttctctacagctggtaccgccccggcggccgcctctcgcccgaggaagtggtggccgagctcacccggctggcgagccgcgtgatcggcctgcgcagcgccaaagaaccgcgttgaagcgaagggcgcgctgccgcgccctccgcggaagtctttccaacgacatcggagacagacggacatgttgaaatccatccgcgcgccgctggcgcccatcgcccttgcctcgctgctggcccttgcgggtgcatcgcaagcccagcagcagacctacaagatcgcctacatcgatccgctctcggggccgttcgcgaacgtgggcgagctgatgctcatgcacacgcaatacgccatcgaggagatcaacgccaagggcggcgtgctcggcggcaccaggctgcagctgctgcagttcgacagcaagctctcggcgcaggaaagccagagcgcgctgcaggcggccatcgaccagggcgccaaggccatcgtcacgggcggttcgggttcctcggtggtcaccgcgctcgtgcaatcggtggcgcgctggaaccagcgcaatccgggcaaggagctgatcgtgctgaaccactcgtcgatcgaccccgagatgacgggcaagacctgcagcttctggcacttccagaccgaggccaataccgcgatgaagatgaaggcgctggccaactacatcaagaagacgcccgacgtgaagaaggtctacctgctgaaccaggactatgcccacggcaagcaatgggcgagctacgggcgacagctcgtgggcctggcgcggcccgacgtgcagttcgtcggcgagacgctgcaccccatcggccgcgtgaaagatttttcgccctacatcgccaacatcaagcaaagcggggccgactcggtcattaccggcaactgggggcaggacatgaccctgctgctgaaggccgcaggcgatgcgggctacaacctgcgctacttcaaccacagcgcgggctcggtgcccggaaccgtgctggctgtgtcgcaagcaaagctggggcagctgacctgggtcgccgaatggcatccgggccaggccgacacgccgcgggtcgatgcgctcgccaaggcctacaaggccaagaccggcaaggatttcctcgcgccgcgcatcgacttcacgccgcgcctgctggccgccgccatcaacaaggccggcagcaccgacacggtgaaggtggcctacgcgctcgaagacatgcgcttcgattccgtggtgggccccatccgcatgcgcgccgaggaccaccagctgctgttgccgcaggtggtcaacaccatcgcgccggtcgatggcaagagcgtcaagtcgggctgggagggcaccagctatggcttccggaccgacgcggtctacaccgggaacgagttggcccagggctccgactgcaagatggtccgccccggcggttgacgcgcgatgcatggggcgtcctaagggaaaccccgtcctgccgcgcacccgtgcggtcgagatactccgggtgtcacaccccggatctccgaagcgggtccacaccaaaggcgcaagaacccatggcaggcaagaactcgctctatccgatcccgcatcctgcaaagaagccgttcgtcggcaacctgctgtcgatcggatcggactctcccgtgctcgacatgtggaggatcgcccaggaactcggcggcatctactggctcgacatgccgggcatgccggtgatcgtggtctcatcgcccgcgctggtcgacgagctctgcgaagaagcgcgcttcgacaagagcacgcgcggcgcgctgcgccggttgcgcgccgcatcgcacgggctcttcacttccgatacgcacgaggaaacctggtccaagccccacaacatcctcctggccaacttcagccagcgcgccatgcaggcctaccacccgatgatgctggacatcgcggaccagctggtcaccaagtgggagcgcctgaacttcgacgaagaggtggacgtggtgcgcgacatgacggcgctcacgctcgacaccatcggcctgtgcggcttcggctatcgcttcaattcgttctaccgcgagggctttcatcccttcgtcgatgcgatggtgcgcacgctcgaaacggtgcagaaccgccgcggcctgccgctggaggaactgatgctcaagaaggagctcgcccagcagcgcaaggacatccgcttcatgcacaagatggtggaagacatcatcgaggagcgccgcgcgggcggggccgacattgccaccaagcccgacctgctgagctacatgatcgcgggcgtcgacaagaagagcggcgagaagctcaccgacaagatgatccgcgacgagtgcatcgagttcctcattgcgggacacgagaccacgagcggcctgctttccttcgcgatctacttcctgctgaagaaccccgaggcgctggccaaggcgcaggccgaggtcgacagcgtgttcgggcccgacacctcccaaaagccgacgtatgcgcaggtcaaccgcctgcagtacgtgacgcaggtgctgaaggaggccctgcgcctttacccgaccgcgcccgcgatctcgatgcgcgcgaaggaagacacgaccatcggcgggcagtacacgatcaagaagaacaacatgatcatcatgcatgcgctggcgctgcatcgcgacaagggcatctggggtgaaaacgccgaccagttcgatccggaaaacttcagccgcgaagccgagcgcgagcgtccggtcaatgccttcaagcccttcggcaacgggcagcgcgcctgcatcgggcgccagtttgcgacgcaggaagccgtgctcacgctgggcatgatcctgcagcgcttcacgctggtcgatcacacggactacaagctcaagatcaaggaagccctgacgatcaagccggagaacttcaagatcaaggcgctgctgcgcgatccggccacgcggccgcgcggcaacggcgatgcggccgccacccctgcgacgccggcccaacccaccgcgcgcaagccgcaggccgcgcggcacggcacgtcgctgctggtgctgcagggttccaacctcggcacggccgaagacctggcgcgccagctggccgaggccggcgaattgcgcggcttctcgacccaggtggcttcgctcgacgactatgccgagcggctgcccgccagcggcgccgtggccatcgtctgcgcctcgtacaacggcgtggcgcccgacaacgccgccgagttccatcgctggctcgacaaggccgacgactcactcaacggcgtgcgcttcagcgtcttcggctgcggcaacaccgactgggccgccacctaccaggcggtgccgcggcgcatcgacgagcggctcgaagcgctcggcgccacgcgcgtgcatccgcgcggcgaaggcgatgcacgcgaagacatggacggcgcgttccaggactggagcgatgcgctctggccgcagctggtgaaagccttcggcattcaatccggcgccgacacgccggccgaggccgagccgctctacacgctcgaggagctgcccccgccgcagaagaacgcgctcgtcgatgcgctgggcgccgtggcattgcgcgtgatcgagaaccgcgagctgcagaaccccggcagcgacaccgagagcggccgctccacgcgccacgtcgaactgacactgcccgagggcgtgaactacatccccggcgaccacctgagcgtggtgccgcgcaacagcccggcccaggtagagcgcgcgatggcgcgcttcgggttcgatcgttccgcgcacgtgcggctgcatgccgcttcaggccgcaagacggcgctgccggtcgaccaggtcattgcggtcgatcgcctgctgggcgactatgtcgaactgcaggacgtggccacgcgcaagcagatcgccacgcttgcggcgcacaccgagtgcccgttcaccaagcccaggctcgctgcgttatcgggcagcgacgacgcttctcaggccacctacaaggccgaggtgctgcacaagcgcaggtcgctgctcgacctgctcgaggaacaccgcgcctgccaggtaccgttcgcggtgtttctcgaaatgctgtcgccgctctcgccgcgctactactcgatctcgtcctcgccgggcatgacaccggggcgctgcagcgtcacggtgggcgtggtgagcgcgccggcgctctcgggcaacggcaccttcgaaggcgtgtgctccaactacctcgcgcgcgccgaagccggcgacacggtgcacggcgtgattcgcgaaaccacggccgaaggcttccgcttgcccgaggacccgcagcgcccgctcgtcatggtcggccccggcaccggccttgcaccgttccgcggcttcctgcaggagcgcgcggcacgggtcgagcgcggcgaatcgctgggcgatgcgatgctcttcttcggctgccggcaccccgagcaggatttcatctatgccgaggagctgaaggcgtggtcgcatcgcgggctcatgaagctgcacaccgcgttctcacgcgcgggcgagcgcaaggtctatgtgcaggacttgattcgcgaacagggcgcggccgtatggaagctgctcgaggccggggcggtgatctacgtgtgcggcgacggttcgcgcatggagcccgatgtgcggcgcaccctcgccgacctggcgagggagcacggccacgacagccaagcctggatggaccagatgatcgccgaccagcgctacgtgctcgacgtgtgggcaggggcatagccccgccgcccccaactcaggccttcaggccttccggtccggatcgggatagaccagcggccccagcaagccgcggttgaacggcttccactggccctccggctgggccaggcgatcggccagggcatagagcactgcgggatgcgcgccgagtccgagatggctggccaccacctcgatgttttctgcctgcggtcccggcttctcgatgctgcagcgccacgcgacgacaccgtcggtgcggctgaagatcgaggtcgtgggcaccggcggcgtgggctgcacgaacttcatgcggcgcgggtcgtgcgagctctggccgctcacgccctcataaacgcgccatgcgttggtggcgcgcgggctgccggaaaacgggctgcccagggtcacgacgttgcgcaccaggtccggctgcgccgacgccagaaggcgcgcatagatcccgcccaggctccagccgatcacgctgaccttctggccgcttttctcgtgcagggacttgagcagcgcaaccatgccatcttccacgccctggcgcggaccgaagttgcggcccaggccccagccgtgcgcgtcgtagccgcggctgcacaggtagcggcgcagcaccagcgtcgagccgtcgcccgccacgaggcccggcagcacgagcaccgggtgcccgtcgccgcgcggcgtgagctgcagcagcggccacatggcgatgccggcacccgtttcccagagtgcgcgcgcttcggccagcatcagcaggcccgatggcggcgcgatgtggtctcgggttgcagtggtcatgagggcagctttcctttctggtctttgttctataggacgagcatggcgaaccaaagtttcaccgccccgtcggacgacagcgatgtttatccgaggtatttgccccgcaagtaatcaaggtaagccctcgattcgctcgaaacatacggggaaatcagggtgagcgtgtaaaaagccgccaatccggggtcggcctgcgccagcgcgtcgcgccccggcaccaggcgttcgaacgaaagccagcaggtggtggtgaagaccatctgcagcgcaaggatgcgcgcctgctcggcgctggtctcgatgacgcccgatgccaccagcccttcgcagagcgcctgggccgccagcaggttctgcgcggtgagcgcctgcgcgcgctgcccgagcgtggggtattcgctggccaggaaggccatgtcccgatagatgaaccggtactggtcgatggcttcgaagcgcaggtgcagcgccagccagaggtcgtcgatggcggtgatcgcaccggaagacccgtcgagcacctcgagccgctgctcgaaacgccggaacagccactcgacgatcagctgcttggccttgaagtgatagtgcaggttgcccggactcatgccgagctcggccgcgatcttgtgcgtggacaccgccgcgaggccttccgcgttgaacagcgcaaggctggcctgcaggatgcgatcgcgcgtggtgttggaactggccacaaccggctgctgcgtgcgtcggtgcttcgctgggccgatgctcagcgcttgccgctgccgcgcgggccggcgttcttggggtcgagttgggcgaggcgttcatgcagccgggccacttcttcgcgcaaggcctgcacctcttcggcgctgggcatgccgagccgctgcaatgcggtggcaacgcgctggtcgaagacgtcttcgaacttgcgaaggccaaagctgtcgaggctcggaaagccgcgcggaatcgccgccttggcgccattggcgacgtcgggcttgacctggccgatgcccagcagcccctcgatcacgttggcctgccgcttggcgacgtcgttgcgcacgttgccaagcaccttcaggcccgcgcgcagcaggccttcggcgccgccggcctttgggtccggacgggcttcgggtggtgtgacagcagcagtttttttcttcgctggcgcagccgtcttcctggctgcgggtgctttcctggccgtggaggctttcttcgcaggcgccgccgccctcttcttttgcagatttggggtcgggtcgggacgggtcgccatgcgttcttgctccaggatcaggctgccttgcgggcagcggtgcggcgaaccggcttcttggcggcggcggccttggccttcacggtgcgcacggtcttggcttcttcggtgccgctcacgcgcacttcgatctgcttggcaccggcaaccaccttgtcggcgatctgcaccgacacgttggcgatcggctggttcagcgcgttcagggttttgaccaccgaggtgacgatgggcgattcgacacccgccacacggccggccacggcttcgatgccgctggtcgtgcccgcggccacgcggtccatcaccgaaacgatgcggccggtgtcgatgtccaggcggttggccaggaaaccgttgatcttttcttgcgcgccgatcaggttggccttgacctgttcgctcaccagcggaatctggcggctgcccaggaattcgctgtagcgcgaagcagcgccgccgagcaggcgatgcacgccggcacgataggcacccaccagggtcttgccggcgtcgttgtactggccgatgacgtggatggctgcggaagagaaagaagcttgcgtggtcatgtggatttcctggaagttgattgatcggtcgcggatttgcgatggagtgatcttcttccagagcgcctaggcctgaaaagctagaaccgtcggaaaactagtccaactgccccaattttccggccatggcctgccgatcatgccgcagcagcggccctggcgcgcttggccggcgcggcgggcttgcgcggcggcgccttgccagcgggcgccttggcgggcactttcctggcggcggtcttggccgccggcgccttggctgcaggggctttcgccgggagcgccttcttggctgcggcctttttcacggcaggttccaccgcgggcttggaggcgggcttggccgctgccttcgcgacaggtgccggctcgggagccgcggccttcggcgctgccgcggggtggctctgcgtcaggctcatcagcagctggtgctcggccagcaggtagtcgccgatctcggtgatgtcgggcaccgcgcggcggcaggcgatgagaccgtagtccatgcggccgttgtagctctgcaccgtgacgttgagcgccgtgccgtggctcgcgatggagaccgggtagtagctggtgaccagtgcgcctgcaaagtacatcggaaacggcgcgccggccacgttggagatggccacattggcggccggcggcagcaggttcacgagcccagagcgcccgaccatcgaggcgatgcccgacaccagccagggcgcggcaaaggtgggaaagtcgtccaggatcaccgccttgaagcggttcatggtcgacttcgagctggtcgacgaggcgttgatggccttgagccgctgcaccgggtcggtgatgtcggtggccaggctcacgaggatcatgctggcctggttgttggcggtctcgtcgccggcttcgcgcaggctcacgggcacgccggccaccagcggcttggcgggcagctcgttgttgtcggccaggtagtggcgcagcgcgccggccaccgtggccatcaccacgtcgttgagcgacacgccgaagtgcttggcgatgtgcttggtctcggccagcgaaatggtgcggcccgcaaaggtgcgctggttcgtgatcgacacgttgagcgaggtgcgcggcgcaaagaggttgaacttcttgggcgcggtggctgcgttcttctcggccgccttctcgtcgggcttggcgaggccgcccagcgcacgcgcaatggccggcgccatcttgaagagcttgacgtactgctgcgccgtgttgcgcagcgccgcggtcgcgagttcggccatgcccagctggtagccgctgctgcgcgggcgtgagcgcggcggcttcaccacgcggcccgtggcttcgaggtcgaagatggccttgccgagcgccacgccggcctgcccgtcgatgcccgcatggtgcaccttggtgtagagcgccacctgcccgctcttcaggccgtcgatgatgaagaactcccacatcgggcggctgcggtcgatcagcgtcgaatgcagccgcgccacgtactgctgcagctgccggttggtgccgggcttgggcagcgtgatgtggcgcacgtggtagtccaggtcgatgtcgtcgtcttccacccacaccgggttggtcaggtcgaagggcatcagcgcgagcttgcgcgtgaacacgtcggccaggtggatgcggctggccatgaactgcttggcgtcctcgtagaagtcgcccttgtaacctttgggcaggtcgagcacgttgagcgagcccacgtgcatcggcatctcgggagtctccagatgcaggaaggtggcatcaagaccgctcaggtgtttcatgtgtcatgtctccttgtgtgcgcaggcgccgttcggcaggatacccgtgcacagccctgcgaatcggggctaaagcattgaacgcgggtttgtcccgagacccctgcgcggtgcgctattaattcaatagctttcgccgggccgcgagacatgcccacttcacgccggattcgtacactgggcccatgacatccatcgcttccacgcagaccgacgagttcctgtggctcgaagacatcgacggcgccgaacagctcgcatgggcccggcagcacaacgccaagaccgtgcaacgctatgcgcaatcgcccgccttcgagcgcatggagcaaggcattctcgaagtgctcgactccgatgcgcgcattccgatggtgcgcaagatcgggctgctcttctacaacttctggcgcgacaagaagaaccccaagggcgtgtggcgccgcaccacgctggccgaataccgcaagccgcagcccgactgggaaacggtgatcgatctcgatgcgctggccgaggccgacaaggaaaactgggtctggcacggcgcagagggcctgcagcccgagtacaagcgctgcctggtctcgctctcgcgcggcggtgccgatgccgacgtggtgcgcgagttcgacctcgagctcaagcagttcgtctccgggggcttcacgctgcccgaggccaagaacagcatcgcatggaaagacatcgaccacctctacgtggcgaccgatttcggccccggctcgatgaccagctccagctatccgcgcatcgtcaaggagtggaagcgcggcacgccgcttgagagcgcgcaggtggtgtacgaaggcggcatggacgacatgacggtgagcgcctggcgcgacaacacgccgggcttcgagcgcgacttcgtctcgcgccagatggacttctacgacagcgaaacctggctgcgcggcagcgacggccggctggcgaagatcgacgtgcccgacgatgccaatgccgacatcacgcgcgagtggatgctggtcgagccccgcagcccctggaccgtggccggcaccacctacaagccgggctcgctgctggcgacgaagttcgacgactacatggccggcaagcgcgagatcacggtgctgttcgagcccgacgacaccaccgcgctcgacgaccattcgtggacccgccaccacctgattctcaacgtgatgcacgacgtggtgaacaagctcgaggtgctcaccccgcaatccggtgaatggaagcgcgaaagcctgggcggcgcgcccgagctctcaaccattgcggccggcggcatcgacgaagacgagaacgacgactattttctgaccgtgagcggcttcctgcagccgaccacgctctacgtcggcaccatcggccagggcgagcccgagccgctgaaggacagccccgccttcttcgatgcctcgcgccatcgggtgagccagcatttcgccacctcgaaggacggaacgcgcgtgccctatttcgagatcgcgccgaagaacctgcaggccgacggcgggaacccgacgctgcaatacgcctacggcggcttcgagatctcgctgcagccgagctacagcggcagcatcggccgcgcatggctcgaacaaggcggcgtctacgtggtggccaacatccgcggcggcggcgagtacgggccacgctggcaccaggccgcgctgcagcagaaccggctgcgcacctgcgaagactttgccgctgtttccgagcacctcatcgcgcgcaacatcacctcgccgcaacacctgggcgccatgggcggcagcaacggcggcctgctgatgggcaacatgctcacgctccatcccgggctctacggcgccatcgtgagcgaggtggcgctgctcgacatgaagcgctacacccagctgtcggccggcgcctcgtggatcgccgaatacggcgacccggaagatccggaagaatgggcgtggatccaggcgttctctccctacgagaacgccaggccggggcagccctacccgccggcgctgttcaccacgtcgacgcgcgacgaccgcgtgggcccggtgcatgcgcgcaagatgtacgcgaaactggccgccatgggctacgacaccagcttttacgagaacatggaaggcggccacagcgcggcggcggacaacaaggaatcggccttcatggacgccctgggctacgcctatctctggaagcacatcggacgcacatcgacatgagcaacgacaacggcaccaccctcgaactgatcggcgcgcccaccgacatcggcgccagcgtgcgcggtgccggcatgggccccgacgcgctgcgcgtggcggggcttccggaggcgcttgcgaggcagggcttcaccgtgctcgaccgcggcaatctcgccgggccggccacgccctggaccgcacccgccaacggactgcgccacctcgacgaggtgattgcctggaaccgttccgtctatgcgtcggtggacgccgcgctgggcagcggccacgtgccgctcatgatgggcggcgaccattgccttgccatcggctcgatcagcgccgtggcctggcatgcgcgcaagcgcggcaagaagctgcgcgtgctgtggctcgatgcgcactccgacgtcaacaccgaaaccaccagtccgagcggcaacctgcacggcatgcccgtgtcgtgcctgctgggccacgggcccgcggtgctcaccggctggagcggcgagcgcgcggcgctcgagcacgacgccatccgcttcatcggcatccgcagcgtcgacgcggaagagaaggaagccattcgcacccttggcctgcacgtgttcgacatgcgccacatcgacgagcacggcatgcgcaccaccatgaccgaggcgctgcaggacgtgggcgaagacacccacctgcacgtgagcttcgacctggactgcctggacccgaacatcgcgccaggcgtgggcaccggtgtgcgcggcggcccgacctaccgcgagatgcagctgtgcatggaaatgatcgccgacaccggccggctcggctcggtcgacgtggtggaactcaaccctgcgctcgacgtgcgcaaccagaccgccgaggtggcggtggagctgatcgagagcctgttcggaaagtcgacgctggtgcgctgagcgcgtcaggccggtctcaacctgggttcggtaccggcttcaccggaaaaggcgtggccggcgccgggggagcgagtggcgcggacggccgcggagcttcgggcgcgacgctgggggttgcgggctcttcgccgccctggccttcgagaaagcgatcgagcagcgcaaagaagcggtcgtagaagagttcgtcggtgagcgtctcgctggccaccttgaccatggcgtcgtcgctgccggcaaaaggcagagaaagcgagccgaaggcgcccactccaacgctggctgagctattgactttcttgatgccgtagcggtcttgcagcgcggtcgcaaaggccacggtgcttcgcttgccggccttgccgccttcgcgcgcgcacaccacgcggaactcgacctccacgtgcacctcgaaggccggctggaaactcttgcgccccgtcacaaggtcggggttggccgcgttgatcatgtagccctggctcagcagggcgcggcgcgcggcttcgcaggtctgggcctcggtggcggcgtagctgcgcgtgtgggtggtggtggagtcgaactcctcggtttcgtacgacacccggcgcgggctgctgccgcaagcggcgagcaatagggccgacaacaggccgaggaccagaaccggagcgcgaacgacggaaaaggcagatgagaagcgaagggacatagtcatggcgcggcgaatcctaaccggcgtctccgccggcgaggttttcgagcatcgccgggcgccggcgttcccagcgcggcgcaagaatttttcaggaccagtgcagcacgtggtgcgcacgcacgcgcgtcgcggcaatcaaccgtgcattgggcgcgtcggttcgggccacccagtcgcgcgccgcctcggcgctgcggccgaactgctggtggcgcttttgcaaacgctcttcgcgcaccgcatcgtcgatgtcgacgtaccagacctcgtcgagcatcgccgccgcgccggcccaggggccgtcgtcgtgcaggagatagttgccctcggtaatcaccagctgagtctccggcagcaccgcgatggcgccagcgatcggctcctcgatctctcggcggaactcgggggcgtagacgatggggtcgtccggcccctgctcgcgcagccgctgcagcagcgccacgtagcccgcgctgtcgaaggtatcgggcgcgcccttgcggccggcacggccgagccgttgcagctcgacgttggccaagtgaaaaccgtccatcggcacggcctgcgcgcggctcgcgcccaccgcctggagtaacgccagcgcgagcgtggacttgcccgcaccgggagcgccgaccagccccaacagcttgcgccgcccgccggccatcagggcatgcagacgggccatgccgtcggcgggaatggagggaagttcttgcgcggggatggtgctcatcccccgagcgtacaaccctccggcgcttcgaaaatcagggatacaggccgcgttcctggcgggccatcaggatgcgctcgcaagccaccgcataagtggcggtgcgcagcgagatcttgtgcttgtcggccgtgtcccagatctggttgagcgcgttcatcatgatgcggtccaggcgcacgttgatctcgtcctcgtcccagaagaaggacgagaagtcctgcacccattcgaaataactcaccgtcacgccgccagcgttgcagatcacgtctggcaccaccagcacgccgcgctcggccaggatgtcgtcggccaccggcaccgtggggccgttggcgccttcgagcaccagcttggcggtcgttttctgcgcgcgctcggccgtgatctggccttcgagcgcggccggaatcaggatgtcgcaggccacttcccagaagtcttcgttcggcacgatgtcgccgccggccttgaagccgaccacgccgtcggtgcgcgagatgggcaccagcttggccaggtcgaggccgttcgggttgacgatggtgccggtgtggtcctgcaccgcgacgatcttggcgcccgcctcggcaaagagttcggccgcgaccgagcccacgttgccgaagccctgcaccgcgatgcgtgcgccgcgcaggtccatgcccaggcgtcgcgctgcttcgcggcccgtgacgaacacgccgcggccggtggccttgacgcggccgagcgagccgcccaggtgcagcggcttgccggtgaccacgccggtggcggtgccgccgacgttcatcgaataggtgtccatcatccacgccatgatctgcgcgttggtgttcacgtcgggtgcgggaatgtcggtgtgcgggccgatgatgatgccgatctcgctggtgtagcggcgcgtgaccttctccagctcttgcagcgacagcttcttgggatcgacgcggatgccgcccttggcaccgccgtacggcaggttgacggccgcggtcttgatggtcatccaggccgacagcgccatcacttcttcgagcgtgacgtcggggtggaagcgcacgccgcccttgcccgggccgcggctcatgttgtgctgcacgcggtagccctcgaagtgggcgatggtgccgtcgtccatttcgatcggcacgtcgacgatcagcgcgcgcttggggcgcttgagcgtttcgacccagcgggccagcgggccgaggtaaggcaccacgcggtcgacctgcgagaggtacgtgccccaggggctgttggcggtcggattgacgaaggagagcttttcactcatgggaggtcccttggtttgaatggatggccgcaacgatagacctctcccgcccgctgcgccatggcttatgcgcgccgcgctgtcgggttatgcaagagaggcttggccggccagcctcggccaggggcctacgccacggcgctcagcagggccgcattgccgccggccgccgtggtgttgaccgtgaccgtctgttcggcgcaaaagcgatacaggtagtgcggcccgccggccttgggcccggtgccgctcaggccctcgcctccgaaaggctgcacgccgaccaccgcgccgatgatgttgcggttcacgtagatgttgcccacgtgcgcacgggtggcgagcgcctgggcgcgcgaatcgatccgggtctggatgccgagcgtgaggccgtagcccagcgcgttgatccggtcgatcacctctgcgggctcgctcagctcgccacggccccagcgcgcgatctgcagcaccgggccgaaaatctcgctggtcacgcggtcgatggagctcacctcgtaggcctgcggcggaaccaggttgccctcggtcgaagaagaagccggtgcaagaaggcgcttcgcttccgagtccagccgcttcaggtcgcgtcggatgttgtcggcggcttcgcggtcgatcacggggcccacgtcggtcgccagcagggccgggtcgccggcggccagttccccggccgcgccgcggatcatctcgatcaccgcgtcggcgatgctgtcgtgcagcaccagaaggcgcagcgccgagcagcgctggccggccgagcggaatgcgctttgcaccacggcatcgaccacctgctcgggcagcgcgctcgaatcgaccagcatcgcgttgatgccgccggtctcggcgatcagcggcacgatcgggccgtccttggcggcgagcgcgcgatggatgattcgcgccacctgggtcgagccggtgaacaccacgcccgccacgccgggtgccgagaccagcgcggcaccgacggtttcgcccggcccgtgcagcagctgcaccgcgtcggccggcacgccggcggcgtgcagcagcttcacggcctcgagtgcgacggccggcgtctgctcggccggcttggccagcacggtgttgcccgtggccagcgcggccgccacctggcccatgaagatcgcaagcgggaaattccaggggctgatgcagacccagggcccgcgcgcggtgagccgcagttcgttgctctcgcccgtcgggccgggcagcgccacgggctgcatgatgcgctcggcctcgtcagcgtagtagcgcaaaaagtcgatggcctcgcgcacttcggcgaccgcgtcgccccaggtcttgaaggcctccttcaccagcagcgcgcagaagcgcggcagctcgcgttggagcgcatcggcggcctggcgcagcatggcggcgcgcttttccaccggggtcttgcgccagctacggaagctggcggcgctggcagcaacggcccttgccgcactggcggcatcgaacgcttcgacgcgaggcacggcagtggtcgccagggccgccagcagcggcgcgcgcatcgactcgaccgcaaggtccaggccttcgctgttgcgccgtgccggcgccggaccgtagagcgccggcggcaacggcaaggcagggttggtggcctcgagccagagcggcgacatgagcagctcgtcgacgtccaccgtttcgtcgcccagctggttcacgaacgacgaattggcgccgttctccagcaggcgccgcacgaggtaggccagcaggtccttgtgttggcccaccggcgcatacacgcgcaccggcgcggccgtgctcttcatcacttcgcggtacacgccctcgcccatgccatgcaggcgctgcagctcgaacggtgcccgcgccgcttcggccatctgcaggatggccgcgatggtgcccgcgttgtgcgtggcaaattgcggatagatcgcgtcgggcgccgaaagcagcgcgcgcgcgcaggccaggtagctgacgtcgctgtggtgcttgtgcgtgaagaccgggtagtgcggcagcccgagctcctgcgcacgcttgatctcggcgtcccaataggcgcccttcacgaggcggcacatcaggcgcagccggtgcttgcgcgccaccgccgtgacatgctcgatcagttcgagcgcgcgcgtctggtaggcctgcagcgcgaggccgaagccgcgccactgcggctgctcggccgccacgcgcgcggccagcgcctcgaacacgtcgagcgacagctcgagccggtcgacttcttcggcgtcgatggtgaggttgaggttggccgcggccgccagctcgcacagctgccacacgcgcggcaccagttcgcgcatcacgcgttcgcgctgcgcgtcttcatagcgcggatgcagcgcgctgagcttgatggagatgccgtcgttgtgctcgggcggcctggccgcatcggcaccggccgcaatggcgcggatggcatgcgtatagctctcgagatagcgcagcgcatcggcgtcggtgcgcgcgccttcaccgagcatgtcgtagctgaagcgcagggcgtcgtgcttgcggtgcgccgagcgggcctcgtccatggcttcggcaatggtctggcccagcacgaactggcgccccagcagctgcaccgcgcgcagcgtggcggccaccaccgtgcgtgcgccgagcttggccatgaggccgggcggatggtcgccctcgggcaggaatttcttcgacatcgcgatggccgcggacgaaaggcgcgacagcgtggaatcggctgcgccgtcgaaatcggcgcggcccagctggtcggccgtgagcgcaatggccgtggcggcgtcgggcacgcgaagcagcgcctcggccagacgcatcaaggccaggccctctgcgctggaaatggggtattcgcgcagcaggctttccatggcccagaagggcggcgggtgccggcgcaccgcctccacccaggggcgcgcggcggcggccgccgcgctccattcgagtgcgcctgccagcgaggcgaggcggtgcgagacgacgtcggcttcgggccggtaagggatgggcaggtgcatggcagttccttggttctatcccctatgatctttggatatagaccgaatcttttgccaaaaatgacaacctcgaccggataattcaccaatgcacgacatggacctggaccgcatcgatctccggctcctgaagattcttcagcaggatggccgcatcaccaacctcaaattggccgaggcggtggcgctctcgcccaccgcggtgctggcccgggtgcagcggctcacgcgggacggcttcatcctgggctacgaggcccggctcgatccccacaagctcgggcgcggcctcaccgtgttcgtcgaaatactgctcgaccgcaccacgcccaacgtgttcgaccagttcaaggcggccgtgcaggtgcgcgacgaaatcatggaatgccacatggtggcgggcggcttcgactacctgctcaagacccgcatggccgacatggcggcctaccgcgagttcgcgggcaccgtgctgtggcaactgcccggcgtgcgcgaaacacgcacctacgcggtcatggaagaagtgaaaagcagcgcgcggctgccgctgggcatctagcggcggccgaagatcgcggtgccgatgcgcaccattgtgctgccggcgctgatggccgcctcgaggtcggcgctcataccgagcgaaagcgtgtccatctcgatgcccgcggcccgaatggcgtcgtagacggcacgggcgcgaaggcagagttcacgctgcgcggcgaaatccggtgccggttcgggaatggccatgagcccacgcagccgcaaatgtggcaaagccaccacagcgcgcgcgagcggcagcgcctcttccggcggcacgccagacttgttcgcgccgccatccacgttgacttgcaggcacacctgcagcggcggcaaatgcgccggccgctgcgccgaaaggcgctcggcaatcttgatccggtcgataccgtgcacccagtcgaaatgctcggccacgggccgcgtcttgttgctttgcagagggccgatgcagtgccattcgagttccgagcgcagatccgaaagcgcctcgatcttgtccaggccctcttgcacgtagttctcgccgaaggcccgctgccctgcctcgaaggcctcgcgcacagcctccggcccgaaggtcttggacaccgccagcagccggacttcggccgggttgcgcccctcggcggcgcacgcctttgctatccggctctttacttgctggaggtcgtcgccaatcatcgtcataatcgtccccaaatcgtatcaaaacgtcaccgaactcgatcgaggagccccgtggacattacccaactgctggcattcagcgtcaagaacaaagcctccgacctgcacttgtcggccgggctcccgccgatgattcgcgttcacggcgacgtgcggcgcatcaacgtcgatgcgctcgaccacaaggcggtgcacgccatggtgtacgacatcatgagcgacacgcaccgcaagcactacgaagagttcctggaggtcgatttctctttcgagatcgacggcctggcgcgcttccgcgtgaatgcgttcaaccaggcgcgcggcgcggccgcggtgttccggaccattccttcgaagatcctcacgctggagcagctgaacgcgcccaagattttcgcggaactggcgctcaagccccgcggcctggtgctggtgaccgggcccaccggctcgggcaagtcgaccacgctggccgcgatggtcaactacctgaacgaaaacgagtacggccacatcctcacggtggaagacccgatcgaattcgtgcacgaatcgaagaagtgcctgatcaaccagcgcgaggtcgggccgatgacgctctcgttctccaacgcgctgcgctcggcgctgcgcgaagacccggacgccattctggtgggcgagttgcgcgacctggaaaccattcgcctcgcgatgaccgcggccgaaacgggccacctggtgttcggcacgctgcacacctcgtcggccgccaagaccatcgaccggatcatcgacgtgttcccgggcgaagaaaaggaaatgatccgcgccatgctgtcggaatcgctgcaggccgtgatctcgcagacgctgtgcaagaccaaggacggccagggccgcgtggcggcgcacgagatcatgctgggcacgccggccatccgcaacctgatccgcgaagccaaggtggcgcagatgtattcggccatccagaccggccagggcgcgggcatgcagacgctggaccagaacctgaccgagctcgtgcggcgcagtgccatttcggcggcggaagcgcgcggcaaggccaagattcccgaaaacttccccggctagatgtggctcgcccccagtctgcgcgcacttcgtgtcgcttcgccaaccccctaccgggggcaacaccagcggcccggcaaagccggttccgcggtgttcccagaatggggatcaccttttaaacgccgcgttcgtcgaataatgacggcacactgaatcaggagtcgcacatggaacgcgatcaagccagccagttcatcaacgacctgctcaagctcatggtgagccgcaacggcagcgacttgttcatcaccgccgactttccgcccgcgatcaaggtcgacggcaaggtcaccaaggtttcgcagcaagcgcttggcgcgcagcacacgctggcgctcacgcgctcggtcatgaacgaccgccagacggccgagttcgagcgcaccaaggaatgcaacttcgcgatctcgccgaccggcatcggccgcttccgcgtgaacgcgttcgtgcagcagggcaaggtcggcatggtgctgcggaccattccggccaagctgccgaccatcgacggcctgggcatgccgcaggtgctgaaggacgtgtcgatgaccaagcgcggcctcaccatcctggtgggcgccacgggctcgggcaagtcgaccacgctggcggcaatggtcgactggcgcaacgagaactcctacggccacatcgtgacggtggaagacccggtcgaattcgtgcatccgcacaagaactgcgtggtgacgcagcgcgaagtgggcatcgacaccgacagctgggaagccgcgctcaagaacacgctgcgccaggcgcccgacgtcattttgatgggcgaaatccgcgaccgcgagaccatggagcatgcagtggcttttgccgaaacaggccacctgtgcatggccacgctgcacgccaacagcgccaaccaggcgctggaccggatcatcaacttcttccccgaagagcgccgcgcccagctgctgatggacctgtcgctgaacctgcgctcgctggtctcgcagcgtctggtgcccaccgaggacgggctgggccgcgtggcggcagtggaagtgctgctgaacacgccgctcatttccgacctgatcttcaagggcgaggtgggcgagatcaaggagatcatgcgcaagagccgcaacctgggcatgcagaccttcgaccaggcgctgttcgacctgttcgagagccattcgatcaccttcgacgacgccatccgcaacgccgactcggccaacgacctgcgcctgcagatcaagctcaacagccagcgcgcgcgcagcaccgacctcgcggcggggacggagcatttcgcgatcgtctagacgcgtgacgcgggcgccgcgttggctttaagctctcgtccatgagcagcatcaactcccgaacctacgaatccaccccctcccagacggtggcctttctgggccttggcgtcatgggcgggccgatggccgggcacctggccaaggccggccacaaggtcactgtctacaaccgcacaccggccaaggcccaggactgggtggccgaattcggcgcccccggccgccatgccgccaccccgcgcgaagcggcgaccgacgccgacatcgtgttcagctgcgtcggcaacgacgacgacctgcgcgccgtggtgctgggcccgaacggtgccttcgcgggcatgaagcaaggcagcgtcttcgtcgaccacaccaccgcttcggccgacgtggcgcgcgagctgtcgaatgcggcgcagtcggccggtttccagttcatcgacgcgccggtgtccggcgggcaggccggcgcgcagaacggcgcactcaccgtcatgtgcggcggcgacaagacgagcttcgaacgggtcaagcccgtgatggccgcctttgcgcgggccgtcacgctgcttggcgcgagcggcgccggccagctcgcaaaaatggtgaaccagatcgcgattgcggggctggtgcagggcctctcggaagccattgccttcggccagcgcgcgggcctcgacatgaaggtggtgctcgacgtcatcggcaagggtgccgcccagagctggcagatggacaaccgcggcaagaccatgatcgaaggcaagttcgactacggctttgccgtcgactggatgcgcaaggacctgggcctggtgctcgacgaggccaagcgcaacggcgcgcgcctgcccgtgacggcgctggtcgaccagttctatgccgacgtgcagcaggccggcggcaagcgctgggacacgtcgagcctgatcacccggctcaagtaaaaaaagaaagcccgcgcaagcgggctttttctttgttttacggtcagcgcaccggcgtgggcgtcgcgccgccgggctgggccggcggcagcggttccatcggcggcagcggcacgcgcgaagaagacgaggatggcgcggggccaggtgcgggcgcaggtgcaggcgcccccgtgccgccgcgctgcgcctggttggccagttccgattcgctcacgatctcgaccacgcgcaccaccttctgcacgcccgagatgccgcgtgcgatctcggtcgcgcggtcggtttcgcgccgtgtggcgatgcccatcaggtagaccacgccgcgttcggtcaccaccttgaacgaattggcgaagatgtccttggcgtcgagcagcgaagccttgatcttgccgctgatgaacaggtcgttcgagcgttcctggaaggtgctggactggccgatggtgagttcgttgaccaccgagcgcacgttgtccacgcgctggatcacgtcctcgacgcggcggcggtcggcctcgctgcccacggcgcccgtcagcagcacctggcggttgtagctggtgacgctcacgtacatgttgtcgttggcaatctcgcgcacgcgcgcggccgcacgtagttcgatgccctggtcgtcgagctgggctcccgagctgcggcggtcggtcgccaccatgcccatgcccaccgcggcggcgccccccaccaccagcggcacgcaggccgaaagcccggcaaccagcacggcccccgaggcaaatgcaatggcgatgcgttggaacggtgtcgtcgtcatgtagaagcttcctgttctccgagtaactgggcatccacgccgtcgcacaggcaatgcagtgcgagcaggtggacttcgtggatgcgggccgcacgttcgtgcgacacgccgatctgtacatccgtttcgcgcagcgcgcgcccaatggcgccgccggttccggtgctgcccgcgccgggcgatgccggctggccggcgctggcgttgcccagcagcgcgaccacggtcatgtcgcgctcgtgcgcggccaataccgcggccagcacggcggccgactgcccactggcgctgagcaccagcagcacgtcgccggcctggccgagcgcgcgcacctgacgggcgaagcggtcggcgtcgatggcgctggcgctgtcggccgcgggatcggtggtgtcgccgggcagtgcgatggcggccagttcgggccgctcgcgctcgaagcggccgacgaactgcgccgcgaactgcgccgcaagcaggcccgacacgcccgcaccacaggccagcaccttgccgccgctggtcacgcacgcgagcaaggcctgcatggcttgcgaaatgggtttgctcaggactgggccggcctggtacttgaggtcggcgctatcgatgaagtgttgctgaatccgttgctcgagcatggggcgggatgataccggggggcgatgaaacaagacgtgtgtggtgtggagcttatgccgagcgctcagttcccgcccgcatcgaatgcggccttcagccaggtgatgcgctcctcgaccagcaccacgtcgaaccggcacggcggcagcgtgcgcaggttgttcaggtaatggcgcgccgcaaagacgatgcgccgctgcttgacccccgtgatgctgccgcccgccccgccgtgcgcgccggtgctgcgctgccgcacctcgacgaacaccagcgtggcgtccttcggatcgcgcatgatcaggtcgatctcgccgccgccgcgcccgggcgttcgataattgcgcgcaaccagcaccaggccggcatcctgcaggtggtcgagcgcggcgtcttccgcggcatcgccacgacgcttcgtcgtcgttgtgatggtcttcatgcgtgctccctgccgttatcttttttgtttcttcggagaaacccattggcttcatttgcacccgcttctttcggcgccgtccttgcggccgcgcgcgacgcctcgggtgcacagcattatccgcagggtacgctgtacgtggtggccacgcccatcggcaacctggccgacatcacgctgcgcgcgctgcatgtgctgcagatcgtggacgccattgcctgcgaggacacgcgccacacacaaagcctgctgcgcgcctacggcatcgaccggcccggcggccagctcctggccgtgcaccagcacaacgaggccgaggcggcgcaaaccgtggttgcgcggctcgcccagggtgagcgaatcgcctacgtgagcgacgccggcacgccgggcgtgagcgatcccggcgctcggctggtggcggccgtgcgcgcagccggccagcgcgtgctgccgctgccgggcgcgagcagcgtgaccacgctggtcggtgcggccgggctggtggccgagggtggaagcgacggcaatgccagcagcgccttcgtgttcgcgggcttcctgccgacgaaggccggcgagcgcgacaccgcggtgcaggcgctcgcgcaagagccccgcgcagtcgtgctgctggaggcgccgcaccgcatcgaggccctggcccgcgcgctggccgcgctgggcgagcgccgcatcaccgtgggacgcgagctcaccaagcagttcgaggagattgcgaccgttgccgccgcagagttgccgggctggtttgccgccggccgcgaccgcacgcgcggcgaattcgcgctcgtgctgcacccggtggccgcatccaccgacgatggcgccgaaggcgaacgcgtgctgcgcctgctgctggccgagctgcccgtgaagacggcggtgcggctcgcggccgagatcagcggcgcgccccgcaatgcgctgtacgaaacggcgctgcgcattcgcagcgaggccggttcggccgacgacgaataaacctcagccgtccagctccgcatagcgcctgaagatcccgtcttcattgaacgcgatgcggcgcgggctttgcaggtagtcgtgcacgcgctggcggcgcctgacgttgtcgtgcagcttctcgactaagggcgtgacggcgagcgccctgcccgcggccttcggaaacgcgtagcgcaggccttccaccagctggaacagcgacaggtcggcataggtgagcacatcgcccacgaggtgcgacgaacccgccggattgcgctgcagcacccgctcgagccagttcaggaacttgggaatccgctcttcgcggaaggcccgcgcgcgctgcacggccgcgtcgcgctggtcttcgtagtaggcgccggtggagatcggatggtgcgtgtcgtgcgcctccgccaccacgtcggcaatggtgagctgcagctggtgcgtccagaggccgtcggattcgccgacgcccgcaaggccgaggcggggcccgaggtacagcaggatggccgcggtctgcccgacgacgatgtcgccatcgatcaggaacggcggcgcgaaggacgggcgcacgatctcggggtcgtcgagccggtcgcccaatgcggactcgccgccgcccttcgattcgggcagccgcgccacgtcgacatagtccgcgccggccgcctcgagcgcgagccgcacgaattccccgcggccctggatcgtgggccagtagtggagttgataagtggtggtcatccggccatggtgtcaggctcggcgcggccccgcaaccgcccgcttttagcccctcacagcctctcggccagttccaccgcgcggcgttttgcatcagtccgcgcgacggcgtcgacctccggtcccatcaacgttttttcgaccacgaccgagcgcacctcgcgcacgccgatgaaccgcagccacgtctcgacgtagggcagctgaaagtcgagttcgtgcgcggagccatcctttcccagcggatagtccaaccctcgcgcgcacaccaccgtcgccatgcgggtctggagcatgcccgacaggcccgaggcgtcgaagcggaacagcacgtccttgtgcgacaccacgtcgatcaggtgcttcagcttgtagggaatgccaaagttccacagcggcatcgccagcacgatatggtccgccgcgtggaaaggcgcggcgatgcgccggacctcgtcccaggccgtttgctgggcatcggtgagcggcacaccgttgatgccggcgtacttggcgtcgagcatgtcttgcgacagttccggaagcgccatcgtccaggggttgagcgtggtgacacggcacgccgggtgcacgcgcttcacctcgtcaatgaatgcgccggccacttcgatgctggcggaacgcgtttgccttggcgatgtctcgatgtacaggagttctttcatggcttgcagggcgtgagtggttcaggtcagccgaggctaggcaccaaccagcgcgcgcacaagcaacataatttgcggcaattcagaacaaactgcactgaacgaaaccatgctcgattcccagcaactgcgcgcctttgtctccgtcgccgaccacggcagcgtgacccgcgccgccgaagccatgcacctgacgcaatcggccgtcagcgcacagatcaaaaggctcgaagaacagctgggctgccgggtcttcgagcgcaccacccgctcgctgcagctcaccgcccagggcagcgtgctgctgagctatgcgaggagcatcctcaacctgcagcagcaggcggtctcccggctcgcggcgccccgccatgcgccgacgaccctgcgccttggatgctcggaggggtttccaagcgaatggctctttgccgcgctcgcaggctttcgccagcgccggcccgacgtgcatgtggagatcaccggcggcctcagcaccgtgctggccaaacaggtgcggcagcgctcgctcgacctgatggtcggcacggtctgcgatgccggaagcgacaccgaaacgctctggatggaaccgctggtatgggccttttccgagcgcgcgctgctcgaccctgacgcgcccgcgccgctggcctttctttcggagccctgcccgttccgcgaagccgcgctcgcctcactggccggccatggcgcggcgaactggcagatcgtgctgaccgcgcagagttctggcgcattggtgtcggccgccgccgccgggctggccatcaccgtgctgacgccttccggcatgccggcgggcctgcgttccatttcgccggggagttttttgccggcgctgccgccggcgcggtttgtgattcagcatgccaaaagcggcatcgcttccgaagccctgtcagcgctggccgatgaagttcgcgaggcttgctttcggtggcgcggggcgcatgttcaagccgcgcgcggcgtaagtcgagcaaatgcgagaccggaaagcttggagtagcgctctaatacatcgcagcgcccgtccccacgcgcatcaaatccacagcagagccttgcttagttctgcctaaaaaccaaatatttacgacgttacgtttgaagatccaatattgaattcgcaagatcgccagagatcgcatttggcggctctaatccgtgttttctaaccgcccgctccaataccgccctcataagcttgaatatgtttctcggcgtcatttcaacaattctttcaagcaccgcatcgaccgcagcctccgaaaatggataatacaaactcggagctataaattcaggctttctaaatccactcaactgctcacgaacaaatttcttcgccgcctctggttccagtgctggcagttcgatgtatttacgagtaagtcgctgcaaaataggagttggaaggacagcctcaatcaacgcagcgtcagcgctaaaaccccaaatcatacaaaaataattcggcaactgattgaggagctcgcgaaaagactgtagaagttgaatcgactctaccgccttcatctcgaccaaattttcttgctcatcaacaaacaaataaacagcctcataggcagcccgttcattgccgatatcggaggtcataaccttaaaaaggcccgccagcgtagcaaccgccggatagtccgcatcaagagatgaattaagacctatatcgggaaagctgagtttttcacctcgcaagtatctccatacatcaaccagtcctccattggccgccttcagcaacaaatgaataaaaggagttaaagatggcggcacgtgttgtcctagcgtacgcgagaccaacaaacttcgatccgccatcagactcgaagcttcaatatgactcaaactctgaaggtaagctgtcgcggcggagttgacctgaacatttacatgcgccgccaaagttgagaaaaaatctcggccaagctgatcgattaatgtgcgataaacatcaacaaacgtaattttttgacttactcgaacagtttgcacgtagatagcttttcctttgaatcgctcgacctcatcttcgttaatcaaagtcgtgagataccgaagggcatgcgactttcccgccccatagtcaccatggactacaacaaattcacttgagccaatatcactggagcgaacactctcaaccacgtccagaagcaactccttttcccgctctcttccggcccacttatgaactgacaactctccgacggtaatcgcgaaagggtcagctatcaggccaaaatctccgatcgtactcatgcttttcctttagaggttaatttgcttgcttgccaaacgtagaacgggaaactcccaaaacccgtaaggcgcttaagctctttctccacagcagcctcatggtctggattgtcaatgcgaaccattgtttcgtcattgcgctcaaaacctccctgagtgaaattcgaacttccaataaacgccgtatatcgtttaggtgcgtcaaattcgaagtgaaacaacttcgaatgaagacttgtttcgcgaattttaaggctcactccttctgcttctagctgcgacgcctccgctcttcttatgacattttgctggccgaccgcggcatcatcagcaggcggacaggtgacaatttcgattcgatcggttccgcgagaaatagcatgccttgcaaactctagcaccgatgaccatggcttaacgggcgttaaaaatggagagacgattgttatagatctcggcccctgcgcaagagcatttcggaactgctgcgcaaaggggcgcgtgcaatggatttcaatctttgacattatttcgcaactgatagtatgccaatgcaccggtgcggctagcaaaaaacgcaaatcgtcctggacgtaaaaccgcgattgacctgaggacttcttcgaagcttactcgatagccatgctcgatctcacacaagatagtaaagtacattgcggcagcgaccgaagcttgcttagcgtggaatagtttaattttcgggaatgaatgctcaagaaaatcggcgaccttttcaagaaaatctctatgcggcgcaatctgtgctgattggggtcgaagcaattctagtgtcgaaccagaagcgcctttaagcacgagaggagattgcgggcgtaaaaactcgacgcattgaggatctggaccgatccatcctgaactgtcgcttggataacctgactgcgtgaggaacttctcccccatggccgtcaatttcgcattatccgcatcataatgtcctaactctacagcccatgttttgcgtggactaaaatgatgccgaccaaaatctgcgctcggcttttcaaagtcgaggcggccgagcctatcaatctttacccaatgcacctgatgagcgccacctttaatcaagcgagttagaactgatttatttggaaaggccgttgccaaccactcaagcctcaccgccctcattgccaagattttttggcgaaactcctcagcctgttcctcacttgtcttttttaagtcctgctttaatatctgaagaactgtcagataagcatcggcatcggcctcgagaattaaatgctcaagaacgatatttgccagtcgaaggtcctcattggacgccgcttttatagcaatcccgctatcggtaagcgcaaggcggctcaaatgcggcgcgttgctcgcacctggcaatttctgaattattccaagctcacccgagaaattcaatatttcaatagcgtatttatctgttaaaggctttccgtcgagtcctgttgcttggagctgcttagttagttcaaactgatacgctgtatgctgcttaaacagctcagcaagcagtgccattcgccggatgctatatgccccagtggtatatccaatttgccgcgtcagtgcatgcaccagctccgcttccgccctcgcccttgaataaacggttgccacgttaacttggggtgttcccaccgtgagctgtaactcggggccggattttggtggcaaaaactcgcccacttgctgcatcagccaatagacactctccaggatccaacgaccgcaggacactctgaatatcgataccctttgtggcgccaatgtcgtaagtaacggaagaccttgtcggcatgcgagcaactgcagcttgcagatctgcgtcaaagccaagatagtgagtaagtgttatatcaacttggctcatcaagcggggatcgactgcagaaggctgttgagtcgcaaacaccatggaaaggccagcatcacgacctcgctttacatagtcgacaacgggtccggttgcagaagtattccccgcagccggaacgacaacatgggcttcgtccagaaaaacccaaagacgatcgggcaattccgcatttaggctttcttttttcaagcggcgagcaacgcgcttttcctggtggtgataactcatgcgatccgaaaggagacgcacgagaactccgacaacgagcgatcttaagccttctcccaattgccgcatcaagattactgaaatacatcccggccttagcagctcatccaaagccacgccatttccgccgatcaattgggactcgactaaggattccaacctccaccgaagggagtcaacagtagaggcttgaaatttttgcaatggtccggcaggtagacagcgcagagccagcgattccggcgtgtcatgtggatacgccttgaccagagttaaaagcgcttgaccgatcggcgaaaagcgctcgatttctacaagggcgagccaatcgtcaccacgaagttgactcggcgcgatctgaagctccgcgacttggctaagcggagttttatagcctgccggcgcccagagcttcacagacgaagccgaggtcggggagtaaccccaagcttttattgcttgaatttgttctacatcttcagacagattttcggctggggtgtgcccaagagtccaaaactgatcttggacgtcgaaaatgacgcttgcggtcggttgtgtcttggtgccccagatgggcccggctccacagacgctctcggcaataacgcctagatcaaaactttttccactgccgcgcgagccaaagatcccaatgacgtgcgggaacgataggtcaagccaaacaccagcatcaagtacgcttgagccttgagcgttctcacagactttcccgagaagtccgacattggcgccgctttgccccaaccttcttccgactactactgctctgtcggccgaatccacgttcaaaaatgcagctgattcgtttgctcgtagagcagcagtcgttataacctttttagttttcaccaaagcgctccaagaaattttttccagccgacgttaaaacagatctccctggcagcaattgaacaaccagatttggttgcagctcgtgtaagagccgccgcggactcgctgtcgcaacgacgcacgccatcccttgttgatcagccaacaaacgaatctttttgcagacggaggcggctgacaaatcgtccaacggctcacagaacgcatcaataaatagcactttgggctcagttgtcagtgcccgcgctatccccaggcggtagagctgtccatcgctaagataggaggagggacgaacgaacagcgacgcctctgctaggccagcattggacaatgccaccaatgcagcttcgatggagacgtcgctcagcaggtcaatcggtgactcggcacttctttcggtcatcacccaagctgcctttgtttgccctcgaatctcgcccgttttcgcgcagacagaggctgggagctttccaagccctttttgtgcggcgtcagccattgctcttagcagtagcgacttccccgtgccgctcggcccggttatcaagataatttgaccttgcgaaacgttgaaactgagaccttcaaatagcggttgctcaagcgccttagaaacaatcccaaaggcttccgcaacttttctcgacctacccgtcgttgaaggctgagcacttgcgtgtagcgaatagttttcgatttctaataacggggtcatgcgcactctggttgctattttttttctttgaatggattttgattcatgagtttgcggtaccacagtttttaaatgcaaacatgcagcaggggtaagtccggcgatatacgtgggctttggcctgcggtatacatgatgcattgcaacccattcttcgtcggaaaggccttctgggctcttcctcaggacattcaataattgctccagcgaccactcacgtcgattcatagtggcgagcagcgttgtcgcgtaagaccgttgcaggtgcatgatcccaccgccaccctttggaaaattggtgtcatccccgctccttattgtgcgtcgcagcaggtaattcatgtcttttaggacacgcgcttcatttccttcagtgtctcccacatacttaaaacccgctccacgcacaaaaggcgtatagcgcagcatgtccgcggtaatttccaaaaacaaaggtctagctccaccgtagtgccaccgctccctcgtatagtttactgcggcctttgcaagaagcgctgcgatacccaatcctcggatttcaggatagacgacacaacgcgatatcctagcgattcgtttcgtctgctccttcgctgttttcatgtcccatcgctgccaaacaatatcgttttctgcgtccgagaacgggcgatcaagcaacggtttgcgcgcagtattaaccagaagagccgaggtaatttcgataaaacccacaacctctggcagcaagggatgatgcgcaaccgcaatcaacggagcgactcgcccagcgacattttgaccacgatagtgatggtgctttaatcttttcagagcataggcctctgcctccgtttcgacttctttgatggtgatttcaataatttcaccagacagccgaacatcgaaatgttcagaccaagccggagccagaggcacacttgtttttcgtttttctaaaatgacttgggggtatacccccttgaagaaaatttcatcgcctttcgccagcggagcaaatggtggcaattcaagaacagcacccgaggagagtttaaatttcgtttcattctcgcctcggtatcttgaatcaacaacctctgttggaccaaataaattctcaagaggcttgttcaaacgagtagttgtgccgacggacataagataaatttttgggaggggtgatatcagtcaacgagggtattttgaaaattggaagcccgtttaaagcctgacattcaatttattagtttcgccacgcaccccttctaagccacccttcagtcttgtagcggaagtccattcgacgtatctatgccgttaccgacatgcgaggcgccgtgcacacatgggtatggcggatgcgtatgcagtggcggatccggtaagtcacattttgtcatccgcatgttctcatcctttgggagaggacagcacgctgaactcacgcaatagccggcaaaaggttgaagcaacagggtctcaccgtctcggcgattcgggccccgaatgctgcgaccgcttcgcgaaggcccggctcgggtgctaactacgccgggaaaggcgttaacttgggtcggggcaacagtgctccttgtaacgtcggccacctggatcacgtctgccccctgcaatttccggcagcggtactgaaaagtcccgacatgagatagctgcgggccaaggagatgcgcttaggcaaaaagaaaacccgccacgctagcaagcgtgcgggttcttaggggttgatgagaccccatggtctcgatatttggtcccgccgccaggaatcgaacctggatctcagccttcggagggccgaattctatccgttgaaatacagcgaggaatctgggctccggcagaaccggagccacgcattatcgcccatcagacggcgacttcttcatcagcttcgttcccgatgcctgctttcgagttccgcacaaagcccaggccggccaggtagacgcggaaggtgcgccggccggtgggcaccaggtcgaaggcctccgggtcgagcagccagttctggatgagcccgctgatcagcgcgtgcaggccctgcgccgccacgtggccgggcacgggcagcttgatgcggtcgcggcgcgctgccgtgcgcagggctttttcgaaatcggccacgcaggcgttgcgggcgtccaggtggcgctgctgcaccgaggccatgtcgtgcgtgtattccaccttgtgggtggccacgtcgaacacgcggcgcacctgggggtcggtggtcatgagggtcagggcgtgcaccatgccctcttcgatctcgcccagggggtcgtcgttgaggccggccgccgcggcggccctggggccggcttccagcggcaggatgacgcgctccatcatggcgttgaagaggtcggccttgtccttgaagtgccaatagatggcgccgcgcgtggccccggcctgctgcgcaatctgctgcagcgaggtctgcgagacgccttgcgcctgaaacagcagctccgcggcatcgagcaagcgatgccgcgtggccagtgcctcttccttcgtacgacgtgccaccaagtctcccgttttgtaaagccaagccctttcggtatcgtggggccattggggttgtcactatacatccatgaatgtatgtaaactagcgggcttccccgatggcccagctgtttacgctggttttctgttcgcttcgcgaacacgccgtctcccgtctttgcttcaaaggattcgcatgcctctcctgcatgtttcgcgtcaatcgtcgttttcgccgcgcctcgcgatcgtggccgccgccgtggtgttggcgcttgcggcctgttccaagggcgacgcgccagccgggcccggcggcgcgggtggcggcggtgcccggcccgctcctgaagtgggcgtggtggttgccacgccaaccgacgtgggcctggtgacggagctgccgggccgcctggaggcctcccgcgtggcccaggttcgcgcccgcgcctcgggcatcctgctgaagcgcgagttccgcgaaggcagcgacgtgaaggccggccaactgctgttccgcatcgatccggcgccgctggtggcggccgcgcagaacgcgcaggccacgctggcccgggccgaagccaacgccgtgcaggccaaggcgctggccgaccgctacaagccgctggtcgaggccaatgccgtgagcaagcaggaatacgcgaccgccgtggcctcgcaaaagacagccgaggccgacgtggccgcgggccgcgccgcggtgcagaccgccaagatcaacctgggctacgccaacgtgacctcgcccatcgcgggccgcatcggccgtgcgctggtgactgaaggtgcgctggtcggccagggcgacgcgaccgaactggccgtggtgcagcagatcagcccgatgtacgtgaacttcacgcagtcggcatccgacgttctgaagctgcgccgcgcactggccgcgggccagtacaagcgggccaacggcgaagaagccgccagcgtgacggtggtgctggaagacggcaccgagtacgcgctgcccggcaagctgctgttctccgacctgacggtggattcgaccaccggccaggtgacgctgcgcgccgaagtgcccaaccccaagggcgagctgctgcccggcctgtatgtgcgggtgcggctggagcaggcgcaggccagcaacgcgatcaccgttccccagcaggccgtgacgcgcacccagcagggcgacacggtgtcggtggtgggcgccgacggcaagatcagccagcgcaccgtaaagatcagcgccgccaaggacaaccagtgggtggtgctcgatggcctgaaggccggcgagcaggtgatggtcgacggcttccagaagctgcagatgatgccgcccggcacgcccgtgaaggcagtgccgtggaagaagccgacgccgaatggcgcggcgcaaccggcagcacaaccagcggcgcaggcggcatccgccccggcggcggcagccagcggtccggcgtctgccacggccgagaagaagtaatcaggagcgcgcccgcatggccaaattctttatcgaccgaccgatcttcgcctgggtgatcgcgctgttcatcctggtgatgggcggcgtcgccatcacccagctgccgatctcgcagtacccgccggtggcaccgccggccatcgtgatcaacgtcgcctatccgggcgcctcggcccagacgctggaggacagcgtgctgtccgtcatcgagcgcgagatgaacggctcgccgggcctgatctacatggagtcggtggcccaggccgacggcacgggcaccatcaccatcagcttccaggccggcaccaaccccgacctggcgcaggtggacgtgcagaaccggctctcccgcgccacgccgcgcctgccggccgccgtgacgcagcagggcgtgcgcgtggacaaggcgcgcaacaacttcctgctgtttgcgatgctgtcctcggacaacccggacttcaccccggtggcgctcggcgactatgccgcgcgcaacatcgtgcccgagctgcagcgcgtggtgggcgtgggccaggcccagctgttcggtaccgagaacgccatgcgcgtctgggtcgatccggccaagctgcagggcttcaacctgtcggccaccgacgtgaacaacgccattcgcgcgcagaacgcccaggtgtcctcgggctccatcggcgacctgcccaacattcccggccaggccattgcggccacggtggtggtgaacggccagctcgccaacgtggagcagttcaagaacatcattctgcgagccaacaccgacggctcggccgtgcggctgaaagacgtggcgcgggtcgagcttggcggccagtcgtatgccacctcggcgcgcctgaacggcgtgcccgcggtcggcattggcgtgcagcccacgcccaacggcaacgcgcttcaatcggccaaggcgatccgtgccaagatgaccgagctcgagcgcttcttcccgccgggcgtgaagtggaccattccgtacgacagctcgcgcttcgtgcagatttccatcaccgaggtggtcaagacgctgctcgaagccgtggcgctggtgttcgtggtgatgttcctgttcttgcagaactggcgctacacgatcatcccgaccatcgtggtgcccattgcgctcctgggcacgttcgcctcgctgctcgcgctgggcttctcgatcaacgtgctgaccatgttcggcatggtgctggtgatcggtatcgtggtggacgacgccatcgtggtggtcgagaacgtcgagcgcatcatgagcgaagaggggctttcgcctctggaagccacgcgcaaggccatgaagcagatctcgggcgccatcatcggcgtgaccgtggtgctgatctcggtgttcgtgccgctggcgttctttgcgggctcgaccggcaacatctaccgccagttctcggcggtgatggtgacctcgatcgccttctcggccttcatggcgctgtcgctcacgcctgccctgtgcgccacgctgctcaagccggtggaagctggccaccaccacgagaagaccggcttcttcggctggttcaaccgtggcttcacgcgcaccgccaagggctatgaaagcctggtcgcgcgcattctgcgccgcgccgcgcgctacctgatcatctacgtggcgatcatcggcgcggtggtgttcacctacatgcggctgccaagctcgttccttcccgcggaagaccagggcaacatcatcgtgaatgtgcagctgccgccgggcgccacgcaagagcgcgcactgtcggtcatgcagcaggtcgaaggcttcatcctgaagcagcccgaagtgcagagcatggtgggcgtgatgggcttcagcttctcgggccagggccagaacgcgggcctcgcattcgtgacgctgaaggactgggacgaacgcaaggacccggcccaatcggcccaggcgctggcgggccgcgccttcggtgcgctctccggcatccgcgacgccttcatctacccgctgagcccgccgcccatccctgaactgggcaatgccagcggcttcagcttccggctgcaggaccgctcgggcgcgggccacgatgcgctcatcaatgcgcgcaaccagctgctgggcatggccgggcaaagcaagatcctgtcgcaggtgcgccccgacggcctggaggacgcgcctcagctgcagatcgacatcgaccgcgacaaggcgaacgccctgggcgtgaccttcgacgcgatcaacgcgacgctgtcgaccggcctgggttcgagctacatcaacgactttccgaaccgcggccgcctgcagcgcgtggtggtgcaagccgatgcgccggcccgcatgcagcccgacgacctgctgcgcctgaacgccagcaacacgcagggccagccggtgccgctgtcggcctttgccaccaccaagtgggtcaagggcgccacgcagacggtgcgctacaacggctacccggccatccgcatcagcggcgacgccgccgcgggcttcagcacgggcgcggccatggccgagatggaaaagctcgccgcccaactgccgcaaggcttcggctttgaatggacgggccagtcgcgcgaggaaaagctggcaggttcgcaggccatcgtgctgtacggcttcgcgatcctggcggtgttcctgtgcctggccgcgctgtacgagagctggtcgatcccgctgtcggtgattctggtggtgccgctgggcgtgctgggcgtgctgctggcaaccatgctgcgcgcctactccaacgacgtgtacttccaggtgggactgatcaccatcatcggcctctcggcgaagaacgcgatcctgatcatcgagtttgcgaaggacctgcaggcgcagggcaagggcatcgtcgaatcggccctggccgcggcccacctgcggttccggccgatcatcatgacctcgctggccttcggcctgggcgtggtgccgctggtgatcgcctcgggcgccggctcggccagccagcgcgccatcggcacgggtgtgctcggcggcatggtgacgggcacggcgctggcggtgatcttcgtgccggtgttcttcgtggtggtgcgcagcctgttcaagggcagtgcgcgccagcatgaagccgacaagcggcatgcggaggcagccggcatcacggaagaaaaagcaacatgaccaagaaactgatccccacagccctggcagcggccatgctgctggccggctgctcgctgattccgacctacgagcgccccgcggcgccggtgccgaccacctttccgggcgatccggcgcagccggccggccaggccgcggcggccgtgccgtgggaagacttctttaccgacgcgcggctcaatggattgatccgcaccgcgctggagaacaaccgcgacctgcgcgtctcggtgctcaacatcgagcaggcgcgcgcgcaatttcaggtccagcgctcgtcgctgttcccggcggtcggcctcacgggcagcggatcgcgctcgagccccaacccctaccaggcgttcgacagcagcgtgggcagcgtgtcgtcgcagtacagcgtcaacctgggcatcacggcctgggagatcgacttcttcggccgcatccgcgcgctgaaggaccaggcgctgtcgcaatacctggccaccgaggaatcgcgcaaggccgcgcaggtgagcctgattgcggcggtcgccaccggctggctcacgctgattgccgacgacgaactgctcgaactcacgcgccagacgctggtcacgcgcgaagaatcggtgcgcctgaccaagatgcgcttcgacaacggggtttcgtccgagctcgatttccaggccgccaactcgcttgccgaaaccgcgcgcgcttcttatgcgcagcagcagcgcacgcgcatgcaggacgagaacgccctcgccctgctgctgggcgcgccggttccggccagcgccacggcaggcggggtcaagggcctggacagcgtgcagccgatgcccgacgtgccggccggcctgccctccgacctgctggccgagcggcccgacatccgcgcggccgagcagcagctcattgcggccaacgccaacatcggcgcggcgcgcgccaacttcttcccgcgcgtgtcgctgaccaccacgctcggcaccgcgagcagcgagttctcgggcctgttcgacagcggctccaaggcctggtcgttcgcgccgtcgatcacgctgccgatcttcgacgcgggccgcaaccgggccacgctcgactcggccaaggccgggcgcgagattgccgtggcgcagtacgagaagtcgatccagaccgcgttccgcgaagtggccgacgccctggccggccgcgccacgctgggcgagcaggtgcgtgcgcagcgcgcgcaggcggacgccgagtcggtgcgcttccggctttccgacatgcgctaccgcaacggcatcgcgagcgcgctcgacctgctcgatgcgcagcgctcgctctacacggcccagcaatcggccgtcaccacgcggctcttgcagctgcagaaccaggtcacgctctacaagacgctgggcggcggctgggccacgcgcaaggctgggtgaacgccgcctgaagcgccttcttcggcgctggtctgggctcgttgcgtcgaggcatcgcggagaggccttccgtcctttaggcggagggcctctctataatcgccggttgattcgaaaaagccccccgacgagcccccgttattgaggacgccaatgagcgcagacccgcattaccaggccaaagaagaagcccattccggcccgatcaagaacccgaagcaactgctgctcgcggtatttttctccttcgttgtacccattctgatcatcgtgggcctcgtggcctatgtggtttcggacaccaagcccgcgggcacggccgagggcgacaacatggcgctctacggtgtctccaaggatgcgcgcgaccgcgaagtggccgagcggctcaagaaggtcggcgccatcgagatccgcgatgccaaccgcccgctcgcagccggcgatgccgttttcaaggcgcaatgcgcggcctgccacgccgcgcccggcattcccggcgcgccccacctgaacgacgccgcggcctggggcccgcgcatcggccagggctacgcgacgctgctcgaccatgcgctgcatggcaagggcgccatgccggcccagggcggcggcgacttcgaagacctcgaaatcggccgtgccgtggtctacatggccaacgccggcggcgccaagttcccgatgcccgatcgtcccgcagcagcagcagccccggccgcgggcgctgcctcggcagccgcaccggcggccagcgcaagcaagtaagcgctacttcactgccaaagagaaagccggcttcgagccggctttttcatgggcgacgcaaagtcgcggcggctactttgccatggctgcgagccggcgcgccgccgggctcagcacatggccgaagcgctgcggcaagtcgcccgcgtgcactgcctcgggagtccacaggccctgctccacggcttcggccgcaaggccaacgtccagcgtatggaccagcccgagcccgagcggcgtggcaaggtagaggcggccctgctcgtcgagcaggcaggccgtgatgctgtcgaccggctgccccgtgtgggcggtgacggcaaagcccttgtcgtcggcaacacgccagacgaaaggcgcggcctccagctcgacgtagacgcgctgcggcccattctgaaagaaccactggccctctccgtcatggtcgtagttgcgctggatgaagtcgatcagcttctcgtgccgcagcatcgaacccttctcggtcgggaatggacccacggcctgcgtgcggtcgtcgcgcatgtaccagttgccgcgcgcgtccaggccaagccagccgtagcagtgcggcacgttgggccacttggcgagcgcctgtttaacgatgtcgtccatgaaagctattgtgctcgcccgcgcgcggaatgggggctgcaaactggctgagccagccgcccactcgctccggcatgccccgcacgtgccctggcggcaccccgagcggaaaacccacgtggccgccgtgcgcgggttgccacagcgtcacgtacgggccgacctcgccggggcccggcaggctgctggccggaatgaacggatcgttgagcgcattcaccaccagcgtgggcacgcggatcgcgcggaggtgcggcttggacgagccccgtgcccagtagtcgtcggtgttgcgaaagccgtgcagcggcgcggtgaacacgtcgtcgaaggcatagagatcccgtgccgcgagcagccgctcgcggtcgaacagcccgggaaactgcgccagcttggccagcgccttgggcttcatggtcgagaggaacatgcgcgtgtagaccagccggttgaagccgcgtccgatggcctggccgccggcggtcaggtcaaccggcgcagacaccgaagccaccgcattgaccgaggcgcgggccgtctcgccggcctcgcaggcccagcgcaacagcgcgttgccgccgagcgagacgcccgccgccagcaccgggccgccgccgcgcagcgcatgctggccgtgcatgcgccgcaggatccagccgatctcttcgtagtcgcccgagtggtaggcgcgcggcgccaggttcatctcgccgctgcagcccctgaaatgcggcaccgcgaaggccatcccgcgcgcggccgcaaaggccgcgaacgcctccgcatagtggctgcgggaagagccctccagcccatggaacagcaccagcagcggctgcgggccgggcaaggccgcatcgacgaaatcgacgtcgatgaagtcgccgtcgggcgcggtccagcgctcgcggcggtacaagggcgccggcccgtcgaagcggcgcgcatacagcgccggccagatggtctgcaggttgccgccgggcagccaccggggcgccatgtagcccatggacgaattcatggagggtgaagagggcgcgtcggcaggcatcgatcagtgcagggtctggggtggatcgttcgaatcgctgggctcacgcgcgctgccggggctcgcatggtgggccaccaggcgccagccttccacggtcttgtgatagacgttggtggccagcacgaaggcgtgcttgggtccttcggcggtgagcacctcgatgcgttcgagcacgttgtgcaccgcgctcgcaagcgactcgatcttgcgcacgcgcgccggcgtcgcatggatggcgccgttgccgaacatctgctcgaaagccgtgcggatggcggtggccccgaccagccgcggcccgcccggatgaacgcagaacacctcgtcctcgtcggcccagcaggccatcaatgcgtcgatgtcgccgcgctgcagcgcttcataaaaggccgcctcgacgtcgtcggcagtgccgccgatggccgcggcggcgcggagtggggtcttgggcatggcgtgattttgccgcgcgatccgtgacgcggagaccgcaccgctttggctccgcgcgcaccgggctgccgcaagcgcggagattcaaatgctccactttggaccaaatggtcaaacaaacacatttataaacagtcaagctattgatttaaaacaactttcttctttggcacggcctatgcatagggctttcggaccttgcaacaggagcttctgcatgaatgtcggcatcttcattcccatcggcaacaacggctggctgctttccgaaaacgcaccgcaatacaagccgagtttcgaactcaacaaggagatcacgctgacagccgagcgctacggcgtggacttcgtgctgtcgatgatcaagctgcgcggcttcggcggcaagaccgagttctgggaccacaacctcgagtcgttcacgctcatggccgggctcgcggccgtgaccaccaagatcaagctctttgccaccgccgcctcgctggtgatgccgccggccatcgtcgcgcgcatggcgtcgaccatcgattcgatctccaacggccgtttcggcctgaacctcgtcaccggctggcagcggcccgagtattcgcagatgggcatgtggcccggcgaccagttcttcggcacgcgctaccagtacctctcagaatacatccaggtgctgcgcgacctctggggcaccggccagtcggacttcaagggcgcgcacttccagatggacgactgccgcctgagcccccggccccaggccgacatgaaggtgatctgcgcgggccagagcgacgccggcatggacttttccgcgaagtacgccgactacaacttctgcttcggcaagggcgtgaacacgcccaaggcctttgcgcccgcggccgagaagctcatcgaggccacgcgcaagaccggccgccacgtcaccacctatgtgctggtgatggtgattgccgacgaaaccgacgacgccgcgcgcgccaagtgggagcactacaaggccggcgccgaccacgaggcgattgcgtggctcggccagcagggcgcggccgacaccaagtcgggcgccgacaccaacgtgcgccagatggccgacccgacctcggccgtcaacatcaacatgggcacgttggtcggctcctatgccaccgtggccggcctgctcgacgaaatggccgaggtgccgggcaccgaaggcgtgctgctcactttcgacgacttcctgcagggcgtgcaagccttcggcgagcgcatccagccgctgatgaagagccgcgcgcacgtgcagagccccgtggcctcgcaggccgaacccgagcgccttgcggcctgaagggaacgaagcgcatggccacgcccgcacgcaacaccacgctcacctcgaccacccccgtcggtgccccgcgtctgcccggcgcacccgcgccgatggtgctgcccgcgcggcccgaaccactcgcgctgcatgccaccgattcagccctggtcgtggtcgacatgcagaacgcctatgcgtcgatcggcggctacgtcgactcggcgggcttcgacatttcaggcgcgcagggcaccatcgccaacatcgcgcgcgccattgcggcggcgcgcgcggccggcatgctggtcgtgtttctgcagaacggctgggacgcggcctacgtcgaagcgggcggcccgggctcgcccaactggcacaagtcgaacgcgctcaagaccatgcgcgccaagcccgagctcgagggcaagttcctcgccaagggcggctgggactacgaactcattgaccagatgaagccgcaacccggcgacatcgtggtgcccaagacgcgctacagcggcttcttcaacagcacgctcgacagcaccttgcgctcgcggggcatccgccacctggtgttcaccggcatcgcgaccaacgtgtgcgtcgagtcgacgctgcgcgacgcgttccacctcgaatattttgctgtgatgctcgaagacgcgacgcacgagcttggcggtgcggccatacagaaggcgtcggtctacaacgtcgagaccttcttcggctgggtctccacggtggaccagttctgcgccacctttgcgcccgaacctgtcgccccgcctgttgcggccgaagcggccattgcctgatttttttcaaaggagcccacaccatgcccaagcaagccatcatcccggccggaaccaccacgcccatcgccccgttcgtgcccggcaccatggccgacggcgtcgtctacgtgtcgggcacgctgcccttcgacaaggacaacaacgtggtgcacgtgggcgacgcctccgcgcaaacgcgccacgtgctcgagacgatccagaacgtgatcaagacggccggcggcaccatggacgacgtgaccttcaacatgatcatgatcaaggactgggccgactacgcgaagatcaacacggtgtatgccgagttctttccgggcaccaagcccgcgcgctattgcatccagtgcggcctggtcaagcccgatgcgctggtcgagattgcctcgatcgcccacgtgggcaacaaggcctgaacatgccgccgctgcactacgaagtgcatgggccggccgatggcgaggctgtgctgctgtcgtcggggctcggcggttcggccgccttctggcaaccgcagcttggcgcgctggtcgaagcgggccatcgcgtgattgcgtacgaccagcgcggaacgggccgcagccccgccgcgctcgacgcgggctacgccattgccgacatggcgcgcgacgtggtgcggatcctcgacgccacgtcgacgccgcgctgccacctggtgggccatgcgctgggcgggctcgtcggactgcagcttgcgctcgacgagccctcgcgcgtggccagcctggtgctcgtcaatgcatggtccaagcccaacccgcattcggcgcgctgcttcgatgcgcggcttgcgctgctcgatgcctgcggcccgcgtgcgtacgtggaagcgcagccgatctttttgtatcccgcggcctggtgcgcggagcacgcgcagcgcgtggccgatgaggtcgaccatgcctttgcgcattttcccggcgaggccaacatgcgtgcgcgcattgcggcattgcgcgccttcgacatcgacgcgcgcctcggcgacatcaccatgcccaccttggtggcggccgccatggacgacgggctggtgccatggacctgttcgcagcgcctggccgacggcctgcacgacgtcacgctccacttcatgccgcacggcgggcacgcgcacagcgtgaccgaggcggacgccttcaaccgcagcctgctcgactttctttcccgggtcagcgcacccggcgttctcgcatgaccatcgcctccgcccccgctctcgacgacgccgcactggcgcttctttttaccgaagcacgcagccacaacggctggaccaccgaacccgtcacggacgcgcagatccggcagatctacgcgctcgcatgcatgggcccgacgtcggccaactgctcgcccgcgcgcttcgtgttcgttcgcacgcccgaaggcaagcagcgccttgcgcctgcgctttccaagggcaacctcgacaagaccatgacggcgccggtcaccgtgattgccgcgtgggaccgcaagttctacgacaagctgcccacgctgtttccgcacgccgatgcgcgcagctggttcaccggcagccccgaggccgcacatgaaaccgcctttcgcaatgcaagcctgcaggcaggctacctgctgctcgccgcacgcgccgtggggctcgatgcggggccgatgtcgggcttcgacaaggccaaggtcgatgccgcatttttcgagggcaccgactggaccgccaacttcctgatcaacctcgggcacggcgatgcggccaaggtgttcggccgcctgccgcggctggccttcgacgacgcctgccttctcgcctgacgcccacgggagtttcttctcatgctgctgaacgcaatggcttccaacaacgtcgcgccaggcggcgcgccgcacgtgctgcccaaggccgactaccgcaatgccatggcgcggctgggtgccgccgtcaacatcatcaccaccgacggcccggccggccgcgccggcttcacggcctcggccgtgtgcagcgtgaccgacgagccgccgatgctgctggtgtgcctgaaccgttcggcctcggtgtaccccgcgttcacggccaacggcgtgctctgcgtgaacgtgctggcggcaggccaccagtcgctctcgggcctgttcggcggcaagacgccgatggacgagcgctttgccgccggccgctggagccgcaaggccaccggctcgccggtgctcgaagacgcggcggcctcgttcgactgccgcgtggtgcgcgccaccagtgcgggcacgcacgacgtgctgttctgcgaagcggtggcgattgcgatcggcggtgcggcgcagagtttgatttatttcgatcggcgctatcacgagatagcaacgccgccgcactgagctggtcttgttccctctcccttgccttgtcccctctccctctgggagagggttagggtgagggcagcggccttcgcaatctcggcgaatctctaagcgccgctgaccctcaccccagccctctcccagagggagagggagtaattcctaacgcggcgcaatcccctgcagcacgatccgctgcacgttctccaccgtctgctcgaagaacgccgcatcttccagcgtatgccccgtcagcgcctgcacctgcacgccgaaatccgcatagtgctgcgtgatggcccagagcgcgaagatcaaatgatgcggatcgaccggcgcgagcttgccggcctcgatccatgaacggatgacctccgactttcgctccaccagcgtgcgcaattcgcgatcgagttcgtcgcgcaggagcggcgcgccctggatcatttcgaggcagaacaatcgtgatgcatccggccggtcgcgcgagatcacgagcttgcggcggatgtagctgccgatggcttcgcgcgggtcttgctcggcactgaatccgcgcagcggctcgagccacagttcgagcaggtcgcgcagcacgctgacgtacagctcctccttgttcgcaaagtaatagagcaggttgctcttggacacgtcggcgcgcgccgccacctggtcgatcgacgtgccgtgcaatccgaagcgcgagaacaagcccagcgcggcgccgaggatggcgctgcgcttgtcctcgatctggcgcagcctgcggctcaccgcggacgcgctgcgcaccgccggttttgcgcgcttgcgcgccgggctggtcttctttgtgctgctggctgcggccagcgccttggtcttcggcatcttccctcgcttctcgattgcggactcttctttcaacgcgcaccactgtaaggccgcggtgcatcgcgacgcgccaagccaacctttgaagcccctgcgcgcgcaccatgctgacgcggtaaatgcgttttgtccatttggtccaactggcacagacgttgcatggcgaaaggcatgccaagcacgaggacgaccgacacatgacgctcctgtccgtacccatcatcgatctcgcgccctactttgccggcacgcccgaaggcaaggccgaggtcgcggcaaaggtcgacgaggcttgccgcagcatcggcttcctcgtcatcacgaaccacggcattccggccgagctgatcgcgcgcgtgtcgcagctctcgcgtgcgttcttcgacatgccactggccgagaagcgcaaggtcgatcggccgcgccaggatgccgtgcgcggctacagcgctgtcggcgaagaaggcctttcctacagcctcgaagaagccgcgcccggcgacctgaaggaatcgttttcgatcggcccttcgaacgtgccggacgacgactaccaccgcggacccgccgctggcccgcacttcgagcccaacagctggccgcccatcggcggattccgcgaggcgtacgagagctacttcgaggccatgagcgatctctcgcgctcgctgatgcgcatcttcgcgctcggcctttcgctcgacgagccgttcttcgacgacaagatcgacaggcacatcagcatgttccgcgtgctgagctatccgccgcagcgcgaagcgccgctgccgggacaactgcgcgccggcgcgcacagcgactacggcagcctcaccatcgtgctgcccgacgacaagggcctgcaggtgttcaacaaggcgggccagtgggtcgacgtgccgcaggtggaaggcggactggtggtcaacattgccgacctgatgatgcagtggaccaacgaccagtgggtgtccacgctgcaccgcgtggtcaacccaccctttgacgtggcaagcaccaaccgccggcagtctctggtgttctttcaccagcccaactacgacgcgatggtcgagtgcctgccaagctgcctcgcgccgggcgaagagccgaagtacgcgcccatttcatcgggcgaccacctcacgtcgaagttcgtcaagcagaccaccttcggcggcaccaaggccgtggcctgagcatggcgcatctgtcttacgtcaacgtctttgcaaaagacgtggttgcgctcagcggcttctaccagcacgtgttcggcttcgccgagatcgaggcgatccgatcgccgatctttcgcggactcgacaccggcaagtcgagcctcggcttcaacgcgctcgaggcctacgagctgctgcacctggccgagttctccgacacgcgaggcgtgaagttcctgctgaatatcgacgtcgacagcaaggacgacgtggaccgcatggtgccggtcgcgctcgaggccggcgccacgctggtgaagccgccctacgtcacctactacaactggtaccagtcggtgctgctcgatcccgagggcaacgtgttccgcatcaacttcatgatgtgacggcacgcggtggcccgcccctccttctttcttccttgacacgctcctcacgaaaggtcgctccatgctgcgcaatcccactcacggcttcaccttcggccttgcactgtcgctcgcagccggcggcgcgacgttcgcgctgcccgccatggcggccgacggcttcacgctgaaggacaagccgaagatcgcgatgctctatttcggcccgaagaacgacggcggctggacgcaggccttcgacgaggcacgggcaaaggtcgagaaggaaatcggccagaagatccagtttgtcgagaacgtgcccgaagacgcctcggccatcaagccggcagccgagaagttcatccagcgcggcgccaacatcgtgatcggcacggccttcggctattccgacagcttcaaggacctggccgccaagtaccccggcgtggcttttctcaacggctcgggcactaccaacggcagcaacctcgaatcgttctacggccgcacctacgagagccagtacctctgcggcatggccgcgggcgcggcctccaagaccggcaagctcggcttcgtcgcggccaaccccttcggcgtcgtgaactggaccatcaacgcctttgcgctgggcgcgcagaagatgaaccccaacgccacggtcaacgtgatctataccggggcgtggaacgatcccgtgaaggaacgcgccgccgccgccgcgctgatcgaccagggcgccgacgtgatcggccagcacgtcgactcgcccacgccgcagatcgtggcgcaggagcgcggcgtgtacggcaccggccaccaccgcgacctgcgccagttcgcgcccaaggccacgctgtgctcgtcggtgtgggtgtgggaccgcttcctgacgcccgagctcaagaagatcatggccggcaactggaagcccgcgccttatggcgccttcatcgagatgaaggacggcggcaccgacatcgcgggcttcggcccggcggtgcccaaggacaaggccgcacagatcacggccgagcgcgacgccatcatgaagggcaagcaggtctacgccggcccgctcgccgaccgcgacggcaaggagcgcgtggccaagggcgcggtgctgtcggacgccgacctctggaagatggactggttcgtcaagggcgtggtcacgcagaagtaagtgcaggcaggcaggcagtgtccaacgcgctcgagctcaccggcatccgcaagtccttcgacggctttgcggcgctgaccgacgcgcacttcgaagcgcgctggggcgaagtgcatgcgctgctcggcgagaacggcgcgggcaagtcctcgctcatgaacatcgcagccgggctctatgcgccggaggccggccagctgctggtcgacgacaacgtggtgcgctttgccggaccggccgatgcggcccggcaccgcatcggcatggtccaccagcatttcaagctggtgcggcctttcacggtggcagagaacatcttgctcaccgcgccggcgcctgcggagtttcaaagccacggggaacgcttgcgcgagatctcgcgcgacatccgcaacaaggcctcggaactgggcttcgagatcgatcccgccaaacgcgtcgatgcgctctcgattgccgagcagcagcgtgtcgagattctcaaggtgctgcttgcgggtgcgcgcatcctgattctggacgagcccactgcggtgctcaccgaccaggaggccgcgcgcctcctgcggacggtgcgggggctcgcacgcgccggttccgccgtggtgctggtcacgcacaagatggccgacgtgaagacgtacgccgaccgcgtgacggtgatgcgcggcggccgcacggtggccactctggagccgggcgccacgccggtggccgagctggtaaagctcacggtcggcgaatccatcgcgacgcagggcttccaagcggcgacgtcgccgcgcggcccggtgcggctcacggtgcgcggcctgcgctcggcggcgtcggcccagggccgccgcgtgctcgacggtgtcgacctccaactgcatgccggcgaaatctacgggctggccggtgtcggcggcaacggccagggcgaactggccggcgccatcatgggcctgcccgatgccggcggcgcgctcgaaggcgagatccatctcgaaggccatggcgatctcaaggccatgggcgcgccggagcgccgcaacgtgggcattgccgcgattccggccgaccgctacgggttggcgctcgcgggcagcctttcggtggctgagaactacgccatagggcgcgtgcacacggggcgctacggtcccgcctggcatctgcggcgcggccgcatccaggacgacacgcgggaagcggtgcgcgccttcgatgtgctgggggtgcgctcggtggcgcagaaggccgcgctgctctccggcggcaacgcgcaaaaactggtgctcgcgcgcgagttcggcaagtcgccctcgctggtgctggcgcacagcccgagccgcgggctcgacgtgcgtgcgagcgccgaggtgcatgcgcgtctgcgcgccgcgcgcgatggcggtgccgccgtgctgctgatcagcgaagacctcgacgaggtactgcaactcgccgaccgcctgggcgtgatgacgcgcggccgcattgccggcgagtttgcgcagcccgccgaccggcaagccatcggacaggcgatggtggaccatggctgacgcatcgctcgcggccattgccgaggcggcgcaaaccagtccggaggccgcgcaccgggcgcggcgccaaccgctggcaggccggcgctatgcgctcgagatccgccagcacatggcatggcggcggcaggcgctgatccttgcagcggctctcctggtcgggcttgcgatatccgccgccatcctggtggcggccggcgtgcccgcggacgagctcgccaacgagttcgtgatgcagactttcttcgacggccagaactttcgcgccgtgctgttccaggccgcgccgatgatccttgtcggcctggccggctcgctggcgtttcgcgcgcgcttctggaacctggggctcgagggccagatgatctggggcgccatcggcgccacggccgtctcgatctggcagatcgggcccgaaccgctgcgcctgccgctgatgttcgcggccgccatcggctgcgggctcgtctgggtgctggggccggcgtggctgaagatcaggctcggcgtgaacgagatcatctccacgctgatgctcaactacatggcggccaacttcctgctgcacctggtctatggcggctggaaggacccgaaggacaactttccctattcgccgcagttccgcgccttcgagcggctgcccgaactgggcgccggcgtgagcagcgcgatcgtgctggcggccgtggtggcgcttttcgcgtggtggctggtgggcgtgagccgcgccgggctgtacctgcgcttcgtcgatgccaatccgcgcgtggcgcatgccaacggcgtgccggtgcgccgcaccatctatggcgccgtgctgctgtcgggcgcgatggccgggctggcgggctttgcggtggcctcgggccaggaagggcggctcacgcaggccttctaccagggctatggcttctcgggcatcctgattgcctttctcgcgcgcaacaacccgctcgcggccaccgtggtggcgctgctggtggcggccttgttcgtcaccggccgcagcctgcaggtgttctaccaggtgccgttctcgatggtgcagctgatccaggccatcatcgtggtgtgcgtggcgtcgagcgatttcttcattcgccaccggctgcgccgcgtgggcggggaggcggcgcagtgagcagcgctattgcactcaactggctcgcgagcacgccagattttgcggtgccctatgcgcttgccgcgctcgggctcatcatcagcgagcgcgcgggcgtgctctccctcggcgccgaagggctgatgctcgtcggtgcgctggccggcatcggcgcacagctggcgctcgggcagccggccgtgtcgctggtgctggccatgctcgcggccagcgcggtctcgctgctgttcgcggtgatggtgatctggctgcgcgtgaaccaggtgatcgcggggctcgcgctggtgttcttctgccagggcctcacggcgctcgtcggctcgctggccgaatggaccaaccacgccaccgaaggcatcggcggcatggcgctgtggccgctgtcgctgctgcccggcgtgggccggctgttcgagcagaacgccatggtgtggctcacgctgccgatcttcgttgcggtggcctggttcttctcgcgcacctcggccgggctgcggctgcgcgcggtgggcgagaacccgcaggctgccgatgccgccggcctccgcgttgccatgtggcggcttgccgcggtgctcgcgggcgcggcgctggtgggcctggccggcgcgtacatctcggtggtcagcaccaagctctggatcgccggcatgaccggcgggcgcggctggatcgccgtggggctggtgatcttcgcgcgctggtcgccgtggaaggcgctggtgggggcgctgctgttcggctgcatcgaggcgctgattccgcaattggccgcggccggcgtgcagctgccgcagtacttcgtgatgatgacgccgtatgccgtgacgctcggcgtgatggtctgggtcgcactgggccggcgcggcggagacgacgagcccggcgcactcggccagccctatgtgcgggaggaacggcgatgaaggcctgggtctacgacgaagagcgcgagctcgacgcggcgcagttcgccgactacctgaacccggccaccaccgcggccatctggacgacagccccgactgcccgtgccccgcgccgcgggcgcgcgacgtggtggcgcccatcgacagctttcatgattcggcgcgcgcgctgggcattcgcatcgtgcacgtcaaatcggtgctgcggcctggcggcgtggacgacgtccaaggcattccgtccgcatggcgccgcacctttccgctgcacgtgggcgcgattctgaacgccgatgcgcatgccatcgaaggctcgcgctggaccgagtgggtgacgcgcgtggcgcccggtgacatgcgcgtggagaccaagcgccggctgtcggccttctatccgaccgacctcgactttctgctgcgcaaccagcgcatcgagacggtggtgctcaatggcggcttcaccgactgctgcgtgctcaacacggccttcgacgccaacaaccacaactaccgcttgatcgtgctgcgggacctggtgcgcggcaccgacgcgcacctggaaagcgcggcgctcgcgatggtgtcgctgcacctcgggctggtggtcgattcgaccgaactgttgcgccactggcgcggttgaccggtcagccggccagacccagccagcgccgggccacggcgtgcacgtcgccctgcgcggactcccacaccagctcgggcgcggccacgtgcacgcccggcggcgcgatgcgcagcgccacgtcgaccagctcggccaccttggaagcgcgcaccggctgctcgctgctcggcaccatgaagcgcacgaccgacagcatccaggccgcgagccgttcggcggggttggcgaacttcgcgttcaggggcttgcgcgccgaacgcacgaggatcacccggtcgaagccgttggcaaccaccgcctgctcgtcgaggctcgcgaggccgcgcttgagcgcctcgggcagcttgccctgatcgtgcggctgcacgatggccagcgtttgcacaccgcaggcgcgcagccagcgcgagagttcgggcaggtctgaaggctccggcacccacagcgcgcgctcgcggtcgtggtacatccgcggtgggtcgaaggcgatcaccgcggtgtcggccgaggtcagtggccattgcgcgatcggcaggccggaactcagatagctttcgacgccgcgcattccgtcgcgaatgggttcgcgcgacagcacgcgcgcatgggcatagcggtggctccccgcgagccggcgcagcagctcctgccccaaggcgccggtcgcgccggcaatgagcagcgtgccggcggtggcaacggccacgggcacgcccgggcgattggcagcctgcagggcttgaagtggatcgatggccatggagccatctatgctaccttccggcaattctgcggaggtaatgcaaatgtcgatcgtgaaacgctggttcctgattcttgctgcggccctgtccctgagcggatgcggctacaacgatttccagtcgctcgacgaggccagcaagtcggcctggagcgaggtgctcaaccaataccagcggcgcgcagacctggtgcccaacatcgtggccaccgtgaagggcgaagcgagtttcgagcaggacacgctcaccaaggtgatcgaggcgcgcgccaaggccacctcgatccaggtgacgcccgagacgctcaacaaccccgaagccttcaacaagttccagcaggcgcagggcgagctttcctctgcgctgtcgcggctcatggtggtggcggagcgctatccggagctgaaggccaaccaggctttccgtgacctgcgcgtgacgctcgaaggcaccgagaaccgcatcaccgtggcgcgcaaccgctacatcgagaccgtgcagaagtacaacgtgctggcgcgcagcttcccgaccaacatcaccgccaagatcttcagctacgagcccaagcccaacttctcggtgcagaacgaagcgcagatctcgacgcctcccacggtcgacttcagcacacccaagaagtaagacacccgcccgatggcacttgccctgattcgccgtgcgctggccgccgtgctgctggcggcggccgcgtgggccggccttgcggccaccgcttgggcgcagggcctgctgccggtacccacgctcacggcacgggtgatcgaccagacgcaaaccctgggcgaatcggagcgcaccgacctcgaagccaagctggccgctttcgagcagcgcaagggctcgcagatcgtggtgctgatggtggccaccacgcagcccgaagacattgcaagctatgccaaccgcgtaggcaatgcctggaagatcggacgcaaggaggtcggcgacggcatcctggtgatcgtggccaagaacgatcgcaagatgcgcatcgaggtggccaagacactcgaaggcgcggtgcccgacctcgccgccatccgcatcatcgacgaggagatgaagccgcgctttcgcaacaacgacttcgcgggcggactgaacgcggcagtggcccggctcatcgggctggtcgatggcgaggcgctgcctgcgcctgccggcgacagcagcagcgagggttccagtgacggcatcgactgggagaacctggcgatcttcctgttcgtcggcgtcttcatcgcagcgccgatcgtgcgctcgattgtcggcaagaagctgggctcggtcgtcatgggcggcggcatcggcgtggtggccttcttcctcacgacgagcgtggtcatcgcggtgctggcgggctttgcggcgctcgtggtgtcgctgttttctgccgcggccacggcgggtgccgggcgccgcggcggtggtggcggcggcttcggaggctggggtggtggcggtggtggctggagcagcggcggcagcagcagcggaggcggtggcttcagctccggcggcggcggcgatttcgggggcggcggcgcctcgggggattggtaggcatggcatcgctcttctcgaagctcggccgcatctggcgccaccagtggatggacgaggccgatgtccggcgagtgctgcccgatgccgccatggaacgcctggcggcgcgcgtcggcgcgagcgagcggcgccacagcggcgagatccgcatctgcgtggaggcgggcctgccctggtcctatctgcggcggaatgcttcggcgcgcgagcgtgccgtgacgctgttcggcaagctgcgcgtgtgggacacccagcacaacaacggcgtgctcatctacctgctgctggccgagcacgcaatcgagatcgtggccgaccgcggcatcgacgcgcacgtggacgacgccgaatgggccgccatggcgcagcgcatgggcgcggcattccgcgaaggccgcttcgaggacgggctcacgcaggcgctggaagaaatgtcggccttgctggtggcgcactttccgctggcggagaaccagcccgacaccaacgagctgccggacgcgcccgtcgttctttgactttctccctcccccactgggggagggttggggtgggggcaagcggcgttgacacggggcacgctctgcctgcccccatcccagccttcccccaaagggggaaggagccacgccttcagtccgatgcgggcagggcccacacggtcttgccgcccaccgcatagaagcgcctccccggcgcccgctccatcagccacccgccggtgaactcaccaaaggctggcagcacggcctgctgcgcatcgctcacgaaacacggcagccgcacgctgtcgcgccccgggccgtgcagcctgcacaccggatgcaggtgcccggcgagcacgaaatgcgtggcatgcgtctgcggatggtggcaacaggcaaaagggccgagcagatgcggctcgtcgaccacgtcgatgccgagcgcggcgggcggatcgcctgcgcggctgtcgtggttgccccgcaccagcgtcatgccgatggacgcatgcgcggcgcgccaggcggccagcgcggccagcacctggggcgtgcgtgcctgcgccgcatgcaaaaagtcgccgagaaacacgatgcgctgcggcgcgcgctcctcgatcagcgcatcgagccgggcgaggttctgctgcgtggtgccgcccggcaccggctggcccagcgcgcggtaggtcgcggccttgccgatgtgcaggtcggcaatgaacagcacgcgcccggcaggccaccagatggcgtgctcgggcagcagatgcagcagctcgccggcccagtggaccgggagcgccgatgcgggaagaaggtgcgacgaggtcacgggcaacgagtgtcgcaaaagacgtgtgggcgggcggccgtcttgcaattcacccctcggaccccagttcttcggtatgaacgaatcgcctccgctgcacatcgtctgtccgcactgccacacgaccaaccgcgtgcgcgcggcgcagctgggcagcgcgcccgactgcggcagttgccaccggccgctgttcaccggtcattcgaccgcgctgccggacgaagcgaccttcgaccgccacatcgcgcgcaacgagatcccggtgctggtggacttctgggcgccctggtgcggcccctgccgccagatggcgccggcctacgaacaggcagcggcccagctcgaaccgagtgtgcggctggccaaggtcgacaccgaagccgtgcccaacctgggcgcgcgcttcaacatccgcagcattccgacgctggcgctgtttcgcggtgggcgcgaagtggcgcggcaggccggggccatgggcgcggcggacatcgtgcgctgggtcaagtcgcacggcgctggctgagcggggcgcgtcacagcggcggcaggggccgtgaccgccgtgatggcggcctgcgctcccgtcgcggtgcggccggcggcttgcccggcccttcctgtccgaacgccagcgtgctcttcacgcgttcgaccccgccagcggtgaccacgccccccgcggctttttcgagctgctcgaccatgcgcgcaatgcggtcggccacgttctcgttcgacagcttttcgcggaacagctcgaccatgagcggaaacgaaaacggcgtgggccgctcgagcgtcttcagcaccaactgctgagtggccatgcgctcaaggctcgcgcgcaggcggccgatttcgagttcttgtgcgagcagctcctgctcggcctgcagcagcagcttgttcgatgggtcgtacttgcggaacacctcccagaacagcgacgacgaggcttgcagctgcctgctgctgcgcttctcgccggggtagccctggaagatcaggcccgagacgcgcgcaatctcgcgaaagcggcgctgcgcgagttcgcccgcgttgagagaagccagcacctcgtgcagcaactgcgcatgcgcatcctcgccttcgggcaggcgcagcacctgcggcagcagcaaaggccagtcgaccggcagggcgctgagcagctcgaatccgtagtcgttcaccgcgatggaaaaggtgcgcgcctcgtgctgcgccacgcgccaggccaggaggctggcaagccccaggtgcacgtgccgccccgcaaagggatagagaaacagatgcgagccttcgcgcgtggtgagcgtttcggccagcagggtttgcggcgtgggcagggccgaccattgctgctggatctcgagcaggggccgcacgcactgcaactcgggtgattcgaagcgcccctcgccggcgagtgcgagctgctgcaccaccgcatcggccaacgtggtcgacagcggcatgcgcccgccgttccagcgcggcaccgcggcgcgcttgccggtggcgcgccgcacccaggcggtcatgtcgtggatgcgcacgagttcgagcagccgaccgccgaacagaaagcagtcgccgggtttcatgcgcgccacaaagccctcttcgacgctgccgatcttcgttcctcccatgtactgcaccgccatgctggcgtcgctcacgatggtgccgatgttcatgcggtggcgccgcgcgagccgcgcatccggcacgcgccagacgccctccgcatcgggcacggcgcggcggtagtccgggtaggcggcgagcgaaggcccgccctgcgagacgaaggccaggcaccactcccagctctcccgcgacagctctgcatacgcagcggtgccgcgcacttccgcatacaggtcgtcgggcatgaagccgccgccgagcgccaccgtcacgagatgctgcaccagcacgtcgagcggctgcgccggcgagtggcgcgcttcgatgtgcccggcagcgatggccgcacgcgccgcggcgccttcgaccatctcgatgctgtgcgtgggcacgagcgtgacgcgcgatggccggcccggcgcatggcccgaacggcccgcgcgctgcagcagccgcgctacgcccttgggcgagccgatctgcagcacgcgctccaccggaaggaagtccacgcccaggtccaggctcgaggtgcagaccaccgccttgagctcgccgttcttgaggccaagctcgacccactcgcgcacagcgcggtcgagcgagccgtggtgcagcgcgatgattccggcccattcgggccgcgcctcgagcatcgcctggtaccagatctccgattgcgagcgcgtgttggtgaacaccagcgtggtgctgctggcggcaatctcgtcgagcacctgcggcagcatcgtgaggcccaggtgaccgccccacggaaagcgctcggcgcggccgggcagcagcgaatcgaccaccagcttcttgggcacctggccctgcaccagcacgccctcttcatcgccgagcaaggcgtgcatggcctcgtgcaggttgcccagcgtggccgacatgccccagaccgcgagccccgggttccagcgcctgagccgcgcaagcgccagctgaacctgcacgccgcgcttgttgccgagcagctcgtgccactcgtcgaccaccaccatcttcacgcggcccagcacctggctcgcatcggcgcgcgcaagcagcagcgacaggctctcgggcgtggtgacgagcacggtcggcaggcgctcgttctgcgcggcgcgctcggccgacgaggtgtcgccgctgcgcgcgccggcgctccagggatgcacctcggcgcccagggcttcgagcggctgcttcaacgcgcgcagcgtgtcggccgcgagcgcgcgcatgggggtgagccacagcacggtgagcggtggggcagcgggccgcgcggtttctttccgggcctgcgagaagacctgcagcgcgcccagccacaccgcataggtcttgcccgcgccggtggtggcatgcaggaggccggactttccttcggcgatggctttccatacctcgcgctggaatttgaagggcttccagccgcgcgccgcgaaccacacatcgagcgccgccttgactgctgtcttgctccttccccttccggggaaaggctgggatgggggcgcgcggccttcgagggacggctgatcgttgatacgccgcttgcccccaccccggccctcccccgggaggggagggagaaatgcggggtccatggggtcggtcatgacggcagcagcgcggccagcgtctgcaaggtatcggcctctgtcaccggcttgtcctcgcgccagcgcagcatgcgtggaaagcgcaccgcgatgccgctcttgtggcgcgcgctgcgcgcgatgccctcgaagccgagctcgaacaccagcgtgggctccacgctgcgcaccgggccgaagctctcgaccgtggtcttgcggacgatggcatccacgcgcgccatctcggcatcggtcaggcccgaataggccttggcaaagggcacgagcttgcggtcgtcctgctcgggcggaccgtcccagaccgcgaaggtgtagtcgctgtaaaggctcgcgcgccggccgtggccgcgctgcgcatagatcagcaccgcgtcgatgctgagcggatcgatcttccacttccaccacacgcccacgtccttggtgcggcccacgccgtactgcgcgtcgcggcgcttgagcatcattccctccacgcccatgctgcgggccgcttcgcgctggcgcgcaagatcgctccacgcgatgcccgtgagcatcgggctgggcagcagcgacggatgctgcgcgcgcgtgacgagttcgtcgagcagcagccggcgctccgactgcggcagcgcgcgcaggtcgcgcccttcccattcgagaatgtcgtacgccagcagcaccaccgggatctcgcgcagcagcttggcgcccagcgccttgcgtccgatgcgcttctgcagctccgcaaagggctgcaccctgtcttcgcgccagacggcaatttcgccgtcgagcaccgtgccgtcgggcagcgcctcgcccagcacggcaagctccggaaagcgctcggtcaccagctcttcgccgcgcgaccacagccagaccgcgccggcgcgcttcaccagttgcgcgcggatgccgtcccacttccattcgacgatccagtcggccggtggaccgagcgcggcatcgaactgttcgagcggcaggttgaacgcatgcgcaagaaagaacggatatggctgtccactggtcttctgcacctgctccgcacccgactccggcgcgatgagcgcgcgatagtcttccgcgcgcggccggccgccgatgtgggtgtagcccatgagccgctgcgccacgcgcttgggatcgatcccgcccaccgccgcgagcgcctgcgtgacctgcagcttcgacacgcccacgcggaaggcgccggtgatgagcttgaagtacaccagccgctcctcggccgcgagctggcgccactgcgcacgcagccgtgcgggcagttcgtccggcgccgacttgccggcttcgcgcagcggcagcaggtgctcgtcgacccagcgcgccagcccgagctcgtgcgcctcggtgggcgggggcagcagcagcgcgatggtttcggccaggtcgccgaccgcttcgtagctctcgtcgaagagccattcgggaaggcccgccgcttcctgcgcaagcaggcgcagcagcttggtaggcacgagctggcgcggcttgccgccggccaggaagtacacggcccacgccgcatcggcggggtcggcttcgcgcaagtagcgctgcagcgcggcttgcttggcaaggctcgatgtgctggcatcgagctcgcggtagagcgcggcgaaatctttcatgcctttgctccttcccctcccgggggaaggctgggatgagggccgccagcgtccgcatcgagcgctgcttgctccctccccggccctcccccggaaggggagggagcttcctggtcatcttcgtcaccgtattcggtcttgaagccctgcgcttccaatccgttctcggtgagccagcgcaccatcactgccacgctgccatgggtcacgaacacccggctggcgcccgtgcccgcaatggcctgctgcaggccgggccaatcggcgtggtcggacatcacgaagccgcggtccacaccgcgccggcggcgcgtgccgcgcagctgcatccacccgctcgcgaaagcgtcggcgtagttgccgaagcggcgtatccatggcgttccctgggccgagggcggcgccagcaccagcgcgcgcttcagcagcgcggcatcgacacccgggtcggtcacgcgcaatgtttcggccaaggccacgcccgcggcgcggtacaccgcgttcagcggctcgacggcgccgtgcaccacgatcggcccgatggaagcgtccacgccatgcaggatgcgttgcgccttgccgaaggcatagcagaacagcaccgacgcgcggccggcctccgcgttgccgcgccaccaggcgtcgatctcggcgaacagcgcagcctgcgtgggccagcggtagatcggcaggccgaaggtcgattcggtgatgaaggtgtcgcacggcacgggctcgaagggcgcgcaggtgccgtccggctctgtcttgtagtcgcccgaggcgacccacacgcgcccgccgtgctcgagccggacctgcgccgagcccagcacgtggccggccggatgcagcgaaacgcgcacgccgtggtgctcgatggcttcgccatagccgagcgtctgcaatgcgatgtcgctgcccaggcgcacgcgcagcgtgcccgcgctgtcggtgtgcgccaggtaatgggcatggccgatgcgtgcgtgatccgagtgcgcatgcgtgatgacggcgcgcgccaccgggcgccaggggtcgatgtagaaatcgcccggcgggcaatagaggccttcggggcgggcgatgaccaagtcgtcgggcatggcgcacatcgtaggccggcgcccggctcttcgcgcagacgggccgacgcgaagccttgtcggcgcgagcctacttcttccttgcgccgcccgtcatctccagcacgttcatcttcatgccgttcgacatcatcatgtctcccggcttctggccggccttgcagggcccgacccacttggcctcgacgatggccgtgccttccttgcgccccatcatcggcgggttgtagctggagcggctttccatgcggtagccggtgccgaagtcgcccgtgatcaccgaatgcgtggtggcggtggtgttgccgattttgcacaccgagtcgaccacgatcctgccgccctcggtgcgcatgtcctgcttggagcaggcttgctggccggtgctgctgcccatctcgcgcatggccttgtcggtggcgccatcgatgcactgctgggtctgcatggcgggggtcttggacgcgccgtcctccgactggatcgacagctcccagagccccggcttgcgcggcgggtagtccagcgcgcgcgccgcgccggcaacgaacaggaggcaggtcgcggcggcgatcccgaagcggatgtgggtcttcatcgtgtactccagcagagacgggtctgaaatgaaagccagccgctttctaacccacaagccggatcggcggaatatggcgatcggccagcagaccccctgcccgccctgcgctcagcgctccggcacgcgcttcaggtcctcgagccagacctccgcttccgagtcgctcggcgcgcgccagtcgccgcgcggagacagcgaaccgcccgagccgaccttgggcgcgttcggcacgcaggagcgcttgaactggctgatcttgaagaagcggtagagaaaggtgcccagatggcgcttgatgtcggccagcgcgtactcgttgcgcgccggctgcagctcgtcctcgggccagcgtccgcgcgtgcggtcgccccaggccgcgtgcgcaaggaaggcgaccttggtcggcctgaagccgtagcgcaacgtgtagtagagatggaagtcctgcagctcgtaggggccgatcacgtcctcggtccgctggccgggctgcttcgacgacccgtcggcggcatccttcgttgcatcgtcgggaatcagctcggggctgacctcggtctggaggatgtcgcgcagcaccgcgctgccgtcggcgcccagcaccccggtcgccgcgacccaatgcactaggtgcttgatcagcgtcttgggtacgctcgcgttcacgttgtagtgcgacatgtggtcgccgacgccgtaggtgcaccagcccagcgccagttcgctcaggtcgccggtcccgaccacgatgccgttgtgatggttggcgagccggaacaggtggctggtgcgctcgccggcctgcacgttctcgaaggtgatgtcgtactgcggcacgccctggccgaacggatggccgaggtcttccagcatctggcggcagctcgggcggatgtcgatctcgcgcgccgtgcagccgatgctggccatgagccggtgcgcctgcgccagggtgcggccgctggtggcgaagcccggcatggtgaagccgaggatgttggcgcgtggcaggccgagccggtccatggcctgcgcgcagaccaggagcgcgtgcgtcgaatcgagcccgccagagacgccgatcaccagcttgtcgatgtggctggcttcgagccgctgcaccagcgactgcacctggatgttgaacacctcgccgcagcgctcgtcgcgccgcgccgggtccgagggcacgtagggaaagcgctccaccgtgcgcagcagaccgcccggcacctggcgcggcggcgccagatcgaactcgacggtgcgccaccccgccagcacgctcttgtgcttctggaccgaggtgccgaagctgttctgccgcatgcgttcgcgcgacaggcgctccaggtcgacgtcggccgcgatgacgtgcgagcggttgctgaagcgttcgctctcgaccagcatgtcgccgccctcgcagatcagcgcctgcccgtcccaggccaggtcggtggtcgattcgccgatgccggccgacgaatagagataggccgcgaggcagcgggccgactgcaggctgaccagccgatgccggtagtccgccttgccgatcgtgatgttggaggccgagagattgaccagcaccgtcgcgccggccagcgcggcgtagctcgagggtggaatcggcacccacacgtcctcgcagatctccacgtgcagcttgaagagaggcatctgccgcgactggaacaggagctcggcgccgaaaggcacgcgctcgccgccgagttcgacctcggtcgagagcgcggtgtcggcgccattgaactgccggccttcatagaactcgccatagttgggcaggtaggtcttcggcagcacgcccagcacgcggccgcccgcgaccaccgcagcgcaattgaagaggcggtggtccacccgcagcggcaggcccacgacagccacggcgccgatgtcccgcgaggccgcggccacttccagcagcgcgcgctcgcaggcatcgagcagcgccgcctggtggaacagatcgtcgcaggtataggccgagagtcccagctcgggaaaggcgaccagcaccgcgccgtcggccgccgcctcgcggtacatgcggatggtctcggccacgttgaataccggatcggccacgcggttgcgcggcaccgccacggcgaggcgcgcgaagccgtgggtgtagggattggagaactcgtgctcggtcatgaaccggattgtggagcagccggcgaaagcggtcacgatcccgcgccgatgcgggccggctcagggcgacgggcacggccaagtgcccgccacgcgcatgccgctaaagagacagaaggcgctggaagaaggagcgatagcgcctcaaggccaggcgcaggttctccgtcgatggctgctccgccgtgtccgttccgccgtcgagcgtgctgcgttcgttcgaaaagcttcgcgacagatcctccaggacttggcgcaccaggtcgtcggcctggcgcaccgcctgcctcggatcatcgacgaagccgatctggagggcatcccagctggcgcggaagttccgcgccgcgtcgggagtgaaaagcggctccagcgcgtcgtcttcgcccctggcgggcaccttcgtctcgggcaccggtacgggcgctggcgcggggcgttccagatcgtccggcgcgacggcgcgctctgcctgggtcgattcgcgattcatgatcgggcctccaccggccttgccggcatcctctcccgctcgacctctctcacttcgagcaggtcatcgaacagggcccggtagtgcaccaccgccctgcgcaattcctccgtgtcggcttcgccgcgcaggtttcgcgcccggatgtcctgtgccgcgcggtagttgctcacgacggcgggatggtcgacggagatgtcggccgcccgacgctcgaagtcgcccatcggatagccgcgcttcagcatcagctcgcgcaccagttcatccgcctgggccaccgccccttgggggttgtcgacgaactcggcctgcaggctgttccaggccgcgccgaatctggcggcttcgcccggtgccagcgcaacgatgcgcagcccttcgactcgctgctgccgcctcttgagttccgcctcggccttcgagcggtcgccaagctcattgacgacgcggccgtattccgaaccgaagtgctcctcgagttgctgggattgtcgttttcgttgatagaggtacacggccagcgcgaccagtgcaaggatcacgacgaccgccaggaccaaccatgtctgcgtgttgacggcatccatacgcgtctcccttcgattgaccgcacccgtggtccgccgtagtcggcggggcatcgcgagtgggtgtagggggatgctgttccggctgccgtggcaagccagcagtccagggcagattcaactgtgggaggccacctacagcgagctcgatgcgcgtgagggcccgacgcgcagcctcaccaggccgtccacttggcctcgctcgcggacgaggccaccgtgcgctcgatgaaccggacacctcgcgcgccgtcttccacgcgtgggtagtcggccgcgagcggatcggctgcaatgcccgcgagccgcgcgcggatgtcggccaccacgccgccgtagatgttggcaaaggcctcgatgaagccttcggggtgccccgcgggcagccggctcgcgcgctgcgccgattcgcaaagccacggcgagccgcgcgtgaggatgcgcttggggccgtcgtgcagcaggtgcagcagctcgctcggccgctcctggcgccattcgagggtgcccagcgcgccggagacgcgcaggcgcagatcgttctccaggccggtgttgatctgcgaggcgatcagcacgccgcgcgcgccgcccttgaagcgcagcagcaggctgccgtcgtcgtcgagcatgcggcccggcaccagcgcgctcaggtcggcgcagaggctttcgatctccaggccggtgacacttgcgacgaggttctcggcatgcgagccgatgtcgccgatggcgccggccgcgccgctgcgcgcggggtcggtgcgccagtcggcctgcttgttgctgccgctgccttcgacgtggctcgcgagccagccctggttgtattcgaccaccaccttgcgcagctcgccgagctggcccgagcggaccatctcgcgcgcctgccgcaccatcgggtagccggtgtagttgtaggtgacgccgaacaccgtgccctgtcttgcgacggcggccaccagtgcatcggcctgttcgcgcgtgtgcaccagcggcttgtcgcacaccacgtgaaagcccgcttccgcaaaggcctctgccaccggaaagtgcacatggttgggcgtgacgatcgagacgaagtcgatgcgctcctccggcgggcgctggagctcgtcggccaggagcgactgccagtcgccgtggttgcggtcgtccgccaggccgaggtcgcggcccgaggcgcgcgccttcccggggctcgacgacagcgcgccggccacgagctcgatctgcccgtcgagcgccatggccttgcggtgcacggcgccgatgaaggcgtcgcggccgccgcccaccatggcgcagcgcagcttgcgaagaggttgatcagtcatcggtaggagatccctggaaactgtcccctctccctctgggagagggctagggtgagggcatgggcgtttacgagcacgctgcctatgccatggccgctgccctcaccccaaccctctccccgaggggagagggagcaaggcagctcagaacggcgagttcgggtggtagaaatctttcgcgttttccttggtgatcagcaccgaaggaatgatcgtggtcgcgggcagcttctcgcccttcagccgcgcttcggccgtgagcttgatcgcgtcgtagatgaacttgggcgaatagctcacgtcggcgccaatgcgcttgtccttgccgtccatgatggtcttgaccatgcccttggcgcccgcgccgccaaagacgatcttgatgtcgtcgcgcttggcctgctcgatggccttgagcacgcccacggccatgtcgtcgtcggccgcccagatggcgtcgatgttcttgaagcgcgtgaggtagtcctgggtgaccttgaaggcgtcgtcgcggttccagttggcgtacttggcgtcgagcagcttgatgtcgggatagttcttcagcactgcattgaaggcgtccatgcgctcgttgtcgagcgtcgtggcaatgccgcgcagggcgaccacgttgcccttgccgccgagttgctttgcgatgtactcggccgggatgcggccgaaggcggtgttgtcaccggccacgtaggcgtcttgcgcgctggtgtcggtgaggccgcgatcgaccacggtcacgtaggcgcccttggccttgacctgcgccaccggcttggtcagcgcggccgactcgaacgggaacaccacgagggcgttgatcttggtgacggtcgagaggtcttgcagctggttcgcctgctcgggcgcgttggccgcggtcttgatcgtgatcttcaggtccttgtgttccttctccagatccttcttcgcctggttggcccagtagttgatgccgcccatgaagctgtgcgtggccgcgggaatcgaaacgccgaggttcactttctcggcggcgaatgccggcaggctcgcgagcgccgcggccgccacggccgtgagtgcgatgcgacgtgtgaagcttgtcatgctggatgtctccttgtggttgatggattggaacgggaacggcctagcggcgtcctctctggaggaacgcgacgatgatgatcacgaagccctgcaccgcggcgttgaggtacacgctgatgatgctggtgaggttcaggatgttgctgatgaccgagagcaggatggcgcccaccacggtgccggtgatgctgcccgcgccgcccttgagcgcggtgccgccgacgatcaccgcggcaatcgcctcgagctcccacaggaggccggtggtcggcgatgcggaacccaggcgcggcacgtacagcagcgtggcaatgcccacgcagacgccgaggagcacgtaggtgaggatcttcacgcggtcgacgtccaccgccgcgtagcgcgccacctgttcgttcgatccgatggcctgcacgtagcgcccgtaggccgtgcggttcaagatgacgccgccgatgatcgcgacgaccacgaacacccataccggcaccggaatgcccgcgaggctggcgtagtacaccggcgcatagaggtccgacaaatcgttgtcgagcgtgagcgcgccgccgtcggcaaagtacgtgaggtaggcgcgaaagatgccgagcgtgcccagcgtcacgatgaagggctcgatgcgtcccttggtgatcaggagcccgtgcgcaaggccgaacagcgcgcccagcaccaccgcgagcaccgcgcccatcaccaccgccatgagcggcgagcccgaggccggcccggcccagttgatgaacatgatcacgctgcccgcgatgagcgccgccatcgagcccaccgagaggtcgatgccgcccgagatgatcacgaagcacatgccgaccgcgatgatgccgatgaaggcggtgcgtgtgagcacgttcatggcgttgtcgacggtggcgaagtcgctgttcagcagcgtgccgccgatgcacagcagcacgaggccgatgaccgggccgaggccgtgcaggcgctcggtccagcgcggcttgctttcgccgcggtgttgcgcggcttcaggctgcggcgtggatgtctgctgttccggtggcatgagcgatgagctcctcttctgtcaaatggtcggcattgagcgtggcgacgaggcggcccgcgcgcatcaccgccacgcggtggcacaggccgatgagttccatcagctccgacgagacgacgatcaccgcgagcccttcgcgggcgagtcgctggatcaaaaagtagatgtcgcgcttggcgccgatgtcgacaccgcgcgtgggctcgtcgagcaccaccaccttgggcctgggctgcagcaccttggcgagcgcgagcttctgctggttgccgcccgagagcgaagatgccttgacgtcgagcgagccggtgcggatgccgtagtccttcacggcctcggccagcgcgccgcgttcggcttcgggctggagccagggctgggcatagcgctcgagcgccatcagcgtgaggttctggcgcaggccgaagttcacgtgcaggcccttgcccttgcgatcttcgctcaggtaggtgaggccgtgccgcgccgcatcgcgcggattgcgccaacccgtctggtgcggcaccggcttgccgagcatctcgacatggccactggcgggccgaaggcccagaaggccttcgaacagctcggtgcggccggcgccgacaaggcccgcaaagccgaggatctcgccggggcgcacctcgaagccgacgtcgtgcgcccaaccgggcacgctgaagttgcgcacgcgcatggcgggcgcatcggccgccaccaccacgtcgcgcggcgggtacaggtcggcgagttcgcggcccaccatgaggttggccatctggtggcgcgtgacctggggcgtgggtgcgcgcgcaacgaagcggccgtcacgcatcacgatcacctcgtcggtcacctgctcgacctcgtcgagcttgtgcgagatgtagacgatggtcacgccgtcggcgcgcagctgcgcaatgagcttgaagagccgctcggtctcgccgggcgtgagcgtggcggtgggctcgtccatgatgagcagacgtgcacggcgcgcgatggccttggcgatttcgaccaactgcttctcggcaacgatgagccgccgcaccttggtacgcggatcgacctgcaggcccacggcggcgagcgctgccgcagcatcgcgttccatcgtcgcatcgtcgagcagccagcccttcttcttttcatggccgaggaagatgttctgcgccacgctcaggtcttcggcaagattgaactcctggtgaatcagcacgatgcccagcgcctcggcatcgcgcgaactcgtgaagtgccggggctcgccgttgatgcgcagcgcgccgccggtgagcgactcgtagcccgcaagaatcttcatcaacgtcgacttgccggcaccgttctcgccgagcaatccgtagacgcgtccgggcgcgagcgaaaagctcacgccgtgcagcacctgcaccgggccgaaggccttcaccacgccgtcgaattcgaccgcgacgcttcccttggtttctgcttgtgccgtcatggcgccaccccgcggactttgagtgtttcgtgcatcgcgagcacgccggcgccgatcagcccgccctgcacgcccagtggcgtgtactggatttccaggtgccgcgtggagagcgcgagcgagcgctggtagacgctctgccgcacggccgcgagaaacagcggcccgatgcgcgtgatgccgccgccaatgaacacatgcgacggattgaagaaattcaccaccgacgccagcatctggccgatgaggttgcccgcgcgctggatgatgccgttggcgaccgtatcgccggcacggctcgcctggcccacatcgacggcatcgatgtgcccatgcacgcgcaggcattcggcgagcaaggcgctttcaccggcttcggccgcctgcacggccatgcgcgtgatggccggccccgcggccatggcctcgacgcagccgacgttgccgcaatggcagcgcgggccctcctggtcgacgcagatgtgccccacgtcgccggccgaaccggccgcgccgcgatagacctcgccgtggcagacgatgccgcagccgatgccggtgccgatcttgatcacgagaaagttgttgagcgagcgcttcagccgccagagctcgccgagcgccatcaggttcacgtcgttgtcgacgaagaccggtgcggcgtagtcctcccgcaggtagtcgcggatcgagaagctgtcccaggccggcatcagcggcgggttcacgagctggccgatctcgaaattgacggggcccggcacgccgatgccgatgccgagcacgtccttggcgccgctgttgcagcgcgcgagcagctcgcgcatgagcacgcgcacccgcgccagcaccaccgccgggccttcgcgcacgtcggcgggttcatcgtgctgcgccagcacggtgaggtcgggacgcaacaccgcgacgtccaggctggtggcgccgatgtcaatgcccacgagcacgcccaggccggtgtgaagctggaggttttcggcgcgccgtccacccgacgagcgctgcaggccggcttcggccaagaggccctggtcgacgaggcccgcgatcagcgcattggccttgctcttggagaagccgagctgctcggccatggcatggcgcgacccgccggccgaccagaaggtggtctccagcaatcgcatttcgtccgcagtgatgccactccagggtgccacgcgctgtctccaatattctttttggcccaccgccccccgtgggtgccgatcggcggaatgggaatactaggtgcgcggcttcagccggacaaggccgaacttcgaccaaattcagatcgaagccgttctctcgacagaacgcggacgaaaaaaagccgccctaggaggcggcttcttcggagcgagagccttggctcttgcttgcttgcttgcttaattacttcttctggcggtacttgcgcagcgccgcgatctgggcggccatgacggccagctcggattgcgccatggcgatgtcgatgtcgctcctggcgttcttgagcgcttcctcggcagccgccttggccttgttggccttctcgtcgtcgaggtccttgccgcggatggcggtgtcggacagcacggtgacggcgttgggctgcacttcgagaatgccgccggccacgaagacgaactcttcgccgccgtcggccgtttcgatgcgcaccgcacccggacggatgcgcgtgatcagcggggtgtggcgcggatagatgccgagctcaccggcttcaccgggcagcgcgacgaacttggcttcgcccgagaagatcgactcttccgcgctgaccacgtccacatgaatggtgtttgccatcttttttcctttgccgttctatggaggaacatcggaaagcaagcagtcggccgtctggtgaggcgccgcgcgcagccgtacacaagtacggcgagcacggcgacgaagccaggcggtcgaccgcgccgctttacgcgaccttcttggccttttcgaacgcttcgtcgataccgccgaccatgtagaacgcttgttccggcaggtggtcggcttcgccgttcacgatcatcttgaagccgcggatggtttcagccagcggcacgtacttgccgggcgagcccgtgaacacttcggccacgtggaacggctgcgacaggaaacgctggatcttgcgggcgcgggccacggcgagcttgtcgtcgggagccagttcgtccatgcccagaatcgcgatgatgtcgcgcagttccttgtagcgctgcagcgtgccttgcacggcgcgggccacgttgtagtgctcttcgccgaccacgttcgggtcgagctggcgcgaggtcgagtccagcgggtccacggcggggtagataccgagcgaagcgatgtcgcgcgacagcaccacggtcgagtccaagtgagcgaaggtcgtggcgggcgacgggtcggtcaagtcgtcggctggcacgtacacggcctggatcgaggtgatcgagccgaccttggtcgaggtgatccgctcttgcaggcgacccatttcctcggccagcgttggctggtagcccacggcggaaggcatgcggcccaagagagccgacacttcggtaccggccagcgtgtagcggtagatgttgtccacgaagaacagcacgtcacggccttcgtcgcggaacgactcggcgatggtcaggccggtcagcgccacgcgcagacggttgcccggaggttcgttcatctggccgtagaccatggccaccttcgagtcctcgagcttctcgaggttcacgacgccggagtcggccatctcgtgataaaagtcgttgccttcgcgggtacgttcacccacaccggcgaacaccgacagacccgagtgagccttggcgatgttgttgatgagttccatcatgttcacggtcttgcccacgccggcgccgccgaacaggcccaccttgccgcccttggcgaacgggcacaccaggtcgatcaccttgatgccggtttccagcaggtcttgcgacggcgagagttcgtcgtaggcaggagccttgcggtggatcgaagcggtgaggtcttggctcacttcgccgcgctcgtcgatcggacggccgagcacgtccatgatgcggcccagcgtggccttgccgacgggcaccgtgatgggcgcgccggtgttggtcacgatcaggccgcggcgcaggccgtcggacgagccgagcgcaatggtgcgcaccacgccgtcgccgagctgctgctggacttcgagggtcagcccgccgccttcgaatttcaaggcgtcatacaccttgggcatctggtcacgcgggaactccacgtcgaccacggcgccgatacattggacaatttttccttcagccatggcgtttccttctggatctcaataatgttgcgacaggttcttgcagaagcgtccttgtgccatcgcgggccgcttttgcaagaatgccggacgggccggcacccttgatttcagatacttcttccgatcagcacttcattgccgccgcctgcgcggcgaaagcatcgctggcagccttgcaggcctggcccagtgcggccttgtcggtgcccaacgaagcccaggcagccttggtctgctccacgctcgccttcatcgcatcggcggctgcgccgctttgtgcggacgcgcaggcctgtgccttggcgaggtagtcgttgcactcttgcggcaggtccgcggccgatgccgtcggcgcggttgcggccggcggtgcagctggcgcaggcgccgccggagcgggagccggtgctggcgtggcggcgggtgccggcggtgccacgggcgcctcttccttcttggagcaggcagtcagcgcggcggccatggccaccagaacgagaagttttttcattatgcagagtcccctaaaaaaggccttcggttatcgggcccgcagagcgggcctcgaatggcaatgtggcccggtacattgcctcatcaaacaccggcggccgcagcggcgccggacacgatttccgaaagttccttggtgatgcctgcctggcgggtcttgttgtagaccagcttgagctcgttgatcacgttgcccgcgttgtccgttgccgccttcatggccaccatgcgggcggagtgctcggacgccatgttctcggccacggcctggtagaccagcgactccacatagcgcaccagcagctcgtcgatcacgctctgcgcatcgggctcgtagatgtagtcccacgaatgctggcccgcctcgacttgcagcgagtctgcggccagcggcagcagctgctcgacgagcggctcctgcttgatcgtgttgatgaacttggtgtagcacaggtacacggccgacagctttccctcggcataggcgtcgagcagcgtcttgaccggcccgatgagcttgtccaggtgaggcgtgtcgcccaagtgggtgacatgggccaccacgcgcgcaccgatgcggttcaggaagcccaggcccttgctgccgatggccaccgagtcgatggcgatgcccgcgctctgcgcttcccgcagctttgccgtgacggcgcgcagcaggttggtgttcaagccaccgcacagtcccttgtcgctcgtgacgatgatgaagccgatggccttggcatcgttcttcttcatgaacgcgtgggtgtactcgggattcgccttgcccaggttggccgcaatgttgcgaattttctcgctgtaggggcgggcggcacgcatgcgctcttgcgccttgcgcatcttggaaaccgagaccatttccatggccttggtgatcttcttggtgttttccaccgatttgatcttgccgcggatttccttaccagctgccatgagtgctccttgtccggccgatcaggcgaacgacttcttgaacgacgtgatggcggcggtcagctcggcttcggcgtccttgtcgagcgccttggccttttcgatcttgtcgagcagcgcagcatggctggacttcaggaactggtgcaggccgtgttcgaacggcagcaccttcttgatgtcgaggtcgtccatgaaacccttgttcaccgcgaacagcgtggcgcccatcagcgagatgggcagcgggctgtactgggcctgcttcagcagttcggtcacgcgggcaccgcggtcgagctgcttgcgggtggcttcgtccaggtcggaagcgaactgcgcgaacgcagccagttcacggtactgggcgaggtcggtacggataccgcccgacaggcccttgatgaccttggtctgggccgacgaacccacgcgcgacaccgagataccggcgttgatggcgggacggataccggcgttgaacaggttggtttccaggaagatctggccgtcggtgatcgagatcacgttggtcggaacgaaggcggacacgtcgccggcctgcgtttcgatgattggcagcgcggtgagcgaaccggtcttgcccttgacggcccccttggtgaaggcttcgacgtagtcggcgttcacgcgggctgcgcgttcgagcaggcggctgtggagatagaacacgtcgccggggtaggcttcgcggcctggcgggcggcgcagcagcagcgagacctggcggtaggccacggcttgcttggagaggtcgtcatagacgatgagcgcgtcttcgccgcggtcgcggaagtattcgcccatggtgcagcccgagtaggccgacacgtattgcatggctgccgattcggaagccgatgcggccaccacgatggtgtagtccatcgcgccggcttgctccagtgcacgcaccacgttcttgatcgacgaagccttctggccgatcgcgacgtagacgcaggtcatgttctgacccttctggttgatgatcgcgtcgatcgccacggcggtcttgccggtctggcggtcgccgatgatcagctcgcgctggccacggccgatcggcaccatcgagtcgatggacttgaggccggtctgcatcggctggtcgacggacttccgtgcgatcacgcccggagcgaccttttcgatcacgtcggtcatcttggcgttgatcggacccttgccgtcgatcggctggcccagggcgttcaccacgcggccgatgagctcggggccgacgggcacttccaggatgcggcccgtgcacttgacggtgtcgccttcggagatgtgctcgtactcgcccagaatcacggcgccgaccgagtcgcgctcgaggttcagcgccaggccgaacgacggcgtgccgtctgccgtgggcgggaactcgagcatttcgccctgcattgcatcggacaggccgtgcacgcgcacgatgccgtcggtcaccgaaacgacggtgccctcgttgcggatgttggcgctgaccccaaggccctcgatgcggctcttgatcagttcggaaatttctgcgggattgagttgcatgactctttccttctttctttgaggctacaagtagagggctgaagaccgtcaggccgccagcgcaactttcatttgttcaaggcgcgctttgacggaggtgtcgagcacctcgtcgccgaccaccacacgaatgccgccgatcagttccggctcctgctggaccgtgacctgcagcttgcggccgaaacgcttttcgagcgcgacggccacattggccagaaccgcggcatcgatgggaaaggcgctgtagaccacggcgtcggacgagccgctcttcgcgttggccagtgcccggaactgcttcgcaatttccggcagcaccgagaaacggccgttgtccaggagcgcgcccaggaagttctgggcgtgggcggtcagcggtgcaccgaaggcgccggcgaccacaccgagaacctgctcggccgtggccttggggttgtcggcgaactgctgtagctccgggctggccgcgatggcggccaccttgtcgagccatgcgctggttccggcgacgtcggacgacgacgccttgaaaagcgcctcggcgtagggacgtgcaatggtggcgagttctgccatggcttctatcagagttcggtctgcagacgggcgagcaaatcggcgtggacgcctgcattcacttccttgcgcagaatctgctctgcgcccttgacggccagtgcggcaacctgctcgcgcagtgcttcgcgcgccttcagtgcctgctggtcggcttcgacgcgtgcagcagcaacgatcttgttgccttcttcggtcgcgcgggccttggcctcttcaacgatggcctgggcgcgacgttcggcgtcggcaagacgttgcgcggactcattgcgtgcctggcccagttcggcttccacgcgcttgttggcggcggacaactcggacttggccatgtcggctgcagcgaggccttcggcgatcttcgcagcgcggtcgtccagcgctttcgcgatcggcggccacacgaacttcatcgtgaacccgaccaggatcaggaacacgatcatctgaacgatcagggtaccggtaatgctcacttttcaccctctctttgggattgaatgcgaagccattccacggaggggaacgacgtcacgggtccgacgagaaagacttacttcggcaggttggcgatctgagccaggaacgggttggccgttgcgaaccacagcgcgataccggtgccgataatgaaagcagcgtcgatcagaccagccagcaggaacatcttggtttgaagttcacccatgagttcgggctgacgtgcggccgactcgaggtacttgctgcccatgatgccgatgccgatacatgcgcccacagcgcccagaccgatgatcaggccggcggccagtgcaacaaagctaataacttccatgatgactcctagaggactttggttgaagagaaaacaaaaaactaaaacgaaaccgaacgatcagtggtgatcgtgagcctggccgatgtagaccagcgccagcatcatgaacacgaaggcttgcagcgtgatgatcaggatgtggaagatggcccaggccgtgcccgcgatgatgtggccgatggccaggccgatgccggtggccgacagcgtgaaggcaccgcccatcagggcgatcagcaggaagatcagttcgccggcgtacatgttgccgaacagacgcatgccgtgcgagacggtcttggcgacgaactcgatcatctgcatggcgaaattgaacgggtacagcgcccagtggttgccgaacggcgcggtgaagagctcgtgcacccagccgccgaggcccttgatcttgatgttgtagaacaggcagaccagcagcacggcaaccgacatgcccatcgtcaccgagaggtcggccgtgggcacgacgcgcaggtaggcgtgatgcgggtcttcaccggcgatgccgaagatcttggcccagattgccgggaacaaatcgaccgggaacaggtccattgcgttcagcaggaagatccacacgaagatggtgagcgccagcggagcgacgaacttgcggctggtggcgttgtgcacgatgcccttggcctgctggtcgaccatttcgaccaggagctcgacggccgcttgaaaacgccccggaacgcccgaagtagccttgcgggccgcgagccagagcagccagcaacccagcatgcccaacgcgatcgagaaaaagagcgagtcgaaattgaataccgaaaagtccgcaacacctccaggcttggagctttgcaggtgcgtcaagtggtgaatgatgtattcacccgcggtctgaccatgttccgcagcgttttcagcagccattcagttactcgtctctatgttgccggcgccggggcgaaaacatcaccgccaaccaggccgccttcattgtcaccaccaaaccgaccagcattgcaggccagctcagcgccgtaatcagcattggcgccgcgaacaacatcgcaagcgacaaggccatcttgaccatttcccacaggaagaacccaaccaccgcagtgcccggattcagggaagaaaaccggccggtcaacccccgtgcgaacaccgcagcaggaatgaccaccgcgatcgcaccgtaagcggcggaccaacccagattttgcctccccgtcagtccccaggcggccaaagccaccagcagaccaacaaccaactgccccgcgatgacccaccaaagggaaatcgagggatgccttgcacgcagttcacgcgcctcatcggcggtcaacggcttgtattccgtgtcgaggtcttcagcgaccctttcatctttttgggcgattgttttcatttcgaatgaagcccggatgacgacccagaatttctacaaagccattgattataagtaaaaacccagcccgtccggccacttgaactgtcgccgttgcaaatcgaggcttcgtcagctgacgagaacccgacttggcgcacgcaaccataattccttcatgcaccctctcactgccgctctccccaccacgctctgctatctcgacggcgaatacaccgccgtcaaggatgccaaggtcagcgtgctcgatcgtggcttcattttcggcgacggcgtctacgaagtcgttcccgcctatggtggccagcctttctgcttcgaagaacacatggcgcggctcgatcgttcgctggccgagttgcagattgtcgatccgctcacgctcgccgagtggcgcgacatcgtgatgcgcctgatcgccccgggcggcgatgcaccgcaagccgtctacttccaggtcacccgcggcgttgcgccgcgcgaccatgcgatggtcaagggcctcaagcccaccgtcttcgtgatggtgaacccgctgccaccggtgtccgatgcggtgcgcgccaagggcgtgacctgcgtgactgcagacgacttccgctggcagaaggcccacatcaagagcaccagcctgctgggcgccgtgctctcccggcagatcagtgtcgaggccggcgcggcagagaccgtcatgttccgcggcgactggctcagcgaggcttcgtcgagcaacgtatggatcgtgaaggacggcgtgctgatcggcccacccaaggacaacctggtgctcaccggcatccgctatggcctgctcgaacgcctgtgccgggaaggcggcattccctttgcgctgcgtcgcgtgtcgcgcgatgaagtgttcggtgccgacgaactgatcctgtcttcggccagcaaggaagtgctgcccgtcgtcgcgctcgacggcaaagacattgggaatggccggcccggccccatctacaagagcttgtatgcggcctaccaggaggccaagcaacgcaacgctgagaagcaaggagccccggcatgaccgagaacaccaccgacgcagtcaccacacccattcccgatccgcgcaaggaatcgctgatcgaatatccctcgcagtttccgatcaaggtcatgggcgtcaaggtcgacgggctcgtgcatgcgatcacccagatcgcagagcgcttcgatccggccttcgacgccaccacggtcgagttgcgcgacagcaaggcgggcaactacctgggcgtgaccatcaccgtcaccgccaccagccgcgagcagctcgacgacctctaccgagcgctgtcggcccatccgtcggtcaaggtcgttctctaggctggacctgatgacgctggcagagcacccggcgggcaccgccctcgcactgcgctggctgggccgcgtcggctatgccgagacctttgcggcgatgaagcagttcacgctcgagcgccagccggaaacgcccgacatgctatggatgtgcgagcacgcccccgtgttcacgcaaggcctcgcaggcaagcaggatcacatcctgaacccgggcgacattcccgtggtacagaccgaccgcggcggccaggtcaccttccatgggcccggccaagtggtcggctatccgttgatcgaccttcggcgggcgggctactacgtgaaggaatacgtctaccgcatcgaggaatcggtgctgcgcacgctggcccacttcggcgtgacggggcaccgcgtgccgggcgcgcctggcatctacgtgcgcctggacgacccgttctcgcatgcggcactgaccggcccgctgcccgccagcgacccgtttcggggcctcggcaagatcgccgcgctcggcatcaaggtgagccgccatgccacttatcatggagtcgcgctcaacgtcgacatggacctcgaacccttctcgcgaatcaatccgtgtggttatgcggggctgcaaacggtcgatctttctacaatcggcattcaaaccacatgggaagacgctgcccgggtcttgagccagaagctcacaacctacctggcgccttagcatccaatgagctctaccgaagtcgtccgggacgcacaaagcgccgaaaactacaacccgctggccaagcagaaggccgcggccaagctgtcgcgcatccccgtcaaggtggttcagggcgaagtgctcaagaagcccgagtggattcgcgtgaaggccggcagccccaccacccgcttctacgagatcaagcagatcctgcgcgagagcaacctgcacacggtctgcgaagaagcctcgtgcccgaacatcggcgaatgcttcggcaacggcacggccaccttcatgatcatgggcgacaagtgcacgcgccgctgcccgttctgcgacgtgggccacggccgccctgatccgctcgacaaggacgagccgctgaacctggccaagaccatcgccaagctgcggctgaagtacgtggtgatcaccagcgtcgaccgcgacgacctgcgcgacggcggcagccagcatttcgtcgattgcatccagaacatccgcgagctctcgccgatgacgcagatcgagatcctggtgcccgacttccgcggccgcgacgaccgcgcgctcgacatcctgaaggccgcgccgccggacgtgatgaaccacaacctcgagaccgcgccgcgcctttacaaagaagcgcgccctggcagcgactaccagttcagcctcaacctgctgaagaagttcaaggcgctgcaccccaatgtgccgaccaagagcggcatcatggtgggcctgggcgaaaccgacgaagagatcctgcaggtgatgcgcgacatgcgcgcgcacgacatcgagatgctgaccatcggccagtacctgtcgccgtcgggctcgcacctgccggtgcgccgctacgtgcaccccgacaccttcaagatgttcgaggaagaggcctacaagatgggcttcagccacgccgcggtgggcgcgatggtgcgttcgagctatcacgcggaccagcaggcgcacgccgccggcgtgtaaggcggcagtcggcggcaaggcgggtgggccgtcgcatgtagctcacccggtccgaggcttcttcgctatcctgccggctggccaagacgaaggatcgattttgcaaacgcaccctgccatccaagccgcgatggaacgcgagttcggcgccattgccgatctggttcgcctccatgcgcaacacacgcccgaccatgccgcgctcgcggacgcccatcgcacgctgacctacggcgctctcgacgcgctgatggaccgtatcgcggccagcctgcagcgcgaagggctcaagcccggcgatgcgatcgcggtgtgcgcgtcttcttcggtgaactatgcggcggtgttcctgggtgccttgcgcgcgggcgtcgcggtcgcgccgctcgcgcccggctccaccaccgccagcctggcgcgcatgatcgaggatgccgatgcgcgcatcctcttcaccgacgcttcggcggccgaggtcgtcggcgccccgaaggaaggcggcattccgcgcgtggcgctcgacggttccgctgccgggcagagtctcgagagttggctggcccccgtgggtgcacggccgagcgcggtcgaaacgcaaccttcctggcccttcaacatcatctattcctccggcaccaccggcgagccaaaaggcattgtgcagggccatggcatgcgctgggcccacgtgcagcgtggcgccaaatacgggtacggcgcggacacggtcacgctgctgtcgacaccgctttactccaacaccacgctggtggttttcttcccgaccatcgccttcggtggctgcgtggtgctgatgccgaagttcgatgcgctcggctacctgcaactggccgagcagcaccgcgtgacgcacacgatgctggtgcccgtgcagtaccagcgcctgatggcgcatccgcgcttcgacgcacacgaccttgcgtcgttccgcttcaagttcagcaccagcgcgcccttcaatgccgcgctcaaggccaatgtgctcgagcgctggcccggcgggctgatcgagttctacggcatgaccgaaggcggcggcacctgcattctcgaagcccacctgcatcccgacaagctgcacacggtggggagcccggccgagggcagcgacatccggctgatcgacgaggacgaccacgagattccgcgcggcgacaccgaacgggccggcgaggtggtgggccattcggccggcatgatgaccggctaccaccgccagcccgccaagacgcgcgaggccgaatggttcgacgcgagcggcaagcgcttcatccgcaccggcgacgtcgggcgcttcgatgccgacggcttcctgacgctgttcgaccgcaagaaggacatgatcatcagcggcggcttcaacatctacccgagcgacctcgagacggtgctgcgaggccatgccgccgtggccgacgtcgcggtggtcggcgtgccgtcggagcaatggggcgagacgccggtggctttcgtggtgcgccgtgaaggcgacggcaccaccgaagaagcgctgctgcaatgggccaacgcccagctcggcaagacgcagcgcctggcgcgcctgcgcttcatcgacgaactgccgcgcagcgccatcggcaaggtgctcaagcgcgaactgcgtgaactcgtcggccactgaagcgcgggcagcggcgccgtccgagcacggcggcggcaacggcctgctgtggctgctggccgccgtggcggtcttgttcgccttcctgcgcccgcgtgcgcccatggactggctgaagctggtcgattggcagaccgtgggcgcgcttgcgggcctgctcgccatcacccagggcgtggaaaagagcggcatgctgcaggccgccgcccagcgcctgctcgcgcgcacgcacagccagcgcagcctggcgctgctgctcactgccagtgccgcattgctctccgcgctggtgaccaacgacgtgagcctcttcctgctggtgccgctgacgcgcgtgcttgccaaccaggcgcacctgccgctcgcgcggctcgtggtgctcgaggcgctggccgtcaatgcgggttcggcgctcacgcccatcggcaacccgcagaacctctacctgtggcaccgctccggcgagagcttcgtcgccttcatgggaatgatgctgccgaccgtggccgtgatgctgttctggctcttcgcggcggtctggctgctggtgccgcgcacgcccatcgcgctcaagcccgaagccgaggccacgccggtgcagccgcgcctgctggcattggcgggggtcctgttcgtcggcttcgtgatcgcgctggaccggcattggctgctggcaggcctgggcgtggtgttcgccgttttcctggtgtcgtatccgcgcgtgctgcgcggcatcgactgggccctgctcgcgatcatcgcgttgatgttcgtggatctgcggcagctggccgagctgcccgccgtcgtggcgctgatgaaccattggcccatcaccgacggatggcgcgcctacctggccgccatcgtcacctcgcaattcatcagcaacgtgccggccgcgatcctgctcgacggccatgtgcgcgacctgccggcactggcggcgggagtgagcgtgggcggcttcgggtgcgtgctgggctcgctggccaacctgatcgcattgcggcttgccagattgccgcacggcctgcgcgagtttcaccgcatcagcattcccttcctgctggtgtgcgcggcttccgcgttgctgctgcggctgggatgacagccgcggagcacggaacgacaattcgatcctgcccatgcgaaccccagccatgctcccgcgcgccgaactgcacagcctttcgctgcgcgactacggcgcttcgcgcggcagccacgcgcatgaccacttccaggtgctgatcggcctggccggtgtgctcgaactcgaagtggaaggccgcggtgcgcacgttggcgccggtgaggcgcaggtggtggtgcccggcgaccggcatgacttcgaatcgcgcagcggcagccggtgcctcgtgctcgacaccacccacccggcatgggcgcgctgcgccgagcgcgcccgcaaatgcgtcgcggctgcaggccctggcgcagtacctcgcgcagtgcgcgcagcacccggacgctttcgtgtcgacgctgcagcatggccccgcgctgttgctcgaagcctggggtgccgccgcgccggcccctgcgcgaagccggcgaatcgactggaccgcgctcgccgcctgggcccgggcgcgctggcacgagccgctgggcgttgccgatctcgcagccgtggcgtgcctgagccccagccagttcgctcagcgctgccgcgatgagcagggcgtgagcgccatgcactggctgcgcatgctgcggctcgcgcatgcccgcgaactgcgcctggccggcatgggcgtcgcggaaacggcgcgccgcaccggctaccgttcgccctcggcgctcacggcggcattgcgcaggctcggcagctgaacggcaacatcgtcgtcacgcgacgattcaccggcgttgcgcgacgacggcgccgcttaagctcggtgcaatgtcgcccacgcttcttgcccttgccgccatcgcgctgtgggccacgctcgcctcgctcggcaccgcgctttcgcacctgccgccgttcctgctgacgggcctcgcgctgatcatcggcagcattccgagctggccgctcgtcttgcgcgaccgcagcgcctggagcgtgccgccgcgcacgctggcgctgggcatctacggcctgttcggctttcactttctgctgttcatcgcgctgcggcatgccccgcccgtggaagccaacctggtcaactacctgtggcctctcttcatggtggtgctggcgccggcgctgctgccgggcgtgtcgctgcggccgttgcatctggttgccgccacgctgggcttcgcgggcgcggcgatcgcgatcctcggtgcgcgcgagggctccgtgtccattcctggcgccacggccgggtactggggcttcctgccggcgctgggctcggcgttcatctgggccagctattcgctctggacaaagcgcgtggcggcgttcccgacctccgcaatcggcctgttcggcctggtctcgggcatgttgtcgctcgtctgccatgcactgctcgagaccccggcaatgctctctgcgaaagactggctgctggtcgcactgtgcggcctcggtccgctcggcgcggctttcttcgtctgggacatggcgctcaagcgcggggatgcgcggcagatcggcatcctgagctacgtcacgccgctgggctccaccgcgctgctgctggccgtgaccgggcgcccgctcacctggagcatcggtctggcggcggcgctgatcatctcggccgccgtgatgggcacacgcgcccgctgaatacgcccgtgtccgacgacaccggtgcatggtttgtggctagagtggaggcttcggaaaaaaaggagccatcacccatggataagaagaacaagaacgatgaattcgagatcacccccaagctggtgttcgacctgaacctggcgctgtacctcgacctggtggcggcactcgaaagcgcgggcgccgtcagctaccgccagatggcggcccgggtgctcaacatcagcatggacgcccgcgccgacggcgacgtgggcctgtcgacggcgctcgaaggcgttgccaagggctttgccggccacggcgacggcctgtcgatcgaaacgctgaaggccgcccacggcctgcgcgaggacgacgcgatgggcgacattccaatgcgccccagcgagccctgagccggcgtcagtcttcggccacctgcaggatcagcttgccgaaattctcccccgcgaacagcttgttgagcgactcggggaaggtatcgaggcccttcaccacgtcttccttgctcttcatctgcccgtccttcaggtagccggccatctcggcgatggcgatgtggtaccggtcggcgtagtcgaacaccacgatgccttccatgcgcgcccggttcaccagcaggctcaggtagttcttcggaccggcgcccggcatgctgttggcgttgttgtactggctgatggcgccgcagatgatcacgcgggccttgcgtgcgagccgcgccagcaccgcgtcgagaatctctccaccgacgttgtcgaagtagatgtccacgcccttcgggcagtgggtcttgaggccgtcgcgcaccgccgcggcgccggccttgtagtcgatgcaggcgtcgaagcccagctctttcaccacccagtcgcacttggcggcgccgcccgcgatgccgaccacgcggcagcccttgatcctggcgagctggcccacggtctgccccaccgcgccggccgcgcccgagatgacgacggtttcgcccggcttgggctggcccacgtccatcaggccgaagtagccggtcatgcccggcatgccgagcacgttgagccactggttgatggtgccgaccctgaggtcgattttcacgaggccgttgcgcttgatctggtcttgcggaatcagtatgtattcctgcacgccgagcatgccgtagacagtagcgccgaccgcgaactcggggttcttcgaagcaatcacgcggccaatgccgcctgcacgcatgacttcgtcgatcgccaccggtgcgatgtagctcttcgcatcgttgagccagccgcgcatggccggatcgagcgagagcgaaagcgtcttgaccagcaccccgccctcggccggttcgccgacgggctcggtggtgaagcgccagttctcgcgggtggccgtgccctctgggcgcttggcgaggcggacctggtggttggtgagtgagctgctcatggtgtctccttgattgacgggcgctggcacggacgcgcatcgtagccccgcattgcgcgtcgactggtagcgcaggtgacagcgcaagacaccgtgagcgaaccctacatgcgcacgacgatctgcaggccgggatgcgcgttgcgcaccacgaatgtcccgccgtgcgcctcggcgatcagccggcacaggtacatgccgagccccacgccgccggtggcacgcgcgcgcgcgccgtcggtgcggtagaagggctcggtcagccgctcgagctgggcttcgtcgacgccggggccatggtcccgcacctcgagttcgacaccctggaccttgccgtccaccaccgcgcgcagcgacacgcacggcggccgcggcgcgtcggtgctgtagcgcaaggcgttgtccagcaggttgcgcaccagaaggcgaaaacgcatgcggtcgatcgagtgcgccggcaggccttccgccaggtcgagatgcacgttctgcgcgcccggcatctcggcgacgatttcgcgcaccagcacggccaggtccaccggttcgcgctgcagcgccgcatgcgggcttgcgaggcgttcgctttccagcaggtcgctgatcaggtcgcgcatctcgttcaggtcgcgcagcagcgcttcgcgctcggccgcgccctcgggcgtggccggcagcagctcggcattgagccgggcccgggtgagcggcgaacgcagttcgtggctcaacgccagcagcaggccgcgcttggcatcgagcatggcctggatgtcgtcggccatggtgttgatgtgtcccgcaaggtcgccgaggtcgtcgttctggcggattggaatgggctgcgtgaactcgccgcggccgaagcgctgggcgccttcgcgaatgtcgatcagcggccgcagcaggcggctcacatagacatagcccagcaccatgagcagcagcagcgcgcagagcgtggcccagcccgccgcgcgcggtgcaagctgccagagcttgggcgcccagccgaagatgacgcggtggccgtcggccgttggacggatgaaccacttgtcgttcagcggctcctcgtcgaggtggtgcatccagccgccgcggccgttgaagcccgcgggattggagtcccagttgaccttggggcccacgatgcggatcgtgatcggcagccggctcaccagcgcctgcgcgcgcgcgatgtcgggcggggtgccgatctcggcgacgagccggtcggcatagtccaccagcatcggctttgcggcctcggcccagccggtagagaaggacttcttcatgccgcccatgaacaccactgccatcaccagcgccagcagcaggaacatcatcacgagccggatgcgcagcgaacggcgccagcggcgcttgccctgcaccttctcgtgccattgttcatgccattgcttgtgcagctccgcacgccggcagctcatgtctcgccacgccttgcgccaacctctcctcgaagatctcatgcggactcgctgcgcgcgacggccagcgcgtagccggcattgcgcagcgtcttgatgcagtccagcggctcgagcttcttgcgcaggcggctcaccacgatgtcgaccgcgcgggtgtagagctcggcttcatggccgcgcaggcggttcaggatgtcgtcgcggctgaagaccttgccgggctcggccgccagcagcgcgagcagctcgaactcggtgccggtgagttccacgcgctcgccgtggcgcagcacctggcgccggtcgagatcgatcgacaagccgtcgaacacgcggtgctgcgcactgttgccgttggccgccgcggcgggcgcgctgcgctggcgccgcaggatggtctgcacgcgcgccaccagttcacgcggctcgaagggcttgggcacgtagtcgtcggcgccgagctccaggccgaccacgcggtccatcacctcgccgcgcgcggtgagcatcacgatcggaatgtcgctttccttgcggatctcgcggcacagcgcaaagccgtccatctcgggcagcatcacgtcgaggatcgcggcgtcgtactggccggcacgcagcttggcgagcccttcgctcggacgcacggcgctttcgagcgtgcagccaaagcgtgcgaagtaggtggtcagcggcgcggcgagatgttcgtcgtcgtcgatcagcaggatgcgcggcatggcgggattgtgcctcctggcgaacaattggctgacgactaggcccgccggcattgcaccgccattgtcatttcgatagccggccaccgcggcgcgctgcattgtgcgaccttcaccacggatcggcccgcccgatgcggccgaggtgcgtggcgccgaagccggctgcgtacttgaggccgtagcccagcgcccggtcgaggccgatgtgcgcgcaccagatcaagccgccagccaccgcccatggcatcgcggcgagcacgccgagcaccagtagcgcaacggcgccggcgtacgagtgcgccgcgttgtagagcgccgcgcccacgcgcgggcccgcgaggtagccgagcatcgagaggtcgggcacgagcagccacagcgcgaacacgccccagccggcgccgaactgcgcataggccgccagcgccgcgcccagcacgaccaccccttcgagccgcagcagcgtgcgcacgccacccgtcgctgccactgcctggtcgtgggataccgcggaaccggcttcgccgggccgcaggtatcgcccccttgcagggggttggcgaagcgacacgaagtgcgcgaagactgggggtgagccaagcctagccacgatggccccagcggcgtccgccgcggtccatgaagtcgcgcaccttctgctgctgcgcggcattcaggctgtcgaagaaatcggcggcggccgcgatgatttcgggactgccgttgcgcacggccgtggtcttctcgtcgacgagccgcgcggcgcccgcctggtcgagcttgttgcctgcgaacagtgccttgaactgcgaacgcggatcgcccgcgccgcccgcgccacgcatcgcttcacgctgggcctgcagcttctcggccagcgcggtgagtttctgcttttgcagagtgtcgagttcgagcttgctgccgactcgctcgaccatcttggtgcggaactcggcagggtcgccgccgccccagccatgccgatggccggcgcagccggcaatgctgcccgccaccaccgcgaggcctgcgaaaccgaagagagtgcgtttgatccagtgtttcatgatgttccttgcggcccggggtcgtgtgcggcgggcgtgagtcttagagcttgctgctgctgttgccggcggctgcggcacgtgcatcgaccgggttctgcagcgtcgagatcaccttgctgttcactcgcgaacccgaggtcacgttctggtcgggtgcggcggcggtgcgcatggcttcgtagacgacgcccgcgcggtctctcgacacggccatggtctcggcgccgcgcgagccgcgcaccacgttctggtccggcgcggtggccgtgcggacggcttcggcgttgacttcggcgcggctcatcgccgatgcgagcggctggacgccttcgtaggattcagccttggcaccggccgcggccagcagggcgaaggagccgacggtgacgatctgggtgagggagagagatttcatgaatcaggcctttctgtcgttgaagaggagacctgatggtgcttgccgcgaggcgacaagtcctttcaccgcagtttcggcgtgtttcgttttatgtcgattcgccctgcttttgagcgaattgagtgcggaagacctaactatcccgccagggcggcggcgggatcgtccgattcgagcacgctcttggcccaggcttcgagcttgccggtgtcggcgcgcagcacttcctgcttgacggcgaggatgcgcgagggatgcatcgagaagctgcgcagccccaggccgagcaagaggcgcgtgaaggccacgtcgcccgccatttcgccgcacacggccacgcccttgccctggcggcggcattcggcgatggtgtcggccacgagcttcagcaccgccgggtgggcggggtcgtacaggtgggccaccgcttcgtcggcacgatcgatggccagcgtgtactggatcaggtcgttggtgccgatcgacaggaagtcgaagtacttcaggaaggtcttgagcgtgagcgccgcggcgggaatctcgatcatcgcgccgagcttcacgttgccgtagacagctccgcggccgtcgagctccgtgcgtgcgaagtcgatcagcgagagcgtctggcggatctcgctggcgtgcgcgagcatcggaatcagcaggtggatttcgccatgagccgccgcacgcaagatggcgcgcaattgggtgaggaacatggccggatcggccaggctccagcgaatggcgcgcaggcccagagcggggttcaggtgctcctgcttgctggccgccttgccgtcgatgggcttgtcggcgcccacgtcgatggtgcggatggtgaccggcatgccctgcatgccctcgaccgcgcgcttgtaggcctggtactgctcttcctcgtcgggcaggcgggtctgtcgctgcgactcgcggcccatgaaaaggaactcgctgcgaaacagcccgacgcccacggcgccggccttgacggcgccgacggtgtcttcgggcatctcgatgttggcgagcagctcgacgcgctggccgtcgagcgtcaccgcgggcttgtggcgcaggcgcgcaagccggccgcgctcgagatcgccctggcgctgcttgaaaccgtattcggccaggatgatgggcgagggatcgacgatcaccacgccggcatcgccgtcgatgatgacccagtcgtcctggcgcaccagctggctcgcggtgcgcgcgcccaccacggcgggaatgtccatgctgcgcgcgacgatggcggtgtgcgaggtgcgcccgcccacgtcggtcacgaagccggcgaacacgctcttcttgaactggagcatgtcggccggcgaaagatcgtgcgcaatcagcaccagcggcgcgtcgatgccgtcgcccgcggtggggtcgtcgtcgtcgtcggaggtggggcgcttgcggcgcggcgggctgggagcgagcaccgcggccgtgccctgcatgcggtgcagcagccgctcgaccacctgttcgaggtcggccttgcgctcgcgcaggtattcgtcctccatctcgtcgaactggcgcgcgatgatttcgagctgcgtggtcagcgcccattcggcgttgtagaggcgctcggtgatccagtgcttcacgccgccggtgagcgcctcgtcctgcagcagcatctggtgcacttcgagcagcgccgcgagttcgtgcggcgcatcgttggggcccatcagcgccacgttcgtctgcagcttggcgagctcgtcggccaccgcgttgcgcgccgtgcgcacccggtcgatttcggtgtcgacctcctcgggcttgatgaagtagtgggccacgtcgatgcggctggacaccaccagcaccgcgcggccaatggcaatgccacgggcaacggggaggccgtggactgcgaaagtcattcgccttcgccgaacttgtcgttcatcaactggatgatggcggccatcgcctcttcctcctgctcgccgttggtctccagctcgacggtcgagccgaggcccgcagccagcatcatgacgcccatgatgctcttggcattgatgcggcggtcgccgcgcgagagccacacctcgcaaggaaagctgcctgcgattttggtgagcttggccgatgcgcgtgcatgcaggcccagcttattgctgatggtcacggatttcttgatcactgtgctttctcttcgcctgattctggggtgccgccacggccacctgcatgacaccggccgtgccgcccgcgatggcgcgctgcaccagcgtttcgagcggctcgtggcggtaggtgaccgcgcgcagcagcattggcaggttgacgcccgccaccagccgcgagcggacaccgtccaccagcttctgggccacgttgcagggcgttgcgccgaacacgtcggccagcaccagcacctgcgagcgcggcgcattgagctgctgctccagggtgatccgggcggcggccagggtttcttcgggtgagacgttgggcagcacgtcgagtgcgacgacggcctgctcgcagtcggggaacacatgcagcgcgcaccgccgcagcgcctgcgcgaacggtgagtgggcgatgatgaggatgctgttcatgcgggtcggaggactacgcgccgattatgcgggggcgcccaaaggaagtaggtatacgacataacgcagcaggccagcaaaacggacagggccgcgtggaacgatcccacgaggtcgagcaaaaagccatcgccgccagcatctcacagcggggcccgctatcaaaacgagagcgcgcacgcgcattccgaacggcgggccgccgctcctgggaagtcaccgtgttcacggaaggcgcaggccttcgaagaaagtcttcgccgcctcgggggacgaaggccgcccgagcacggtggcctggtagagcgcgacgctgccgtctttttgggattgggcgaaccagagcacctggacgggcgcggcgcccttttgggctggctgcgcatcgagccgcactggcgcgggggccgcggtggcgcgctgcaatgcggcggggccttcggtcagctgcgcgccgcccaactgattgcgcgtggccgcgcgccacgcgacgagccaggcctcggcctgcgcggggctgccggcggatgcatgggcaacggcgaaggttgcgcccccggtctcgcagccagccatgtcgaccttcaccgattcggcaccgaacggcagggcacggttggcacggtctggcttgcagggcagcagggcgaccaggcccgcgtcggcaatcggcacctcgcgccagttgaaggtggggctgcaggcggccagggcgacggcggtggtggcggcgagcagcagaggccaggagcgggaagcgaacgacagcatcggagggcgattatcgagccgcccacggcacgccccggcacgttccgcccggcggaactaaaatcccgacgcccctctctctcagttgccatgaaaaaatacatcgccgtcgccgcagtcgcgcttgcattggccgccggcgtgggcgtgtacctggggtcgggcgccacagctgcgccagcgtcgaccttcgtgctgctcgacggaagcaagaagagcacggacgacctcaagggcaaggtcacgttggtcaacttctgggccacgagctgcgtgacctgcgtggccgagatgccgaaggtcatcgccacctacgacaagtacaagtcgaagggctacgacacgctggcggtggccatgagctacgacccgccgagctacgtcgtcaactttgccgaaacccgcaagctgccgttcaaggtggcgatcgacaacaccggcagcgtggcacaggcctggggtgacgtgaagctcacccccaccacttacctggtcaacaagaagggcgagatcgtgaagcgctacgtgggcgagcccgatttcgccgaactccacaagctgatcgagaaattgctcgccgaagcgtgaaccagaaggcgctccacggagcgccttctgtctttttgcgacggcttactggttgcggaagctgtcgtggcaggccttgcagctccctgcggtcgagccgaactgggccttgagcgcgtcgatgttgcccgccttggccgcgactaccagcttgccggtctcggcaatcatcttgtcctggtgttccttgaacttcgcggtttccttccagacctcgggcttgctcttgccgccttccgtgccggcagcgaaaccggcccagggaaacttggccacttcggccacgatatcggcgttggcgatagccgtggccgcgtcgtaagggatgcggccgttggccatggcaccgatacggctgaaatgctggcccatcacgaacagcgcgctctggcggtacttgatggcgtcctcgggcttggcgaactgggctgcggccggcagggaaatcgcggcacatgcagcggccagggcgaacgaagcaagtcgaatcatcgggggtccttgtaggtagtggagcaccgtcgaaagcggtgccgcgccgagtgtagaggcaccgttacagcgcgcatagcaacaacccgaagcatggagccgccggactttgctaatctgcgccttccgcagtttttgcgcaccttgccttctcgatgaccgactcttccgtggcctccatgccggccgcagcgtccgatccccccgtccgggcacgcatctgggacctgcccacgcgggtttttcactgggcgctgagcgccgcagtcgtcggcctgatcgccaccggcctcggcggcgtgatggagtggcacttccgcctgggctacacggtgctcgccttgctgctgttccgcctgttctggggcttcgtgggcgggcgctggtcgcgttttgcctcgttcttctatggcccgggctccgtcgtcgcgtatctgcgcgggcgggcccatccccatcatgtgatcggccatacgccgctgggcgccctctcggtgttcaccgtgcttgcggtgcttgcggtgcaggtaggcacagggctggtggcggacgacgaggtctcggccgcggggccgctgacgcgcttcgtttcgagcggcgtggtgagccttgccaccggctggcacaaatcgcaaggcaagacgctcgtgattgcgctggtgagcctgcacgtgctggcggtgctcttctacgtgctggtcaagcggcatcgcctggtgcggcccatggtttcgggcgacaagctgatcgccgcgaccggtgccgcaggccaggtggcgccaagccgcgatgacgccgtgtcgcgcgggcttgcgctggtgctgttcgccgtgtgcgcaggcgtggcgtattggattgcgtcgctgcgcgtatgagttcctcggtttcacgcccgctgccactggccgacacgccggccgtcgtgcttttgacgcccgacgaagctcacgagatcgatgcaacgcgcgcgatctttcgcgactacgccgcttcgctgggcatcgacctgtgcttccagaatttcgacgaggaagtggccggcctgcccggcgactacgcagagccgcgcggcgccctgctcctcgcgctggtcgatccggcccatatcaaggaggccaccggacaacaggcgccgaccctcctgcgatccgatggaacgctggcgcacgtggcgggctgctgcgccctgcgcccgctcgacaatgccgactacgccaattgcgcggaaatgaagcggctgtacgtgcggcccggctttcgcgggctcggtgtcggccggcaactcgccgaagccatcctcgacgccgcgcgcagcgcgggctatgcctgcgtgctgctcgacacgctggacgacatggaatcggcccgcgcgctctacgaagacctgggcttcgcggaagtgccgccctactatcacaacccgattgcgggcgcgcactacctcaaggcggagctttagccgcccctttggccgccagtcctcagccgcgggcttgcgccagcagcgtctctgcgttgctgacctcgaacttgcccggtgcctcgacgttgagcgaggccaccttgccgtccttcacgagcatcgaatagcgattgctgcgcaggcccatgccgcggccggtcaggtcgagcgtgaggccggtcgccttggcgaaatcggcgctgccgtcggccagcatgcgcaccttggtgccggtcttctggtcgcgcgcccaggcacccatcacgaaagcgtcgttcacgctcacgcaccagatctcgtccacgccggcggccttgaagtcgtcgaagtgctgcacatagccgggcacatgcttggccgagcaggtcggcgtgaaggcgccgggcagcgcgaacagcgcaatggtcttgccggccgtggccttgctcacgtccaccgggttcgggccgatgctgcagccttcgccctcgacctcggaatactcctgcagggttgccgaaggaagggtgtcgccgactttgatcatctgaatgctcctgaaaaagaaaaacggcccacattgtgggccgtttccggatgggttgccttcacgaggcttcccgaggtcgatcaaccagtgatcagaccagcacggccttctcgaccagacgggtcacgacccagttcttggtcttcgagatcggacggctttccgtgatttcgatggtgtcgcccagcttgtactcgcccttttcgtcatgggcgtggtacttgctcgtcttggccacgatcttgccgtagagctcgtgcttcacacggcgctcgaccagcacggtcacggtcttggcacgcttgtcgctgaccaccttgccaatcaaggtgcgcttgagggattttttagcttccgtcatgttcactccttacttggcggcttgggtttcttgctgcttctgagcaagaatggtcttggcgcgcgcgatgtcgcgacgcgtcacgcgcagcgtcgaggtgttcgacagctgttgcgtggctttctgcatgcgcaggccgaaatgggccttttgcagttccttgacttcggtttgcagcgctgcgacgtccttcgtgcgcagggttgcagccttggtcaccttggccggagccacggtttcttttttcttacgtgttgccatggatgttctcctctcaggcgccgagctggcgagcgacgaacgtcgtgcgcagcggaagcttggcggcggccaggcggaacgcttcgcgggcgagttcttcgggcacgccgacgatctcgaacacgatcttgccaggctggatttcagcgacgtagtactcggggttgcccttaccgttacccatccgcacttcggcgggcttggtagagatcggcttgtccgggaacacgcggatccagatacggccaccgcgcttcacgtgacgcgaaatcgcgcgacgagcggcttcgatctggcgcgccgtgaggcggccgcggtcggtgcatttgagaccgaaatcaccgaaggcaaccgagttaccccgggttgcgacgccggtgttgcggcccttttgttccttgcggaactttctgcgtgcaggttgcagcatttttaatactccgtagttctaagaccgatcactcggtcttggcaccgtcagctgctgcagctggcgcggctttgcggacgcgcttaacggcgggtttcgagtctgcacccggagcagcgggagctgcgccagtggcttctgcgggcttgtcgctgccgtcggccggggcggtgttgccaccgatcgggccacgggcaccggcgcgcgggccgggaccacgacggtcgccacccggacggtcgccaccagggcggccatcacggcggggaccacgcggacgacgctcatcgtcgggacgcggcgtttcgacggccggcaggtcgttacgacccagcgtgtcgcccttgtagacccagaccttgacgccgatgacgccgtaggtggtcttggcttccgaggtgccgtagtcgatgtcggcgcgcagggtgtgaagcggcacgcgaccttcgcgataccactcggtacgagcgatttcgataccgttcaggcggccagccgacatgatcttgatgccttgggcacccagacgcatggcgttttgcatggcgcgcttcatggcgcggcggaacatgatccgcttttcgagctgctgcgtgatgctgtcggcgatcagctgggcatcgatttcaggcttgcgcacttcttcgatgttcactgccaccggcacgccgagctgcttgcccagttcgcgcttgaggttctcgatgtcttcgcccttcttgccgatcacgacgcccggacgagccgagtagatcgtgatgcgtgcgttcttggcgggacgctcgatcatgacgcgcgacaccgaagcgttcttcagcttcttcttcaggtattcgcgaaccttgatgtcttcggccagcatgcccgcgaaatcgcggtcgcttgcgtaccagcggctggaccaattacgggtaaccgcaaggcggaagccggtcggatggattttctgtcccatatttcttccaggcgttcttagttgccaaccgtcacgtacacatggcacgtgggcttgctgatgcggttaccgcgacccttggctcgcgccgtgaagcgcttgagcgtggcaccttgttcgacgtagatggtcttgaccttcagttcgtcgatatcggcgccatcgttgtgctcggcgttggcgattgccgactcgagcaccttcttgatgatcacagcggcttttttctgcgtgaattgcagaacgttgagcgcttgatcaaccttcttgccgcggatcaggtcagcgaccagacggcccttgtcgaccgagaggcggacaccgcggaggactgcacgtgtttcagacatggtcgttccttacttcttctggactttcttgtccgcggggtgccccttgaacgtgcgcgtgagcgcaaattcgccgagcttgtggccgaccatctggtcggtgatgtagacaggcacgtgctgcttgccgttgtgcacggcaatggtcaggccgatgaactcgggcagaaccatcgagcggcgcgaccaggtcttgatcggcttcttgtccttcgtcgtcacagccttgtcggccttggccacgaggtgatggtcaacaaacggaccctttttgagagagcgagtcatttgctatcccttacttcttgcggcgcgacacgatgaagacctgcgtgcgcttgttgttacgggtacggtagcccttggtcaggttgccccatgggtcgacaggatggcggccttcgccggtcttgccttcgccaccaccgtgcgggtggtcgaccgggttcatcaccacaccgcgaacggtcgggcgaatacccatgtgacgcttcacaccggccttgccgagttggcgcaggctgtgctcttcgtttgcgacttcaccgatggtggcgcggcattcgatgtggatgcggcgcacctcacccgaacgcatgcggacctgggcgtagacgccttcgcgagccagcagcgtggccgacgtgccagccgaacgcgcgatctgcgcgcccttgccgggttgcagttcgatgcagtggatcgtcgagccgaccggaatgttgcggatcggcagcgtgttgccggcgcggatcggggcttccgaaccgctcagcagcgttgcaccggcttcaagaccgcgtggggcgatgatgtagcggcgctcgccgtcggcgtagcagaccagggcaatgtgggcggtgcggttcgggtcgtattcgatgcgttcgaccttggccgggatgccgtccttgttgcgcacgaagtcgacaacgcgatagtgatgcttgtgaccaccgccgcgatggcgaatcgtgatgtgaccgttgttgttgcgaccggcagcctggaactgcggctcgagcaacggcgcgtgaggggcacccttgtacaggtggtcccgcgaaatcttcaccgcgccgcgttggcccggcgaagtgggtttcatcttgatgacagccatgattaagcgccttccccgacgaggttgagctcttgaccgggcttcagggtcacataggccttgcgaacgttgtcgcggcggccgatggacttgccaaagcgcttggtcttgcccttggtgttgagcaccgacacgccctggacttcgaccttgaacatcagttcgacagcggccttgatctcgggcttggtggcgtcttgcagcaccttgaaagtgacagcgttcgacttctcgccgaccatcgttgccttttcggacacgatcggggcgaccagcaccgccatcaggcggccttcttcgaacgtacgttcagcggcggtagggttcacgcggctcatgcgaacatctccttgagcttgtcgacggcacccttggtgaccagcaccttcttgtagtggaccagcgacaccggatcggcgtagcggggttcgaccacgagaatgttgaccagattgcgcgaggcaaggtacaggttttcgtcgacttcttcggcgatcacgagcacggactcgagattcattgccttgaaacgggctgccagcggcttcgtcttgggcgaatccacggtcagcgaatccaccacggccagacggccttcgcgagcgagctgcgagaagatggcggccatgccggcgcggtacatcttcttgttgatcttctgcgagaagttttcgtcaggcatgttcgggaaaatccggccacccccgcgccacagcggcgaggacgtcataccggcacgggcgcggcccgttcccttttgcttgaaaggcttcttggtcgagtgcttgacctgttcgcggtccttctgggcgcgcgtgccttggcgggcgttggcctggaatgcaacgacgatctggtgaaccaggtcttcgttgtagtcacggccgaacacggtctcgggggcgtcgtacttcgacgcggcctggccttgttcgttcaggagttcgagttgcattacttcgctccttcggccgcttgcggcttggccttgatggcgggacgcacggtgacgaagccaccctttgcgcccgggatcgcgcccttgatgagcaacagttgacgcgcttcgtcgatgcggaacacatcgaggttctgcgtggtcttggtgacgtcgccgaggtggcccgtcatgcgcttgccggggaacacgcgaccggggtcttgtgccatgccgatcgagccgggaacgttgtgcgaacggctgttaccgtgcgacgcgcgttgcgagctcatgttgtggcgcttgatggtgccggcgaagcccttgccgatcgaggtgccttgcacgtcgaccttctggcccaccgagaacacgctgctcgcggcgatgacgccgccagccttgtgctggtcagcggtgtcggcggtcacgcggaattcgcggatgatttcaccagcttcgacacccgccttggcgaggtggccggcttgcggcttggtcacgcgcgatgctttgcgcgaaccgaacgtcacttgcagtgcgacgtagccgtcggtctcttgcgacttgatctgggtcacacggttgttggacacatccaccaccgtgacaggaactgcgtccccgtcatcggtgaagagacgcatcatccccaccttgcggcccagcaacccgagggagttgctcagactcatttgttttctccaaaaatggaagctcccttcgccgctgccacttcaattggcgacagcgtttggccgattccctgggggcaccggcctgcgaaagaaggttgataaatctctactcccatggcgtccgcatagacgcaacaagggcagagccagcgattatagcccgctatgcatgcgcagtgcaagcagcgttgtaaagcgatcccggggcgtgttcagccccgaaaagtgctgctttttacctatttgaccggcatcgtgatgatgccgtcaccgcccggcgtgcgcttcatctcacccgtggttttctgggccggcgttgctgttccggtctggatggggacggaaatcgcgctcgacgccccgccctgggtgatgaacacattgaggtaggccaggccttcggcctcgctcaccacgacgacggtggccgtggttcgcttgcccgacggcagcgtcagcgtgctgcttccctggagcgtcagcccgcggtcggcactcaggcgcaccgtggcgccttcagcctcggtcacgtcatcgaactgcagcacgacgggcgtcgcccggcccacctgcggcgtggcgtcgaggcggtattggagcctgacgccggaacttccgggcttttgcggtgcggtggtcatgggcgcggtgcggtgctgtgcccccgcatgcctgggcttggcgctgcgcgccgcagggtcgccgtccgccgcggccggcgccggcaacgtggccagcgccaggcacgcgatggccatcatcgaattcgaacggatgttcatggcggcctttcttgcctttcctgctactggatggagactttgaagcatgtcagcgctccggaattgttgaggtccgacacggcaagaacgtattcgccggacgacaggctgactgcgttgctttctcgagcgatgaacccgcccctgaagaggtcgaaatcgggattcgagccggccggacctccgttgaccacgatctggtagctgcggctggcgggcgcggtgaagcgaaggtaggagaagctgcccagcttgttgtcggtaccggccgaactggaaacgcaggcctgggtcggggcgccgcctacggccgcgagcctgtacatcggcagcgtgatcgggattccgccatcgttcgtctccgcgccgccatagggatcgttgcccgtcgcgtggatgtcttgcccggcgagcagggttgccagcgatgcggcgctcgtcggcgccgtcgcattgaaggccgccgcgaacggatgaatcgacgtgacggcagtaccgctcctgaactgacttccggtcagcgtgtcatggatcggcttgaaaccgacctgctggttgagattccagaaaatcgactggatcgaaggctcgcggtaccagcccggcgtggtcggggggcccgcagcgaggtcgatgttggtgctgaactgcgccgccgactgctgggggccgcccgagtcgacatagttccggcgctcgagcgcgatgcccgaccaggcgttgccccagccctcggagaaggcgagccggcgatcgaggcgctggccctgcgaatgggagccgcccatcgagtcgtcgcggctgaaggccgattggtagtaatggccccattcatgcgcgatcaccgaattgtcgtattcgtcggtatccacgtcttccttgccgagcacatagatttcgcggccgctgcttctgttgacgaagaatgtggtgccgatctgccctgccgcgacgctgccgggagaaggcgcattgttgatgctccagtacacgcgcagcaccggaaacgccgtggccggggcgaccgacaccaccttctgcatggcggcgtagaccgtgtcgaggatggcaaaaggtcccgccacccgatcgcccgtatagcctgagccaccccaacccgagggcgcatggatgtcgcgcaccattgccaccgcacccgatgagaaagcggggctctgcatgctgtacagcgtgccggaccggacgttgtcgcgcacggtgacatcccagctcgcacctggaccgctacgggccagttgggcgttgacgcgcaccgcgatcgccgtgtttgcgggcacggacaccgagtaggcaccgttgtcgtcggtggtcgccgcggccagttgcacggagcttgccgcatcgagcacttccagcagcgcaccgcgcaccggcttgggcgtggcgctggcataaaccagcgtgccattcgggttcggaacggattcataggtggccgtgccgctcagcgtcaccgcgctcgacgtgccgggcgctaccggcaagaagggcagaccaccaccgccgcctccgccgcccccaccaccgcaaccggccagcagcgctgctgccgtgatgcacgccatcacccccgacgcaaaagagataccttgtctcatgctgtgctgcctcttgcctttccactgacccgtgccttcccatggatggagaggccgccgccccggcgaggatgccacatcggcgctacaaaaaaacaaagcccgcctgcatttctgcagtcgggcttcatcaagaacgcggcgcgaggccgcggtgcttattgcagcttgatttcgacgtccacgccggccggcaggtcgagcttcatcagcgcgtccacggtcttgtcggtcggatcgacgatgtccatcaggcgctggtgcgtgcggatctcgagctggtcgcgcgacgtcttgttgacgtgcggcgaacgcaggatgtcgaaacgtttcatgcgggtcggcaggggcacgggacccttgacgatcgcgccggtgcgcttggcggtatcaacgatttcggctgccgactggtcgatcagcttgtagtcgaacgccttcaggcggatgcggattttttgcttggtagccatgatgattcctttgcgtccggcttagatgtcgaggatcttggccacgacgcccgaacccacggtacggccgccttcgcggatggcgaagcgcaggccttcttccatcgcgatcgggttgatcagcttcacggtgatgctgacgttgtcgccaggcatgaccatttccttgtccttgggcagctcgatcgcgccggtcacgtccgtcgtgcggaagtagaactgcggacggtagttgttgaagaacggcgtgtgacggccaccttcgtccttggacagcacgtacacctcggcggtgaagtgggtgtgcggcttgatcgagccgggcttgcacagcacttggccgcgctcgacttcttcgcgcttggtgccgcgcagcagcacgccgacgttgtcgcccgcctggccttggtccagcagcttgcggaacatttccacgccggtgcaggtggtcttgacggtcgggcggatgccgacgatctcgatttcctcgccgaccttgatcacgccgcgctcgacggcgccggtcacgacggtgccgcggccggagatcgagaacacgtcttccacgggcatcaggaaggtgccgtccacggcgcgctcgggcgtcgggatgtaggtatcgagggcttcggccagcttcatgatggcttcttcacccagcttgcccttgtcgccttccagggcgagcttggccgagccgtggatgatgggggtgtcgtcgcccgggaattcgtacttgtccagcagctcgcgcacttccatttcaacgagttcgagcagttcggcgtcgtcgaccatgtcgcacttgttcaggaacacgatgatgtagcccacaccgacctgacgggccagcaggatgtgctcgcgggtctggggcatggggccgtcggcggccgagcacacgagaatggcgccgtccatctgggccgcgccggtgatcatgttcttgacgtagtcggcgtggccggggcagtcgacgtgagcgtagtggcggttggccgtttcgtactcgacgtgggcggtgttgatggtgatgccgcgggccttttcttcgggcgccgcgtcgatctggtcgtaggccttggcttcgccgccgaacttggccgacagcaccgtggcgatggccgccgtcagcgtggtcttgccgtggtcgacgtgaccgatcgtgcccacgttcacgtgcggcttggtgcgggtgaatttaccttttgccatttttcaatccttgaaagagcattcccgtgtattggttttatgtctgcacccgattgctggttcgcctcgcacgggaacgcggcggcaccggatcgcagacaacgagagccgcgcactgcgcgaccccacattctttttagtcagttggggacagagcaaatttgctgcgcaaatcctggtctgtcccgcaaagacattacttagcgcgagctgccacgatggcttcggcaacgttgcgcggagcttcagcgtagtgcttgaactccatcgtgtacgtggcacggccttgcgacatcgaacgcagcgtggtcgagtagccgaacatttccgacagcggcacttcggccttgatggccttgccgccaccgatcatgtcttccatgccctgcaccatgccgcggcgtgaggacaggtcgcccatcacgttgccggcgtagtcttcaggcgtttcgacttccacggccatcatcggctcgagaatcacggggctggccttgcgggcgccttccttgaaaccgaagatggcggccatcttgaacgccatttcgttcgagtccacgtcgtggtacgagccgaagtgcagcgtgaccttgacgtcgacgacggggtagcccgccagcacgccctgggtcagcgcttccacaacgcccttttccactgcggggatgtattcgcgaggaaccacaccgcccttgatggcgtcgacgaactcgaagcccttgcccgcttcctgcggctcgagcttcaggatgacgtggccgtactggcccttgccgcccgactggcgaacgaacttgccttcggcatcttcgaccgtcttgcggatcgtttcgcggtaggccacttgcggcttgcccacgttggcttccacgccgaactcgcgcttcatgcggtccacgatgatttcgaggtgaagctcgcccatgccggcgatgatggtctggcccgattcttcgtcggtcttgacgcggaacgacgggtcttcctgtgccaggcgttgcagggcgatgcccatcttttcctggtcgaccttggtcttgggctcgacggcctgggagatcaccgattccgggaacaccatgcgctcgagcgtcaggatggcggcgggatcgcacagggtttcgcccgtggtcacttccttcaggccaatacaggcggcgatgtcgccggcgcggatttcgctcacttcgacgcggttgttggcgtgcatctgcacgatccggccgatacgctctttcttgccacgcaccgggttgtagacgctgtcgcccttggtcagcacgccggaatagacgcgaacgaaagtcagctggccgacgaacgggtcggtcatgagcttgaaagcgagcgcggagaacttctcgtcgtcgtcggccttgcgggtcgtcggcacttcgtcttcgtccatgcccttgaccggcgggatgtccgtcggtgcgggcatgtattcgacgacggcgtcgagcatggcttgcacgcccttgttcttgaaggccgagccgcacagcatcggctggatttcgccagcgatggtgcgttggcggatcgcagccttgatttcggcttcggtcagctcattgccttcgaggtacttgttcatgagctcttcgctcgcttcggcagcggcttcgacgagcttttcgcggtactcggcgcacacctcggccaggtcggccgggatttcgccgtacttgaaggtcacgcccttttcttcgtcccagatgatcgacttcatcttgaccaggtcgacgatgccctggaagcgctcttcggcgccgatcgggatctggatcacgacggggttggccttcaggcggtccaccatcatctggcgcacgcgcaggaagtcggcgccggtgcggtccatcttgttgacgaacgcgaggcgcggaaccttgtacttgttggcttggcgccagacggtttcggactggggctgcacgccgccgaccgcgtcgtacaccatgacagcgccgtccagcacgcgcatcgagcgctcgacttcaatggtgaagtccacgtggccgggggtgtcgatgatgttgatgcggtgttcgtcgaacgtgcccgccatgcccttccagaagcaggtggtggcagccgaggtgatcgtgatgccgcgctcttgctcttgctccatccagtccatcgtggcggcgccatcgtgcacttcaccgatcttgtggttcacaccggtgtagaacaggatgcgctcggtcgtcgtggtcttgccggcgtcgatgtgcgcggagatgccgatgttgcggtagcgctcgatgggggtcttgcgggacatgatttactttcgggttaaatgcgttgagcgctgggccctgagcccgggcgacatcgcccgacactcaacgcccaacgcccaagcgaagtttgattcttagaagcggaagtggctgaacgcccggttggcttctgccatgcggtgcacttcgtcgcgcttcttcatggcgccgccacggccttccgtggcttccatcagttcgttggccaaacgcaaggccatcgacttttcgccgcgcttgcgggcagcttccttgatccagcgcatcgacagggcgaggcgacggacgggacggacttcgaccggcacttgatagttcgcaccgccaacgcggcgcgacttcacttcgaccatcggcttcacgttgttgatggcaacggtgaacgcctcgagggggtccttgtccgggttcttcttctcgatgaattcgagggcaccgtaaatgatgcgctcggcaacagccttcttgccgccttccatgatcacgttcatgaatttggacagctcgacattgccgtacttgggatccggcaggatttcacgtttggggacttcgcgacgacgtggcatgttactaacctctttgcttcagttggcaccgtttccggcaccgcgagagccattccggactctcacttactcgacccgacattgggtcactccgttcgatgtgcccgccaaggcaaccgaacaccatttgtttgttttttacgacaggaaggcttacgccttcttgggacgcttcgcgccgtacttggaacgcgactgcttgcggtctttcacgccttgcaggtcgagcgagccgcgcacgatgtggtagcgaacaccgggcaagtccttgacacgaccgccgcgaaccagcacgacgctgtgttcctgcaggttgtggccttcgccgccgatgtaggaaatgacttcgaagccattggtcagacggaccttggcaactttacgaagcgccgagttgggcttctttggcgtcgtggtgtagacgcgggtgcagacaccgcggcgttgcggcgagttctgcatggcagggctcttcgaattgatcttttcgaccgttcgaccctgacgcaccagttgattgatggttggcatgaatgaattagtcccaaaacaacccggctttggctgtgaaccgcccttgtcgtgactcaaggaagccgggaataacgaaaacgtgaaacccttcggaaaattccgaaaagcccacgagtatagcagtccaccccgccgtcagcaattgctatgcgctggcatcacttgatccagagccggacggcatcccaggcgcggccaaaaatacccgcctgctcgacgccttccagcgccaccagcggcacatcggccaaaggctggtcgtccagggtcaccttgagcgagcccacgggctggtacttggtgaacggcgccaccagcggatcggggcgcgccacctgggtcttgatcttgttggcggtacccgccggtaccgccaccacgatcgcttccggacggcccagcttgagcgtgttggccttgcccttccagaccgccggcgtggcggccggctggccggcgtcgaacaggcggacggcgtcgtaggcggtgtagccccagttcagcagcttttgcgactcgttggcgcgcacggtttcacccgaggtgcccagcacgatcgacagcaggcggcggccgccggtcaggttggggaagtcgcgcttggcggtggcgatcatgcaatagccggccgcctcggtatggccggtcttgaggccgtcgacggtcgggtcgcgaaacagcagcaggttgcggttggtgtcgttggtcgagggcgtgccggggtagcggtacttcttgatggcgtagtacttggcttcttcggggaagtctcgcaccaggcgcgtcgcaagaatgctcaggtcgcgcgccgtggtggtgtggccgggcgccgtgaggccctcggggttcttgtaggcagtgttcttcatgcccagcgccttggcctgcgcattcatgagttcgacaaaatgctccaccgtgccgcccacgccttcggccagcgccaccgtggcgtcgttgcccgactggacgatgagccccttgatcaggtcttcgaccggcacctgcatcttcgggtcgatgaacatgcgcgaaccgggcatcttccaggcgcgctggctgacgggcaaggtctgggtcagcgtgatcttcttggcgcgcagcgcgtcgaacacgatgtaggccgacatcagcttggtgagtgaggccggctcgaccgggctgtcgatgtccttctgggcgaggatctggttggccgtgatgtcgagcagcaggtagctgcgcgcggcaatttccggcggtgccggcacctgggcagcggcaatcatgcagaccgaagcggcggcgcccagcaccagggcgcgaaacgcggcaagaaaacgattcatgggagagattgggagaaaacgaaaacaagcccgcagggctttcatgcgatgcccgcgcgcagatggcggacgaccagacttttgagcagcggcaattgtccgtgaaagaaatggccgcccccggggacaaccgtgacaggaagtgactgcggccgcgcccagtccatgacagccgacagcggcaccgtgtcgtcggcttcgccgtggaccaccagcgtgcgctcatgtgcttcggccggcagcgtggccacggaaaagcgcgaggccgccgttccaacgagcacgagctgccgaatgtcacgagacgcccagagcttttcggccgcgcagctcgccacgaaggcgccgaacgaaaacccggcgatggccagcgggccctcgggggcgagccgttcgacgacgttcagcatgtcttcgcgctcaccgcggccttcgtcgtgcacgccctcgctcgcgcccacgcctctaaagttgaagcgcaccgcggtccagccgcaggcgacgaatgcacgcgccagggtctgcaccaccttgttgtccatggtgccgccgaacaacggatgcggatgggcgatgaccgcgatgccgcgcgcgccgtcggccgcggacggctggtcgcgctgcacctcgatgacgccggcggcgccctggaggcggatcttttcggtctgggagttcatggggctgggaatggaacggcccggcggcggcgggctgggtggacggtacgagcgcgggacttccggaaaagttcagcggccgacatcgggaggcagcacgaggcgctcgacgaccttgccgttcttcagatgcgactcgacgatttcgtcgatgtcttcggcatcgacgaaggtgtaccagaccgcctcggggtagaccaccgccacgggcccgccggcgcaccgatcgagacagccggccttgttgaccctgactttgcccgggccggccaaccccgcttcctttacctttgccttgcagcggtcgaagccttgctgggcgttgtgcagggcgcagcagtcttcaccgttcttgcgctcgttgaggcagaagaagatgtggcggccgtagtagccgtgcggcgcggcgggagtggaactgggcatccatcgattttagtgacgcccgccatgcgccatcgatcaccctctcaaccggcttggcggccgcggcgcgacagggcggccaccacataggccagtaccgcaaacggccacacccaacccagccactgcgccaggccgtgaaagcggatgaagcgcccctgctcccaggtggccagggtctgggcgaaatacgcgctctcgggcgcctggttcaaaaggctcagctggatcaccaggcccaccagcagcaaggccgcgcacagccggcgcggagctcccagcagcagcatgcctgcgaacaaggcgctcgcaatgccgacctgcaccggcaggcccagccaggcccatgcatgttccggcccgtaactcatggccgccgacagcgccgaggcgccaatgccggccagcagcgtgagcggcagcagcacggcacgacgggccaccgtgcgcgtcaccaggaaggccagcaggcaaggcaccagggccccgagcatcacgcacagcagttcggcggcgggcaccagcggctcgagctcgaactgtcgaagcggcatccagtcgatgaaaggcgtgtcgagcagccactccgagattgcgacctcgagccgctcgaacacctggccgagcccgaaggtcacggccgccggaaacaaaagcgcgatgggccacagcgccagcagcaccagcgcgccgcgagactcttcgacgaaccattgcgagcgcgtgcggctccagtgcgccaccgcgccaaggcgctccaggcccaccgccagcatggcccccagaagggcgccggaggtgttcagccccaggtcgacattggaaggaatgcgcgccggcaaatagctctgcagcgtctccatcgcaaaggccaccgctgcgccggccaccgtggcgcgcagcatggcgcgccagacgctcgcgtcgcgtcgcgtgcgcagcacggccagcgcgcaaagaaagccgaagggcacgtagccgccgacattgaccgcgaaatcgaagcccgtccagtacttgggccacgacgccgacaaataggcccagggtgcaatgccctggtcgcgccagtcggcaaacggataaaggctggcatagacgatcaacgccgcataggcgagcgcaaggggcagcgcggcggtcttgtgctgcgtctccaccttggcggctcagaacggcttgacgaccaccagcaccacgatgcaaagcagcagcaggacgggcagttcgttgaaccagcggtaccagcgatggctgcgctgctggcctccggccacgaagcggcgcagcagcacgccgcagccatggtgataaccgacggcggccaggaccagcgccagcttggcatgcatccagccgttgcccggtccgcgtccgatgccgtagcccagccagagccaaagaccgaaacccaaggccggaatggccaggaaagtcgtaaaccgcaacagcttgcgcgccatcagcagcaagcgctcacgttcggcaacggactccggcggcaccatcgccagattgacgaatatccgcggcagatagaacaaccccgcgaaccagctcgcaatgaagacgatgtgaaaagatttgacccagagcatgccggcagtttagtggtcggctgcgcccttccggcctttgcccgccggaacgggcgcagcgggcaaaaaaaagcccgacgtctgcacgtcgggctgggaagcccttttgctgtcacacatcaaggcacccgctcagggaggaaaagcggggagcggcaagccgcccgctttagaatttaacaaagacgaaacaaggtttcaagcgaaacggccactttctttgacatttccacgcaaaaaaagagaaccttcgggctaccgattcgaggggtgatcagagcgccttctcgcaggacggctcatacgtggattggcgcttcaggcacaattttccgcttatgacgccctcctccttctcctcctttgccatgtaccccgccggccggccgcgccgcctgcgccgcgatgccttcacccgcaacctggtcagggagcatgcgctgacggcgcacgatttgatctaccccgtgttcgtgcaggaaggcgagaaaaagcgcgatgccgtgtcttcgatgcccggcgtggaccgcctgagcctcgacctgctgctgccgctggcggagcagtgcgtggaagccggcattccggtgatggcgctttttccggtcatcgacgccagcctcaagacaccgtcgggcgacgaagccttcaaccccgacgggttgattccccgggtggtcgcggcgctcaagtcgcgctttccggagctcggcgtgatgaccgacgtggcgctcgacccctacaccagccatgggcaggacggcctgctcgatgagaccggctacatcctgaacgacgccaccgtcgaagtcctggtgaagcaggcgctcgcgcaatcgcaagccggcgtggacatcgtggcgcccagcgacatgatggacggccgcatcggcgccatccgcagcgcgctggaagcccgcggcgacgttcacacccgcatcatggcttacagcgccaagtacgccagcgctttctacggcccgttccgcgatgccgtgggctcggccgcgacgctcggcaagagcaacaagaaggtctaccagatggacccgggcaacagcgacgaggcgctgcgcgaagtcggcctcgacatcgccgagggcgccgacatggtgatggtgaagcccggcatgccctacctggacatcgtgcgccgcgtgaaagacgaattccacgtgcccaccttcgcctatcaggtgagcggcgaatacgcgatgctcaaggccgctgcgcagaacggctggctcgaccacgacgcggtggtgctcgaaagcctgctcgctttcaagcgcgccggcgccgacggcgtgctcacctacttcgcacttgacgctgcacgtttgctacaaaaacaatagctcaccaccttctggatccgcggaggcgggcccgaacggcaatgaaagagagcaacaaggcggtccatgcgcatcattgaaatcaaccgctcgcaggtgagcgagcaccaggcgctggcgccgctcacggtgccgggcgcctgcggcgcgcaaggctatctctggatttcgctgacgcgggaggagtttcgcgcctcgctgccggaagttcagcagatcctgcagtcgctctgcctcacccaactggtcgacctgcatgtggccgacctgctcaacgaccagttgccttcgcacttcgactacacctcgaaatacgacgtgctggtgttccggcgcctctcgagcggcccaggccagacggcgccgggcaacggcaaggggacggtcagcggcgagccgccccttgccgggcgccgcggcccgccggtgctgcgccgggtcgacacccgcccggtgggtttcgccgtgttcgaccgcgtgctgctctcggtgcaccccgaggacggcgcggtgcgcgacgcctttgccgcccggctgctggcggccgggtcgcccgacggcctgggcgccccggcgctcgacgtgcgcgccacctcggcccgggtgccgaccggcactgccgacctgatgcttcgggtcatcaaccagatcgtcgacggttacctggacatgcgccgcgagctcacccgccagctcgaccattggcagaccgagctgatcgatccgcgcagccgcttcaccaactggggcgcgctgatggaaacccggcagtcgctgcaccacctggacgaaatctgcgaggaccagcgcgccgccatacaggactggatcgatttgctcgaaaccttgccgtcgccgaaaggcgaggcagagcagcgcgagcgggaactgatcatggtgcgaagccgcgacgtgctcgagcacatcgagcgcgtggtgcatcacgtgcgccggctcgagcagaacgcggaaaccgcggtgcagatgcatttcagcgtccagggccaccgcgccaacgacatcatgcgggtgctcaccgtgctgaccgccatcttcctgccgctcaacctcattgccggcatcttcggcatgaacttcgagttcattccgctggtgcacaaggcggacggtttctggatcgcgatgggcgcaatgttgaccatcgcggtgctgctggtcgtgattttctggcgcaagcgctatctcgcgcgaacacgctgaccacccgccccaacaaaaaaagccacgctttcgcgtggcttttctttcttcaagcagccccgaagggcccgcttgccttgccggcttacttggcgacggcgcccgagccttgctgggcttgaacgcgtgcgtccatcgggtggggcatcgtcgagatgaccttgctgttgacgcgcgagccgccggtcacgttctggtccggtgcgtaggcggtgcgaatcgcttcggcttccacgatggcacggtccttcgacacggcaaccgtttccgggccgcgcgaaccgcgggtcacgttctggttcggagccgctgcggtgcgcacggcttcggcgttcacttcgtcacggctcttggtcgagacggcggtgttcacgccatcgtagctttcagcttgggcgccagtggcggccagcagggtcagggcggcggcagcgaggatgtgcgaggtcttcattttcagttccttgtgttggttggatggttcgtccaccaggctcgctcgttcgctcacctgtgcggcgagtttccagctgaaagagccccgcaaaacacgtggaacagagacaccgtgtttcctctattgaaacaatgacaacccaaaggcatgcacccgattgagtgagcgcttcgcggctgcaaaagccgctttcccggaaaatcaaggcacgccggtcccggaacggaaacaatgggcactttgacatggacagtctcgatctgatcagaaccttccgggaggttgcttcgcagggcagcttttcgaatgcggccaagaagctcgacatgtcgaaagccaccgtcagcaaatacgtggcggaactcgaaacgcgcttcggcgtgcgccttctcaaccgctccacgcggtcggtgagcctgaccgacgccggccaattgctgctcgaacgcagcactcccgtgctcgagatggtcgaactcacgcaggccgagttgcaggagcgcgccaggcagcccggcggacgcctgcggatttcggctccgcacggcatgggcaatggcgaatttccgagccttttggccgacttcatgcgctactacccggacgtgagcatcagcctgcagctgaccaaccgcacggtcgatctggcggaagaaggcatcgacgtcgacatccgcagcggcccggtcgcggatgccaacctgatcgtgcgcaagctgatgctcatggagatggtggtctgcgcatcgccggtctactggaagaagcacggcaagcccgagcatccgcgcgaccttgccggtcacgaggcgctcacgcattcgttgctgggcgcccaaccggtctggcgcttcgacgatggcggccagccgctggacgtaccggtgaagagccgcatggactgcaccgagggcgcgccgctgatccgggtcgcaatgcgcggcttcggcgtgatctacctgccgtcgatcctcgtgcagtcgcacatcgaccacggcgaactggtgccggtgctgcaggactatgcgcgcaaggacatgtggctctcggccgcctatctgcagcggcgccacaacagcgccgcgttgcgtgcgctgctcgactttctccagacccgcgtcggcaaggggcccggctcccagaagaaatagaaaagcccggcgcgggccgggctttcttagcttggcgcaggctcgttcagccgacgtgcttggcaaaaaactcgagcgtgcgcgagcgcgcgagcttggcggcctcggcgttgtacgaaccgcgctggtcgcagttgaagccatggcccgattcatagacatgcacctgaacctcgggatgcgccttcttgaaggcctcgatggtgtccagcggaatccagtggtcctggttgccgaaatgcgccagcaccggcaccttgggctggcgcgcggtttcttccggcgtcgtcatgccgccgccgtagtaaggcgccgcggcggcaatgcccggaaccaggctcgcggcgcgccacaccagcaggccgccccagcaatagcccacgatgcccaccttgccggccttggccgcgtaggccacggcggcctcgacgtcctgcagcacgccgggcgcgggcagcgcctcgaccgcggtcttcagggcgaagccggccttcatgtcctcgtcgctgtagccgagctcgacgcccggcttcacgcggtggaaggtcgagggagagacggccaggtagccgtccgccgcatagccgtcggccaccgagcggatgtgcgagttgacgccgaagatttccggcaccaccaccacggcgccccgcggcttgccggcaggttcggccacgtaggccgggaagacgaagccgtccttggcggtgagatcgatgaattgacccatggttgtcatgctccttgatagcgaatgagttgaatcgaatgaaagggttgccgctagcgtttttgctgcagcgcgcgctcgacgaaatcgagccggtcctggccccagaatatctcgccgtcgatgacatagcttggcgcaccgaacacctggatgtcgatcgcttcctgggtgtaagcctcgtaacgctcctgcacggcctggctcagtgactgttccgtgcgcttgggcggtaggccgcattcggcgaccagcgattcgagcaccttgggatcgccgatgttgcgctcctgcacccacacggcggcaaataccgcgctgcacacctgcatggccacgtcggtgccgtcgtgcaggtcgaccgcgatgatcagccgcgcggcgtcgtcgcccgagaccggaaagaatttgggcttgaggttcagtggcagatcgagatggcgcgaaaagcgcgccagttccaccagccggtaggcctggcgctgcggtgcccgcttgccgagcgggagcccgcccgagatcggatagacactgcccaggtccaccggccgcacgcgcaccgtggcgcccgccgcggccgcgatggcggcaaaccgggcatgccccagatatgtccagggactctgcggcgcaaagtaatagtcgatcgtatggctcatgcgctcgccctcgatgatgtaatccaagccaacggttttaactgacacgcagtttttgtgcaggaggtcggatttggaccaggtactcttgatcacgggtggcggccgcggcatcggcgccgcaaccgccttgctggcggcaaagcgcggctacgcggtggccgtcaactacgcgagcaactcgctcgccgcggacgaggtggtgcgcaccatccgcgcgggcggcggcaccgccgtggccgtgcaggccgacgtgggcgacgaggcgcaggtgaccgccatgttccagaaagtcgatgccaggctcggccgcctcacggcactggtcaacagcgccggagtggtcgacgtgcaggcccgtgtcgatgaaatgaccgcgctgcgcctggagcgcatgttccgcaccaacgtgatcggcagcttcatctgcgcgcgcgaagccgtccggcgcatgagcacccgatacggcggcgcgggcggcgccatcgtcaatgtctccagcgccgcggcgcggctgggctcgcccggccagtacgtcgactacgcggccagcaagggcgccatcgacactttcaccatcggcctggccaaggaagtcggcgccgagggcatccgcgtgaacgccgtgcgccccggcctgatcgacaccgagatccacgcctccggcggcatgcccgaccgcgccttcgagctggcgcccaccgtgccgatgcagcgcaccggcagcgcggaagaaattgccggcgccatcctgtggctgctgtccgaagaggccagctacaccaccatggccctgctcgacgtgaccggggggaggtaagtgagtacctcgatggatctgatcaagccgctggtcacgctggtggccatcgtcaacccgctggccatcgtgcctttcttcatccactacacgcagggctattcggatgcacagcgccggcacacggtgcgcatgtcggccttcagcgcgttcgtggtgattgcggtcagcgcgctgatcgggctgcagctgctggcgttcttcggcatctcgattgccagcttccaggtgggcggcggcctgctgctgctcatgagttcgctgtccatgctgaatgcgaagccggccgagagcaagaccaacgtggaggagctgcgcgcgaccgaggtgaaagcctccatgggcgcgtccatcgcggtggtgccgctcaccattccgctgctcaccgggccggccacgatatcaaccgtggtgatctacgccgacaagacgcagcacctgtgggagctcgggctgctggtgggctacggcgtggtggtggcactggccaccgcgctggccttttcgctcgcgcagccgattgcgcgcgtgctcggcaagaccggcatcaacatcatgacgcggctcatgggcctgatcctcgcggcgctcgcggtcgaggtcatggcagacggcctgggcaagctgtttccgatattgcagcgcgtgggctagcgcctgttcaggccagcatcttctcgatgatccgccagtgcgtggggtcgaccggcgtgatcgacagccggttgcccttgcgcagcacgacgaggtcggccagctcgggcctggcgcgcagctcgggcagcgccagcagccgggtcttgcgaacggcctgcacgtcgaccagcagccagcgcggatcgtcctccttggaggccgggtcgtagtacggcgattcgggatcgaactgcgtcgggtcgggcttgatgcccgaggccacgcgcgcaatgcccgcgatgcccggctcggggcaactcgagtgatagaacagcacgccgtccccgaccttcatgccatcgcgcatgaagttgcgtgcctggtagttgcgcacgccggtccacgccaccgtggccttgggtgcggcaagcgcgtcgtcgatcgagacctcgtcgggctcggatttcatcaaccagtactggggcatggcaatctcgcgaaggagtttcgcgagggaatatagccgccctccccggtactggcgagctctgcttacggcgtcacgtaatcagaaaccacgacccatttgccatccttgatttgcgacaggcgcgactggtcgttgcccaggcgcttggtggcggtgtaggtgctcttggcgctgccgaacatgtcgggctcgaaggtcatgctgtccatcgccttgatgaagctgtcggtcgtcaggttggggccggccttctgcgccgccttgatgaacgaatcgatgatgatgtagccgtacaccgagaacaccgtcgggtcttcgttgaacttggtcttgtacttgttggcccagaagcgcagcggctgcgactgctcgtcggtgtaggggttctgcaccgtcatggtcgcgtagatgccgtccatcgccttgccgccgagcttgtggatcaggtcggtataagcggcgctggagcccaggaaggtcgggttgaagccggtcttgcgcgcctcgcccacggtgccgatggtctcgcggatgatggtgccgagcaccacgaggtcgcagttggcggccttcatttttgcgacctgcgagctgaagtcggtggcgccgcgcttgaaagatgttttctcggccagctccaggcccgccgtcttcaggccggcctcggcaccgcgctgcacttcgagcccgaactcgtcgtcctggtagatggtgcagaccttcttcgcgcccttctccttgatcatcttgggcagggccaggcggatctggtcatagtaggtggccgcgaacgagtacttgagccggttcagcggctcgtacatttcacgcgccgcggtgatcggcatgaagttgacgatgttcttctcgaactgcaccggcatggccgccatgttctgcgcggtgccgatgtggcccgccatgatgaagatcttttcctggttgaccagcttctgcgccgcgagcacggctttcttggggtcgtagccggagtcttcgacgaagagcttgagcttgcggccgtggatgttgccctgctcgttgagttcgtccacgcgcagctgcatgccgttgcgcgcctgcttgccgaagcccgcgagcgggcccgacaggtcctggatcgtgccgatgcggatctcgtccttgctcacgccttgttgttgctgctgcgcggacgcgaacgttacgatcaggcccagcacggccaaggtcgtcagtgtcttgagcttcatcatggcgttgtctcctcgggttgacaaaaaacggttcggcgatgccggtggtcagcggtacatcgcctcgatgcgctcggcatacttggtctgcaccagcttgcgcttgagcttcatcgtcggtgtgagctcttcgtcctcggcactcaactgcgtttcgagcaggaagaatttcttgatctgctcgacccgcgcaaacttggcattgacgcggtcgatctcgccctggatcaggtccagcacctcttgcgcgcgcgtgaggctttcgtagttgctgaaaggcacatcgtggtcctgcgcaaatttttcgacgttctcctggtcgatcatgacgatcaccgtcaggtacggtttcttgtcgccgatcaccaccgcatcggtgatgtaggggctgaacttgagctcgttctccagttcgctcggcgtgatgttctttccacctgccgtgatgatgatgtccttcatgcggtcggtgatgcggaaataccctcccgcgtcgaccgtccccacgtcgccggtgtgcagccagccgtcggcgtcgatggtctcggcggttttttcgggcaggttgagataccccatgaagacattggggccgcgcaccaggatctcgccggtttgcggatcgagccgaacctcgttgtagctggtggccgggcctatggagcccggcatgatgcgcgacggcggcacgccggtggaggcgccgcacgattcggtcatgccccacacctcgagcatgggcacgcccagcgccaggtaccagcgcacgaggtcgggcgagatcggcgccgcgccggtcacgagaaagcgcgcacggtggatcccaatgagcttgcgcacgttgtccagcgccagccagcgcgccaggcgaaacttgaaccgcagccccgcacccaccggctggccctggagcacgcgttcggcaatctgccggcccacgccgatgctccagccgtaggcggcctgctgcagccggctcgcctccttcagcgcgatcatcacgccggaatagaacttttcccacacgcgcggcacggcggtgaacaccgtgggcgaaatctcgcgcacgttctcgggcaccgtctcggggttctcgacgaagttgaggatcgagccggtgtacatcgcgaagtattcgccgcccatgcgctcggcgatgtggcacagcggcaaaaaacacatgcgctcgtcgccctcgccttgcgacagcagggagttgtagccgcgcatggtgtacaccagcccgcggtggctgtgcatcgcacccttgggtttgccggtggtgcccgaggtgtagacgaggatggcaaggtcctcgggccggcaggcggcaatgcgctgctccagcgcctgcggatggtcctgcagatgcgcccggccgagcgcgcgcagtgcgtccaggctgatgacgccggggtcgtcgagctcgcgcaggccctccatgtcgaacacgacgaccttgcgcagcagtggcagtcgggcgcgcacttcgagcgccttgtcgagctgctcgtcgtcctcgacgaagagcacggtggtgcgcgagtcctcgcaaagatagtgcacttgcgaggccgcatcggtcgggtagatgccgttcgatacgccgccgcagctgagcactgcgatgtcgcacagcacccactcgatgacggtgttggccagaatcgaggcgcattcgcccggcccgaagccgagcgccagcaggccgcccgcaatctcgcgcacggcctcggcggtttggcgccaggtccaggcgcgccagatgccgaattccttctgccgcatccagaccttgtcggcgcgcagttccacggccttccagaacacggccggaatggtgtcgccgggcacgacgacgccgggggtaggctgcaggtgcgccaggtcccacaggccggcgggcgggcgcaaggcggtggtggtggtgctcatctcgctcatctccaggtcttcttctttttccagcgccgctcgccgcgcacgccatcgtccttgacgccgaggtagaactccttgatgtcttccttctcgcgcaggcgttcgcaggtgtcttccatgacgatgcggccgttctcgagcacgtagccgtggtccgaagcgttgagcgccatgttggcgttctgctccacaagcaggatggtggtgccgcgttcgcggttgatgcgcacgacgatctcgaagatctctttcgtcagcttgggactgaggccgaggctgggctcgtcgagcaggatgagatgcggcgcggccatgatggcgcgcgaaatcgcaagcatctgctgctggccgcccgagagcaaaccggcgtcctgcgtggcacgctcgcgcaggatgggaaagtagctgtagacgctctccatgtcccgcgccacgccgtcgcggtccttgcgggtgtaggcacccatgagcaggttttcccgcaccgagagcaacggaaacacttcgcggccttcgggcacgtggctcaggccctgctgcacgatgtaggccgggtccttggcggtgatgtctcggccctggaattcgatgctgccttttcgggggtcgatgattcccgagatggtcttgaggatggttgtcttgcccgcgccgttggagcccaggaccgtcacgatctcgccctgcctgactttcaggctcacgccgcggatggccttgatggggccgtaggcgctttcgacgttgagcagttggaggacgacgtcggtcatggcgttgtccctcttgctccgggcggggaacggcgttggggcccctgccccgggcgggccgacgtcaccggcccttcgggcttccctgcgctgctcacgacaagcggggtctcgcagaactcgcttcgctcaaacagctgcgagccctgatccgcctgtcgctccgctgctcggcggcgcctcaacggcccgcccggggcaggggccccaacgccgtggatacgctcagggtgtttcccccactccttgagcccggtgtgcggtgcggggtgggcgccccctctgcgccgctgaggagcgcagctttccgcggataagggctcgcccttgtttgagcgaagcgagtttgggcgagaccccgcggaaagcgagcaccggaagggagcccgaagggccggcgtagtgggggcgaacgcgccgtgccgcacaccgggcgcctccaacgaagcagcggacatgacgttcatgccgccaccctcctcaagctgctcacgtcatccacggtcccgagataagcctcgatcacccgcgcatccgcctgcacttcacgcggcgtgccggtggccagcacctcgcccatgttcatcgccagcacgcggtcggacaccttcgacaccagcgacatgtcgtgctcgaccatcagcaccgacacgcccagttcttgctggatgtcctggatccagaacgccatgtcggccgtctcctcgacattgaggcccgacgatggctcgtcgagcagcagcagcttgggctcggtgcacaaggcccgagcaagctccaccaccttgcgaacgccatacggcaagcccgccaccatcgaatcgcggtgatgctgcaggtcgagcagttcgatcacctgctccgccttctcgcgcgccgcgatttcggcgcgccgcgtggcgggcgtgaagaacacctcgctccagaaacccgtctgccggtgcgtgtggcggccgatcagcaggttgtgcaacacggtggcgtgctcgaagagctcgatgttctggaaggtgcgcgcaatgccgagcgcggcaatcgcatgaggcgcctggtgcgtcaaggccagcggaccggccgcttcgccgtgccacgtgatctcgcccatggtcggcgtgtagatgcggctgatgaggttgaacaccgtcgtcttgcccgcgccgttggggccgatcagcgtgaagacctcgccgcgccgcacgtcgaagctcaccttgttgaccgcgagcacgccgccgaagcgcacgctcaggtctttcgccgaaagaagaatgtcgccgctgctgctcatctcagccgatccgacttggtgaatgacttctgccgcttgaacaaacccttgcggtagaacgggaagagctgcagccaggtgcggatcttgagccaacggccataaagccccagcggctcgaacagcacgaaggcgatcagcaccaggccgtacaccagcccttgcaggcccggtgcctgtccgatcacgggcggcagccagtccttgcccatggagatcaactgcggcatcgcgatcaggaagatcgcacccaggaacgcgccgtgcaccgaacccagcccgccgatcaccaccatcagcagcaggtcgatcgactgcaggatgttgaactggtccggcgagatgaagctgagcttgtgcgcatacagcgcgccgcccagccccgcgagcgcggccgaaatcgcgaacgacatcgtcttgtagcgcgccaggtgaatgcccatgctctgcgcggagatttccgaatcgcggatggcgacgaaggctcgccccgtcggcgagcgcagcaggttcaggatgcccagcgtgctgagcaccgccaccaccaggcacagaaagtagaagccgttgcccgaccccagcgaccagccgaagagctggggcgacttcacgtgcagccccgaattgccgcccgtgacgctatcccagcgcgcgaacacttcctcgacgatgaagccgaacgacagcgtcgcgatgccgaggtagatgcccttcacgcgcaaggccggcaaggccaccaccacgcccaccgccgccgagagcgccgcggccgcgatcagcgcgatcggaaacggcacgcccaggttggtcagcacgccctgcgtataggcgcccgcgccaaggaacgccgcatggccgatggagaactgccccgtgaagcccgccagcagcatcaaccccagaccgacgatgccgtagatcagcacgaaggtcagttgcgcgagccagtattcgtcgatcacccatggcgcgacgatgagaaacgcgaccaggagcccataccagaacacatggccgccgtgccgcgcaaggcggatgtcctggtcgtagctggtcttgaagatgaagcgcatatcggactaaaccttcttgcgcagcttttcgccgaacaggccattgggtttgatcatcagcatcaagagcaccacgatgtagggcgcagtgtccttgaagccgtcgggcagataaaaccccgcaaacgattcgacgatgccgatcaccagtccgccgacgatggcgcccggcaggctgccgaagccgcccaccactgcggccggaaaggccttgagcccgatgaagcccatgttcgcgtgcacgaaggtgatgggcgcgagcagcatgcccgcaatggccgcgaccgctgccgccaggccccacaccagcccgttgagccgcttcaccggaatgcccatgtagtaggcggctagctgattctgcgaagaggcctgcatggcgatgccgagcttgctatagcggaacatcgcgaacagcagcccgcagagaatggcggtggcgatgatgatggccagttgctcgaggttgaccaccaacccgcccagcttccagatctggtccttgtagggcacggccagcgtgtgggtgtcggtgccgatgcccggcaccatcgtgatgagcccgcgcgccacgtaggcaatgccgatggtcagcatcacgatcgagaactgcggctgcccgaggatcggacggatcaccaccagctcgagcagcacgccaaaggccgccatggccaccaccgcgaggatggccgcgagccagaacggcaggccgaacagcgacatgccggcaaatgcaccaaaggcgccgagcatcatcaagtcgccctgcgcaaagctcacggtttcggttgccttgtagatcagcacaaaccccagcgcgatcaggccatagatgcagccctgcgcaatgcctgacagaaggagctggagagtctgcatgcggcttctgtctctctgtatgtctagtgcctgaagccgccggccgcgtcgtgcagcgccaggcggcgcgagccggccaggatgtcgctcggcttgagcccgtagacctggcggatcgaatggctgaagtgcgtcgaatcggggtagccggcgtccagcgcgatgtcggtcagcgtggtggtctggcgcacgtagcgcagcaagctgcgcgcgcgcttccaggcccggaaggcacgaaacgccatgccggtttcctgcttgaacaggtgcaggaagcgcgagaaggacaggtgcaccgaggccgcgcagtcttcggccgaggtgggcgcggccgggtcggcgttgatggcgtcgatgaccttgcggatgcgtgcatcgagcgcgcgcggcgccagcgcctcgccgaagaacaggcgatcgaactcgaggccttcgaagccctggcgacccgagagcgcaagcaattgggcgtgggcatcgcgcacgcgctgcacgaacgccggcgcatcgaccggcccgcaatgctggagaaagcccggcagccgcgccggatcgaccgattccgactcgatcagcaggttgaagatgaggggatgcgcgctttccacccggtgcggcacctgcggcggcaccaccagcagctcgcccgtctgccaggcgcccccgccgatgcagaggcggttgggcggcgcaccggccggcgacacgtacacgccgtgcccgcccaccgtgcgttcggccgcggcgccgagcagccctgcgtagaacacccgctgatgcgtgagccacatcaggcgctccccgcgctctgcgccgccgctttcgggcggcgccgtcttcgttcgctgcatggtgtccgtctcctgcatccggccgccgtcggccaggggccggcgttgcgttggctggatcgtagcggcgggggccggcggcgcggcgttcatttgcgcggggactttccctaggccggcgcaagtgcgcggcggagttcggcactgcacagcgcgatggccgtatcggcctcgtcgagcaccctgcccatggtgatgaagccgtggatctggcgctcgaagcagacgcatgcggcgcggttgccggcggcggtcagcgcctcggcgtaggccatgccttcgtcgcgcagcgggtcgaagccggcggtgagcaccagtgcgggcggcaggcccgaaagatcggcgtgcagcagcggcgacgcgcgccagtcgaggtcgtgccgggggtcgtcgatgtagtggtcgtggaagtaggtcatcgtgtcgcgggtcagcaggtagccctggccgttggcctggtgcgacgggtggccgcggcgctggtccgtggcgggatagatcagcagctgaaaggcaatcgggaggtcgcccgcatcgcgggccgcaatggccgccaccgccgcaaggttgccgcccgcgctgtcgccgcccaccgcgaggcggccggcatccaggccgagcgaggcggcctcgcggcgcacccagcgggtggccgccagcacgtcgtccacggcggccggaaagcgatgctcgggccccatgcggtagtcgatcgaggcgaccgcgcagcccgcgccgttggcgagcgagcggcacagcacgtcatgcgtgtcgaggtcgccgatgacccagccaccgccatggaagtaaaccagcaccggcagcgccgcatcggctgtggaacccagcgggcgatacaggcgcaccgggatggtgccgtgcggcccttcggccttcagctcgcggacttgggcaacctgcggggcttcgggttgcgtggtggcgcgccgttcgcgatagaacgcacgtgcctcggccggcgaaagcgtgtgggtcggcgggatgccgcgcgcctcgatgaagtcgagcaaggcgcgcgcctgggggtgcagcatggtgtctccggtgggtcgggctggggtgctcccgatctcatccacacgatgcccgcaggcgccggtcgccgcttgcgaaaactggctgtaaaaccgcctgtgccggggctcgcgcccttcaggcgatgcgcggcttcacgcgcgaggcggcttccttggccagcttgcgggcggtgccggtgtcggccgcatgcaccagggccacgcccatgcggcgcttggcaaagctctcgggcttgccgaagaggcgcacgtcgctgccgggcacctgcagcgcctcggccacgccgtcgaacgcgatgccggtggcatcgacgccgccgtagatcaccgcgctcgcgcccgggctcttgagcgaggtgtccaccggcaggccgaggatggcgcgcgcatgcagctcgaactcgttctgccactgcgtggccatggtcaccatgccggtgtcgtgcggccgcgggctcacttcgctgaaccacacgtcgtcgcccttcacgaacagctcgacgccgaacaggccctggccgccgaggtcggccgtgacggcctcggcgatctgctgcgccttctgcagcgcggccggcgccatgcgatgcggctgccagctctcgacatagtcgccgctcacctgcacgtggccgatgggttcgcagaagtgcgtctgcaccgcgccggccgcgtccctggcgcgcacggtcaggagcgtgatctcgtagtcgaagtcgatgaagccctcgacgatcacgcggccatggctcacccggccgccggccatggcgtagtcccaggccttctgcacgtcggccgggccgtcgatcttgctctggcccttgccggagctgctcatcacgggcttgacgatgcaggggtagccaatgccggcatcgatggccgcctgcagctcggccagcgagtcgcagaacctgtaggggctggtcggcacgcccagcgtttcggccgccaggcggcgaatgccttcgcggtccatcgtgaggcgggcggcgcgggcggtgggaatcacgcgcaccacgccggcgtcttcgagctgctgcagcatcgacgtggcgatggcctcgatctccggcaccacgagcaggggcttctcggcctcgatcagcgccttgagctgctccgggtcgctcatggtgatggtgcgcgcatggtgggccacctgctggccgggcgcgttctcgtagcggtcgaccgcgatggtctcgacgcccaggcgctgcagggcgatgagcacctccttgccgagctcgccggagccgagcagcatcacgcgggtggcggagggggaaagaggggtgccgagggtggtcatggtcgggatcgaaaagagagaagaaaaagcaaccgccgcactgtaagccacccgcgggcggcccgtgtcacgcacggcaacggcggcctggcggggctgcttcacaatcgatctcctgtcgcggtggcggccagcgccccacccgctcccctttcccctgttttttcttcaaggagttttctcatgacgatccagactgtcggcatcatcggcgccggaacgatgggcaatggcattgcacaggcctgcgcggtggccggcgtcaacgtggtgatggtcgacatcgcccaggcagcggtcgacaagggcctggccaccgtttcgggcagcctcgaccggctgatcaagaaagagaagctcacggccgagcagaagagcgcggcgcttgccctgatcaagggctcgacgaattacgacgacctgaagagcgcgcaactcgtgatcgaggccgccaccgagaaccatgcgctcaagctcaagatcctgaagcagatcgacgagctgctggcgcccgaggtgatcattgcctcgaacacgtcgtcgatctcgatcacccagctcgcggccgccacctcgcggccggaccgcttcatcggcatgcacttcttcaacccggtgccgatgatggcgctggtggagctgatccgcggctacctcacgagcgacgccacgcacgacgccgtcaaggcgctggccgagacgctcggcaagtcgccgatcacggtgaagaacgcgccgggcttcgtggtcaaccgcatcctggtgccgatgatcaacgaggccttcttcgtgctggccgaaggcattgccacggccgaagacatcgacgccggcatgaagctgggctgcaaccagcccatcggtcccctggccctggccgacatgattggcctggacgtgtgcctggccgtgatggaggtctacctcgagcagttcggcgattccaagtaccgcccctgcccgctgctgaaggaaatggtcgcggccggccagttgggccgcaagaccggacgcggcgtgtacgcctactgagcgtcatccaacaaaaacaaaaggagacaaaaaccatgaccgccgtgcccaccaacccaccgccggaaggctgcatcgacacccaggtgatcgaccatgtgctgctgatcggcatcaaccgcccggccaagcgcaacggctggacgccgccgatgttcaagcagctggccgaggcctacacccggctcgacgacgacccggacctgcgcgtgggcgtgctgcatgccttcggcgatcacttcacggccgggctcgacctgccggcggtcaccgagtacatgaagcgcggcgaaaaagccattccggccgggctggtggagccgcacgacttcggcctgcccgactaccgccgccgcaccaagccgatggtggtggcggtgaagggcatctgcttcacggtcggcatcgagctgatgctgggcgccgacatcgtggtggcggcggacaactgccgcttttcgcaaatggaagtgcagcgcggcatcatggcgacgggcggcgccacgctgcgcatggccgagcgcgcgggcgtgggcaatgcgatgctgcacctgctcacggccgacgagttcgacagcgccgaggcctatcgcctcaacttcgtgcagaaggtggtgccggccgggcaggagctcgacgcggcactggccattgcgcagcgcatcgcggcgcaagcgccgctggcggtggtggccacccggctcaacgtgatcaaggcagtggaacagggcccgctcgcggcggtgtcggaattcatcgagacgcaaaagcgcctgtcgaacagcgaagacgcagccgaaggcgtgcgttccttcgtcgaacgccggcccgcgcgcttcagcggccgctgatgaattcaccggagccttgcccatggcctttctccaacgcgcggcgctcgctgccgccttcacactgcttgccgtgaacacctccaccaacgcccaaacagccgcatcactgcccgaccccgcggccacgtcggtcgaggccatgggctggatgaagggctttccgcccccgcccgacaagctgatcaccttcgacaaccccgccggcggcgcgtttccgcgcacgcgctggagcttctcgcacgtgcgcgaaaccgtgcccaccgccaacgtgtggcgcggcagcggcgcggccagccccctgccggcggcaccgcgcagcgacctcgaagccgtgaccttcaaaccgctgggcagcaacgagacggtgaccttcgcccagatgatcccgcgcacctacaccgacggcatcctggtgctgcaccgcggccgcgtggtctatgaaaagtacttcggcgcgctcacgcccgagcggccgcacctcgcaatgtcggtcaccaagtccttcgtgggcacgctggcggccatcctcgcggacgagggcaagctcgatccgtcggcaccggtcacccgctacctgcccgaactcaaggacaccgcctacggcgacgccacggtgcgccaggtgatggacatgaccatcggcgtgcactactcggagaactacgccgatccgaaggccgagatctgggattacgcgcgcgccggcggcatgctggtgcaggggccgaactacgccgggcccaggtcgttctacgaatttctcgccacgctgaagaaggaaggcgcgcacgacgccgcctttgcctacaagacggtgaatgccgaagtgctcgcctggattcttcgccgcgtcagcaaccagccgcttgccgacctgctgagcgagaagatctggcgccgcatcggcgccgagcaggacgcctacttcatggtcgaccgcatcggcaccgagtcgggcggcggcgggctcaacaccgtgctgcgcgacattgcgcgcttcggcgaaaccatgcgcaacggcggccgcgcgcccaacgggcagcaggccattcccaaggcggtggtcgaggacatccagcgcggcggtgatcgggcccagtttgccaaggccggctacgcgctgctgccgggctggtcgtaccgcaacatgtggtgggtcacgaacaacccgcacggcgcctacatggcgcgcggcatccacgggcagagcatctacgtcgatccgaaggccgagatggtgatcgtgcgctacgccgcgcacccggtggcggccaatgcggggaacgacccgctcacgctgccggcattccaggccgtggccgaagcgctcatgcgcccttgagtcttgagggctcagcccgcggctcgctcgcgggcaatcaccaggagtccgtccatgatcaggctttcgaccagttcgaagtccccgttcatgacgggcgccatcttccagcccgcgccgcccgtcatgtagcaggcgggctcggcgccgcaatgcgagcgcacgtgctgcaccatgcgctcgacggcgccggcaatggcgtaggtgccgccgctggtgagggcgtcgctggtgttggtggggaattcgcgcacctcgccggtgggcacgtgcagcccggccgtgcccgattcgagcgcgcgcagcatgatgccgtggcccggcaggatcaagccgcccagaaacttgccgccggcgtcgatggcctcgaccgtgacggccgtgccgatcatcaccaccaccatcggccgcgccggcccggcatccagcatccgctggcgcgcaccgatcatcgccacccagcggtcggcgcccagccgcgtgggatggtcgtagccgttgacgatgccggcctcggctgcgctcgacaccacccagcgcggcgcgcagtcgaagcgctcctcgatctgctcctcggcgcggcggcgcaccgcgtcgcccgcgaccacgcagcccagcatggagccgggcgcgggcaggtcggcccaggggccttcggccagccgctcgatgtggtccaggaactcggcaccgtgcgcctgcagcgcagcccccggatgcgcggcatcgtagagagcccatttgaggcgggtgttgccgatgtcgatcgcgaggaagggggatgccatgcgcgggattattgcgactttgtcggcattcatgctggcgcgtcgttgacacacgcggcgcgggcctacgccggcacctcccgttccgccgctacattcgccagttccatccaccacggcacaaggagatcaccatgggattgctcagtttcatcaaggaagccggtgaaaaactgttcggcggatcgtcggcccaggccgccgagccggacgccaacaccaaggccgcggcggccatcaagacctacatcgagacgcagaacctcggactcacgggcctcgaggtgacctacaccgccagcagcggccttgtgaccctggccggccaggcgccctcgcaggaggccagcgaaaaagccgcgctcgccgcgggcaacgtggccaacgtgacgagcgtcgacaacaagctggtcgccccggccgcgccgcccgcccagtaccacgacgtggtcaagggcgacacgctctcggccatctcgaagaaatactacggcgaccccaacaagtacaacgcgatcttcgaggcgaacaagccgatgctgagccacccggacaagatctatccgggccagaagctgcgcattccggcgccttgaccgccccgcccccatgaaaacgcccgccgcgcttcggcgggcgtttttcgtttcagttctgcttccagggcagtccccgcttgcgccagccgccgatcgtgccgcggtgcccctggtcgtcggggttgccctcgaagccttcgagaatgttgtaggcctcaaagccgagttcggtggcgcgcttggcggcggcaatggagcgcacgccgctgcggcacagcagcaccagtttctgcttgccctcgcccgcggcacggatgccgtcgtcgaaagccggattgggcaccatgcccggccactgcttccaggccagcgccacggcgccgggcacgtagccgacccattcgcgctcggcatcgctgcgtatgtcaaccagcacggcctcgccgctcgccatccacagcgccgcctgttcgggcgtcacatcgccggcatagcccttttccccaacgggttcggtcatttctttgcgtcctttcgatagacagggtaactacgtgggacggctcccttgagctttgccccagccccgtccggatgatggaatttttcaccagttcgtgaaaaccctgtttgtcgcatattgcgccgagccaaagatgcggattgggcctgccgaacataactccaggaaggtgggcaggatttcttccggtcagaacttgtttggagagagacaacatgacaaacagcaaatcgccccgccgccgcagccttctcaagggtgcggccgtggccgcaggcgccatgtcggcgccgatggtcagcatggcccagaccacctcgctgcgtttccagagcacctggccggccaaggacatcttccacgagtacgcgcaagacttcgccaagaaggtcaatgacatggcgggcacccgcctgaagatcgaagtcttgccggcgggctcggtggtgcccgccttccagctgctcgatgcggtggccaagggcacgctcgacggcggccatggcgtggtggcctactggtatggcaagaactcggcgctcgcgctctgggggtcgggccccggctacggcatggacgccaacatggtgctggcctggcacaactacggcggcggcaaggcgctgatcgaggaaatctacaagagcctgaacctggacgtggtgtcctacctctacggccccatgcccacgcaaccgctgggctggttcaagaagccggtggcccgcgtggaagacatgaagggcctcaagttccgcaccgtgggcctggcggtcgacgtgttcaccgacatgggcacggccgtgaacccgctgccgggcggagagatcgtgccggcgctggaccgcggcctcatcgatgcggcggagttcaacaacgcttcgagcgatcgcgtgctgggctttcccgacgtggcgaagaactgcatgctgcagagcttccaccagtcgggcgagcagttcgaggtcttgttcaacaagggcaagctcgcggcgctgccggccgatctcaaggccatcatcgattacgcggtgcaagccgccagtgccgacatgagctggaaggccatccagcgcaattcgcaggactacatcgagctcaagaaggccggcatcaagttctacaagacgcccgacgcgatcctgcgcgcgcagcttgcatcgtgggacaagaccgttgccaagaaggcggccgagaacccgatgttcaagaaggtgctcgactcgcagaaggctttcgcagaacgcgccggccagtggcacaacgactacacggtcgatttcaagatggcctacaaccactacttcggtccgcaggccaagaagagctgaaaccgacccgatgacccgagggcaccccagcggtgccctcttttcacggctgcccatgctgcgccggccgcggcgaggagttctcttcgatgcaatctttcctgttggccgtcgatcgcttttcgacctggatcggcaagaccttcgcgtggtgcgcgctgctgctcacgctgctgatcagctgggaggtgttctcgcgctacgtgctgaaccacccgcatgcgtgggtgctcgacgcgcagatcatgctgtacggcgccatgttcatgaccgccggcgcctacacgctgtcgaagaacggccacgtgcgcggcgacgtgctctacgggttcttccgcccgcgcacgcaggcgctggtggacctggtgctctacatcgtcttcttcctgccgggcatcgtggcgctcacctgggctggctggatctacgcgggcgagtcgctcgccatacgcgagcagaccttctcggccgagccgctgccgctgtatccgttcaagttcatcattccgctcgccggcttcacgctgctgctgcagggcgtggtcgagatcatccgctgcgtgcagtgcatccagaccggcgcctggccctcgcgcgagcaggacgtggaagaagtcgacgtcgagaagctcaaggagatggtcaacgtcaaggacgaggacattgccgcgctcgaccgcgtggtggctgccaaggaggccgcgcgatgatccgccgcgaactctggttcggcctctcgttcatggcgctgatcgtgatcggcgctgcggcggtgctcgtgagcgccgacaccatcaccaacggccacctgggcctcttgatgctctcgctggtggtggtggccatcatgctgggctttcccacggcgttcacgctgatgggcatgggcatgctcttcacctggctggcctatgaccgcgactggcaccgcacgctcgacctgatggtgcaggcagcctacaagaccatggccaacgacgtgctcattgcggtgccgctgttcgtcttcatgggctacctggtggagcgcgcgaacctcatcgagtcgctgttcaagagcctgcatctggcgctcgcgcggctgccgggcgcgctggccgtggccacgctggtcacctgcaccatctttgccaccgccacaggcatcgtcggcgcggtggtcacactgatgggcctgctggccttgccggcgatgctgcgcgggggctacagcgtgccgctggccgcgggtgcgatcacggcggggggctgcctgggcatcctgatcccgccttcggtgctgctgatcgtttacggcgcaacggccggcgtttcggtggtgcagctgtatgcgggcgccttttttccggggctgatgctcgcttcgctctacgtggtgtacgtgatcatcgtcgcccgcctgaagccgcaatgggcgccgccgctgtcgcaggccgaacgcgtggtgccgctgtcgccaatgtcgcagcggctggccgaaagccccgccgcgcacgcggtggtcgggctgctgaagggccgtcgcaacgcgggcgtgccgttctcccacgtgctgcggcagttgggcatcgtcgcgatgcccggcgtgatctttctcttgctcgccggctacagctacaaggccgtgaccacggtcgaggcacaggcgcgctacgacatcgaggagatcggcgccacgcgcagcggccccgcggagggcgcgggcggactgcaggagcccccctctacaggcgggctgcaggaaccaccgtcggcaggcggcttgcaggagccgccttcgggggaggcgccttcctccggtccgctggcggaaccgccgggcgcatccaccgcgccggccgaagcagcctccgcggcgcaaccacccgccgcaagcccggccgcggccgcaaccgcgccagaaggcgcctcggtacgtccggcacccagctggtggtgggtcaccttcgccatcttcggcgcgctggtgacgctgttctatctgttcctgagcttcgcacggctcgagatcttcaagatgctgctggcctcgttcttcccgctggtgctgctgatcctttcggtgctcggctcgatcgtgctgggcctggccacccctaccgaggcggccgcgatgggcgcgctcggcggcatgctgctggccgcggcctaccgccggctcaatctgtcggtgctcaaggagtcggtgttcctcaccgccaagacctcggccatggtgtgctggctcttcgtcggttcggccatcttctcggccgcattcgcgctgctcggcgggcaggcgctggtggaggagtgggtgctgggcatgaacctcacgaaggtgcagttcctggtgctgagccaggtcatcatcttcctcctgggctggccgctggagtggaccgagatcatcgtgatcttcatgccgatcttcattccgctgctcgacaacttcggcgtcgatccgctgttcttcggcctgctggttgcgatgaacctgcagacggcgttcctgagcccgccggtggccatggcggcgttctatctgaagggcgtgagcccgccgcacgtgacgctgaaccagatcttcctgggcatgctgcccttcatgggcatccaggtgctggccatcgtgctgctctacatctggccgcaaatcgggctctggctgccgcagctgctctacaagtagccaaccggccagctcagcggcgccgctccacgtaggggcgcgcctgcagcagcacgatgcggtcgcccaccgtcgcccattcgatgtcctggtcgaggccgccgaacgagcgcttcacggccgcaccgacgctcgcaaggcgcagcaccagttcgtccgtcagcacgttgcggccaagctccaccggcacttccttcacgccgccgtccttgtcgagctgcagcgccgtctcctcggccgagcggctcagcacctggatcgccttcgaccagctcgaatacatcacctgctcggccacgcgctggccctcgaccacgcggatgccgatgccgcgcttggccgagatgtaggtgacgtgcggatgcccggcgtcgaaggggtcgcgcgtgatcatcacgccggcgttggtcgaatcgatggcggtctgcacgaacacgcccatcagcaccgactcggcgccgaagcccgcggcgctgcgcgcctcccaggcctcggggttgaagaccgaggcccagaccttcttcaccgcgagctcgagcgcgtcgccggtcttgacgttgggcatcgtcgtgtagagccccgcgccgctgaagccgggcaggtcttcggagttggacgagctgcgcacgaacacgccaccgccgcccagctgcgattgccatgcggcgcgccacgacgccgcggtggcgggatcgaccggccatttgacgatctcgtcgcgcagttgcgccagcgccttctgcctggtctgcgggtcgcccgcaaacccgggctgctgctgcatgcgcgcgatgcggtcggcgaggccattggcgcgcatgaagcggtcgtagtgcgcaaagggaatgcagaaaccgtcgggcaccgtggtggagggaatgcgcgcggccagcacggcgcccagattggcggccttggaaccgcactgcgcgctgttgcgcgcgcgcagcgaggaaagcggcagcagacgggtttcgcgcaggtcgggcctggcggctttcgcgctgccgggcaccgcgccgatggccgcggtgcgcacgttgcgcggcggcagcgcggcaacctcgtcgggcgtgaggcggcgcacctggtagcccgaggccgcgaccttgagcgccacccactggcccgcatgctcgcgcagcacggatgcggcatcgcgcacataggcattgggaatgccccaccccttggccagcaggttgacgtgcgagagcgcggtcgacagccgctcggtcagcacgccggccacgggcggcaggttgatcggcacctggcgcagcacggcgatgtcgtcgggcaacagcgcattcaatgcgttcgcgcccgaggcctcgtccacgatccggacgcggcccgtggccgtgcccagattcatcggcatgtagggctgttcgcggatcagcgcttcctggctgacgaagtcgatgccggcttccttggcgacccgatcgtgcagcgtcgagttggtcttgaacttgacgggcgcgaagaaactggctttcgcctctgcgtccgcctggcgcagcagcgcaggggtgagctggtcgccctcccagaactcgtaggtgaagctgccgatgttctgctgccagctcagcgtgccgaacaggaagcggcgatcgggcacgaggtagttgcggtcgatctcgcgcttgcccgcgctcggcgcaagcccggtgtcccgcacgaagcgaacgtgcaactggtagcgcggcgtgtcgatgtaataggtgcgcaccggcctggcctggcgatcgaccgcgaacagcacgtgggccagctgcatcggcgtgccggcgtcgtagatgcgcgccaggctgtcgaaatcgccccggctgcgcagcgcgggcagcgacgcaggtgccgccacgcgctttgcgggctgcccggccgcgccttcgggagcggccgtgttgttctgctgctgatagtaggaaggcttgcgcgccagctgggcttgcgccggcaggatggcgacggccatggcgcccagcgccagcgtcgcgagccagcgcggcttgctcttgtttcggtagcgtggttggcccgatgcgccttgatatttgtcgtttttcatgcagggtccctcattacaagcggttgccgaatgtgcgtgcgcttcaccaagcagggggcttgcgctgacagcggcagcggattctcgcgcgttacatatgcattgctttcatccggtcccgcgaaccagagacaaaccatgaaacgccccgctctttccatccttcctccccggccgctgcaccggtggctgctcggactggcgctgctgtgcctcggcgcggcggccagcgcacaacaagacccgccgggccgcgtggcccgcctgaacctgcacgagggcgcggtgagcttcgcgccggccggcgaagacagctggtacgacgcgcagcccaatcgacccatcaccaccggcgaccggctctggaccgaccgcaatgcgcgcgccgaagtgcacatcggctcgtcgacgctgcggatggacggccagacgcacgtcgagttctccgagctggacgacgacaccgtgcgcctcaccgcgaaccagggcaacctgcaattgcgcgtgcgcgacgacctctcgggccagcgcgtcgagatcgacaccggcaaccttgccgtggtgatcgacgcacccggcgaataccgcattgcggccgacccggccgccgacaccacgtggatcgcggtggcctctggccgcgtcacgctccatggcgagaacggcgaatcgcaatcgctgggcgcgcggcagcagatcacggtcggtggccgcaacctggccgcggtgggcggtgcgccggcgcagaacggcagcttcgatgcctgggtggcggagcgcaaccgcatcgaggaccagtcgatttccgcgcgctacgtgtcgcgcgaagtcgtcggctaccagcagctcgacatgtatggcgactggcaaagcgaccccacgtacggcgacgtctggtttccgcgcaacgtggacgccgactgggcgccctaccgcgacggccagtgggtgaacatcgcgccctggggcctgacctgggtcgatgccgcgccatggggctttgcgcctttccactatggccgctgggcccgcgtgggcccgcgctgggcttgggtgccggggcgcacgaccacgcggcccgtgtattcgcccgcactggtcggctttgtaggcggcggcgcgaacgccaccctgcagatcggcgacggccgcagcggcgtgggctggttcccgctggcgcccggcgagccatggcggcccgcctatcgcgcgagcccgcgctacgtggaccaggtgaaccgcatggccgcctaccggaaccggcaggccgagctgcgcaacgacttctatgccaaccagcggatgccgggcgctgtgaccgtgctgccggccgaccgcttcggccgcggccccttcggccggcgcgacctggtgcgtgtgccggacgaccgctttgcgcgcgtgccggtggtgccagcgccgggcgtgcccgtgcacggcttcggcagcggcttcggccggcccgcggccgtgctgccgccgccgaccccgccgatgctgcgccaacagcaggaacagcaatacgaacaggcgcggcaggcccggcagatgcagcaggcgcagcagcgcgcattgcagggtcaaccgtcccagcagctgcagcaacggcagcaaatggaatggcagcgcgagcagggcttgcgccagcagcagcaacaggagtggccgcagcgcggcgcccaggagcagcagtggcaaaacaggcgacagccgcaagagcaccagcagatgcaactgcagcaacagcaacaggcacagcggcaacagcaggagatgcagcagcgtgcggcagcccaggcacaggcacaggcacaggcacaggcgcaagcccagcagcagttgcagcagcaacagcgcgcggcgcagcagcaggccctggctcagcaacagatgctgcgccagcagcaagaggcgcagcaacgcgcagcccaggctcagcagcagctccaggcacaacagcaggctcaacgccaggcccaggaagcacaggtgcgcgcgatacagcagcaacgcggttttgcgccgccacctcaagcccaacagccccaggtccagccccaccccccggcccaaccgggccaacgccccggcgacgaccgtcgccggctcgtgacctctcccgaccagcgctgaacggcgggcgcgcggcgctgcatcgcaccgcgcgcaggccccgccagcaccgacgcctccttggcggctacagtcgccgccaaggagcgtcttttccatgcccacattcgacttcgatcttttcgtcatcggcggcggcagcggcggtgttcgcgccgcgcgcatggcggcgcagcaaggcgcgcgcgtgggcttggccgaggcggccgaactcggcggcacctgcgtcaacgtgggctgcattccaaagaagctctacagctacgcagccggctatgccgaatccttcgaggaatccgccggctacggctggaagctgcccgaagcgccgcagttcgactgggcctacctcaagacccagcgcgccaaggaaatcgctcggctcaacggcgtgtatgcctcgctgctgaagaattccggcgtcaccctcgtcacgggctgggcgcagctggccgacggccacacggtcgaaatcgacggcaagcgccacacggcccgccatctgctggtggccaccggcggcacgccctacgtgccggagattccgggacgcgagcacatcgtgacctccgacgcgatgttcgatctcagcccttttccgaaacgcctgctggtggtgggcggcggctacatcgcctgcgagttcgcgtcgatcttcaacggcctgggcgccaaggtgacgcagctgcatcgccgcgcgcatctgctcaccggtttcgacgacgacgtgcggcagttcgtggcgcacgaaatgggcaaggcgggcgtcgacgtgcggctcaacatcgaagccacgtcgatcgcgcgcggcccgcacgggctcgtcgtcacgctggcgcgcgggcagcagatcgacgccgacacggtgctctttgccaccggccgcgtgcccaacacgcagggcctcggcctggaggccgcgggcgtggcgctcgacgagcgcggcgcgatcgcagtcgatgcgcactaccgcagttcggtgccgtcgatctatgcggtgggcgacgtttccacccgcgtgcagctcacgcccgtggcgctggccgaggcgatggtggtggtcgatgccctgttcggccaaggcaagcgcgccctcgactacgaatacattccgaccgcggttttcacgcacccgaacatcggcacctgcggctacaccgagatcgacgcgcgcgccaggttcggcgaggtcacggtgttctcgagcgaattcaagtcgctgcgccacacgctttctggacgcggcgagcgcaccttcatgaagctggtggtgcagaaggccaccgaccgcgtggtcggcctgcacatggtgggcgccgatgcgggcgagatcgtgcagggctttgccgtggcgatgcgcgcgggcgcaaccaaggcgctgttcgacagcaccgtgggcatccacccaactgcggccgaagagttcgtgacgatgcgcgaaccaatgccaggctagaggaagggctcgcccccagtcttcgcgcacttcgtgtcgctacgccaaccccctaccgggggcaacaccagcggcccggcaaagccggttccgcggtgtttcgcgaatgggcccctcaacaagaccgcggcttgctttcgagcagcttcaccagcgtgaacagcacgcggttggcgggcgtgcgcacgccgagcgcctcgccgcgccgcacgacgaagccgttgaggtgatcgatttcgctcggcttgccgcgtgcgaggtcctgtgcggtcgatgagtattgcgagggcatcgtctgcgcaatgccgcgcacggcggcgtcggtgtcgccgggtatggcgacgccttcggctttggcgacggcaaggcattcggccaccacgtcgcggatgacctcggccacgccctggcccttcaccacctcgccatagggcagttgggtgatggccgatagcgcgttgtaggcgcagttcagcaccagcttggcccagagcgagccgcgcacgttgtcagagatttgcgtcggcacgccggccgcggccaggtgttgcgccacctgctcgctgctgcgtgaaggcgcaatcaccagttcgccgcggccatggtgcttcacgtggcccggccccgccatctcggtggccacgtagaccacggcggcggccacgtcgttggacggcagcaccgagcgcacgcgctcgtcgttgtcgaccccgttctgcaaggtgagcaccagtgcatcgggcgagagatgcggcttgatctgcgccgcggccgattcggtgtcggtggacttcacgcagaacagcaccaggtgggcgccctgcaccgcattcgcttccgtgcttgccccgagcttcacctgctcgtcgaaagccttcgtctccagccgcagcccgttggcgcgcacggcctccacatgcgagggccgcccgatcagcaccacctcgtggcccgcgcgcgccagcatggcgccgtagtagcagccgactgcaccggcgcccatgactgcgactttcattgcttcacctttcgcggttgttgatggaatctgtccaggttaacggtttgaagccgggcacaatgcgcgcggcccgccgtctccaaccccactaccccagagtttccgccatgcccgtttccgcccttcgtctgcgcgaaaacctgtctgtcgcgttccagcgcggcaagacaagcgagcagcgcatcgagcaactgggtgcgccggccgtcgaaggcgacgacccaccggcggtttacgactacctgggcgacatgcagctgcgcttcatgttcacggcgtcagacggcaccaatgcggtcgccaaagagtccgacctgcaacgcctgaacctcacacctcaactcgcgatgacgcaggtcaccgtgaactcgcgccgtgcgcgcggagcgcccaagcatgggctgttcggccagggcgtctatcagttcacgggccgtggcgacgcggacaccgacgccagctacctgctggatcgcggcttctggcgcacccagctgcaggcctttcccaagggcgtggtcgcggcgataccgcggcgcggcagcctgttcttcgcggatgccggcgacagcgccgcgaccgaagaactcgcgcgcatggctgcacgcctgcaccatgcggcgggcgagcatcgggtgtccaattttttgtacatcttcggcgcgcgcggctgggaagtccttggcaccctgcccgccgaggcgcctgcgcccacctccgccgcgggaggccgcaccaggccggccagccgccaaccggcccgcgaatccgtcgagccgtacgacgaacaggagctgtcgctgtcgctcgtcgccagcgggcagaagaccgtcatctactgcctcatcgcgaatttcgtgctgtcggccgccgcgcggggaggatcgctcccgccgctggttgcctcggcgctgtacatcgccacggcggcggtgagcctgttcggcatcgtgcgcatctgctccgggctgggccacggcacctcgggcaagatcctgttcatggtgctggcattcgtgccgctggtgaacctgatcgccctggtctacctgagtgccaaaaccaaccggttgctgcgcgccgccggctggcgcgtgggcctgcttggcgccaaggcatcgtgaagaagaaaaccggaggcccacgatgagcggcaacagcatgttcgcaatccctgccagccagcaggccggcctgtggctgagctacgccgtcgtgctgctgctgttgcccgtatgcgcagcgatcgccggcgttgtcgtgggcgtatcgaaccgggaccagtcgcccgaggacggcagcctggtgcggcagttcctgttgttccttgccatcttcgcggccgcgacctggggcatcagccgcttgccgtcggttcagtcgcgcatcaatcccgaggtcaaggtccgggaacagctgagtgcgaaccccgcatacgaagccatccggaaatacgcaccgagcgatgcggccaaggtgcaggcggcgctgggcagcgaggtcggcagaggggtgaagctcgaggacgccttcgtgcgcattcgccccctgttcgcgacgctggttcgcgagcggctgggcttcgtcgaccagtccacggccgtggcatgggcgcacgtgatgcgcgacacgctgcagcagatgaaggcggccgatccgcagaagtgcgtccgcacgctgtaccctgagccaggcgtgccgcatccgttgtcggagcgggtgctgagcgacgccagcgctgcggccttcctgcaggcggtagcggatgtatacgcctccgccgacgctggcatgcgccgtgacacggttcgcaccgatccgcaggtggatcttcaggcgctccagaccgagtaccgcctggtacaggaacagacgaaaggcgagttcggcgacgacgcgggccgcaccaaggaccgccagtggcgcgaagcgaatccggccgcctactgcgacatcgtgctgcgcaagatgcagctgatgctgcagcgcgaaccggccctggcgggctcgctgctgcgccagtatttgcgcggcgactttcacggcgacatcggctgatcggatcgggcaggcattgcacaatgccgacatgccctacatgcccaccttcgtcgcccccgcccgcttcaccgacgccgccgccgctctcgaacaggtcaagtccatctaccaggctggcctcgcgcatctgcgggagtcgatgctgcgtttcgtggccggggaggcgctgccggggcgggtgcgggcctgctaccccttcgtgcgggtgcacacgcacaccgtgtcgcgccacacgccgccggccaacgcggggctgagctacggcttcgtcgccgggccgggccgctacgaaaccacgctcacgcggccggatcttttctcgcgctattacctcgaccagttccgcctgctgctcgaaaaccaccaggtcgacatcgaggtcggcaccagcacgcagccgattcccatccacttctcgtttgccgagaacgaccacatcgaaggcacgatgagcgatgagcggcgcgcgctgatgcgcgacgtgttcgacctgcccgatctgggcgtgatggacgacggcattgccaacggcacctacgaggcgcaggccggcgaggcgcagccgctctcgctcttcacggcggcgcgcgtggactactcgctgcaccgcctgcgccactacaccggcacggcgcccgagtggttccagaatttcgtgctgttcaccaactaccagttctacatcgacgagttcgtgcgcctcgggcatgaggccatggccgacgaaaaaagcgagtacgtcgctttcatcgagcccggcaacgtgatcacgcggcggcgcgggctgcctgcgggcgcaagcaccaactacggcggcctgctcgacggcagccagggcacggcgccaccgcgcctgccccagatgccggcctaccacctggtgcgcgaggactgcagcggcatcagcatggtgaacatcggcgtcggcccggccaacgccaagaccatcaccgaccacatcgccgtgctgcgcccccacgcctggatgatgctgggccactgcgcggggcttcgcaacgcgcagcagctcggcgactacgtgctggcccacgcctatgtgcgcgaagaccacgtgctcgatgaggaactgccgctgtgggtgccgattccggcgctttcggaaattcagctcgcgctggaaaaagcggtggccgacgtcacccgctacgaagggcccgacctgaagaagatcatgcgcacgggcacggtggcgagcaccgacaaccgcaactgggagcttttgcccggcaaccagccgcagcggcgcttcagccagagccgggcggtggcgctcgacatggaaagcgccaccatcgcggccaacggcttccgctttcgggtgccctacggcacgcttttgtgcgtgagcgacaagccgctgcacggcgagatcaagctgcccggcatggccaaccacttctaccgcgaacgcgtggagcagcacctgcgcatcggcatgcgggccatcgacatccttcgcgaacagggctccacgcggctgcacagccgcaagctgcggagcttcgcggaggtcgcttttcagtaatagttggcacttcctagggttttcacctacttccgggtgtaggcgggcgacgcaattcgcgtggatcattcggttaccgttctcaacaactggaaacaaaatgcctcgttcgtcgctcgcgggcctttcgcgccgcaatttcaacgcatggatggcgggcgcggccgccgtcgcgggcgccgggcatgccgctttgtggccccgttcggccggggcggccgagccgcaactcgtctccaagctgcgcatcgtcattccggccaacgaaggcggcggctgggaccagaccggccgtgcgctcggcgcggcgctgctggcctcgggcgcggccggcgaggtgacctacgaaaacatcggcggcaagggcggcaccatcgggctggccaagtacgtcgaaaaatacgatgccgatcccgacacgctgctgatgagcggcatggtcatggtcggcgcggtggcactgcagaagccggccgtcaccatggcgcaggtcgcgcccgtcgcgcgcctcaccagcgactacgaagtggtggcggtgaaagccgactcccttatcaagacaccgaaggacctgatcgcccagctgcgcgccgacgcggccaagaccgtcatcgccggcggctcggcgggtggcgtggaccacatgtacgccggcatgctggcccgcgtggccggcaacgccgcgaacctggtctaccagccgtaccccggcggcgcccaggtggtggaggcactcatgaccggcaaggccgttgcgggaatctcgggcttcagcgaattcagcgaaagcctgtccagcggcaagctgcgcgccatcggcgtgtcgtcgaagcggccgtttctgggcattccgtcggtgcgcgagcagggcgtggatgccgacctcgccaactggcgcggcgtgctcaccggcaagaaggtgcccgcggaccgcaaggccgtgctgctcgaagccgtgcaccgcgccaccaccgccgacgtctggcagaagaccatcaagcgcaacaactgggatgcgtactggatggcgggcaaggatttcgagagcttcctcgagctggacctggccatggccgggccgatgatctacttgctcaaactgaaggcctgaagacgcttttcaggcgaacaactccggcatctcgcgctgcgccttgggcgtgagcgtcagttcgcgcccgtcgagcgcctgccgcacccagccgcggcgcagcgacagctggagccaggccgcaccgagcgcgccgcccaggtgcggacggcgctcgctccagtcgaggcaggcacaggcaaagcgccgccgcgatcggcgcaccgcgtcgatctcgacacccaggctctccagcgcgatggcgccttcggccgtgagctcgtacgacccgctctgcagtccgctgagccagccctgcgcatgcagccgatcgtgcagcgcgacaccggccgtgcccgccatgtggtcgtagcaggtgcgcgcggtgcgcagccggcttggggtgctcggcttgaactcggccgcgcgcggcgcgccggccaccaccatgaggctctcgagcgcggccgcgacgttgtcgccggccaggcggaaatagcgatgtttgccttgcaccagcaactcgaccagccgctcttccttcaggcgcgcgagatgcgcactggcggtggaggcggccacctcggcgacggcggcaagctcggtggcggtgcgcgcgtggccgtccatcaggcaactcagcatgcgggcgcgcgcgggctcggcaatggcgccggccaggcgggccagctggagatcggcgttcgatgaagaggacgtgtccatgcgccgatcctaaggcgcagccgcaatccacacttcgttcgcgggcgaagtgtggcggcggcttcaaccgcacactgcggcccatgaatccaagccccaattctttcgccgatacgcccgtcgccgacccggtcgcggccgtcacgcatgccgacccctaccccttctatgccgggcttcgcgcgggtccgccgctcgtgtggaacgagaggttgcgcgcgtgggtcgcgagccgcgcggacgtcatcgagtcgttgctgctcgcgcacggcgcgctgcgtgtgcggccggccgccgaaccagtgccgcgcgccatcgtcggcagcgcggccggtgaagtgttcggccacctggtgcgcatgaacgatggcgccgcgcaccaggcacaccggcccgcgctgcaacgtgcgctggccgggctggacctggatgccgctcacgcggccgccttgcaggtcgcgcgcagcgtgcccgcacaacccttgtccgatgcgctgttttcgatgccggttcgtacggtggctcatctgctcggcttcgccgacgaggcgctgccgaaggtcgaccactggatgcgcgatttcgtcgcctgcctgtcgccgctctccagcgccgaccagctgcaaggcgccagcgtcgcagcgaacgaactcatggcgcgcttcgaggccttggccgcgggcgcgccgccgcgacacggaagcttgctcgcggcggtgctggccgaaagcgatgatgccggcgcgcctctttcgcgttcgctgctcgccaacctcgtcggcctgctctcgcagacctgcgatgcgacggcgggcctgctgggcaacagcctcatcgccctgatgcgcgagccttcactgcgtggagccgcaagaacacgcgacggattgcaggccgttgccctggaaaccgcgcggcacgacccttcggtccagaacacgcgccgcttcgcggtcgaacccatcaccatcgcaggcacgacgctggcggcgggcgatgcggtgttgctcgtgctggcggctgcgaatcgcgacccggcgttcaaccccgaccccgaccgcttcacgctcgtgcgcgcacggcgccgcatgctgggcttcggccacggcgtgcacgcctgtccggggcaggcgctggcctgcacgctcgcagccgcggggctcgaggctttgctgagtcgcgcgcccgatctcgatgcgatgcgcgaacgcggctggagctaccgcccttcagccaacgcgcgcatccccgtctttcactgaggggcccagcgccccgagcccgccaggtgcggcgacagctcggcatcgccccagcgcagcggcagggcggcgggccggcgcaatgcatggtcgacatgcagccgcagcaggcgctcggccccttcgaactgcgcgagctcgggtccgtccagcacgatctcggccgtggccgccacgtgcagaagctcgccgctgtcgaagtcgatgaacagcaggccagcgcgcggatgggccaccaggttgcccagcgtgttgaagaagcggttgccgttgaagtcgggcacggtcagcacgccgccttcgtcgacgcgaacgaagcccggcaggccgccgcggtgcgacacgtcgacaccgtgcgaccttgcatcggcatcgtcgccgaccgccgcttcgtcgggataggccgtcgcgatgaacagcgtgtccgcgctgccgatgagccgctgggcggccaggtcgagcgtgtcgagtcgctgcaccggcacgctgtgggcgttgcgcgcagccgcgaacacgggctcccgcgcctggatgtagcgcgggcagttgccgaagctctgctgcacctcgaccatgaagcccgcggcatcgagcaactcgaccgtgccgttcatgcggttgcgccgccgggtgtgcggctcgatgcccaagaggcccagcgaagcgccttgcgcgagctggccggccagtggatcgccggccgccggcagcgcatcgatgcgcaggtgcgtggcatcgggcgaatgcacgaaccccgcgggcgccgcgagcacgctggcccagggctgcaggctggcatcgaggctgcccaccacgaggaacggcagctgcgcgaagaattcgcggtgctggtcgggcatgtagtcgcggatcacgcgcgggcccaaggcctccatgcgatcgcgccagccggtctgggcttgcagcgcgcgctcgcccgcatggaacggcgcggagatcatgccgccatcccgacaggcgtgcgcaccatcggcacgaaaccgggcaaggcctccacgcgcgcgagccaggcccgcacatgcggatacggttcgagcgacacgctgccttcgggcgcatgggcaacgtaggcgtagttcgcaatgtcggccagcgtggcggaaggggcggccaggaagggcagctgctccaggtggatctccatcaccgcgagcagcgcgtgcgaacgcgtcactgcttcaccggagtcggcgcggccgaacagcgccatgacgcgcgccgccgcagggccataggccagcgggccggccgccaccgagaaccagcgctgcacgcgcgcggcgcccaccggatcacgcggcatccaggccgccggatcggaggcgtagcgctcgttgaggtagaccaggatcgcgttcgaatcggccaacgtgacctcgccgtcctcgatcaccggcacctggccgaaggggttgcgcgccaggaactcaggcgtacggctggcgcgctgcttgaggtcgagctcgattctctcgaagggcaggccgagcatcgagagaaacaaccgcacccggtgcacgtggcccgagatggcgctgccgtagagcttgatgggttgtgcgggaaggcgggcgacggcgttcatggagaggtcctttttggaatggtggatggcgtgccccgattcttctctcttgcggcaaatgaatgaatagccattcctggatttgactgctgcgttttccggtttaattgcgccatggaccgcttcaaagccatgcagaccttcgtgcagattgccgagcagggcagcctgacccgtgccgccgaatcgatgggcagttcgctgcccgcggtggtgcgctctcttgccgcgctcgaggcgcacctgggtgtgcgcctgttccaccgcaccacgcgccgcctctcgctgaccgaggaaggccgccactatctgcccagcgcgcgcgaggtgctgctcgcggccgacgccgcggacctcgcgctcaaggccgaggctcacgagcccgcgggcctgctcaccatcaccgcgccggtgctgttcggccacatgtacgtggcgccggccatcacgcgcttcatgaagcgctacgacaaggtgcgctgcagcgtgctgctgtacgaccgcacggtgaacctgctggaggaaaacatcgacatcggcatccgcatcagcccgctgcaggattcatcgctcgttgcccagacgctcggcaccatccggcgcgtggtggcggcgagccccgacttcctcgcgctccaaggcacgccgcggcacccgcgcgacctggccggcgccccctgcgtgcgcggccgcatcgacgcgccgccgcagtggcagtttcacgagcgcggcaagaccgtgagcgtgacgcccagcaaccggctcgagttcaaccacctcgcacccgccgtggaggcttgcgctgcgggcatgggcttcggcaccttcttctcctaccaggtgcttccgtacgtggcgcaaggccggttgaagctggtgctcgaagactacgaaccgccgccgcggccggtgagcgtgatctacccgaacgcgcggctgctgccggcgcgcacgcgggctttcatcgactggatgaagagcgagttcagcggcctacggatgtagggcgccaatggccgggggccgctccgaacgcgcaggggttgtccatcggttgaagcgatggcggcaagtgtcgcgagcctgggccagaatggccgcgtgccatcctcctcttccacccccctcttccacgccagccatctcctcaagcgctatggcggcaccaccgtcgtcgacgacctgtcgttcgagatcgcgcctggcgaatgccttggcgtgatcggcccgaacggcgcgggcaagaccaccacgatccgcatgtgcctgggcctgaccacgcccgacggcggcgagatctcggcgctgggcttgcaaatgccgcgcgatgcgctggccatcaaggcgcaacttggcgtggtctcgcagttcgacacgctcgaccccgacttcagctgcgccgagaacctcgtggtgtacggccgctactttggcttcaccaaggcgcaggcgagcgagcgcgtgccgcagctgctggagtttgccgccctctcgcacaaggcgaacgcgaagccaggcgaactgtcgggcggcatgcggcggcgcctgtcgctggcgcgcgcgctggtgaacgaccccaagctgctgctgctcgacgagccgaccaccgggctcgacccgcaggcgcggcacctgatgtgggagcggctgcaggtgttgctgcagcaaggcaagtcgattctcctgaccacgcacttcatggacgaggccgagcgcctgtgctcgcgcctgctggtgctcgaccacggccgaaagattgccgaaggacggccgcgcgacctgatcgccgaacacctggagcccgacgtggtcgaggtgtatggcaacggcgcgctctcgctggccgagtcgcccgaactcaaggccatggcggcacgcgtggaagtgagcggggaaaccgtgttcttctacacgcaggatgcgcgccgcctgctcgatgcgctggcgcggcacggccggctgcgcaccttccatcggcccgcgaacctcgaagacctttttctcaagctcacgggccggcagatccgccaggagggctagtcaatgaacaacaccacgacgacgacaacaacgacaacaactgcaaccggcgccacgccgccatcgccttcggtgtggcgcgcgcccgaactctcgctgcgctggtggccggttttcctgcgcaacctgctcgtgtggaaaaagctcgcgatcccgagcctgatcggcaacatcgccgagccactgatctggctcgtggccttcggctacggcatgggtgcgcttgtcggcgaggtgtcagtgaacggaacgcgggtgccctacatcctctttctggcgagcggttcgatctgcatgagcgcgatgaatgccgcgagcttcgaggcgctgtactcggccttctcgcgcatgcacgtgcagaagacctgggacggcatcatgaacgcgccggtcgggctcgacgacatcgtgctggcggagatgctgtgggccgccttcaagtcgatcttcaccgtcaccgcgatcctgttcgtgatgctcgggctgggcatcagccacagcccgaagctggtggtcgcgtggatggtgctgatcggcgccggcatcaccttctcgtccattgcgctgatcttcaatgcgctggcgaaggggtatgacttcttcacctattacttcacgctgttcatgacgccgatgatgtttctgagtggcgtgttctttcctctggagcaattgccttctgctgttcgggctgtggcggcttggttgccgttgactactgcggtggcgctggtgaggccgttgttcatggatcagtggccgacggactggtggctgcacgggggagtgttggcggtttatgcggttgtggctttttggattgctttggctttgactcggaagaggttccggggatagctgtttttacgggttctttttctttcccgaggccgggtctcgccccggcctcgggaagcaaacacccaaagtacccaaaaatattacattgcacacaattgaattgcacactacaattcatcccatgcctacccaacatacctcggacgaaatgctcaagctggacaaccagctctgcttcgccgtctattccgcctcgttggccatgacccgcctctacaagccggtcctggaaaagctgcagctcacctacccccaatacctcgtgatgctcgccctctgggagcaagacggccccacggtttccgcgctgggcgaacgtctctcgctcgactccggcacgctcacgccgctgctcaagcggctcgaagccaacggctacgtggcccgggtgcgcgacacggccgacgagcgccgcgtgcacatcacgctcaccgccgccggccgcaagctcaaggcccgtgctgccaacgtgcccgaatgcctgatggccgccgcccaatgctcggtgcccgaactgatttcgctcacccagcagatccagtcgctgcgcgaccgcatcaagaaggcggcctgacgacgggacaacccggttttctccccgcttcgatcgaaaaagagagaagcttttttcaccctccccctcctccatcatcatcaaaggaatcaccatgaccaccaagctcgacaaggttctctacaccgctgaagcccataccgtcggcggccgtgacggcgcaggcaagtccagcgacggcgccatcgacgtcaagctgagctcgcccggttcgggcaagcccggcaccaaccccgagcagctgttcgcggtcggctatgccgcctgcttcatcggtgcgatgaaggccgtcggcccgaagatcggtgtcaaggtgcctgaagacgtggccatcgactcgaaggtttccctcggcccgacgaacggcggcgctgcctatggcatttccgtccagctcgcgatcacgctgcccggcctcgatgccgaccagaagcagaagctggtcgacaccgcccaccaggtgtgcccgtactcgaacgccacgcgcggcaacatcgacgtcgaactgacgatcgcctgagttcgcgctaagcaaagcgcagcgcagctcaacgcagcaaaaagcgtcccggccacaagccggggcgcttttttcatgcgcgccgtcgtgtctcacgggtgacgccgaaacgccctgtgcgatagcgcgtttcatcaagcttggctaatgtggctgcacgcaacgaaactcacaccaccgtggagatcgagacaccatgagcaccaccagcctcctgatccgcaaggaccagctccccgccacgcgcctgcacaccgccaccgacgagcctttggccgacggccaggtgcgtgttcgcatcgacagctttgcgctcacctccaacaacatcacctatgcggcctttggcgatgccatgagctactggcagttcttcccgtccggcgaagagggctggggaagcattccggtgtggggcttcggcagcgtggtgcagtcgctgcacccgggcgtggcggtgggcgaacggctctacggctactggccgatgtcgtcgagcgcggtgctgagccccgaccgtctcacgtccgcgcgcttcaccgatgctgctgcgcaccgcgcggcgctgcccgcggtctacaaccagtatttccgctgcaatgccgatccgctctacaccgcggacaccgaagacctgcaggcgctgctgcgcccgctgttcatcacctcgtggctgatcgacgacttcatggccgacaacgatttcttcggcggcaacaccatgctgctgtcgagcgcgtcgagcaagacggcctacggcacggccttccagctgcaccagcgcaaaggcatcgaggtgatcggcctgacctcgcccgccaacgtggccttctgcgaaagcctgggctgctacgaccgggtggtgacgtacgacgcgctcgacaccatcgcggccgagacgcccgccgtgtacgtggacttcgccggcaacggcggcctgcgcaatgccatccacgcgcgcttcgcgaacctcaagtacagctgctcgatcggcggcacgcatgtcgaacagctcgccgcccagggcgcgggcaaggacctgcccggcccgcgcgccacgctgttctttgcgccggcgcagatcaagaagcgcaccgccgaatggggcgccgacgaattcggccgccgcatggtggccgcctggcacgacttccttgccaccgtgaccaatgcgaagaccccctggctgcgcgccgagcaccaccacggcggcgaggcggtgcaggccgcttacgcgcaggtgctggccggcaagggcgacccgcgcatcgggcatatcctttcgctttacaaacaacccggcgggttgtgacgccggggagggcccgtgtagcgacaattgctgcatgaccctttcccccgcgacgcccgccaacacacatccttacgagagcctcacgcccgacgtggtgctcgacgcgctcgcgacgctcggcctgcacggcgatggccggctcaccggcctgaactcctatgaaaaccgggtctaccaggtgttcctggaggacccggatccgcatccagccgtggtggtcaagttctaccggcccgagcgctggagcgaggccgagatcctggaagagcacggcttctcgcttgaattggcggcggccgaagtgcccgccgtggcgccactggccttcgacggcaccaccctgcaccaccacggcggcttcgccttcagcgtgagcccgtatcgcggcggccgcgcgccggagctcgacgatttcgaagtgctcgaatgggtcggccggtttctcgcgcgcatccacaccgtgggcagcgccaggcctttcgaggcccggcccgcgctcgacctgcagaccttcggcatggcctcgcgcgactggctgctcggccacgacaaggtgccgctcgacgtgcagcgcgattgggaaaaggcctgcaacgaggcgctggacatgattgccgccaccgcgctggcggtgaacgcccccgcctccgacttccagccgcgcaagctgcggctgcatggcgacgtgcaccccggcaacatcctgtggacgcccaccgaccgcccgggtggcggcccgcacttcgtcgacctcgacgacgcgcgcacgggcttcgcggtgcaggatctgtggatgctgctttcgggcgagcgcgcgcagcgcaccgcgcagctctcggggttgctcgacggctacgagcagttccgcgaattcgaccgccgcgaactcgcgttgatcgagccgctgcgcaccttgcggctcatccactacagcgcctggctcgcccggcgctgggaagacccgatctttccgatcaactttccgtggttcggctccagcgactactggaagggccagatcctcgtgctgcaggagcagtgcgagcagatggccgaagagccgctctacgcctgagcgagcgcccggcgggcgactgcgctatgccgcccggctggtcttcaggccctgccccgccgcccaggcggccacgtcttcgcgcttgatggccgcggccatcaggcccgggaacgcatccggcgtgcaggcgaacgacggcacgccgagcgcggccagcttggcggccaggtcgcggtcgtaggcgggcgcgccctcgtcgctgagcgccagcagcgcgatgaactgcacgccggcctccaccagttcgttggcgcgccgcagcaggttgccttcgaccccgccctcgtacagatcggagatcaggatcaggatggtgttgcgcggctcgcgcaccaggctctggcagtagcccaccgcaccgttgatgtcggtgccaccgcccagctgcacgccgaacagcaggtcgaccgggtcttgcagctgctcggtcatgtcgaccacggcggtgtcgaacaccacgagcttggtcgagaccgccggcaggctcgccatgacggcgccgaagatgctcgaatagaccaccgaggcggccatcgagccgctctggtcgatgcacaggatcacctcgcgctgcggctggcgggccttccggccatagccgaccagcgtctgcggcaccacggtgcggtactcgggctgccagtggcgcaggttggcgcggatggtgcggttccagtcgatctccgaatggcgcggccggcggttgcgctggctgcggttgagcgcgccgctcacggcactgcgcatcggctcttcgagccgcttcatgagttcgtcgaccaccttgcgcaccacggcgcgcgcggtgtccttggtgccggccgggatcacgctcgacaacgccacgaggttggcaaccaggtgcacgtcgggctgcgcgttctcgagcatctcgggctgcagcagcatctggcgcaggttgagccgctccatcgcgtcgcgctgcatcacctgcaccacctggctcggaaaatacttgcggatgtcgccgagccagcgcgccacgctgggcgccgaatcaccgcgtccgccgcgctggccgccctggcccaggccgcggcggccgtcggcttcatagagcgcggcaagcgcctggtcgatctcgcgcacgcggccctcgacggcgccgcagctggcgttggcctcgctgccgagcacgagccgccagcgctgcaggcggccagtgggtggcggtgcctcttcttcgatgtcggcggggtccggattcacgctcatgctttcactcccagcagttcccgcagcagcggcagcgcgagcaccgcgcgtgtttcgtcccagtcggccgcggcggtggccgtcgaagccgtaccgcccgcagcgccgcgcctggcgcgctcgcccagggcgcgccggtcggcgcccgaaaaatccgcgaagctgcggcgcaccagcggcagcacctgcacgaagtgctcttcgccgagccccgagagccagccgtcgaccagcgaccagacggcctcgtcgtgcagcagcaccatcgcgttgcggttgagaaaaccttcgagccacgcagccgcttcggtcggcggtgcgccggaagaaaggttgcgcgcgagctgctgcgaagcgccatcgctgtcgagctgcgcgtcgtcgagcagcagccggcagctcacgccgcgcaagagcgaggccgcgctttcgctgaaggcgatggcgcgcagcgcagcacgccaggcggcggtggtctcttcgccgtcgcgcaggcgcaccgcatcgtgcgcggcaatgagccttgtgcgcagcgcctcggcggcttcggcatcgagcgcgccgcaggcaatcggcaggccgatggcgccgcgcacgatcaggctgtcgagcacgtgcgagagcagcgcgctgtcggtctggcgcacgctgccgtagcggaacacgttggccagcggcggcaccgcgccgatgagctgcaccgcatcgccggtgagcgcggcgcggtcttcgagcgcgcgggtcacggcctgcacggctactggcaggtcggccagcagcacggtgtcgacctgctcggccagtgcggcgagcgaggtttccgcggccagtccttccatcacgcgcgcgctcgcggcgtgggccacggtggcgccgaagcggctggcttcgatgatgcgcagcgcgaactcgggctgccactgcaactgccacacctcgtggaaggtgccgcggctcgcgcgctggccggcggtgatctcgccccagggcaggtcgagcaggcgcaggcggtgcagcaggtggctgcgcgccaggtcgttgggctggcgcaggtcgaggtcgagcgtcttggcggttgcctcgggtttcaggcgcaggcttttctgcgcctgttcgatgtcgcgctgcagcggcacggtcggcacttcggccggcacctggcccatgcggtcgccgacagtgaggcgctcgcggatcagcgtgagcggtgcctgctcgcccatgcagatgacgctgcgcacggcctcgtcgagctcgggcaggccaggcgcggggcgctcgcgcagggcggccagggtgtcggcgaggcgcgtggcctcgatcagatgggcggacgaacaatcgaggtcgtgcgcgcgcagcagcctggcgacacgtgcaagccagcccgtcgtgcggccggccacatcgtgcccctgctgccacaggtgttcgtaccagccgggcgaatcgatgccggcgccgtagccgctggcgctcgtgaggtggcgataggtccacggcacccaggtggcaagcaccttgagcttgggcaggcccttgagcagcgcggcatcggccttggcggtggctgcgccttgcagcgcgggcacatgccaggcgccgcagacgacggcgatgcgctggtggccggctttcacggcctcgcggatcgattgccgcatgaaggcctcacgctgctgttcgcgttccatggcgcgttgcccgcgccggtcttcgggcgtctcggcgcgcacggcggtcatggcctctgcgatggcgccgaacaggtcttcgccgtcgccgcgctcctcgaccatgtggttccaccagctctcgccgtcggcatagccggcggcgtgggcgagccagtcgaaagggtcgtcgggcagtgccgcggcggccactggttcctgctctggcgcttcgaccgtttcggagacgggcaccttgtcggtctcgtcgtcgtcgagcggcgtttcgaccggtgcttcagccttggcctcgtcggcctcgcgcgctgcctggtcgatggccatgcgatgcgcctgcggcaggtcgatgaagcgcgtgggcaggccgtgcttcacgccccattgcagcgcctgccactcgggcgagaactcggcgaacgggtagaaggcagccaggcgcgtgtcgtcgttcgcatgcaccagcatcgcgaccggcggacgcagctcggcatgcgccatgaaggagagcaggccctcggcctcgggcggcccttcgaccaggatgcagtcgggctgcagcgattcgaaggcgcgcagcaggctgcgcgcgcagccaggcccgtggtggcggatgccgaagtagtgcagcggtgaagccggcttgctcgaagtcatatcgatggcctcactgcgcacaaagcgacccggtttttccgtggaacgccgcggaaccggctctgccgggccgctggcgttgcccccggcgagggggttggcgaagcgacacgaagtgcgcgaagactgggggagtcatcaaagctgttcgcggcaggcgcggtacagatccttccagtcggtgcgttccttcaccacggtctccagatactccttccacaccacgtggtcctgcaccgggtccttgatgacggcgccgatcaggcccgaagccacgtcggccgagcgcagcacgccgtcgccgaaatggcccgcgagcgccatgccgctgttgatgacggagatggcctcggcggtggagagcgtggaggtcggcgacttgatgcgcgtcttgccgtcctcggtctggccgttgcgcagctcgcggaagatctgcaccacgcggcgcacttcctgcagcgcgggcggctcggccggcagcgcgagcgcgcggccaagttcggacacgcgcttgaccacgatctgcacttcctccgcttcgctggccggcactggaagcaccaccgtgttgaagcggcgcttgagcgcgctggaaagttcgttcacgcccttgtcgcggttgttggcggtcgcgatcaccgaaaagccgcgcacggcctgcacctcgctgccgagctcgggaatgggcagcgtcttttcggacagcacggtgatcagcgtgtcctgcacgtcggccggaatgcgcgtgagctcttcgacgcgcgcgatcttgcccaggcgcattgcatgcaccagcgggctcggcaccagcgccttttcggaagggccgttggccagcagttcggcgtagttccagccatagcgaagctgctcctcgctggtaccggccgtgccctggatcagcatggtcgagtcgccgctcacggcggcggccaggtgctcagacacccacgacttggcggtgcccggcacgccgtagagcagcagcgcgcggtcggtcgcgagcgtggagaccgcgatctccatgagccggggattgccgatgtacttggggctgacctcgaagccgttggccagcttgccgcccatcaggtaggtgagcacggcccagggcgagagcttccagttggccgggcgctggcggtcgtcgaccttctggagcgcatcgagttcttcggcgaattgctgttcggcatgctggcgcaggacattgctcatggacggccttgggaagatgaagaggggggctgggaacgaagggttgaaaacagctggcgcgcgcgcacgatgcgtgcggtgtcgcccagtgcgttggcaaggccggggctttcctcggccgcgcgcggcaggtcggccagcaggtgcagcgcactcgcatgaagcagcgcggccgcatcgccgagcacctggcgcagcacgtagtcgttgacgagatcgccgcgttcgacgcgggtgcgcagtgcgctcgcaagcttcagcgagagttcggcggaaggggtttcgccgggcgcgcaggcctgctcggcgaaggcgaccacctcctgcacgccgttgcccgattcgccgagctcgcggacccagtgacgctcgcgccgttcgcgcggcaacagtgccagcagctggcccacccacgcgcgctgggcgcgcgcgcggtcgagcatggcgtcgcaccagtcgaaatcgggggtcgccacgatcgcgtcgttccagccgcgcagcagtgcgtccttccagtcgcctttcgcggcccagtcgagcagcgcggcgggcgccatgccggtgcgcgcggtccaccatgcgagcggggcctggcgcacgagctggtagagccaccaggcgcgttcaccgaggctttcgtgggtcggacgcgcggcgtcgatggcatcgtccttccagcgcggatcggcggcttcgggtgctttcagctgccatgctccgccctcctgcgagagcagcggcgcaaagaaggcctcgatgcgctgcacatgggcgctcgcgggcaaccgctgcagcagttcgaccgcggcctgccgcacgtcgcgggcgcgatccttgagctgggcgtcgagcagggcttcgtcatcggggccgatgttctcggccagcgcgcccagcagcgcggcgcgctccttcgccgggagttgtggcagttccgccgcaaggcgttcgcgcgcggcggcgggatcgatgcggcgctgttcggccagcaccgcgcgccgctgttcgaggctgccctcatcccaccgtgtctgtgcgtcggcctgctcactggcaccgacggcatagcgccactcgtcgttgcgtgcggcaagccagagtccgcgctcgccgagcgcaggaatcacggcgggccgcaggtcgacggcgcggcggccggcgtcgagtgcggcgggcagcaggctgtgcggcaggcgcaggccggcggcggccagcgcggcgaggccttcgtgctgcaaacgcagcggtccgctcgcgagtgcgtcgacgatggcggcttgcagcgcggaatcgttcagcacggggcgttcgtcggcggcggcgaccggtgcgtcggaaggcgagaggcccggcgccacgaagccggcacggcggccgatggccacggcgcccgcggcgcgcaggagctggccttgtgcttcgccgtcctgtatcgcttgcagcagcgcggcgaattcgccgcctgccattccttgagctgccggcacgggctgacgggcggtgccgaccagcgcggtctgcagtagcgagttccaatggctcattcgataacctccgcgctcacgcgctgcggtattcgccttggggcggcccggcggctcatgtccgcactccgctcaaggtccagaccggcgcgctgcccgctgcggcgcccgaggcccaggcggtgagcggcgcgaactgctcgccgtcccattcgccgaagacacgcagcggcgcgccgcccgaatgcgccagcaactgccacgcctcctgcgtcgccaattgcattggcagcgcctgcggtgcggcatcgagtcgcagccaccattggtcgccatgccgcgcgggcacggcttcggcccacaccatcggcagcaggggttgccaggggttggcggcaatctgctgcgccatgcgttgccattcgtcggatgcgttcgatgcggactctgccgatgcagcgggtgcatccgccagcagctcggccaccagcgcgcgctgcgacgcatggccggggtagaagcacagcactgcggcgcgctcgctgccgctgacccatccggtttcgaaaccccggccgccatgcgaatagtcgagcagcagggcacgccgcccgctcgcgcggccttgcagccagacatggcgctcgaccagcttggtgtcgcgctcgtcggtgcactggcccagcacgagccagtggtcggcaacgcgctcgccatccgccagcagggcttcgcggtcctgaggccagccgagcgcggtgcgcaggtcggccagcgtggcgggcgagagcgattcgcggcgcggcaccgcatcgacgatcagttgaagccggcccagccggtcgagcagccgcgccggccagccttcaccggcgccgatgagttcggccgcctgcgcgatgcgctggccgagcccgggcgcctgcgcatcgaccatgcgcgcggccatcgagccccaggcctgttgctgctcgctgccgagcgaggcaaggccgcgctgggtctggtcgtcgagccagcgcgcgagctcctgcgtgccggcctcgatgcgcttccagcgctgcgcgtcgcgcttggcggccgcggcgggatcgggcgcggccggcgcttcggcggcgcgggcttccttcttctcggccttgtcgcgccgcgaagcgatccactcggacacccaggccggcggcgtgcccgcggtgaagctggcttcgctctgcgcgcgcagcagcatcagcgcgaggccgtgcttgcaggggaacttgcggctcggacaggagcagcggaacaccgggccggcgaggtcggcctgcgtctgataaggcttgctgccgctgccctggcattcgccccacaccgcatcgtcggaatatccgagcgtgggccatttggctggtgcaagcaggcccttggcggctttcgccgaggcatcgtcgggcgcgagcgccaggacggcttctgtgctgagagtcatcagggcaccctcgcgccggtccgcggcgcggaagattggaaaagcgcggccatcaaggcgcgacgggattgcccggcgtgccgaggctgccggccggaagggccgcggcatcggccggcgtgcggtaagacacgcgcaccgcggaaggctgcggcgccgcctgcggtgcggaagcggtgaccggcctggtcacgccgcccttggtgaccgtgaccggcgcagcgggcggaatggttgccacgggagccacaccggcaatgcctgacgtaccggataccgggaccgtagccccgatcgccgccgtcgtgactggcgcggcgccgcccgccggcgcgtacccggctttccccgcattggggtcgtgcagcaccacgctcttgcccacgccgacgccggtgccgatcggcccgatgccgacgccgacacccacgcccgcggtgccggccaccacgccggcgttgttgactaccacgcccgcgccgagcgggccccagccggtgttgagcccgacggagaaattgccgtccttggtcgcgccaagacccagcgagagccccggcaccagcggtatgccgatgtgatagtgcgaacagccgcccaccaggagcaacagcgccaccgccacggcggcggctgttgcccgactggagcgcggccgggcgttcacaccagcagcgcgttcacgcgcctcacgtaggccgcggggtcggccggcaggccgccttcggccagcagcgcctggtcgaacaggatgttggcaaggtcgtcgaaatgcgccgagccttcgagcttcttcaccagcgcgtgctcggcgttcacttcgagcaccggcttgaggtcaggcgccggctggccggcctgcttgagcatgcgcgcgagctgcgtgctcatgccgccgtcattcaccaccaggcaggcgggcgaatcgaccaggcgcgtggtcacgcgcacgtcctcggccttgtccttgagcgcttccttgagcttctcgagcagcggcttgaaggactcggcggcttcctcggcggccttcttctcggcctcgtcctgcagcttgccgagatcgaccgcgcccttggccacgctttgcagcggcgtgccgtcgaactcggtgaggtagttgagcgcccattcgtcgacgcggtcggtcatgagcagcacctcgatacccttcttcttgaagacctcgagctgcgggctgttcttggcggcggcgagcgtgtcggccgtgatgtagtagatcgcgtcctggccttccttcatgcgcgccttgtagtcggcaaagctcacgctcgccgtgtcgctcgtggtggaggcaaagcgcagcagcttggcgatgcggtcgcggttggcgaagtcttcgcccaggccttccttcagcacggcgccgaactcggcatagaacctggcgtacttgcccgattcgtcggcgtactcggccgccgcctcggcagccggcatggctttcttgtcgaccacgtcggtgacgtcggccgcaatctcggtcggatcgggcgcgggcaccgattccccggagccgacgtcgatcttgccttcggcgctttcgggcgcggtcttctgcttcttcgccaggtcttcgagcatggagagcacgcgcttggtgctgccctcgcggatggccttcacgtcgcggctttcctgcagcaattcgcggctcacgttgagcggcaggtcggacgagtcgatcacgcctttcacgaagcgcaagtagctcggcagcagcgcctcggcgtcgtccatgatgaagacacgcttgacgtagagcttgacgcccgcgctcttctcgcggttccacaggtcgaacggggccttcgaggggatgaagagcagctgcgtgtactcggtgctgccttccacgcggttgtggctccaggcgagcggcgcctcgtagtcgtggctgacggtcttgtagaactcttcgtactgctcgggcgtgatgtctttcttgttgcggctccacagggcgttggccttgttgaccgtttcccattcgccggtcttgaccatgtcgccgggctggtcgttctcgccttctttccactcctctttttccatgaggatgggcagcgagatgtggtcggaatacttgccgacgatctgcttgagcttccaggcgttgaggtattcgtcagcgtcgtcgcgcaggtgcagcgtgatgcttgtgccgcgctcggcgcgcgtgatgtcggccacttcgaagtcgccggcgccgccgctcacccatcgcacgccctgctcgggcggcaggccggcgcggcgcgattcgaccgtgatcttgtcggccacgatgaagcccgagtagaagcccacgccaaactggccgatgagctgcgcgtcggctttctggtcgccgctgagcttgctcatgaagtccttggtaccactttttgcgatggtgccgaggtggtcgatggcttcctggcgcgacaggccgatgcccttgtcggtaatggtgatggtgcgcgcggccttgtcgaaggaaaggcgcacgtccaggttgggctggtcttcgtacagctcgggatggtcgatggcctcgaagcgcagcttgtcgcaggcgtccgatgcgttcgagatcaactcgcgcaggaagatttccttgttggaatacaacgcatgcgtgacgaggtgcagaagctgcgcgacttcagcctggaacggtagtttcgtgttggaggaatcagccatgagaaagaagaaatatcgaactgaaaaattctaagccgggcggccgccggggcgcgttcggcttatcaactctgcgagttggggcttccgccccaaaaaacaatatctgccggaagcgtgctttttttaggcctatctcggttgcgattcgacttcgcgggtccagcggtcgatcagccgcttgcgctcggcggccttgccgtatttctcgaagtcgtacttgatgagcttcacgtcgctcatcgacggaatgcgcgcatcgggcttgaaggtcttgttggccggcgactgcaggctgccgacctgtccgccggtcgcctggccggccggactcatgagccagtcgtagtagcgcttggcattctccttgttgcgcgcgcccttgaccagcgcgataccgcccacctcgtagccggtgccttcgcagggcgcggccgtcttcaccggaaatttgtcgtagcgccagcgctcgaatccgaagatgaagctcacgccgatcgccacctcgcccttggccacgttgggcgcctgcgcctggccgctgcgggtgtagctggtgacgttgcgatgcagcttcttcaggtagtcgaaggccgcgtcttcgcccatctgctgcaccaggcccgcgatgatggtgtaggccgtgccgctcgaggccgggtgcgagatctcgatctcgcctcggtactcgggcttgacgagatcagcccagcacttcggctcgggcagtttctttttcttgagcaggtcggtattgaagccgaagccgatggcgctggtgtagaagccccccaccatgttctgcgacatggcgtactggcgcaccgcccagtcgtgcaggtcgttgatgtaggccggccggtagggctccagcagaccctgctcggcggcctgcaggaacgggtctccggtgccgccccaccagatgtcggtcttggggttggccgcctcggcacgcagctgggcgccgatttctccggtgcccttgtgcgcctgctgcaccttgatgccggtctcgcgcgtgaaggccgcggcggccgcttcgcaccagccggcatcggtgctgcagagcgcgttgaccgtgccctgcgcggccgcgcagggggaaaagaaaaaggccatggcgcccgcgcatgcggcaagggccgcggcattcctggtggcaaaggggcgcatgcgttctcctccggcaaatggttttattggaaaggccaggccgcaggatagccggcaacgccgctcagcgggccgccagcagcggcggcaggtgctcggccagccagtcgaccaccacccgcgtcttgtgcggcaggtagcggctgcgggaacggatgacgttgagttcgaagccgaacggccgcggctcgtcgaacacgcgcaccagcgtgccggcggccagcgcatcggccgcgagccaggccggcaggcgcgccaggcccatgccgccgatggcggcttcgagcagcacctccgcgctgtcgcagcgcagccgcgaaggcggtgccatctcgaccagccggccttcggcgtcgtgaaagcgccagggcgagatctgcccgtcgcgggcatagagcaccgcctcgtgcgccgaagcgccgagctcggccacgtcggcggggcgcccgcgctcggcaagataggcgggagcggcgcacagcaccatccattgcgtgccgaccggccgcgccaccaggtcggcgctgtcgggcagctcgccgcttcgaatggcgaggtcgaggccctcttcggccaagtccacgcgccggtcgttgaaagaaagctccagcgaaagccccgggtgccggcgcgccagcgcgagcagcagcggcccgaccttcaggcgcccgagcatcgccggcatgctgaggcgcaccagcccggccgcggtgctgcgcgcggcgtccgccatggcttcggctgcgtcgagctcggccagcgcgcgccggcagcgctcgtagtagccgtggccttcttcggtgaggctctggctgcgcgtggtgcgcaggaaaagccgagtgcccagccgcgcctcgagccgcgcaatgctcttggccaccgccgagcgcgtgacgtgcagccgctctgccgcacgcgcaaagctgcctgcttccaccgcggcgacgaactcttcgatgctttggagacgttggctcattggatattttcaggcgccatgaagttgaaaattatccaccactggataaatcaagtcgccaatagcatgaaggctcccttgtttcttcgaaggagtcttttttcatgcaggaacctcaaacgcttcgccgctggcaactctcttccttcggccgcgagcagctccagcaggtcgaactgccgctccccacgcccggcccgggccaggtcctggtgcgggtgggcgcggtgtcgctcaactaccgcgacctcctgatggttcgcgacggcatgggcatgaagttcgacatgccgttcacgcccggttccgatatggcgggcaccgtagtggccacggggccgggcgtgcagcgctttgccatcggcgaccgcgtggtcaacaccttctggggcggctggatcgacgggcagtggccggcaggggccgtgctggccggcgggcccggtccgggcatgctggcctcgcacgtgcttctcgatgcggcctgggccgtggcggcgccggccacgctggacttcgccgaagcgagcacgctgccgtgcgccggcctcacggcctggttcgcgctggccgagaccggcgcgaaccaggccgtgaggcccggccagaccgtgctgatccatggcaccggcggcgtggcgctgttcggattgcagctggcacggctgtacggcgcgcgcaccatcgtcgtctcgggcagcgaagacaagcgcgcgcaaacgctcgcgctcggcgcaacccacgtgctgatgcgcgacagcgactggccggccgaagtgcggcggctcaccgaaggccgcggcgcggaccacgtgctcgaactcgcgagcgggccgaatctggatcgttcgctgcaggccacggcgcagggcggccgcgtgtcgatcatcggcatgctgggcggcgagacgctgagtgcgtcgttctatgcgatggtgctcggccgcatcacggtgcagggcattggcgtgggccatcggcgcgcactcgaagagctggtgcgcgccatcgacgtcaatgcgctcaagcccgtgatcgcggcgcgccatgccttcgccgagctgcccgatgcgctcgaccatctcgcgcgcggcgcgttcggcaaggtcgtcgtcacgctttgatgagacctattggtctcttgcacgccccgtgtcagaaacaaaagaccgtcgatttgtgaacaggttccgttagccgcaacaacatgcatggcgcatgcgtgttccgttcctagaatccgcccgcacgatggccgggaggccatgcgcttttctcaacttcaggatggaacagcatggaacatagcacctacaaaaagtggtcggccgagttcataggtactttctggctcacgctgggcggctgcggaagcgccgtcctcgcggcggcctttccgggcaacctgggcatcggcttcctgggcgtttcgctcgcgttcggcctcacggtggtgacgggggcctatgcgctcggccccatctcgggcggccacttcaaccccgccgtgtcgatcggcctcgcggccgcggggcgcttcaaggcctcgcagctcgcgggctacatcgtcgcgcaggtgctgggcgccattgccgcggccggcgtgctctacctgattgccaccggcaagcccggcgccgacatcggcggctttgccaccaacggctatggcgagcactcgcccggcaagtacggcatgaccgccgcgctggtgtgcgaagtggtgatgaccgcggtgttcctgatcgtgatcctcggctcgaccgccaggcgcgcggccggcggcttcgcgggcctggccatcggcctgtgcctcacgctgattcacctggtctccattccggtgaccaacacctcggtcaacccggcgcgcagcacggggccggcgctgttcggcccctcctacgccctgccggaactgtggctcttctgggccgcacccatcgtgggcgcggtcatcggtgcggtgatctatcgcgtgctgctcagcaacgccaacgacgactgacggaagccgcaggcaaccgatcaactgccgctggccgactgcacgagcggcagcgaggtcgattgcccgatcgactcggtgccggtggcgtgcgacgccgcataagcaccggcctgcacatcggacaccgggatagtcgagttcatggccggcgcgctggtcgactggccgatggactcggtgccgctcggccgcgcggcggccatcgcacccgcctgcacttcggggttctcgggtgagttcatctgcaacgggtggtagtccgaaccgtcggtcgtctcggccgatgcatggacggcaccgagcgccgcgaacgcggcaaaagaaccaagggcaataagcttgacggaagtgcgcatggtgtgtgctcctgaatggcgggtggttgtctccggccgcgtgccatcgcgcgaactgcgcgtggcagggcctgaacgcactctaggcagcctgactgagcgggccgtgagcaaacaattaggccggcgtgagcggcatggatgacgaaggcaggtgcacccgcgccatcagtcccgggccgcctccgcctccttcttcttcatcgcggttgcgcagctcgatgcgcaagccatgcctttcggcggccgtgcgcgcaatggccagcccgagtccgctgccgcccgccggcgcgcccggcacgcgaaagaaacggtcgaacacgcgggctatcgacgacgctggaatgcccggcccgttgtcgagcacgtcgaccaccgcatggccttcgaactcgtgcagccgcacgtcgaccacgccgccttcgggcgcatagcgcagcgcgttgtcgatcaggttgtcgaacacgctgcgcagctcggcgggcggcgccatcaccacgggcgcaatgcggccttcgaatccgatgtcgacgcggcgcgcatcggccagcaccatcagctggctcacgctctcgcgcagcagggtttcgatgtcgacgggctcgcacgacgtggggcggcccggcgcatcctgccgcgagaggctcagcaattgttcgatcaggtgctgcgcgcgggtgacgccggcctcgagctggttgaagcgctcggtggcttcgccggcggggacgtgcgcgcgcaggttctcgatctgcaggccgatggcggccatgggggtgcgcagctcgtgcgccgcgtcctgcacgaagcggcgctgcgtggcaaaggcattgcgcacgcgcgacaacaggtggttgaacgcgtggaccagcggcgcgatctcgtcgggcacgcgcgccagcgacagatcggtcgggctgcgctcgtcctgcgaggccacgtcgcgcgccaccgccctgagcgaacgcgacgccgccgacacgatgagccacaggatcaacaacgccaggggcagcagcaacgcgatgggcaggccttcgagcagcgcgcgtcgcagcgttcggcgccggcggtagtcctcgttctgcaagacctgcacgcgcggctggtcggcgtgcgcaccgggttcggccgtgagcacgcgccagcgcgaatgcggatgcacgccggtgtccacatcgccaaagcccggctgcggctgcaagggcaccacggccagcggcggccaggaactcgcgcgcagcgtgcggccgtcggcgctccatagctggaccacgaaggcgccgcgcaccagggcggcctcggcgtcgagcgggcgcggggtccggggcgggtcgccgcccgcataggaatcggccaccagccgcatctgctcgtcgagcgcgttgtggaccaggtcgccataggccacgaaggtgaaccacgccgtgatcgccgccgccgccaggtgcagcgtgacgagccagaacagcagttgcgtgcgcagcgagcgcgggcgccaccagcgaccgccgcccgcagcgctcattggcaaaccttcgtgcttcgcgctgcggcgcgagcccccttcggaacggccgggcgagcgctcatgccgcgacgcgccagcccagtccgcgcacgttgcggatcgaatccgcgccgagcttgcggcgcatgccgtggatcagcacgtcgatggcgttgctggtcacttcttcgccccagccgtagatgcggttctcgagctgctcgcgcgagaggatggcgccgggccgctcgagcaaggcgtgcagcagcgcgaactcgcgcgccgtgagcgcctcgcgcgcgccatcgaccaccacctcgcgcgtggtcaggtcgagctgcaaggtgctccccccgatcagggaatgcgcggcgccgtcgcgccggcgcaccacggcccgcatgcgcgcgagcagctcgcgaaactcgaaaggcttgagcaggtagtcgtcggcgcccaggtcgaggctgtggacgcggtcgtcgagcccgtcgcgcgcggtgagcaccagcaccggcgtggcatcgccgcgttcgcgcgcgcgccgcagcacctcggtgccgtcctgccgcggcaggcccaggtcgagcagcacgcaggtgtagtcgccgtcgccgagcgcgctttgcgccagctcgccgtcgcgcacccagtcagccgaccagcccgcgccttcgagcgcctgcttcaggctgcgcccgatcatctcgtcgtcttccaccagcagtacacgcattgcgtcgactccttgggctgcaaggtagcacgtgatcgggatgatcggtagtggccctgcgccgcggcgcagcgtagaggcgaagtcttaggcggggcttagacgccgtgaaggcacaagggtcacgccacgcggacgtcgtgccgctcgccctcgccaccggcggcgaaggccagcaggcgcatggcctcttcctgcacgccgagccggtcggccttggaccaccgcgcgaagggctccagcaccaccgtggctgcgttcttcgcccgctcgatcttccagatgcccgcgacgaaaccgtcgagcagcaccgtgccgcgcacgatgccattgacggtgaacacccggctgcgatgcacctcgctcatcacgcggctgcggtcggcatgcgagagcagcaggttgtcccattcggcgacgaggcgcggcggcgcgggggtgtcgggaccggggcgcggcgcacgcggcaggtcgaacagctcctggccctgctcgccggtaaacgtgcgcagctgcggccggaggcgctcggccacggccttccagcccgtgaggcccgaccacgcgccggcatcggcgagcgtggcgggaccgaaggccgccaggtagcgcagcagcaggtcgtcctgcgtggcggctgcggcatcggcagcggaatcgccgagccactgtccgatgggctgcagctgtgcgctctggtgcgagttccagctgcccgcgggcggcagatgcaccagcggcaggttgttgcggatgagtgcggcgagcgaggcgggctggcggtctttccagcgcgccgcgagtgcctgcccgagctcggaaccggtgagcgggccttcgcgcagcaacgcccaccccgccttcaccacggctgcacggtcgatgccttcgagagcccgcgcgtgctcgcccgagaggccgcgctgatgcacgggttcgagcagcggccgccaggacagcgcatccgatgcggccatcaggtgcagggtcgcacgcatcgtcgacatgcgcacgacgcggcgcttctccagggcttcagtcagctgcgcgcggcgaaagccttcgagccggctccagagcccgatgtaaggcgggttcggcgcctgcgcctgcaggcccgccagcttttcgatggcctgcgcgaccgtcgccttgcgccgctccagcagcatctgccgcgccagcgtggcccggttcagcgcgcgctggctcagcaccacggccatcggcgaagactcagaacttctcgtgcggaccgaggtagcgccactgccccacgggcaggttgccgagcatcaccttgccgatgcgcacgcgcttcaggcccaccactttcaggccgaccagctcgcacatgcggcggatctggcgcttcttgccctcggtgagcacgaagcgcagctgctcggggttctgccactcgacccgcgccggcttgagcggctgtccgtcgaggctgaggccgtggcgcagcctggcgagcatggccggcggaaagaccgcctgcacattggtggtgacgggatcgtcgtcgtccatgcgcacgagctggccggtgggcgcgggctggccgaggccgtgatacgccacgcgcaccaggtattccttctccatcaccgagtcttcgccgatcagctggcgcgcgatgcggccgtcctgcgtcatcaccagcaggccgatggaatcgatgtcgagccggccgcacggcgccaggccgcgcagttgctgggggttgaagaagaagcgcgtgttgtcttcggcccagcggttctgcggcgtgaagagcgagaccgccggctcatggccgtcttcggcctgcgcgctcacgtagccgatgggcttgttgatgaggatggtgacctggttcgcctgctggcccttggcggccttgtcgacctcgacgcggtcggccggcgtcaccttcacgcccatttcggccggcttgccgttcactttcacccagccgttggcgatccactcatcggcctcgcggcgcgagcagatgccgagctcggccatgcgtttgttgaggcggatcggagcggtggcgtcgtcggtcatgcgggtgcgcggtcggttgggggcaggtcacgcccggtggagcggtgcgcagcggcattttcgtccattgcagctgcctccggaatgtgtcgcattgcatagggataatgcgcgccaatggcccgccgacggcccggacccgcatgacaaaaatcctgatcctcagtgtgagcgccggcaacggccatgtgcgcgcagcgcaagccctcgaagccgccgtgcaatcgaccccgccgcacacggccgtccacatggacgccatggcccacgtggccagcggtttccgcaaggtctacaccgactggtacatccagctcgtgaaccgcgcgccggagctgtggtcgtacctgcaccagcgcgccgacgccacgccgcaccatgcgccttcgcagcgcctgcgccgcggcatcgagcggctgagcaccggcactctgttgcgtgagatccgccgagagaagcccgacgcggtggtctgcacgcatttcctgccggccgagctgctgatgcgcgagcgcaatggcggccgcatcgactacccggtgtggctgcagatcaccgactacgacctgcacaacatgtgggttgtgccgggcatggcaggctacctggccgcgacggacgaagtggccttcaggctgcgcgcgcgcggtattcccccggagcgcatccacgtgacgggcattccggtgatgcccgccttctccgaacccgatgcgccagcgctcgcccacgatgcctgcgccaaggcgctcggcctcgaccccgcgcggcccgtgctgctgatggcctcgggcggcgcaggcgtcggcgacctggcgagcatggtcgaacgcgtgctcctgctcggcagcgacagcggcctgcaggtgattgccgtggccggccgcaacgccgaggcccacgccaagctccaggccctggccgcgcgccacccgggccgcgtggtcgccatcggcttcaccaacgagatgcacaagctcatggccgcggccgacctggtggtcaccaagcccggcgggctcacggtgtcggaatgcgtggcgctgggcaagccgatgctcctgatttcgccgattccggggcaggaagagcacaacgccggtttcctgatggaagaaggcgcggcctggctcgcctacgacgcgatcgggctcgactacaaggtggcgcgcctgatggccgaccccgccaagctggcggacatggcccggcgcagccgtgcgctcggcaagccgcgcgccgcggccgcggtgctgcgccacgtgctgggaaacaaggaatgaaaggaatgaacagccccgccgagaagaccagcgtggcccgcaccatcggctacctggcctgggtcgtggtgatggccttcttctttgccaacgccgagatccagatcgaaggcggcgccggctgggccacctcgctgcccacgtggcgcatcgagaacagcatctggctcgacattttctggggcgggcgcgccatgacgggctaccacgcctgggtgttcaccttcatgctgctggtgttcttctcgccgctggcgttcaacggccgctggacgctgcgcgacctggggctggcggctgcgggcctgatcgtgttctgggtttgcgaagactttttgtggttcatgatcaacccggccttcggatgggcacgcttcaatccggccgacggtttctggcacaagcactggatctggggcgcgccggtggactactggggcggcctcgcggtcgccctgctcatactgttgcggcgccactggccccgctcgacttcatgacaaccactccacgcccctcgcactgggcagacccgctggacgaactgcaggtcgagaacctgcaccgcatcacgccgacgctgtaccgcagcgcgcagccgcgcgtcgcgaacgtggcggcgctcaagtcgctcggcatccgcaccatcgtgagcctgcgctccttcaacgacgacaagaaggtgttctcgggccacgacatccgcctggtgcgcgtgccgatcaacacctggtcgatcgacgacgccaaggtgctgcgcgcactggtcgccattcgcgaagccgaaaagcagggcccggtgctgatccactgcatgcacggtgccgaccgcaccggcgtggtcgcggcggtctaccgcatggcggtgcagggctgggacaaggagagcgcgcggcaggagatgtttcgcggcggctacggctaccacacgctgtggcgcaacatcccgcgctacatcgaccggctcgatccggagaagatgcgccgtgcgctggcccacgcgccggtgattcccgtggtgtcctgaaggcggcagcagctttcgtacgccgctcctatactggccgccccgtggccctgggccatgttcgaacttgcctttttcacaaggccacaaggggctcatccatggcactccaactccgctccctcatccgcgcgaacggcgaactcgagctctcgctgcacgacgaaccgattcccgaaccgcagccgcatgaagtggtgatccgggtcgaggcgtcgcccatgaatccgtcggacctggggctgctgttcggcgcggccgacatgggcaccgccaaggtttccggcacgcccgagcgccccgtcgtgacggccacggtgcccgagcgcggcatgcccgcgatggccggacggctggaccagtcgatgccggtgggcaacgaaggcgccggcgtggtggtcaaggccggttcgtcgccggcggcgcaagcgctgctgggcaagacggtggccgcgatcggcggcgcgatgtattcgcagtaccgcgcggtggcggcggcccagtgcctggaactgcccgcgggcacgccgccggccgaaggcgcatcgtgcttcgtgaatccgctcacgtcgctcggcatggtcgagacaatgcggcgcgaaggccacaaggcgctggtgcacacggccgctgcctccaacctgggccagatgctcaacaagatctgccagaaggacggcatcgccctggtcaacatcgtgcgcaagcccgagcaggaagcgctgctgcgcggcatcggcgcgaagcacgtgtgcagcaccagctcgcccacgtttctcgaagacctgacgcaggccctggtcgagaccggcgcgacgctggccttcgacgccaccggcggcggcaagctcgcgggccagatcctcggctgcatggaagcggcgctgaatcgcaccgccaaggaatacagccgctacggctcgaccacgcacaagcaggtctacatctacggcgggctcgaccgttcgccgacggagttcgtgcgcaacttcggcatggcttggggcatgggcgggtggctgctgtttccgttcctgcagaagctcggggatgaagggacgcagcggttgcgggcgcgggtggtggctgaattgaagaccacgtttgcgagccactacacgcgggaagtttccttgttcgaggcgctgcagctggatgccattggtgtgtatggcaagcaggcgacgggggagaagttcttgttgaatccgaacaggggtgtggggggctgatcttctcttggggattttgtggtggcgtgaatgccgctgccctcaccctaaccctctcccggagggagagggaacaagagggaacaagacggagcggtgaggcatcgggtattgccccctctccctctgggagagggctggggtgagggctctgtgcccacgatgaggcgcgcccttaaaaacctaaaccaccaaccgataccccaccgcagtctccgtcaacagatgcttgggctgcgccggatccgcttccagcttctgccgcagatgccccatgtagatgcgcaagtagtggctctggtccgtgtgcgacggaccccacacctcgcgcagcagttgtcgctgcgtgagcacgcggccggcgttggcgaccaataccgacagcagccggtactcggtcggcgtcaggtgcacctcggcgccggcgcggcgaacgatgcgcgcggcgcggtcgagttcgacctcgccgaaacggaacagcgggtccgcgggttcgtccccaccgccggccgcgcgcgggcggcgcaggttggcgcgcacccgcgccagcagttcgccggtgccgaagggcttggtcaggtagtcgtcggcgccggcatccagcgcggcgatcttgtcggcctcgtcgctgcgcgcggacagcacgatgatgggcacggccgaccagccgcgcacatcgcgaatcagcgaaacaccgtcgccgtcgggcaggccgaggtcgagcaccagcaggtcgggctggcgcgtgccggccgccgccagcccaccctgcagcgtgccggcctcgtgcaccacccagccttcggcctcgagcgcgccgcgcacgaagcggcggatctgcggctcgtcctcgatcacgatggcggtgggggatggcatggtttcagagttgtgcttcggccggttcgggtggctcgcggcgcggcaatgtgaccgtgaattctgcaccgccgccctctgcattggccgccgcaatctcgccgccatgcgcgctcaccacggcgcggcagatggccaggcccagccccacgcccggcgtggccgattcggtctcgccgcgggtgaacttgtcgaacagcttctgctcccggcccagcagcgcggcgggcaggcccgggccgtggtcgcgcaccgtgagcaccagcgtgccgggctcggcccgcgcaccgacgacgatgggcggcgcgccatacttggcggcgttctccagcagattgaccagcacgcgctcgatcagcacggcatcgaattcgacgaggggaagatccgggtcgagcgcggtttgcacgatgctgttgcccaacgacgtgcgcgccgcgcgaatggccgagcccaccacttcctcgaccgattgccagtcgcgccgcagattcaccgcgccgcccgcaatgccgctttcgagccgcgccatgtcgagcaggttgttgaccagcgcgtgcagttcatgcgcctgcgcgacgatggcgcgagccgcctcggcgtgcgcttcgggcggcagggtctgcagcgattcggccagcgcaatcagtgccgtgagcggcgtgcgcacgtcgtgcgaaatggcgccgagcagggcgttgcgcaggcgctccgactccatctcgaccacggcctgctgggctacctccacgtagtgcacgcgctccagcgcgatcgcgatctgccgggccagcgtgtcgagttgctgtgcctgctcgggaatcagcagccagcgcggctgcgccggtgacagcgcaagcacgccgcgcacgcgcatgggcgcctgcagcggcacgtagtgccagggctgagctgcgagcgtggcggtggcaaggccggcgggctggccatggcggaaagcccagtcggccacctgcgcatcgaagccctctggcggattcctgggcagcacgagctggtcggccgcgtcggtgaccagcaccagcgcatggccgccaaagtggccctgcaccgcggcagcgcccagcgcgacgacctgcgtgctctccagcgccgccgagagttcgcgcgtgagttcaaacagcgagcgtgcccgccgctcgcggctggtcgacacgccggccgcaaagcgcagtcccgccatgagctggcccaccagcaggcccacgcccagcatgatcgcgaaggtcagcacgtactgcacgtcgctcaccgcgaacgacaggcgcggcggcacgaagaaatagtcgaacgccgccacgttgaggagagccgcgagcgccgaaggcccgcggccgaagcgcatggccacgccgatcacgcccagcagcaacagcatcacgatgttggacagctccagcacgttggccaggggcgcgcacaccagcgtgagcgccacgctggcggccgtcgcccaggcgtagcccggccaatgaacgggcgccttctcgtgatcgccctcgtcggcacgcatgccgttgatggcggcgcgcgcgaggcgccgcgaactgtcggcatggcccacctccaggatgtcgagcgcgggcgcgcgttgcgccagcgcgcgcggcagcggcatcggcgtggcgggccaccagcggcgccagcccttgaggggctccgagcgtcccagcaccagcgttgcgcaattgagccgccgcgcctcttcggccagctgctccgccacgtcggaacccgtgagcaccgcggtggccgcgcccagttcctccgcgagcttgagcaccgcgaggatgcggtcgcgctcctgcgcggcaagccgttgcagccgcggcgtttcgacataggctgcatgccagcgcacgttgagctggcccgccagccgcgccgcggtgcgcaccgtctgtgcggcgccctcgtgcggtccgacgcatgcgaggatcgcgcccgaggtgttccaggcctgcagcgctccgccgttgccgttgccggccgcgcccgattgctcgacgcgccagccgcgcacgtcgtcttccacgtgctcggcggtgcggcgcagtgcaatctcgcgcagcgcgatcaggttgcccttgcggaagaagttctgggcggcgcgctcggcctgctgtggcagatataccttgccggcggcaagccgcgccgtgagctcgtcgggcgtgacgtcgaccagcaccacctcgtcggcttcgtcgagcacggtgtcgggcacggtctcttgcacccgcacgccggtgatggcccccaccgtgccgttgaggctttcgagatgctgtacgttgagcgcggaccagacctcgatgcccgcggccagcagctcctgcacgtcctgccagcgcttggcatggcgggatccgggcgcgttggtgtgggccagttcgtcgaccagcagcacggcgggcttgcgggccagggcgacgtcgagatcgaactcggccagtttgcggccgcggtagtccacctcacgcatcggcaacgcgtccagccccgcgagcagcgccgcggtttcgctgcggccgtgggtttcggccacgccgaccagcacgtcgcggcccgccgcgtgctcgcgctgtgcagcgctgagcatggcccaggtctttcccacgcccgcgctggccccgaaatagatgcgcagcttgccgcgctgcgcgcgcgccgcatcgctgcgcaattgcgcaagcagggcgtcgggatcggggcgggcgtcggacatggcggtggcagcgcaggttagcgcatcggcccgctcccatcgagcgcgagattcagtgccagcacattgacgcgcggctcgcccagcaagccccagagcggcgcctgcgtgtggctggcgaccagcgcgttcacctgctcgaccggcacgccgcgcacgcgcgccacacgcgccgcctggtagcgcgcggcggcggggctgatgtcgggatcgagcccgctggccgaggccgtgacgagatcgaccggcaccggtgcggtgttgcccgggtcggcggcacgcagggcttcgacccgcgccttgaccgcatccaccagcgccggattgagcgggcccaggttcgagccgcccgaagcgctcgcgttgtagggctgcggcgcagtggccgacggccggccccagaagtgcttcggatcgctgaagttctggccgatgagcgtcgagcccaccgtggtgccgccctgcacgatcaggctacccgcggcctgcgacggaaacagcgccttggcggcaccggtgacggccatcggatagaccaggccggtgagtgcgctcagcaatgcgaagagcacgagcgcgggacgaatgatgttgttcatgatgaagcgcttctcaagcaaggtgtacggcaacgagcagccagtcgatcagcttgatgccgatgaagggaacgagcaggccgcccagcccgtagatggccaggttgcgccgcaacagcgcggccgcgcccacgggccggtagcgcacgcccttgagcgcgagcggaatcagaaagacgatgaccagcgcgttgaagatcacggccgacaggatcgccgacgacgggctcgcgagccgcatcacgttgagcgcgccgagctgcggataggtcgagacgaagatcgccggaatgatcgcgaaatacttcgccacgtcgttcgcgatcgagaaggtggtgagcgagccgcgcgtcatcaagagcgctttgccggtctccaccacctcgagcagcttggtcgggttcgagtccaggtcgaccatgttgccggcctctttcgcggcctgcgtgccgctgcccatggccacggccacgtcggcctgcgcgagggcgggtgcgtcgttggtgccgtcgccggtcatcgcgaccaggcggccttcggactggtacttgcggatcagcgccagcttgtcctcgggcgtggcctcggccaggaagtcgtcgacgcccgcctcggctgcgatggccgcggcggtgagcttgttgtcgccggtgatcatcaccgtcttgatgcccatgcggcgcagctcggcaaagcgctccttgatgtcggtcttgacgatgtccttgagctcgaccacgccgagcacgcgggcaccctcggccacggccagcggcgtgctgccgcggcgcgcggtttcctcggacgcgcgcagcacttcagccggcatggcgccgccgagcgactccacatggcggcgtaccgcatcgaccgcgcccttgcgcagcaggatggcgtcggtatccaggctgctgggtgcggccggcaggtcgacaccgctcatgcgggtctgtgcggtgaagggcacgaaccgggcgccctcgacagatgcggcctccaggccgtcgcggcgcgcgaggtcgacgatgctgcgcccttcgggcgtctcgtcggccagcgatgccagcatcgcggcgcgggcgaggcggcccttgggcacgccaggcgcgggcaggaaggcgctggcctggcggttgccgtgcgtgatggtgccggtcttgtcgagcagcagcacatcgacgtcgccggccgcttccacggcgcggcccgaagtggcgatcacattggcctgcatcatgcggctcatgccggccacgcccacggccgagagcaggccgccgatggtggtcgggatcaggcacaccaggagcgccaccagcgcggtgagcgacaccacggtacccgcgcccgcagcctccacgctgaaaagcgagaacggcagcagcgtgaccgtgaccatcaggaacacaagcgtcagcgccaccaagaggatggtgagcgcgatctcattgggcgtcttgtggcgcttggcggcttcgaccatgccgatcatgcggtcgaggaaagactcgccggggttcaccgagatacgcaccaccagccagtcggacagcacgcgggtgccgccggtcacggccgaaaagtcgccgcccgattcgcgcaccacgggcgccgattcgccggtgatggcgctctcgtcgaccgaggccacgccttcgatcacttcgccgtcgagcgggatgacgtcgccggtctcgaccagcacgacgtcgccttttcgcaagtttggcgcctgctccggaagccagctgtgagcccccacgcttgccactgcgtgtgctgcgctgccccccgagggggccgcttcgccttggggcggcccggcggcgaagcgcgcaccatgatgcggctcctgcagcttcttggcccaggtgtccttgcgcaggccgcgcagcgaggcggcctgcgccttgctgcggccttcggccagcgcctccgcgaagttcgcgaacagcacggtgaaccacagccacacggacacggccagcacgaaggccggcttcatgccggtgtcgcccgggaaggtcagcgaatgcacccagagcagcgtcgtgaggatgctgccgatatagacgatgaacatcaccgggttgcgccactgggtacgcggatcgagcttggcaaaggcgccccagagcgcgggcttgaccagcgcggcgtcgaacagcgaaagggaagtcttggtgtttgtcatggtgcgctccttcacttccagagcacgaggtgttcgacgacgggcccgagggccaatgccggcacgtagttgagcaggccgaccagcagcacggtgccgatcagcagcgagacgaacagcggcccatgcgtgggcaacgtgccgccggtgaccggcaggcgttgcttggccgcgagcgaaccagcaatggccagcaccggcacgatcaccgcgaagcggccaaaccacatggcaagcccgagcaggccgttgtagaacggcgtgttggccgagagccccgcgaaggcgctgccgttgttgttggcggccgagctcagcgcatacaggatctccgagaagccgtgcgcgccggggttcgcgatgccggccttgccggcgccggccatcaccgccaccgcggtgccggccaacaccaggatcggcgtgaccagaatgacgatggagatcagcttcatctcgcgcacctcgatcttcttgcccaggtactcgggcgtgcggccgatcatcagccccgcgatgaacaccgcgagcatcgcgaagatcagcatgccgtacaggccgctccccacgccgccgaagaccacctcgccaagctgcatcagcaccatcggcaccatgccgccgatgggcgtgaaggagtcgtgcatggcattcaccgcgccgcaggatgccgcggtggtaatggcggcaaagagtgccgaggcgtcgatgccgaagcgcacttccttgccttccatgttgccgccgctttgcagcgcgctcgatacctggtcgacgcccaacgcgccgaagagcggattgccggcctgctcggccgggatgatgaccgccaccgcgacgacgaacatcaccgccatggccgcgagcaccgcccagccctggcgcaggtcgccgaccacgcgcccgaaggcgaagcacagggccgccgggatcaggaagatcgcgagcatctgcagcaggttgctgagcgcggtcgggttctcgtacgggtgcgccgagttggcgttgaagaaaccgccgccgttggtgccgatcatcttgatggcttcctgcgaggcgaccgggcccatggcgatcgtttgcgcgctcgccgtcgcctcgaccgtgtgcacggtcttgtagccgtcgaagttctggatcacgccctggcccacgaagagcagcgcgagcacgaacgacagcggcaccaggagccagagcgtgatgcgcgtgaggtcggcccagaagttgccgaccaggccacggctcttgccgtcgccgcggcgcgcgaagccgcgcaccagcacgaaggccaccgcaatgcccgtggcggccgagaagaaattctgtaccgtgaacccgagcatctgcgtgagatagctcatggtcgattcgccgccgtagccctgccagttggtgttggagacgaagctcaccgcgctgtcgaaggccgagtcgggcgacaccgcgcccatggcggcgggattgagcggcagcgaaccttgcatgcgctgcagcgcgtagagaaagatcgcgcccacggcattgaaggccagcagcgcaagcgcataggtcagccagtgcatcgactgccccggctgggtgccggcgagcttgtagagcggcgcctcgatgcgctgcatccagcgcggcatgcgctcgtcgcacagcgcagccaggaacttgccgacaggccaggccagcagcaaaagcacgacgagaaaggaagccagcaaggaccaggcggaggcggtcatgtcagaactcctcggcgcagatcagtgcgaacacgaggtacgcgaacagcaccacggcaatcaatgcgccgaaaccatagagagcttcgaggctgatcatggccgttctcccacggcggctttcggcgcgcctggcgcgttcggcccgttgagccggttcagcccgacggccatggccgccaccaccgcccacagcgccagcaaggcgcccatccagacgaaatccattcatcactcctgcagcgaaacaaggcctcgagtctcggcaggcgcccgtaaaaacagggaacagagtcggctgcggcgcataaagaaaccgtaaaggcgtcccctctttttcaaagtgctcgacaacggctggcgtgtcccttgataatcaaagaaccatctttgaataaaagaaaaaggatgaccacgcgccccttcgatgccaagcccgcctggatgccgcaccagccggcagaccgcatcctgtccacgctcaagacgcgtggcgcgctcggcattcccgacatcgccaaggtgctcgacgtcacggtggaggccgtgcgccagcagatggccaagctgcaggccgagggcctggtcgatgccgagagccgtccggcgggccgcggccggccgacgcagatatggcggctcaccggcgccggacacgcgcgctttcccgacacgcacgccgagatgacggtgcagatgatcagcgcggtgatcagcgtgttcggcgagaagggcatggaccagctcatcggcgcacgcgaggaagccatgcgcgccagctaccgcgaggccctgcaaggcgcgcgcagcctcaaggccaagctagagcggctggccgacatccgcagccgcgaaggctacatggccgagttccggcccgagggcgacggcttcctgttcatcgagaaccattgccccatctgcaccgcggcgcgggcctgcacgggcttttgccgcagcgaactgcagctcttcgacgccgtgctggggcccggcgtaagcgtgagccgcgtcgagcacgtgctcgcgggcgcgcggcgctgtgcctaccaggtgagcccgaagaactcgccttgatccatttccagacccctacctagacgctaaaggaaaaacccaccatggaacacaccctcccacccctgccttacgccctcgacgcgctggcacccgagtactcgaaggagaccctcgagtaccactacggcaagcaccacaacgcctacgtggtgaacctcaacaacctgcaaaagggcaccgaattcgagtcgatgacgctggaagaaatcgtcaagaagtccagcggcggcatctacaacaacgccgcccagatctggaaccacaccttcttctggaactgcatgaagccccagggcggcggcgctcccggcggcgcgctggccaaggccatcgatgccaagtggggcagctacgacgccttcaaggaagcgttcgtgaagtcggccgtgggcaacttcggctcgggctggacctggctggtgaagaaggccgacggttcgctggacatcgtgaacatgggtgccgcgggcacgccgctgaccaccggcgacaccccggtgctgacggtggacgtctgggagcacgcctactacatcgactaccgcaacctgcgccccaagttcgtggagaccttcctggccaagctggtcaactgggacttcgcggcaaagaacttcggttgacggcagccgaagttcctgccggcggcatcctcactcgttgacgaggttcaggatgttgccgtccgggtccttgaaccaggcgaccttcatcttgtccatgacgtggatgtcgcccgtgagcgttgtgttcggcatgtcgtagtgctcgaagcgtacgcccttggccttgagcgccgccacgacccgctccaggtcgtcacccactgcccaggtcacggccgtggcctggttggtgccggcgaatgacgactggtagacattgatacgggtgttaccgctgcggtaggcgatcatgccctcgcaatccgtgtcggccggcgacaggcccagcgtgtcttcgtagaagcggcgggccgcgccaaggtctttcaccgcgaggttggccacggcattgatgtttccgagcatggctgtctcctgtgtggatggactcccatcttctgcgccgcagtggccatgtcaagccgccgctacccgatagggcccccatctcgaacgaagaaaaccacacggctgcgccctgcggcacactgcacccttggtgcagtgcccgacgaggcctgaagcctgacccaccgatttgctcccccgatacagagacaaacccatgatccgcaaactcacccgctcgctggccctggcgctggcgcttcccctggccgtttccctcacgttcagcacggccgcccacgcgcaggcctatcccgccaagcccgtgcgcatgatcgtgccgttcccgcccggcggcggcaccgacatcctggcgcggctggtggcgcagaagctcaccgaggctaaccactggaccgtggtgcccgacaaccgcgcgggcgccggcggcaccatcggcattgccgaagccgcgcgcgccgcgccgacgggctacgacatcgtgatgggccagaaggacaacatggtcgtcgcgccctggctctacaagaacctgagctacaacccggtgaaggacctcacggccgtggcccacgtggcctacacgccggtggtgatcgtcacgcaggccaactcgaagttcaagacgctgaacgacgtggtgaccgccgcgcgcgccgcgcccgacaccgtcacctacggctcgccgggcaacggcaccaccatccacctggccggcgagatcttcaacggcgccgcccagatcaagatgcgccacgtgccctacaagggctccaatgcggccatgatggacgtgctcgcgggcaacgtcgacctgatggtctcgtcggttccctctgcgctggcgcagatcaaggcgggcaagctgcgcccgctggccgtgacctcggccaagcgcagcacctcgctgcccgacacgcccaccgtggccgagctcggctacaagggcttcgacgtgtccacctggtacggcctcttcgtgccggccaagacgccgaaggacgtggtcgccacgctgaataccgaagtcaacaagctgctggccacgcccgaaatgaaggccgccatcgtcgcccagggcgccgagccgcagagcatgacgccggaacagttcgagacgctcttgaagaccgattacgagaagtggaagggcatcgtgcaagcctcgggcgcgaccatcgaataagcgcccggcgtcgcagaatggcgtctccacaacaagccgcatcgacggcatggagacagcgatggcagcacagcgcaagaaatccgggaacgcctttccgctgaagacaaccgccctggcagcggttgccgtcgccctggcgcagggctgcgcgcagacatcgccgcagcagcaacaggcgccgtcggaggcctccgttgcggtgcatgtggcggccgccacccgcgccgcgcgttccgacctgacggcgctgctgaccctctgcaaaccggctcccgccgcgcggccgccccaggccgagctggacaggggccttgccgcattcatcgccaggcccgcaccgccgccgggccaggctttcgacaacctgtacttcgtgggcgccgactgggtcagcgcctgggccatcaagacctcggacggcatcatcctcatcgatgcgctcaacacccaggccgaggccgcggcgctcatcgaaggcggcatgcgcaagctgggcctcgatccggcgcagatcaagtacgtgatcgtcacgcacggccatggcgatcactacggcggtgcgccctacctggcacagaagtatcgcgcgcgcgtggtgatgagcgaggccgactggaccatgaccgaaacccggctcgagttcgccacgccgatctggggggcgccgccgaagcgcgatgtgtcggtgaaagacggcgaccgcatcacgctgggcaatacctccgtctcgatgtacatcacgccgggccacaccatgggcacgatctcgccggttttcgatgtgacttccaacggccagaagcaccgcgccatgctctggggcggcacgggcttcaacttcggcaaggacgtgccgcggctcgacgcctacatcggcgccacgcagcgcatgggcgccgtggtgcaaagccagcgcatcgacgtgctgctgtcgaaccactccaacatcgacggctcgcaggccaagctggccgcgttgcggcagcagcccgcaccggcggcgaacccgttcgtactcggcaccccgaccgtggaacgggcactggcggtgatgggcggatgcgcgcaggcgcagcgcgaccggttcgcgatgcagtgatcccgtcctgctccttccccctctgggggaaggttgggattgggggcggctcccgcgttcgcggctgcgcggaggccgatgccgctgtgcccccacccctgccctcccccggaaggggagggagagatgcaaggggtcagtcgggcgtgaacttcttgttgaagatgtccacgtccgacgccagctcgaaggtcgccacctgccccatctttccgtcgctgaggcggcaggctgcgaacaggctgtagcggcccttgaaatagaactcctccatcacgatcagcgcgtacggatacggcacgaagacctggtgttcgaagatgacgcggtgcacgttcctcggcgaaggaaagagcttgtagtcgctggtgtcgatcgactttgcggtggccatgtctttgtgctcgtactcgttttttttgtgttcaggcggggtcgcgcacgtcggccacggggttgctgccgaaatccgcgcgcgccaggtacctgagcaccttggccgcggcggtggcggggctgtcgagcatgccatcgttcttcaggcgctcgaagcgcgcgcggtccggaaacttctcggccgatgcgccgcgcagctgaacctgcatgtcggtgtcgatcacgccgggtgcgagcgagacgatgcgcgcgccgttcggtgcgccggcttcctcgagcgccacggcgcgagagaagtggtccatgccggccttcgccgcgcaatagggcgcctggctgcccatggcattgcggcccaggcccgacgaaatgttcagcaccttgcgcgcgccgcgccattcgcgcgtggcgccgaggaacgcggccgtcagcagcatcggcgcctccaggccgatgcgcagcgcctgcgacagttcggcgccgacggcactcgccagcggtgcggggttgccgacggtgccggcgttgttgatcagggtcacgctgtcgaagcgctggccgtcgagcgtcttgagccaggccgaaacacgggccgacgcggcgacgggatcggacaggtcctgctcccactggacgagttcggcgccggcccgttgcgccagctcggcgagctgcgggtcttgccggcgcgaaatgccgagcaccatgtggcccgcttgcagcagctgttcggccatggcatggcccaggccgcgcgaggcgccggtgatcagggtgaggtgggaagcggtcatcgagagagtctttctgaaacggagccggggagcgtaaaggggttcgaatacttgcgaggcgcgttcaaccggtgcggaactgcttgcgcaggaaagcccggtggcgcgcaatgtgctgcagctgcgccggggcaatggtgccgccaaggtcgacctcgtccgcgccgttgagcaccgcgttggcatgggtcatggcacgcgcgaccacttcttcctcgctcacgccgagctgcgccgcaagatcgagcgccacgcgccgcatcgcgcgctgcgagagcatccacatcgcgccgaagcggtcccaggccagggcggcctcgtcggccttctcgcgctcggcaagaatctcgacgagcggcttggccagcacggcgtcgagcgcgtcgatcttctcgctaagggcttcgttgcgtgcgatggcttcctcgagcgtaggcccggcctcgccggccttggccttcggtgcctcgggcggcggaatgaaggccgcttccgcattcgcggaaacgacctggagctggtcggacagggtcatgagttttccgtttcccgtgaagggtgcttcttgttcgagatcgcggtggcgcgcaggcccggcaggtcgagcacgcgcagcccaccgtactccacgcggatcaacccttgcgccgacaggccgttgagcgcctcgttcacgcgctggcgcgagaggccgaccaggtacgccagctcctgttgcgtgatgcgcagcacctcgcccacgccggggtacagcaccgggttgaacagcgacaccaggttgcgcgccacgcgcgcgtcggggttgttgagccggtcgatctccagcgccgcaatgaactggccgagccgctcgttgagctggttcatcacgaagcggttgaagccgatggaatggtccagcagccaatgaaagccatcgatcggcaggcccgccaccacgctgcgccgcagcgcctgaatgttgtagcggtagggctcgcgcttcatcaccgtgccttcgccgaaccagccgccgggcggtatgccggcataggtgacggagccgccgtcggcgttgtcgttgctcatcttgagcaggccctcgaccacgccgaaccaataggtcggcgagcggccgacgcggcacaccaggtcgccaacctcggcctcgcccaccaccagcgcggcctcggcgcggcggcgctcggccggcgtgagcgcgggcagccacggaatgccgtcgagctcggcggcattgggagaacgcgcgcggtccttgatcgaagcgccgtgcacgctgtggtgtgaatcgccgtgaagcatcgggaaactccggggagtagtgtccctaggattgtcgttggaacgacaacccaacgtcaaagtgaggcctacgatccggccactgtgcaaaccaccgcccccaccttcccccgtctgttgctcgctcacgcccaggcccagcccgaggcgcccgccatccgcgagaaggacctcggcatctggcaaacctggacctggagcgccgtggcgcaggaggtgcgcgagatcgcgtgcggccttgcgagcatgggcttcaaggccttcgacaacctggccatcgtgggcgccaaccggccgcacctgtacatggcggtagtcgcggcgcagagcctgcgcggcgtgccggtaccgctctaccaggacgcggtggccggcgagatggtcttcatgctgcaggacgcgagcatcgagttcgtgatcgtcgaagaccaggagcaggtcgacaagctgctcgagtgccgcgagctccagacgggcaagcagcccagcatccgccacatcatctacgacgaccccaagggcctgcgccactacgaccagcccgggctcatgagctacgagcagctgcgcgagctgggccgcgaattcgacaagacccacgtgggcacctacgaccgcgcggtggcgagtggcgaagccaccgacgtcggcgtgatcctctacacctcgggcaccacgggccgtcccaagggcgtgtgccagacgcatgcgagcttcatcgcggcgggccgcggcggcgtggagaccgacaagctcggccccggcgacaacatcatgagctacctgccgatggcgtgggtgggcgaccatctgttctcggtggcgcaatggctggtgggcggcttcacgctcaactgccccgagtcgtccgagacggtgatgaacgacatgcgcgagatcggcccgagctattacttcggcccgccgcgcaccttcgaaggcctgctcactgcggtgtcgatccgcatggaagacgcggccgcgccgaagcgctggctgtatgccaagttcatggcgctcgcccagcgcgtgggcgccgacatcctcaacggcgccccggtgagcacgggcgaccggctgatgtatggcctgggcaacctgctcatctacgggccgctgcgcaacgtgctgggcatgagccgcatccgcgtggcctacacggcgggcgcggccatcgggcccgacctgttccgcttctatcgctccatcggcgtgaacctgaagcagttctacggccagaccgagacctgcgcctacgtgtgcctgcagcaagacggcaaggtcaagctgcagaccgtcggcaccgcggcgccgggcatcgaactcaagattgcggacgacggcgaggtgctggtgcgcggcgtgtcggtgctcaaggaatactacaagcgccccgacgccacggccgaggtgctcgatgccgacggctactttcataccggcgatgcgggcgtgctcgacagcgaaggccacctgcgcatcatcgaccgcgccaaggacgtgggccggctcgtgagcggcgcgatctttgcgcccaactacatcgagaacaagctcaagttctttccgcagatcaaggaagccgtgtgcttcggcaatgcgcgcgacgaagtctgcgcggccatcaacatcgacttcgaggcggtgggcaactgggccgagcggcgcggtctggcctatggcggctatgtcgacctggccggcaagcccgaagtgctggcgctgatcggcgaatgcattgccaaggtgaacgccgaccttgcgagcgaagacggcatgggcgacacgcagatcgcgcgcttcctggtgctgcacaaggagctcgaccccgacgacgacgaactcacccgcacgcgcaaggtgcggcgcggcttcatcgccgagaaatacgcggtgctggtcagtgcgctctacggcggcaagaccgagcagtacatcgagacccaggtcaagttcgaggatggacgcaccggcgtggtgaatgccacgctgaagatcgtcgaggccaggaccttccccatcgtgaaggcggcggcatgagcagcaatagaaaagtcggcgacgtcatcctcgacgtgcagaacatcagcttgagcttcggcggcgtgaaggcgctgacggacatcagcttcaacgtgcgcgagcacgaggtgcgggccatcatcgggcccaacggcgcgggcaagagctcgatgctcaactgcatcaacggcgtgtattggccgcagcagggctccatcactttccgcggccagaccttcaagcacatgaactcccgcgaggtggccgagatgggcgtggcgcgcacgttccagaacctggcgctcttcaagggcatgagcgtgctcgacaacatcatgaccgggcgcaacctcaagatgaagagcggcctgttcgcgcaggccctgcgctgggggccggcggaacgcgaggagctgcggcaccgcgaattcgtggagcacatcatcgactttctcgagatccaggcgcaccgcaagacaccggtgggccgcctgccctacggcctgcaaaaacgcgtcgacctgggccgcgcgctcgcgatggagccgcaggtgctgctgctggacgaacccatggccggcatgaacgtggaagagaagcaggacatgagccgcttcatcctcgacgtgaacgacgagttcggcgccaccatcgtcctcatcgagcacgacatgggcgtggtgatggacatctccgaccgcgtggtggtgctcgactacggcaagaagatcggcgacggcacgccggacgaagtgcgcagcaatgagaacgtgatccgtgcctaccttggggtcgaacactgatggccttctttctcgaaaccctctttggcggcctcatggtgggcatgctgtattcgctggtggcgctcggcttcgtgctgatcttcaaggcctcgggcgtgttcaatttcgcgcagggcgcgatggtgctgttcgcggcgctcgccatggcgcgttttgccgaatggatcccgatgtggaccggcatcgagagccgctggttcgccaacggcgcggccttcgtggtggcggggctggtgatgttcgcggtggcgtggctgatcgagcggctggtgctgcgccacctggtcaaccaggaaggtgcaacgctgctgatggcgacgctcggtatcgcgtacttcctggacggcgccggccagaccttgttcggcagcaacatctacaagatcgacatcggcatgccgaaggacccgatcttccttctcggctcggtgttcgagggcggcatcctgatcaacaaggaagacctgtacgccgccgcgatcgcggccgcgctggtggcgctgctctcgctgttcttccagaagaccggcaccggccgcgcgctgcgtgcggtggccgacgaccaccaggccgcgcagtcgatcggcattccgctcacgcgcatctgggtcatcgtgtggtgcgtggccggcgtggtggcgctcgtggccggaatgatctggggcagcaagctgggcgtgcagttctcgctcaccacggtggcgctgcgcgcgctgccggtggtgattctcgggggcctcacctcggtgccgggcgccatcatcggcgggctgatcatcggcgtcggcgagaagctgtcggaggtgtacctgggcccgtacgtgggcggcggcatcgagatctggttcgcctatgtgctggcgctggtgttcctactgttccggccgcagggcctgtttggcgaaaaaataattgatcgggtctgaacatgttctatagagaaaatgggcagttcaagtccagctaccgcgccgaccagcaggtcttcccgatccttcaggaccgcgtggccatcggcctggtgctgatcttcgcgttcgcggtcgtgcccttcgtcgccagcgactacctgatgcgggcgatcctgattccgttcgtgatcatctctctggcggcgctcggcgtgaacgtgctggtgggctactgcgggcagatctcgctgggctcgggcgccttcatggcggtgggtgcctacggggcctacaacttcttcgtgcgcttcccggggctgccgctgattcccgcgctgatcctgggcggcctgtgcgcaacgctgttcggcatcctgttcggactgcccagcctgcgggtcaagggcctctacctggcggtggcgacgctggcggcacagttcttcagcgactggatgttcctgcgcatcaagtggttcacgctcgacacgccttcgggctcggtgtcggtgtcgaacctgcaggtcttcggcttgccgatcgagagcgccgcgagcaagtacctgctctgcctggcgatgctggtggtgattgccgttttgaccaagaacctggtgcgcggcgccatcggccgcgagtggatggccatccgcgacatggacgtggcggccgcggtgatcggcatccgtccgatgtacgccaagctcagcgccttcgcggtcagctcgttcatcatcggcgtggccggtgcgctctgggccttcgtctacctgggtgcctgggagccggcggcgttctcggtggaccagtcgttccggctgctcttcatggtgatcatcggcgggctcggctcgatcatgggggccttcttcggcgcggctttcatcacggtgctgccgatcatcctgaaccaggcgctgccggtcatcgccggctggttcggcgcgcagatttccactgtcggcattgcgcatgcggagctgatgatcttcggcggcctgatcgtctggttcctgatcgtcgagccgcacggcctggccaagctctggtcgaccggcaagcagaagctgcggctctggcccttccctcattgaccgccaccgcgcaccgacatgttttttttcgaagcgcccattttttccagcgtgacttcccattcaaccaggagacaaccatgaaactgaaatcactcgcacttgccgtggctatcgtgtccgcgctcgcgggcgcggcccctgcgttcgcgcaggccaaggagcagttcatccccgtgctgtcgtaccgcaccggcgcctacgcgcccaacggaacgccctgggccaatggctatgtcgactacttcaagctggtgaatgcgcgcggcggcatcaacggcgtgaagatctccttcgaggaatgcgagacgggctacgacacggcgcgcagcgtggagtgctacgagcgcctgaagggcaagaacggcggcgcctccctggtgcagccgctgtccaccggcgcgaccttcgccatcaccgagaaagcgcccgtcgacaagattcccgtggtgaccgtgggctatggccgcagcgaaagcgccgatggcacggtgttcaagtggaacttcccgatcgccggcacctactgggtggccgccgacgcgatcatccaggccatcgccctgaaggaaggcgggctcgacaagctcaagggcaagaagatcgccctgatctatcacgacagcccctacggcaaggaaccgatcccgctgctgcaggagcgcgcgaagatgcatggcttcgacctgcagctgctgccggtgacggcgcctggcgtcgagcagaaggccacctggctgcaggtgcgccaggcccggcccgacttcgtgctgctgtggggctggggcgtgatgaactcgaccgcgctgaaggaagcgcaggccaccggcttcgcccgcgaaaaaatgtacggcgtgtggtgggccggcgccgaacccgacgtgaaggacgtgggcgacggtgccaagggctacaacgccgtgaccatgcagcacggtgccgagccgcaatccaagctcgcgaaggacgtggtcgcgatgctgcacgacaagaaccagggcacgggccccaaggaagaagtggggcaggtgctctacatgcgcggcgccatgagcgcgatgctcggcgtagagggcatccgcgccgcgcaggaacgcttcggcaaaggcaaggtcatgacgggcgagcaggtgcgctgggggctggagaacctgagcctcacgcaggccaagctcgacgctctgggctttgccggcgtgatgcggccgatcagcacctcgtgcacggaccacatgggcgcggcctgggcgcgcatccacacctgggacggcaaggcctggaagttcacgtccgactggctgcaggccgatgagcagatcatcaagccgctcgtgaggtcgaccgccgccaagtacgcggccgagaagaagctgacggcgcgtacgccggcagattgccagagctaggcccacccccagtcttcgcgcacttcgtgtcgcttcgccaacccccttcgagggggtaacacccgcggcccggcaaagccggttccgcggtgttccgcgaaggggctgctgggcggcttcgccagttattggaagcaatatgagttcaccgaacatcgttctcaacgtcaacggcatcgaggtcatctacaaccacgtgatcctggtgctcaagggcgtatcgctcacggtgcccgaaggcggcatcgtggcgctgctcggcggcaacggcgcgggcaagacgaccacgctgcgggccgtgagcaacctgctcgcgggcgaacgcggcgcggtgaccaagggcaccatcgaactgcgcggcgaccgcatcgaggcgctctcgcccgccgagctggtgaggcgcggcctgatccaggtgatggaaggccggcactgcttcgcgcacctgaccatcgaagagaacctgatgaccggcgcctacacgcgcaccgacggcaaggccgcggtgcaggagacactggagaaggtgtacgcatatttcccgcgcctgaagacgcggcgctcttcgcaggccgcctacacctcgggcggcgagcagcagatgtgcgccatcggccgcgcgttgatggccaacccgacgatggtgctgctcgacgaaccgtcgatgggccttgcgccgcagatcgtcgaggaggtgttcgagatcgtgaaagacctcaacaccaaggaacgcgtgaccttcctgctggccgagcagaacaccaacatggctctgcgctatgccgactatggctacatcctggagaacggccgcatcgtgatggacggcgaggccaagagcctgcgcgagaacgaggacgtgaaggagttctaccttggcgtcggcggcgcggaccggaagagctttcgcgatgtgaagagctacaagcgccgcaagaggtggctggcttgatggcgcgcatttcgtgttgtcccctctccctccgggagagggctagggtgagggtgcagcggctgcggccctcaccccagccctctccccaaggggagagggagcaagaccgaacagaaagacaaagggtacggacatgaccgaccattacgacgccctcgaaatccgtgaccccgccgagcgcgagcgtgacctgctggccgcgctgccgaagcagatcgcgcaggcccagaccgccgcacccgcgtttgcaaagatcctcgatggcgtgaagccggcggacatcaccacgcgcgaagcgctcgccaggctgcccgtcacacgcaagaccgaactgctcgagctgcagaaacagcgccgcgccgacgaccccttcggcggcttttccgccatcggccgcggcacccgcatgccgcgcgtgttcgcaagccccggcaccatctacgagcctgaaggcgaggcgcgcgactactggcgcacggcacgtgcgctgcatgcggccggctttcgcaacggcgagctcattcacaacagcttcagctatcacatgacgccggccggctccatcatggaaagcggcgcgcgcgcgatcggctgcaccgtgtttgcgggcggcaccggccagaccgagcagcagctcgaggccatggccgacctgaagcccgaaggctatgccggcacgccgagcttcctgaagatcctgctggagaaggccgaagaaaaaggcctgaagctgccttcgctcaccaaggccctcgtgtccggcgaagcctttccgcccagcctgcacgactggattgccgcgcacggcgtgaagggcacgcagtgctacgccaccgccgacctcggcctcatcgcctacgaaaccagcgcgcgcgaaggcctggtgatcgacgaaggtgtgctggtggaaatcgtgcggcccggcaccggagaccctgtacccgacggcgaagtgggcgagatcgtggtgaccaccttcaaccccgactatccgctggtgcgcttcggcaccggcgatctttcggccgtgcttgcgggcgcctgccccaccggccgcaccaacaggcgcatcaagggatggctgggccgcgccgaccagaccaccaaggtgcgcggcatgttcgtgcacccttcgcaggtggcggaaatcgcgcggcgctttccggaaatcctgcgtgcgcgtctcgtggtctcgggcgagatgggcgacgaccagatgaccttcaggctcgaatgcgacggcgcaccggccgggctcgatgcgcgcattgccgatgcggtgcgcgaagtgaccaagctgcgcggcaccatcgaactggtggcgccgggcacgttgccgaacgacggcaaggtgatcgaggatgcgcgcagctacaagtagcggcggtagaagcggcgcgtgatcatgcgcaccaacacgaccagcagcacgaggtagagcgccaccatcacggcggcgagcgccacgaggcggctgtcgctgctgccgcccgagaagctcccgctcgcgatccacagcagcccgccgagcgcgagcgcgacgcagaccgcctgcagcagcacgaaggccgacacagaggccgccacggcccggaagggacgcgcttgcgtgggccccggcgcggcgccgagccacccaccccagaacgccagcgcatagaccagcagcggcaccgcgaaccagcccagaagaagcggcatcacgtccgaatccctcgaggtgtcgacccagccgctcgcgatgttgccgatccacatctgcaacgaaacgaatatcgcggcggccacgagagccaccgcgcggcgaggcggtgccgtgtccgggccggcctccgccgcgccgggtggtgacgcatccgcgagcgcagcggcgccgcgctcgcgcagcgcgaaccgggcggcaagccacacgcccgcgacgaggacgagcacctggatgaccgactggaccagcatcgacatggccatgagcgagcgcaagccgtacgtgtcgacgcgctcgtgcagcgggccgcccggcatgaagagcacctgcgcctgatagaacagcggcgtcaatgccagaaggttgacgaccatcgccgcgaggtacacggcggcaaagcggctgccggggctccgaagccgcgcgatgcggggcgcaccgcgctcgtcgagcgccttgcgcgcatggcaccacgcaagcgtggcagccagcagccacaccgtgacgacgcgggacaagagcggaatccacacgcccggctgcgcatacacactgcgcatgtgctcgctgtgcggcgacgaaggcagcagcagcaccaccatgttcaccacgaacagggccgcatcgaccacgagtgcgatccatgcgaaatgtctgggcaggcgctgcgcgcgctcgaacgaagaagatgccgccatgggttggaatactttcgccttgcagaaccaccgcgccgcacgggccgtgcgggcgatgcgaagaaaaaggcgagcgtaccggaacgtggcggcgttccgaagaccgggcgctgcagcgcgcgttcagtgcgcgagcgcggcttcggcctcttccggagcgggccccacgtacaccgattgcggccggatcagccgccccttcttcacctgctcgcgcgcatgcgccacccatccgcacacgcggcccgccgcgaacacgcaggtgaaactctcgcggccgaagcccagcgcttcgagcagcagcgcggtatagaactcgacgttggtttccagcgcgcgatcgggcttcttctcgcgcaggatgtcgagcgcggcctgctccgctgcttcagccagttcgaagcgcgcggcctgaacggtgtccgcgttgccttccgcgcccagccggcgcagggcccccttgagcgcatcggcgcgcggatcgcgcacgcggtagatgcggtggccgaaacccatcagccgctggccactggcgacagcgccttcgagccatgcccgggcattggccgcggttccgatggcatcgagcgcatcgagcaccgggccgggcgcgccgccgtgcagcggccccttgagcgcgctgatgccggccagcacggccgacgccaggcccgcgccggttgacgcgaccacacgcgcggcaaaggtcgacgcgttgaggccgtggtcgcacacggtgacgaggtaagtgtccagcgcggcaacctgtgcttcggtgggcgcgcggccatgcagcatgcgcagcatgtcggcggcctgcggcagcgtttcgtcaggcgcaagggcctgcacgcccaggcgccagcgcatgaccgcagcggtgtagaccgcgggcgcggccaccagacgcagcgcggtggccaggtcgtcgccatcgggcaggcgggcaagcagggcgcgtaccgcttcgatgggcggcagcttgcgcaaggcggcatcgtcgttcggaggcaggcgctcgaaggcttcgcgccgtgcgcggcccagcgccgcgcgcaggccaaccacgctgggcagcgtatcgaagaagccctggaacagcagcgccaccgcgtcttcgtaccgccagtgccgtgcgatctcgtcgagctggtggccgcgaatcaccagccggccggcggcgccatccacctcggacagcaccgtgcgcgcggccaccacgccttcgaggccgtcttcgtcgtcgttcatcgctgtactcctgtgtttgcgtgacgaagttgattctggcggcgctaatattgacgtcaatcttgatttattgcatcaacatggcgacgaagacaccgctctggcttcccgctgccgaagccctcgcgctgatgcaggtgcgtccgcagacgctctacgccagcgtgagccgcgggcgcgttcgcgccaagcccgatgcggcggaccctcggcgcagcctctatcaccgggacgacgtgcagcgcatcgcggcgcgcacgcgcggccggcgcagcagcgaggcggtcgcgagcgaggccattcgatggggcgaaccggtgctggcgtctgccgtgtccacggtgtccgaagggcgcctctggtaccgcgggcaggatgcctgcctgcttgcggaacatgccacgctcgaagacgtggcagggctgctgtgggaaagcgcgccgccgcgcttcgccccggcccacgctcccgagccgttgcatggcgaacgcgcgacgccgctgcaggccggcctgctcgcgcttgccgcacgcgccgggaccgatccgccctcgcgcggccgcgccgccgcggtgctgaagtccgaagcggcggaagtgatcggcacgctggccgatgcattgctcgggccgtcgccttcgcgcaccgctccgctgcacatgcgcattgccgcggcatggcgccgcccgcgcgcagccgatgtgttgcggcgcgcactggtgctgctggccgaccatgaactcaacgcctcgaccttcgccgcacgcgtgacggcatcgacgggtgcctcgctcgcggcgtgtctgctcaccggcctgtccacgctcacgggtcccttgcatggcggtgccgcggcggcggtgcaggcgctgatgcgcagtgcgacggccatgggcagcgaagccgcggtgcgcgagtggctcgcgcacgaccggccgctagcggctttcggccatccgctctacccgcagggagacgcgcgctgcgccgccctgctggccggcatcgagctgccgcccacgctcgcggcactgcgcgccaccggcgaaacgctggtgggggaagcagcgaacgtcgatttcgcgctggcggcactggctgccgtgcacaagctgccggccgatgcgccgttgacgctgttcgcgctggcgcgcacggtcggctggacggcacacgtgctcgagcaacaggcctcggggcaactgatacgcccgcgagcgcgctacacggggccaggcgtcgcaaccctcagtgaatcgccacttcgtgcgcgagctcgaacagcttcgtcatctcgcggttgaatgccggcaggtcgtcgggccggcggctcgttaccagaccgcgatcgaccaccacttcctggtcggtccacttcgcgccggcattcatcaggtcgatgcgcagcgaaggccacgacgtcagctttcggcccttgacgccatcggcgttgatgagcgtccatggaccgtggcagatggcggcaatgggcttgcccgattcgacgaaggcgcgcacgaaggccacggccttctggttgatgcgcagtgcgtcggggttgaccacgccgccaggcagcagcagcgcatcgaagtcatcggcattggcgttcttgagcggcacgtcgacctcgaaggtgtcggccggttcgaggtgcctccagccgcgcacgctgccgtccagcggcgagacgatctgcgtctctgcgccggcactttcgagcgccttgcgcggctcggtcatctcggcctgttcgaagccgtccgacacgaggatggcaaccttcattccgtccagcgaggatgaggtgatgggcatgggtgaaattctccttgttggatgcctgatgacggcaacaaagacttcaccctagaacccacccccgcggcgggcatcggcacgcgccgggtctgcctgtcggacagttcgacggccggcaaacttctcttacgactgtatatgtcgttcggtttgccgctatttgcggcaggcgctcggcagtgccttgtcagccaggtcgtcaccagccacgcagttccatgcaatgccgtcatcggtggccgagggctccatgcgcagcgtgcctgccgcctttggaagcgcgacgtcgaccaccatggtgtccggatcgagcgtcaactccgcgccgccgggcaggctttcaggcgcgccggcgatcgagagcgagtcgggaatctcttccttctgcttgtagtagttgccgagcgcttcgcgcaccggcgcggcctccgaccaggcctgggaaacgaccgcccgggactggtattccttgtaggccggaatggccaccgcggccagcacgccgatgatggcaaccaccatcaccaacgccagcgcaccgccgccggcacggccggtgtacggcacgaagatcgcgagcaggtaagccacgggattgcggctcggcagtttcgcatccgcgtcgatggtgcgcgccacgcgcttggtgagccaggggtagccggcgatcacttcatggaacgagccccagaagccgctgttgcccgccgactggtcggcgtagcgctgcaggtcgacgttgcgccattgctgcgcaccggcggccagcgccacgagtgcgcggggcgcggagtcgggctgctcgcagcaggcggcgccgtgcaggtcgcaggtgtattccttcgcgcgagagtaggcggcgccgagcagtggcagccagagcaccggggcgcgccagatgtgacccgtgaggtggccgcgccggatgtggccgagctcgtggccgatgtagaagttgatgccgtcgggctgggcttccatcgcatcgaccacgtcggacagcagcacgacgaagttgcggccgaagaagcgcgtggcaaaggcattgaacatgccgtcgccatgcagcaggtaggcctcgggcgggttctggatgccgagatagccgcagcaggcctcgaagcgcgcatgcagctcgggcagctgggtgggcgaaagcttcacggccgtgcccttgatccaggcaatgacggccgattgcgcgaacacgtaggcgatgaagccgaacagcacgtagatcagcgcaatgcccagagtgccgagcaccagcagcgcccagaccagaaggccgagcacgagcgtgatgatgccgagcgagcgctcgcgcgggtagacccatggatccatttggaaattcctcctcgatgcggcccgtgggcctgcagtgtttatggttttttttcgcgcctccccaggcgcgacttgcgagcgcgcatcatgcccgaggaaagtgcggtttctggcacgtccctagggctattcgctatgggtcaggtcatggtcagcctttatgatcgcggccgttttcaattcaatcgtcgggagacatcatgaagaaattgcttgcttttacggcgattgccgctgccgccgcgggcgcctatgcccaggatttccccgcgggcaagaccgtcacgctggtagtgcctttcacagccggcggcccgaccgaccgcgtagcgcgcgacttggccgaagccatgcagaagaccctcggcacgacgatcgtggtggacaacaccgcgggcgccggcagctccatcggcaccgccaaggtggcccgcgccgcaccggacggccacacgctgctgttgaaccacattgccatgtcgacaatgccggcgctgtaccgcaagctgccattcaacgtggagaacgacttcgaatacctcggcatggtcaatgaagtgccgatgacgctcatcggcaagccgggcctgccggccaacaactacaaggaactgacgagctggatcgaggccaacaagggcaagatcaacctcggcaacgccggcctgggcgctgcctcgcacctgtgcggcctgctgttccagagcgcgctcaagaccgagatgacgtcggttccctacaagggcaccgcgccggccattgccgacctgctgggcggccagatcgacctcttgtgcgaccagaccaccaacaccacgtcgcagatcgaagccaagaaggtcaaggcctatgccgtgaccacgtccaagcgcctgagcacgccggcggtcctgaaagacctgcccacgctcgccgaatcgggcctgaaggacttcgaggtcaccatctggcacggcgtgtacgcgcccaagggcacgccggcgccggtggtgaagaagctcaacgaagccatcaaggccgccatgaaggacccgggcttcatcaagcgccaggaaggccttggcgcggtgatcaccaccgacaagcgcgtcgaaccggccgagcacaagaagttcgtttcggctgaaatcgccaagtggggcccgatcatcaaggctgccggcgtgtacgccgactgatcgctccgatccgccgacaacaacaaaaaagccgccgggccttcaggcccggcggctttcttcatggtggcgagggcgtcacttcggccggatcgcgtccgccgtgccctggatgaaggccttgatgctctcgatctcctcgcccgagagcttgcccgtgaagtcgggcatgccgcgccccacggcagggccgttgagaatgaacttgtccaggttctggatgtaggcggcgtccatgtagccgaggttcggaatgttgccgccgcggtccacgcccggcacgccgtggcagaacacgcagttgctcacatagagcatggtgccggcctgcaccttggcggggtcgtacttcaccccctccaccagcttgctcatgcggtactgcacgaactcgggcatcttggccgtgccgccgaccgcgaaggtgtagaccgtgcccggaccctgccgctcggtcgcgcgctgcgcgaggccgtagacaccgccccagcccactgcgaccgacacgtactgcttgccgtcgaccatgtaggtggacggggccgcgaccacgccggtaccggtgggggtctcccagagcttctcgccgctcttggcgttgtaggccagcaggcgtccgtcggccgtgccctggaacacgaggttgcctgccgtggtgagcgtgccgccgttccagggcgaggcgtagtccacgccccaggcttccttctgcgccaccgggtcccaggcgatgagacggccgaagggcttgctcttgggcggctcggcattggcgaacatcgcggtgttccagcccatccctccgtgcgggcggcccggcacgttctggtcgaacttccagtccttgtcgtccatcaggttgatcggcacgttctgcgcgggcaggtaggcgaggccggtctgtgggttgaacgacatcgggtgccagttgtgcgcgccgaaggggccggggatgctgtcgccgggcttttcgttctggcgtgcggcggcgatctcgatgggccggccgttcttgtcgtagccggtggcccagttcacctcgacaaaattcttcgccgaaatgaacttgccgttggtgcggtcgatgacaaagaagaagccgttcttcggcgcgtgcagcagcaccttgcgcgccttgccgcccagcttgacgttggccaggatcatcgactgggtggaggtgtagtcccagttgtcgcccggcgtctcctggtagtgccacacgtacttgccggtgtcggggttcagggccaccaccgagcccaggtagaggttgtcgccgcccttggggctgcgcttgctgtgcgcccagggcgagccgttgccggtgcccacgtacatcaggttgagttcgggatcgaaagcgaagctgtcccatgcggtgccgccgccgcccgcctcccagtatttgccgctcggatcccaggtcttggcggcgcgcgccatcgattcgtcctcgaaaggcttgcttggatcgcccggcaccacgaaccagcgccacttctggtcgccggtcttcgcgtcgtaggccgtgacgtagccgcgcaccccgtattcggcgccgccgttgccgatgatgaccttgcccttgaagacgcgcggtgcgccggtgatggtgtaggagcccttctgcccctcgatggtgttcttttcccagaccttctggcccgtggccgcatcgagcgcgatgagccggccgtcgtaggcggccacgtagacccggccctcatgcagcgcaaccccgcggttcaccacgtcgcagcagccccggaagcccttggacttgtcgacctgcggatcgaaggtccagagcttctgcccggtgcgcgtgtcgatcgcgtgcaccacgctccatgacgcggtgacgtacatcacgccatcgaccaccagcggcgtggcttccacgccgcgcgtcgactcgaggttgtaggaccagaccaggccaagctgcttcacgttgccggcattcacctggtcgagcttgctgaagcgcgactcggcgtagtcgaggccgtagctcggccagtcgggcgtcttcttctgtgccgcgttggcgcggatgaagtcgccgttcacctgcttgacggctgccgcggcgcggtcctgcgggttgcccggagcctgggcggaaaccgtcgacgcgcccaggcacagccatgcagcggcgagcggaagcagcccggcgtggatctttttcatcgtgagtctcctttgtgccgcaaggatcgtttttgtcgcccttgccttcaccttcgggatttccccagtccggcgctgttccattgcagaacacattcgagaggggccagcgatttccgattccccattttcctgattcccccgacttcgaggagcagcgaacagcatggctttcgaaaggctgggcacggcaaccgcgccgcgccaactcttttccaccacgcccgcgcagcgcgtggcgcttgcgcggcagcagttcttcgaggaaggcgtgcggccctcgggcctcgtcggcgaagcggtgatccagtcatggctgcgctgcacccgcaaccacagcgaccggcaacgcatcgtgcccttcgatgcggtcacgcccagccggctgcacgccacgctggcgcgcaaccgcgaactgctcgaggtcgcgcggcaagagctcgcgagcatggaaagcgcgctctcgggcaccgattgccgcgtgatcctgacggacggcgaaggcgtggtggtgcatgtcacgcagcacccggccggggcgcaccagccggtgctgcgcaagaccgcgcgcgtgggcgtgaacatttcggagcgcatcgtcggcaccaccgcgccgggcatcgtggcgaccaccggtcaggcctgcaccgtcgacggcgcggagcactatttcgacgtgctgtcgcagatgcaatgcgccgcggcgcccattcgggacgtgacgggccagcttgccggcgtgctcgacatcacgatggaggcgcggcgcttcggtttcgacgcggcctcgatggtggcgctgtacgccaccaccatcgagaaccggctgctgcaggcgcagtcgcgcgaccacctgatcctgcgcttccaggccagccccaccttgctgggcacgcccatggaagcactggccggcgtggcgcccgacggcaccatcgcgtggctcaacggcgccggcgcgcggctgatcggccgcttgcccgaggaggcctgcgagcgcgatgtcgagtccatgctgggccatgatctcgccagcctgctgcggctcgaacggcgcgacgccgcgcagccgctgcgcctggccagtggcctcggcgtgtgggtgcaggcgcggctcaaggcggcggacggcgcggacttcaggcatgcggtggccatgcccggcgagaccggcgcggtaatgtccatcgagcccgcaacgccgatcgacgcctgtgcggccgaagacagcgcgggagcggtggttccccgccacgcgcacatggaaacagaaatgccgcagggcgaaaccctgcgcgagcacagccgcaagctgatcgaggaagcgctggcggcgcagggcggcaacgtgtcgcaggcagcgcggcagctgggcgtgtcgcgcggcacgctgtaccggcggctgcgcgactggcgcgaagcggacaagggcacgccgaccgcgccggactgatcgcgtactggcccccgtcgccggtctttcaggccgaaggaattcggtactcgcgcgcggcgcgggcccggcgcgcgcgcgcatcgagctgaagaggccgcaggtactcgtgcaacgccagcgcggccgcgcccaccgcgggagccagctcgccatagcgggccaggcgcaggtcgggcgcgggcatgccggccgcatcggcatggcgcttcaccctctcgaaagccgcttgcgccaggccgcgatggtgggtgcacgacttgccgccgagcacgatggcgcgcggatcgaaggtgacccacaggttctgcagcagcacgccgaagaaggcggccgcacgcgccgtgtcgggtgcctcgcgctccagcgcgcgcgagccgaagaaggcttcggcgcagcctcttcgcccgcacgagcacagcggcccgtcgatctgcaggatggtgtggccgatctcgcccgccatgccttgcgcgcccgtgaacaggcggtcgttcagcaccacgccggcacccacgccgacgtcgcagctgacgaagatcagcgggtcgccgccttcgccgccgaagaactcgtactcaccgagcgcggcggcatcggcatcgttctgcagctgcaccgtgacgcccggcaggcccgctgccgcaaaggctttttcgagcgcgggcagcaggctcacattgcgccagccgaggttgggcgcaaagcggaccacgccggtgcaatcgtccaccgcgccgggcacgcagacgccgatgctcgacaggcgcagcccccgttcgttcaactgccggtgcccctccgcggccatgcgcgcgacctgcgcgcagacgccggccggggcgctgtcggtcagcgcgtgcgtgtcggcatggagcacctcgccctgcagcgagacgcaggccaggcgcaccgtttcaacggcgatctcgacgcccatcaatgcgcgcacgccgacgttgatctgcagcggcgtggaaggccgccccaggccatcggcaaccgtcgtacccgcttcgctgagccagccctcgtcgagcagctcgcgcaccagcaggctcacggtcgatttggtgaggccgctttcggtggcgagccgcgcacgcgagagccccggccttgcgcgcagcagccgcaacaggacgctgcggttcatccgcttgagcagctgttgatcgccgatggtcacgaaccgaccctcagcctgcgaaccacgagcgcgcctgcattcaccggtgcgcctgctcttttccttcagggcgcttgccggcgatgatcatgccgagcacttcgtcttcggtgacgtccgcggtgcggtaggtgccgacgagcttgccgttcttcatgaccgcgacgcggtcgctcagcgagaagacgtcgggcatgtcgtgcgtgatcaggaagatgccgacgccatcggccttgagctgcttcacgaggccgccgaccatcgcggtttcttcggggccgagcgcggcgcagggttcgtccatgatgaggatgcgcgcattgaagtacagcgcgcgcgagatcgccaccacctgccgctgcccgcccgagaggcggcgcaccggaatgcggatgttggtgaagttcttgttcaagcggttaaacaccttgcgcgcctgcacctccatgaagtggtcgtcgagcgtgttccagcgcgtcatcttctcgcggccgagaaagaggttggacaccgagtcgaggttgtcggccagcgccagcgtctggtagatggtctcgatgcccagcgcctgcgcctcggcgggcgttcggatgtggaccttctcgcccgcgatcagcgtgtcgccggagtcgatcgggtaggcgcccgcgagcatcttcatgagcgtggacttgccggcgccgttgtggccaagcaccgcgaccacttcgccgggatggaggttgacgctcacgccgtccaccgccttcacgccgccaaaggccttgcggatgtcgcgcagttcgacgaggggtctggatgtgtcgatggtgctcatctcagttctctccgaaacgcttgcgatagagaacgtcgaacaccaccgccacgatcagcacctgcccgatgatcaccatgcgcttgccgatgggcacgtcgagcagcagcatgccgctgtcgagcgactgcatgatgagtgcgcccagcaccgaaccgaagatcgaaccgctgccgcccgcgagcgccgtgccgccgatgacggcggccgcgatcacgtacagctccatgcccgtgccgagcgagttggtgccggcattgagccgcgcaatcgacacgatggccgccaccgtcaccagcaccgcaagcagcgcgaacagcatcagcgtgacgcgcttgaccggaatgcccaccagcgccgccgcatcggagttgccgcccatcgcgaacacgtagcgcccgaagcgcgtgcggtgcacgatgaacgacagcacgatggccaccacggcccagatcagcaccggaatcggcaggccctggggcgcgtctttcgaggcgatctggtagttgttcatgacggccgcaaaaacgaacaccaccgccaccggcacggcggtcagcagcagctcgagccacagcggctcgttgggcatctcgtgatgggcgcgcgcgcggcgcttctgcagcatgcgcgcgaacagcaccaccgccacgaacaccgcgagaacccaggtcgcggtggtgccgatgccgccgtcgtacccgccgcccaggcgctgaaagaactcgtcgttcaccggctgcgtcttgccgtcggccaccaggaaggccgcgccgcggaacgacatcagcccgcccagcgtgaccacgaacgacggcacgcccagcatcgccgtgagccagccctggtagatggacaccagcagcgccaccgcaagccccgccaggcaggccgtgggccaggaccagcccgaggtgtattgcaggtaggcgatcagcacgccgacaaagcccatgaccgagcccacggacaggtcgatgtggcgcgccacgatgaccagcaccatcacggtcgcgacgatgcccaccacggccgtctgctgcgcgacgttgtagaggttctcgggcgacaggaacacgccgccggacatcacgttgaagacgatgcccatgacgaccagcagcacgctcatcagcagaagccgcagatcgacgcccgcacgccgccaccagcctggcgtttgattgctcatttttcagatcctctcgaagaagaaacggaggtgcgcggccgcgcgccggcccggccttcgggccgaccggaaccgcgagacggcacggatcggggagcgcctgcgggcgcacccgctacttgcaggcggctggcgcgctggcggccgggacgcccttgcagagctcgtccttcttgatccagccggccttcacgaccacgtcgaggttgtcgcgcgtgatcggcaccggcgtgagcaggcgcgacgagagcgagatcttcttcggaccggaattccacggcgcggccttctcggccggcttgccctgcgtcagcgcgatggcggcgctggcggcttcgcggccgagttcgcgcgagtccttgaagacggtggcggtctgcgtgcccagcgcaatacggttgagcgccgcaaagtccgcgtcctgtcccgacaccggaacgccgcgcaggcccttggccgtgagcgccgccaccgccccgccggccgtgccgtcgttggccgccaccaccgcatcgaccttgttgccgaccttggtgaggatctgctccatgttcttctgcgcgacctcgggcttccagccctcggtgtattcgtcgccgacgatcttgatgtcgcccttcttcacggcggcgtccagcacctcttgctggcccgcgcgcaaaaagtcggcgttcgggtcgctcggcgagcccttgatgatcacgtagttgcccttgggcttgaccttgaagacctcgcgcgcctccatgcggccgacctcgacgttgtcgaaggtgatgtagaagacgcccggcgcctcgatcaaccggtcgtacgcgaccacgggcaccttctggcgcgtggccttggtgatggctggcaggatcgcgtccttgtccatcgccagcacgatgagcgccttggcgcccttggacatcaacccctcgatgtcgcccagctgcttctcgggcgagccgcccgcgtcggcactgatgtacttggcgccgagcttctcgagctgggccttgatggcggcctcgtcggtcttccaacgttcttcctgaaagttggaccagctcacgccgaccacggtctgggccagtgcgcccactgcggtgaggccgaaggccatggcggccagggtgtgcttgagttgcatcgatgtctctccttggaggatttgcccggcgaaaaagccgtgtaagaaattagttagtttgaagggcgaactaactatcccatcgccgccggacgatgggcatccgggaattcccggggaacaggcgcgcgcggaggcgtggcgaaacatcgaaatattcaatgctcagagaaaaaatatatcgttttcggttatgtgattcgctgcttaaagttcggcgctcctgaactcacagatgcgattcgaaccatgaccgcgcccaccgaaagaattccgttccatctggcttttcccgttcgcgacattgccgaagcgcgcgccttctatggcaagcttctgggttgcccggaaggccgcagcgcgcccgagtgggtcgatttcgatttctacggccaccagatcgtggcgcacctggcgcccgatgaatgcggccacaaggccagcagcgcggtggacggccatgacgtgccggtgcgccacttcggcgcgattcttccgatggacaaatggcaggcgatggccgacaagctggtcgcccggaaaacccgcttcgtgatcgagccctacatccgcttcaagggcgagccgggcgagcaggcgaccatgttctttctcgacccctcgggcaatgccattgagatgaagtcgttcgcgaacctggactcgctgttcgccgtctgaaagcgccagccacagcagatggtgatgactcattgaaccgcgcatcgattcttgagatgctcggttcatgatcaacgagctcagaaccttcatctccgtctgccgccacggcaccttcgccgccgccggagaacggatcggcctgacccaatcggcggtcagcagccagatcaagcggctcgaagatgccttggggttcgagctcttcgacaggaccgggcggtcggccaccttgaacgccgccggggagacgaccctggcacgcgccgaggagatctgtgcgctctatgcaaagctcggcgagctgccggacgacgcctcgaacggcgggctgctgcggatcggcgccatcgcttcggcccaatcgacgctggtggcgcgggcgctggccaagctgcgcgccacgctgccgctgctgcgggtccacgtgtcgccgggcgtgtcgatgcggctgatggacgagctcgacgcgggcaagatcgatgcggccgtgatgatccggccgccgttcgggattcttccggacctgatgtggcaatcgctggtgcacgagccttacgttctcattgcgccgacgaaggtgcccggaaaagactggcgcacgctgctccaggagcagcccttcctgcgctacgaccgcgcgtcgttcggcgggcgcatggtggaaagatttcttcggcgcgaagggcttgtggtgaaagacgccatcgagctggacgagatacccggcctcatccacatgaccgccaagggactgggcgttgcgctggttccgctggtcgaggcgcaccttccccttccggcgggcgttcgcgtgctttcgctgggcgagctcactttctatcgcgaggtggggcttcttcaacgcaagccgcgggcgagtccgccggtggttgcgcagtttgcgcagtgcttgcgggaggcggcagaagccgcggaagaaaaggcccggcctccgaaggcgaaggccgaaggcgccaagcgccgctaggccgtcgcccgccgcatcagcggttggcgagcggaaattcttcggcgctgaacaccgtgtgaaagaccgtgccgtcgaacatctcgaacagatgcttggagagctcgcggctttcgtagcgcacgggcgaatcgagcgccagcgcgatgtcttcgcggctggcatagcgggtcgacagcaccatggccagttcgggatcgctcacatcgctttcgatctggcgcagcacgcgcacttcgagcacgccgggaaaacgggtccagagcggcaccagcttctcgtgcacgtgccggtcgaaagcctcttccatgccggccttgaccttgccccggaaaaacgcgcaacggatgaacatgggtgtcttctttactggttgaaatgtgttgtcgggccgcgcgcagggtgcggccaatgcgtgcttcagtcgcgcgcgtagccgttgaactggcgcatcatggccgccgtgtcctcggccccgagaccggccgccacgaaggcgcggtgcagctcggagaccgcgcccgccagtggcagcggcaggcgttcggcttgcgcaaaagcctgcacggcctcgaggtccttgagcatgttgtcgatgcggccggtgggcgtgagatcgcgtgcggccatcttggggccgaactcgcgcaggatctggctgtcggcccggccgccggccagcgcggtgtgcagcttcgacgcatcgacgccgccggcttcggccagccgcaccgcctcggccacggcctggaagccgatggcgcagagcagctggttgaccagcttggtggtctgcccggcgccgctttcgcccatgcgggtgtagttggcgcacaggctgtccatcacggcgcgagcacgtgccacgtcgtcttcgctgccgcccgccatgaccgtcagctggccgacgagggccttgggggcgccgcccgagagcggcgcatcgacgaagcccatgcccgtgcgttcgcgcagcagctgcgcgagccgacgcgtggagaccggatcgatggacgacatgtcgatcagcagccggcgcgaatccgcgggctcggcggcggccacgccggtttctccgaagagcgcacgctccaccacggccgccgaattgaggctggtgatgacgaagtcgctagccgccgcggccatggccgcggtgccggcgacgtgcgcgccgtgcggctccagcgcggcgaccttggcggtgtcgaggtcgaacacgcgcaccgtgtggccgcattcgagcaggcgccgcgcaatggccgagcccatgatgccgacgccgatcacggccacgcgctggcttgggaatgtcatgcggcaactttcagtgaggcggagcaattctgtgcgaacgcgatcaggcgcgcgcccacagaggccacgatcagcggcaccggctcctcgatgccggcgtgcagtacctccggctcgtccgcgccgggtttctcgaagctctgcagctggctgtcgagcagcgcgggcggcatgtaatggccggtgcgttcctccagccggtgccggaccagtgcgcgcggaccgtccaggcagacgaagtgcaggccgggtgccgccgtgcgcaagcggtcgcggtaggcgcgcttcaatgccgagcaagccaccaccacgcctgccggcgccgcagcttcgtcgctcaatcgcgcaccgatgcgttccagccaaggccagcggtcctcgtcgcagagcggcacgccgccgcgcatgcgcgccaccgcctccggcaggtgcaggtcgtcgccgtccacccagggcacgcccagcacacaggccaggccggcggccacgctgctcttgccggtgcccgagacgcccatcaccaccacggccagccttgcccggtgcggttgctgctgaaggggggccatgggaatcagaggctggcggtgatgccgccgtccacgtacaggatgtggccgttgacgaagctcgatgcgtccgacgcgagaaagatcgccgcgccgcccagttcttccacgtcgccccagcgcccggcgggcgtgcggccggaaagccacgcggtgaatgcctcgtcggcgaccagcgcctgcgtcagctcggtcttgaaatagccgggccccaggccgttgacctggatgccgtacttgccgaggtcgatggccatgcccttggtgagcatcttcacggcgcccttggtggccgcgtagggcgcgatgccggggcggcccagctcgctctgaaccgagcagacgttgatgatcttgccgcgcttgcgctcgatcatgcgctgcgccacgaagcggccgacgaagaacacgctgtcgatgttggtggtggtgatcttgtgccaggcgtcgatcggaaactccgcgaacgcgccgcggtgctgcatgccggcgttgttgaccaggatgtcgatggggccgacttcggcttcgatgcgtgccacgcccgcttccaccgcggcggcgtccgtcacgtcgaaggccatggcttcggccgcgacgccccgggcgcgcaaggcgtcgcgcgcggcttcgagcgcgccggcatcgcgcgcattgagcacgatgcgtgcgccggccgagcccagcgccgcggccagcgcgaagccgatgcccttgctggagccggtgatgagggcggtgcgcccggagaggtcgaacagtttcaagcggggctccaggaggaatgggcggaatgcgcacgaggcggcaatgcgaatacgttaccggtatcctattggagcgtcaagggtgaaaaccttggtggaacttcctttggacgacctcaggcaaaggttaaagttaccggtatctttattgcgcccagccgcgccacccgcaggagaattcgcttgaccgctgccactacacccccgcacgtgctgatgcccggcccctatccggaatgggacatggcgccgatggcggcgagctacacgctgcttcgctggtgggaggcgccggaccggcaggccttcatcgccgaacacgccccgcaaatccgcgcggtggccacgcgcggcgagttgggcgcgagcgccgagctgatcgcctcgctgcccaggctggagctggtcgcctgctacggcgtgggcaccgacggcatcgaccttgcggcctgccgcgcgcgcggcatccgcgtcaccaacacgcccgacgtgctcaatggcgacgtggccgaccttgccgtgggcctcacgctcgcgctgcagcggcgcattccggccggcgaccgcttcgtgcgcagcggcgaatgggcccagggcccgatgccgctggccacgcgcgtcttcggccagcgcgtgggcattgccggtttcgggcgcatcggcagcaccatcgcccggcggctctcgggcttcgagatggagctgggctacttcagccgcacggcgcgcgaagacagtgcgctgcgccacttcaacagtcttgcggccatggccgaatggtgcgacgtgctcatcgtcatcctgcccggcggcgaggccacgcgcggcatcgtcgatgccgaggtgctgcaggcgctgggccccaagggctggctggtgaacgtgtcgcgcggcaccacggtggacgagggcgcactgctgcaggcgctcgagcagcgcagcatcgcgggcgcggcgctcgacgtgtttctgaacgagccgcgcatcgacccgcgctttgcggcgctcgacaatgtggtgctgcatccgcaccatggcagcggcaccgaggagacccgccgcgccatgggcgaactggttcgccgtaatctgcaggctcacttcggtggccagcccctcgtcaccccggtcgcctgacggcctgaaggagaaccccatgcgtatgcgttgtatgtgcctcgtgatccatgcccccgatgacctgcgcctggaagaacaggacgccggagacatcggcccgggccaggtgctggtcaaggttggcatgggcggcatctgcggctccgacctgcattactttcacaacggcggcttcggcaccgtgcgcatcaaggagccgatggtgctgggccacgaagtggcgggcaccgtggtggccacggcgcccggcgtcgacagcgtgcgcatcggcgacaaggtggccatcaacccgagccgcccgtgcggcgcctgcaagttctgcctcgaaggcctgcccaaccagtgcctggacatgcgcttctacggcagcgccatgcgcacgccgcacgtgcagggcgcgttccgcaacatgctgctgtgcgaggccacgcagtgcgtgaaggtggcggcgcacgtgccgctgcgcctcgcggcgctggccgagccgttctcggtggggctgcatggcgtgtcgcgcgcaggcccgctcctgggcaagcgcgtgctggtgtcgggctgcgggcccatcggcgtgctggccattgcggcggcgcgtgcgcacggcgcggccgaaatcaccgccaccgacgtcgtcgacgaaccgctcaccttcgcgcgcgccatgggcgccgaccacaccatcaacgtcgcgcaggacaaggcctgggtgtcgcgctattcggccgacaagggcaccttcgacgtgatgctcgaatgctcgggcaacgagcgcgcgctgcgcgacgggctggaggtcatgcgcccgcgcggcgtggtggtgcagctggggctgggcggcgacgtgagcattccgcagaacatggtggttgcgaaggagctcagcatctgcggctcgttccgcttccatgcggagttcgcgctggcggtgcggctcatcaacgaaggccgggtcgatctgtcgccggtcgtgtcgcacaccttcccgatgcagcaggcacgcgaggccttcgaactggcgagcgaccgccagcgtgcgatgaaggtgctgatcgactttgccgacaccggcgcggaaaacgccgcggcctgatcggcctcaggagctttcccgctgcacgacgcgaaacgggatcagcaccgtttccgcgggcggccgattgccttcgcgggcgccgtcgatcacccgcagcagcagttcgcccgcggccctgccgatgcccacgcaatccaccgccacggtggtgatgcgcggatggcaggcgcgcgccacctcgaagtcgccgaaacccgcgatcgcgatgcggcccggcacgtcccagccgcggcgctggcattccatcagcgcgccgaaggccgagagatcggacacgcacatcacggcatccacgtcgggccattgatggatcagctgcaccacggcctcgcccccttgcgccatcgagatcggcggctggccgaagctgatgacgcgcccatcgggcaggcccagttcgcggatcgcctcgacatagccgcgctgcctgtcggccccgcgggtgtcgcggttcgaggtgccgccgatgaaggcgatgcgccggtagccctggccgtgcaggtgccgcaccatcgcggcggccgcttgcgcgttggagaagccgaccgtgtgctcgatgggggtggcgggcagatcccaggtctcgaccaccggaatgccggccgcctgcagcatggcgcgcgcggcggacgtgtgcgcgcctccggtgaggatcacgccctcggggcggcgcgcgagcatcgcacggacaaggcgttcctcggtctccacgcggtagtcggtatagcccagcagcagctgcaacccgcgcgcttccagggcggcggcaatgccttgcgcggtttctgaaaagttggagttgttcagcgacggaatcagcaccgcgacgaaacccgagcgcttgctggagaaggtgcgcgcggtctggtcgatgacgtagcccatctcttcgcaggcctgcaggatgcgctggcgcagcgcctccgaggtggcgcggtcgctgcccgtgcgccggttgagcgcacgcgacacggtcatcttcgagacgccgacgcgcgcggcgacgtcggccatcgtcgccggacgaggcaggggggcggaggctttggtcgagggcaaggtgctttctctggatgcgggtccgaggataggcgaggacgggcgggaacagaggcttaaggttaccgatatcgcaaagcaagggactacatgcatccctggttcagcgtgctggcgccatcacgttgctcctcgccagccttggcctctaagggggaggtccggcacatcaacataggacaactttgcgttgagaaaaataccaatcactattcttctcagaaaaaataaagtaaactatttttttcttcccatagggcacttgccatggcagcaacggttccgtcttatgcagacgtcgtgatcatcggaggcggcgtggtcggatgctcgatcgcctatcacttgaccaagctgggcatccgcgacgtgctgctgcttgaacgcagacaactcacctgcggtacgacttggcacgcagccgggctggtcggccagcttcgtgcgacgcgcaacctgacagagctggccaaatacacgaccgatctgatctacaaactggaggcggaaaccggccaggccaccggactcaagcagaacggctcgatctccgttgcattgacgcaagagcgaatggaggagttgaagcggcaggcttcgatggcgcagaacttcggcctggaggtggatgtcatctcgccacgggacatcttgcagcggtacccgtacatcaacctcgacagcgtggtggggggtgtattcctgcacaaggatggccaatgcaatcctgtagacgtcacccaggcttatgccaaaggtgcgcgcatgggcggggcgaagatcatcgagaacgtcaaggtggaacgcatcctcaaggaaggcggcaaggctgtgggtgtggtcaccgaccaaggcgaggtgcgttcctccaccgttgtgattgccgccggcatgtggtcgcatgagctgggccgccagaccggggtgaacattccactgcatgcggcggaacatttctacatcgttaccgaccacatcaaggatttgccagggaatctgcccgtgctgcgtgtccccgacgaatgggcctactacaaggaagatgcaggcaagattctgcttggttgcttcgagcccaaggccaagccgtggggaatgaaggggatccgcgaagacttttttttcgactccctgcccgaggacatggatcacttcatgcctgtcctggaaaaggccgcttcacgcatgcccgcactcgaaaacacgggcatccaaacctggttcaacggcccggagagctttacgcccgacgaccgctatctgctgggtgaaaccgcggaagtcaaagacctgttcgttgcctgtggcttcaattccatcggcattcagagttcggggggcgcaggcaaagtactggctgaatggatacgggaccgccgcccaccgctcgacctggtcgacatcgaggtgcagcggatgaatccgtttcagggcacccggcaatatctgcatgaccggaccgtcgaaaccttgggtttgctctacaagacacactggccgttctaccaatacaccacggcgcgtggcgccaggcgcagtcatttctacgacaagctcatgcaggaaggtgccgtgtacggcgaactcgccgggtgggagcgccccaactggtttgcgccaaaaggcgtggcgccagaatacgaatacagctacggtaaacaaaattggttcccgcatgttgcggccgagtgccgcgcgacgcgggacagcgtcgcgctgtatgaccaaagcacgatgaccaagtttctggtcgaagggcgagatgccttgacggtcctcgagaccatttcgtgcaatcggatcgacgtcccgttgaacaagctcgtctatacgcagtggctcaacccgcgcggaggaatcgaggcggacttgaccatcacccgaacgggcgaacagcagttcctggtcgtatctgctgcggcgacacacttccgggacctgtcctacctgcgccggcacgccgaggcggcgagccactgcttcgtcgtcgaccagacggcaggtacgccaatgctgggcctgatgggaccgaaggcgcgtgcggtgctggaaaaggccgcaccgcacaccgacttttccaatgacgccttccctttcggtacatcgcagatgatcgagatcgggtatgcgcaagtgcgcgccagccgtatcacctacgtgggcgaattgggatgggagctttacatcccaggtgaatttgccctgcatgtctacgaacggctgcgtgaagctggctcggaattcgggttgtcgctggccggcatgcatgcgatgaacgcctgccgcatggaaaaaggctaccgccattggggtgacgacatcagcgtcgaagacaccaatatcgaagctggcctcggctttgccgtcgcttacgacaagccaatcgatttcattggcaaggacgcgctgctgcgtcaaaaagccgagggcacacccaagaagcgcctgctccagttccggctgaaggacaccgaccgcctgctttacaaggaggagccgatctgggtgaacaacgcgcgtgccgggtcgatcacttcgggcatgtacggccaccgcatcgaagcgtcgctaggtatgggctatatacgcgcgtccgaggcgatcacagccgaatggctgacggcacagaagttcgagatcgaaattggatgggagcgctacgaggcgcaggctcaactggcacctttctacgatcccaaacagcagcgcgtcaaggcatgaacggcgtcaggacagccaaacccaaacggagaagccgaacgggggaaacctctgctgcttcgatcccccttctctctggagccaccgtgaacttgccttctctttcctatgtgctgagcctgacctgcaacgaccggcgcggaatcgtcagcgccgtttctcgattcctgagtgatcgcaatgggaacatcgaagaggccgcgcagttcaatgatcaggaagccaagcgtttcttcatgcgcatagctttcaccatgcaggaagaagccgtcagcctgcaggacttgcgctcgcaatttgcgaacaccgccgaggaattcggcatggagtggcagttagtggacacgcaggtgcgcatgcccaccgtcatcatggtgtccaaactcggccattgcctgcatgatcttctgttgcgctggaagaccggactgcttcccatcgacgtcagggcgatcgtgtcgaatcatcgagacttctatcagttggcggcctcctatgacatcccgttccaccacattcctgtctcgcctgacaccaaggcagaagcagaagccgagctgctgcggatcgttggtggggaaaaagcagagctggtcgtgcttgcccgctacatgcaagtcctgagtgatgacctttgtagaaaacttgccggcaaggccatcaacattcaccacagctttctgccaggattcaaaggcgcgaaaccttactatcaggcttacgaacgtggtgtgaagctgatcggtgccaccgcccactacgtcaccggtgacctggatgaaggccccatcatcgagcaaggtgtcgaacgcgccgaccatgccatgagcccagcggcactgacgtctcttggcagggacgtggaaagcgtcgtattggcccgagcggtcaagtggcatgccgagcaccgcctgatccccaatggaagccgcaccgtcgtcttcaagtaaacggcttcgctcatccgcgaagcgattccccgcagcgcgaagtcccgttttgccagcaggaaaaaactgcaaaccttttgttcttggaaggaaaagccgctcggttattatgtgcttcggtgatgaagacagacaatatccttgcaggcggagattcggcaccggcaaatgtcgacggtgcgagcctgggtgaagagatcagaaaacttcggaaggcgcgaggctactctttgacggacgtggccacggcaatttcgcgttcgatcagcttcatcagtcaacttgaaagaggcaacgcgtccccatccatcgcagacctcaggggcatcgcgcaaaaattggaagtgcccttaggctggttcttctcgcacgatcaggttccatccaacgagcgcggaaaaatcgtaaggagcaccgagcggcgacggctaggcactgtgacgagcgggctgctggaagagttactttcgcccgatataggcggtgcgtttgaaatgttcctcagtacctttgaaccgggcgccgcacttcgaactttcaatcagcgcgacaccgaagaagaaggctatgtcgtcagaggcagtctgaacctctggatcgggaaaaagcgtttcacggtaaatgccggcgacagtttcagaatcgtgcgcgagccctttcgatgggccaaccccaccaaggaagatgcggtggtggtctgggtgatctcccctccaacctattgatcattggcacacctgccgctcgcttgactgcccctcttcaagccggcgctgccctcccaatcacgccgaccatcaattccgccgggcacgaccggtgaagttcgcccgtgccagtgaaccgcggaactcgatgcgccggggactccagttgcggtcggcaccgagtggcttgtcgcttgcagagtgttccggtcttcactagcgcctttctcctgcgaaggttcctggcaggtaaccgggggcgccccaatcggttccttgacttctggcgatcgcccgcggattgcgcacgcgtctgggttgagaaaaatattgccttgcttttttttctgatcaataattagttcaacgtttttatttttcgggatcaggagaatttcgtccgaataaggacccgccgacgacgtaggtgttcagcaccagggtggttggctcatgtgtcgcttggtcggatgacacagcgagaagtgcgatcagccggatgtcggacgatgacaacgttgccaaccctcttcactccaggatccgacatgcaactcaatcacctccaactcgcggcgctttgcctcggcttagtcgtcggcaccactgcacagtctgcagaacaggtcgtcaagatcggcatgaccggccccctgtcgggcggcaatgcgtacgctggcagagacaatcagaatggcgtcgccttggccattcaggacttgaacgcaaagaagatcgtggtcggtggccagacgatcaagttcgaactccagtccgaggacgatcaatgcgatccgagggctggcgtgacggtcgcacagaagcttatcgacagcggcgtcaagtacgttttcggtccttactgctcaggcgtcgctataccggcatcgcgcatctacagcgaaggcaacgcgatgctgtccacggtcggcagcaatcccaaggtcacgcagggcgggtacaaaaatctgtttcgcatcattgctggtgacaaccaagttggagcgagcatggccacctacgcggccaaggcactcaaggcaaagaccgtcggcgtcatcgatgatcggaccgctttcggtcagggcctggcggatgaattcatcaaggaggccaaagcactgggaatgacggtggtcggtcaggaattcaccactgacaaatcggtcgacttttctgcgattctcaccagtctcaagagcaagcaacccgacgtcatcttcttcggcggctacaccccgcaaggcgccccgctggtgcgccagatgaagcagcttggcgtcaatgccaagctactgggaggagacacggtctgcacgccggaactcggcaagattgccggaagcgcggctgacgataccctgttctgcgcgcagggcggtgccatcttgaacaaaacggcaaacggcccgcaatttcgggcgacgtaccaaaaacgcttcaatcaggagcccgatgcctatgctgcgtcgttctacgaccagaccatgcttgtggccgaatcgatgcaaaaggccaactcgctggacgtcgacaaggtcggcgccgaaatgtacaaagcatcctataaagggatcgcaggactgtatgagtacgacgaaaagggcaacatgaagaaggcgcccgtcaccgtttacgtattcaagaacggggtgcccgtgcccctcgaaagttattgaggcgatcgcacggccaaccgtcgccctggacacgcccatgtacgagtcaatgcgtgcctgcaggtacagcttgcgccacaacttcgcgatgggccacatgaggctcgattgaacggggtgactttttggacgagaaatttgtccagcaggcctgccgcaccatcgactaggtgcgggcgagccacttggtcgcgctgacggcactgacaccgggcaagacgacggcatttgatgcgctgacgccatgctcagtgacgtcttgaaccatctccgggccgcgcaggtacgtcacggcgtatctacttgcttccgacatgcactcggcagttttgggtgtgttcatgaaatcctttagcccggcggggtaagccccgtgcccgatttccgtctcgtttgatacgatttttgccaaagccgccggtttcaaaggcgttggagacaagatgggttcgagcatttcaccgagcggcgccggccaggcgctgtaccgcaccatggtgcgcatccgcgcctttgaaaatgccgcggaagcggcgagccagggtggcgtgagcgcctatggccagcaggccgccggttccgccaaggtgcgcggaccgctgcacctctcgaccgggcaggaggccgtgcccgctggcgtgtgcgcccatctgcgaacgagcgactacctcacctccacgcatcgcggccacggccatacgctggccaagggcgcggacctgacacgcatgatgtgcgagctgttcggcaaggccaccggtttcaatggcggcaagggcggctcgatgcacatcgcggatttttccgtcggcatgctgggcgcgaacggcgtggtggcggcgggactgccgattgcagtgggtgcggcgcatgcgcagaagctgctgaagaaaaatggcgacatcacggtctgcttcttcggcgatggcgcgatcaaccgcgggccctttctcgaggcgctgaactgggcgcgcgtgtacgacctgccggtgctcttcgtctgcgaagacaaccgctggagcgccaccaccgcgagcggaccgatgacggccggcgaaggtgcatcggcacgcgccgcctcgatggacatcgcggcgacgcaggtcgatggcaacgacgtgttcggggtgcacgaaaccgcggccaggctggtcgccgaggtgcgcggcggtgacgggccgcgcctgctgcatgcgctgacctatcgggtgaaggggcatgtgtcggtcgacgtcgcggcttaccgcgatccggccgaactggctgccgcgctcgaaaccgatccgatcgcgcgggcacgcgggcatctcctctcgcacggcgtcagcgcagccacgctcgatgcgatcgagaacgcggcgcgcgacgaagtcgataccgcgctggccgtggccgacgcggcgccctggcccgagcccggcgacgccttcaccgacgtgcagaccatcggagccgggcaatggcactgacgatgacgcaggacctcagctattccgaagccgccgtgctcgccatccagcgcgagatggaggccgatccgcgcgtggtggtgctcggcgaggacgtgggccgcggcggcatcttcggccagtacaagggcctgcagcaggccttcggcgccgagcgcgtgatcgacacgccgatcagcgaggccgcgatcatgggcgcgggggtgggcatggcgctggcgggcctgcggcccgtggtggaaatgcgcgtggtcgacttcgcgctctgcggaatggacgaactggtgaaccaggccgccaagaaccgcttcatgttcggcgggcagggccgcgtgccgctggtggcgcgcatgccgggcggcatctgggatgcctcggccgcgcagcattcgcagtcgctcgaagcctggtttgctcacctgccgggcgtggtggtggtgagcccttcgacgccgcaggacaactacagcctgttgcgcgcggcgctgcaatgcggcgatccggtggtctacatcgagcacaagacgctctggggccagcgcggcgaagtgaacgaggacatggccgtgccgctcggcacggcgcggcgcgtgcgcgagggcgacgcgctcacgctcgtgagctggagcaagcagatgcaggcgtgcgccgcggcctgcgacacgctcgcggccgaaggcattgcggtcgacctgatcgacctgcgcacgctctggccctgggaccgcgaaacggtgctcgcatcgtgtgcgcgcacgcggcggcttttggtggtgcacgaggcggtgcaggtggcgggcttcggggcggagattgcagccagcgccgcggaggccacggggtgccgcgttgcgcggctcggcgcaccgcgcattccggtcggctatgcgccggtgctcgaggcagagtcgcgcgtcggcgccgaagccatcgcggccggcgcgagaaaactgctgggctgagccgccgtgcgccatggacccgctgttcttcaagctggtgcgggtggtcaacctcacggcacgcccgttccatgagaaggtcggccgcgagcaccatctcacgctcaacgaatggcgcgtgatggcggtgctgggcagcgagcccgggctcaacgcgacgcagatcgccgacttcaccggcctcgacaagatggcggtgagccgcgcgctggccggcctgaagcgccacaagcgcgtgcagcgcctgggcgaccccaccgaccggcgccgtagccggctctatctcacggcggccggcaaggcgctgcacgaaaccgtcggcgcgctgggccggcagcgcgaggccgtgctgttcgagggcgtgaacgccgacgagctggcccgcctcgacgccaccctggacaagctcgttgccgccgtccagcgcgccgactgaggcgcctggtcaggctgcgaagccgccgtcgatgttgaggctggcaccggtgacgaaacctgcctccgggctggccagataggccaccatgccggcaatttcctcggggcgcgcatggcgggccagcgccatcaggccgtgcatggcggcggcgttcgggccgtcgacggggttcatgtcggtgttgaccgggccgggctgcacgttgttgaccgtgatgccgcgcggaccgaggtcgcgcgacaggccctgcaccagccccttcagcgccgacttgctcatggcataggcgctgccgccgggccagggcatgcgctcggcgttggtgctgccgatgttgatgatgcggccgccttcgcccatgtgccgcgcggccgccttggcggccacgaacacggcgcgcacgttgatgtccagcgtgcgatcgaaatcctcgagcgagaaatcttccagggtgccgggcaggaacacgccggcgttgttgacgagcacgtcgatgcggccaagcgtgcgtgcggcttcatcgatgccggcggtgagcgcggcggcgtcggcgctgtcgatcttcagcgccagcgcgcggccgccttcggcttcgatgctgcgcgccaattcgtcggccggcgcgctcgaactcgcgtagctgaaggcgacggcggcgccatcttcggccaggcgccgcacgatggcggcgccgatgccgcgcgaaccgccggtgacgaaagcgactttgcccgcgaggatgggagaggttgatttgctgggagccatgatgggtattcctgtcggttgtgaggttgaaggccttcagtgtcgtgattcaattaccttcgcggtagccaccaattgacgcaatcaaattcaaccaatggttgaaaatagcggtccatggaaccgctcaatcacctcgagtccttcgtccagagcgcggagagcggcagcttctcggctgcggcgcggcggctcgggctcacgcctgccgcggtcagcaagaacgtcgcgcggctggaagcccggctgggcgtgcggctgttccagcgcagcacgcgccgcctcacgctcaccgaaagcggcgaacgcttcctgggccagattggcggcgcgctcgccacactgcaagatgtggtggccgatgtttcgaagaacgacgggcagcctgccggcacgctcaaggtgagcatgggccaggcgttcgggcgcgagcacgtgctgccgatgatgggcgacttcctggcgcgctatccgtcgatcctgcccgactggcacttcgacaaccagcaggcggacctggtgggcgaaggcttcgacgcggccatcggcggcggcatcgagctgtcgccgggcatggtggcgcgagagctgtcgcgcattcacgtggtggcggtggccgcccctggctatctggcgggccgcacgctgccggcgcaccccacggagctggtgcggttcgacgcgctgctgcgccgctcttcgcccacggggcggctccgcagctggacgctgcagcatgccggcggcgaccagaccacggtggagctgcctcgcccgcgcgcgatcttcaacgaccccgaagccattgcgcatgccgcgctgatggggctgggcgtggccatgctgccgatgcctttcgtcgagcgcggccttcgcagcggcgaactggtgcgcctgctgcccgaatggcatttcgacgcgggtgcggtctggctctactacccgagcaagaagctgctgcccgcgaagacgcgggtcttcatcgacttcgtgctggagcgctttcgcagcgagcgcttcgcggagcggatgcaggtggcatagcagacgcggccaccggggttttaccggcggcgcccgccgccgttcacctgtacaaacagacgcatgacttcttcaactttcaaaacgaatcgccgtttggcgcttgctgcatccgcggctgcggccatcgcttttgcagcctcaccttcctgggcccagaacacctggccgaacaagccggtgcgcatcgtcgtgccctttgcggcgggcggcaccaccgacatcctggcgcgcgccattgcgcccgaattgtcgaaggccttcggccagcagttcatcgtcgacaaccgcgccggcgcgggcggcaacgtgggcgccgagatcgtggcgcgcgcgccgaacgacggctacacgctgctgatgggcacggtcggcacgcatggcatcaaccgggcgctctatcccaagctgccgttcgacccgatcaaggacttcgtgccgatcacgctggtggcggccgtgccgaacgtgatggagatgaacgccgacaaggccaaggcacttggcatccgcaacgtgcaggatttcatcaagtacgccaaggccaatccgggcaagctcaacatggcgtcgagcggcagcggcacctcgatccacctggcgggcgagctcttcaagagcatgaccggcaccttcatgacgcacatcccgtacaagggatcaggcccggcgctgctcgacctggtgggcggcaacgccgacctgatgttcgacaacctgccctcgtcgatggcgcagatcaagggtggcaagctcacggccctggccgtgaccagcgcccagcgctcgccggcgctgcccgatctgcccacggtggaagaagccggcggcccggcgctcaagggcttcgacgcgagttcgtggttcggtttgctggcacccgccggcacctcgcccgacatcgtgaaccggatccagcaggaagtggccaagtcgctcggcacgcccgccatcaaggaaaagatgctggcccagggcgcgattccgagcggcaatacgccggccgaattcaccaagctgattgccagcgagcacgtgaagtgggcgaaggtggtgaaggactccggcgcaaaagttgactgacgctcaggtcttccaggtaacgtctttcttgtcggccagggaatccctcagcatgtggagcaggggggctgcgcgctggtgcagtcccacgtgctgcttctcggcctcggcggcgtggccttcgacggcgtagtcgtcgttattgtggggattgccggcctcgcgtgccagcgcggattcgagcgccgcaatggcggcgggaatctgctcgacggtgacgatgcccttgggcgcgatgtccttgccgatgatgtcgaacagctggcgcgcatgcacctcgagcatcacgaagtcaggggaggcgcgggactggaatcggtacagcatgattgttttcactcacttgtagatgtggtcacgggcaaaagggtacaccgattgcgagccgcgcaaaacaccgtgctcgaccctgccgtcgggcttggtggaaagcatctggtgcagtgagatccagccttgctcgaagctcatggcggagcccgccaggtagaggcgataggcgcgcaggatgcgctccgcgttcgcgccctgccggccacccgctcgctgaagcacctcgcgtgcggcgccgagttgcgactccagcgcgtcggaccaggcccacagcgtgcgcgcgtagtgcggtcgcaggctttcggtgtcgaccatctccaggcccgcggcggccgtttcgcgcagcacgtgcgtcacgtgcaggagttcgccgcccgggaagatgtacttctcgatgaaatcgcccatccccgcgcccagctgccggtagtcgagctggcccgaggtgatgccgtggttcagcaccaggccgccgggtttcaggagcgaatggatcttgcggaagtaggtgggcatgttggccgcacccacgtgctcgaacatgccgaccgacgagatcttgtcgaaaggcgcgtcggcggacagctcgcggtagtcgcgcagctccacgcgcacgcgtccctgcaggcctttttcctcgatcaggcgctgcacgtgcgcgtgctggttcttcgacagggtgatgccggtggcgtcgacgccgtagtgctccgccgcccacagcagcaggccgccccagccggagccgatgtccagaaatcgctcgccgggctgcagcaacagcttgcggcagatgtggtccagcttggcttcctgcgcctctgccaggctcagctcgggcgtacgaaagtacgcgcacgaatagacccggcgcgggtcgagccacagcgcgtagaagtcgtcggaaacgtcgtagtggaactggatctgctccgcatccttgttcaatgaatgggagccgcgggacttggccatccgcagcaggcgggtccaccaggtggtgtcggtttgggcggggttgccgggcagcatgccgaccgttgcgtcgatcaggtcgcgcatggcgccctcgatctgcaccttgccttccacgtaggcctctccgatggcgcccacttggtgcgccgccagcttggccagcgccgaccactcgctgaatgccagcgtcacgcgcgaccccggcttggccactcttcggccatcaggcaattccagcgcgatgggcacgggcagcgacgcaagctgcgactcgatcttgggtatcaagctttgcatggtgagcccatagtattgattttttcggttttttgcatgacatcacacgacttgcggggtacccctgtggtatgaccccgttgacaccagattgtttatgcttaaactattcaatcatgaacagcctcaccgccggcctttccgccgcccccgccatggaccttcaacgcatcctgtgcataggcggcggccccgcgggcctctacttcgccctgctcatgaaggcgcgcaacccggcgctcgaaatcaccgtggtggagcgcaaccgccccttcgacaccttcggctggggcgtggtgctgagcgaccagacgctcgccaacctggcggcggccgacgccgagactgcggcgctgatcggccatgagttccaccactgggacgacatccaggtgttcttcaagggccggcaggtgcgctcgggcggccacggcttctgcggcatcggccgcaagcggctcttgaacatcctgcaggagcgctgcctggcgctgggcgtgaatctggtcttcgaaaccgacgccaccgacgaccaggcgatcgccgcccagtacaacgccgacctggtgattgccagcgacggcctcaacagccgtatccgccagcgctacgccgatgtgttcaagcccgacatcgacctgcgcaattgccgcttcgtgtggctcggcacgcaccagaccttcgacgccttcactttcgccttcgaacagaccgagcacggctggttccaggcccacgcctaccagttcgacgacaagacctcgaccttcatcgtcgagacgcccgaggcggtgtggaaggcccacggcctggaccagatggagcagcccgaagccatcgccttctgcgagaagctgtttgccaaatacctgggcggccacccgctcatcagcaacgccacgcacctgcgcggctcggccaactggatccgctttccgcgcgtggtgtgcgagcgctggacgcaccgcatcgacgtggaaggccgctcggtgcccgtggtgctgatgggcgatgcggcgcacacggcgcacttctcgatcggctcgggcaccaagctcgcgctcgaggacgcgatcgacctggcgaacgagttcgagcgcggcggcacggtcgaccacgtgctcgaaggctacgaggcacgccgcagcgtcgaggtgctcaagatccagaacgccgcgcgcaactcgaccgagtggttcgagaacgtgcctcgctacaccggcatgcagatcgagcagttcgcgtactcgctgctcacgcgctcgcagcgcatcagccacgagaacctgcgcgtgcgcgacaccgaatggctgggcggctacgagcgctggctcgccgggggcaagcccgtggcgcccatgctgatgccgttcacagtgcgcggcctcacgctgaagaaccgcatcctggtgtcgccgatggccacctacagcgccgtggacggcgtgccgcaggattttctgctggtgcacctgggcgcgcgcgcgctcggcggcgccgcgatggtgtgcgtcgaaatgaccagcccgacgccggagggccgcatcactcccggctgcacgggtctctacaacgacacgcagcaggcggcgttcaagcgcatcgtcgatttcgtgcacacgcagtcgagcgcgaagatcgccatgcagctcggccacagcggtcccaagggctccacccgcgtgggctgggaaggcaccgacgagccgctggagagcggcaactggccgctgctggccgccagcgcgatcgcctatggcgagcagaaccagctgccggcggcgatgacgcgcgagcagatggacgacatgcgcgaacgcttcgtcgactccacgcgccgggccgccgaatgcggcttcgactggctcgaactgcactgtgcccacggttacctgctgtcggccttcatgagcccgctcaccaacctgcgcaccgacgagtacggcggcggcatcgaggcccgctgccgctatccgctcgaagtgttccacgccatgcgtgcggcgtggcccgaagacaagccgatgagcgtgcggatttccgcacacgactgggcgccgggcggcaacaccgacgccgatgcggtcatcgtcgctcgactcttcaaggatgccggcgcggatttcatcgacgtctcttccggccagaccacgcgcgacgccaagccggtgtacggccgcatgtaccagacgccattctcggaccgcatccgcaacgaggtcggcatctcgaccattgccgtgggcgccatcaccgatgccgaccaggccaacagcatcatcgcggccggccgcgccgacctgtgcgccattgcgcgcccgcacctcgccgaccccgcctggacgctgcacgaagccgccaagctgcaaagccgcgacgtcgactggcccaagcagtacctgagcggacgcgaccagatgtaccgagaaatcgcgaagcagcagcagatggctgcggccgcgaatgccgcgctggcatcgccaaaccccgaggagacacactgacatggacctcgaagcacgcgcccacagcgagcaccccgaggccctgcgcctctggctgcggctcctcacctgcacccaactgatcgagaagcaggtgcgcaacgaactgcgctcgcagttcgcgaccacgctgccgcgcttcgacctgatgtcgcaactcgagcgctcgcccgacgggctgaagatgaacgaactctcgcgccgcatgatggtgacgggcggcaacgtcaccggcatcaccgaccagctcgtgaccgaggggctggtcgagcgcatcaacgtcgagggcgatcgccgtgcctggcgcgtgcggctcaccgcgcgcggacgcaagctcttcaacgacatggcgcagcagcacgaagactggatcgtcgatgccttcgcgggcctcagcgccaaggagatcgcgcagcttcacaagctgctcggcaaggtcaagcaacactcacacagccagatggcggaggccgaatgaagcactacatcggcgcgggcaatcccatgcgcgcgcaattcgaggccaaggcgccttacgtggccaggcacttcgcatggaactacgaggccggtgtcggcaccatcacgctgaaccggcccgagcgcaagaacccgctcaccttcgactcgtacgccgagttgcgcgacctgtttcgcgcgttgaactatgcgaccgatgtgaaggcaatcgtgatcaccggtgcgggaggcaacttctgctcgggcggcgacgtgcacgagatcatcggcccgctcaccacgatgcgcatgcccgagctgctcgagttcacgcgcatgacgggcgacctggtgaaagccatccggcattgcccgcagcccatcgtcggcgcgatcgacggcgtgtgcgccggtgccggcgcgatgatcgcgctggcttgcgatcttcgctatggctctccttcgacgcgcacggcgttcctgttcacccgtgtgggccttgccggcgccgacatgggcgcctgcgcgctgctgccgcgcgtgatcggccagggccgcgcctccgagctgctgttcaccggccgcgcgatgacggcgcaggaaggccaggcctggggcttcttcaatgcgctgcacgagagcgatgcattgctcgaagcggccaccaaggtagcgcgcgagctggccgagggaccgagcttcgcgcatggcatgaccaagaccatgctgtcgcaggaatggtcgatgaccatcgaccaggcgatcgaggccgaagcgcaggcgcaggcgatctgcatgcagaccgaagacttcaagcgcgcctatgaagctttcgctgccaagcgcaagcccgtgttcggtggggactgaagtcatgatgaccaggattcccgcaccgccttcgacagcgcaccttgcactgccgttcttcgacgacgcccaccaggcgctcgcacgcgacctgctgccctggtgcgcagcccaggaggtggacgagcgcgacgaccgcgccgcttgccgcgaatgggtgcgccgcctcggcgacggcggctggctgcgctatgccgtgcccggcagcgcgggcggcgcgctcgatcgcctcgattcgcgcgcgctggtgctgctgcgcgagacgctcggctaccactcgccgctggccgacttcgcgttcgcgatgcaggggctgggcagcggcgcgatcacgctcgcgggcacgcccgatcagcaatcgcactacctcacgtccgtcggcaagggcggcaagatcgcggccttcgcgctcagcgaacccgaggccggttcggacgtggccgccatggccatgcgcgccgaggccacggccgacggttggcgcctccatggcgaaaagacatggatcagcaacggcggtatcgccgacttctattgcgtgttcgcgaagacggagccgacggccggcacgcgcggcatcaccgcgttcatcgtcgatgcgaattcgcccgggctcgatacgtccgagcacatcgacgtgatggcgccccacccgctcgccaccttgcggttcgagaactgcatcgtgccgcgcaccgcgcagctcggcgagctcaatggcggcttcaagctggcgatgcgcacgctcgacatctttcgtgcgtccgtcgccgcggctgcgctcggcatgggccggcgcgcgctcgccgaggcgattgcgcacgcgaagggccggcgcatgttcgggcagacgctggccgacttccagctcacccaggccaagctcggcgagatggcggcgctgatcgacagtgccgccttgctcacctaccgcgccgcctggatgcgcgacgacgccgaacagcgcggcgccccagcggtgggcgatgtttccgctgccgcggccatggccaagatgtgcgccaccgagaacgccagccgcgtgatcgacatggcactgcagatgcacggcggccttggcgtgaaggtcggcacgaagattgaaagcctctaccgcgacatccgctcgctgcgcatctatgaaggcgcgacggaggttcaacaactgatcattggcaaatccgttctgcggggataaacaccgtgtctgcacaagtcgaccgcttcgttcacgaccgcctgccgcctgccgagcagttgccggtctttcgctacgacctgccggagttgcggctgcccgatcagctgaacctggtcgaagagctgctggacaaggcgcccgccaaggggttcggcgacaagccgatgctgcgttcacctgccggcacgctgacgtattcgcaggccgccgttgaagtcaaccgcattgcgcaggtgctgacggaagacctgggcctcgtgcccggcaatcgcgtgctgctgcgcggcggcaattcggtggccatggcgttgtcatggctggccgtggtgaaggccggcttgatcgcggtggccaccatgccgctgctgcgcgccaaggaactgggcgagatcatcgagaaggcccgtcccgtggcggcgctgtgcgatggccggctgctcgacgagctggtgctcgcgcagcgcgaacatccagtgcttgccacggtggtggcgttcaacaagcccgatgcgcccgattcgttgtcggcacgcgcggccggcaagagcggcgtgttcaccgcatgccccacggcgtcggatgacatcgccctgctcgcgttcacttccggcaccacgggcaagcccaaggcaccggtcaccacgcaccgcgacgtgctggcgatgtgcgaaacctggccgcgccacgtgctgaaggcgcaaagcgacgacatcgtgatcggctccccgccgctggccttcaccttcgggctcggcggattgctggtgttcccgatgtgggccggcgcctcggtgtactttgccgatgcaccgttcacgcccgaaggtttggtgaagctcatcaacgaggtcggcgcgacgatctgctacaccgcacccaccttctaccgccagatggcgcccttcgtccgccagcacggcgcgccgagcctgcgcatctgcgtgagcgccggcgaggcgttgcccgacgccacgcggcagctgtggaaggaagccaccggcatcgaaatgctcgacggcatcggcggcaccgaggtgttccacatctatatttccgccgcgggcgaccaggtgcgccgcggcgcggtcggcaaggtggtgcccggcttcaccgcaaaggtggtggacaaccaaggcaacgaagtgccacgcggcacggtcggcaagctcgcactgcaggggccggtgggctgccgctacctcgacgatccgcgccaggccgactacgtgaagaacggctggaactaccccggcgactccttcgtgcaggacgacgatggctacttcttctaccaggcgcgcgccgacgacatgatcatcacggccggctacaacgtgggcgggcccgaggtggaagatgcgctgctcaagcacccggccgtggccgagtgcggcgtgatcggcaagccggatccggaccgcggcatgatcgtgaaggcattctgcgtgctgaagcccggccacgaaggcgatgccgcactcgtcaaggcgctgcaggaccacgtgaaggccaccatcgcaccgttcaaatacccgcgggagatcgaattcgtgacggtgctgccacgcaccgagaccggcaagctccagcgcttcaaactgagacaactcgacaacgacaccacatcatgatgaacaaactcttgcagccaccgggctggttgccccccaagggctatgcgaatggcgtggccgcacgcggcaccatggtgttcgtcggcggccagatcggctggaatgcgcagcagcaattcgaatcggacgacttcatcgaccagtgcggcctggcgctgcgcaacattgccgaggtgcttcgcgcagccggcgccggccccgagcacatggtgcgcatgacctggtacgtgacggaccgcgacgaatacagccgccgactggcggaactcggccccgtgtaccgcgatgccatggggcgcaactttccggccatgacctgcgtgcaggtggcggcgctggtcgagacgcgcgccaaggtcgagatcgaggtcacggccgtcatccctgactgacgcaaacactcgacccataaaaaagccctcttcgcgagggcatttttattcattcgaattcttcgacccaagaaaaaggccctttgaaattcaaagggccttttaaattggttgcgcgagcaagatttgaacttgcgacctttgggttatgagcccaacgagctaccaggctgctccatcgcgcggcaagatggaattataccttattcagcagcgccttgctcggcggcttcttctttaatttcagcacggtcgaccagttcgaccagagccatgggtgcgttgtcgccaacacggaaacccatcttcaggatgcgggtgtagccgcccggacgcgcggcgaaacgcgggccgagttcgccgaagagcttgacgacgctgtcgcggctgcgcaggcggtcgaaggccaggcgcttgttggcaagcgtgggcttcttggcgagcgtgatcatcggttcgatgacgcggcgcagttccttggccttggggaccgtggtcttgatgacttcgtgctcgatgagcgaattcatcatgttctgcagcatcgcaaggcggtgcgagctggtgcggttgagtttgcggagtccgtgtccgtgacgcatggtgctttcctttactttatttaaacaggcagccgtatcaggtactgcccggtgcacgagccctcatgggctctcttcaaaaatcaacgcttgtcgagaccggccggcggccagctttcaagcttcatacccaaggtcaggccgcgcgaggcaagcacttccttgatttcgttgagcgacttgcgacccagattcggggtcttgagcagctcgttctcggtgcgctggatcaggtcaccgatgtagtagatgttttcggccttcaggcagttggccgaacgcacggtgagttcgagctcgtcgacagggcgcagcaggatcgggtcgaattgctgtgcgctgcgcggtgccggcgtatcgaatgcagccagttcgccgccttcgagctgtgcgaacacggccagttgctcgaccaggattttagccgaggcgcgcacggcgtcttcggcggtgatcgcgccgttggtttcgatctcgaccagcagcttgtccaggtcggtgcgctgttcgacgcgggcgctttcgaccgtgtagctcacgcgcttcacgggcgagaacgaagcgtccaggacgatgcggccaatcgacttggtcggctcgtcggcgtagcggcgcatcgtgcccggcacatagccgcggcccttttcgaccttgatctgcatgtcgagcttgccgccttgcgacaggtgcgcgatcacgtggtcggggttgatgatctcgacgtcgtgcggggtctggatgtccgatgccaggaccgggccttcgccgtccttgcgcaggctcagcgtgacttcatcgcggttgtggagcttgaacaccacgcccttgaggttcagcaggatgttgacgacatcttcctgcacgccgtcgatcgacgagtactcatgcagaacgccggcgatcgtgacttcagtggccgaataaccgaccatcgacgacagcagaacgcgacgcagcgcgttgccgagcgtgtggccgtagccgcgctcgaaaggctcgagcgtgaccttggccttgttggcggcaagttgctcgacctgaatggtcttgggtttcagcagggtggtttgcatgcagacttcctctcaatacccccggctcgttacaccggtaaggctggtgaagcacccgtcgagagtgcctcccgatgggaacaaaaaaatcaaattcgggccgcgaagggcggcccgttatcgtctgtttagcgcgagtacagttcgacgatcagcgattcgttgatgtcggctgcgaattcgtcgcgatcgggcaccttcttgaaggtgccttcggccttgtcggcattcacttcgacccaggccgggataccgacttgttgggcgagctggagcgcttcggcaatacgggtctgcttcttcgacttgtcgcgaacggcgatcacgtcgccggtcttcaccaggtacgacgggatgttgaccgactggccattcaccgtgatcgccttgtgcgacacgagctggcgtgcttcggcgcgcgtcgagccgaagcccatgcggtagacgacgttgtccaagcgcgattcgaggatgaacagcaggttggcgcccgtgttgccacggcgacgatcagcttcttcgaagtagcggcggaactgcttctcgagcacgccgtacatgcgcttgaccttctgcttttcgcgcagctgcaggccgtagtcggaggtgcgctgacccgaagtgcggccatgctggccgggcttggaatcgaacttggccttgtcctggatggagcggcgggcgctcttcaggaacaggtcggtgccttcacggcgggagagtttggccttggggccgaggtagcgtgccacgagttttcctttgtgtcatctgccgcagttgcctgcgggagccatcggcgcggacgcggatggcggtgggcttagtaaaaaaacaaatgcgcagccgctcaaaagccggctgcgccttgcggactgacgatcagatgcggcgacgcttctggggacggcagccgttgtgcggaacgggcgtcacgtcggcaatggaattgatccggatgccgagcgcagccagtgcgcgcaccgacgattcgcgaccggggcccgggcccttgatctcgacgtcgaggttcttgataccttgttcgacagcagcacggccggccacttcggaagccacctgcgcagcgaacggcgtcgacttgcgcgagcccttgaagccctggccacccgacgaagcccacgacagggcgttgccctggcgatcggtgatcgtgatgatggtgttgttgaacgaggcatgcacgtgggcgataccgtccgcaacgttcttgcgaaccttcttgcgaacgcgctgtgcggcgttgtttgcaggtgctttagccatgctggtctatccttatttcttcagggactgcgcagccttgcgcggacccttgcgggtgcgggcattggtgcgcgtgcgctggccgcgcatcggcaggccgcgacggtgacggaagccgcgatagcagccgatgtccatcaaacgcttgatgttcatcgtcgtctcgcgacgcagatcgccttcgatggtgaagagagcgatctggtcgcggatcttttcgagatcggcgtcggtcagatccttgatcttcttcgaatattcgatgccgctcgcttcgcagatttgacgggcgcgggtgcgaccgatgccgaagatggcggtcaggccgatttcagcgtgcttgtgcggcggaatgttgatgccagcaatacgtgccatgtgcgtcctctaatactcttcaatcaaccctggcgctgcttgtggcgcgggtcggtgcaaatcacacgcaccacacctttacggcggatgaccttgcaattacggcagatggttttgaccgaagccgaaactctcatttcattctcctaaaactgtttaacgtggcggtacaccgcccacacccaaattctcaatactgaaactcacagccctacgatgtcttgaagttggccttcttcagcagcgattcgtactgctgggacatcatgtagttttgcacctgggccatgaagtccatcgtgacgaccacgatgatcagcagggaggtaccaccgaagtagaacggcacgttgtacttcaggatcaggaactcgggcagcaggcagacgaaggtgatgtacaccgcgccggccaacgtcaggcgaaccagaatcttgtcgatatagcgagcggtctggtcacccggacggatacccggaatgaatgcaccgctcttcttcaggttgtcggccgtttccttgctgttgaacacgagtgccgtgtagaagaagcagaagaaaacgatcgcggcagcgtacagcagcacgtagatcggctcgcccggacgcagtgcgccggcaatgtccttgatccaccggaaaccaccttcgccggcgctgaaccagccgaccaccgttgccggcagcaggatgatcgacgaggcgaagatcggcggaatcacaccggccatgttcagcttcaagggcaggtgcgacgactggccgccatagaccttgttgccgacctggcgccgcgcatagttcacgaggatcttgcgctggccgcgttcgacgaacaccacgaagtaggtgaccagcaccacgaccgcgatgatgaagagcgcaatgatcggattcattgcaccggtggtcaccagcgaagcgaggccgccgatggcgctcggcagaccggcggcgatacctgcaaagatcaggatcgagatgccgttgcccaggccgcgttcggtgatctgctcgccgagccacatcaggaacatcgaacctgccgtgaggctcaccatcgcggtcaggcggaagccgaaaccgggggcgatgacgaggccagccgacgattcgagggccactgcgatgctgaacgactggaacagggccaggccgagtgcgccgtagcgtgtgtactgcgtgatcttgcggcggccggcctcgccttccttcttcaattgctcgaaggtcggaagcacgtaggtcatcagctgcatgatgatcgacgccgagatgtacggcatgatccccaacgcgaacacggtgaagcgcgacagcgccccgcccgagaacatgttgaacaggctcaggatgccgccctgctggccctggaacaacgcagccagctggtccgggttgatgcccggcacaggaatgtgcgcgccgatccggtagaccacgagcgcgagcagcaaaaagacgagccgacgacggaggtcgccgaacttgcctgtttttgcgatcgttgccgcgttagttgccacgaagaacttctttcagtccagtgtgatcaggcgatgctgccgccggctgcttcgatggcagccttggcaccagcggttgcgcccacgcccgtcagcttgacggccttggtgagttcaccggtcttgatgaccttgaccaccttggcgagctggcccacgaggccggcttgcttgagtgccaggacatcgacttcggccaggccgagctgctcgagggcagtcagcgtgacttcggcgttgaacttcagcaggtgcgacttgaagccacgcttcggcaggcgacgctgcagcggcatttgaccgccttcgaagccgaccttgtggaaaccgcctgcgcgcgacttctgacccttgtgaccgcgacctgcggtcttgccgataccggagccgataccgcggccgacgcggcgcttggcgtgcttggcgccatccgccggcttgatgccattgagttccatatcagtctctcttacagaactttgaccagataactgatcttgttgatcatgccgcgcaccgccggggtgtcttgcagctcgctcacgctgttgagcttgcgcaggccgaggccacgcacggtcgcgcgatgcgattccttggtgccaatcgggctcttgaccaattgcaccttgagggtttgttgttgcgtcgtcatttgaatgcttccttcagccttgcgagagcttgcgctcaggcgaagatttcttcgacggtcaggccgcgcttggcagccacttcggacgcggtcgtcgagttcttcaacccgtcgagcgtggcgcgaaccatgttgtaggggttcgacgaaccatggctcttggccacgatgtcggtgatgcccatgacttcgaacacggcgcgcatcgggccgccggcgatgatgccggtacccttcggggcggggatcatgacgaccgaggcggcgccatggtgacccgtcacgcggtgatgcagcgtgccgttcttgatcgagatcttggccaggttgcggcgggcttcttccatcgccttttgcacggcagcaggcacttccttcgacttgcccttgcccatgccgacgcggccttcgccgtcgcccacgacggtcagtgctgcgaaaccgaggatacgaccacccttcaccaccttggtgacgcggttgatcgcgatcatcttctcgcgcaaaccgtcttcagggccttcgttctgcgttcttgcttgaatctttgccattttgaatctcgtgtccggttagaactgcagaccggcttcgcgagccgcatcggccagcgccttgacgcggccgtggtacgcaaaacctgcgcggtcgaaggcgaccttctcgacgccggcagccttcgccttttcagcgatgcgcttgccgatggccgttgcagcggcggcattgccgcccttgcccgagccgccgagtgcggtgcgcacttcggcttcggccgtcgatgcggtggcaatcaccttggtgccgtcgtcggagatgacggtggcgtagatgtgcaggttggtgcggttcaccgtcagacgggccacgccctgcgtcgcgatgcggatgcgggtctggcgcgagcggcgaagacgctgtgcttttttggtcaacatcattttgctgccccttacttcttcttggtctctttgatcacgatcttctcgtccgaataacggatgcccttgcccttgtaaggctcaggcggacgaacagcgcggatctcagcggcgatttgaccaacgcgctgacggtcagcacccttgatcacgatttcggtcggggtcgcggtggccaccgtgatgccttgcggcatttcgatgttgaccgggtgcgagtaaccgacttgcaggttcaacttgttgttggaggctgcagccttgtagccgacgccgaccaggttgagcttcttctcgaagcccttggtcacgccaaccaccatgttgttcaccagctgacggatcgtgccgctcatcgcgttcgcttcacgcgactcgttggcgggctcgaagttcagcttgccgtcattgctgacgaccttgaccagggcattgcgtgcaaggttgagcgtgccgcccgtacccttgacgctgatctggtcttccttgatcgacacatccacgcctgcggggatggtgatcggcatttttcctactcgggacatttcagttactcctcgatgtctcggttaggcgacgtagcacagcacttcgccaccgacaccggtagcgcgtgccttgcggtccgtcatcacgcccttgggggtcgtgacgatcgcaacgccgaggccgttctggacttgcggaatggaagcactggccttgtagacgcgcaggccgggacggctcacgcgctcgatgcgctcgatgaccggacggccagcgtagtacttcagggtaatgacgagttcggtcttgccgtcttcggtcttgacctggaaaccgtcgatatagccctcgtccttcaggacctgcgagatcgcgatcttcaccttggaagacgggaccgacacagtgggcttcgccaccatctgcgcgttacggatacgcgtcagcaggtcggcaatgggatcactcatgctcatgttgtttgctcctgcctggcttaccagctggccttggtgacaccggggatgtcgccattgaaagccagttcgcggatcttggcgcgggccagaccgaattgacggaaggtgccacgggggcgaccggtgatttcgcagcggttgcgctgacgcgtggggttcgcgttgcgcgggagcttttgcaggcccaggcgggcagcagcgcgctcttcgtcgctcttcttcacgtcgttggaaattgccttcagttccgcgtgcttcgcagcgtacttggcgaccagcttgtcgcgcttgagttcgcgctggatcaaagatgctttagccacagatcacctcagttcttgaacgggaaacggaaaccagcgagaagcgccttggcttcttcgtcggtcttggccgtcgtcgtgatgctgatattgagaccgcgcagggcatcgaccttgtcgtattcgatctcagggaaaatgatctgttccttgacgccgatgttgtagttgccacggccgtcgaacgcacggccggagatgccgcggaagtcgcgaacacgcggcagcgcgatggtcacgaaacggtccaggaactcatacatctgcacgccacgcagcgtgaccatgcagccgatgggctggttttcgcggatcttgaaaccggcgatggccttcttcgacttggtgaccacgggcttctggccggcgatcttggtcaggtcggcgacagcgttgtcgagaaccttcttgtcggcgacagcttcacccacacccatgttgagcgtgatcttggtgaggcgggggacctgcatcggcgacttgtagccgaacttttccgtcaggtctttcgcgatcttttcgcgatagtgttgttggagacgtgccatgtgagtacctcttaggcgaacttgatttcgtcgccgctggacttgaagacgcgaacagccacgcgcttgccgtcagcaccctgggtgatcttgatgcccacgcgatcggccttgccggtcgcggcattgaagatcgccacgttggattggtggatgggcatggtcttttcgacgatgccgccggtcgtacccttgagggggttcggcttggcgtgcttcttgacgatgttcacgccctcgacgacgaggtgcgaatcgtccttgcgaagcgagacggtgccgcgcttgcctttgtcgcgcccggccaacacgatgacctggtcgcctttgcgaatcttgttcatggcgttgttgtccttaaagaacttcgggggccagcgacacgatcttcatgaacttttcggtgcgcagctcgcgcgtcaccggtccgaagatgcgggtgccgataggctccagcttggcgttgagcaacacggctgcgttgccatcgaatttaacgagggagccgtcggcgcgacggatgcccttggcggtgcggaccaccactgcgctgtagatctcgccctttttgacgcgaccacgcggagcggcttccttgatgctcaccttgatgacgtcgcccacgctggcgtaacgccgcttggagccaccgagcaccttgatacacaggacggacttcgcgcctgtgttgtcggccacttcgagccgggattcagtttggatcattgctagtagttcccaacttgtaccgatgcgtctccgggagggaaacgctgcggtcagtcttgggcccgtcgtctgcacctcgaaccactcgaggcacttccgctttgggctgaaagcttcgccttttttgaagcgaagcctgcgattgttgcacggtgaccagggcatgtcaactgccttctgacgcgaaatgcactggaactagacttggcggcgtgcgtaccgtcaattcaggccccgtagtagctcccgcgtctcccctgcgccgcaggctgctggccagcacggccgccgctgcggcggggctggcggggctcggaggactggccggctgcggcagccctgtaatcccgccgcctgccgcagcgtcacggttgcgccgcgtggccgaggcgtactggccgcaccggctgaatattatacaaggcacaacggcgggtggcctctccggcatcgactacgacacggaaagaagtgagtacatccttctcagtgatgaccggtcagacctgaaccccgcccgtttttataccgctcaatgggcaccgccgtggctgcagccacccgcgccgaagagcgtcgtggaattgcaacgccccggcggcggcccctggctcgcgcgccgacgggtcgaagcccggatgcccgtacccgaccccgaggcgctgcgcctgcggcccggcgccggcaccctgctttggaccagcgaaggcgatgtgacacgggggttcggaccggctttctacgaatcggcgcgcgatggccggctgctgcgcgagtttcccctgccggccatgttcaatgccgatgcctcgcagcgccgtggcctgcgcgacaacctgggcctggaaggcctggcgctgacgcccgacggccgccacgcctggcttgcaatggaaagcgcgctggtccaggacggcccgattcccaccaccaaggcgccgggcgggccctgccggctgacccggatggacctggaaaccggccaggccacgcgccagatcgcctatgttcccgacgcgatcccgctgcggccgctgattcccggcagccatgccgacaatggcatcaccgaggtcctgatgctcgatgccgaccgcatgctggtgctggaacgcgcctatgccacgggcgccggaaactcgctgcgcctgtacgagatcgacacccgtgacgccaccgacgtgctggcgaccgacacgctcgccgcgggcaaccatcgtcccgcggcaaagacgctggtcgccgactttgcccagctcggcctttcgcgcctcgacaacaccgaaggcatatgctgggggccggcgctgccggacggcaagcgcatgctggtggtggtgagcgacgacaatttcaacccgctgcagacaacccagttcgcggcattcgaatacaccgaccgaccatgaccattgccgtcacattcctgccccgcaccggcccggcgccgcttccccccattgccttcatcggcggcggcaacatggccagcgccatcatcggcggcctcatcaagcagggcacgcccgccgacgccttcgaggtggtcgaacctttcgaggaggctcgccggaagctggcgcagtccttcggcatcatcgcgcgcgccgaggccggcgaagccctttcgcgctgcgcggtggtggtgtgggcggtcaagccgcagacttttgcggacgccgccctgccggtgcgcccgttcgccgaaaacgcgctgcacctgagcgtggcggcaggcattccgtcgggcagcattgcgcgctggctcggcgccgaacgcgtggtgcgcgccatgcccaacacgcccgcgctggtcggccagggcatgacgggcctctatgcacgcgccggggtggacgccgccgaccgcgccctggtcgggcagctgctggcaccgaccggcgaactgctctgggtcgacgacgaagccgcgctcgacgcggtcacggccatgtccggctcgggcccggcctacgtgttctatttcatcgaggccatgaccgaagccggcatcgaaatgggcctgccgcccgaccaggcccagcggctggccatcggcaccttcaccggggcctcggcactggcgcacagcgccaccgagccaccgtcggtgctgcgcgaacgcgtgacctcgaagggtggaacgacccatgcggcgctcagctcgctcgagggggccgacgtcaaggcgaagttcaagaccgcgattcgcgcggcgcagaaacgcgcggccgaactgggcgaggaattcggcaaggcctgagagccccgctcatcgccccatctacttcagcgcatagccggccgcgacgccggcgaacaccgtgaagccgagccagtggttcaggcggaaggccttgaagcagccgtcgcgggtgcgaccgcgaatcagctgccagtgccagacggcctgcgccacggcgatgccgatggctgcgaaaaacacggccccgaggccgcggccggcccaggcccagaccgccagaaatacgccgtagctcgccatcacggccgccacgtcgaattggccgaaggtgatggccgaggtcttcatgccgatcttgaggtcgtcgtcacggtcgaccattgcgtattcggtgtcgtaggccagcacccagaacaggttgccggccagcagccaggcagcgaacaccggaaccgtggattgcaccgccgcaaaagccatcgggatgccgaagctgaaggcgatgccgagcaccgcctggggaaccgacacgaagcgcttggcgaacggatagaccagcgtgatggccagcgccgcgaacgaccaaagaatggtgagccgattggtcgtgagcaccagagcgaaggccgcgagcgccagcaccgcaccgagcagcagcgcttccctgaccgaaaccgcgccgctcgtcaccggccgctccgcggtccgcttcacgtggcggtcgaagtcgcggtcggccacgtcgttgacgcagcagcccgcgctgcgcatgaggatggtgcccagcacgaacaccgtcagcagatgccagcccggccagccctcggccgcaaaccagagcgcccccagcgtgggccagagcagcagcagccagcccgcggggcggttccagcgaatcaggtcgagatagagcgcaaaacggcgggcaagcatgcggcaggcaaaaaaagagcggccattgtgccgctctcggtgccggggctcggaggccccgggcgctttttcagtcttcgagcagcgaacgcagcatccatgcggtctggtcgtgcaccgtgcagcgcgcggtcagcatgtcggccgtcgggtcgtcaccggcctcctcggccacgggaatgaattcgcgcgcgatgcgcgacacggtctcgtggcccttgaccaggatgcgcaccatctccatcgccttgggcggggtctgcggcacgtccggcacggtggcgatcttgctgaactcggcgtaagagcccggcgcgtagtggcccagcgcgcgaatgcgctccgcgagcacgtcggtagcgccccagagttcggtgtactggcccatgaacatcgcatgcagcgagttgaagtgcggccccgtcacgttccagtgaaagttgtgggtcgtgaggtagagcgtgtaggtgtcggccagcacgcggctcaggccttcggcaatggcggcgcggtcctggcgctcgatgccgatgttgatgatgggcgcgttgcggctgccggactcctgcgccaccagagcgccgcccttcttgggcaccttgcccgacgacgttttcttcaatgcttttgccatggcgtgaaactctttcttcaactattgacggacaccttgattctgaaagccgacccgcggcttcgcaacagcgtcactctatcccggcgatgaacgaaatcgaacggtcgccgcgtaggccgagttcgcaattcttctatgacagccgcttgacgcccggcagctcgcacgcatagatagcgttgcgcaacgcggcaatcgcttcatagcgcgtgaaggtgcggcgccaggccagcaccacgcgccgcgtgggcggatcgcggtcctgcgcgtcgcgcaccggcaggtaacgcaccatctgctcgggctccttgcgccccttcaccttgagcttgagcgcttcggcaggcaccgacaggcgcggcaccagcgtcacgcccatgcccgaggccaccatgtgcttgatggtttcgagcgacgagccctcgaagctcttgcgaatgccctcggcattgctcgagaagcgcgcgaactcgggacacacctccagcacatggtcgcgaaagcaatggccggtgccgagcaacagcatggtttcgttctgcagctcttctgaagtgatggattcgcggtccgcgaacttgtgcttggtgggcagcgccgccatgaagggctcgtcgtagagcggcgccatcgccaggcccgtgtcgggaaaaggctcggccatgatcgcgcagtcgatctcgccggcacgcagcatctcgagcagcttggcggtgaaattttcttgcagcaccagcggcatctgcggcgtgcgcgcaatcacctggcgcacgaggtcgggcagcaggtacgggccgatggtgtagatcacgccaaggttcagcgggccggccaacgggtccttcccgcgcttggcaatttccttgatgctggcggcctggtcgagcacgctctgcgcctgctgcacgatctgctcgccgagcggcgtgacggtcacttcgccggcgctgcgctcgaagagcttgacctcgagctcgtcctcgagcttcttgatggccacggagagagtcggttgggagacgtagcaggcctcggccgccttgccgaagtgccgttcgcgggcgactgcgacgatgtatttgagttcggtgagagtcatagcttgcgtcaattatgcgcaagcctccgtgaccgggcattgtctggggtcggcctacgccttcaggtactcggccttggtgccgagccagcgatcgatgtggcgctgggccaggtcggggtgcttctcgagcatgcgcggcgccagctcgcgcgcccagtcgagcagcatcacgtcggtggccaggtcggcaaagcgcagcagcggcgcgcccgactggcgtgcgcccaaaaattcgcccggcccacggatctcgaggtcgcgccgcgcaatctcgaagccgtcgctggtttcggccatggccttgagccgcgcgcgtgcggcttcgcccacgcggccgctgtcgccgggcgcatagagcagcacgcaggccgaggccgcggcaccgcgccccacgcggccgcgcagctggtgcagttgcgagaggccgaagcgctcggcatgctcgatcaccatcagcgaggcgttgggcacgtccacgcccacctcgatcacggtggtgctcaccagcacctggatttcgttggcggtgaaggccgccatcaccgcctgcttctcggccgtgggcatgcgcgagtgcagcagcccgacgttgaccgccgagcccaatgaacccgcgagctcgtcgcgcgtttcggtggcgttgcgcagatcgacggcctcgctctcctcgatgagcggacagacccagtagacctgccgcccctgcccgagctgtgcctggatgcgcgcgatcacctcgtcgcgccggtggtcggccaccagcttggtgacgatgggcgtgcggcccggcggcagctcgtcgagcgtggaaacatccaggtcggcgtagtagctcatcgccagcgtgcgcgggatcggcgtggcgctcatcatcaacaggtgcggctcgagatggcccacggccttgccgcgcagcgccagccgctgcgccacgccgaagcggtgctgctcgtcgatgatggcgagcgccaggttcttgaagcgcaccttttcagaaatgacggcgtgggtgccgatgaccagcgcggcctcgccgctctcgaccgcggccgacatcgcgtcgcgctccttcttcttctggctccccgtgagccaggccacccgcaggccgcgctcggccagcagcggatcgagccagccgaccagcttgccgaagtgctgggccgcaagaatctcggtgggcgccatcaacgcgcactgaaagcccgcgtcgatgcagcgcgccgccgcgagcgccgccaccacggtcttgcccgagcccacgtcgccctgcagcaggcggtgcatcggaatctcgcggcccaggtcgcgcgtgatctcttcacccacgcgctgctgcgcgcccgtgaggccgaagggcagcaccgcgagcaactgcgcatgcagcgaggccggccggggctcgggcgaagcgggcagcatcggcgcgcgctgcgccgcacgctccagccgcgcctgcagctgcgacagctgctgcgccagcagctcctccgccttgatgcgctgccacgccggatggctgtggtcttcgagcgtcgccatcgccacgtcgggcgtggggtagtgcagaaaggtcaacgcactgcgcaggtcccatgcgccgcgcagtccgatctgcacgggaatcgtctcgtcgagcaccgcgcgcgccagccccgagcgcacctcgcgccggagcaccggctgcggcaggccggccacggtggagtacacgggcgtcagcgcttcgggcagcgcagtaccggccgccttgaccgtcggatgcatcatctgccgcccgacgaaaccgccacgcacctcgccgcgcacgcgcacccgcgcgccgaccgcgagctgcttttgctgcgagggatagaaattgaagaagcgcagctggcaggtgtcgctgccgtcgtcgatggtggcgagcaactggcggcgcggtcggtacaccacctcgcactcggtcaccacgccctcgacctgcgccatgtcgccgtcgcgcgtgtcggccagccgcacgatgcgcgtctcgtcctcgtagcgcatcggaaggtagagcgcaaagtcgatgtcgcgcacgagcccgagcttgcgcagcgcgcgctgcacgaggctcagcccggcgccgggcgcggctggggcgacggtgggcgggtttgcggtcttttgggggcgcactgacttcgcggaagcgggcatgggacaattctgcccggctccagccttgttcttcttcctttccatgcctccttggcacgggcccgtccggccctcaagcaccatgcgcgccttcacgctctccgatttcgatttcgccctgccgcccgaactggtggcgcaacacccggcccccgaacgcacgtcctcccgcctcctcgacggcacaggcagcgccccggtcgaccgcatcttcaagaacctgccttcgctgttgcgcgcaggcgacctgctggtcttcaacgacacgcgcgtcgtcaaggcgcgtctcttcggcgagaagccgaccggcggcaagctcgaactgctggtcgagcgcgtgctgcagggtcatgaagtggtggcccacatgaaggtcagcaagaagccgccggtgggcaccacgctgcagatggtgggcggcttccgcgcgacgctcctggggcgttggcccgaggaagacggcgcgctgttccgcttcggcttcgagagcgacgcgggcgaagacccctacgcgctgatggcccgctgcggccacgtgccgctgccgccctacatcacccacaccgattcggccgacgacgagtgccgctaccagactgtgttcgcgcgcgtgcccggcgccgtggccgcaccgacggccgcattgcatttcgacgaagcgctgctggacgaactcgaaacccgcggcgtgcagcgcgccaacgtcaccttgcatgtgggcgccggcaccttccagccggtgaagaccgagaacatcgcagaacacacgatgcacgccgagcgctacgaagtgcccgcggccacgcagcgcgcgatcgccgagtgcaaggcacgcggcggccgcgtcgtcgcggtcggcaccaccaccgtgcgcacgctcgaatcgtgggccaagagcggcgaggccacgggcgacacgcgcatcttcatcacgccgggctttgcgttcgagcacgtcgacctgctggtgaccaactttcatttgccgaagagcacgctgatgatgctggtctcggccttcgcgggctacgagcgcgtgatgtcgctgtacgcccacgccattgcccaccgataccgcttcttcagctacggcgacgccatgctgctggcacgacaacgacaagattgaagacaacgaccatgctgaacttcgaactcctcaaagccgacaccgacagccacgcgcgccgcggcacgctcacgctcaaccacggcgtggtgcagacgccgatcttcatgcccgtgggcacctacggcaccgtcaagggcgtgatgccgcgcagcctggaagagatgggcgcgcagatcatcctgggcaacacctttcacctctggatgcgccccggcctggacgtgatggcgagctttggcgggctgcaccagttcgagaaatggaacaagccgatcctcaccgactcgggcggcttccaggtctggtcgctgggcgccatgcgcaagatcagcgaggaaggcgtgaagttcgcctcgcccgtcaacggcgacaagctgtttctcacgcccgaggtctcgatgcagatccagaccatcctgaacagcgacatcgtgatgcagttcgacgagtgcacgccctacgacaccaagggccacatcaccaccgaggccgaggcgcgcatctcgatggagctgagcctgcgctgggccaagcgctgccagcacgaattcgcgcggctcgagaacccgaacgcgctgttcggcatcgtgcagggcggcatgttcgagaacctgcgcgaggagtcgctcgccgcactggtggagatggactttccgggctacgccatcggtggcgtgagcgtgggcgagcccaaggaagagatgctgcacatcatgggccacacgccgcaccggctgccggcccacaagccgcgctacctgatgggtgtgggcacgcccgaagacctggtgcagggcgtggccgacggcgtcgacatgttcgactgcgtgatgcccacgcgcaatgcgcgcaacggcacgctgttcacgcgcttcggcgacctgaagatgcgcaacgcgcgccacaagaacgatccgcagcccatcgacccgagctgcacctgccacgcctgcgcgggcacctcgggcgtctcgtggaacgacggtgggcgcgaaggcttcagccgtgcctacttgcaccacctggaccgctgcgccgagatgctgggcccgatgctcaccaccatccacaacctgcactactacctgaatctcatgcgcgaaatccgcgaagccctcgaggcggacagcttcacggcattcagggcccgcttcaaggccgaccgcgcgcgcggcgtgtagccgccgcgcatcggcgcaccgtttccgtttacttcgcggctgccggcgccttgaccgccagcggcgtggtgtaaggctcgatgcgcagcagctcgttcttgaagaccgccacctgccgcagcggggcctgcaccaaggcgccgccggcgtccttctgcgatgcgtattgccagagcgtgagatgccccttggctgccagcaattcggccaggcgctgcacggcggggcccgagcccgtgccgagttgcgcggcctccacgccgacgacgatctcgtcgcgtggcgaaaccagtttgaagagttgaacggacgcgggcgtttgtgcccggacgggctgcacggcagcggccagcggaagaatcgccagggcggcgaggccggtcattgcacggcgacggtaaagggtgttcatgggccgcaagcgtagccacgcaagtgcccgttgcccacatgccggaagccatacgccacgtacgccagaggtatgcaggagtacaccgggtgcgcgccgattcgttcatccgctacgctcaacggcatgaccaccgcttcctcctcaccacccactgcctacaccgccagctatccctcgctggccggccgcaccgtgttcatttcaggcggtgccaccggcatcggcgaagggctggtgcgggcgttccacgcccagggcgcgaaggtcggcttctgcgatctcgacgctgccgcgggccaagcgctcgcgtccagattgcaaggcagcaacccggcgctgttttgcgagtgcgacgtgaccgacacccccgcgctcatcgccgccattgccgcggttcgcgcgcagttcggtcccatcggcgtgctgctgaacaacgcggccaacgaccggcgccacgacatggccgacgtgaccagcgaagacttcgatcgcctggtggcggtcaacttcaagcaccagttcttcgccgcgcaggccgtggcggacgacatgcgcgcgctgcgcggcggatcgatcatcaacttcggctcgatcagctggatgatcaagggccggggctacccggtctaccaggcctgcaaggccgccgcgcgcggcctcacgcgttcgctggcgcgcgacctgggcaaagagaacatccgcgtcaattcgatcgtgccgggctgggtcatgaccgagcggcagatcaagctgtgggtcaagccggagtcgggcgccgagatcgatgcggcccagtgcctgccgggccgcgtgatggccgaggacattgccgccatggcgctcttccttgccgccgacgattcgaagatgtgcaccgcgcaagacttcgtggtggatgccggctggacctgagcctctcgcgccctctccccaaaagcaagaagcccggcatgccgggcttcttgcgtcgaggggggcggacgatcaatcgcgcagttcggccggaaccttgccgccgttggccgccagcttggtcatgacctggcgatgcagccagatgttcatcttggcgctgtcgctcgtatccgcgccgtagctgagttcggcggccagctgcttgcgcgcgtcgaggctgctgtccagcccgagcagcttcatcaggtcgacgatggaggtgcgccagttcaggctgctcgcgccgggcatgccgtcgagcagggcctcgacgtccaccaccgtgatggcgggcggcggtgccgccgcggccggagcgcccgcgggggcgggttccggagcagccgcaggtgcgttggcggcgtttgcggacgggaagatcttggaaagaatgctgccgaaaatgctcatgcgtgtgctccatcaatgttgaaaactgaaaacccgcggccacgtcggtgtcgcagccggacgttgtagcacggtggtgcggcgcttccgctacacggcgggctgagccggtgcgccgggtgtgaacgaatccacagaccctgcagccgatgcgagcggcacccgcggcgcagcggaggtgccgcaggcatggcagaacttcgagaacgcgcccttgcgggtttcacactggccgcaatggtcgaacaggccgatgccgcaatgcgggcagaagtcgatctcgttgttcttcaggtccactggccgctcgcagccggggcaaacgttcttgccgagccgcgtgagcgcggtgtcgtagctgagctcttcgcgccgcacctggtcgggctgctgctcggccagcttctggcgcgcaaggtagcggttcagcgcgacgatggcgtagcgtcccacgagcactgtgaccaggatgcccaccacgtagcgcacgtagccgccgtaactcggcatgtagggcaccagctcgacgaagaaagcgaacagcgcaaagaagatgaagccccagacaaagggccagtaggtgcccttgcgcttcttcacgaacaaccagcccgccaccgccagcaggggcagcgtgagcgcaagcctgtagccgaacacgcgcagttcgacgcggcggtactcggcgtccagcttgtcctgagcggtgcgctccagcaccgccagcgattcgcgggcgcgctgctcgccctgccgcgcatcgatcacgatctgatgctgcgcgtccaccttgcgctgcacggcgtcttccttgttcttgagcgcgtcgagcgccttggtgcgcgcgatgagctccgggtcctggtcgggctgcgcggtggcgcgtcgggtggcaatccagttgccgaaggtctcgcgtgcgttggcgctcgcctggtgcgcggcactgagctgcaggctgatctgctcgagctcccgcgacgcggccagttcggtcttttccgccgccttgatcgtctcgcgcagcggcgcggccgcggcacggtcgatgaagtcgtcgagttcgagcgctcgctcgacccgcggcagatcgccaacgacggtgccgccgagcccgatcaggaagcttgcgaacaccaaggccaccagccacaggccgcggcgaaaccacttttcggacagacgcaatgacttgctcatttcttttctttctcgttttccttgcgaagcgcgaacgccccgttgcaacctacagcttgaacgccaccggcgccgcacccagtcccgcgcgcggcagccatgcgaacaccgaatcgaccgtgaccgtttcgatgcggtccgaaaaccgcttgtcgttcgggtgatcgtcgaacgccacgttggccgagcctactcggccgcccaggcgcgtgagtgggccgagccgcagtgtcgtcggttcgtagcccttgaactgcatccacgcctgcgcctgcccgcgattggcgatggtggcgggctccatggctgcggccagcgtctcgacggcccactggttcgactgctggtatttctggccccagacgtagctcacgatgctgtagggcgcaatgttcagccgcacgatgcgcgacggcgattcgtgcaacgcggccagcagctgcgtttgcacctgcggcgtgggcaccgcccaggccgcttcgtagcgccacagatcgtcgaggaaaaactcgccgagcccctgccggtacaccgcggcctcggacgtgccgcactggttgagcttgtgcaccacgcgccacggaccctgttcggtcttgtaggcgatgccaaggtgcgaatagcgcaggccgtacttgccgaggtcctgcccggcccgcgccagcagcacgacccgggcgccgctcgcatccagctgctgcgacgtgcgctcggccagctgcatgcccttgacgatcagctcggcagtcggcttggcctgttcgcaggagcggccggcctgtgcctgcagcggcatggcgatcgcgagcgcaagcagcagcgatgaaacaagcgcgcgcttcatgacagcctctcgttgtgcagcagcgcgcggccgatggcgttgggcacgaaggccagcacctcgcccgcggccgacagcaccacgccgctgccgatcacgctgaccagcacgcccgtgccgaccgccgcggacacgccgttggcggcgcgcgccatcaccttgacgctggcgcgggcgccgtccgaagcccgttccagcaggtagacggtgccatcggccgaagcctcgaccgcaatcaccgtcagcatcgagccgcccaccgacagcgcagcaggcaccgcgaccaccgccgtggccgaagcgcccacggctgaagcggcacccacgaccgacgccacggggagcagcgagagtgcggccgaagcctcggaaccccgggcttgggcctgggcatgaagagggagcgtggcgcctgcgaatgcggtgcaagcggcgatcagaagagaagcaatcgacttattcatgacggtctttcgttggttgatgtgcgggtcgagatgaagcaaggagaagcagaagcggcactcattcggccgaggccgaagaagcagcgctttcctggcgggcggcgcggcggccttgcaggcgcgcttcgaccaggtcggcttcgtggcggtcgcgcagcgtcttggccagcgtgaaggccgagctgatcaggaacagccagctcacgcccaggaaggccttgtaggcgtcgttgatctccatgcggacgaggccccagccggtcaggcccatggcggtgaagaagctgccccagaccaccaggcgccacatcggcacgtcgcggcctgcggcgccgccggcgtccgcgtgctggttgtctcgaatgaacttggccagcatgaaggcggtgctgaggcagaacacgtagcccatcaccatgaacgcacggtccagcgcctcgcccggcagccagctcaagccggtggcgcacaggaacacggcaatcgcgaaagaagcccagacctgcagctgccaggcccgcgtgtcgcgctggatcgaaacggtggtggaagggaagggttgcatgaaagcctcgcggcgtagtgaaggtgagcgaatgatggttcgctcccgcaccgcgaggatcaaatgcttcaaccagttctggtttgagccgctgcaggtatcttggaaagatacttttttgatgccgggcgtgccggcaaggccgggcctaggtggccagcaagccactcacgcgctgctgcagcgtctcgggccgcacgtcggctggcggcaccgcgtggccgacatggagccccacgcggctgtagaagccgcggcggaagggcttggccatggccacgttctggccgccgcgcagctcgatgcggctgaagtaggagccccagaggttggtcagcgccatcggaacgaccggcggctcgatgccctcggcgcgcgcggcttcgatgatcttcatcacgccgcccttgaagggttgcagcgtgccgtcgcgcgtgatggcgccttcgggaaagatcgccagcaggtcgccttcgcgcagcacctgcagcgccctggcaaaggcggcttcgtaggcggcggggtcttccttctgcggcgcgatgggaatggccttggccagcttgaacagccacccgagcaccggcaccttgaagatccggtggtccatgatgaagcggatcgggcgcgggctcgccgccatcagcaggatcgcgtcgatgaagctcacgtggttgcacaccagcaccgccgcgccttcggtcggaatgtgctggtcgcccttgatctcgaagcggtagacgaagtgcgacagcagccacgcgatgaagcgcagcagatactccggcaccagcatgaagatgtagaacgccaccagcgcgttggcgatgccggtgaaaaggaagatctgcggaatcgtgaagccggcgccgagcagcgcgcccgcgatgaccgagctgccgatcatgaacagcgcattgaggatgttgttggccgcgatgatgcgcgcgcggtgcgtgggctggctgcgcagctggatcagcgcgtacatcggcacgctgtacaggcccgcgaagagcgacagcagcgccaggtcggccatcacgcgccagtgcgcggcctggctcacgaaggtgccgagccccatgaccgccgaggcggcaagagcacccgccgccgcgggtgcgggcggcagaccgcgcgacgcaaagtaaaggtcgatggcaaacacgctcatgccgatggcgcccagcggcacgaggccgatttccacctgccggcggctcagcgtctcgcacagcagcgagccgatgccgatgcccacggagaacaccaccagcagcagcgaagcgacctgctcgtcgccatgcagcacttctttcgcgaagctggggaactggctcaggaacaccgcgccgaagaaccacatccacgaaatgcccagcagcgaccggaacaccacgatgttgccgtgcgcgagcttgaggttgcgccaggtctcgctgaacgggttccagttgatcaccagccccggatcggtcgcgggcgccggtggaatggcctgcgccacgccgcgcccgaccagcgccagcagcaggcaggccacggccaccgtggtgtggccgacctgcggcaaggccaccagcagcccgccagccacctggccgagcaggatggcgacgaaggtgcccatctcgaccatgccgttgccgcccgtgagctcgcgcgcatcgagcacctgcggcaggtaggcaaacttgaccggcccgaacagcgtggaatgcaggcccatgaggaacacgcagcccagcagcaccaccgcatcggccctgacgaagccccaggccgcgagcagcatgatcgcgatctcgaggttcttcacgaagcggatcatcttcgtcttgtcgaacttgtcggtgagctgcccggccgtggcggaaaacagcaggaacggcaggatgaacaacgcgccgatggccaggcccgccatggccggcggcatccaggtcagctggagctggtaggtcaccatcacggtgaaggcgaacttgaagagattgtcgttcgccgcccccgcgaactgcgtccagaagaagggcgcgaagcgccgctgcccgagaagcgcgaactggttggcgtgcgcgttcgcttcgtgaggcgcggtaacggcagcagcagcggcggggttcgtcattcgaagcatctcctcttgttatctacacacggtctccgcttcttcgtcgtggaacaccgaggatccggctccgccggtcctctggtgttgcccccggcagggggttggcgtagcgacacgaagtgcgtgaagactgggggcgagccaatgtcacgccgttagaacggctgcgtccggattgtgccgcagcagggccctgcgccagctcacgtcgagcttcctgagcgccgcaagcacaggcaggccggccagcgatgcggccaggtgcttgaggctgtggccggagatcagctgcccggtcatctcgtagatcggctcgtccgccagctcgaagcccttggccagcacatagaagaagatcacccagccgagcttgagtccgaccgcgccgcgcatcggcgtggccagggccagcgtcagcaccacggccatgccgccaaactgcacgatcgcccagggcaggacattgccgctctcatggaacacctcggccgccagcaggccgcccgccagcacgaaccaggccgccggccaaccggcgcgctggctcacgcgctcgcagaccgcgatgccgatcaggcccgcaaaggccacggccatgccggcgcggtcggccgcgagccgggacgcgtcgggcatcaggtgaaagaaggccgagcccgcggcggtggcgatcagccccgcgaagaaaagccaggcgcagtcgagcgtgttgtccggcggatcattggccggcggtgccagcgggaattcggccagcgcctgctgatgggcacggtcgatccggtggagccggtacaggccccagcagccgacgagcgcaaagggcaggttgctgagcacgtccatcgcgttgggcaggccgtaccaggcgcggctgtcggcaaacaccgaggcgatcgccacgtcggcggccggcagcgcgggcccgaagagggccgccaacgcgagcagcgcaaaggtgaaaagcaatccgcgttcgcggcggctgagggtggtcgggagcatggcggtcctcgtgggttgggtacgagtcgcggaatttagttgccagcctctctacaggcatcgagaatcgatacgaggcattaattcacacctttcggtatcttcttttagtacccctttgccagcaagctacttttcatgagcaccaccgtcgacctcgtccaagccctcaagaacgaactcaagagcgcccgcatgacttacgccgacctggcgcggtcgctcgacatggccgaatccagcgtgaaacgcatgctggccaagagcgacatgccgctgtcgcgcgtcgacgcgatctgccgcgccctcaagatcgactttgccgagctggcgcgccgcgtggccgacgcccagccgctcctgaaggagctcacccaggagcaggaaaaagcggtggtcaaggacaagaagctcctgctggtggcgatcagcgtgctgagccagtggacgctggagcagatcgtgtcctcgtaccggatcagcgaggcggaatgcatcggctttctggcgcaactcgaccgcatcggcatcatcgagctgcgcccgctcaaccgctaccggctgaagctggccaagaccttccgctggcggccgcacggcccggtgatggagttctttcgcgagaacgtggtgctcgactactaccgcggtggtttcgatggcccggccgaagggctgctgctggtgcacggctcgatcagccggtcgctggcgccggcgttcctggagcggctgcagcgcgtggcgcaagactttgcgcagcagcaccagacggaccagaagctctcggccaaggaccgcgagggctacacgctgctgctgggcatgcggaactgggaattcgaagccttcacgcgcctgcgtcgcggctgaccctcagggcttgcttcagggcttggcggcttccagcgcgtcgcgcgtggtgcgtgcggcgttcttcgcggcggcggcgaagtcgtcgccggacgaggcatagatgatggcgcgcgacgagttcacgatgatcggcgcatcggcgcgccagccggcacgcaccgtggccaccgcatcgccgccctgggcgccgacacccggaatcagtagcggcaccgtgggcgcgagttcgcgcacgcgttcgatctccgccgggtaggtggcgcccaccacgaggccgagctggccgttgaggttccaaggcccctgcgccagcttggcgacgtgctcgtagaggaaaggctggccctcgatgtccgcgaggcgctgtccctgcaggtcggagccgccggggttgctggtgcggcagagcaaaaaggcgcccttgccttcatgcttgaggtagggcgccaccgaatcgaagcccatgaagggcgacagcgtcaccgcgtcggcgccatagcgctcgaaggcctcgatggcgtactgctcggccgtggagccgatgtcgccgcgcttggcgtccaggatcacgggcacgtgaggcgcattgcggcgcatgtgctccatcagttgttcgagctgggcttcggcgcggtgggccgcgaaataggcgatctgcggcttgaaggcgatgaccaggtcggccgtggcgtcgacgatgcgcgcgcagaagtcatagatgcggcccgcgtcgcccttgagctgccccgggaacttggctggctccggatcgagccccacgcagagcaacgaaccgtttttttgctgtgcagtggccagcttgtcgaggaaagtcatggggcctgattttaaggaccccggccgccggcccttaattcgacggcgattgctgttcagcggccaggcacaagtcggcccaggcgcgcgccttgtcggcggggtttcgcaacaggtacgcggggtggtaggtggccaccaccgatacgccctggatcgatgccagcggcacggcacggccgcgcagcttgccgagcggatcggcgctttgcatcagcccttgcgcggccagcggccccatggcgagcaccagcctcggtgccagcgcggcggcctgttcctcgaaggcctcggccatgggacgcgggctgccggactggccggcggccacgccgcggtgcgtgcgcatcaggtgcaccggcgtcttgccgtcgtgcagcttgagggcgcgcagcatgttgtcgagcagcttgccggcgtcgcccgcaaagggctcgccgtggcggccttcggcctcgggcggcatgtcggccacgacgagccagccgccctgggccggccccgctccggcctcggcgtaaaggcggcggggtgcctcgaccagcaccgcggcgccatgggcgatcggcgcggccgcggggcgggccgccggggccgttgccgcagcgggccttgcggccggggcgggcgcctcggcgacgaagcgttcgcgcgtttcttcttcaaccggcggcggctccgcggcaaccgctttcgtttccacggcgacccttggcgcttcggccacttcgggcatcggccaccagaccttcacgcccatttcgtcgagcatcgcgcgctggcgcgcatcgagtttcaatgtctgtatcgcgctcatcgcaaagctccccaggcggagcctgtttcattcagtcgcaggctcatgaccacggcgtcttcgcgcttgctgtcatgggccgggtagtagcccttgcgcacgccgacactgcggaaaccctggcgcacgtagacgtcgagcgcacgctggttgctctggcgcacttcgagccagagccatagcgcgccttcgccgcgcgaccatccggtcagcgcctcgagcatcagcggcgcccacccctggcgctggaaaaccggcgccaccgtgaagttgagcagatgcacctcgtccacgcctttcatggcgacgaagtagccgatcagcgtttcgccgaggctggtcaccggcgtggccaggtcgggcacggagaccggcgcgagcaggcattggcagtggtagccgaccgccatcgagtcgatgaagttggcccgcgtccacggatggctgtaggccgtctgctcgaccgcgcagacggcatcgagccgctcgacggtgagcggttcgaggcgggcttcgacgggctgaagaacggcgctcattcgattacctccgtgcttcgcactgcgatgcgagcttgcttggggcggcccggcgcggcgctcattcgattacctccgtgcttcgcactgcgatgcgagcttgcttggggcggcccggcgcggcgctcatgtcttgctggcaacaggtgaaaccgcgacggcggcggccgccttgatggcagcgcgctcatcggtcgtttgcgccactttatcgcgaacatagagcggccaggcatgtgccgcgtccaccgtgcggccggcggccagcagcgcgggcgcgaggcggagcatggcggtggcggtcggcagcacttcatggcgcgccgcggcgggcgccaggcgcgggccataggcggcaaaggcgttaccggccagggaccagccggcgggcacttcgagcgcttcgggcgcgagcagcagcggctcgccgccatcgccttgcagggcgcccagcgcgccgccgccgtcgaagtcgtagcgcgcggcatagagctggtccatgcgcgcgtcgagcgcggccaccacctggcgggcgccgaatgtgtggcgggcttcctcggccacggccagcagcgtgtcgaccggcagcagcggcacgccggagccgaaggccaggccctgcgccaccgagcaggcggtgcgcaggcccgtgaaggaacccggcccgcggccgaaggcaatggcgtcgagcgcggccagttcgagcccggcctcggccagcaattgcaggatgagcgggatcagcgtgctcgacgcctgcgcgccgccggcgccgctgtgcgtgaacaggcgctcgccacgccgaaccgcgaccgacaggtgctcggtgctggtgtcgaaagccaggagcttaggcatcgcgtcgtcccatggcggtggccggaaccgtgggcatcggggcattgcgcgccccggccgatttctgcacgccgaacaggatgccggcggtcaccagcagcaggccggccatcaggttccagtgcagcggctcgtcgagccagatcaccgcgccgaaggccgagagtccgggcacgagcgccgtgatcatggtgctgcgcaccggtccgaagtactggatcatcttcgtgaacgtgatgcccgagatgacgaccgagcccaggccctggaacagcatctggaacgccacctcgccccacggcgcggaaccgatgcggctcgcgaccgcaccgcccgccaccagcaggctgtagacgggcacataggtcagcaacgcgaagacggtgatggcgatggtcgcgcgcacggcgtcgagcccatggcggcgcgccaccacgctgtagcaggcccagcagaaggcggccgacatgaagagcaggtcgcccttccagacctcgccgccctcgaaggcgtgcagcaggctgcgcccgccgaccaccagatcgccggccacgatcagcgccagcccgaaagcgcggcccggcgtgatgcggtcgcgcagcaccagggcggccagcagcgtggtccacagcggcaggctgccgggcatcagcaccgaggcatggccggccggcgcgaagaagaagccgctgtaggccagcgcggcataggccacgccgccgaagatgccggcgctggcggtcacgcgcagcgacaggggcgagaggccgaaaagcgaggaggcggtggtaccgtccctttgccggaggtccttcatcaccatccaggcaccccagggcaccagcaccaggctggcgccgcagatgcgcgccagcgccaggtcgaagggggtgagcgagcgtgcggccgaggcccgggcaatcacgatgaaggccgtccagaccagcacggtgaccacggccgcgccgatgccgagcgtgcggggcgagaggcgtggcgtggcgggcatccccccattatcgagggcccgcccttggccgcgccggccaggggcgaatcggcgccgaatgcggcgatcagccgccgtcgctgcgaaggatgtcgagcccggccttgcgcaacggcgccagcgcggcctccggtgcttccggcgacaccagcaggcgggtggccgacgacacggggttgaccatccaggccgaggcggcgccgatcttttccgacgaggccagcaccaccgtctcggccgcggcggccatgagcgcgcgcttgatcgcggcctcctcggcatcgccggtggtcagcccggcctcggcatgcacgccggtcacgcccaggaagcaggtgtcggcgtggatgcgcgagatggcgtccatcgccgccgcgcccaccgccaccatcgaatgcctgaagaggcgcccgccgatcagcaccacctcgacgtccgcgtggcccaccagctcgaccgcgaccgacgggctgtgcgtgaccacggtggcgcgcaggttcttcggcaggtgccgcgccatctggacggccgtggtgccgccgtcgatgaacaccacctgcgcgggccgcaccaggcgcgccgcggcgcggccgatggccaccttctccgcggttgcgagctgcagccggcccgcgaaatcggcttcggccctggcgagcggcagcgcgccgccgtgcacgcgctgcagcaggccctcggccgccagctcgcgcaagtcgcggcggatggtgtcttccgacagcccaagctcctcgctgagcgacttggcgacgacgttgccgtcgcgttgcaggaccgagaggatgtgttgcttgcgctggcgggtgagcatcggtcgatggtagctggcgaggaggtcgattgcacgaattttcttgtttctgcacgaatttgcgcataagctgcgcgccatgacccttcaagaccgcgtccgggtgcacgaagtcaccctgctttccgacaactggtacacgctgaagaccaccgccttcgactggcggcgcagcgacggcgagtggcagcgcatgcaccgcgagacttatgaccgcggcaacggcgccacgctgcttccctacaacctggcgcagcgcacggtgctgctgacgcggcagttccgctatccggccttcgtcaacgggcacgacgacctgctgatcgaggccgcggcgggcctgctcgacaacgcggcgcccgaggaacgcattcgcgccgaagtggaagaagagctgggctatcggctcggcgcggtgcagaagatcctcgaagccttcatgagcccgggctcggtcaccgagaagctgcacttcttcattgccgaatacgagccttcgatgcgcatcggtgacggcggcggcctggccgacgagggcgaggacatcgaagtgctcgaactgcgcatcgacgaggcgctggccatggtggcggacgggcgcatcgccgacgccaagacggtgatgctgctgtatcacgcgcagttgcatgttttcgcgccgagataatcggccgatgcttcttcttcgcctctcctttcttcgtaccgcctgcgccctgtctttgaccgcatgggccgcctcgagcgcctttgcccagcaggctttcccgaccgaagtagaggctgccctcgcgcgcgccaaagtgccgcgcgattcggtgacgatgctggtggccgatgccgacggcgtgcgtccgcctcggctggcctggcgctcgcaggtacaggtcaatccggcgtcgatcatgaaactggtgaccacctacgccgcgctcgatcttctgggcccagcctacagctggagcacgccggtctatgtcgacggcacggtgagcaacggcgtgctcaatggcaacctctacatcaagggccagggcgatcccaagctggtgctggaacgcgcgtggctgctgctgcggcgcgtgcaggggctgggcatcaccaccgtgagcggcgacatcgtgctggaccgcagcgccttcgagaacacggccgagaacgaccccggcgccttcgacggcgagccgctgcggccctacaacgcctcgcccgacgcgctgctggtcaacttcaagtcggtcaacatgaccttcacgcccgagcgcggcggccagcaggcgcgcgtgagctacgagcccccgctcgccagcgtgtcgacgcagcccgcggtggcgcttgcgcccggcgaatgcggcgactggcgcacagcgatcaagcccgacttcagcgacccgaaccgcatccgcttcacgggtgcgcttccggccgcctgcggcgaaaaaagctgggccgtggcctacgccgacccgcgcacctacggcctgcgcgccatcggcggcctgtggggcgagatgggcggccgcgtcggcggccagatgcgcgagggccgggtgcccgcgggcctccggccggccttcgaattcggatcgccgccgctcgcggaggtggtccgcgacatcaacaagtacagcaacaacgtgatggcgcagcaagtgttccttacgatcgggctcacgcagaagaaccgcggcagcttcgaggcctcgcgcagcgcgctgggccaatggtggcgcgaccgcatcggcaccggcgaggcgccgccggtgttcgacaacggctcgggcctgtcgcgcgacgagcgcatcagcgcggcggcgctcggcaagatgctgcaggtggcctggcgctcgccggtgatgccggaactggtgtcctcgctgcccgccactggcgtggacggcacgctcaggaagcgcgcgctgcgttcgggcggcgcggcccacctgaagacgggctcgctgcgcgattcggccggcgtggccggctacgtgcacggcgcgagcggccggcgctacgtgctggtggccattgccaacggcgagaacgcgggggcggcgcgcgccgcgttcgacgcgctggtcgactgggcttcccaggacaactgagccgccggctggcggccgtgtactgaaaacttctctaggtattcgcgccgcttgcgtgcgggcaggtcgctgcacagaatcggacgcccgttcggtccgactgacaaaacatcaagaggcacgccttgaaccagccccaacgacaaccttcttctccgctgcgtggtctttcagcgctcgccggcgtcaccttgctgctggccgcctgcggtggcggcggaggaggcggcggcatcggcgtggggcttccgccgccggtcggcgacaccggccgcggatcggtcgtcaccgacccgcccgagcagaccgcaaagctgacggccgaccagttcaggaccaacctgcaggccagcgaccagggcaaggccttgctgcaggtggccggcacgcccaagtgcggggtcgaggtgcgctatctcgaataccgcacggtgggtggcaagggcgaagcgaccaacgcgacggccgcgatcatgctgccgtcaggggccgacgtggcctgcaacggcgcgcgcccggtggtgctgtatgcgcacggcaccaccgccgcgcgcaattacaacctcgccaggtggaccgactcgacccagccggccgccggcgaaggcctgaccatcgccgcgatgttcgcggcgcagggctacatcgtggtggcgcccaactatgcgggctacgacaagtcgacgctgccctatcacccgtacctgaacggcgaccagcagggcaaggacatggtcgatgcgctcacggcggcgcgcaagactttttcgggcatcgacgcggcggacgcgggctcgctgctgatcactggctattcgcagggcggctacgtggcgatggcggcgcaccgcgagatgcaggccacgggcaaggcggtgacggcgtcggcgccgctctcggccccgtcggccatcggcctgctggcggattacaccttcctgggctggccggccctcggcagcacgctcttcgtgccgctgctttcggccagctggcagcagcagttcggcgatgtgtacggcagcaccgccgacatctacgaagcccagtacgccaccggcatcgacaccctgctgccgagcctgacgcccctggccaccctgtatgccaatggcaagctgccgcagctcgcgctgtttccagccggcgcaacgccggggccggtgagcccggagctgtcgatcttctatggcgccaacaacctgatccgccagacctacctgacgcaggcggccggcgacatcctggcgaatccctgccccggcaatgcgctgcccgccacggccggctcgctcagcacgacctcgccgctggactgcaggccggccgtgggcttccgcaaggcggcgcgcgccaacgacctgcgcaactggctgccggcccggccggtgctgatgtgcggcggcgccaacgacccgaccgtgaatttcctgagcacccgcgccacggccggctacttccgcgcccgcggcatgcctgccgccgcgctgacggtgatcgacctggaagacacggccaccaccgacgcctactccaccgcgcgcgccggcttcgcgcaggccaagagcaccctggcgcagaacacccccggcagcgacgccgacaagcggcaggccgtcaccatggcctaccacggcacgctcgcgccgccgttctgcctggcctcggcccgaggtttcttccagggcgtgctggccgccggcggttaagaggggctcccttccagaaatgccgtggaaccggcttcgccggtccactggcattgccccctgaaagggggttggcgaagcgacacgaagtgcgcgaagactgggggttagctcagggacgcgcgctggaggcggtcgcgcacgccttcccactcgggcgtgtcgggcggcgtctcgacccagatcagcttgacgccctctgcgtcgaactggcgcagcaccgcgaacagctggtgcgcgctggccactgcatcgtcgggcatgcgccgttggagaacccgctgcgaggggctgcgcagtacggcacgcgaccacaccgcaatgttggcggcgcccgcgccgagcacgtcgagcgcggtctggatggccttggcgtccatcaaccgcagtttggcgttgggcgcgtagtgcgcctccagcgtgcccggggcgcgcgggtcgggcgtttcgagcacctcgcggttgctgaggcgctcgccaagggcggcctcgatctgtgcgcgcgtgatcaggcccgggcgcagcaacacgggcgcgccgcggctgcagtcgacgatggtcgattcgatgcccacctcgcaggcgccgccgtcgatcaccggcagcgaatcgccgaactcgtcgaccacgtgctgcgccgtggtcgggctgacgcggccaaaacggttggcgctcggcccggcaaggcccggcacgccctgctcggcgcaggcctcgagcagcgcctgtgccaccggatgcgaagggcagcgcaggccgatggtgtcctgcccgccggctgccgcgccggccacgccaggctggcgcgtgacgatcagcgtcagggggccgggccagaaggcctgcaccagcttctgcgcgaaaggcggcagcggctgcgcaaagcgcgacagcgcctcggtgcccttgatgccggccgcaacgtggacgatcagcggatggtcggccggccggcccttggccttgaagattccgcccaccgccatgtcgctggtggcatcggcgcccagcccatagacggtctcggtcggaaacgcgaccagcccgcccgcgcgcagcacgcgcacggcttcggcaatggcgtggggatcctgcccgtcgagaatcatgcgaaatcggccgccgaaaggggcggcaggccaagcagcgtggcggcctgcgaggccgcggcgcgcacgctttccagcgtggcgccggtaagggtcaggtggcccatcttgcggccgcggcgcggttcgatcttgccgtagagatgcaagtgcacgccgggcagcgcgagcacgtcgctccagcgcggagcggccggcttggtgccgcccgcggtgaaccacaggtcgccgagcaggttcagcatgatcgccgggctgtgctggcgcggcggggccagcggcaagcccgcaagcgtgcgcacctgcagctcgaactgggacacgtcgcaggcttccatggtgtagtggccgctgttgtgcggccgcggcgccatttcgttgaccaccagggagccgtcggtcaggacgaagaattcgacgcacagcacgccgacatagttgagcccggtggcgatgctcttggcggaattgatggccgcctgcgccacggtcttgggcatgttctgcgcatgcacctcggtcacggccaggatgccgtcccggtgcaggttgcgttggggcggaaagtgcacgatctgcccgtcgcggccgcgcgcgacgatcaccgagcattcgaactcgagcggcagcatcttctcgagcacgcagggcacgcagtgcgcggcctgccaggcgtcgaccagctcggcgcgcgtggtcacgcgctgctgtcccttgccgtcgtagccgaggcgcgcggtcttcaggatgccgggcagcagcccgtcttcaccggccgcgagctgggccgcggtctcgatgaccgcgtacggtgcgcaggccacgccgcagcgtgtgaaatgggccttttcggcgatgcggtcctgcgcgatggcaatggcggcggcatcgggcgacacgggccgggcggccgacagcttgtccagcgagggggccggcacgttctcgaactcggtcgtgaccgcatcggccaggcccgcgagccgcgccaggccgtcgacgtcggcgtagtcggtgtggatgtggtgatggctcacgcggccggccggactgtcggcgtcggggtcgagcacggccgtgaaataacccatgcgctgggcggcgtgggcgaacatgcggcccagctggccgccgccgagcacgccgagcgtggcgccgggaagaatgggcaggccgttgttgctcatagggcacccccgccttgcggcgaaaaaggcgacacggcgccgccgtcgaccggcggcggcaacgccatggcttcggccgcggccgtttgcgcggcgcggaaggcatcgagccgggcgcgcagcgccgggtcgttcactgccagcatggccaccgcgaacagcgccgcgttggcggcccccgcattgccgatggcaaaggtggccaccggcacgcccttgggcatctgcacgatgctgtagagcgaatcgacgccctgcagatggcggctggccaccggcacgccgagcaccggcaccgtggttttggcggccagcatgcccggcaggtgggccgcgccgcccgcgcccgcgatgatcgcgcagagcccgcgcccggcggcgctttcggcgtacgcgaagagcgcatcgggcatccggtgggccgagaccaccttcgcttcgtgctggatcccgaattgctggagaatctcgaccgcgttgcgcatcgtctcccaatcggagctcgagcccatcactacaccgacctgaatggtttcgttcatggtttcaattttacgtttcacccccagctggttccgatgatcgacatcactctcgaaaattttcaggccgaactgatcgaaggctcggtcgccacgccggtgctgctcgacatctgggccgagtggtgcgggccgtgcaagcagctcgggccggtgctcgaaaagctcgaggtcgagtacgccggccgctttacgctggccaagctcgacgccgacaaggtgccgcagatttcgtcgcagctgtccgaaatgttcggcgtgcgcagcattccgttctgcgtgatgttcaaggacggccagccggtcgacggcttcgtcggtgccattccggccgacaagatccgcgaatttctcgacaagcacgttcccggcgccgaggaagcggaggctgcttccgagggggccgcggcgcaggaggcgctggctgaaggcgataccgagggcgcgctcgagcggctgcagcatgccgtggccaccgaccccgccaacgacgacgcgcgtttcgactacgtcaagctgctgctgcagatgggccgcatcgacgacgccaaggtggcgtttgcgccggtgattgccaagaccacgctggtgcgccgcttcgattcgctgcagcgctggatggacgccatcgattttgcggcgccggcctcgggccccgcgcccaccctggccgatttcgacgcccgcattgccgccggcaaacgcgacttcgatgcccgcttcggccgcgcgcagctgctgatggatgcccagcgctggaccgatgccatggacgagctgctcgagatcctgatgcgcgacaagagctggaacgaagaactcgcgcgcaagacctacatcgcgatcctcgacctcatcgagccgccgaaggtcaaggtggccgatgggcagattccgccggatgacccggtggtggccacttaccgccgccgcctcagcagcgtggtgctgagctgaacgccagattgcgcaccttgatcagtgcgcaattcaacgaaaaagcgactctcgggtcgctttttcattgctccgctcaccgcttctggacgcggccagcgggcgccgcggcattggcgggccagggcggtctcgaatacgatggcgccgattcaacttgttgcaattgagaaggaaaaatcggccatgcgcttcctcgcccgcctcgcgcttcccgtcttcgcgaccgcactggcagccgccctgtccgcctgcggcagcggcatcagcctcgacgagccgatcgaaggcccggtctggcgtctcgcgcagctgggcggcgaacccgtggcgcccggcggcgatgcgcagatccagttcgaccgcagcagcggccgcgtcagcggatcgggcggctgcaaccgggtgtcgggttcattcacgcgcagcggcgtcacgctgcgcatcggccagctggcatcgacccgcatggcctgcgcggacccggtgcgcggcgccaacgaagcgcaattcgtttcggcgctgcagaccaccgccagctaccggctcgccggtcccgggcggctcgcgctgctcgacgcgagcgggcgcaccgtggcaatgctgaacgcggcgacgcgctgaaggctgccgccgggagcgctcttcgcgctcttttttttcctcagccggtgaggcgttccagtgcttcgcggtacttggccgcggtcttctcgatcacctcggccggcaggcgcggcgccggtggcgtcttgtcccagggcttgccgttgatcttggtggcttcgagccagtcgcgcacgaactgcttgtcgtagctcggcggattggtgccggcggccagcgcggcttggtagccctcgaccggccagtagcgcgagctgtcaggcgtgagtacctcgtccatcagcaccagcgtgccggcctcgtccaggccgaactcgaacttggtgtcggcaatgatcattcccttggtcagcgcgatctgtgcggcggtttcgtagatctcgaggctggtctcgcggatctgctgcgccagcttgggcccgacgatctcgaccacgcggtcgtagctgatgttctcgtcgtgctcgccggccgcagccttggcggcgggcgtgaagatcgggcgcggcagcttgctggcgttggtgagcccttcgggcagcggcacgccgcagaccgagcggctttcctggtattccttccagccgctgccggccaggtagccgcgcaccaccgcctcgaccggaatcggcgtcaggcgcttgaccagcatcgagcggcccgtgacctgcggcacctcttcaggcgtgaccgcgctttcgggcgcgtcgccggtcaggtggttggggcacagctggcccaggcggtcgaaccaccacagcgccatttgcgtgaggatttcgcccttgcccggaatcggctcgcccatgatcacgtcgaaggcgctgagccggtcgctcgcgaccatcaggatgcggtcctcgccgacggcgtagttgtcgcgcaccttgccgcgcgcaagcaggggcaggctctggatggaggaggtgtggacggtggtcatgaggcggtgctgtgcggaaacgggtgacgggaaaaacggattgtgcgcgcagaaaaaagccaccgcgaacggtggcctgcgaatcgcgaaaaaagtttccttagacgacttcttgcgcgagctcgcccttggcgtatttggcggcgacgacctgcagcgtgtcgcccttgatcttggcgccctggccttcgcagccgaactcgatgtagcgctgcttgcagatcagcttggcggcttcgcgcgcgggcttgagccattcgcgggcgtcgaacttctcggggttctcggccaggaacttgcgcaccgcgccggtcatggccagtcggatgtcggtgtcgatgttgatcttgcgcacgccgtgcttgatggcttcctggatttccttcacgggcacgccgtaggtttccttcatgttgccaccgtactggcgaatgatggccagcagctcctgcggcacgctcgacgagccgtgcatcaccaggtgggtgttgggaatgcggcggtggatttccttgatgcggtcgatcgccaggatgtcgccggtgggctcgcgcgtgaacttgtaggcgccgtggctggtgccgatggcaatggccagcgcgtcgatctgggtgcgcttgacgaagtcggcggcctgctcgggatcggtcagcagctgttcgcgcgtcatggtgtcgtcggtgccatgaccgtcttccttgtcgcccttcatggtctccagcgagcccaggcagccgagctcgccttcgacggtcacgcccaggcggtgggccatgtccgacaccttcttggtgacgtccacgttgtagtcgtagctggcaatggtcttgccgtcggcctcgagcgagccgtccatcatcaccgagctgaagcccaggtcgatggcgcccttgcagacgtcggggttctggccgtggtcctggtgcatgaccagcgggatgttggggtactgctcgatcgcggcctggatcaggtgcttgatgaaggcttcaccagcgtatttgcgggcaccggcgctggcctgcaggatgacgggcgcgccggtttccttggcggcctccatcacggcctggacctgttccaggttgttgacgttgaaggccggaatgccgtagccgttggcggctgcgtggtccagcagttcgcgcatcgagacgagtgccatgggaaatacctcgcggaaataggggaaaaagaaggcggaaagacgagagaaaactgccgcaattctatcgagcccccttgtgggacggcactgacaggtacctcaagccggtggcaaggcggtcgcgggcgcctctagatcggcagttgcgtggtcgacagcacctgcttgagcaccacgaaagtccggatctgccgcacgccgggcaagtacagcagctgctcggcgtgcaggcggttgaagctgtcgttgtcgcgcgttcgcacgagcatgaagtagtcgaactcacccgtgaccacatggcattcgaggcagccggacaccttctgcgcggccttctcgaaatcggcgaacgagtcgggcgtcgagcggtcgagcaccacgccaatcatcaccagcatgcccagatccagcgccttcgcatcgagcagcgccacgatgcccttgatgagccccgcggccttgagccgctcgacccggcgcaggcaggccggcgcgctgagattgaccttggccgccaaggccacgttcgacaccgaggcgtcgcgctgcagggcgcgaaggatggcgcgatccgtgcggtcgagctccaccgccgcctcggccgcctgcgccggcgtggtacgcaactttgttgtgctcatcttttcctttgcaaaccaaaaacattcaatctggcgatcttgtcttttttttgctcgtatttccatcgaagtttgcaaccacgtttcttcgccttctttctacgatcgaggtcattcctcctccttttcatttcctctggagcacatcgatgaacctcaagaaatttccccgccataccctgaccttcggccccacgccgatccatccgctcaagcgcctgagcgcgcacctgggcggcgaggtcgagctctacgccaagcgcgaggactgcaacagcggccttgccttcggcggcaacaagacccgcaagctcgaatacctgatccccgaggcgatcgagggtggctacgacacgctggtgtcgatcggcggcatccagtcgaaccagacccgccaggtggccgccgtggccgcgcacctgggcatgaagtgcgtgctcgtgcaggagaactgggtcaactattcggacgcggtgtacgaccgcgtcggcaacatcgagatgtcacgcatcatgggcgccgacgtgcggctggacaacgcgggcttcgacatcggcatccgcaagagctgggaagaagccatggacgacgtgcgcaaggccggcggcaagccctttcccattccggccggctgctcggagcaccgctacggcgggctcggcttcgtggggtttgccgaggaggtacggcagcaggaagccgagctgggcttcaagttcgactacatcgtgacctgctcggtcacaggcagcacgcaggccggcatggtggtgggctttgcggccgacggccgggccgaccgcgtgatcggcatcgacgcatcggccaagccgcagcagaccttcgagcagatcgtgcgcattgccaggaacacggccgaactggtcgaactgggccgcgacatcaccgacaaggacgtggtgctcgaccgccgcttcggcggccctgaatacggtctgcccaacgaaggcacgctggaatcgatccgcctttgcgcgcgcctggaaggcatgctgaccgaccccgtgtacgagggcaagtcgatgcacggaatgatcgagaaggtgcgcctgggcgaattccccgcgggctcgaaggtgctgtatgcgcacctcggcggcgtgccggcgctgaacgcctacagcttcctgttccgcaacggctgagcgaactcggctcgcgcggcagatctccgtcatgtaggcagccgctcagcccgcctatccttccgacaatttgcctcgatcggtcatcgcggtttgacgcgcacatactccccagagggcttggccgacttgtccgccctgacacacaagtgtccgtcgcacagcgtgacatcggcctcgttgtaagccttgagcaatgtggcagaaatttggttcttcgagatctcgtcgtagtagtgactcgacaaccaaacaccgcccgacagcatcaacaccaggctgcccagcgtgatgcctgcgaccttccagatcaggtggcggtgcaacgcctcggcacgtcggagctgcgcgctcaaggcaagagaagactgatggatttgttcgcctgcttcgcgcaggcgccgttcatagtcggaaaccggccgctcgatgccaccgcgaacatctgcaagcaccgcctctggcagccggcccagctgctcgttggcggcttggcgcaccacggccggcacctgttgggaaagcctctgcagttccgagccggattgctcgcatcggcgctcgaacttttcgaccagcgcgctcatcttgctggccaacgccagcatggtttgatcgttcacttttatttgcctcgcctgttccgcgcgtggatgggctcaatggcgcatgaccatcgccggcgcattcattgcaggctgctgctgcgcttgcgcctgttgttgcgcaacccattgctcctgccgattcacttccgcaattccctctgcgatcacctctcggcccggcggcaggtccgccaacgtctgttgcattcttctgaaggtggcgtcatcggcgctcagcatgcggtccagaaatgcggacaggtcgtcagtgggtgagggctccttggatggcgtctgcggcgtgcgttgcgcttcgcccgttgcttctgcaggcgcggcgccaggcagcatgcggctcgcctcgacttcacagaattggccgtaggtttgcctggtgttcgatgtgacgttgcccctgttgttctgagccagcgcatagacggccgcctccatgacctgagtggcggtcatgtggccgggttcttcccgggcggcatccgaaatgcgtctggcgatcaggtggtcctggccttcgccgcggctaccgtgcaccccttcaccgcgccagcgggattccagttgaacttcctgttccgtaaggggccgttgctcgagctcggcggccaagcgattggtttccaggatttcttcgcgcactttgacttcgttgtagtgggcgtagccttcggtcaggtggcaggcgctctcgtaagcggccttgtcttttcccgtcagggcgttggagcgcgcggtcgcgatggcggcattgggttcttcaacgcgaaagtgcccgagttcgtgggccaggatgctgactgtgccttcgggggtggtgaagcggtcgagggcgatgcggaggcggccgggattgtccttatccaccggcgtcctgtactcgcccgcaccggcttctgggttgatccttccagcggccgtgtaatcgctggaggcataggcgcgcatgtcggccttgagcgtttccgacctgttgatcattgcgagcgcctcgggcgaaatcttgtacgccttgaatttgttcttctcgtcggccaaccactctgctgtgatggccgtggtgaaagtgctcattttttggttccctctctctgattctttagtgattcaaggtcgcgctgaacggtgatgcctcccacgcattcgtagtaactgaaatcgaattcaattcgcccgttcctaggccccttgaagaagcggggagtgacatagaagatgccctggagctttcctgtttgaaagggcggcgttggcaccccccctggcaacgccacagcaggcgctacgggacggtgtggcgagacggtgaagccgtcgccgaaggtggcgatcacatccgccagtgtcacgcatgatttcctgatgtcgacgtcaaagctgaaataccttttccccccaaaccttggtctgtcgtcatctgcacgcttgtagtaaaagttgctgacgcccgctggcaaatgttgaagctcttctgcgttccccgctcccgccgagatccgccaaggaacatttctggactcgctgtagtcccggtcgttcttgatccccagggtttcataaaacaggtggcttggatcggagaggtcatccgtccgtgcgatgcaccaggccagttcgacgatcgggtgtttcggcggccgggcttcggcgctctgaaccgcgcatgatgctgccgtcgaggagttgaaattcgacacccccggcagaacgccgcaccctgcgacggacaccgccgtcgccaaggccagcagcaccgctttgaatgcgtgcaattgcttcattgatttcccgcccttccggatgtcgcgatcacatccgcagtgtcacgcaggatttcttggggtcggttcaaaaccaacgcgccttttcccgctgatcgtgaacttatcgacgtctatgcgttggaaggattgaaattcgacacacccggcggaacgccgcaccttgcaacggacagcgccgtcagcaaagccggcagcatcgccttggatgtagcaattccccatttgatgtcccccgcccttccggcgctcgagacatcgtcgatgcccgatcgatcagctcgcgcggcagatcttgagcatgttggtgccgcccggggcacccatcggctcgccgcaggtaatcgcatagacgtcgccggtctgcacgatgccgcgcttcttcaagtgggcttcggcctgctcgagcgcggtgtcgcggtcgctttccgaatccatcagcagcgggcgcacgttgcggtagagcgccatcctgcgctgcgtggcaaggcgcgaggtcagcgcgtacatcggaatgtgcgcgcggtggcggctcatccacagcggcgtggagcccgactcggtgagtgccacgatggccttggcgccgagatggtgggccgtgaacagcgcgcccatggcaatcgactggtcgatgcggctgtaggtcttgccgctgaagtcggcgtcgagcatcttgtcctcggccgattcggcggcctcgcagatgcggctcatctcctgcacggtttcgagcgggtagcggcccgaggcggtttcggccgagagcatcacggcatcggtgccgtcgagcacggcattggccacgtcgctcacctcggcgcgcgtgggcacggggttggtgatcatcgactccatcatctgggtcgcggtgatcaccaccttgtccatgtcgcgcgccatgcggatcatctttttctgcagcgcgggcacggcggcattgcccacctccaccgcgagatcgccgcgcgccaccatgatgccgtcgctcgcgcggaggatctcctccagcttgggaatggcttcggcacgctcgatcttggcgatcaggcccggcttgtggccgaattcggccgcggccacgttgcacagctggcgcgccatttccatgtcggtggcgttcttgggaaagctcaccgccacgtagtcggcctggaagctcatcgcggtcttgatgtcttccatgtccttggccgtgagcgccggcgccgtgaggccgccgccctgcttgttgatgcccttgttgttggagagctcgccgcccagcttgacggtggtgtgcaccgcctcgccgcgcaccgcgtcgaccgtgagcacgatgaggccgtcgttcagcaacagcttgtcgccggggcgcacgtcgcgcggcaggtccttgtagtcgaggccgaccgcgtcggtgtcgccgggttcggtgcgcgaggcgtcgagcacgaacttggcgcccggctcgagccagaccttgccctgggcgaacttgccgacgcggatcttggggccctgcaggtcggccatgatcgccacctcgcggccggtcttgcgggccgcctctcgcaccatggccgcgcggtcgatgtggtcctgcgccgtgccgtggctgaaattgagccgcaccacgctgaccttgttcaggatcatctgttccagcagctcgggcgtattggacgccgggccgagcgtggcgacgatcttggtggcgtggcggggaaggcgatccgtgatcattgagctagtctccattttgtatccgctactgtatacactttgtgtgactacaggaagtggacgcggcgcccacgcgagaaaaatcagcccgcggcgcgcttggcaagaatctcgaaagccggcagggtcttgccctcgagcacttcgaggaaggcgccgccgccggtcgagatgtagccgacctgcttttcgatgccgtacttggcaatggccgcgagcgtgtcgccgccgccggcgatcgagaaggcgctgctttcggcgatggcctgggcgatggccttggtgccacccgcgaaggcatcgaactcgaacacgcccaccgggccgttccagacgatggtgccggcttcgcgcagctgcgcggccagctgcgcggcggtcttggggccgatgtccaggatcaggtcgtcgtcggccacgtcgttcgcgtccttcaccgtggcgggcgcatcggccgcaaaggtcttggccgtgaccacgtccaccggaatcggcacgtcggcgccgcgggcgcgcatggattcgatcaccgccttggcctggtcgatcaggtcgggctccgccagcgacttgccgatcttgaggccggccgcgagcatgaaggtgttggcaatgccgccgccgacgatcagctggtcgacgttggccgacaggctcttgaggatggtcagcttggtgctcaccttggagcccgccacgatggccaccagcggccgcttgggcaatgccagcgccttggagatggcgtcgatctcggccgcgagcagcgggccggccgcggccaccttggcgaactgcgcgatgccgtaggtggtggcttcggcgcggtgggccgtgccgaaggcgtcgttcacgtagatgtcggtgagcgcggcgagcttgcgggccagcgcttcgtcgttcttcttctcgcccttgttgacgcggcagttctcgagcagcacgacctggccgggcttcacgtcgacgccgtcgacccagttggccaccagcggaacctcgcggcccagcagctcgcccaggcgcttggccacgggagccagcgagtcctcgggcttgaattcgccttcggtcgggcggcccaggtgcgaggtgaccatcacggcggcgccggaatcgagcgccagctggatgcagggcaccgaggcgcgcacgcgcgtgtcttcggtgatgttgccggcgtcgtcctgcggcacgttgaggtcggcacggatgaagacgcgctggccggcggccttgccctgcgcgcagaggtcggtgaatcgaatgacgttcatggatctggaggtggtggaagacaagtcgcccgcattgtaggtttcgccccgcggcggctctacccgcgtcatgccgtgcgccgatgctttttcagccagccttttgctgttcccgggcaaagcgctcgaggacctcgacaaagctcgcggcggcgggcgagagggtgcgccgcgcggcgctgtagacgcagacttcgcggtggaagtcgggcgactcgagccgcaccatctgcaggccgtgggcgcgcaccagcggcgccgaataggtcgggcacacggtgagccccaggcccgaggccaccatgccgagcgccgtggtcatgtacgacacctcctgcgtggccgggcgcagcatgtagtcacgttcggcgggcgccagttcgggcagcacgcgctggcggaagtcacgcgtgggcgcgatgaaggtgtagggctcgagctcgtgccagcgcaccttgcgacgcctggcaaacgcatggccgggcgggcagatcagccagtgccggtcgcgcaagagcgtgcggcgctcgatggcggcatccaccgccacgtcctgccccaccgcaagctccacgtcgccggccatcacgccggccagcaggtgctccggcagcgtgtcagccaggcgcacgtcgacatcgggataggcctcgcgatagaccgcgatcacgcgcggcatcagcgtgcaggccatgagttggggcgctgcaagacgcaacacacctttcttcttgtcacgcaaatccgtcacgccggccaccgcggtcgtgaggtcgccgaggagccggtgcaccgaaggcagaaactcgcggccggcttcggagagctgcacgcggcgcgtgtggcggtcgagcagctgcacgcccatttcgcgctcgagctcgcgcaccagcacgctgagcgccgactgcgtgaggtgcagctgctgcgccgcggcagtaaagctgccggtctcggccacggccgcgaaggcgcgcaattggcgcagggtcagattcatatggttatttcatcaatcgatgaattaatttcgattgcatcataagacgcggcatcgcccaatcacggcttaccggagacaagccatgccgacgactgccaacgcggcccccccagttcgcgggctgcaccatttcgcctggcgctgccgcgacagcgaggaaacccgccgcttctacgaagacctgctgggcctgccgctcgcccacgtcatcaagagcgaccacgtgccgagcacgggcgagtactgcccttacgtgcacatctttttccagatgcgcgatggctcgtacatcgccttcttcgacctgggcgacgacattgccgcactgccttcgcccaacacgcccgcgtgggtgaaccacattgcgctgcgtgtggattccgtcgaagacctgctggccgccaaggcccggctcgaaggcgcgggcgtggaagtgctgggcgtgaccgaccaccacatcatcgagtcgatctatttcttcgaccccaacggcatccgcgtggaactcaccacgccgaccgtgccgcaggccgagatggatgcgcatgcgcggcgcgcccgcgcggacctcgatgcgtggaccgcacgcaaggcgcagcttcgtgcagcgaaaggcggtgcgaatgtctgaactgcagctcgccgtcatcgacgtgaaagccggcgcggccatggaaagccagtcgggcctgcagatgctgcgtccgcgcatctacggcgcctttcgcgcgccgccgggccccaggaagatcgcggccatcgtgatgcacccggccagcaacttcatgggccactacctgatcggcccgctggccgagcgcggcatctgctgcatgggactgaactcgcgttacgtgggcaacgacacagtgctcttgatggagcgtgccatccaggacctgggcgccggcgtgcagtacctgcgcgcggccggctacgaaaaggtgtttctcatcggcaactcgggcggcgcggcgctcgcgagcttctaccaggcgcaggccgagaagctcacggccacgcacctgcccgatggcgacccgacccacctgcacccgagcgacctgccgccggtggatggcattgcgctgtgcgccgcgcacttgggccgcacgcggctgatgcgcgactggatcgatccctctgtcaccgacgagcacgatccgctttcggtggacgccgagctcgacatgtacgacccgcgccaccgcgtgccctacgactcggactttctcacgcgcttcagcacggcgcagaaggcgcggctggatcgcatcgagcaatggtgcatcgaccggctcgcgcagttgcgcagcaccccgggcgcgccgcgcgaccaggccttcgtcgtctaccgcacgcacgccgatccgcgctgcgtcgatctttcgctcgacgccaacgaccgcctgccgggcagcgtgtggggcgatgcgcggcaggtgaactattcggccaacgcgatggggcgcaccacctcgctcacggcctttctttcgcaatggtcgtcgcgctcgcaggccgacgggcccaccaacctcgcgcgcaccacggtgcccaagctgctgctgacctacacgggcgaccagtcgacctttccgagcacgcgcgatgcgtggctggccgccggcggcgggcgcatccgcaacgtcgacatcgtgggcggcaaccactatctcgcggggcaacccgagctggtgcccaaggccgcggatgcgatcgccgagtttgcccacgcgctgtagaagaaacatggaaagctttgcatttgcaccggcctacgagcttccgagctggcccttcacgccgccgcccgaactgggcagcccccggatcgttcgccacccgatcgtgatcgtcggtgccgggccttcgggcctcacgctggcctgcgacctggcgcaacgcggcgtgcgcgccgtgctgctcgacgaagacgacaccgtcggcgtgcgcggcgcctcgtcgcgcggcatctgctatgcgcagaagagcctggagatcttcgagcgcctgggcatctacgagcgcatcgcggccaagggcgtcacgtggtcgttcgggcgcaccttctcgggcgaacaggaggtctacaacttcaacctgcaggcgaacagcgtctccaggcagccgccgttcatcaacctgcagcagttctacctggagtggttcctggtcgagcgcattctcgaactcgggctcaccgacctgcggtggaagagccgggtgacgcgcgtggagccactccgcgacggcgtgcgcatcgacgtcgagacgcccgcgggccgctacacgatcgaggccgaccggctgatcgacgccacgggcgccaacagcccgatccgcacgcagctcggcatcgatgcgcattcgtcgcgcagcaccgaccgctggtgcatcagcgacgtgcgcttcaagaagcccttgccggtcgaacgatggacctgggtcgacgcccccttcaacgaaggccgcggcgtgtggcagcacctgatggccgatggcgtgtggcgcatcgactaccagatgcccgaagactgcgacccggccaccatcagccagcccgaagtggcgggggcgcggctgcgcgagcagctcgggccgggcgtggagttcgagttcgtgtggatcggcccgtatggctaccgcgaccacctgctcgacagtttccgccacggccaggtgtttttcatcggcgatgccgcgcacgtggtgagccccttcggcgcccgcggcggcaacagcggcatccaggacgcggccaacctcggatggaagctcgcgctgatcgcgcaagggcaggccagcgatgcgctgctcgacagctatgacgccgagcgccagcccgcggcacggcagaacctcgaagtgacgagccgctcggcgcgctttctcgcgccgcggtcgtcggccgagcacacgctgcgccgcgccgtggtggcactggctgcgcgccatccgttcgcgcgggcgctggtgaacaccggccgcatgtcggtcgccaacgactatccgtccgcgccccaattgcccgagggtgggcgcaccgtgcagaacctgccgctgcgctggaccgatgggcgcgagacgacgctgatgcagttgctggccgagggcacgcagtgcattgggctatggctggcgccgacacgcgccgaagcagaagcggcattggcagcgaccgcctcgcttcccttgcacttgctggccatcagcggcgacagcggcctgccgacgctgcaagccgacgatcggctcaccagccatctgggcatcggcgatccgggcggctttgtgctcgtgcgtcccgatgcctatcgcgcggcgctgctcgcgcaggccacccccgaatcgattgccaacgcgttgcgcacggcccttgcccggaacaccaccccatgaccaccgagccccgcatccccgaccccgacggtttctacgcagccatgctcaccgcgcatgaaggcctggacgaagcgcagagcgccgatctcaacgcgcgcctcgtgctgctgctggccaaccagtgcggcgaccaggacgtgctgctggcctgcatccgcgcggcggccgaagactcccccacaagcaaagccccatgaacgccaacgtctccttcgcctctgcctccgacacgcgcgagcagaaaccccgactgcgggaactcgcgcccggcgtgtacggctacatcagcgatttcgatccgaactgcggcttcgtcgtcggcgacgagcaggtggtgctgatcgacacgcgtcccacgccgcgcatggcgcgcgactttctcgcggccatccgtacggtgaccgacaagcccatcaagaccatcgtgctcacgcactaccacgcggtgcgcgtgatgggcgccagtgccttcgacgaggtcgaggccatcgtcgcgagcaacggcacgctcgactggatccgcacgcgtggacaggccgatttcgattcggaggtcggccgctttccgcgcctgttcgcgggcgtcgaggagattccgggcctcacgttcccgacgatgagcttcgagcgcgagatgagcctgtggctcggccctcgcccgggcctgggtcgcgagcttcgcctgatggcgctgggccgcggccattcgagcggcgacacggtcgcgtggctgcccgactgcggcgtgctgttctcgggcgacgtggtggagaaccactgcggcgtgtatgcgggcgacgcctacatcggcgactgggccggcacgctcgacgccgtgctggcgctgaagccgcgcgtgctggtgccgggacgcggcgcggtgctgcaggacgaagccgcttgcgccgaggccatcgggctcaccaaggcatttctcgggacgttgctgggcagcgtgaaggccggcattgccgccggcgaaacgctcaagggctgcttcgcgcgagcagaggcggcgatggcgccgcgcttcggcacctggcccgtgttccagcacgtgctgcccttcgacgtatcgcgcgcctatgacgagctgcgcggcatcgagcatcccgtggtgtggacggcagagcgcgaccgcgagctctggcagacgctccgcggcgaatgacccgcgaacgatttcaagacaagcaacggagacaaaagacgatgaagcgattccttcccctcctggccgcagccctcgcgctggccaccagccccattgcgtccgcgcagcagcaggcggcctacccgagccagcccgtgaaatggatcgtgccctacgtggccggcggcggcaccgacaaccttgcgcgcgcactggcggaggcgatgcagccgtcgctcgggcagccgctgatcatcgacaaccggccgggcgcatccaccaacatcggcgtgtcggtgctgatgcaggccaagcccgacggctacacgatcatgcaggccgagaacgcggcgctgctcttcaacgaacacatgttcgccaagctgccctacaagcccgcgagcgatttcacgtacatcggcaccatcggccgctttccggtggcgctggtcgtgcaccccgactttcccgcgaagaacgtggccgagttcgtgcgctacgtgaaggccaacccggagaaggtgagctacgcctcgccgggcaacggctcgccgcaccacatggcgatggagctcttcaagcagaaggccgcgatcagcatcacgcacgtgccctacaagggcgccgcgcccgccatgaccgacgtgatgggcggccaggtgccgacgatgatgctcgacctggcctcgggcctgccgatcatcaaggcgggcaaggtgcgcgtgctggccatcgcgctgccgcagcgcgccagcgcactgcccgatgtgccgaccttcatggaagccggcttcaacgacgtcaacgcctatgccttccacggcctgatcggcccgggcggcatgccgcccgacgcggtggcgcgcatcaacggcgaactgcacaaggcgatgaaggcgccgaaggtggcgaaactgttctcggaattcggcttcgaggcgctgccgggcacgccgcaggagttctataagctctcgcgcgccgaaagcgagcgctggggcaagatcatccaggccgccggcgtaaagctggattaaaagggccccccgcttttcactccgcttcgctgcgtgtaactccaccccccgagggggaggcgcggcccggcggcagccgccggctaccagccgagccccaggtgcaagggcaggtacaccgccatgcccgccagcatcgtgccgaacacgccgcgccgccagtagtaataagcggcgccgaccaccgcggcatacaagcgggcgtcgtgcaacgtggtgatcaggtgcccctgggtcatcacgatctcgggcgcgatcacgcccgcgagcgcggcggccggtgcgtagtgcaaggcgcggtgcgcccagtcgggcaggccccagggccggtcgagaatgaagaagaagcagcgggtgaggacggtgaccgcggccaggccgacgatcacgcccagcgtccacaggtcggtgcccctcacttgtcgtcctccgcgtcggggtcgagcccgaactgcttctcgagccagaagcacagcagcaccgccacaccgatggccaccacgatgttgagcttgagcggcaaggcataggcggccacggcggtgacgctggcaatcagcgcggccagcacgcgcagccgcgtggtcgccatcgagcagacgatcgccaccaggctcagcacgccggcaaagccgagtccccagttctgcggaatgaaattggccagtgcgatgcccaggaggctcatgcccatccaggagcaccacgtcacgaagtagttgccagtgaggtaggcctcctgggccttctgctcatcgccgacgagcggtggcgaggggtactttctcgtgaagagcgcgtagctgaggtcggccgtgagatagccgtgcgtcatgcggcgccagcgcggcatgtgcatgaggtacggccgcaggtgcaggctgaacaccacgaagcgcaggttgacgcaaaagcccgtggccaggatcacccaggccggcgcgcccgcgaacagcagcggaatggccgcaagctgggagctgccggcatagaccagcagcgtcatggccaccgactcgagcacgctcatgttcgacttgaccatggccacgcccgtcatcaggccccaggcgccgatgcccagcgcggccgacgacatgtcgcggatgcccgcgcggaactcgggccggcggcggatggcagcggacaggaacatcagccgaagcgctgcccgggcttcaggtcgaagccgcgcaggaaatcggccacggccaggcgcttgccgccgggacgctggagttcggtcgccatcacgatggcgccggccgccgccaccgcaacgccggcgtcggtcacggccaggagggtgcccggcgcggcagacacctcggccgcgaccgcgcgcgcggaccagagcttgatggtctcgccgtcgagtgggctgttggcgcccggaaagggatcgaacgcgcgaatgcgccgcacgatggcgtcggcgggctggttccagtcgatctgggcttcgtgcttttcgaccttgttggcataggtgacgccttcggccggctgcggcgtgcgcgccagctggccgatgctggccagcgcctggacgatcatgcggccgcccagctcggccaggcggtcgtgcaggcgggcggtgttgtcgccgccgatctcgaccgcttcgcgcagcagcatgtcgcccgtgtccaggccggcgtccatctgcatgatggtgatgccggtctgcgcgtcgccggcttcgatggcgcggtggatcggcgccgcgccgcgccagcgcggcagcaggctggcgtggatgttgaggcagccgaacttcggcaggtcgagcacccattgcggcaggatgagcccgtaggcggccaccaccatcacgtcgggcgcagcggccagaagggcctcgcgtgcggccgaggcatcttccgggtacttgccgtccagccgcaggctgcgcggctgcgccaccggccagttgtgggccacggcgcattgcttgatgggcgaagcctgcagcttcatgccgcgtcccgcgggccggtcgggctggctcagcaccagcgtgatttcatggccggcggcggcaatggcttcgagcgcgacgcgcgcgaactcgggcgtgcccgcgaaaacgactttcagcggggtcaatcgcggatccgatcgagttcgaggtcgtcccccgtgtgataacggcgaaccacgcctgtcgggtcgatgtagatatagagcatgcggcgctcgttcaccgccttgtagcgccaggtccagacggtgccgtcgaaggagctcacgcggctggtttcatagggccggccatagaaggcgagcacctcgttctggcgccattggtcgaccttgatgtcgtggccgaagcgcgcctcgttgagcacctgggtcacggaaacgaccttgcccgaggcatcgacgtcgatgtcggtgacctcgaaacccgccggcatgcgcgaatactggagccgctccccgccgccgttgagcggatagcggcccgtgggcgcacccaggcgctgcagcgtttcggccgccgtggtacccggaacgatgcgcgtgggttcgctggcgcagccggccaggacgacgacaagccccgcggccagaacggccacccagggccgcagggacggcatggtcacgcccggccctctttggcctcttcccgctgctgcttgagcagcttgctcttgatgcggttgcgcttgagcggcgacaggtattcgacgaacaccttgcccaggaggtggtcgagctcgtgctggatgcagacggccagcaggccatcggcctcgatggtgcgcatttcgccgttctcgtccagggcctggaccttgaccgacgtggagcgcatgacgccgtcgtagatgccggggaccgacaggcagccctcttcattcagcactttttcgtcgctggcccagataatctcggggttgatgagaacgatcggctcgttgcgctcctcggaaacgtcgatgacgaccagccgttcatgcacgtcgacctgggtcgcggccaagccgatgccgctggcgtcgtacatggtctccagcatgtcggcaaccagcgccttgatgcgcgcgtccacgccctgcacgggcttggccaccgtgtgcagtcgcttgtccgggtaactcagaatgattcgtttggccatgaaaaaggggaaaagttgtggctattttcgccaattccgcgacgcgatgagccgggatcgcctgaaaacgttgccctcccaagggcttcgggcgcagaattcgtagcaaattgtgagattcgtatgtgcaccgatactcggtgcgctcacccatccagacatgaaaaagctccgaaaccctgtccgccagcgcacgcctctcttcgccacgttggcagcccttgcagtgatcagcagcggcacgacggcctgggcgcaaagctatccagtcaccccgcagcagcgcgccacggcccagcagaccgcccagaacggcgttccgttgagcgaactggcgcccaatgcgcctgacgaatacacggtaaaacccggcgacacgctgtgggccatttcccgcctctacctgctgcgcccctggcgctggccggaactgtggggcatgaacatcagtgaaatcgcgaatcctcaccgcatctaccctggccaggtgctgtacctggacaagagcggtggccgtgcgcggctgaccatgcgccgcggcgcgggcggcagcggcgacggcggcaccatcaagctgtcgccgcgcacgcgcttcgattcgctggccggcatggcgctgcccacgctcaacccgagcatcatcgagcccttcctgagcgagccgatcgtggtggactccgacacgctgcagagcgcgccgcgcatcgttgccggcaacgacagccgggtgctgctgtcgcgcggcgaccgtgcctatgcgcgcggcaatgccgagacgccgctgctcgaaaccccgggcccgctgaagaacttccgcgtgttccgcagcgccacgccgctcaaggaccccggaaccggcgaaatcctcggctacgaggcgcagtacctgggcaaggcccagctcaagcgtggcgaatcgaccacggtcgagacccagaaggacaaggacgtcatcaccgtggtgccggccagcgtcgacatcatcgcggcgcgcgaagaaatccgcgccggcgaccgcctgctgccggaaccgccgcgccagttgctgagctacgtgccgcgcgcgccctccacgcaggtcgagggccggatcatctcggtctatggcaacgcggtgcagttcgcggcgcagaaccaggtggtggccatcaacaagggcacgcgcgacggcatcgacagcggccacgtgctggccatcctgaagaacggcgaaaccattctcgaccggaccggcgaacgcaaggagacgatcaagctcccgaacgaacgcatcggcctcctgatggtgttccggcctttcgaaaaggtgtcgtacgcgctggtgctcgaaattaccgacaccccgcgtgccggcgacttcctcgtcaatccctgacgctttcgccttcgcttggaacgcgctgaactcgctggctggctgcggctttcactgacgccgggcatcggcgacggtggcgctcgccggctgctggccgccttcgggctgccggagaaaatctttgcggagaccagcgcggcgctgcggcaagtcgtgtcggcggcgcaggccgatgccttgcatctggtgccctccggccttcaggcccagatcgaccagacttggcaatggctgcaacccaacgccgacgacggcaccacgacgcgccgcctggtgacgctgggcgacgccgcctaccccgcgtcgctgctcgaaatggccgacccgccgctgatgctctacgtgctcggtgcggccgccttcgacctgacacagctcgaaaacagcattgccgtggtgggcagccgcaacccgaccccccaaggcgcggccaatgcgcgcgcgttcgggcgcgcattgggtgaagcgggtttgccggtggtgtcggggctggcgctcggtgtcgacggtgccgcgcaccagggtgcgcttgacgcggccggcgacgccgtgcggcttgcgaccgtggccgtggtgggaaccgggctcgatcgcgtctatccggcgcggcatcgcgatctcgcgcaccgcatcatgttgcaggggttgatcgtgagcgagctgccgctcggcacgcccccgctcacgcaaaattttccgaagcgcaaccgcttgatcgccggcctggcccgcggcacgctggtggtcgaggccgcgctgcaatcgggctcgctgatcaccgcacggctcacctcggagcaaggcaaggaagtgttcgccattcccgggtcgatccattcgccgcaatcgcgcggctgccatgcgctgatccgccagggcgcgaagctggtcgagtcggtgaacgacatcctcgaagaactgcccgcgctgcgcgctgccggcggcgcggctgcgggtcttttcgagaatgcgagtgcgggcgatccggcctcctcctccgggccggagaatccgcttctcgaagccctcggcttcgatccggtgagcctcgacgcattgagcgcccgcaccggctggagcgccgccgcgctgcaggccaagatgctcgaactcgagctcgacggccacgttgcgcgcctgccgggcggcctttttcaacgagcggcagcggcataaccgctctttctctctctgtcaaagagaaagaaggggcagcgcacgaagctcgcgagcgagccaccggcttcggctatattgggcccatgttcgaagtgctcgtgtttgtctacgaaaactattggcgcggcgatgcctgccccgaacccgaacagctgggccgcaagctcagcgcgcacggcttcgaggcagaagaaattcgcgatgcgctgcaatggctcgacggcctgagccttgcaacgcaaggcttgcagttcgagcgcagcgcaatcgacgacgcggtcgccacggtcacgctgcggggcgcgcccgaaccggccctgccgcagtcggacaacgccatgcgggtctattcgcaggccgagcaggagcacctgggcgccgattgccttggcttcatccgctttctcgagtcgtcgaatgtgctgtcctgcggcctgcgcgagatcgtcatcgaacgtgccatggcggccccgggcgacccggtcgcgctcgacgaactcaagatcatcgtgctgatggtgcactggagcacgggcatcgagcctgacgcgctggtgctcgatgaactctgcgaaagccgcgagggccgaatcgcccactagttgggctagttcagcagtcgttccggattggcatccagcttggccagcgcctcgcgcgtcgcgcgcactgtgagggtttcttcctcggccggcaccagcaggccggcctgcaggtagttggccagccggccgacctggatcaggaagctgcggccgtcggccgttgcaaacaggtgcagttgcttgcggtcgctgcgccagacgaactgcacctggctcacgcgatcattgtggtcgagcatgaaccagttgcccacctccagctcatgggcccacgccagcatgtcttcggccggcgtgccgcccgcgatgtcggccacgacctcgatcgaggccgcgtcgatgcccagcagcaattcgatgctgttcgcgtcgagcggcaggctggatgcgccgccgtcgtcgctcacgaaatcttccaggtgcgccaggcgctcggccatggcttcgatcttggccgcgggaatggcttcggtcttggacaggaaggcatcagacaaggttgcgccgatggtcttgatgtgagcttcctgcggctcgtcgatgatgccgagcaggttcatgcccaggcgcaggcgctgcagcagctgcggcaggtcctggatcacgcgcgcacggtcggcgcggttgggcttggcgctcgcggcccacaccagttcggaggccacgcgcttgagcatcacggtctgctcgccctgtgcgccatagcgcaatgcggcaatcgccagcacctcggcccagaccttgaagaggaactcgcgtatctcttcgcgcaccggcatgtcgttgagcatcttgcgcagttcgatggtgtactggatcgccatcgtttccttctgctcgacctgctgcgccacgctcatgacgcgctgggtggcgtcgctctgcgtgagatagcggttcaggaaggcgacgaactcgtcgaacaccagcttgaacacgcgctggccggtttcggggtactgctcgatcacctgaaccacgcgccggatctcgccctcgagcgcgctgccggaaatggcggcggcgtcgaagcccatcacgcaggagcccatgcggtcgatcagcatgcgcgccggatgctgcagcgtgccgaagaattcgggctcggcaatggccacgcgcagcacaggcatctgcaggcgcgcaaaccagacacgcgccgagaaaggaatgcgctcttccgcgaggatggcctggaacatgagcgccacgatctcgaccgtggccttgtcggcggtggtgggcgcccttttcttgagctccgcgctgcgccgccgcaggtcgaccgaggcctgctggatgacggtcgcctgctccgcggagccttccatgtactgcgtggcggccatccggtaggcgacttcggcttcggcgatgagccctgcaaaggtcttggaagccgcgcgcgaagaaccgtcgccggcgccggccggtccggcacctggcacgcgtccatccattcccgtcgtcgtcggggaggaggaggcgttcggcgcttccgcgccaatgcgggcggcaacgaagcgcttgaggctcaggagcgccgtctgcgcacgctggcgcgcgaccatcaagggcgaaccgccggtggtcgcggccggcacggaaggagcaaaggcccgcggctgcgacagcgcatcgaagccttgctgccgatgcacggcgccggtggcctggggtgcgcccgcgttctggggggcgccgggcgcgtaagggggcgcgggcaccgtcgacggtccgccgccggaagcgccggtgcgccggacaaagctcttgagatcgatttccggcatcacgcctttggaaatcaggaacgcgttggcgtcttcgtaagccttgacgaccacgccgacgagatgctgctgcacggtgtcctgcacccgcgcccacagggtgcggctcaagcccgccgccagccactggtcgaccagcagcttggccatgctttcgggccggagcacgtcgtgggcgtccagttcgctggaaccttccaggtgctggatgcgcagccgaaggtcgctgagctcgaagctggccttgtcgtggatcagctgcgccaggcgcgacgacagaatgctgctctccatcgcgtcgtcgtcgatgagttcgagccgcagcttcgcattggatgacgcgcccggcaccgcgcccggcgcatcgaccgccttgcgccagcccgtttgcgcgagcgccacccattgcgatgcctggccctggaaggccacgaaatcgtcgcggctctcctgcatggcgcgtgcattgcccatctccgaagcctgctgcgtcaggcggtcccggatggcttgcgccaacggggcgatcacgcccccggtcgccagaacgaagcgctcgcgcgtctcgcgtgcgagctgcaaagaagaggcggaccgcgcaatgctcattgaaggatcgggaagaccagtggggctccgtgggtgggcgatgaccgcgagcttgcatccggaaatgcaaccgcacaagtgtgcatcagctccgtcattctcgctggctccggcggcgcgttcctctcgaattcgatcggggtcagaccaccgcgccggcgttcggatcgtccggtccgccgtcgcgcttgaccgggcccttgacgagatcttcgcgcttgacgccgagccacatggcaatcgccgcagccacgaaggccgacgaatagatgccgaacaggatgccgatggtcagcgccagcgcaaagtagtgaagcgtcgggccgccgaagaagaacatcgagagcaccaccagctgcgtcgagccgtgcgtgatgatggtccggctgatggtcgaggtgatcgcgttgtcgatgatctccaccgtgttcatcttgcggtagcggcggaagttctcgcgcacccggtcgaagatcacgaccgactcgttgaccgagtagcccagcaccgccagcaccgccgccagcaccgcgagcgagaactcccactggaagaaggcaaagaaccccaggatgatgaccacgtcgtgcaggttggccagcacggtggccacggcgaacttccattcgaagcggaacgccaggtagatcatgatgcccaccaccaccatgcccagggccttgagaccgttggtggtgagctcgtcgcccacctgcgggccgacgacctcgatgccgcgctgcgtggccgacgggtcgaccgccttgagagcctgcatcacctgtgcgctctgctggtcggagttcatgcccttttgtgccggcaggcggatctgcacgtcgcgcgaggtgccgtagctctgcacctgcacgtccggatagccgagcttgccgacggcctcgcgcaccttgccgatgtccgcggactgctggtaggccacttccatcacggtgccgcccgtgaactccaccgacaggtgcagcccgcggtgcagcaggaagaacaccgccagcgcgaaggtgacgaaggaaatgatgttcagcaccagtgcgtggcgcatgaacgggatggtcttgtggatgcggaagaattccatggcgcttgtccttgacctttacttgccttcggccacggccgtgccgtcggtcttgggccgccaaaccgtgccgatggacaccgacttgagctttttcttctggccgtaccagaaattgacgaggccgcgcgagaagaacacggcggagaacatcgaggtgacgataccgatgcagtgcaccaccgcaaagccgcgaatcggacctgagccgaaggccagcaaggcgatgccggcaatcagcgtggtcacgttggagtcgagaatcgtgccccaggcgcggtcgtagccggcatggatggccgcctgcggcgaagcgccgttgcgcagttcttcgcgcacgcgttcgttgatcagcacgttggagtcgatggccacgccgatggccagcgccatggctgcgatgccgggcagcgtgagcgtggcctgcagcatcgacagaatggccaccagcagcatcaggttgacggccagcgcgatcgacgagaacaggccgaacagcgcgtagtaggcgcacatgaacaccatgatggccaggaagccatacatcacgctcttgaagcccttctcgatgttgtcggcgcccaggctcggaccgatggtgcgttcctggatgatttccatcggcgcggccagcgagccggcgcgcagcagcagcgcgaggtcggcggcctcgaccacggtcatcgaacccgaaatctggaagcggttgcccagctcgccgttgatcgacggggccgtgagcacctcgcccttgcccttctcgaagatcagcatggccatgcgcttcttgaagttctcgcggctcacgtcgcgcatgatgcgaccgcccttggcgtccatggtcaggtcgaccttgggctggttgctctgctggtcgaagccaggctgcgcgtcggtcaggttttcgccagtgacgagcacctgcttcttcacgatcaccgcgcggccgttgcgctcgaagaatttctcggagccgaagggcaccggcccgccgctcagttcggctgcgcggccttcggcgctctcgtcgaccaggcgcatttcaagcgtggccgtgcggcccaggatgtccttggccttggccgtgtcctgcacgcccggcagctgcaccacgatgcggtcgagcccctgctgctggatcaccggctcggccacgccaagctcgttgatgcggttgtgcagggtggtgatgttctgcttcagggccgcgtcctgcagccggcgtgcggcctcgggcttgatggtggccgtgaggcgccagacgttgccgtcctggctgtcggtggtcgtgagatcctggaactggtcctggatcagctgcttggcggtttgcagcgcggccgcgtcgcggaacgaaacctcgatcgtctggccgttgcggttgaccgacgtgccgcggatacccttgtcgcggaaggtggtgcgcaggtcgcccgcgaaggattcggccttcttgtcgatggcacccttcatgtcgacctgcagcaggaagtcgacaccaccgcgcaggtcgagacccagatacatcgggaacgcatgcagcgccgtgagccaggccggcgaccgcgaaaccaggttcagcgccacgacgtaggaagggtcggccggatcgggcaccagtgcgcgctgcaccgcatcgcgcgccttgatctgctcgtcggcggtggcgaagcgcgcgcgcagcgagccgccctcgagcgtgaacatgtcgggcttgaccccggctgtcttcagcgcctcctcgacccggccctgggttgccgcgtcgaccttgacggtcgacttggctgcggacacctgcacagcaggcgcctcgccgaagaaattggggagggaatagatcaaccccacaagcagcacgatcacgatgatcgcgtacttccagaccggataacggttcatgagaaagcgcttttagaaacggaacaccgcgtgacttgaggccttgcgccaggaagcgcaaggccgggtcgcgctttgattttgattactgcttgacggcgcccttgggcaggacctggaccacagcgctgcgctggatcttgatttccacgccattggcgatttcgaggccgaggtactggtcgccgatggaggtgatcttgccgagcacgccgccggcggttgccacctcatcgcccttggccagggcttcgatcatggcgcgggcctctttctggcgcttcatttgcgggcggatcatgacgaaatacagcaccacgaacatgaggaccaggggcagcatgctgccgagcgaggacaacatgtcgccaccgccggaagcagcgggcgcggtttgggcgaaagcagaggaaatgaacaaaagagtctccagcagagagaagaggaatgtcagaagcgcgagccgggcccgcggttccgcggccctgtaaaaaagggccgcgaaccagcgcttgaagcggcatcggccgcgaacagcaccgggcattgtattcgtggcaacgccccgcgctccgcgcttatccggcgcggagggcagggctttccaggggcggcaggcgcgcctcggctgctcttctttgaatagcggctccgcaagcgggccggcggctcgaggggcgttctttcagaatctcaggcggccgagcgctgggcctgttgcgggttgcgccacttggcgagcaggtcgctccagcgggtgcgggcggccgccaggttgcggtccttcacgtggccgtagccgcgaatctgctcgggcaggctcgcaatctccagcgccagggcgtggttcccggcgttgaggccggaaacaacctcctcgatggccgcgcggtactcgccgatgagcgcgcgctcggtcttgcgctcttcggtgcgcccgaagatgtccaacgccgtgccgcgcaggcccttgagccgggccagcagcctgaatccggtgagcatccaggggccgaacttctgcttttgcagttcgcccttgccgttcttcttcgcgatgatgggcggcgcgaggtggtagttgagcttgaagtccttgcccatctggccctcgaacatgccttcgacccggtcgaggaaggcgcggtcggtgtgcaggcgcgccacctcgtactcgtccttgtaggccatgagcttgaacaggtagcgggccacggtttcggagagcgcggtcttgcccagcaccgattcggcctgccgcaccttgcccacgaactgccggtactcgtcggcataggctgcgttctggtagcccgtgaggaattcgacgcggcgcgcgaccaggctgtcgacggtttcgcgcttcttgaattcgaccacctggcccgggcgcacgcgcttttgcaacgcggccggattcgcggccgcctggcggccccatgcaaaggcggccttgttgttgtcgatggccacggcgttgagctcgatggcgcgcatcagcgactcgagcgccagcgggatccagcccttttgccaggcaaagcccagcagcatcggattggcgtagaggctgtcgcccatcaaagtggtggcggcggcatcggcgtcgaaggtgccgagcgcatcggtgccgacgacacgcgcaatctggttcgcgcagtcgtcttgcgggttgacccagttggcgttgcgcacaaaagcggccgtgggcgtgctgtgcgtgttgagcgccacgtgggtgcggccctcgcgcatgcgggccagggtttcggcgttcacggccaccagcggatcggccgccaggatcaggtcggccgcggcggtgccgacgcgggtggtgcggatcgcgtcctgcgattcgccgatcagcgcatggctccaggtggcgccgcccttttgcgccaggccggccgcgtcctgcgtgacgatgcccttgccttcgatgtgggccgccatgcccagcagctggccgatggtgatgacgcccgtgccgccgacaccggccaccacgatgccccagacctggtcgcgcgccagcgccggcacggccggttcgggcagcgggccgagctcgagcggcgaatcggccttgttcctggactttttcttgagctgcccgccttcgaccgtgacgaagctggggcagaaacccttgaggcagctcatgtccttgttgcagctgctctggttgatggtgcgcttgcggccgaactcggtttccagcggctcgaccgacaggcagttgctctgcacgctgcagtcgccgcagccttcgcagaccaggtcgttgatgaccacgcgcttggccggatcgacggccgtgccccgcttgcggcggcggcgcttctcggtggcgcaggtctggtcgtagatgatggcggtggtgccggccatctggcggaactcgcgctggatctcgtcgagcaggtcgcggtgcttcacggccacgtggtcgccgggaatgttcacgccttcgtacttctcgggctcgtcggtgacgatgacgaccttcttggcgccttcggcatgcaggctctcggcaatctgcagcaccgaatggccctcgggccgttcgccgacctgctggccgccggtcatggcgaccgcgtcgttgtagaggatcttgtaggtgatgttcacgcctgcggcaatgctctggcgaatggcgagaaggccgctgtggaaatacgtgccgtcgcccaggttcgcaaagatgtgctggtcggtggtgaagggctgctggcccacccacggcacgccctcgccgcccatctgcgtgaagccaatggtggagcggtccatccaggtcgccatgaagtggcagccgatgccgcccatggcgcgcgaaccttcgggcaccacggtgctggtgttgtgcgggcagcccgagcagaaccatggctggcggtcggcgccctgcacgccgcccaccttgagcacttccatcgagcgctccttggcttcgaggatggcgatctgcgcatcgatgcgcgcatgcatgtcggcgccggcctggtccaggatgccgagcttgcgcaggcgctgtgcaatggccttggcgatcagcgccgggttcaggtcggcgttggcgcgcagcagcgtgttggcggtggggttgggcatggcccattcgccgccggagaaatcgccgtccagctcgttgaacttgcccagcacggtgggccgcacgtcggcgcgccagttgtagagctcttccttcagctggtattcgatgacctggcgcttttcctcgaccaccagaatttcctgcagcccggtggcaaagtcgcgcgtgagctgcgcctcgagcggccacaccacgcccaccttgtgcagccggatgcccagctggcggcaggtggcgtcgtccaggcccaggtcgatcagggcctggcgggtgtcgttgtaggccttgccgctggccatgatgccgaagcggtcgttcgggccttcgatcacgttgtggttcagccggttggcgcggatgtaggccagcgcggcataccacttgtagtgcatgaggcgcgcttcctgctccagcgcatggtcgggccagcggatgtgcaggccgccgggcggcatctggaaatcggtgggaatgacgatctcgacgcggtcggggtcgatcatggccgtggcgctcgactcgacgatctcctggatcgtcttcatgcccgaccagacgcccgagaagcggctcaaggcaaaggcatgaatgcccaggtccaggatttcctgcacgttggtcggaaagaacaccggcgtgccgcaggccttgaagatgtggtcgctctggtgcgccgccgtgctgctcttggaaatatggtcgtcgcccgccaccgcgatcacgccgccccattcggtggtgcccgccatgttggcgtgcttgaagacgtcggagcagcggtccacgcccgggcccttgccgtaccagatgccgaagacgccgtcgaacttgttggtgcccgcgggcgagaagcccagctgctgggtgccccacagggccgtggcggcgagctcttcgttcacgcccggctggaagacgatgttctgttccttcaggaacttgctggccttccacagcgcctggtcgtagccgccgagcggggagccgcggtagccactgatgaagcctgccgtgttcttgccggcctgcttgtcgcgcagtcgctgcagcatcggtagcttgacgagcgcctgaacgccgctcatgaaagcgcggccgtagtcgaggctgtatttgtcgtcgagcgtgacggtttccagcgccttgcgaatgtgctcgggcagcggtgcgttcatgtgtctgtctccgtttggcagggcctggtgggcctggctgatggggtgtgggtctgtgcccgggtagggcgcgagcccatgatcacgcaaagtgtatgccggggtgcgcgacaggtgtttgcgttctttgcccctaaaaaccggctttcagaaagaatcttgcttaagatcgatccttatggaaagcattgacaagttcgaccttgcaatcctgcaagaactgcaggccgacggccgcctgaccaacgccgagcttgcgcagcgcgtggggctctcggccgcgccctgctggcgccgggtccgcgcgctggaagaagctggcttcatcaagggttaccgcgccgagatcgaccgccacaagatcggacttggcgtgctcgctttcgtgcgggtggacaccgagcgcgtcaccaacgaagccacccgcaagctggaggaggcgatccgcaagatgcccgaggtggtggcctgccactacatcagcggcaccggaaccttcgagctgcaagtggtggcacaggacctgaacggcttctcggccttcgcgcgccagcacctgatgaacctccccaacgtgaaagacctgcacaccagcttttcgctgggcgaggtgaaggcgagcagcgcgttgccgctcgggcacctggcacgctagcggcatcagggccgttgcccctccctgcgattgccggttttgcgaccggtttcgatggcatcggcacaattggggcacatgccaccgatatcgcccgaagagacacccatcccccccacccggccgcagccaccgaaattcgcggcgctcgtgccgctcaagctgcctgtgttccgcatgctatggagcacctggctcatcgccaacatctgcatgtggatgagcgacgtggcggcggcgtggatgatgacctcgctgaccacctcgcccatctgggtggcgctggtgcagtcggcctccaccttgccggtgttcctcttgggcctgcccagcggggcgctggccgacattctcgaccgccggcgctggctggtggccacgcagttctggctggcgggcacggccatcgtgctgtgcgcggccattgcgctggacatgatgaccgcgccgctcctgctggcgctcactttcgccaacggcatcggcctggcgctgcgctggccggtgttctcggccatcgtgcccgagctggtgccgcggccgcagctgccggcggccctgggcctcaacggcatcgcgatgaacgcctcgcgcatcatcgggccgctcacggccggcatgctcatcgccagcgcgggcagcgtctgggtgtttgcactcaacgcggtgctttcggtcgcctcgggcttcgtggtgctgcgctggcggcgcgagcacaagcccaatccgctgggccgcgagaagctcatcagcgccatgcgcgtgggcgtgcagttcgtctggcagtcgcagcgcatgcgggcggtgctctcgcgcatcacgatcttcttctttcactccacggccctgctcgcgctgctgccgctcctggcgcgcaacctcaagggcggcggcgcgggcaccttcacgctgctgctggcggccatgggctcgggcgcgatcatcgcggtgctgttcctgccgcggctgcgccaggcgctggggcgcgaccagctggtgctgcgcggcacggtgctgcagtcgctcgccaccgcggtgatggcctttgcgcccaacgcatggatcgcggtgcccgcgatgttcttcggcggcatggcctggatcacggtggccaactcgctctcggtgtcggcgcaactcgcgctgcccgactgggtgcgcgcacgcggcatgtcgacctaccagatggcgatcatgggcgcgagcgcgatcggcgcggcgctctggggccaggtggcgaccgtcacgtcgctctacctgagcctcgccatcgccgccgccagcggcacgctgctgatgctggtggccctgcgctgggtgaccgacggcgtcggcgaagacgacacccgccccgccgaagccggctgggccgccggcccgccggccgaggcgccgcaggaagacggccgcgtggtgatcacggtcgaatacctcatcgagccgtcgcgcgccgcggccttccacctcgtgatgcagcagacgcgccgcgcgcgcctgagccagggcgccatcggctgggagctgctgcacgacatcgggcagcccagccgctatgtggagcagatcgtcgacgactcgtggaccgaccaccttcgccgcttcaaccgcgccacggccagcgacatggcgctgcgggagcgccggctcgcattccacatcggcgaagcacagcctgtcgtcacgcgctacatcgtgcggcgctgagcggcccgccaggccgtcagtggaagaacagcagccgcgtcaggaaggtatggccggcctcctccgccatgagccagaccaggaccagcaggcacaggggcggcaccaggatggcatagaccagcgacagccgctcccacgccatgtgcatgaagaccgcgacgatcagacccgccttcagcaacatgaaggtgatgatcaggctccagcgcagatacccctcgaaatggaagtagtcgaccatgtacgacatcgcgctgagcacgaacagcagcccccagatcttgagatagaggctgatcggatgttgttggcctgtgacggagttcatggtcgtcctcaccagagatagaacagcgcaaagatgaacacccacaccaggtccacgaagtgccagtacaggccggcaatttcgacgatctggtagttgccgccgcccttgtcatagtcgccgcgcaacagcttgaaggccacgacaaacaggaaaaccacgccggccgacacgtgcagcccgtgaaagcccgtgatcatgaagaaggccgagccgaattgcgccgcgcccatcgggttgccccagggccgcacgccctcttcgaggatcagcttggaccactcgaaggcctgcatgccgacgaagagttcgccgaaggtcgcggtcacgagcatgagcgtggcggcgttcaggcggtcgccgcggtaggcgaaattgacggccatggccatcgtgccgctgctggtgatgagcacgaaggtcatgatcgcgatcagcagcaacgggatgtcggcgccccccacgtggagcgcgaatacctcgctcggattgggccacgacgcggtggtcgagacgcgcaccgtcatgtagccagtcaggaagcagctgaacacgaaggtgtcgctgagcaggaagatccacatcatcgccttgccccacgagacgtggaacgcctgacggtcggaagaccagtcggaaatcagcccgcgccagccactggcggcgatctcgggagtcaacggcgttgctgcgacggttgcggtgttgttcatgaaaaacgcctcctcaggatgtgccgcagatgaagcgcgccacctccggcgtcacccagcccagcagcccgaacagcaccagccacaccgccagcatgaagtgccagtagcgcgcgcacagcgcgatgcgccaagcggcccgggcagggtcgggccacgcggcgcgtgccgtccatgcccagccggccagcccacccgccaggtggagcccgtgcatggcggtcaacagatagaagaagctgcccgccggattgccggccggcatcacctgtgcgcccagcagcgcctgccaggcccacagctgcacgcccaggaagcccactgcgcaaaggccgccggccagcagcaggcgacgggcccgcatcgggtcgaggccgcgcgatgcgttaccggcccattgcagcgccacgctgcccgccacgagcagcgccgagctgagccagagctgccacggcagtgcgatcgtgatcgcgtcgtcgccgctcatgcgcatcacgtaggccacgatgaagagggagaacaacgcggtggccacgcccatgaagacccacaggccgatgctggccgcgctcgcgtgggcatcgcgagggcggccgccgcgctccgcaccgtggagcgcgcctgccagggagcggcccagcgctgtgctcatgccggtgctccccggacctcgctctggccctccggctcgggctcccctgccgcgggcttcggcggtgtgttctgcggaatgaaatcttccgtcgcacccggctcgccataggcataggcccacctgtagaccaccggcagctgcgggccccagttgccgtgacccggcggcgttgcgggcgtctgccattcgagcgacgcggcgcgccatggattggcgtcggccggctggccgcgccaggcactccaggcaaggttgaagatgaacagcaactgccccacgccgacgatcaaggcgaccacggtgatgaattcattcatggtgaatgccgacggcggaatgaagtcgtagccgtcgaagttgtagtagcgccgcggcatgcccagcacaccgaggtagtgcatcggaaagtagatcgcgtaggtgccgaggaaggtgatccagaaatgcagccggccgagccggtcgtccagcatgcggccggtgaccttggggaaccagtggtagatgccgccgaacaccaccaagagcggcgccacgcccatcaccatgtggaagtgcgccaccacgaagtaggtgccggacagcgggatgtccacgctcacgttgcccaggaacagcccggtcagcccgccgatgaggaaagtgcacaggaaggacagcgcgaacagcatcggcaccgtcaggtggatgtcgccgcgccacagcgtcaggagccagttgtagaccttgatcgcggtgggcaccgcgatgatcagcgtggtggtcgcgaagaagaagccgaagtacgggttcatgccgctcacgaacatgtggtgcgcccagaccaccacgctgagtccgccgatggcgatgatggcccacaccatcatccggtagccgaagatgcacttgcgcgcgtgcacgctgatcaggtcggagacgatgccgaaggccggcagcgccacgatgtagacctctggatggccgaagaaccagaacaggtgctggaacagcagtgggctgccgcccttgtagcctgtcacctggcccatcgacaccagcgccggcatgaagaagctggtgcccatcgtccggtcgagcagcagcatcacgccgctgacgaacagcgccgggaagccgagcagcgcgaggatggtggccacgaagatgccccacaccgtgagcggcatgcgcagcagcgtcatgccttcgcagcgcgcctgcagcacggtggtcacgtaattgaggccgcccatcgtggttgccacgatgaagatcaccagcgacaccagcatcaggatgatgcccccggtatggcccggcgtgccgggcaggatcgactgcggtggatacagcgtccagcccgcacccgtggggccgcccgcgacgaagaagctcgccatcaggaccaccaccgacagcaggtagacccagaagctcagcatgttgaggtaggggaagaccatgtcccgcgcccccaccatcagcgggatcaggtagttgccgaagccgccgaggaacagcgccgtgagcaggtagatcaccatgatcatcccgtgcatggtcacgaactggtagtagcgctccgcgttgatgaactcgaactggcccggaaagccaagctgcagccgcatcaggttggacaggaccacgcccaccacgcccaccgcgatggcggtacaggcgtactggacggcgatcactttgtgatcctggctccagacgtagcgggtcagaaagctctgcggcgcgggatgcccggcgtcgtcgtcgtgggtcacggcgtgccccgtgggtgaaggagtgttcatcgcggcgccttctgttcggcggcagcctgcgccggcgggctgcccagactctggatataggccaccagcgcggccagctcttcttcgctcaactcgaccttgggcatgacgggcggaaagcccttcacatggcgcgcctgcgggtcgcggatgaagctgcgcaggaaggcttcgtcgaccagtgcggtggaaccgtccgccatgttttcggtcttgccgtacagccccttccaggtcggtcccacgcgcgggctgccgtcgaccgtgtggcaggccacgcagcccttgctgtccgccagcgcgcgtccctgctgaacgcgtgcgtcgccgcccgccgccacggcaccggccggggcctcgggcgccttgatctgcgacttggcaaaggtcggcagcgccgcctgccaggccccgtaggccgccgggtcctccaccaccacgtggccgcgcatgttcggatgccccacgccgcacagttgcgcgcaaagcgcttcatagcggcccgcgacggtcggcgtgaaccagaagcggctgacctgccccggcaccgtgttcatccgggcgcggaagttcggcacgaagaaatcgtgcagcacgtcgtgcgagcgcatcagcaccagcaccggcttgccgagcggcagatgcacctcggtgccggcgatcagcagatcgtcctgcccggcccggtcggcggggtcgatcccgaacggattggtggcgctgaagaagcgcgcatcggtcgcgcccagcttgccgtcctcgcccgggaatcggaagcgccattgccattgctgggccagcacctccagcacgagcgcatcgcggggctccctgacatagttcgcgtacaccaggagaccgggcgccagcagcgccatgatggcgacggtggtgccgccgatcagccagcgctcgagcttcctgttctcgggctcatatgccgcgcggcgccccgcgcgatggcggaagcgcaccagcatgtaggcgatgaacacgttgatgacaatgaagaagatgcccgtgatcgccagcgtgatgccgagggtgtcgtccatcagcttccagttcgaagcaaggggcgtcgtccaccacggattgaaaacgtgaaacagcaccgagccggccacgatgagcaacagggcaacggccatggtcatgtgcgcttcctcggctcggcatgggctcggggctcattcgcgcttcagaggagagccgggacttggggctcttcaccctcgaaccgggcttcgggatgcgcggactgcagcagcgcctcgatctcccgcacgcgcgcacgcggcaggtccaccatcagcaggatctgcccctgtgcgatggcgccctcgaaacgttgcagcctggggctcgggatggaaatgccgaccatgctggccgaccaggcgccgaccacgccgcccaggagggccacgaacacggccacctcccattcggggtcgtcgccgatgatcggaaacatcagcgcggccaccaggccgacgacgatgccgcaggcactgccgagcacccacccggtcttggctgcgtggacgaggtcggaggtttgccatacgttggccgcgtggagcccggccatgtccaggccttccggtccggcgaaatggatgtgcgccacgtcgacgcgcgcccggaccagatcgtccatcgcccgcctggcgctcgccaggtcgggcatcaaccagtagatgcgtctcttcactgcatccccctttcgtcttgcgacgagtcaaggaaccatgaacgacttatatgcccaaggagggccgccatcaagtaggtaccgcatttcaggcggcagcggcacggggtaaccgccatcccacctttttttgaccgaacggataatttagctcatcatccgctccttattgcccgtcaccacgaggtacgccacgatgaacccggtccccttgcgcagccgcttctggtccgacctgaccagcgaagagttctcccgcctcgaccgcgaacggctcatcgccgtgctgccggtgggcgccaccgagcagcacggtccccatctgccgatgtcgaccgacacggccaccatcgacggcatggtgcgcgccacgctcccgcacctgccccccgacctgccggtgctcttcctgccgaccgtgccctacggcaagagcaacgagcattcgcgctacccgggcacgctcaccgtctcggccaccacgctgatctcgctgtggaaggacatcggcgcctgcgtggcgaaggccggcgtgcgcaagctggtgctctacaacagccacggcggccagatgagcgtgatggacatcgtggcacgcgacctgcgcgaggaacacggcatgatggtcgtcgccgccaactggtacacgctgggcctgcccgaagggctcttcaccgcgcacgagggcaggcacggcatccacgctggcgacctcgaaagctcggtgatgctgcacctcacgccggacttcgtgcgcaaggaccagttccagaacttcagctcgatgaccgagcaactggcggccgagaacaagttcctctcgatcacgccgagcggcaagctcggctggcagatgcacgacatcaacccctcgggcgcggccggcgacgccacgcgcgccacggccgaaaaaggtgccgcggtgctcgaccacgtgggccggcgcttcgtcgaactgctgcacgaggtcgaccgctttccgctctcccgcctttccaacgagcccgcctggaaatgagttccgaactcacgccaccgctggtcagcctgcgccacgtcagcaagcgctttgccaacggcacgctggcgctgcagggcatgacgctcgacatcggcgagcacgacttcatcagctttctcggcccttcgggctgcggcaagagcaccgcgctgcggctgatcgccgggctcacccggctcagctccggcgagatgcagtggtccggcgccaacaccggaaagacccgaagcgaccgcgacctgggcttcgtgttccaggagcccacgctcatgccctgggccaaggtgttcgacaacgtgtggctgccgctcaagctggcgggacagagccgcgacgcggccgcgcccgtggtgcggcaggtgctggagatggtgggcctctcgcgcttcgccgacgtgtatccgcgcgagctgtctggcggcatgaagatgcgcgtgtctattgcgcgcgcactggtcacgcacccacgcctcctgctgatggacgagccctttgccgcgcttgacgagatgacgcgcatcaagctcaacaacgacctgctggccatctggcgcgagcaccgcttctcggtggtgttcgtcacgcacagcgtgtacgagtcggtgtatctgtcgaaccgcatcgtcgtgatggcggcgcgcccgggccgcgtgatcgacgagatccgcatcgacgaaccctatccgcgcggcgaggactttcgcacctcgagccgctacaacgcgcactgcacggcggtgtcgcggtccctgcatggagcgctgcatgacatcgatcactgagcccgccgtgccggcagaggttccgatggatgcggccgacgtcgcgccctcggaagcgatgctgcgcgcgcacgaagacaagctgcgccggcgcgagtcgatgctgcgcatcgcggtgccggccggcatcgtcatcgtgcttctgctggcgtgggaatggatggttcgcgccaacaacattccgcactacatattgcccgcgccctccctcatcctgcgcacgctgttcgacaactggggctcgctctccagcgcgctgtggttcaccgtcaagctcacgctgctcgcgctcggtgcggccatcgtgggcggcgtgctgctggcaattgcgttcgcgctcttcaagtgggtggagatcggcctcttcccgatcgcggtgatcctgcaggtgacgccgatcatcgcgattgcgccgctcatcttgatctacgtatcgagcaccacggcggcgctgctgctgtgcgcgtggatcgtcgccttcttcccgatcctgtcgaacaccgtcatcgggctgaaaagcgcggacagcaatctgcgcgacctgttccagctctacaaggcctcgccgtggcagaccttccgctaccttctcgcacccagcgcgctgccgtatttcatggcgggcctgaagatcgcgggcggcctgagcctgatcggcgcggtggtggcggagttcacggccggcaccgcgggcaaggagaccgggctggcctcacgcattctcgaatcgagtttccgcaccgagatcccgatgatgttcgcggcactgctgctggtgtccctgctcggcatcgtgatcttcatcgtgttcgccgcgttgtcgcggttggtgctcggccactggcacgagagcgagatgcgccgtgaacgctaggaccatcgtgcctgcggtcgattgggacgccgtacgcgcggacctgcgcggcctcaacctgattaccgcgcccagccagcgcaagcagctctccaaggacttctactggtacagccccatcctcacggcgcagctcgcgggctgcgtggccgacctcgtcgtcaaggtcagcactgaagacgacgtgcgccaggtcgccgccacggccgcgaagtggaagctgccgctcaccgtgcgcgcgggcggcaccggcaactacggccagtgcgtgccgctcgaaggcggcatcgttctcgacgtgacgcagatgtgccgcgtgctcgacatccagccgggccgcatccgcgtcgaggccggtgcgcgcatgcacgacatcgacctcgcggcccgcgagaccgggcaggcgctgcgcatgtggccctcgacctggcacgtggcatccatcggcggcttcatcgcgggcggcttcggtggcatcggctcgttccgccacggcatcctgcgcgacccgggcaacctgctgcgcgcgcgcgtgatgaccgtggagcgcgagccgcgcatcatcgagctgcacggcgacgagatccagcaggtgcaccacgcctacggcaccaacggcgtgatcctcgacgtggaagtggcgctgagccctgccgtcgaatgggtgcactgcacggtgctgttcgagacatactgcggcgcgctagccttcgccgtcgcggcgcaggcgcccacgctcgacatcttcctgctgtccacggtcgaggcgcgcttctcgccctactacacggcgatgcacgaccgctttccgatcgaccggcacgcggcgttcaccatggtctctcccgattcgatggccgacttccgcgcgctcgccgccgcgcatggcggcaccctctccgtcgcgggcaccgagcccgagctgctggcagagggactgccgcccgcctacgaatgcgcgttcaaccacaccacgctgcaggcgctgaaggccgaccgcggctggacctacctgcaggtggcctacgcccagcccttcgatccttcggtggtcgagcgccatctgcggatcttcggcgacgacgtgctgcagcaccaggactttgcgcgcgccggtggcgagtgcggcaccttcggcatcctgctggtgcgctggaagggcgaagcccaccagtacgacgtgatccgcgaaatcgagtcgcagggcggctgcaagatcttcaacccgcacgtcgtcaccatcgaggacggcggcatgaagaccatcgacacgcagcagatcgagttcaagaaacgcagcgatccgatggggttgatgaaccctggaaagacgcgcggctggacatccgacatggctgtcgagcgttgaaatgaagccttgctttgtcatccgtcgcgatggttctgaacgctgttgttcgtggtgcgctcccgccgacggggtaccttgctccgcgaatgtcccccggcctgcggcctcctcctttatttcgctgcgcaaggcaccccatcgacgggagcgttgttcagagcggtcgttgatcagccagcacaacgacggcgctcggcgtgcacagggcgccgggtgctccccgcagcgaaataaaggaggaggcgaagccgggggacattcgcggaggggagtacccggtggcctgtgcacgcgccctgaacaacagcgccctgaacagaacacaagcgccccaaaaaacacgccctcaaaaagtccgttccatcacatgatcgacggcgacatgaaaatcccccgcagcattcaacccaggagtccactgccatgcgcgttcccgctctgaccatccgtccgcttgctctcggccttgccctcgcagctgccgccttcgccgcgcaggcgcaggaaaaagtggtatttgccaccaactggaaagcgcaagccggacacggcggcttctaccaggcgctggtggacggcacctacaagaagtacggcctggacgtcgatatccagcagggcggcccgatggtcaacaaccggccgatgctgccggccggcaaggtcgattttctgatgaccggcaacctgctgcagtccttcgacaacgtgaagaacggcgtgcccacggtggtggtcgcggccttcttccagaaagatccgcaggccatgttcgcgcatccgggccagggctacgacaccttcaaggacatggccaaggcgcccgtcgccttcatcggcaaggacggccagttcagcttctggcagtggatgaagtcggagcacggcttcaaggattcgcagctcaagccctacaccttcaacgtgggcccgttcctggccgacaagaagtccattcaacagggctacgccatctcggagccgctctcgatcaaggcgcaggccggcttcgacccggtggtgcaactgctggccgacaacggcttctcgacctactcgaccaccatcgagacgcgcgccgacctggtcaagaccaagcccgaaaccgtgcgcaagttcgtcgaggcctcgatcatcggctggaacaactacctctacggcgacaacaaggccgccaacgaaatgatcgccaagatcaaccccgactcgccggttgccgcatcgctgggctccatcgagctgatgaagaagatgggcatcgtcgacagcggcgactcgctcgccaagggtatcggcgccatggacgaagcccgcgtgaaggacttctacgacaagatggtgaaggccggcctgtacaagccgggcgagatcgacctctccaaggtcgtcaccacgcaattcgtcaacaagggcgtcggtgtcgacgtccgcaagaagctcgctggaaagtaagcaggcaggcaagagtttcaccgtttttcccgtgggtcgcgcggggcttgcgccggggtcagatgccggtgcctgggttgccataaggcaccgcgcgacttttctcttcttgggctctgaccccgtctcgccgacaggcgatgcggccctctttcatgaaaacgctcgtcgtccactgccatccgaatcctgacagcttcaaccacgcgctctatcgcacggccctcgaagccctcgagccccggcatcccgtccgggccatcgacctgtatgccgaaggcttcgaccccacgctgacccgcgaagaacgcatcgcctatctcgagaaccccgaactgatccgcgaacgcgtgaagccgcatgtcgacgcgctgctgtgggccgagcacctggtgttcgtctatcccacctggttccacggaccgccgtccatgctcaagggctggctcgaacgcgtgtggctgccgggcgtggccttcctgccggccgagcgcaagggacagctcgcgaagtcgggcatgcggcacatccggcggctgacggtggtgaccacgggcggctcgccgcgctggttcgtgatgatgatcggcgacccgggccggcggctcttcacgcgcgcgctgcgggtcctgtttgcgtggcgctgcaaggtgacgtggctgcagctgcacgacatgaacgccgtgaccgaacgcgaccgcacccatttcatcgagcgcgtttcgcgcaagctgcaccgcatctagccacggagacacaacacaccatgagcctcgaacgcacgctgaccgtccgcgtcgaacgcatctcgcgccagacgcccgagatcctcgccttcgagctgacgcatccgtggggccgcacgctgccgggctacgaagccggcgcgcacatcgacgtgcacatgcccggcggcttctcgcgccagtactcgctggcgcgatggcctgcgggtgcaccgtcgaacgccgcgtcttatgtgatcggcgtaaagcgcgaggccgcgagccgcggcggctcggcctcgatgcacgagcgcgtgcacgaaggcgacctgctggctatcagcgcgccgcgcaacacctttccgctgcgcgaagaagcgaaacaccacctgctgctggccggcggcatcggcatgacgccgctgctggcgatggcgcaggcgctcgcggcgcgcggcgctgacttcacgttctgcgtgttcgcgcgcagcgaagaacacctggcctttgccggcgcgttgcgcgaccccgcgctggcgccgcatctgcggctgcacctcgaccagggcgacgtctcgcaacgcatcgacctgcgcgcgctgctggccgagcgcgcatccggcacccacctgtacgtctgcggccccggcggcttcatgcaaaccgtgcgcgaggccgccgcacactggcccgatgacgcgctgcacgccgaatacttcgccgcaccggccgacgccaacaccacgacgggcctgcccttcacgctcaagctcgcgcagcgcggcatccgcgtgccggtggcggccgaccagaccgccgtcgatgcgctgcatgaagtcggcatcgacattccggtgtcgtgccagcaggggctgtgcggcacctgcgtggtcgagggcgacggcgaaggcgcggagcatcgcgacttctgcctcacgggcagcgagcggcgcacgcgcgtggccctgtgctgctcgcgcgccaaaggccaggaactggtgctgcagctgtgagcatcgacgaagaaagcgacggcgaggcgccccccacgcgcgggcgttcgcgcaagtacgcccaggtgctcggcctcatcaaccaggccgccatcgaagtgttcgcgagcgaggggctggccggcgcttcgacgcaggccattgccgacaaggccgggctctcgaaggcgcagctgcactactacatcgagagcaaggaggcgctctaccggcagatcctgcaggacatcctccacgactggatcgtggtgttcggctttgccgatgaagccttcggtccgcgcaaggtgctgggcgacctgatccgccgcaagatggcgttctcgttcgagcaccccttgcgctcccgcatcttcaccgccgagatgatgcgcggcgcgccggtgctcaacaccatgatggacacgagcaagcagcacaccgaccaggccgctgccgtgatccagaactggatgaaccagggcctgatggacaaggccgacccgatgctggtgctgttccacatctgggcggtgacgcagttctatgccgaccacgccacacaggccgcctactttcgcaatgtggcccaagagggcgacgacgaggaccggcgctacctgatcgagcaggtgaccgaatttttgctcaagggcgcaggggtcaaataggccggtgctgcggcaggtacatggtggcctccacttccaccagtacctcgtcgcccggcaggaagcgcgacacctcgaccaccgtgctgaccggcggctcgcccggatagaacagcccgcgcacgcggttgtagaacgcatagtgcggcaggtggcggaaatactgcaccagcttcaccacgtcttccatggtgccgccatgctcggccgcgatctggcggatgcgttcgagcacgaaccagctctgcgcgacgatgggcgcttcgaagatgtcgaccgacatctggcccgtggcatagcccacgccctgcagggccgtgcgggcttcttcgggaatcgcgtcgtagccggcgaccgcgcggcgcgtggccggatcgaccgccaccacgccgctcatgaagacgaaatcgcccacgcgcttggcggcggcgtagttggccattggcttgcccatgctcattgtgttttctccaggattcggccgccgcggatcacggtgcgctggcgcccgcgcgggccgatgagttcatgctcgccggtcgccgcaagcagcaccaggtccgcggggcagcccggcgcgatgcgtccgtcccacgcgagccccagcgcctttgcgggactaatggtgatggcgtcgagccaatcgtacgcgggcgcgagatgcgccatctgcacgccgagcccgaaggtctccagaaggtcgtagctgccgtagggatagaaggcgtcctgcacgttgtccgttgccaggctcacacgcaagccccgtgccgccgcttcgtgaatgcgcgtgatgccgcggggcacgggcgtgcggtcccaggcgccctgaagatagagattggtggtcggcagcgcgacgatgtggatgccggccccggcacacagcgccagcgtttcgttggccaccgcgtcgtcctgcatggccagcgagcagcagtggccgcagaccacgccgtgccggaattcgcgcgcacgcatcagctgcgcgatgctgcgcaggccgctcgcatcggcatcgagtccttcgtcgacatgaaagtcgagcccgaggccgtggtgctgcgccagttcgaacacgcggcccagcttgtgcatgaggccctcgttgcgatagacgaaggcacccaacgtgccgcccgcccgcttgacctcgcgcgcgatgcgctcgccggcggcgaggtcggcgaacaggtccagcggcgtgagcgagacgaactgcaactcgatgcggccgcgccactcatgccgcagggcctcgaacacggccagcgcggccggcgggtcgccctgcacccagtcgatgtgcgtgcgcagcgcccgcgtgcccgactgccaggcctcgtgcagcgcacgctccatgcgcgggcgcagcgtttcgccggtccagcccgcacggtgcttttccatgcgttcgatggccgcgaacaggttgccctgggcggcgccgacttcctgcacggtgtagttcttgtcgatgtgcgcatgcgcctcgaccagtgcgctcagcagggtgccgcgcgcctgtgcctgcgatgcgctcggcacgatggcctgcacgcgatcgccggccagcgtgacgtcgaaaacctgcgcatcgtccgcggcaaaaccttgcagccgcggtggaatgcgcacggcctcgagcttcatgcgcgctgttgcaatgcccgcagccagcccaggccggccgaagtgccgccgggttccatgccgcgcttggggcggtactcgcagccgacccagccctgccagccgcattgcgccgacacctcgtcgatcaggtcgaacaggtacgggtagttctgctcgccgatgtcgggctcgtggcgctcgggcacgccggcaatctggatgtggccgacgcggccggtgggcaggtatttgcggatcttcattgccacgtcgccctcgacgatctggcagtggtacaggtccatctgcaccttgagattgggcgcgcccaccatgtcgacgatttcgtgcgcatggtcttgccggttgagaaagaagcgcgggatatcgcgcgtgttgatcggctcgatcagcacgtcgcggccggccttggcggcctcggcggcggcccagcgcaggttgtccacgtacacgggctgcacggcctcgcgctccacgccttccggcaccaggcccgccatgacgtggatgcgcgggcagtcgagcgccacggcgtagtcgatggccttggcaatgccttcgcggaattcggtctcgcggccgggcaggcacgccaggccgcgctcgccgcggtcccagtcgcccggaggggcgttgaagagcacctgctgcaggccgttgtccttcaggcgggccgcgagctggcggcgctcgtagggatagggaaaaagatactcgacggccttgaagccgtctttcgcggcggcttcgaagcggtcgaggaaatcgagctccggatagagcatcgagaggttggcggcgaattgaggcatggtgtgtttttactcttgctaccagcgcgcaccgaaagtgcggcgcagttcatcgatctgttcgttgctcaacggctcgggtttggcggggccggcgagcagatggagcttggcggtttcttcgagttcctcgagcacggccatggcggcggccgggctctcgtgccagacgttggggccgaggcgttcgagcatcacggcgcggatcggcgtgccggcggcaccgtggcgctcgatggcctgtgccaccagctcggccgcttcgggtgcgcccgggcggtggtacggaatgatcggcacatggccgaccttcatcacgaaatacggcgtgagcgcgggcagcagttcgtcgtcgcccggtgcgttcagcgtgagtgcgacgcaatgcgtgctgtgcgtgtggatcacgcaggccgtgccggcatcgaacctgcgcgcagcggcgtagatgcgcgtgtgcagggcgatggtcttgctcgcccggtcgccgccggtctggttgccttgcgtgtcgagcttggccaggcgcgccgggtcgagaaagccgaggcaggcgtcggtcggcgtgatgagaaaaccgtcatcgacccgaacgctgatgttgcccgccgtcgcatgcacgtagccgcgttcgaacaggctgcggccgacgcggcagatttcttcgcgggcttgggtttctgtcatgtcagttttccacgcgcgctgtgtttgttgtgctgttcagggcgcgtgcacaggccaccgggtactcccctccgcgaatgtcccccgccttcggctcctcctttatttcgctgcggggagcacccggcgccctgtgcacactggacgctgcgcttgttccgctggatcaatcgccgcactgcccaacgctcccgctggcggggtgccttgcgcagcgaaataaaggaggagcccgaagggcgcgggacattcgcggagcaaggtaccccgtcggcgggagcgcgccacgaacgtgctcgaacgctgaggttgaacgtcatgccagcactgtaaatgccttggtgaagaaatcatcccccccaaagttgccggacttgagcgcgatgtgcacgggcgtgccttctgccacgtcggtacgcgcatggcaccacggcacgccggggtcgatctgcggaccgatctgcatctgcgcaatgcccagcgcctgcacgcaggcgcctgaggtttcgccgcccgccaccacgagctggcgcacgccgcgctcgaccaggccgcgcgcaatagcggcgatggtgcgctcgaccatggcgccggcttcctcgacgccgagccggccttgcaccgacttgacggcaccggcctctgccgtggaatagaccagcaccggttgcttctcgacaagcggcgcggcccaggccagcgcctcggccgcgacatccacgcccgcggcaatgcgcaacggatcgacggccagcgccgcgccgccgcgctggataaagtccagcacctgccggttggtcgcgagcgagcagctgcccgagaccacggcgcacaacccacccgcggccggcaacgcgctggcctgcgacgacggcgcaaggccgaagttggccggcagcccgatggccacgcccgagccggccgtgaccagcggcatcttcgcaatcgccgggccgagccgcagcagatcgtcgttcgacaccgcatcgacgatggcgaccgacacaccctcgcccttcagctgttcgatccgctccgaaatggccgccgcgccgcgtgccaccaccgcatggtcgatgagcccgaccttgcgccggcactgcgcctgcagcacgcgcacgaggttcgggtcggtcatcggcgtgagcggatggttctgcatgccgctctcgctcagcagcacgtcgcccgcgaacaggtagcccttgaacacggtgcgcttgttgtcagggaaggctggcgtggcaatggtgaagtcgcagtggagcgcttccatcagcgcctcggtcaccggaccgatgttgccctgcggcgtgctgtcgaaggtggagcagtacttgaagtagatctgttgcgcgccttgggcctgcagccagcgcagcgcgtcgagcgattgcgcaatggcctcggccggtgtgatggtgcgcgacttgagcgcgacgacgacggcatccacgtcggcgtcgagcggaccctcgggcacgccaatggcctgcaccacgcgcatgccggcgcgcacgaggttgttggcaaggtcggtggcgccggtgaaatcgtcggcaatgcagcccagcaatagttttgccatggctcagtccttcgcgacaggcagtttcacggcctgcgggttctcgcgcacatagtcgcgcaggatggcgtcgaagctcgcatcggcctggaggcccagcgactcggcgcgggccgcatgaatgcggctaggccagctggtcacgatcttcgcgatgccggcatcgggctcccagtcgatcagcccggtggcgtcgcggcccgcgatgcgttcgagcgcctctgccatttcgcgcacggtggtggtcagggcgggcaggttgacggccgtgcgcgcgccccattcggcggcactggcggtggccgcgcggacgatgccggcgacggtgttgccgggcgacgcgagggcgaccgccgtatcgggcgacacggggcagcgcgcacgttcgccggccagcggctcgcgcagcatgccgctcaaaaagctggaggctgcaccgttgggccggcccggccgtaccgagaccgtcatgagccgcacgttgcggccctgcacgaagcccttgcgcgtgaagtcggccacgagctgctcgccgatgaacttctggatgccgtagctgttctgcggcgtcggcagcgtggtgtcttcgatcaccgccggcagccgctgctccggcgaatcgccgaagacagcgaccgagctggagaacacgaacaccggcgcatggcccgcgcggcggcaggcgtcgagcagcgcgcgcgtggtgtcgagattgctgcgcatgccgagatcgaagtcggcctcgcattcgccgctcacggccgcggcaaggtggaatacggcttgggtatcggccagcggcagtgcgccgctggtggcctgctcgtacaggtcaccctgcacgaactgcacgcgggcatcggcggcaaggtcggcgggcggcggcacacggtcggccagcgtaatgcgcgagaggggttcggcaacgccgccggccagtgccagcggcccacccgccagcagcgtgcgggccagccgcgctccgacgaaaccgcagccgccggtgatcagaatgttcatggtgctcgtcttccttcttcttcaggctttcttgtcggcggccggcagctcgatgccgggaaaaatcttgatgaccgcgctgtcgtcctcgcgcgcaaagccggccgtggacgcctgcatgaacatctggtgcgcggtggacgagagcggcagcggaaacttgctggcgcgcgccacgtcgagcaccaggcccaggtccttcacgaagatgtcgacggccgagagcggcgtgtagtcgcccgccagcacgtgcgccatgcggttctcgaacatccagctgttgcccgcgctgtgggtgatgacttcgtacagcgcggccgggtcgacgccttcgcgcaggcccagcgccatggcctcggccgcggcggcgatgtgcacgccggccagcagctggttgataaccttgaccttgctgcccgcccccgcgcggtccccgagacgataaaccttggccgccatggcgtcgagcacggcgccggccttttcgtaggcggcaggcgtgccggcggtcatcatcgtcatctggccgctcgcggccttggcggcaccgccggaaatcggggcgtcgaggtacaggatgccctgttcggccagccgcgcttccagcgcgatcgaccagttcggatccacggtggagcacatcgcgaacaggctgccgggcttcatcgacgccgcgcagcctggcgtggtgccgtcgccgaacagcaccgactcggtctgcgccgcgttgacgaccacggaaaccacgatgtcgcattgcgcgccgagcgcggccagcgtgtcgcaggccacgccgccgtcgcgcgcgaaggcctgggccgcttcggggcgaacgtcgaagacgcggggcacgtggcccgcgcggcgcagcgatcgcgccatgccgctgcccatggcgccaaggccgacgacgccgacgacgggggtgttgatctgggtgttcatggtgtgggttctccggtcaacggttgacgagttgcttgggcgtgagccacacgccgatggctccgagcaccagcgcggcggccagcacgtacatgccgatctgcgtgctgcccgtgaggtccttcaggtagccgatgaggtaggggctggcaaaccccgcaaggttacccaccgagttgatggccgcaataccggccgccgccgccgtgcccgaaagaaaggcggtgggcagcgaccagaagagcggcgcgcaggtgagcacaccggcggcggcgagcgagagaaacgcgagcgacacgacggtgttctgcgtgtacgaggcggcgacggtgaacccgatggcacccatgagcgccggcacgatcaggtgccagcggcgctcctgccggcggtcggcgctgcggccgaaaagattcatcgcgacgatcgcgcagatgaacggaatggcgctcaggaggccgatgtgcaggttgcccttcacgcccgtggccttgaccagcgtgggcagccagaaagtcagcgcatattggcccatcacgaaggcgaagtagatcagcgccatccaccacacgcgcgcatcgcggaacactgcggccaccgagtgcgggccttttgcgccgtgcgcctggtcgcgctcgacctcgcgctgcagcaggcgcttttcgtcagggtcgagccagcgcgcatgctggatgccgttgtccaggtagagcagcaccatcacgcccacgatcacggccggaatggcttcgatgatgaacatccactgccagccctgcatcgacgacacgccgtggaaggcatccatgatccagcccgaaagcggattgccgaagatacccgcgaccggaatggccgacatgaagaccgcgatgatccgtgcgcgccggtgggccggataccaatgggtcaggtacaggatcacgcccgggtagaagcctgcctccgccacgccgagcagaaatcgcaggatgtagaagctggtcgacgtttccacgaaaacgaagcaggccgacagcacgccccaggtgatcatgattcgcgcgatccagatgcgcgcgccgactcggttgagcagcaggttgctcggcacctcgaacaaaaagtagccgagaaagaagatgcccgcgcccaggccgaacacggtttcgctgaagcccaggtcctgccccatctggagcttggcaaagcccacgttcacgcgatcgaggtacgcgaccacgtagcagagcatcagaaaaggaacgaggcgccagaacactttggcgtaggcgcgcttctcgagcgcgacgtcggcctgcatgccgcctgcagtggcgaccagaggcgcctggagtgttgaagtcattgggaggtccattggaatgaggaactgagccgtgcggattgcccatgcgatgagcccgtctcttatttgtcaggtcatcatacaaatctgatgcggcttgcccgatccgggtaaacccgcaagctacacctcgtttctttttccctacttgcccacgggccagccttcgaccagcggccgcgcgagctgtgcgccttcctgctgccagaaggcggggtcggcctgttcgatgcgccggatggcgttgtccatgtgggacttggcggcctcgcgggcgcgcagcgggtcgccggcctcgatggcctcgacgatctgcgcgtgctcttgcgccacctcgcgcgcaaagtcggcccggcgcgcctcgttggcgcgcgtgacccgcgtggcgccgtgcaggaattgccgcaggtactgcagcgtgccgatcaggaacggattgcgcgccgcctcggcaatggcgcggtgaaagcgcacgtcttcgtccgccccgttgccaccggccgccaccgcggcgtgcagcgcctcgatggcttcacggatgcgctgcacgtcttcgggagtgcgccgctcggccgccagcgcagccacctcggcttcgagcgcgcggcgcagttccaccatctggatcaccgcttcgcgcgaggccacgtgcggcatctcgaagcgcagcggctcgacaccggcggcgcgcacgtacacgccgctgccctggcgcgaatcgagcagccccagcgacttgagccgcgagaccgcctcgcgcaccacggtgcggctcacgccgaattgctcggccagcgcagcctcggtcggcagccggtcgccctccgacaggcgcccgctgcgcacctcggcggccagcgcgtcggccacctggtcggcaaggcgaacggtgggagcaacggattggaaacgtgcggtcatgagctcgggtgtcggtcgggctgcgactctaacgcaggcacgtgcggcgaatctctggaacttaagaactacccaatgccgacaggtgttgtagcgcggcacgctggagctgtgagaaatctggcgctttcagcctcaatctgtgcgggcctttcgcattttgacctccggcgcccacatgtaacgagaaaatccgatccgcgcgcatgtgcccccgattacgaggcatgcgatcactataaaaaagcacgccaaccggaggagcaacatcatttgacttaaatcgttctcacctgcagttggcgattacttatcactcccccaatttttacttctcatgaaaatcaattcttcgatctcatcgctcgtgctggcagcggcacttgcagttctctctgggtgtgccagcctgccttcgccagaagcaatgaaggctgaaactgcgtcctttcagctccccaaaatgccagagcctggaaaagcaattgtttatgtcgtacggccttccggagtaggtggcctggttcgattcaatgtcttcgtggacgatcaagaagccacttcagagatgggtcacacccgctcaagtcagtacatctatttcaacgtcacgccgggtactcacaagatttactccaaggcggagaactgggctgacacgcagatcactgccaccagcggcgacatcatctacatacagcaagaaccttcaatgggcatcatcatggctcgcaacagcgtgagcaaaatcgatgacgtccaaggcaagtaccaagtgaagaagctgcaggtcggcacgattatcaaaactgacaagtaaggcaagcaagttcggtagccaagctactctctggctaggctaccgaacgcgactcaggttatctgcagcgaatgccgcgccgcccccgcaatgctcgccgcatccaccccgaagaacttgcgcagcgccgcgcgcgtgtcgctgcgcccgaacccgtcggtgcccagcgtgaggtagcggcggccttcgggcaagaatgcgcgcacgctctcgggcacggcgcgcacgtagtcggtggcggcgacgatcggtcccgcgccggcgccgagctgccttgcgatgaacggcacgccggcttccttctcgcccgccagcgcccgctgctcgcaagccaggccgtcgcgcgcgagttcgctccagctcgtgacgctgaacacctcggcctcgatgccttcgtcggtcagcagttgcgccgccttgaccacctcggtgaggatcgcgcccgatcccatgagcgtgaccttcttcttcgccttgccagaggctggaccatgcacgccgaagcggtagcacccgcgcaggatgtccgcctccgcgccttgcggcacgtcgggctgcgcgtagttctcgttcatgagcgtgacgtaataaaacacgtccttctgctcgaccatcatttcgcggatgccggcatcgacgatcaccgccatctcgcccgcaaaggcggggtcgtaggccttgcagttgggaatggtcgcggccacgaggtggctgctgccgtcctggtgctgcaggccttcgccgccgagggtggtgcggcccgaggtggcgcccaaaaggaagccccgcgcgcgctggtcggccgcggcccagatggcatcgcccacgcgctggaagccgaacatcgagtagtagatgtagaagggcagcatcgccaggccatgcacgctgtagctggtggccgcggccgtccagctggcaatggcgccggcttcgctgatgccctcttccagaatctggccgtcggtggcttcgcggtagctcagcacggagccgatgtcttcgggcgcatagcgctggcccacgctcgaatagatgccgacctgcttgaacaggttggccatgccgaaggtgcgcgcctcgtcggccacgatgggcacgatgcgcgggcccagcgccttgtctttcatgaggttgcccagcatgcgcacgaaggccatggtggtgctcatttccttgccggctgccgctgtcgcgaactgggcgtagctcgcgatgtcgggcttgggcaccacctcgcacgcggtctcgcggcgcggcatggcgccgccgagcgcggcgcggtggctccgcaggtactgcatctcggcgctgtcttcgggcgggcggtaaaagtccatcgctaccgcctgcgcgtcggtcagcggcaggttgaagcggtcgcgaaactcgatgaggtcgacgtcgcccatcttcttgtgcgagtgcgtggtcatcttgccctgcgcggcgctgcccatgccgtagcccttcttggtgtgggcgaggatcacggtgggctggcccttgtgcgcggccgcggcggcgtaggccgcatggatcttcacgaggtcgtggccgccgcgcttcaggcggtcgatctgctcgtcggtcatgccttcggccaggcgcgcgagttcggggttctggccgaagaagttgtcgcggttgaagcggccgtccttggccgcgaaggtctgcatctggccgtcgacggtttcggcgaacacgcgtgccagcgcaccgctcgcgtcctgcgcgaacaggccgtcccagtcgctgccccagaccagcttgacgacgttccagcccgcgccggcaaagagtttctcgagctcgtcgatgatgcggccgttgccgcgcaccgggccgtccaggcgctgcaggttgcagttgaccacccacacgaggttgtcgagtttttcgcgcgcggccagcgtcagggcgctcatcgattcgggctcatccatctcgccgtcgccgaacacgccccacactttgcgaccctcgcagtcgagcaggttgcggtgcgtgaggtagcgcatgaagcgcgcgtgatagatcgagctgatggggccaatgcccatcgaccctgtcggaaactgccagaagtccggcatcaggtacggatgcggatagctgctaaggccgcgcgcaccgctgccttcggtgaaggcgggcgcggtcagttcctgcctatagtgcttcaggtcttcttcgccgaggcggccttcgaggtaggcgcgggcatagacccccggcgcgctgtgcggctgaaagaagacaaggtcaccgcggtgctgttcgctgcgcgcgtggaagaagtggttgaagccggtctcgaacagatcggcggcgctcgcatagctcgcgatgtggccgccgagttcgccatacgcctggttggccttggccaccattgcgagcgcattccagcgcatgagcgaagccaggcgttcctcgatggccaggtcgccgggaaacggcggctggtcttccaccgcaatggtgttgacgtagggcgtggcgagctcgggctgccagccgatgcgttgttgccgcgcgagccgggcaagctccaccagcatctgccgtgcgcgttgggggccatgcgtttgcgccagcgccaggaaggcatcgcgccattcagcggtctcggcggggtcggggtcgtgcgagagcggcgtgtcgatcagcagcgcacgcatctggtcggtggaaatcggggcgttcatgccggcactttaagccgccgtgcagcaaattagctaccggtacgggcaatcccatgcggtcttcgcagcataaaattccggccactctagatttcacggcatttcatgcaactcgatgccatcgacctgcgcattctcgacgagctgcagcgcgacggcgcgctgtcgaacgtggagctggcgcgccgcgtgcacctctcgccctcgccctgcctcgcgcgcgtgaagatgctcgaggcgaatggcgtgatcgaccgttatgtggcgcttgcgagcgcgaaggcgctgggcttgggactcaacgtgttcatctcgatcagcctcacgacgcaaagcaagcagtcgctcgccgatttcgaacagcgcattgccgagcacgacgaagtgatggagtgctacctgatgacgggcgacagcgactacctgatccgcatcgcagtcgccgacatggcgtcactggaaaaattcatcctggaacagctcacgccgattccgggcatcgagaagatccgctcgagctttgcgctcaagcaggtcaggtacaagacggcgctgccgttgccccggtagggcgctaccccaggctgcgcacaacctggggtatcaatcagcgaatcagcgcaatcggtcagaggccgatcaagccgccgtcgtccttcgtgatgaccacggtcgccgagcgcgggcgtgccgtgccgccctgcggccagtggctgccgaacttcgtcgggtcggagatgttggcgcgcgccgtggtctctccgggatgctggatgttcacgaacagcgcgcggccgtcgcccgattcagcaatgccggtaatttcgcagtcggacgggccgaccaggaagcggcgcaggccgtcggtgccgggtgccttgccgacgaaggtggcctgcgtggcggtggtggcgccgtcgacgttggtgatcgtcttcgccgcgccgtctcccacctggcccggcagtgccgcgagcatcatgcagttggtcacgtcggtgtacttgccatcgtcggtctgcagccacagcaggccggcggtcgcatggctgaaccacatgccgtcggggctggagaagtcgttgtcggcaaccaggttggacaggttgacgtcggccgatgccgtcgagcgtgcaccgaacagatagacgtcccagttgaagctgacggccgcggggttgccgccggcatcggcaaagcgaacgacgtggccgttcgggttgcccgtttgcgccgtctgggccacgcccttggggtcgttgtaatagcgcgggttggcggcatcggtcgtgctgatggtgcgcgcggcgttgttggtgagggtgaggtacacctcgccgttcttcgggttgacggcggtccactcggggcggtccatcttggtcgcgccggcaacatcggccgcgaggcgcgcattgatcacgacgtcggccgcatcggcaaaggaataggccgcgttgccggaggtgatgccgttcacgccgagggagagctcgagccagtcgccggtgccgtcggccttgaacttggcgacgtagagcttgccgtcgtccatgtacttgtcgccggccgcaatgccgccgccgatgtcggccgcgtcccaggccttggtggagacgaacttgtagaggtattcattctgcgagtcgtcgcccatgtaccagacgaggggcttgccgacgacgacggggccgaggcaggcgccttcatggccgaagcggccgagcgcggtgcgcttcttgggcgtgctggtgggagcgaacgggtcgatctcgaccacccagccgtaggtgttggaaccgttgcggtagtcgtcggtcgcggtggcgccgaggacttcggtgttccagcggccatagagattgtcggcagtgtcgggcgtcaccgtcgcccacagttcgcggccggtgccggtgtcgacgccactgctgtttttcgcgccgatgccgtatcgcttgaaggaggccagttccttggcacttcgctgggcgtcgtcggtcgccgtgatgcggcggaagtagccggcccagttttcttcgcaggtcagataggtgccccagggcgtggtgccgttggcgcagttgttgagcgtgccgcgggtcttgctgccgtcggtcgagtacttggtcttcaggtagtcggtcttggcggccggacccgagaagctcatctcggtcagcgtgtggacacggcggttgaagctcgaatcctgcttgtagctccaggcgctgccgttcttgttgacctcgatcacgctcacgccgtgcaggtagaactcgcgcagcacttcatcggcgacggtgcggactgccgcggtgccgctgccggtgatggtctggccggtgggatgcaggaacagcggcgtgatggcttcgtggttcatcacgagcaggccgcgcgacgcgttggcggcgtcccatttgttcgaggcattcatgccgaagaaggtcatgccgtcgtggtggtccccggcgcggcggtcgtaggtggccggatcgtcggtgccgtcgttcttgtaggcggccacgcccgaggcgatcgggtcgcccaggcgatagagcacgctggcggtgtagccggcgggcacggtgaccacgtcggccaggctcttggccacggcattgaagcccagcttggccgatgcgggtgccggcgaaggagctggtgccggtgccggtgcgggagcgggcgccggtgcgggcggaatgatcggaaaagccacgccgccaccgccgccgcctccaccgcacgcctgcagcagcgcggtactggcggtgccaacgcccaggccgaacagatggcggcggctcaggcgcgaagcaatcaggtcggtgaaggacggattcgaagtggggttggtgccgacgtcgtcgagatcgatgccgttggcgtcggtacgggtgtttgcggtcatgcgcaattgctttcgtgggttgaaaaggaaatcaacccgcgaagttaggcacttggcatgacatccgcgtgaaacgctcagcttccagtcagaagtagctcgcccccagtcttcgcgactttccccttcagggcgcgggcagctgcctcggccagagggcccagaggcgcagcgactggttcatgctggcagcgaggcggccggcgtcggcaccggtgccggcgaaatagtcggcgcgcaccgccccgacaatggcgctgccagtgtcctgcgccaccaccagcttctgcaactgggccgcggggccgctggacgcaagccacaccggcgtgccataaggaatgctctcgcggtcgaccgcaatggaacgccccgccgtcagcggcacgccctgcgcgccgcgggggccgaaagccgcgtcgagctcgctcatggtttcctcgcggaagaacacgtagcgcggattgctccacaagagctgcgacacgcgctgcgggttctgcgccgcccatgccttggtgtcgtcgggccacttgccgatcttggccacgccttgcgagatcagccattgctgaacgctcttgtagggctgctcgttggtggccgagaacgccacgcgcacggtgcgctgcacgccgttggcctcggtgatgcgaagccgcccggagccctggatgtgcagcatcagcgcgtcgatgggatcggccatccacgcgatctcgcggccgcgcagcgccgcctgcgcctccggcagggtttcgatctcttgccgggtgtaccaggcgcggcgcggcaccagcccctccggcgcctggtagatcggaacgctgaaggtggcggtgggcacgcgcgaagcttcgtacaccggctcgtagtagctcgtgagcttgccctcgctcgaacccgcgagcgactcgatccggtagggctggagcctctccgtcatccactgccgctgttcttccggcgtggcgatggccagctggcgcacgtcgcggcacagcggcgcaaaggcggcgttgggccgggcgcaattggcgagcagcgcaatccaggcttcgtgcagcggatcgtcgccgaaacccggcagttccgaccagcccaccggcacccatcggctcttgggatgcgccagcgagccggtcagcggcccgaggtcgcgcgggggtgtggcggtgggccgcgccggtgtgtcgggcacgcgcgggccaaccgagcagccggccagcgttgctacgatcgcgagcccaaccagccactggagtccatttctcatgggtctgattttgcttgaagccctcggggccgggctcgtattgatattgatcgtctggtggaccatgttttcgggtcggaagaagggtgagctgcaggatgaggacgaggccgcccatgacgacaacggctccgccgaaaaggacccgccgccgaaaccgtgaattccttgcgtagcccaaagtcggcgtggagtgtcggagaacaggctatcagctattactttagtagcaatcatcgcagtattcacggggctttgcagaaggttttcctctttcctccaaggcaggaaggccgtaccatcgcgtgctcgccgacgctaagctgtcccgcctgattcaaccttgaaagggattgccatgaaaaagttcgtactcgccaccaccgccgccgctctcgtcctgtccggatgtgccggcggcatgaccgacacccagcgcaacaccggcatcggcgccggcattggcgcactgggcggcgcggccatcggttccgccactggcggcaaccgcggcgccatcggcaccggtgccgtggtgggtgccgcagccggcgcactcggcggctacctgtggtcgcagcgcatggaaaaccagaaacgccagatggaagccgccacccagggcaccggcattgctgtaacgcaaaccccgaacaacgagctcaagctgcagatcccgagcgacgtgtccttcgacgtgggccgttcgaacatcaagtccaacttcgcgccggtgctcgaccagttcgcgagcggcttgcgcaacaacccgaatgccgaggtgcgcatcatcggccacaccgacgccaccggctcggacgcagtcaacaacccgctgtcggtcgaccgtgccgcaagcacgcgcgactatcttgtgacgcgtggcgtgagcacggcggctttccgcatcgaaggacgcggctcgcgcgagccgattgccgacaataacagcgacgccggccgggcgcagaaccgccgcgtcgaaatctacgtgggcgagcgcgcgccacgcggctgaccgaacacatcgacagataaaaagacagatcaaaaaaaagaaaaaagccggccgggcgggagcggccggcgctcatcgccatcgtttcaatgtcaattcagagggaaaactcatgaggaagtttgttgtttcgggtgcggctgcggccgcattgttcgttgtggggtgcgcctcgcaatcccccgcgccagggtcggccgcagcgccggctgcacaggcggccgcaccagccaacagctggaccgcgcgcctggcctcgctcaagaccgagctcgaaaactcgaccaagggcacgggcgtggtgatcgagcagaccacggacaaccagctgcatctcgtgattcccaatgaactctcgttcgacgtgggccgcgccaacgtgaagcgcaacctcgcccaggtgctggacaaggtggccgaaggcctgcgcagcgccaccgcggccagcgtgcgcgtcgtgggccacaccgacaacaccggcagcgaagaaggcaacgagcgcctctcggtgagccgcgccgacagcgtgcgcaaccacctggtgggccgtggcgtctcgacgacggccatcaccaccgacggccgcggctcgcgcgaacccctggccgacaacagcacgccggctggccgtgcccagaaccgccgcgtcgagatcttcgtcgcggaaaaggtctgatctcctagagatcccgcaggcggttggccagctcgaccgccgacttcacttccatcttgtcgaacacgcgcgcgcggtggacctccaccgtgcgcacgctgatcgccagctgatcggcaatcagcttgttgggcaggccctcgaccacgagccgcatcacgtcgcgctcgcgctcggtcagttcggcaacgcgtccggccagactcttgcgcgcgcgctgcacttccagcgcccggagcgaagcgcccagcgcctgctcgatgcggtcgaccaaggcgttgtcggaaaacggcttctcgcaaaaatcgaaggcaccgcgcttcaccgcgtccaccgcggtcggcacgtcggcgtggcccgtcaggaagatcaccggcatggcgtccaggaggccgcgttccgcgagccggtcgaacagcaccaggccgctggtgccgggcatgcgcacatccagcagcaggcacagcggctgctcgggcagcggaccctcggccaggcgctgctcgaaagcctccgcgctcgcgaagtgctcgctctcgaggcggcgcgaacgcagcagccaggccagcgcctcgcgcacgctggcgtcgtcgtccacgatgaagatgagaccgtcgatcagcggttgcatatcgattccagaaacgagcgcgaagcctgggggtgaatcatgtacttggcagggtaaaccggaacacggtgccccgggggctgttgggctcgaacacgagcacgccgccatgctgctccaccaccgtgcggcacaggctgaggccgagccccatgccgtcggcccgcgtggtgaaaaacggcgtgaagagacggctcgccacttcttcgctgatgccgctgccgaagtcggccaccgaaaactcgagccagcgtcgcgcgtcttccgcgcccgggccgccgacggccacgacgcgcgccacgcgcagccgcaggatccggtcgccagtgttgtccgccgtgtccatcgcctgcatcgcattgcgcgccaggttcaacagcacctgttcgaccagcgtgcggtcgcacatggccttggccaagccgtcttcgagcgccacctcgatgctcacgcccagcttgcgcgcctgcagccgcaccagcggcagcaccgcatcgatcagcgcctgcggtgcgacggcctcgcgcgtgcggtcgcgccggcgcacgaagtcgtgcacgctgcggatcacctggccggcacggtcggcctgctcggcaatgcgccgcaccgccatggcgacctcggcctgctcgcccttggcatgtgggcccagcatgttgagcgagccggtcgcatagctggcaatagcggccagcggctgcgtgagctcatggctcagcagcgaggccatttcgccgacggtggcgagccgcgcgctggcctgcaggcgctcctggctggcccgcgagagttcttcgacgcggcgctgctcgctgacgtcgatgaaggcgctcatccagccggtttgcacgcgctgcgcattgatcagcggcgcttcgaagatgagcaccggaaaacgcgtgccgtccttgcgcatgaagaccgactcgaagccttcgcgcggcggcatgccgccggccagccgccgggcctgccgctgctggtattcgtgcgccaactcggtcggccagtagggggcctcgatcgattcgccactgccggccatcagctcctcggggctgaagccgaccatttcgcagaacgcgggattcacgtaggtgatgcgcccctgcaggtcgcgcgcgcgcaggccggtgatgaccgaatcttccatcgccttgcggaaggcgagcgcatcggccaggtcgcgctccgcgcgcagccggcggcgcgtgtcgcgcgccagcagcaccagcacggacaccagcgcgatggaaatggccgtgaccagcgcggtcagcacgttggggaacagatcgggcgcggcacgccagccatcgacgcgcagcatcagcgcggcaccgggcaggtcgatcagctgctgcgaggtgaagacgcgcgttcccgttcggcgcgacgtgccgagcgccaccaggcgcgtgccgtcggcttcggtgaatgccacctcctgcccgcgcgtgagcgtggggccgaccagctcgacgagcgtgtcgcgcagcgagtagctggccacgaggaagccgcccgcatcgatgggcacgcagagctccatcacctcgacgccgcccccgccgaggatcggcacgtagtggctcggcgaataggccggcgcgccgagcttgcgcgcggccgcgcaggccagcgccacgtcggactggtcgggcccgcggctctcctcgccgatcagccgcatgcggtagggcgtgttgacggcctccagcggtcgcagcgcggcgtcgcgccactcgagccggagccattcgcggtgctcgcgcagcaggctggccgcggcttcgggccagtgcgtgcggtccaggccggaggcctgcgtggcgcgcaggctctgggcattgcgctgcaggccgttgcgcaggtcggacaccgcatcggcggtgtcgcggtcgagcgccgcctgcacctgctcgacctcgtgccgccccgcgagccacaccacggtgatcagcaaggccgacaccaggacggccaggatcagccagagaaaccagcgctgccacagcgaccgcaggcgcgcgaacgcggacagcgcccaccgcggcggtgcgacgtgcaaggcatcctccatcgctagagtacgcagtgcgagagaaccggcaactgggcgcgcacgcgctcgatctgcccggcatcgatgtcgaacagcaccatgccttcgtcgctggcctgctgcgccaccaccgtgccccatgggtcgaccaccatcgactggccccaggtctggcggccgttctcgtgcgtgccgccctgcgcgggtgccaccacccaggccaggttctcgatggcgcgggcacgcagcagcacctcccagtgcgcggcgcccgtggtgcgggtgaaggcactgggcaccagcagcagctcggcgccctgcctggcaagcgcgcgatagagctcgggaaagcgcaggtcgtagcagacgctcatgcccacgcgccagcggtgcccgtcgcgcgagggcaggtcgaacaccacgggcgtggcgcccggtgcgatcacgcggcgctcgtcgtagcgctcggtgccgttgtcgaaatagaacaggtggatcttgtcgtagcgcgccacgcactggccatcgggcgaatagcacagcgagctgttgaacacgtgctcggcgtcggtggtctcgatgggcagcgtgccgccgacgatccagagcccgaactcgcgcgccgcatcggcgagaaagccctgcacggcgccggcccccgcggtttcgcgcaggcccagcttgtcggtgtcgcgcgcgcccatcatgcagaaatactcgggcagcaccgccagctcggcaccggcctcggcggcttgggcgagcaggccgtgcgcacgcgcgaggttggcttcgcgggcgatggccgacaccatctggatggctgcgactttcattgcgtggtctccgttttcttgcctgcaccgcccgcgggcggggcgggaacggccgaggcgttcggcaggatggatcgtggcaccttggcgatcttggggtcggcccaggtgccttcgatgtggaactcctgcgtggcggcggtagcaagcggcttgctaagcacccactgcgcgaggaaggtgcccaggccgatggccgggttgatggcggtggccaccaacgcggcggtgccggcgttgatttcgggcaccaccaccacgcgcaggtcttgcgtctcgcgcacgatgtcggccgagccgtccatcagcgcggcggcgttgacgcccttcatctgcaggttgttggtgctcgcgatgccgttggtgattctcgcgtcgccgcggatgaagtcgaaggcgaagccctggctgaacacatcgcggaaatccagcgtgagccggcgcggcagcgcctgcaggctcaacacgccgagcagcttggcaaggccgggatcggccttgaggaactgacccgattcgacgttgacctggatctggccacccaggctcgggtagtcgagcgagaacggcgagccgcgccaatggacgtcgccctcgagccgtccgctgccgcgccgcaagacgccgggcatgccgaagcgcgtgagcaggttgccggcgtccgagatgtcgagcgtgaaggtcatggccgtgcgccgccgctcggaccgcccgggcgtggtgaccgagcttgcggcccaggtgcccttggcggtgaagttcgcctcgggcatggtgaagctcagtttgttgagcagccattcgcggcccgcgccgccgcggttgacggcgtcgatttcggcacggcccaggcgcttgcccagcagctcgaaatcatcgaccacgatgtcgagcgcgggcagcgtgcccggctcctcgtcgagcagcgcttcgacctgcgtggcctcggccggcgcgatcttgagccgcgcgagccgcgcatagagccggccggcctgcgcgtggcggtattcggcgtagccgctgagctcggtggcgtcgatgttggcgcgccagagcgtgccttcgcgcgtgccgccgagcaccacgttgtgcagcgtgcggcccgcaatgccgagctgctgcgcgcgcaccgcgatgcgcgtgggcacgtagctcatggccgcgtcctcggtgccgcccggcgcctcggccgcaccggtgctggtgcccgcgtcgcccaccagggcttgccatgcgggcatgtcgagcttggcgatgttgacgttggccgtcacgcccctgtcgggcacgctggcggtttcgcccggtgcgaggccgatggcgacgcttccgcgcagcacccgcgcatcggcgcccgagatgtcgcgcacatactggaccgcgccaatgcggccgagctccagcgagagctggtcctgcaccgcgacggcaacaccggcgcgggtttcgcgctgcaacaccttcttctcgatgcgcagcggcatctgctcgtcggccgtcttcaccaggggcgcaggcaactgcagggccaggccttgcagcgtgctggtgagagaaaactcgggtgcgccgtcgcgcatcgagaaggtgaccgcgtagggcgtgctgccgctggccttggccgcgatccgggtgagccactcggcctcgcgcgcgccgcgcaggccctcggccgtggccgtgccctgcgccttcagtgccacttcgcggttggcaccggcgaagcgaccgcggccctcgaggcggatgtcgccgcccagcagccgggcctggacgccggccagcgaaaaacccgtttcggtgaagctcacagtgcccttggcctgggagaacgacggcgcttcgggcgcgaactgcagttcgttgtcagacagcgcaatgctggcctggaccttggccgcgtccagcgcggcgagcggcagttcgaggtgcaggcggtagtcggccacgccggtggcgcgtgcgcgggacagcagctcgccggtttcgccggccagcggggcgcccacgcgcagcagttcgccaagcggccccttggcctgcgcatcgacgcgcagcagcgaggcatggtgcgacatgtcggcaatctgagcttcggccttggtcacctcgatgccggatgcgccggccagccgcccgcgcgcattgcgcaccagcatgcccgcgcgctcgaacaccagctcgcccgagagcccggtgagcggcggccagaccggggcgggcgtgccggtgcgtgttgcggaggccgcagccttcgacgcggtcgacgcggcaatggccgacgtgggcggcacgtaggcgtagttcacgtcggccaccttggccacgatgcggaattcacccttcttggggtccatgaagggcatgtcgtgcaggtcgccgcgcacgcggaaatcgacgctgctggccgtgcccttggtgaccgcggtgcgcacgtagtcgcgcgtgtgctgggggatttcaagcggcaggtagcggaacacgcgcgttccgtcggcgcgcgtcagcttgccttgcaggtcgagcacgccggggtagcgcgcgcgcccggacgacacggccggatcgctggtgcgccagctggcttcggcctcgccctcggcgtcggtgttggcgaagcgcagcttggagacctgcagctgcgcgttgcccttgtcgagcttccactggagctgggcggcgagccggtcgatcggaatcaccggctcttcgaacacgcccggaaattcgagcgtgccccgggccattgtcagtgccgcggtgccgccggcgtgggtggcctcgaactcgaccgtggcgccgctcacgccgggcgagccggcatgcgggtgttctggcgccggggccgtgctgcccgcggttttgccggcagcgggtgcggcgggcgcagttgcagcggtttgcggcgccccgggctgcgaggcgacgcgcaggccgctgacccgccccttggcctggtagcgctccggcgcgccgagcgacccctgccagttcaggtcgatgcgctcgaccagcccgcgcggcgcataggcatcgagcacgcggtgcgtggcctcgcccagcggcaggcggtcggcaatgagggccagcgcggccaggtcgagccggtcggcacgcaatgcgccgtgctcgggcgtgcggccctgcgcgggcgagtgctgcagccacaggttgccgccgggccagcgcatgccgtcggcggtgtcgaactgcagcgccgcggtcgagaactcgaaggtttcttcgttccggtggcccgcgagccggccggtcaccgaccgcagcaccagcggctggaggccgcggcccagcgaggcgtcgatgcggttgaggccgaggtccgccgcgccgcccacgatctgccctctcttcatgtcggcccacaggcgcagggcaccgctgccttcgcggatgcgcgcgtcgatggagacgtagcggcccaggcgggtgacgtccatgtagggcaggtcggcgtagatctggccgtcccacgtctgccaacggccggatcgcaccgacagcagcggctggcggaattggccgcgcagggtgaagcgctcgccccatccggccggcggcgtggcgtcgagccggaggccgtggcgccgggcggtattgcgcgccacgaagcgcacgtcgctcagcagcaggggctctgcctggcgctgctcgtcggtccagcgcacggtgccgccttcgacgaccagctcgcgctgggcaaaaaaccagtcggcggcgcgggtctctccggtggtgtcggtgtccatgtggaggccggccacgtgcagcttgccgagcacatcgcggcgcacgtcgacctgcggcccctcgatgtagatctgctcgaagttgaggcgccacaaggaacgcggcgagacgctcgccaccacccgcacgaggcgcagggcttctcgcttctgggcatcgtgcaggaccacgtcgcgcagttcgaagacgggaaagaggctgtccgaacgggcggtgatcgacccgatgcgcacgggtaccccgatggccttgctggcttgcgcctcgagcgcaccacggtaatcgccgattcgcggcacaatccacgcgtgtaggacaaccactgacagtgccagcagaagccatgcagcgatcagtaaacccaacagccagcgtgccgtcgcagcggtgatcttgagcagacgtgaaggggaagacgccgtgtcgttcattgaggatcgcgctgtgtcaggaattatgaccgccagcactcagaggggttccacggaaaccgatatcagcgtgaaccagttgccagccacgccacccaccgcgatcgaggtcgcgttttcttcttactcgcgcttcgttcagcgcctgcgccgcaggtatgcggcggagcttgcattgcttccccctggcgcgccgctgcgcgagtcgatgtcaaaggcctacgaggcattgcgcgaacgcggggatggcgtcggcgatgcgcttcggattgtgcgacagctggtggtggagcggcttgtaacgctcgattgcgatgcccaggctccgctggccgtggtgaccactgccgtgaccgagctcgcggaattcgcgctcgatgtcgcctgccgcgacgcctgccaggagctcgacgccacgcatggcgcaccgctcggccccgaaggccagcgctcgcagctctgggtggtgggcatgggcaagctcggcgcgcgcgagctcaacgtgtcgagcgacatcgacctgatctacctgtacgacctggacggcgaaacccgcggcgacgcagacggccgcggccgactctcgaaccaggagtacttttcccgcgccgtgaagcgcatctatgcgctggtgggcgacatcaccgagcacggcttcgtgttccgtgtcgacctggcgctgcggccgaacggcaattcggggccgagcgtggtgtcgctcgacgccctcgacgagtattttcaggtacagggccgcgagtgggagcgctttgcctggatgaagagccgggtggtcgcgccgcgcgacatcgtttcggaaggcctcgcccaaggcctgcgcgccacggtgctgccgttcgtgttccgccgctatctcgactacagcgtgttcgattcgctgcgcacgctgcatcggcagatccgcgagcagtcggcgcggcgcagcgcgggccggcccgagcgcgccaacgacgtcaagctgtcgcgcggcggcatccgggaaatcgaattcaccgtgcagctgctgcaggtggtgcgcggcgggcagtttcccgagctgcgcacccggccgacgctcgacgccttgcagcgcgtggcacgcgccggactgatgccgcaggaaaccgccgatgcgctggcggcggcctatgaatttttgcgccgcgtggagcaccgcatccagtacctggacgaccagcagacccacgtgctgccggtggccgacgacgatctgcgctggatcgcccagaccatgggctatgccggctgctgcgcctttctcgagcagctcgacacgcaccgcgagctggtcgcgcaggaattcgacaagctgctcggcggcgtgaagccctgcaacggcaaatgcaacggcaagaaggcggccgcgcccgccgacctggccgatctgctcgacgatctgccgcccgcctttgccgcgcgcatcggcaactggtgcgagcagccccgtgtgctggcgctgcgcgaggaaacgcggacccggctgcgccagctggtgcagcgcaccggccaatggctgaaagaacccgatggcgacggcccgggacaaacgccgcgccacgtggacgccgccttgcgctgggccgactggatcgagccgctgctgcggcgtgagagctatgtggcgctgctggtcgagcggcccgccgtgcaggagcggctgctgcggctcctgggcgccgcgaagtggccggcgcgctatctgatgcagcaccccggcgtcatcgacgagctcgcgagcgacgaaatgctgtcgggccgcttcgtggcggcggagttcgagcgcgaactcgaagcgcgccatgcctcgctcagccgcaccggcgaagccgacgaggaacgcctgctcaacctgctgcgccatgcccaccatgccgaggtgttccgcacgctggcgcgcgacgtggacggccggctcacggtggaacaggtggccgacgacctgagcgcgctggccgacaccacgctgcgcgtgaccgcccgctggtgctggtcgcacgtgcgcaaccggcaccgtgaggtgccgcagttcgcgatcatcggctacggcaagctgggcggcaaagagctgggctatggcagcgacctggacatcgttttcgtctacgaggacgacgacgagcgcgcgggcgaggtctacgcggcctatattcgcaagctgatcaactggctcaccgtgaagacgcgcgaaggcgacctgttcgagatcgacaccgccctgcggcccaatggcaactcgggcctgctgacgaccaccttcgaagcctacgagcgctaccagctcgggcgcggcagcaacacggcgtggacctgggagcaccaggccatgacgcgcgcacgcttcgtgctcggcagcgccgaactgggcgcgcgcttcgaccaggtgcgcgaggccgtgatcgtggcgccgcgcgaccaccaggcactccgggccgagatcatcgcgatgcgcgacaaggtgcgcggtgcacggccggtgaaggccgagcgcttcgacgtgaagcacagcccgggcggcatggtggatgccgagttcgcggtgcagttcctggtgctgtcggagtcggccgggcaccgggaactcattcccaacgtgggcaacatcgcgctgctggtgcgcgcggaagaagccggcctgctgcccgccgccgttggccgcaatgccgccgcggcctatcgcgaactgcgccgcgtgcagcatcgcgcgcggctcaacgaagagccgacgcaggtcaccccgcccgcattggcccatgagcgcgaagccatgctggcgctgtggaaggcggtatttggctgacagcacccgcacccgcgccatatcggcgatggccgcctgcgcggtggctgtcgccgttcttctcgccggctgcgcgagcggcccgcgcagcggcggcggcgctggcggcagttcgggcgggcgtgacggccccggcagcaacattcccgcggacctcgaccgcgtgcccgatgccgagccccgcgtcgaacccatccgcaacagcggcggcaccagcaagccctacacggtgctgggccggggctaccagccgatcaccgacgacaggccgttccgcgaatcgggcattgcctcgtggtacggccgcaagttccacagcgcctcgaccgcgagcggcgagccctacgacatgtacgccatgacggccgcgcacaagacgttgccgctgcccagctatgtgcgcgtgcgcaacccggccaacgggcgcgaggcgatcgtgcgggtgaacgaccgcgggccgttcgtcgacggccgcatcatcgacctgagctacacggcggccctcaagctcggcctgctgcgcggcgtggcgccggtggagatcgaacgcatcacgaacgaggacatccgcaccggcgcgtggcggcgggattcggggacggcgtatgcctcggcggccccggccccgcaaccgccgcgcgcaacggcggctgcggcggtgccggttccctcggcatgggtggcgccggtggcgatgaacgcgccggctgcttccaccatgccggtcgcaccgcagaccgcgatgacaccgatgacagcggcggagcctctgatggcgcaagctgcgccgccggcaccggaggccgcatcgccccggcagatcgaggtcgccgagctgccgccaatggcgcccatcgcggcgccggcgtccatggctcgttcaacggctgcaagctcgtccgccgccgccacggcgggcttctgggttcagcttggcgcgttccgcgagcgcgatggcgcacagaacctgctgagcgaggccgcgcgcggcctgcccacgctggcaccgcaactgcgcgtgttcagcgaagccggcacgcaccgcctccaggccgggcccttcccctcgcgcacggcggccggcgaggccgtcacgcagttgcgcgagagcctgcgcatcgcgccgatggtggtggagcgccgctaggccgcaacttcaaaacggcggcatcggagacacgggctcagggcatcgccttggccagcacctgcgagcgcatgccgacgcccatgcggttccaggcgttgatctgcgcaatggcgatcgagagttcgacgatttcgagttcgctgaaatttgccttgagcgcctcgaactcggcgtcacgggcttcatgacggtcggcgaggcgcgtcagtgtttcagcccagtcgagcgccgcgcgctcgcgctcgttgaaaaagctcacctcgcgccaggtggccaggctgttgatgcgctgccagtcttcgccctgctggcgcaggtcgcgcacgtgcatgtccaggcagtaggcgcagccgttgatctgcgagacgcgggcaaagacgaggtcgatcagcaccttgccgagcgtgctcgattcgatggtgccgttgacggcgatcatggcctggaaggccttgggggcggtcttgtaccaggtgaggcggggggcgacggtgttgctcatggcgtgtactccaggtggttgagattgaaaaatctgcttgctacctgttgaagacgggccggcccccggccctgtgacacgccgggcgatttatttcgaagaaaagtgctgggcgatgcgcgccagcttgtcggggttgcgctgtgcgcggatgcgcacgatgcgctcgccctcgatctcgaaggtctgcgccgattcgagctgcccgtcgacaaagcgcagcagcccgggctcgccattgatttccgccagctccatgcgcaccgccgcgcccaaccggcgccagagcgcgaagtacagctgcgccagccgctggctgccgcgcagcaccttgctgaagctctgcaccttgccgccgccgtcgccgatgagctcgacgtcttccgccatgagcgccttcaggtcatgcaggctgccgcgcgcggccgcatcggcaaaggcgcgcagcaggcgctggtgggtttcgcgcgacacctgatagcgcgggcgcgcctcttgcacctgcgccttggcgcggtgcaccagctgccggcaggcggcttcgcttttgccgagcgtgagcgccacctcgtcgtagtcggcgtcgaacacctcgcgcatcaggaaggcggcacgcgcctcgggcgccaggcgctcgagcacggcaaggaacgcgacggagatgttgtcggcgcgctccagcgattcttccggcgtgtcgggcgattcggtcagcgtgggctcgggcatccaggccccgacgtagtgctcgcgctggaccttggcggcgcgcagccgatcgatcgaaaggcgcgtgacaacggtgaccagccaggcttcggcgctgtcgaaaccggccttgtcggcctcatgccagcgcagccaggcatcctgcaccacctcttcggcctccgcaacggagccgagcatgcggtaggcgatgccctgaaggcgtcggcggtggctatcgaaagtgagggtggcgtcgtccatgttcggctagacggccggcaacgcgtctttgtgacaccactgcccgcaatccggccgaaattatcggggaacggcccgccgctacgcgccctggtattcggccttggggccgatggatgcggccaattccttgcggtagcggttgagctcctgcacggtcttgaagctgcggtccatcaagaggctcaggttgtgcaggatgcgctcgccgaccttgctttcccagacggcatcgaacttgatctgcttgtcgagccagtgctcgagccagtccgggtcgggcatgcggctctggatggtgtcgttcgggaacagcgccttgttgacgtgcaggttggtcgggtgcagcgcctgggcggtgcggcgcgcgctggccatcagcacgccgaccttggtaaacgcggcccgggcctcgtcgccgaacttttccatggcgcgcttcatgtagcgcaggtacgcgccgccgtggcgggcctcgtcctggctcagcgtggtgtagatgtgcttgatgaccggctcggtgtgccactgggccgcgcggcggtaccagtggttgaggcggatctcgccgcagaaatgcagcatgagcgtttcgagcggcggcgcggggtcgaagtcgaagcgcacttcgtgcagctcctgctcggtaggcgcatgctgggggctgaagcgcttgaggtattccatcagcaccagcgagtgcttctgctcctcgaagaaccagatcgacatgaaagccgaaaagtcgctatcgtggcggttgtcgcgcaggaacatctcggtggccggcagcgccgcccactcggtgatggcgttcatcttgatggtttgcgcctgttcttcagacagtagcgaagcatcgaacgactgccagggaatgtccttgtccatgtcccagcggacagattcgagttgtctgaagagttccggataaagcatcaaaatctttctaaggccgccgattttagtcggcccgtttggcgcgtcgatgacagacgcgcgatgatgcgaatacgtgcttgcctggcggcacggattcacacccccatttttgtatcaggagcccccatgcgaaccccctcccgattgtcggcgcccaggcgctgcactccggccgccgcactggcagcatgcctgtttgccctcgggacggcgggtgcccagaccccttccgcggcccctgctgcagcggcatcggccgcccctgccgacggcgttgccaccgcctgtcccgcaaccctgcaacacaccttcccgcggctgcaggacgaaaaaccccaagatttgtgccagtactccggaaaagtggtgctggtggtgaataccgcgagcttctgcggctttaccccgcaatacaagggcctggaagcgctggacaacaaatatcgctcgcgcggcctggtggtgctgggctttccctcgaacgatttctcgcaggaatcgggctccaacaaggaaattgctgatttctgcgaaagcaccttcggcgtgaagtttccgatgttcgccaaatcgtcggtgcgcggcgccagcgccaacccgctgttcaagcagctggcgctggcctccggcaccacgccgaagtggaacttctacaaatacctgatcgggcgggacggcaaggtggtccaggcctggtcgagcatgacggcaccggacgaggcggccttcgtgaaggtcatcgagagccagctggccgcgcattgacgcgctgggcgcaaaccagtcgtcacaaacgtttaccactggagggggaaccgggctggcacactgtgctcatatcgagcgtgggcagcaaatgccctccggtttcatgttgcgaggtcttctgggcgtcttgtctggttgaaatcccgaggcgattcttctcctcctccctccctccctccttcgcgtcggggcgcctcgcagcatttttgtatttccctccggggcggggcgccgcaacacaggcgccctgaaacgaaaaaggcgccagaggcgccttttttcatggttgggtgtcgatgaagctgggccgaagcagcagcttgtcgtacaactttgccaggttggagtgctggctgcgccagtcgatctcggggaagcggagcccgacccagcccagcgcacagcccacggcgatatcggacaggctcaggtggatgccgctgcaaaagggcttgtcgttcagccccttggccatagcggcgatgccgccttcgaccttggcgcgctggcgttcgatccaggccgcgctgcgctcgccgtcgctgcggccggtccacgtggcttccaggcgccagagcacgccggcgtccatgacaccgtcggccagtgcttcccaggtcttgacttcggcgcgctcgcggccctgctgcggaatgagcttgcccacgggcgacagggtgtcgaggtattcgacgatgacgcgcgaatcgaacatcgcgtcgccgccttccatgatgaggcagggcaccttcccgagcgggttggagtgggcaatggtggtgtcggcagcccagacatcttcgatcacgaactggtagtcgagccgcttttcggccagcaccacgcgcaccttgcgcacataagggctggcggccgatccgatcagtttcatgaaagctctctccctaggctttgatttacgtttattcaacttcattttaggggaacgccaaaagggcggcctcgatctgtcgcgaacgcacgtcgccgcgggccgcctaaaattcgggcatgagcttctccaccgtttccgccctctccccacttgacggccgctatgcggccaaacttgcggcactgcgcccgctgatgagcgaacagggctatatgcaccggcgcgtgcaggtcgaagtggcgtggttcattgcgctgtccgactgcggctttgccgaattcaagccgctcacgggtggcgcccgcaagtacctgctgggcctggtggcccatttctcggaggccgacgcactggccatcaaggaaatcgagaaaaccaccaatcacgacgtgaaagccgtcgaatactggatcaagtccaagttcgacgcccggccggagctgctggccgccgccgaattcgttcactttgcctgcaccagcgaagacatcaacaacaccagccatgcgctgcagatccaggccgcgcgcgagaaagtggtgctgccggcgatcgacgggctgattgccaagctgcgcgagatgtcgcaccagttcgccggcgtgtcgatgctgtcgcgcacccacggccagaccgccagcccgaccacggtcggcaaggaaatcgccaacgtggcggtgcggctttccaaggcgcgcgcgcagattgcctcggtgcagctgctcggcaagatgaacggcgccgtgggcaactacaacgcccacctggcagcctggcccgatttcgactgggaggcgttcagccgcaaggtcatcgaaacgcccgcgccgctcggcctgggcctggccttccagccctacagcatccagatcgagccgcacgactacatggccgagctgttcgacgccgtggcgcgcaccaacaccatcctgatcgacttctctcgcgacatctggggctacgtgagcctgggctacttcaagcagcggctcaagaagggcgagatcggctcctcgacgatgccgcacaaggtcaaccccatcgacttcgagaacgccgaaggcaacctgggcctcgccaacgcggtgctgcgccacctgagcgagaagctgccgatcagccgctggcagcgcgacctgaccgacagcacggtgctgcgcaacatcggcgtggccttcggctatgccacgctggcctacgcgagcctggccacgggcctgggcaagctggagctcaacgaggaggcgctggccgaagacctcgacgcttcgtgggaagtgctggccgaaccgatccagaccgtgatgcgccgctttggggtgcagggcgcctacgagcagctcaaggaagtgacgcgcggcaagacggtgacggccgaggcgctgcacggactgatccgctcgctcgacattccccaggcggaaaaagagcggctcctcgccatgacgcccgcgagctacgtgggcaaggctgcggagctcgccagtagaatctgaggcttcccgcaccgacgctccggccgcctgaaggcggctgcctgcgtcgcttcacgcccctcttcagccaacgcgcccttcgcggtgcgccagccaacaacctgacggggcttcaaagcccctgttgttcatgctgcgcgcccccctccgacgcctctggctcaaggttcaccgctggatcggcctctcgctcgggccggtacttgccctcacggcgctgctcggcgcggtgctggtggtggccttgccgatcgaccgctatgcgcatcccgagctcttcgtggcccggaacacggccgttgcggcgcccgcattgccgctcgagccactgcgccaacgcatcgtggccgagttcgggcctgacgccaccctcacactgcgaccgccgcgcactcccggcgagacgctctgggtgtatgtgcgcgggccttgggacggcacgctctatctcgatcccgccaccggcgcggagcaaggccggcgcgggtcgcatgagggcgcctacaacctgcttttcgagctgcacagcagcctgctgctggaagacaccggcaagggcatcctggccttcgtggcgctggcctacctgtgcctgctggtcaccggcgtggtgctctggtggcccacgcgctggccgccttcgctacggattgcgctcgaccgcggcctgctgcgcgggctgttcgacctgcaccgcaccggcggcgccgtgctcgggctcttgattgcggtgtcggtcttcacgggtgcctacatggcatggcggccgctcggcaacttcatttcggccgccatgggccaggagccgatcaagccgcccacggttcccaagggcacggccgcagggccccggctttcgctcgacgaattggtcgcccgcgcgcagaacgtgttcccgggccagccgatcggctacgtgcaggtgcccgccaggccgaaccgcccgatgcgggtgcgcttccgtctggccgacgatccgcatccgaacggcatcagctcggtgtggctgcatccgctgaccggcgaggtgctggcggtgcgccgctggcaggacctcgaccccggcaacggcgcggtggtggtgatctatccgctgcacaccggcgtgctgggcgggccggtgcaccaggcattcgtcgcgctgcttggcctggcactcgccggcctgggcctgagcggcgtctggctctggtggcgacgccgcgccgtggccgccgcggcccgcggcaccgcgctttcgaacaacaaccgcacgacgtcctgaacgggacgtctgctgcggtcgattttttattgatatccgaggagaacccgtgttcaagcagaagaaatgcgccgccctggtcatggcgctgttccccatcagtttccagagctttgccgccgaagccgagccggcgaccgatggcacgaagtcgctggaggccgtgaccgtcacgggcgactggctcggcacgcccagtgaaaccaaggtgctcgagcaccccggcgcgcgcagcatcgtcgagcgcaagcagatccaggagagcggctcgagcagcgtgcgcgacgtgctgcgccaggttcccggcgtgcaggtgcaggagagcaacggcacgggcggcagcgacatctcgctcaacgtgggcgtgcgtggcctcacctcgcgcctgtcgccgcgctcgaccatcctgctggacggcgtgccgctggcctatgcgccctatgggcagccgcagctctcgctcgcacccgtgtcgctcggcaacctggaggcggtcgacgtggtgcgcggcgcgggctcggtgcgctatggcccccagaacgtgggcggcatcatcaacttcgtgacgcgggcgattccgaagcagttcgcgggcgaagtgggcgtgggcgtggaaagcgcgagccacggcggcggcatcaagaccacgcccaccctcttcatgggcggcaccaacgagaacggcctcgggcttgcgctgctgtattcgggcacgcacggcgacggctttcgccggagcaacgaccacaccagcatcgacgacctgatgctgaagggcgcctatcgcctctcgagcacggacgacatcgccgtttcgctgcaccacttcgaaggcaagggccgcatgcccggcggcttgacgactgcgcaatttgccgcggacccgttccagtccgaccgccctttcgacgaattctccgggcgccggaccgacggctcgatcaagtacacgcacaacgacggcgtgaacaagttcgaaatgctgagctactacaccgactcgttccgcagcagctacctcgagcaggaaggcacgggcgccaatgccggccggcggcgcctgaccagcgcaccgcgcaactacaagacctacgctttcgagccccgctactcgcgcttgatcgattcgggcagcgtggtgcaggagatcagcgtcggagcccgctatctcaaggaagaggcctccgaggtggcgacgcgcagcacctactaccggccgcgcccgggcttcgatgcattcacgctcgcgcagcctgcgtaccagtcgagcaaaggcggcacgaccgcgcacgcgttctatattgatgaccggatcgactttggcaactggaccatcacgcccggcgtgcgctacgagtcgatccgctcgcacaacgacgtctacaccctggccaacaaccgggtcacgggcgcgaactttccgaagatcgactccaacgaggtgctgccgacgctgtcggtgctctaccgcatgaacgagcgctggtcggtgttcgcgaatgccggcgtgtctttcggcccgcagcagtacgcccagcttgcgcagtccaccaccggcctgcaccccgagaaggccaagacctatgaaatcggcacgcactacaagggcgaggcctggagcggcgagctgaccctgttcaacatcgatttcgacaaggaactactgctcgcgcgttccatcaccggcgacgtcggccaatggaccgacctgggcgccacgcggcaccgcggcgtggagtcggccctgcgctacgaccttggcacgctgagcgaatcgctcaagggcgtgtcggtgtccgcgacgtacacctacacccaggccatcgccaaggccggggcttttgccggccgcgacctgccgttctactcgcgccaggtggcgacgctcggcgcgcgctacgagcgcgggccgtggaccttcaatgccgacgtatacgcgcaatcgaagcagcgttcgccggggtcgcccgacgacggcgcaaactacgtgacgatggaagactcgaccggccgcctgggcaacattccgggctacgccaccatgaacctgcgcgccgcatacgacttcggcccgtcgatgagcaacctgaagctggccgtcggcgtcaagaacctgttcgaccgccgctactacaaccgctcggtcgacaacaacggcggcaagtacgtgggccagccgcgcaccgtgtacctgcaggcgtcggtggcgttctgatgaagcccatgggggcgcatacactcgcgcacccatggccctcaaatccaccatcttcaaggccgccctcgcggtggccgacatcgaccacggctactacgccgaccatgcgctgacactggcgcgccacccgagcgagaccgacgagcggatgatcatccggctcgtcgcgctcgcgctcaatgcgcacaagctgcaggacgtgtgccagggcgacggcacgctggcctttggcgccggcttgtcgaacgtcgacgagcccgacgtgtggctgcgcgatttcaccggcgagaccaagctgtggatcgaggtcggccagccggaagacaagcccatcatcaaggcctgcggcaagtcggacgaagtgatcgtctactgcttcaaccacgcggccgagatctggtggcgcggcatcgagaccaagctcacgcggccgcagaacctgcaggtgtaccgcgtgccgaccgaggcctcgcaggcgctggccgcactggcgcagcgcagcatgcagctgcaggcgacgatccaggaaaacacgctgacgctgggcgacggcacccacagcatcgacgtcgaactgctgcggtggaagtagcgccttaaacaggcggcatcatcgcgccgcagtgccagcactgctcgaagccgccttcgatccgctcgccgcacacgcattgccagttgcgctgaggcctgtgctgcgccgcatgcagcacttgctgcgcgcgctcgaactgagcttcgtcgtcgatccagatttcaggcaggcattggtctggcggcagctggcccatcacggcgccgagaaattcacgctgcaccgtcgcttggacgccctcctcttgcaacgcgtgcacccacaaggtcgcaatcgcgagattgggtgcttgggcgaggcggcgcattcggcggcccctttcagggcgtgtcgtcggggccgaggggctcggccgggtcgtcgggccattgcggcggctcggcctcgcgcgcgcgctcggcgtacttgttgaagcgccaggccgtgtcttccatggtgatgcggcgccaggtcacgcgcttttccgccggcgacatggcgggccaatgctgcacctcgtcgaagctgcggccgcagcccttgcactcgtcgtcgccctggctggtggagcagattgctatgcagggggtgtcgggcgtgctgtgataccagtcgagccaagcggcccaggcatcggggggaaatccgaactcgtcgacctcgtcttcgtggtggaacaccatgagcgcgtagacctcggcaagcgcgcgcaattcgggcgccagggtaacgccgtcgggcgagggactcttctcgcgccaatgattgatggcggcctcgatgtcgatgatgtgaatggcggccatggagagagaaaaaacagcgagcggcgatcatagtccggcaatgccccgcggccgctgaaggttataggcgctacaaaattcatagcttcatgcccttttgaaccaggctcttcaaggcattgcttttgcagcatcggaaatttcaggttgccagaacaccggtcaggatgctctaattcgccccacgaaggggagtagctcccaactgccgcacaacggcgggaatcgactggtcgtcaatacgaagcacaacacttccggcctgtcgggcaacacgtgcccccgggcatgcgctgtcgagcaagaccttcgatttgaacctgcgcaggtttggtcgaagcgttccagaatccccggtcattcgcccggtcttcgccatcgcttcgacattcctgcacgggatggatcgaaatgcaacgcatgcgccggactgtcgccatccaacccaggatggacggaccgcgcgaagacaagaggaacctatggaacagttcatgaccccggaattctgggtcgcggtcggtcagatcatcatgatcgacatcctgctcggcggcgacaacgccgtcgtcatcgccctggcgtgccgcaagctcccgcctgcgcaacgcaccaagggcatcctgtggggcacggccggcgccatcgtgctgcgggtgatattgatcttcttcgcgctcaccctcctggccattccgttcctcaagctggtcggggccgcgctcctggtgtggatcggcatcaagctgctggcacccgaccatgacgacgcgcacggcaacatccagagcagcgacaagctgtgggccgccgtcaagaccgtgatcgtggccgacctggtgatgagcgtggacaacgtgatcgccattgcaggcgccgctcagggcgccggccagagccaccagatgccgctcgtgatcttcggcctgctggtgagcatcccgatcatcgtctggggcagccagctggtcatcaagctgatggaccgtttcccgatcatcatcacgctgggtggcatgctgctgggctggatcgcaggcacgatggcggtgtccgatcccgcgctgtcgaacaccgcggcctggacatgggtgccgaaggtgccgcagaccgacatggtcaggtatgcagccggcatcgccggtgcgctgctggtgctggtcatcggcaagtgggtggcagtgcgccaggcgcgccaaaagcccgccgaggccgtcacgtcgagctgaacgccggcaggcgccggcaaaaatgcccttcccctttcggccagtctctgccactctagctacctgaaggagcgcaccgtggaaacgatcattctctatgtcgacgacgccggctatgcctgcgagcagttcgccgaactgactcccgacgccaacagcgtcgtggctcgtcattgggtgctcgtggcctgcgcaccgcgcatgacgcatcgcatcagcaaatgggtgagccacagcgcacgagagaactggcgcgccaagtggttcagcaaggtgcaggcgcagctgctgccagtgctcgaacgcaatggcggacaggtgacaccggtgcttgccaagggcccgctggccgatctcacgcagcagctgaagcgcgagcatgcagccacccacgtggtcgatgcgcgccgccccaagatcggtgtcgacctggaaccggtcacgcccgaccagacgccgccgcgtcaatcgggctgggcctttccgggtgccgtgatgggcatgggcgccctgctggtgctcgcgaacgaactggccgaataaacacacactgcttcacgacgagccccggtgcggcaacgcgccggggctctcgtttttttgcgggccggtggggtatcctgcggcgcatgcgcatcatcctcaaatggctgctcagcgccgtcgcgctgctggcggtggcctatctctacaacggtgtccaggtcaacagcttcggctccgcgctgattgccgcggcggtcatcggcttgctcaacatggtcgtgcggccggtgctggtggtgcttacgctgccggtcaccatcgtcacgctggggctgttcctgttcgtgatcaatgcactgctgttctgggccgcgtcgggcctgctcacgggcttccaggtcagcggcttcgtggctgcgctgatcggctcgctgatctattcgctgctgggcttgatcatcgaagccgcgctgggcgggcttctgtccaggcgctgagccgccggcccgttcgtcgtcattgcctgagcggcggctcttcggcctgccgcttcaccaatgcttcgacgtcccgcgcgcgggtgtcgatgatcgacgcctcgtagtggtcgatgggcgcgccgggcttgcgcaccagttcctgcgcggccttgaagcggtcgcgcgcggcggggtagtcgaggatggccacgttggcttcggcatcggcacgcaccgcgcgcagcgtgtcgttctgcgcgccatacagattggccagcgcccgccaggcggtggcatcgcgcggatgggtggcgacccaatcgcgcagcaccggcaccatgggcgcgggctggcgcgtggccacggccgtgtcggcggccagtagcatctcgggccgctccttggacttcgcatccagcaaagccgcggccttggaagcgccgccgccggcgagttcgatttcggccatgagccagcgcgccagcctggcggccgacgggtcttccgcggtgcgtgccgtcagccgctcggccagggcgcgcgccgccttgaaatcgcgcagatccttggccgacagcgccgctgcgtagagcgtgccggcctgctgggccggaccgctcctggcgaactcgccgctggaagccgcttcgaccccgagccgcagcacgtcgacacccggccgcgtgagcacgcgcgcacgcgcggcaatcatggcgtggtccatggccagcggcatggccggcgcggcatcgaggcggaactggaaccggccctgcatgtcggaaatgcgctctgacgtgagcggatggctgcgcaggtagggataggagccgttgtcgttgaggcgcgaggcgtactgcagcttttcgaacatggcggccgcgccctgcggcgcaaagccggcctgcgtcatcacgccgaagcccacacggtcggcctcgcgctccatgtcgcgcgaaaagctcagctggttctgcatgaagagcgcctggctgcccatgattacggcctgccccgcatcggcgttgcggctcttgctggccgcgatcatgccgaggatcaggccggccagcatcaagggcatctgcttgccctgccggctcatgatgcgcgagatgtggcgctgcgtgacgtgcgacagctcgtggccgagcaccgttgccagttcgtcgcggctgcctacggtggcaatcaagcccatgttcaggcccaggtatccgccgggcagtgcaaaggcgttgacgttgcggtcgcgccccagcaggatggtccacgcaaagcgctcgtccagctcgggcgtgagttcgccgcgctgacgtgcggcggccaggagccgctgccagatatcctgcacgtaggcggcgatgacggggtcgtcgatgtagtcggtatcgcgatagagctcgcgcgcgatctggtcgcccagattgcgctcggcgctggcggtcatctcgccgccgtcgcccaggcctggcagcgcttgcagttgcgcgcgggcgggtaccggcagcaggatctgggacgctatgagaaccgtagcgcacagtgcccgcaatgcgggcacggcagaattttttttcgtgtcagaaggagtcaagcgcggcattcctcgtccatggctcgggctcgtatgatgcacctccacaccgatcgttcacacatgagttccctcacccattttgacgctcagggccaggcccacatggtcgacgttgcggccaagcccgccacccatcgcgtggccgtggccaccggccgcatcgagatgcagcccgcgacgctggcgctgatcgaatcgggaaccgcaaagaagggcgacgtgctcggcatcgcccgcatcgcgggcatccaggcggccaagaaaaccagcgacctgattccgctgtgccacccgctggcgctcacgcgcgtggcactggcctttgcgctggccgaaaaaggcaatgcaccgcaagtggtctgcaccgcgacggtcgagaccgtgggccccacaggcgtcgagatggaagcgctgaccgcggtacaggtcgcgctgctcaccatctacgacatgtgcaaggccgtggaccgcgggatgcggatcaccgatgtgcatgtgctggaaaagcatggcggcaagtcgggcagctacgtggcggagtaaaggcggggtcgagccaggctgtcaaggcatatcggcctcgaccggctggcccttcagccagcgctcgtactcattcggaaaggcaatgcggaagcgttccgcctgatcctgggcttcatggcctcggcccatcagttcggcgctttcgatcagcttgacgatcacgcgcggctcgggtgaaaagtgcagcgtgcgctcggccagcgaatgcagcgcggccgcgttggcgggggtcaccgccgtgagcgtcagttccgcaaaacccacctgccttgcgaagagccacgaccccttggccttggccagcgtgctttcttcataggccggcaagcgctcgtcgcgcggcagatatatctggctgatgcggatgtagtcccacgtggcatagccgaccatcgccatcaacacggcagccgcggcggaagagaacacaaccggctccgcccaccggcctttgccgaagcgctgctgccgcaggggcgatgaagcgtggcgcctggcgggccacagcattcccaggcacagcccgaacgccagctggaacggcccataccaaagcggatattcgagcaggctgtgcaatgcaatggcgcccagcatgccccacgccatgagccgcgccggatcccgctcgcgccaaggtttggccgccagcaccatccagatgaagccgccgcagatcagcaccgacaccgggatgcccagctccacggcaaggtgcagcggcaggttgtgcgcgttgtccaggatctccgggaaccgtggcccttcgtacagcgtgctgtagtgcgcgaagctcagctcgccccagccccaccccgcgagcggatgctcggcgatcagcgtgagcacattgcgccacaggatgaaccgcgtgtggtcgccgggcgcgccctcctgcaggcgccgcatcatgccttcgacctcgcccgccgcaagctgcggcagcacccaggcaatggcgaaatagaccggaatcatggccagcagcacccacggcggcggcaagctgaagaagcgaacaacctccgccgcactttcttcggacacgccgcggcgctcccgccgcgcgatcaaggcggccacgccgacgatcgaaagcaattgcagcaagcccgtgcgcgacgtggacgccgccgcggccaccagcaacagcaaggccgccgccaccagccagcgccgcgcacgcaccgaaggctgcgtggcgtaaatccacagcgccgccaccagcgccatgctgatcagcgtggcgaactggttgcgctggcgcaagttgccgtaggcctggcccagcgcgggcgtggtggtccagggcaccagcggctccgccaggccgtagtactggagcaggccgagcacggcgctgaccaagccagccaccaggatgcccaccgccagcgccgccgaagccgaaggcccgccacgcgccatgccgaccccgacgcaggccgaaacggccacggcgcccagcgccgcgacagctggcagccacgaagcggcggcggcttgcgaggagaagaaagaagaagacagcacgatcgccgccgctgcggccgccagccagagccagacgctccgcgccggcgcgcccggacgaatcaccagaaccatcgccgcgaggcaaacccaggttgcaaacagctgccaggcctgaaccgaggggcccgccacgagcgggcagagaaagggaaacgcgaccaggccggcgcgcagggcgccaagggccttcgatgggaggacggccacctcgagaggtgctgtgcgggacgtcatccggtcgattgtgccggccgggggccgggtgagccgacgaatggctacgggcgggagacgagcggttttgcagaaaaacacaattagagacattctttgacaactgtctacaactgctgtccgcctcccaaaaagggattgcggccacgaaaggtgtcaatgaaacaacaagcgattccacgcgaaaccgtggcaaatcgacacggctctcgcggcttcacgctgatcgaaatcatgatcaccgtggtcatcatcggcgtgctggcggccattgccattcccagctaccaggactacgtacggcgtggctatgtggtggacggcaccaatgccctggcgaccatgcgtgcagacatggagcgctacttccaggacaaccggacctacgcgacgacgccgggaggtctggttccgccctgtgacgccactgtggtcgccagcaagcgcacctttggcaatttcgtcgtgacgtgtccggcgcccaacgcgcccactgggaccacctatacgctcagggcagcaggaagcggcccagccaacggcgccatctacacgatcaatcaggagaatgtgcgcgctacggtggacatgcctcccgcgtggggctggaccaggacatgcacctcctcctggatcgtgaaaaaggggcaggcgtgctgatgcagcagggctcccatcggcgccagaaggccttcaccctggtcgagctgatcgtcaccgtcgcgatcatggcgatccttgccgctctcgccacgccctcgatgattgggtgggtgcggaacaacaagatccgcactgtcagcgattcgctgcagaacggtctgcgcctcgcccaagcggaagccacccgccgcagccggcaggttgtcttctcgctgacgaacgacaaacccactgccagcggctacacggctgcgaccaatggcagcaattgggcaatcaacaccgtgacgttgatgaccgagggcgaaaccagcgcattcgtcgaggccggagtcctgcgagacgtcggctcgaacgtcgcgatctcggggccggaggcgatttgcttcaactcgctcgggcgccttgttccgaatgcctcgccaggcgtgaccagcgctgtttgcgaatcgccgccgatggccgggtattcatacaccattcaaatgagcgatagcgtcgaaggcgatcgcccgctgcgagtcacagtcgccctgggtgggcaagtccgcctgtgcgacccggccagaaccctttcggacagccagcccgacggctgccccgccgcgccatgaaacgtacccgcacctcttctcgccgcggccaaaccggcgttgcgctgctcgaagttctggtttcagtgctgctcttctcgctgggcgtgcttggcttgatcggtcttcaggcacgggcgatcaacctgtcgatcgatgcggaagaccgcaaccgcgccgccctgatcgccaacgacatcgcagcagccatgtggaccactcggacggtggcgatcgacgccgctgcctggaccacccgcgccagcaacccgctggccggcggcctgcccgggggaagcgtcgcgatcacttcggacgccacgaccaacaccgccgacatcgtcatcacctggacccccccccagcgcgcaacaaccggcgaacaggccagccgcctcaccacgcgcgtcgcgctgccgcccaccccatgaacgcccgctccatgccctttgcccgcgccgcgcagcgcggcctgacactgatcgaattgctggtggccatggtcatcggcctggtcgtggtgctcgcagtgaccagcgccgtcacgttcggcgagtcgcacaagcgcagcaccacctcgaccaacgacatgaaccagagcggctcctacgccgtctacaaaatcgaccgcctgctgcgaagcgccggctccggcttcgcgcagaccggcacgcgcgggatgttcggttgccggctgagcgccgcgcgcctcatcggcggcacggccaccacaatcctgccgcgaaccgcatccgcgtttccggcgccgttcaacacgctgctcggcggttccggggccgccgcggcggggaatctgcggctggcaccgttcctgattgccaagggcgcctccggcgcttcggacaccctcgtggtcatgggcggcaacgcggcggcgggcgacgtgccgcgccgtatccgctccgggattccgggcaacgacaacctgcggctggacaacaccatcggcctgagcaacggcgacatcggactggtgagcaaagaaggcacggccgactgcctgctcgagcaggtgagttcgacgaacgcggaactggcaacggcggggaacgaagtgctggggatgggagggcgctacttcacatcgaccggcgccaccacgtcgcttgccacgctcgcggcggacggcacggcgctcttttcgccgctcggcaatgtgggtgccaacaacctgcagttccagctggtcggcgtgaacgccaatcgcacgctcgtcgcctacgacctgctgcgggcggccggcaccggcagcgacgagggcaccgacgcatcggccatgcaggcgctggccgacggcgtcgtcgccctgtatgcggtgtacggtgtcgacaccgacagcaacggcgtcgtcgacacatggatcgaccctgccgccacgggttatgcgattggcacgctcatgctcgcgcccgacaccatgcgccacatcgtggcggcgcgcgttgcgctggtcatgaaaagcagcctgttcgagaaggaacccgtcacggcgggcagcctgaccgtcttcagcgacctcccgacggatcgccagcgcacgctgaccatcgcgacttccgaccggaacttccgctaccgcgtcatcgacaccaccattccgcttcgcaacatgctgttgctgcctttcccatgaagacacttttcaagatacacgggccggcgcgcgagcgcggcgtggtgctgctgttctgcctgatcatcctcgtggtgctgctcgccggcggcgtggcggtcatgcggtcgatggacacctcgctggtcggggccggcaacctcgccttcaagcgcgacctggtcaaccagggcgaactcgcaatcgcgaaggcgatgcgggagttccaggccagcggcgcgctcgctgcgacgggagcgacctccagcagcctgcccggggcgaactacagtgcgatccagctcgttgccaatgcccaaggcatcccggaggtgctgctcaagaagaccacgctgaccggacccgatgtggtgggcaacaccttcgcgccaaccggcacccccatatcgggcagcggcggggtcaccgtgcgctatgtgatcgaccgcatgtgcaacgccaccggcgcgttctcgaccatcggcaagagcggctgcgtctacaccccgtcgaccaccgaaacgctgggtggcgaccagagccagctgagcacgcccggcccgtccattcccagtccgcccatctaccgcgtctcggttcgcgtcgatggtccgcgcgacacgcaggcgttcctgcaagcctccttcaccaagcccgaatagggcacaggcgagtcatgaaaacaagaattcgttcgtccgttcgcgcggtgtgccgcgccggcatcgccaccggcctggcgctcggcagcgccatgttcgcgtccgcgatcccgctcgccaaccagcccgtgttctcgacctcggaggttccaggcaacctggcactggcgctgtcggtggaatggcccacggcatcacgcacggcccacgtcggcgactactccagcaacaccaactacctgggctacttcgatccgggcaagtgctacctgtaccaggtcgacgccaccgccaacggcgtcagcacgaccgacaagggcgactccagctacttctacccggccggcgccgccaccaatcgcacctgcacgggcgacaacgacgacaagtggagcggcaacttcctgaactgggcctccaccgccaccatcgaccccttccgctgggccatgaccggcggaaggcgcgtggtcgacacggccaccaccaccatcctcgagaaggcctggcacggcaaccgcagcctctttccggaccgcaacctcacggcatcggccatcgcaggcgccacccccttcaacagtgccaccgcactgggcgtgagcatcaccaaccgcggcttcaagatgcgcatgactgccacgggcggcggcacccgcacgatgtcggcgcagtacttcaacaacatcagtcttaccaatccccggttcgccctcgtcgatacggacaccgccgaccacgattggggcaacggcagccccgtgaccggaatgaatgccgacaacttttcggcgcgcttcaacgggacctatacggcgcccgagaccggcaactacacgttccgcaccatcagtgacgacggcgtgcggctctgggtcaagaccggcaacggcaacaatttcggcaacagcgacctccggatcgacaactggacggatcacggtccgaccaccaacgattctgcgaccatcgctctcacggcgggtcaggagttccgcgtgcagatcgagtactacgagcggggcggcggcgcggtgatgcagttccattggcgcacgccctcgtcgaccgccttcacgccgttctccgtgaccgggccggtcgatggcgacttcacgatgcgcgtgaaggtatgcgacccctcggccgcagccggtggactcgaggccaactgcaaggcctacggcaccaactacaagcccgaaggactgatccagaagtacgccgacaagatgcgcttcagcgccttcggctacctgaacgacagcagtgaccagcgcgacggcggcgtgctgcgcgccaggcagaaattcgtcgggccgaccgcgccgacccccggccaggcgccctcggccaacgcgaacaaggagtggagcgagaccgacggcactttcatcggcaatcccgacgccgccgatgcgaccgcgaccacgacggcgaccggcgtggccatcgcggacagcggcgtgatgaactacctgaacaagttcggccagatccttccgggcgactacaagaactacgaccctgtcagcgagctgtactacgcagtcatgcggtattacaaaaacctcggcaacgtcgcgggctggagctcgatgggcactgccgacgcccccacgaagaccagttgggtcgacggtttccccgtgatcaccaactggggcgacccgatccagtattcgtgccagcgcaacttcgtgctgggcatcggcgacatctacacccacgtcgacaagaacgtggccggcaacaccacctaccgcacccgcgagccggccatgcagaccgaggtggagaacgacaacaccgtcaatgcggtcacggccaccaaccgcgtcggtgcgctgcagggcctgggcgacctcggcaactccaacgactacagcggtcgcaacaactccgcctacatcgcgggccttgccttcgacgccaacaccaaggacatccgtcccgacgtggcgggacaggccaacaccatcggcaagcagacggtcagcacctactgggtggacgtgcttgagcagcccttccaatacaacaaccagttctaccttgctgccaagttcggcggactggaccagaagaagctgccagccgacttcgacccctacaccttcgctggcaccattccgctggactggtggtccaccagcggcgagacgctgaccgacgcacgcgccgcgaacctgacgcagccgcgtcccgacaactactttgccgcaggccagcccgacacgctggtccgcggcctgacgcaagccttcgaacgcatcgtgaacgccattcaggcgtacaccacctcgttctcgctctcggccctgcaggtttcggccacgggctcggcttcgtatgcctcgcagtacgacgcccaggactggaccggcgtggtgagcgcgagcagcatcagctttgccgccgacggcacgccctcgctcacggcggcatggaccagcaccgacaagctcgcgacgcagttcgccggcacgggctggaacaccaaccggcgcatcgccacctggaacggcacggccggcgtgcccttccgcatcggaagcctcaccaccggaacgggcagccaggcggccgcgctcgacacgctctacgtcaccggcgacgacagcgccaactacctgaattacctgcgcggcgatcgcagccaggagaagacggcgatcgatggaaccaagccctaccggcttcgcagcaagctgctcggcgacatcgtcaacgcgaaggtgaagcccgtgggcccgcccgcatcgagctactccgacgctgtgaaccgcggctacgccgccttcaagacggccaaggccacgcgccccacgatggtctacgcggccgcgaacgacggcatgctgcatgcattccgcggcgaactcaccggcaccagcgccggcctcgaacagtttgcctacgtgccgaacgcgctcttcaacggccccagcaacccgaccacgccggccgcggacggcctggcccagctgggcaacccgaactacctgcacaagtactacgtcgacgcgacgcccgaggtggtcgacgtcgacttcgaccgcgccggcggcaccttcgcggccaccggctcggactggcgttcgctgctggttggcggccttggcaagggcggcaagagcttctacgccatcgatgtgaccgatccggccacgatgaccgatgaaaccatcgttgcaagcaaggtgctgtgggagttcaccgatgcggacatgggcttcagctacggcgcgcccctggtcctcaagaccaagcgctatggctgggtggtggtgctgacctccggctatcacaacgacaccagcaaccacaacggctacctctacctcgtgcatccggaaaccggcgcactgctgcagaagataagcaccggcgcgacggccaacggcatgacccacgccacggccttcatccccgacctgaccgacggcacggccgacgcgatctacgtcggcgacctcaacggccagctctggcgcttcgacgtgaccgcgcccgcgggcacgaccacggactacccggcaccgaccaagatcgccctcttcaccgatggcgccaccaccccgagagcccagcccatcacctcgcgcccactggtgcagattcagcccacgacccgcaagcgctacgtgatggtcggcaccggccagttgctcgatgcgagcgacatcaactccggcgcgacgcagagtttctatgccgtcatcgacggaaccgccaccgccttcaagccggccgacagcaccatgccggtgacacgcagcgcgctcaccgctgtcaccaacctcgtgagcggcaccgtcgttccgaccgattcgcgcggctggtacctcgatctaggcacggaaggcggcatcgggcttcgcttggtggcgagcccgaccgccttcaacggcatcgtggcgttctcgtcgctgctcaccagtggcgatgcctgcagcccctcgggccagagccggatctacgccatcgacttcaacaccggccgcacagcgctggccagcggcgccgcgttcgtgcagtccaccaccgcgatcaccgacctcaagttcgtgggcgtcgacggcaccgtgcgcctgatctccggcgacgtgcgcggcaacctggacaagatcggcttcaggccgccggctggtaccacgctgcggctgctgaactggcgggaagtgccgacggcggattgatcgactagctagttggtcgaagcgcaccctggtacgagatcgatctttgaaagcgctgccagagtacctctgtgtagcgcttttttttgcgaggccttggtgttcagatgctcaggcttgccacccgtatgcgagcgacaaggaaaggcgcaacccgatcatgtgtaacgagtgatgcgggggtagcccccgctgcgcaatttgggctcaagcagtctgaacggcgttggactgcaatctaccagcgggggccgcgctctcaactcgacttgccgaccgcgtgatggcaaatggcgacatcgaagatgtcatcaacgcaactgaatgctcatcgagcagcactgagtgcttgttcgatcaggttcgatgtcatgagcattgcggcgatttgaacgacgcaggcacactgctgagacatgtccaatttcctgccgcgttgcgctgccaagttaatgtttggcctgcgagcacggtagcggccgaatttccaaaagtagcagtcatcactgcgacctgatcgcctgcggcaggaaaagtcacagccggcactccggcgccggcggggagctctgacaacgaaggagcggcgccgttcgctgcgggcatggtcatgagcgaagagcccgcggcgccagggtcgcattgcgaagctcccacgcctacactcgtacgcccctcgatgacgcaggtttcaactatcgtccgcaaggcggcgacttccgacatgacgcgagttacttgaacgcgcgatacgtatgtctgatattgcggtagtgcgatgcttgcgagcacgccaatcaccgccgcaacgatcattagttcgatcaacgtgaatccctgatcttttcccaatctcttcttcatgcgttctctcctcagttggaagattacattgcaggtcgcatgccaagatgcggagaccgggcctcctgacgtcttgtgcttgatgatcgttcaggcgaaagagtgtctgagcctagcgcatagatcgcgtttaatgccctcaaaatacgggactcggagggatcagatcaattccgcgccgaaagcgcagatcgtcgcaattcgcaaattttctgccaaaggtccgtaaatgggaggagcatctgggatagatactccgtatggtcgaccccctctacaccgagcttttcgttgcaaggcccaggaacatagaaagttctgaaagcgcggtcgaaaacgctgaacacagtagcgtagttgctatacatgccttgtcccgcgcgaacgtgatgccatcggtgcattgccggcgagactaacaaccagccggcaattccgagcgtccaaggcctatttatgtgaacaaacattccataaaaatgtcgaactgaaccagcaaacgcgattgcccaaagcggaaatccgagaagaaataaaacaccgtaatctataacagcagtcgaaacccgattgatcggatgaaatctaaacaatgtgaaccaagtcatttcctcgtcgctgtgatggagcgaatgagctgaccagagtataggagagtgttcaagccggtgacgccaatatccgacgaaatcaccggttgcaatacaaatcatgccggccatccacaccggcatagcatccagcgtgggggcaaagaatatcaacccccttgagtctagcacccgataaataacgccgaccagcacggagattggcgccgccacaatcaaagcgtcaacgaaatacaccatcagattgactcgaagactcgaagggcgcagtcttcgtagctcatcccgccaattgcacttgttaatcaaaatggcgattagtactccgcccgtcgtcaaaaggatgagttcttttacacaatcccattggtaccatagcgtattaaggattgactcaatcgattcgttcatttacaccccaccgtagcaacgaaaaagccgcccgaaggcggcctcttgtgacgtaaatgtaaattacggcgaggcagcgacggcagcgccgcaggcagccgtgttgtacttgacatcagcggtgctggtgcaagtccacgtgccgttggcatcacggttccaggtgattgccttcgcggtgccggccgtcagcgtgttagcggccttgttgccgaaggtacccaggatcgaagccgtgccggcagaagcggtgatcgtcaccactggatagcctgcgccggtcacagtcggagcgccagcttgcgcagtaccggagaggatgctcgaagcggtagcaccaggattgcactcgccagcagctgcaccgatggtggtccggccgttgttcatgcagtcttcgatagcagtcttgatggcgccagtttcgccaacagcgcgcgagacctgcgacttggcgatgtacgtttggtactgggggatagcaatagcagccaagataccgatgatcgccacaacgatcatcagttcgataagggtgaaacccttttgcacgttgcgtgcgatcaaacgacggttcattcaaaaactccaggttggttggtagagcccgggaaccagcccggagcgcagtttcttccgcagcatctgtgccacccgtccgggaggccacttcgccatggaaatgaacacttttgttaacactaaatttacatcaagtgacacattccgctccgagatgctacagaacgtgacaattttgtcatgcccggtcgtccgccggactcaaaaagtcaatactccgtccgccttaagccaccgaatgtcccgctgcgccaagccggccacctgatgccccaccagcgcgtcgatctggttcatgatttcttcggtttcggcgggcttggtgtgggtgatgtagatcgggtatttcctgcctggctcgatgtgcgccagctcgtcggccagcaccttgggtgacaggtggaggctgcggtcggccagggcctgctcgcggttgctgaaggcggtttctatgacgagcatggccacgtccagcgcgttgacgcggtcccagaagggggcgttgcgctcggtgtcgcctgaaaagacccagttcgcaccgccttcggcgcggctcacggcaaagccgcaggcgggcacggtgtgcacggcgggcagcacttcgacgcgcttgggcgtggcgctgcccagttgcagggtctggccgacggcgatgtcgtgaaaactcacgaagggggcttcggggctgggaatgctctcgaaatcgggccagatgacgttgttgaacacatgggcgcgcagcgcctcgatggtggcgcgcagggcgtgcacgcgcagcgggcgggtgcggcggccgcccacggcgtcgagcatgagagggagcgcggcaatgtggtcgaggtggcagtgggtgagcaccacgtcgtcgatgcgggccatctcgtcgagcgtgaggtcgcccacgccggtgcccgcatcaacgagcaggtcggtgtcgacgaggaacgaggtggtgcggcagtccttggcaatggcacccgagcagcccagcacgcgaacctgcattgagaaagaccccccgcttgtgtttgtggtcatttggtttcaaaccgggttgcgccgtcccattcggggtcttgaggccgcaacgccatcgaggctaatcgctgggcgtagagctggtaaaggacttttttggcatctgcggcgagcaatgggtccagcagggtccggcccatcgcccagtcctggcggcggtaggcgtcaagtacctgcgcccagcgctgcaagtgctgggatcgctgctcggccgcggggccttgggcttgttcggtgtcggcggccaggggcgtgaagacggcaacggcctgtgccttgcccttgacgagcacgctgtcgagctcctgccagaggcagcggggcgcgagttcgcgggtggcgccgctggcgacgatctccacgccgtagtgcgcgctgaggccctcgaggcgcgacgcgagattgaccgcatcgccaaccacggtatagctgcgccgtgccacggagcccatgtcgcccacgcacatgacgccgctgttgatgccgatgcccacgctgatttcggggcgcccgacggcgcgctgggcctggttgatgtcgcgcacggtgtgcgccatttcgagcgcggcccgcacggccagcgtggcgtggtcgggggtgtcgacgggcgcgccccagaaggccatgacgcagtcgcccatgtatttgtcgacggtgccgcggtgcgcgctgatgacattggtgaggcggctgaacagggtgttcaaaaaggcctggagctcggccggtgccatctgctccgacagcctggtaaagccgcgcatgtcgcagaacatgacggtcatctgcttgctctcggcatgcatgctgtagcggccggggtccctgagcatttcgtcgaccagctgcggcggcacgtaggtgccgaagagccgcaccagcccacggcgcgcgcgggactcgatgaagtaaccccagcccatgttgagcacgaaggccagcgccgccatggccagggacgtggccagcggcagcacaaggccgtggcctaggtaaagccaggcgtttgcgccgaccagcgcagccacggtggcaatgcccagcagaagggcgcgcgtggctggcagcagcgagaggcccagcgccagcaccaggcccgcggccaagaggctcagcacttcgtagccggcggcgtagtcgggcaccgcgagcaggcggtggtcgagcatggccgacacgacgttggcgtgcacctccacacctggaaaaccggcacccacgggcgtgacgcgcaggtcttgcaggccaggcgcagtggcgccgacgagcacgatcctgtctttcagctcgcctggtgcgagccggccttcgagcacgtcggcggcggccacgtagcggaacgagccgccattcgcgccgccggggccgcgaaacggcacctgcatgctggcggtttcgtcgaccggcacgcgcaggcggcccaccagcagggattggagccggggcacggcgccaccggaggcaaaggccggcagcacaggcgggccgccgttggccagccggtagacggcgagaccgagcgattcgtagtagccggaccgcgccgcatcgccttcgtagcgcgcaatgaggggtgcggcgcggatggcgccatcgcccgtcgacgagaccagtgtgttgacgaaccccgacgcaggcgcggcggcggccagcacgggcaggttggcgccaaagccgttccaggccgttgcgtagccgtggcccggcggaaatgcctcgggctggagcaacggagccgcgggcaactggcctttcgcgctcggcttttcggtgcgggtgaagtagtagccgagcgccacgcgccggccttcgagcgcgcgggcaaaggtggcgtcgttgtcgagcgcgggtgcgagccgttcgatgcccgtggcaaggccgggcatgtcgcgcagcggcccgcttgcgatctggcgcagcttgtcgaggccggagctccggtcgggctcgatgaacatcacgtcgaagcccagcaccgccacctgctggcgcccgatgagctcttccgtgagccgcgccaacttgtcgcgcgcccagggccactggccttgccgcgccaggctggcatcgtccacatcgacgatcaccacgcgcgggtcgagcgtgcgcggcatggtggcgcgcaggcgggcgtcgtagagcaggtggtcgagccgatcgatcgcgccgaggcgccaggcgcccgtggagtgggcaagcgccagcaagaccggcagcaaggtgatggctatgcgcggccaatgccgcttcagcgctttcatggcgtcgcacgcacgcgggccgcgctgtggaaaagagaagaaaaaccgaagaaaaagaaagcgtcagacccgcacgaactgcatgcgcgtggcgccgccgagttccagcacgtcgcgctcctgcaagtccacggcgtcggtgcccagcggggcgccgttgagcgtgaccccgcccatgacgctggcggccacgtagccttgccggcggcgcgtgacaaccgccacggcaacgcccggcttgccgacggtggtgaccaccttctgcagcggcacgtcctggccctcgttggcaccggcaagaacgcgcagcaccggcacgccaagctcgatgagcgcgccggattcggtcggtgcggaagacaagggaatggaatccacgaagtcgccggtcgtgtcggtgtgcgccgcgccgccgccaaccgccaggtggctgtcggcgcggaacttgatgcggcagccgcccagttcgatgatgtcgtagtccttgagcacctgcttctggacgacgagtgcattgacgtaggtgccgttggtgctgttgaggtcttcaatttcgacttggccgtcgcgcatgtgcaccacggcatgctcgccgctgaccgcgagattgtcgatcacgatgtcgttgtaggcgcgtcggcccagcgtcgtccggtctttggcgagagccagttgcccgatgacaacaccatcgatcgaaatgatcattttcggcattgccgataccccgattagcagaatttgatcgaccgcaagcggcgcgacgggtgtcgccaaggcctgcaactagacggctccaggcgtgtcgtcgacacgcgcttttgccagaacaactgaaatgttatctcggccgccattgtcgtttgcaattgcaaccaaaagtgaggctttctgccggagcccgatatcgtggctcaaaagcgtgaaaagctgcgcatcggtgatcatctcgctgagcccgtcggagcacagcatgtagagatcgtcaggccttgccgtgtgctcatgcatttcgagcaggacctggggctccacgcccatcgcgcgcgtcaccaggttgcggtggggcgagttcagggcttcttcggcggtgatggcgcccgcatcgagctgctgctgccgcagcgaatggtcgcgcgtgagctgctcgagcttgttgttgcgaagccggtagcagcgcgaatcgccgatgtggccgaccaccacgcgctgcggcctgaaggcggccagcaccagggtcgttcccatgccttgcacttcggggttggtcatgccggcctcgaagatggctgaattcgcctcgtcggtggcggcctgcaatgcgcgccggatcacccgggcgggcgcctgcgagccggcctgtgcgtaccagcgggcgaagctggcatgcaccatcgtaacggccatggcgcttgccacctcgccgcccttgtagccccccatgccgtcggccagcacggcgagaccgcgtgccgggtccaccttgaggtcgtcctcgttgtgggcccgggcgcgcccgacgtcggtcagggccgcgaactcccagctcagcgagggccgattggaaaagagggacgcgccgacgctcgccatgtcttacaagcgcgagcgcgtcgccatcagtgccccgcagcggcgcgcgcacgccgttgcagcaagcggcccgcggccaccacgaacagggcgccggcagcggcggcggcgtagtgcagccacgggttggcaaccagcgcgccctgaagcgacacgtcgccagcaatggtttcgccgccaacccagccgatcagggcggcgcccagcatgacgatgatcggaaaacgttccataagcttgatcatgagcgtactgccaaaaatcaccagcggaatgctgatggccaggccgagcaccagcagcaccatgctgccctgggccgcagcggccaccgcaatcacgttgtccaggctcatgaccaggtcggccagcaggatggtacgcacggccgccatcatgccgccgtattccttggcctcgccgccaccctcttcttcttcgcccagcagctgcaggccgatccacagcagcagcaggccgccgaggatctgcaagtagggcagcgcaagcagcttggccgcgacgatggtcagcacgatccgcagcaccacggctgcgcccgagccaaacagcacggctctttgctgctgcgcagccggcaacgagcgggcagccatggcaatcaccacggcgttgtcgcccgaaagaatgatgttgatccagacaatcttgaccaggccgatccagaaatcggtgctttgaaggagttccatgcctcttgttccactgtgttgtagtgaaaaaagcgcccgcaagatttgcgggcgcttttttctttttgcgtggtgcgcaggagaggagcgccgctgcggtttttagagctgtgccttcagcagcttggccagttccgagaagttgcgcgtgacggtgaagccgcactcttccatgatggcgagcttggcatcggccgtgtcggcgccgcccgagatcagcgcgccggcgtggcccatgcgcttgccgggaggggcggtcacaccggcgatgaagccgaccaccggtttcttcatgtgctctttgcaccagcgggctgcgtcggcttcgtcggggccgccgatttcgccgatcatgatgacggcgtcggtgtccggatcgtcgttgaaggccttcatcacgtcgatgtgcttcagaccgttgatcgggtcgccgccaatgccgactgccgacgattggccgaggccgatttcggtcagctgcgccacggcttcatacgtcagcgtgcccgagcgcgagaccacgccgatgcggcccttgcggtggatgtggccgggcatgatgccgatcttgatttcgtcgggcgtgatgaggccggggcagttggggcccagcagcaaggtcttcttgccgccggccgcttccttggccttcatcttgttgcgcacttcgagcatgtcgcgaaccggaatgccttcggtgatgcagatcgccaggtccaggtcggcctcgacggcttcccagatggcggcggctgcgcctgccggcggcacgtagatcaccgacacggtggcgccggtttgcgaggcggcgtccttcaccgaaccgaagatcgggatgttgaagatcgactcgccggccttcttggggttcacgcccgcgacgaagcagttcttgccgttcgcgtattcctggcacttttcggtgtggaactggccggtcttgccggtaatgccttgcgtgatgactttggtgtctttgttgatgtagatcgacatgacttgttccttaggcctttttcactgctgcgacgaccttctgggccgcgtccgccatggtgtcggcgctgatgatgggcaggcccgaatcggccagcagcttcttgccttcgacttcgttggtgcccttcatgcgcacgaccagcggcacttgcaggttcacggccttgcaggctgcgatcacgccggtggcgatggtgtcgcacttcatgatgccgccgaagatgttgacgaggatggcctcgacgttcttgttcttcagcatgatcttgaaggcttcggtgaccttctcgggggtggcgccgccgcccacgtccaaaaagttggccggctcgccgccgaacagcttgatggtgtccatggtggccatggccaggccggcaccgttcaccaggcagccgatgttgccgtccaggctgatgtaggccaggtcgaacttcgaggcttccacttcggccgcgtcttcttcgtcgaggtcgcgcagggccacgatttcggggtggcggaacagcgcgttgctgtcgaagttgaacttggcgtccagcgccatgacgttgcccttgctgtcacggttgagcgggttgatctcgaccagcgaggcgtccgtctccatgtagcaggcgtagagcttcttcaggatgtcgaccgtttgcgcggtcgagtcggccggcatgccgatgccgtcggcgatctgcttggcttgcgcgtcggtcaggccttccttggggtcggcgaacaccgtgatgatcttctcgggcgaggagtgggccacttcctcgatgtccatgccgccttcgctcgaagcgatgaacgcgaccttctgggtcgcgcggtcggtcacggccgaaacgtagtattccttgttgatgtcggcgccatcttcgatgtagaggcggcgcaccttctggccttcggggccggtctggtgagtcttgagctgcatgccgaggatctcgccggcgagcttcttgacgtcttcgatggatttcgcgaccttgacgccgccacccttgccgcggccacccgcgtggatctgggccttgacgacccagaccgggcctccaagtttctgggcggcctcgaccgcctcctgaaccgtataggccgggatgccgcgcggcaccggcacgccgaacttggcaaggatttccttgccttggtactcgtgaatcttcatgagggatgtctctcggaaggaggaagttgagaacgggagatctggggtctgaggcgtctttggctctgttgctcgcgggcgacggcagcctgacggctgggggcggcgaacaaccgcggactgtatcatggtgcgccgcaccaatcccgacgtgtccttgcggtcaatacgtactttcttctagccacactacgcatactccgatatggccaaggttttcatcgacggcgaagccggtaccaccggcctgcagattcgcgaacggctccagacgatgccgcagatcgaactcgtgagcatcgcgcccgagctgcgaaaagacgtgaacgccaagcgcgagctgatggccggcgtcgacctcgtggtgctgtgcctgcacgacgacgccgcccgcgaatcggtggcgctgatcgaccagttgcaaggcaagaagcccaagatcatcgacgcctccaccgcgcaccgcgtggcgcccggctgggtgttcggctttcccgaactcgccgagggccactggcaggccgtggccaaggccgaccgcgtcggcaaccccggctgctacgcgaccggcgccatcgccatggtgcggccgctggtcgacgccggcctgctgcccgccgacttcccgatctcgctgccttcggtcagcggctattcgggtggcggccgggccatgatcgaggactacgagagcggcaaggcgccgcttttcgagacctacgcgctcggcctcaagcacaagcacatccctgaaatcatgaagtacaccggcctcacccgccggccggtcttcattccttcggtgggcaacttcaagcagggcatgctcgtgcaactgccgctgcacctcgacctgctgcccggcaagccgaagtccggcgacctgcacgacgccctggctgcgcactacgccaggagcaacacgcccgagcagttcgtcaaagtgctgccgcccaccgaggacggcaagctcgacgcgctggcgctgaacgacaccaaccagctcgagatccgcgtgttcccgaacgaggaccaccgccacgccgtggtgatcgcgcgcctggacaacctcggcaaaggcgccagcggcgccgcggtgcagaacctgaagctgatgctggcgctctgagcgccagccgtttgcaattcgcctcggttcagttgacgagccagaggcccacgcccagcagaacggcgtgcgcgcccagcgcaatgtagagcggcttgcgcgatggcgtcgacatctcctgcaaggtctcgttgatgcggcgcgtgagcagcgcgcgcaaggccgggtcttgcgcagcaccctccgctgccaccggctctccgtgcgccgcacggccttgctgccattcggccagcatgtcgctcatcggcagccggttgagcacaaagccgaccaccgagcgcacggccttgccttcgcccagaaccggcgcaagctgcttgctcaaggcatcgaccgacagccagtcggcggcgcgctgcagcgtgccgtgggtacggggcatggattcgatgcggcccgcgatcgcaccggccaggcgctcggacacggcctcgccgcgcgcggccaccaggtgctgcatcgccttggctcggccttgctgcacacccagcatcacgtagacgacaacgaaaagaagcagcagcaccgcgaccagcagcggcggcgacgtgaccagcgcaagcaccgcgccggcgccgcccgcgcgtgccgccgtgttgccggggccgtgcagctggcccaggtaatagaagaaagcgccgccgccgagaatcagcgcgagcaggccgcccttgatgaccgagccgacgaaagcggccccggccttggcgcccgtgcgcacgagcgacggctgaccagcaggtcctgaagacatgggatttcctcctccgaagttttgtgaaggcggtcctcgcacgggaccggccggcgccgatcatgccatcgggttgggcccacagcacggcgccggctggcgcgcggcaatgtggccggcgattcagccggcttcgagcaggtgccgcagcgactgcaagtcgcgcgcgatccacccggcatcgcgctcgaaggccgcatcgtccatgtgcggctggcgcagcagcgtgaactgcagctcgcaaatgcccggcgcgacgccgatcacgcggaacggcagatagatttcgggcacgccttcgggcgccacccaatggtcgagcacgccgaaatcgttggcgggtgcgaagcgcaggcgggcttcgccgtcgggcgtcgtggccatccagtgatcgccatgagggaccaatgtgctcttggccaggccgctggcccagtcgggcagccgcgccggctcggaggccagcgcataggcgcggcgccagtcgcaggccacgcgctgcgtgacgacgcgggactgcacggcatcttcattcgcttgattcgtcgttgtcggcatcgaaatcgctcctgagtaccttggccaccacggcgcccgaaaaaccgcgcgccagcagaaaccgtgtttgcctggcgcgctccttcgcatcagcggggggcgcgtcgaaacggcggcgccagagggccgtggcgcgctccacttcggtatcttgcaggctggccacggccgctgcaatggcgtccggcgcaatgcccttggcctgcagctcctggcgcacccgcaaggcgcccgaccgggcagcgcgctggttgagcaccgaggccaccacgcgcggctcgctgatgaagtccttggcggccagctcgtcgagcgcgcgggccagcgtgccgggttcttcttcgtgccgggccagcttgcgctccagctcggcgcgcgaatgttcgcgctggctcaggagccgtaatgcgcggcctttgagggagggggcgccgaaagccatgccttatggtcgcttgcgcggccccgcaggaggccgcgtgtacttgtgcttgcttactcgcccttgtcggccttctccgccttggccgccttcgcgggcttctcggctttttcgggcgcgggggcgccggcatcggccgccagcagcggaatgcccagcgactcgcgcaccttgttctcgatttcgcgcgacagctcggggttctcgcgcaggaactcgcgggcgttgtcgcggccctggccgatcttttcgccgttgtaggcgtaccaggcccccgacttgtcgaggatcttggcggtcacgcccatgtcgatgatttcgccttcgcggctgatgccttcgccaaacaggatgtcgaactcggccgtcttgaacggagggctgaccttgttcttcaccaccttgaccttggtttcattgccgatggcctcgtcgcccttcttgatggtgccgatgcggcggatgtccaggcgcaccgaggcgtagaacttcagcgcattgccgccggtggtggtttcgggcgagccgaacatcacgccgatcttcatgcggatctggttgatgaagatgaccatgcagttggtcttcttgatggtggcggtgagcttgcgcagcgcctggctcatcaggcgggcctgcaggccgggcagcgagtcgcccatttcgccttcgatttcggccttgggcgtgagcgcagcgaccgagtcgatgacgatcaggtcgacggcgcccgagcgcaccagcgaatcgacgatttcgagcgcctgctcgccggtgtcgggctggctgatcagcaggtcggacaggttcacgccgagcttctgggcgtactgcacgtcgagcgcatgctcggcgtcgacgaaggcgcaggtgcccgcctgcttttgcatggcggcgatgacctgcagcgtgagcgtggtcttgcccgaggattccgggccgtagatttcgatgacgcggccgcgcggcaggccgcccacgcccagcgcgatgtccaggcccagcgagccggtggagaccacctggatgtcctcgagcgcctcgccttcgccgagccgcatgatcgtgcccttgccgaactgcttttcgatctgggccagtgcggcctgcaaggccttggccttttcgctgttggcgaccgagatgcttgcgcccttgacaactgcgtccatgtggaaatctccttgaaaatcaacggtttgtgtgtgactgccatccatctgcttttaatcacaggctggatgcttgaacagtagtgtaggggttgattggtttgagtaaacccattttttggtcagtttgctttactatttagtcgatggccgaaaccgcttttccaaccgatcccgacgcctggcggcaaacccacctgggccgcctgctgggccatgcgatgcgccgcttcgacgagcgcgtgctcgaactcatggcgcacgacgtcgacgtgccgctggcgctgtcgaaccttgccgcccgggcccaggtgagcgccgcgcacatccacatcacgcggcacctggcgcgcgagggttcgcgcctgaccgagatggccgagcgcgccggcatgaccaagcaggccatgggcgcgctggtggaccagtgcgaggcgtggggcctcgtcacgcgtgggcccgacccgctcgatgcgcgggcgcggcaggtgcttttcactgccgacgggctggcgtggctcgacgccttccgcggcgcggtgacgcaggccgagcgcgaattccgcgccagcgtcggcaatgacgttgccaccgtggtcaccatcggcctggaagcgtacacagaggagggctagactcggccgggagagacagagacatatgtgaacgcggcgccagcgcggtgcccgaacggccggaggtggctcatgcggattctgattgccgaagacgaccaggtgctggccgatgccctgctgcgcagcctgcggacctcgggcgcggcggtcgaccatgtggcgaacggctcgcaggccgatgccgcgctcatgacgcacagcgagttcgaccttttgatcctcgatctcggactgcccaacctccatggcatcgagattctgaagcgcctgcgcgcgcgcggctcgcaactgcccgtgctggtgctcaccgcggccgacagcgtggaagaacgcgtcaagggcctggaccacggcgccgacgactacatggccaaacccttcagcctgcaggagctcgaagcgcgcgtgcgggcgctcacgcggcgcggcatgggcgccaccagcaacaccatccggcacggcccgctggtgtacgaccaggccggccgggtggccaccatcgacggcaagatggtcgagctctcggcgcgagaactcggcctgctcgaagtgctgctgcagcgcgccggccgcctggtcagcaaggaccagctggtggagcgcctgtgcgagtggggcgaggaagtgagcctgaacgcgatcgaggtgtacatccaccgcctgcgcaagaagatcgagaaagggccagtgcgcatcgccaccgttcgcggcctcggctactgcctggaaaaaatccagcaatgacgcccgggcatgcccggcggctcgggaggccgtaagccttgaaactgtttcagcgcgcccagcgctccctgttcggcgagatcctcgactggatgctcacgccgctgctgctgctggtgccggtgagcatcggcgtcacgtggctggtggcacagggcattgccaatgcgcccttcgaccgcgcgctcgaatacaacgtgcagacgctggcgcggctcgtcacggtgcagcagggccagacgcagttcgtgctgccgcagccggcgcgcgagatcttgcgcgccgacggcgccgaccgcgtctactaccagttgctcgacagccacggcaagctgctcagcggcgagcccgacgtgccccaccccaacaccgacgagccgccggtcaccggcgtggtcacgcttcgcaacggcgaaatgcgaggcaagcaggttcgcgtggcctcgctctggctggccgacggcaacgacgattcggccccggccctgctgcaggtggccgagacgcgcgagaagcagtcggtgctggccaccgaaatcatcaagggcgtgctgctgccgcagttcgccatcctgccgctggccgtgctgctgatctggctggcgctggtgcgcggcatcaagccgctgtcggtcgtggaggcgcgcatccgcgagcggcgcccgggcgacctgagcccgctcgacgagtcgtcggtgccgctcgaggtggtgccgctggtgtcttcggtcaacgagctgctcgacaagctcaacgattcgatccacacgcaaaagcgcttcctggccgacgcagcgcaccagctcaagacgccgctcgcgggcctgcgcatgcaggccgacctggcccagcgcgaaggcgccaacgccgacgaactcaagaagtcgctcaagcagatcggccgcgcgagcgtgcgcgccacccacacggtgaaccagctgctttcgctggcgcgcgccgaaagcaccggcgccggcaccggccgccagccctgcgacctggcacggctcaccatcgaggtggtgcgcgaagcggtgccgcgcgccatcgaaaagcgcatcgacctgggctacgacggcgccgaggccggcgcgcccggcgtggtgatcgaaggcaacccgaccctgctgaaggaactggcgcgcaacctgctcgacaacgcgatcaactacacgccatcgaccgccgagcggcccggcgtgatcaccgcgcgcgtgctggccgaccccttcggccacgtggtgctgctgcaggtggaagacaacggcccgggcattgcggaatccgatcgcgagctggtgttcgagccgttctaccgcgtgctgggtaacgaagccgacggctcggggctgggcctgccgatcgtgcgcgagatcgccaaccagcaccatgcgcaggtcaagctcgaagacgcgcacccgggccggcagccgccaggcgcccgcttcacggtgcgcttcgcggacgaagaaggagcgccctgaggcgcacaacggacgcgcccggtcagggagcggcgctgctgctcttgccgtccttgcgtatctggagccagtcgggatgaacctggcgcgcgaggcgctgcggttcgcgctcgttgaggctcgcgggcgccaagccaaagccggccagatcgccgcgcgaccacagccagtagccggcattggcaaggagcagggcaatcagcacgaggcgcagtttcatcgtgaatctcaaaaggccatgccgcgcggacgcacgctgacctcgtcgctcgagatcatctgcaggccgtcggccgtgcgcacctgcagttcgccgccccaggcgacgccctcgcacaagccgacgctgccgtcgctgagctggacctcgcgcccccgcagcgcgtcgcgcgcggcaaagcgctcggcaaatggcacgaaaccctcggcctcgaaaacctgcacgccgcgcaccagcggtgcggccagctcggcaagcacctcgggcgcggtgacgccggggcgccattggcgcagccacgcgggcggggtgcgcatgccctcggcttcgcgcgggccgatgttgatgccgatgccgatcaccaggtagcgcggcacggccggcccctcggcacggcccacgtgcggcatggcggtttcgatcaggatgcccgcgagcttgcggtcgtccacccacaggtcgttgggccacttgagcgcgactttcgcatcgcccgaggggtcgaggctttcggccacactgacgcccacggccagcgagaggcccgaccagtcgcgcggcgcaagcggcaggcccagcgagaaggtgagggaagcggcgccgtcttcgctttgctgcgcactctgccagggccggccgagccggccgcgcccggcggtctggcgctcggccaccagcagcaccggcggggtgtggccggcgcgcgcgcggcgcatcagctcggtgttggtcgaatcgatttcggccacggcctcgatcgcaaagccgggcagcagcggcgccaccgccgcggcaatccggtcttcgagccaggcggtctgggtgcccatgctcagcccttgccggcctcgtccttcctggacttctttttttccgacttcttttcggccttcttctcggcttttttgtccgcctttttggcttcctttttctcggcctttttcttctcggccttctttttggcctttttcttctttttcttttcttcgtcttcgtccttgggcgtcagcaaggtgccgcggcaactctccgagccgcaccagcagggaaactcggccagcagctttggcgtgtagggctcgtcgatgatcaggccgtagtcgtagttgagctcttctcctgcagcgatgtttcgcagcgccttgatataaacgcgcccattgacctcgtcggcctcgcagttcggctcgcaggaatgattgatccagcgggcggcgttgccgttgacgttgccgtcgatcacacgcccgtcgtcgatgtggaagtaaaaggtgtggttcggctgggccgggtcgtgcgggtggcggcgcagcgcctctttccagttgatgacctcgcccttgtattcgatcagcgtctcgccttccgccaggtcctggacggcgaacacgccgttgccatgaacggtggagcgccgcgtctggatgcggcggccgctggccggcccagaggcaagccgtgcttccccctcgggagggcggagggcttccgtgtcgcggccgccggaaagtggggatttggaaggcatcgccgaagtctgttaggttgaatatgcacacatgcgcgtgtgcgcgtgcgcacgcgggaagccgcagattgtatgtggcccccacgctcccgcactgcgtgtcgtcgctgcccccgagggggccgcaggccgccttgaggcggctcggcgccggcctgggaactcttttaggaatgttgatgaagactttggtaattgcagaaaagccgtcggtggcacaggacatcgtccgtgcgctcacgccggtggccggcaagttcgaaaaacacgacgagcatttcgagaacgagagctatgtcgtgaccagcgctgtcggccacctggtcgagatccaggcgcccgaggagttcgacgtcaagcggggcaagtggagcttcgcgaacctgccggtgattcctccgcacttcgacctgaagccggtcgacaagacaaagacgcgcctgaacgccgtggtcaagcaggccaagcgcaaggacgtgacgcagctcatcaacgcctgcgacgcgggccgcgagggggagctgatcttccgcctgatcgagcagtacgcgggcggcaagaccggcctgaacaagccggtgaagcgcctgtggctgcagtcgatgacgccgcaggccattcgcgacggcttcgacgcgctgcgcaccgaaaagcagatgcagggcctggccgacgccgcgcgctcgcgctccgaagccgactggctggtgggcatcaacggcacgcgcgccatgacggccttcaattcgcgcgacggcggtttcttcctgacgaccgtgggccgggtgcagacgcccacgctgtcggtggtggtcgagcgcgaggaaaaaatccgcaagttcgtgagccgcgactactgggaaatccacggcgtgttccaggccgaggccggccagtaccccggcaagtggttcgatgccaatttcaagaagccgccgccgggccccgacggcacggccgacgcggagattcgcgccgaccgcgtgtggagcgagcgcgaagcgcgcgagatcgccgatgcggcgcgcggcaagcccgccaccgtcaccgaggaaagcaagcccaccacccaggcctccccgatgctgttcgacctgacctcgctgcagcgcgaggccaacggccgcttcggcttctcggccaagaccacgctggcgctggcgcaaagcctgtacgaacgccacaaggcgctgacctacccgcgaaccgattcgcgcgcgctgcccgaggactacctgccggtggtgaaagacacgatgaagatgctcgccgacagcggcatgaagcatctcgcgccttttgcgcagcaggcggtcgacggcagctacgtgaagccgaacaagcgcatcttcgacaacgccaaggtgtcggaccacttcgccatcattcccacgctgcaggcgccgagcggtctctccgaggccgagcagaagctctacgacttcgtggtgcgccgcttcatgtcggtgttctttccgagtgccgaattccaggtcaccacccgcatcagcacggtggaagccggcggcaggaagtaccccttccgcagcgacggcaaggtgctggtcaagccgggctggctggccatctggggcaaggaagcgatcaacgacgacgacgagaaggacggcaagaacctcgtcgtggtgaagccgggcgaaacggtgaagaccgaatcggccgacctgaaggcgctgaagacccggccgccggcacgctattcggaagccacgctgctcggcgccatggaaggcgccggcaagaccatcgacgacgacgagctgcgcgaagccatgcaggagaagggccttggcacgccagccacgcgcgccgccaccatcgaaggcctgatcaccgagaaatacatgctgcgcgaaggccgcgagctgattcccacggccaaggccttccagctcatgacgctcttgcgcggcctgggcgtggaagaactctccaaggccgagctcacgggcgagtgggaatacaagctcgcgcagatggagaagggcgcgctgagccgcgacgccttcatgcgcgagattgccgagatgacggagcacatcgtcaagaaggcgaaggaatacgaccgcgacaccgtgccgggcgactacacgacgctgtcgaccccgtgccccaactgcggcggcgtggtgaaggaaaactaccgccgctatgcctgcaccggcaagtccggcaccggcgaagatgcctgcggcttctcgttcggcaagtcgccggcggggcgcaccttcgaagtggccgaggctgaggcgctgctggccaacaagcacatcggcccgctcgagggcttccgctccaaggccggctggcccttcacctccgagatcatcctgaagttcgacgaggaagcgaagaattggaagctggagttcgacttcggcgacgacaagaacggcgacaccggcgagatcgtcgacttcagcgagcaggacacggtgggcccgtgcccggtctgcggcgcgccggtgttcgagcacggcagcaactacgtctgcgagaagtcggtgcccaccaatgcgcagccgacgccgagctgcaccttcaagaccggcaagatcatcctgcagcagccggtggagcgcgcgcagatggaaaagctgctcgccaccggcaagaccgacctgctcgacaagttcgtgagcatgcgcacgcgccgcgccttcaaggccttcctcacctggaacgccgaagagggcaaggtgaccttcgagttcgcgccgcgcgaaggcggcagcaagttcccgccgcgcaagaccttcggcaaggcgccggctgccggcaagaccgcggcggccaagaaggtggctgcgaagaagacgcccgctgccaagaaggcgccggccgcgaagaaggccgccgcaccgcgcaagcccggcgccggcctgaagcccagcgactcgctggccgcagtgatcggcgccgaaccggtggcgcgcaccgaggtcatcaagaagctctgggactacatcaaggccaacggcctgcaggacgcggccaacaagcgcgcgatcaatgccgacgccaagctcaagccggtgttcggcaaggaccaggtgacgatgttcgaactcgcaggcatcgtgggcaagcacctctcggcgccgtaacttcgtgctacgggccggaaaaagcaccggcctatagtgatctcagtctcaccattgcctggagttttccgtgaagccattcattgcagctgttcttgccctcgcgatgggcgccctggcagcgggctgcgccggcacggggtcggcgggcaacactgaccgcgccacctcgtcgtccggtaacggcatcacggtatttggcaccatcgatgccggcgtcagcggcagcacgaaccgttccgaccggcgctagccagtcggtgtgtcagcgccgcagcagcgcctggcgcagcacgcgcgccgcgcgatcgcggatgcggcctgatccggtatcgagcgaggtctgaggcgccaccctcgcggtggcgcaggcccagagaaagtcgtgcaggatgggcgtgtcgtccacggtctcggtgctgccgtatttgtggaactcggggtgccactgcgtggcggagatgtagctgcggcccttgtcggtgcggcggcgaatggcctcgggcacgcggtcgggcaggctccaggcctcgacctcgaaaccgggtgcgagatctttcacgccctgatggtgaatgctgttgacctttgcagtcttcacctccggatagagcttggccaggcgcgtgccttcgacgatctcgatctggtgaaaattctggtcgtaggtcaccgggtcgcggtgccggatggtttcgggatggtcgtgctgcgcctcgatgtcctggtacagcgtgccgccgaaggcaacgttgatgagctgcagcccgcggcagacgccgaagatgggcttgccggcctgttcgaaggcttcgaccagcgccaggtcgtacaggtcgcgaatgcggtcgccgacccatgcatccttgagcggctcctcgccgtagctgccgggccagacgtcggcgccgccatgcatcacgacgccatcgagccattcggcgtagtgagagagcttggtgtcgccgcgcgcggtttcgcccgtggggcagggcaccatcaccaccatggcaccggccgacatgagccagtgcgcgatggactgctcgacgtactgcagcgtcttgttggtgaacagcgagcgcgccggatccgcatgggaaaagcaggcagacaggccgatcttcagccgggcggaaacgggttgcggcatctcgggactggcaggacgtgctgtgcgaaaaggaaagtccattttggcgctttggcctctcgcacggggtcggacgacacgccaagtatgctttcaacgccgctacgaccaagaaggaagacaagccatgaagacgatcaagggcccggccatttttctggcccagttcgcgggagaccaagccccgttcaactcgctcgacgccattgccggctgggccgccggactgggctacaagggcgtgcagatcccgagctgggatgcgcgcctgttcgacctcaaaaaggccgccgaaagcaagacctactgcgacgagatcaagggcacgctggccgcgcacggcctcgagatcaccgagctgtcgacccatctgcaggggcagctggtcgcggtgcatccggcttacgacgccggcttcgacggctttgcggcacccgaggtgcgcggcgatccggtgcggcgccagcaatgggccgtggagcagttgcacttcgcggccaaggcctcggccaacctcgggctcacggcccatgcgaccttctcgggcgcattggcctggccgtacctttactcatggccaccgcgcccgccgggactcatcgaggaagccttcgacgaactggcgcgccgctggcgcccgatcctcgatgccttcgatgccgcgggcgtggacgtgggctacgaaatccaccctggcgaagacctgcacgacggcgtgagctacgagatgttcctggagcgcgtgggcaaccatccgcgtgcctgcctgctgtacgacccgagccacttcatgctgcagcagctcgactacctggcgtacatcgaccactaccacgagcgcatcaagatctttcacgtgaaggacgccgagttcaacccgaccggcaagcagggcgtgtacggcggcttccagagctggatcaaccgggcagggcgcttccgttcgctgggcgacgggcaagtcgatttcagcgccatcttctcgaagatggcgcagtacgacttccccggctgggcggtgctcgaatgggaatgctgcatcaagcacccggaagacggcgcacgcgagggcgcggccttcattgccgaccacatcatccgcgtggccgagcgggctttcgacgacttcgcggcgggcggcgtggacgtagccgcgaacaagcggatgctcggcctcggctgaggcgcgctgttgagctatatctttagtagcaccagacacttgtttggcgggggtctggtgcctaattcacaggtgcgttgtttttaagacaagcaactgtcatgccccgcgggctataatgtcgggttcgtttcgataccacgacgaagcacttttcgtcactccgccggctgacctgtaccgtcccttggatttttcaggcctcttttttcaagccggcttcacagtgtgttggagcgccagaccgggcgcccatgattgccaccactgccttcgttcttgttgaagcgaatagcgcgtccgccgcgccgttctggccggcccacgcccgttttcaatcattttttcggcattttgcgcacacttttcgcgcagggtgccaaggcttcatggacatcattcaacacagtatcgcggtgggcaagtaccttgtttccccgctcattcgccaccaggacgacggcaactacgccgcttccgtctcgatccgctccggacggggcagcggcatgcacgaccgcgtgatgcgtttcacgccgcgctttgccagccacgccgccgcggtgcgctacgccatcgaccagggcctttgctgggtgcgcgaacgcagcagccctcttggcgttgccccgctcgcacttccgtgcgcaggctgaaacaattacgcccatcttcatctccaacacacatcgaacgagaattcagaggtaatcacacatgcccaaggaagaactgatcgaaatgaacggcgcagtgaccgaagtcctgcccgactcgcgctaccgcgtgacgctcgacaacggccatcagctgatcgcctacagcggcggcaagatgcgcaagcaccacatccgcatcctggcgggtgacaaggtgtcgctcgaactctcgccttacgacctgaccaagggtcgtatcaccttccgccatctggagcgccgcggcccgccgccgacgaactccggaaacaacaacgcacctcgccgctgatccgcgacggacgaagggccttgcggcgccccgcgaagggtgccggcaaggcctttgtttttccgggtccggctgccgccgaacgatgaccacgaccaattctccagccggcggctccccagcccaggcccccgccgaccacggctttgccacgctggcgctctcgccccagatgctggccaacctcacgcagctcggctacacgcagatgacggcgatccaggcggccgcgctgccgccggcactgctcggcaaggacctgatcgcacaggcaaaaaccggcagcggcaagaccgccgcctttgcgctggcgctgctctccaacctcaacccgcgccgttttgccatccaggcgatggtgctgtgccccacgcgcgagctggccgaccaggtcacgaccgaaatccgccgcctggcgcgcgccgaggaaaacatcaaggtggtcacgctctgtggcggcgtcgcgctgcgcgggcagattgccagcctggagcacggcgcgcacatcgtggtgggcacgccgggccggatcatggaccacctggaacgcgagaacctgaacctcgaggcgctcaacaccctggtgctcgacgaagccgaccgcatgctcgacatgggcttcttcgacgacatcgtgaaggtggcgcgccagtgcccgaaggaacgccagacgctgctgttctcggccacctacccggaaggcattgccaagctcgcgcagcagttcatgaagagccccgagcagatcacggtgcaggcccagcatgaaggcagcaagatccgccagcgctggtaccaggtgaaggacagcgagcggctgcacaccgtgagcctgctgctcgaccatttccgtcctgtgagcacactggccttctgcaacaccaagcagcagtgccgcgacctcgtcgaggtgctgcaggcgcagggcttcagcgcgatggcgctgttcggcgaactggagcagcgcgaacgcgaccaggtgctggtgcagttcgccaaccgcagctgctcggtgctcgtggccaccgacgtggcggcgcgcgggctcgacatctcgcacctcgaagccgtgatcaacgtcgacgtgacgcccgactccgagatccacatccaccgcgtgggccgcacaggccgcgtgggtcagcagggcggctcggaaggcctggcgctgaacctggccagcatgaacgagatgggcttcgtcgggaagatcgaacagctgcagggccgcgagtccgaatggcacgacctggccgagctcacgcccgccaagggcgcgccgctcacaccgccgatggccacgctgcagatcgtcggcgggcgcaaggaaaaaatccgcgccggcgacgtgctgggcgcgctgaccggcgactgcggctatgccaaggagcaggtcggcaagatcaacgtcaacgagtactcgacctatgttgcggtggaccgcagcattgccgaagaagccgcacgcaagctcgacaacggccgcgtgaaaggcaagagcgtcagggtccgcctgctgacaccgcagtcgacctgacacccctcccacccctttttcgcctcttggcatgtgaaatctgccgatgtggcctaattgagggtcgaacatcttttttatccgagctttccatgcccaagaaaatccgtaccgaagccgaccgtcttgccagcccgaagccgatccccatgcccggctacaccgcgcctcgcaccggtggtggccaaaaggtcagcctggaacgcggcaccgccacgcgcagcaagaagaacccgggcaagcgccccaccaagggcggctgatccagcccccacggctctttcttcggagccacgacgaacgcgcctccgggcgcgttttgtcattgggcccgctacaaacaaggccgccatgtccgacgacaaccagatcttcatcccgccctcgttcttcgcggtttatagcgatgcgcgccagcgcctcctggagccgatcggcgtggtgcgcgagcgctacgagatctgcgaagacctggccaaccatctcgtgggccatgcgcagatccagcaccacaccgaggtgccggtcgagagcgagatcctgcgccgcatccacgccggcctggccacgcccgaagccggcgtatcggcggccgaggccggctggatcgtgcagcggctggccgagctgctgggctggcccggacccgagccggtaccggccgaggattgacgcgaaggcgcgccgcccggccgccggtgctggcgaggccccccgggcctatttgtcgatgatttttcgagcgaacagttcgaggtagtccatcagacgattggccccggcagtggctgccgcctcgttgccggtcgcgatgccttgcgccagttcgaggtgggcattcgcaccctcgacgatctcgccttcatgctggtaggcgtaccagaagcgccggcactgcacgatgagcggggtcaccgccttcaccgccgaatcgttgtggctcgcctggtggttgacgaggtcgagcgcgcggtcggcctgcatgtagtcgttcaggtcgccgcggtgggcggccttcaccatcagctcggcgcagcgcacgatctccttgcgctgcagcgcggtggcgcggtggcgcggcgcgcggagcaggccgcaatcagcagttcgagcacgcgccgggtctggatcacgtccaggtggtcggccaggtcgatggtcgacaccaggaggccgcggcgcggctgctgcacgatgaggccgatcgacaccatgcgcatcagcgcctcgcgcaccggcgtgcggccaaggccggtgcgctcggccaggtcggcttcgacgatctggctgccgggctccagctgcagcgtggagagcagcgtctcgatcgcgtcataggcgaggtcggcggcccgtcgtttgggctgggggcgaggcacggtcttcggaggggccattgttttcttctggtgctgcttcggcttcattgtcggtccacatcgccagggcccgcgaggccggccagggttgcgatgcgcgccggcgacagcggcggacgcggcgcgggcggcgtccagccgaaaaggaactgcgcggcatcgccgcagacgcggccctggcaggcgcccatgccgcagcggcggtggagcttggcgtcggtccagccgctgcaacctgcgagcgccgagaacggcacgtcttcgcagcggcatacgagggtgtcgggctgcggcatctggcggatctcgggggccagcgcgaagctgcggtgcaactgtgcggcgaaggcattccagcgggcacgcgcgcgttcgtgctgctttgcggcgccttcgttgccgacggccgcgtagccggcgatggcgccctgcgcgagcgcgcgttcgctgccgccgaaaccggtgcattcgccggctgcgtagacatccggcaggctggtggcctgccgcgcatcgacagccagtgcctgcgcgccgatgcctccggacgtgagggcgcagccgagcatctggcccagttgcgtgttggggacgaggccgaagccgcaggccacgcgatcgcattcgatttccacgtcgcggccgccttggcgcaaccgaaccgattcgacctgcatgccgccttgcaccgagacgatgcgcgacgaagtgcggtactgcgcgttggccagcgtgatcgcctgcacagccttgcccggccatctcggcaagctggccgcaaaccctgcgaccgcctcgaacgaggcctgttcggcgatgcgcacgaccttcgcacccgccgcgcgcgccgttgccgccgcggcgagcagcaaagggccgctgcccgcaatcacgatgcgttcgccctcgaccggcaaccccgccttgacgagcgcctgcaggccgcccgcgcccgtgacgccgggcagcgtccaaccggggaagggcagcagcagctcgcgcgcgccggtgcaaaggatcagcttgttccaccgcatgcgccagccgcgctccgcgtcttcgagcagcagttcgtttcgcgatggcgccgcgacgacgcgcgtgccgctgcacacgcggatgttggcgtggcgttcgagcgcatcgcgccacttgcgcgcggccggcggcagcgtggcgccgggaccgtcgcgccagatctgcccgccgggtgcggggttgtcgtcgatcacgacgatcgatgcaccgccgggcgcggccgccactgccgccgccatgccggcggggcccgcgccgacgatcagcagatcgcaatgcgccagtgccatgtcggtcactcggaggtctccacgcacatgccctcggcgcagaccgtctggcaggcgagcctgcgccggccgtcgatgcgcactcggcattcctggcacacgcccatgccgcagaacggcgcacgcggctgccccgtgaccgacgtgcgcgccacgccgatgccaccggcgacgcgcaaggcagcggcgactgagctacccgccgtcacgcggacgagccggccatcgacgtgcagcaaggtctcgccgctcatgcgcacctctccagcagcccgcgcggcgcatagggcgcagcgtcgaatccgggtgcaccgccggtcatcagcgccgcgagcagatgcgcgctgcccggcgcggtggtcacgcccaggccttcgtggccgacggcgagccagagcctgtcgcgccacgggtgcttgcccagcagcggcagtccatcgggcgttgcggcgcgcatgccggtccacgagcggaccgcgttgaggtccgcgaggcccggcaagtagtcgagcgtgcgctgcagcatgcgcgcgagcatcggtgcttcgacggcgggatcggtggtgtcgaactggcgcgaagagccgatcagcagttgcccggtcggccgcggctgcacgttgaacgcgaccgagtcgccgtcgctgtggtgcgcgctggtcacgtagccgagctcgaccagctgatggtgcaccgtgcccggatagcggtcggtgatcagcaggtggcccttcttggggcggatcggaagctcggggcagagcgtcgtcgcctcgatgccgctggccagcacgatctgcggcgcgctgcgacggctcccgtccgcgagccgcagcgtgccgtcgtcttcgatcgcatcgaccttcgcatgctcgatgcggatcgaatctgcgccctgcgcgagcagccagcgcgccgcattcggtgcatagaggatgccgtcgccgggcacttcgagcgcgcccgcaaggcccttgcgcaaggcgggctcggcgcgggccagctccagcgcaccgagcaggcggctttcgataccgtgctcacgcagccgctgctgcttgcactcggcctcggccatttcttcttcgttggccgcgatccagagcgtgccgcaggcgctgtacgcgcagtcctcgctcatgcgcggcgccagggcgcgccattgcgccgtcgaatggctgctcaatgtaagctcggccgggttgtcgtccatcaccacgaggtgccccatgcctgcgcccgtggcgccgccgatacgcgcatcgagcaccagcacccggcggccggcctgcgccagcgcatgcgcgcaggcggcaccgacgatgccggcacctatgacgatgacttcggcgtgcacggcctacactgcggaaccggctttgccgggccgctggtgttgcccccggcagggggttggcagagcgacacgaagtgcgcgaagactgggggcgagcctcatatccggattccccacccgaaaggatcgttgtcgtcgatcaagagcgtggcctcggcgctgatgtgcgcacggccgcgcagcgttggaatgaccttgccgtcttccagcgcgtagctggcctcgaagcggctcccgatcacgctcgcctgtgtccacacctcgcccggcgccagcttgccgtcggccgcaaggcaggcgatcttggcgctggtgccggtgccgcagggcgagcggtcgtaggcattgccggggcagagcacgaagttgcggctgtccgcgccttcgctgtcgtgggcgaagagttcgatgtggtcgatctccgcgccatcggcgcccgtgatgccttgcgccgccagcgccttgcgcagcgcggtggtgtagccggtgagcgcggcgaggttgtcactcgccacccgctggccgtgttcgctcaccaggaagaaccagttgccgccccaggccacatcgccgtgcacggtgccgtggcccggcaggtcgaccgcgacccggtgcagatgccggtacgccggcacgttgcgcacactcaccgagccatcggcatgcagcctggtcgtgaccatgcccaccggcgtctcgatcctgtgctcgcccacgccgatgcgcccgatgtgcgcgaggcttgcgaccagcccgatggtgccgtggccgcacatgccgatgtagccggcgttgttgaagaagatcacgccggcggcggcatctttcgacaccggctcgcacagcagcgcgccgacgatcacgtcgctgccgcgcggctcgagcaccgtggccgcgcgccatttgtcatgccgctcggccaggagcgcgcggcgctcggccatgctgccgccgcccagatcggggaaaccgccgatgaccaggcgcgtgggctcgccgcccgtgtgcgaatcgatgatctggatgcgttgcatgtgtttctcgaactcagtagctggcgaggggaaagggcgctgcgttcttgaaggtgaacaccgtgatcggcgcctgtttcatgttgcccttgtcgtcgtagctgtaggttgcggccacgcccttgtaagtggtcttgtagagctcggcgcctactttgtcgggatcgatggagttggccttctgcatcgattcgccgatgaacagcacctggtcgtagtacgaagcggcatacgcgtccgcgtcggcgttgaagcgcttcttgaacttggccttgaacgccgggccgctctgcgccttttcgagaatggagccgccttgcgcgcagaacaccaggtcgttgaccgcatcgccgcccagcttgccggtggccgggctgcacagcgtgtcgccgcccagcagcttgccgggcacggccagctgcttcatctggcgcgccatgggtgcggcctgcggcgcgtagccgccgaaaaagatcgcttcgggcgccttggccttcatgttggtcaggatggcggtgaagtccacggccttgtcggtggtgaactcctggcccacgactgagaggccctgcttcttcgcttccttggtgaactcttccgcaaggccctggccgaaggcggtgcggtcgtcgatcacgcccaccttcgtcaccttgagcaccttggccgcgtacaccgccatgctggaaccgatctggttgtcgctcgcgatgatgcggtacaggttcttgtagccgccctgcgtcacctttgggttggtgcccacggtggagaccatggtgccgccatcggcgtagatgcgcgaagccggaatggccacgcccgagcagtacgggcccatgacgtacttgacgccgtcgtccacgaatttctgcgccacgctcacgccggacttggcgtcgcactggtcgtcttcggacaccagctcgaacttcagcgtcttgccgccgaccgcgagcttcttcgcattgagttcctcgatggcaagacgcacgccgttctcgttgtccttgcccgcgaaggcattggggcccgagagcggcccgctgtggccgatcttgacgacctgctcctgctgcgcattggcgtggcccgccacggcgatggccacgaggccgagaaacggaatcatgtgtgcgttggacttcatgcttgttcctttgtagaggacgagagggtttatgccatgaccgactggtactgcaccggccgcgtggccagcgccttcttcacgatcgcctccaccgccgcgcgctcctcgcccaccagcggcagccgcgggcggcgcatgtgctcgctgcccacgcccaccagcacgtcgatcagcttcaggttctgcaccagcttgttcgatacatccaggtgcagcatcggcgtcatccactggtacagcgccagcgcctcggcgaactggcccgccttcatcaggtcgtacagcgccacggtttcccgcgggaacgcgcagcccaccccggccaacaggccatccgcgcccagcgccagcccttcgtacgccaggtcgtccacccccaggaacagctggtagcgggtccccaccgtgttgcgcaggtccgtgatgcggcggatgtcgcccgtgctctccttgatcgccgcgatccattcgcagtccgccagctccagcatgtgctcgggcttcaggtccacccggtaggccaccgggttgttgtagaccatgaccggcttctgggccgcatgggcgatggtgcgcacattcagcatagcctcgcgcgcatcggccacgtagatcaccgagggcatcaccatgaagcccgccacccccagcttgttggccccgtccacatagcgcagcgcttcgcgggtgctggtttccgacacattcgccagcaccgggatgcggccgtcggccgcttccagcgcgatctgggccacctgcagcttttcttccaagctcagcgtgctggcctcgcccagcgagccgcaggtcaccaggccgtggatgccgttgcggatctggaagtcgatgtggcgcgcggtgccttcggcatcgatgctttcgtcggcgtggaacttggtggtgatggcgggaaagatgccttgccagcgggggttggtcacgtgatgggctcctgggttgcgcgacaagaaacggtcgcggtttaaatatattaacaatatatcttcaggatatgcgtggggcaagcgctcttttggaccggggtcttctgtgatatccgggaaaagggcggggggcgtccgctgatggggcgccgctacttgtgcgcgtccactgggcgctgcgctttattcacgctcatgcgttcggggcgcgctcccgccgacgggagcgttgtttggagcggtggttgatcgagcggaacaagagcagcgctttgtgtgcgcagggcgccgggtgctccccgcagcgaaataaaggaggaggcgaagccgggggacattcgcggaggggagtacccggtggcctgtgcacgcgccctgaacaagcgtgccccgaacaagagcgccgaacacgaatccaggtcagtcgatcttcgccccagaagccttcaccaccgcccccatcgcatcccagtccgcgcgcagcaccttctggaactcttccgcgctctgagtgcgcggctccacgcccaggcgcttgaagcgctcctggatcgccggatcggccagcaccttgttggtggccgcgttcaggcgctcgacctcggctttgggcgtgccggcgggtgcgagcaggccgatccatgaatcgaaggcgtagcccggcaggccgctttcggccacggtcggcaaagtcggcaggaaggggctgcgcgcctggccggtggaggcgagcagcttcaagcgcggatcggcctggaaacccatcacgccgatgctcgacgagatgaccgcctgcacccggcccgcgagcacctcgttgaccgcctcgccggtcgacttggtcgggatgtgcgtcatctgcagccccgccttcgcgaggaacgacgccatcgccaggtgcgtggcactgccgttgccggccgaggcgtagttgtacttgcccgggttggccttgacctccttgatgaagtcggccgtgttcgacacgttgagcccgctcgacaccgccaacacgtagcccgcgttgccgatgctggccacgcccacgaaatccttcagcgggtcgtaggacagcttgctatacagaaagcctgcgatgtggtggctcgcggccgcgagcaccagcgtgttgccgtccggcggagccttggcgaccacggctgcacccaccgtgccgcctgcgcccgcgcggttctcgacgatggcgctggcgttgagcgccgcgcccagttcggcgttgaaggcgcgcgccaccgtgtcctgcacggcacccgtgccgaagggcacgacgatgtggatcacgcgctgctgctgcgcgtgcacgggcgtgatggcgcccagggccgtggcgactgcgagagcagccatcgaacgtcgggtgaacagggtggaggtcatcggggtggccgctttcaacatcgtgaacggaaaaaagttagccgcccgaaggcagccagcgctgcaccagcttcacgaagtagctggcgccgatcggaatgatctcgtcgttgaagtcgaacgaggtgttgtggatgatgcaagggccgggcccatggccacccagccggtggtcgccgtcgccattgccaagaaaggcgtagcagccgggccgcgcgagcagcatgtgcgcgaagtcttcggcgcccatcacggcgggaaagttgtcggtcaccatgtcatcgcccaccacctcgcgcatcacgcccgcggcaaatcgcgcttcggccacgtggttgaccaccggcggcgaggagcggttgaagaaaacctccgccgtgcagccatgcgccgcggccacgccggccgccacttcgcgcaggcgcgcctcgatcttgtcgatggcctcgatggagaaggtgcggatggttccgccgacggtcgccacgtctggaatcacgttcggcgcgtcggagccctgcagctgcgtgaccgcgagcagcgcgcgctcggtgctgggaatggtgcgcggcacgatggtctgcagctgctgcgcgagcgtgaccacggcggccacggggtcgatgccggtgtgcggcatcgaggcatgcgtgccgcgcccgcgcagcgtgatcttgtaggtgttgctcgacgccatcagcgcgccttcgttgagcgcgaagcggcccacgtcaccgaccgggaagttgtgcagcgcaaagaccgcgtcgcacggaaagcgctcgaacaggccgtcctggatcatcttcttcgcgccggccttgcccatctcctcagcgggctggaagatgaaatgcacggtgccgtcgaagtcatccggcccctgctgcgacaggtgccacgcggcagccagcagcatggtggtgtggccgtcgtggccgcaggcatgcatgcggccggcgtgggtggacttgtgggcgaactcgttggcctcgtgcagcggcagcgcgtccatgtcggcgcgcaggccgatggtgcgcgagccggtgcccttgcgcagcacgccgacgaggccagtgccggcgatgccgcggtgcacctcgatgccccattcggcgagcaggcccgccaccttttcggaagtgcggtgttcttcgaaaccgagttccggatgggcgtggatgtcgcgtcggatatcgacgaagcgggaggcgttgctggcgaaggagtcgacgatgttcatggtggcaaaggtcgtaagggcgaacgattctggcccaacgcggcactggccgccatgcccgccgtcagagccccgccagcacttggtcgagcgtctcgacgagcaggtcggcgttggcttcgctgaacaccaggggcgggcggatcttcaacgtgttggcatgttcgccggtggcgctcagcagcacctgccgctcgcgcaggccgttgacgacgcgcgcggtttccgcggtggcggccgtgcgtgcctgacgatccgtgaccagctccacccccacgaacaggcccgcgccgcgcacgtcgccgatcagcgcatggcgctcggcgagcttcgcgattccggcacgcagatggcggccgacgcgctgcgcattggccatcaagccttcgcgctcgatcacgtcgagcaccgccatgcccgcggccatcgacaccggattgccgccgaaggtgttgaagtagcggcactcgcggccgaaggcagccagcacctcgggccgcaccgcaaggccggccagcggatggccggcgccgagcggcttgcccatcgtgacgatgtcgggcaccacgccgtgccgctggaagccccagaacgcatcgccggtgcggccgaggccaggctgcacttcatcggcgatgaagaggccgccggcttcgcgcaccgcgtccacggcctcagccatgaagccgggcgggtcggtgaagatgccgtcgctcgaaaacacggtgtcgaccatcagcgcggccggacggatgccctgcgccttcaggtcggcgatggcctcgcgcacgccgttcgcaaatgcgcggcccatgtcaccggccaccacgcggtagctgtccggcgcgggcacggtgcgcaccgcatcgcccagctgcacgaacttgccgagcgagggcgaagcctctgcgatcgatgcagtgacgccgtggtacgcgaagcgcgtgacgatcagcccgtcggctttcgtatgcgctctggcaatgcgcatcgcgaggtcgttggcctcgctgccggtgcaggtgaacatcgcatggccgagttcggccggcatggtggcgagcagccgctcggcatagtcgagcacgccttcgtgcaggtagcgcgtgtgggtgttgagcacgcccgcctggcgcgcgatggcctcgaccacgtgcggatggcaatggccgaccgaggcgacgttgttgtaggcgtcgagatagcgcttgccgtcggcgtcgtacagccacacgccttcgccgcgcaccgggtgcagcggtgtttcgtagaacaggcggtaggccgggccgagcacgcgtgcgcggcgctcgacgagtgactgagtctgggggtcgagggaagtcatgggcgatctctcagaggttcacggcgccgcgaaaggctgctgtcgcggcggcagcgccgatgcgctcgcaggcctgcagccgggcccacgacagcgggttgttgcgcagcaggtagggcgcattctcgggatagcgcgcggcgcgccatccgctgatcgccaccaccatcacgagccgcgccgtgatcaggttgaacagcacgccgacctcggccggcgacagcggccgcaccgcgtggtacgcagcgaccagcggcacgatggccgcgagcgggtcgtcaccggtgccggcctggtacgcggcggccacggccaggtcgttgatgcacggcgcgcgcaccatgtcgccgaagtcgaggatcgcggcgatgcagtcggtgtcggccggatcgaccagcacgttgtagatgttgaagtcgttgtggatcggctgcgcaggcaacgtgcgcagcacgggcttggcgtcgcgctcgaagcggtcgagtgctgcggtggccagggcgcggcgctccggctcggcgatgtgcgcgagcaggccgcgcacgctgtcggcgcgctgcaggtcccagggcagcggcagtgcgccggccggatggtcgaagcccgcgagcgcgacgtcgagccgggccagcatgcgcgcgaggttctgctgctgcagcggcgtacgcggcgcctcgggcagcggcaagccgggcaggtaggtgaagaggcgcaccacgcgcggcagtccgtctcccgggtcgcacacgaaagaggcggcgccgtccttcgtcggcacgatgcgctgcaccggcaggctggggtcagtggcctcgaggtacagcagggcctgggtctggaagtcggcgaccaaggcggtttcggccgggtgcgagatcttcagcatgaagcgggcgccgtcggtggcgcgctcgaagcggtagttgcggtcgcgctcgccggtcagcggcttcatctcgccttcgatgccgtagcgctcgcgcgcgagctcgcgcacccaggcgtcgtcgagcgcgggcgagccttcgctgagtacctgcgcgtcggcgaattccgcaattctcattggtgcacccttggcgctgtgcgccttcccgccaagcgggagcgagcttgcttggggcggcccggcgctgcgctcatgccgcgctctcgaaaccgcgcagcgcgctcgcgatgttcgggcccaggtcgtcggaaaggtagccgccctcctgcaccagcaccgtgggcaggccgaggcgcgcgatctccgccagcagcacggcaaatccggcggtctggatcttcatgcccttgtacggatcgcgctcgtgcgcatcgagccccagcgccaccacgagtgcgccgggcgcataggcgcggatgctgtcgcatgcgtcgcgcagtgcgggcaggtagccgtcgaggtcggtgcccagcggcagcggcttgttgacgttgtagcccaggccttcgccttcgccgcgttcgtgcgcatggccgatgaagaagggcgtgaagttgcgcgggtcgccgtgcaacgagatggtcagcacgtcggcgcggcggtagaagatgccctgggtgccgttgccgtggtgcacgtcgatgtcgaggacggccacgcggtcgtgcacgccgcgcaggtgctgcgcggcaatggccacgttgttgaggtagcagaagccgttggcgcggtcggcgtaggcgtggtggccgggcgggcggcacagcgcataggccacgcgctcgccatcgagcaccagctgcgccgcatgcgtcgccatgttcgccgaggcaatggcggcctcccacgtgcgcgcgccgatcgagcacgcgttgtcgcccatgtggaaaccggcctggccgaccacgctgtcgggataggtgcagggctggcccggaaagggatggatgttgggcatcacctcttccgagggatcgtccagcagctgccagcgcgcgtaggctgttgccagaaagcgcaggtactcgggcgtgtggatggcggcgcgcgggccggcgccgaagtcgcgcgtggcgacgatctcgtggccctcctgctcgaccgccttcagcagccggaaggcgcgctcgggctgctcgttgctgcgcttgagcttgccgcgcaccatgaagagctgcgggtcgtggtccttgtgcgtgtcgctgtagacgactttcatcgggcggtttctccggtgtcaggcgttggtgggaaggggcgccgcgccgtgctgcttgacgaacaacgcgcgcacgtgctgccaggcgtcttccaggtgcacgcgcatcgcggccttggcggcctcggggttgcggcgcaccagggcgtcgacgatggggcggtgggtctccgccatcgcggtggggtcgtggtagaccgcatcgatcagcgcgatgatcatctgcatctcggtctgcgtgttcatgaagatgcggtgcaggtgcgcattgcccgacagctcgcagatcagcgtgtgcagcgccaggtcggtggcaatgcggtggtgctgcggctgcgtgctggcctcgcgcaccatggcttcgaccagcgcctgcacgcgcgcgatgcctgcatcgtcggccttgcggcaggccaactcgatcgaagtgagctccaggctcaggcgcacctcgaacagatcgtcgatctcctgcacgctgatggtccgcaccgcgaagccgtggcgcggtttggcgaccagcacgccctggcgttcgagccgccgcgccgcctcgcgcaccggtgcacggctcacgcccatgcggcgcgcgatgtcggcctcgacgatgcggctgccaggtggcaggcggccttcgacgatggcgcgcgtcagctgggcctcgaccagcccgacgagatcggtcgattcgaccgactcgaagagggccgtatcggaagaagaaggaggagaaattacggaagttgccatgttgcttgtctcgtcatttggtatgcgccgggagtgattcttcaccggatggcgtctgccgcagccggtacggtcttcagcccccgccccgcacgggccagatagatgcccgccgccatgatcagtgcgatgccggccatggcgatcgcatcgggcggcctgcggaaccagaaggtgctgaagcccacggccagcagcagctggaagtagttgagcggcgccagcgtggaggcctccacgcgctcgaaggcggccagcaagagccattgcgccgccgcgctgcaggcgccgcccgcgagcagcagcgccacgtcgctccacggcggctggtggtcgggcaggaagaagggcgcaggcagcagcgtgacgacgaagcagaccagcgcggtccaggcgtactgcaccggccccgcgaccaggcccgcgagccgccgcgtgagcagctggaagatcgcgtagcagacggccgccaccgccatcagcaccgttccgagcaggggcaggtcggccccgggccgcacgatcagcagcatgccaccgaagccgaccgtcaccgccacccagcggctgcgccgcacctgctcgccgagcagccacggcgacagcgccaccatcaggagcggcgcggtgaagtagatggcggtggcctcggccagcggcatccagatgagcgccgtcatgaagcaagtcgccaccgttgcgagcatcaagccgcgaagcagcagcaagggcttttgcggcgtgcgccacatgcgcaggtcgccatggcgcagcagcatcgcaaaggcaatgccgctcaccgcgacgtagcgcatcacgttgacgaagggcgccgggtagaactgcagcatgtacttgcagaacgcatcgtaggaggcaaaggccaccagtgcgcagaagaacagcgccacgccggcgcttttcgagcccgccgggcgcagcgggagggcagtggctgcgctgctcatcgcgcggcctggaagccccgcaggaaattgtcgagcgcggggccgatggcctccaccatgtagccaccttcctgcaccaccacggtcggcagcttcagcgcaccgacgcgctcgccgatgtggcggtaggcgtcgaggtcgagcttcagcacgctgatcgggtcgtccttgtagctgtcgaaaccgagcgcgagcaccagcgccttgggcgcgaattcgcgcagcgcggccgcgccttcatccaccgcctgcaggaacgtcgcgttgtccgcgccgtgcgccagcggcaggttcaggttgaagccttcgcccgcccccacgccgcgctcatgcgcatagcccgtgtagaacgggtagtagcccgagggatcggcgtgcgtcgacacggtcagcacgtcgctacgcgcatagaaaatgttctgcgtgccgtcgccatggtgcgcatcgacatcgaacaccgccacgcggccgtgccgctcccacaggcgctctgccgcaatggcgctgttgttgatgtagcagaagccacccgcgcgatcacggtgcgcatggtgacccgatgggcggcacagcgcataggccgcgtcgccgctttccagcaccgcatcggcggccgccaccgccgtgtgcgccgagcgcagtatcgagcgccaggtgtgtgggcccagcgggcacgagaggtcgctgatgtagtagcccgtgcgcgccaccagcgatggcgaggggcacggtgcgcgcgccacgcccggcgtgccgttgtagtagggcgaaagattcggcagcacctcgatgccgggctccacaccgggcacctcgagcttgcgccacagcgcgtaggccgtttccaggtagtcgagatagtcggcgctgtgcacggcctcgagcggcgcgcggccatagtccgcgggttcggccagcgcaatgccgcgcagggccaacgcgtcgcgcagcgcgtgcgcgcggctcggcaggtcggtcggcttgcagatgcggcccagccgcatgaactgctgtgggtcgtgcagcagctgctcgtccgtgaagaaggccttcatgcgaaggtgtcttcgaacaccgccatggcgcggccgaagcgcgcgaacatgtcgtcgatctgttcggccgtgacgatgagcggcgggcagaaggcgatggaatcgcccatcgcgcgcacgatgagcccttgcgccagcgcgagctcggccagccgggcgccggccttcaatgcggggtcgaatgtcgtgcgcttcgcggggtcggcatacagctcgatggcgccgatgagccccacgccgcgcacctcgccgacgtacttgcggtcggcgtggctctgcagcccttgctggaagtgcggtgccagcgactgcacgtgcgcgaggatgttctcgtcctcgtagaccttgagcgtctcgagcgcaatcgcgcaggcgaccggatggcccgagtaggtgaagccgtggccgaaggtgccgatctttccgctgttggcggccaccgccgcatgcaccttctcgttcaccatcacggccgagatcggcacgtagcccgacgacagcgccttggccgcggtcaggatgtcgggtttcaggccgaaggtggtggagccgaacatctggccggtgcggccgaagccgcagatcacctcgtcggcgatcagcagcacctcgtacttcgcgagcaccttctgcaccttgtcgaagtaggtggccggcggcaccagcacgccgcccgcgcccatcacgggttcggcgatgaaggcgccgaccgtctcggggccttcgtcgaggatgcgctgctccagcgcgccggccagccgcgtcgcgaagtcttcctcgctttcgccggcctcggcatagcggaaatggtgtgggcaatcgacatgcaggatgcggtcgatcggcaggtcgaagtcgcggtggttcggcaccaggccactcaggctcgatgccgcgacggtgacgccgtggtaggcgttgcggcgcgcgatgatctttttcttctcgggcttgccgatggcgttgtggtagtaccagaccagcttgaccgcggagtcgttggcctccgaacccgagttggcgaagaacactttcgacatcggcaccggcgccatggacaacagcttttcggccagcgcgatggcggccgggttcgagcggccgttgaacgtgtggtagtaaggcagcccgtacagcgcatcgctgccggccttggccaggcgctggttgctgaagcccagcgaagcgcaccacagtcccgacatcgcctcgagataacggcggccctggtcgtcctccacgaagatgccgtcgccgcgctggatcaccagcgggcccacttgcggatgcgtggcaaggttggtgaagggatggagatgcgcggcgatgtcggtggcggcgttctcggcatgcatgcttgcgttcatgaaggcggttccgttgtggagggaattcaatagccgcgcgccaggtcgacctggttggcggggcgctggccctgtcgcaccgacgcgagattgtcgagcgtctggcgcgcgatcacgaggctgtcggtgcgcgtggcgatgtgcggcgtgacgaggatgcgcgggtcgccccagaacggatgctccggcggcagcggctcttgcgagaaggcgtcgagcgtggccgccgagagctggcccgcgtcgagcgccggctgcaggtcggcctcgaccaggtggtcgccgcggccgacgttgatcaggtgcgcgccgcgcggcagccttgcgaacagcgcggcatcgagaaagccattcgtctcggcggtcagcggcagcaggcacaccagcgtgtcgcagcccgaaagaaattggtcgagctgcgccgcgccgtggaatccctcgacgccggccggcagggcctccttcgcgctgcggctccagccgcgcacccggtagccgatggcggcgagcgcctcggcgcaggccatgcccagcgtgccaaggcccgcaatgccgacgcgatggtggcgcggcgacacgaccggctgctcttcccaccggcgggcctgcgaactcgcgacgtaggcttgcatgccgcggtgccgctgcaccacggcccagcagacataggccttcatgccggccgccatgccggtgtcgacgatgcggcacagcggcaagtggcgcggcaactccgcgtcggccgtgatgtgctcgacgcccgcggccagcgactgcacgagccggagcttcggcatctgcgcgagcaggccaggcggcggaaaccagcacacggccgcatcgatctcgtccagcgcgcccagctccgcgcccaggcgcaggtcgatgcccggatgggcctcgcggaaggccacggcaagatactccatgtccagcaccgcgctgagaagcgcaacacgcggcatgccggcttcgtcgtccagcgccatcacgcgaccagcgcctcggccggcgacgcggaggacaccagccgcggcacggcctcgatcagcttgcgcgtgtaggcgtgcttcggatcgccgagcaccttgtgcgtctcgccgtattcgacgacctcgccgcgttgcatcaccgcgatgtggtcgcacatctggccggccacgcgcaggtcgtgcgtgatgaagaccattgcgagctggaactgctcgcgcacctgcgcgaagagttcgagcacctgcgcctgcaccgacacgtcgagcgccgacaccggttcgtcggccaccagcagttcgggctgcatggccagcgcgcgcgcaatgccgatgcgctggcgctgcccgcccgagaactcgtgcggatagcgctcggccgcgtcggcgcccaggcccacgagcttcagcagctccatggcgcgcgccatggcttcggccttgccgacgccctgcgcaatcggcccgcccgcaatggccgcacccacgcggtggcgcgggttgagcgacgcgtacgggtcctggaacaccatctggatcttgcctgcggcctcgcgccggaaggcgggcccctgcgacaggctgcggcccttgaagaggatgcggccgctgtcgaacggcgagagccccaccaggcagcggcccacgctcgacttgcccgagcccgattcgccgaccagccccagcgtttcgccgcggcgcagttcgaagctgacgttcttcgcggcctgcaccgagcggccgcgcttgaagaggccgttgcccgaggtgtaggtcttgcagaggtcctgcacctgcagcacgcgcgtgacttcgcccgttggcgtgtcgcgctcggcattgccggtgggaatggctgcgatcagcttgcgcgtgtaggggtgctgcggcgcatcgagcacctggcgcaccggcccgctctcgaccaccttgccggtctgcatcaccaccacgtggtcggcgatttcggacaccacgccgaagtcgtgcgtgatgaacagcaccgccgtgccacggcgctgctgcagatcgcggatcagcgtgaggatctgcgcctgcgtggtcacgtccagcgcggtggtcggttcgtcggcgatcagcagcacgggctccagcaccagtgcgcaggcgatcatcacgcgctggcgctggccgcccgagaggcggaacggataggcgtcgatcagcagctccgggtccggcagccccacgtcggccagcgcggccaggatgcgccgccgcttctcggccgcgggcacgctgccgtgcgcgtcgaagacttcgccgatctgctcgccgatgcgcatcacggggttcagcgccgtcatcggctcctggaacaccatgccgatgcgccggccgcgcagctcgcgcatctgcggctcggtgagctgcagcaggtcgcggccctcgaacaggatctgccccgccacaggctcgacgtgcgggcgcggcagcaggcccatcacggcgttggcgatcatcgatttgcccgagcccgattcgccgaccacgcaaagcgtctggcccggcagcaccgacagcgtggcgccgtcgacggccagcgcgcggtccgcgcccttgggcaggcggatgcccaggttgacgacgtcgagcaccggctgcaccggcttcatgggtgtgacggtggcgctcatttgcccctcccgtcgagccgcgtgttgagcccgtcgctcaggccttcgcccaccaggttgagcgcgagcacggtcagcacgatggccaggccggggaacagcgccatccaccaggcctggcgcagcacggtgcgcgcggcgcccaccatgtagccccagctcatctggttcggatcacccaggccgagaaagctcaggctcgactccagcaggatggccgtggccgtcatgagcgaggccatcacgatgatgggcgacatggcgttgggcaagatctgcgtcaagatgatgcgcggcgtcgactggcccgcgagcagcgcggcctgcacgaagtcgcgctggcgcagcgtgaggaattcgctgcgcaccagccgtgccaccggcggccacgagacgatggcaatggccacgacgatcgagttgaccgagggctggaagatggccaccagcacgatggcgagcgcgaagctcggcacggcctggaacagctcggtgaaccgcatcagcgccgcgtcgatccagccgccgaagtagccggcaatggcgccgagcgtcacgccgatgagcagggccaccacggtggacaccagcccgatcagcagcgagatgcgcgcgccgtagatcacgcccgagaggatgtcgcggcccagcgtgtcggtgccgagcgcgaagccgggctccgtccacggccgcaggaacggctgctcgaccatgttccacggatcgttggtcgcaacccacggaccgatgatggccaccacggccaccagcagcagcaccgccatgccgagcacggcgcccttgttgcggcagaagcgccgccagaaaggactttgcagcaatgtcatagctctatccgcggatcgaccaacgtgtagacgaggtcggtgatgaggttgaacagcacggccatcgccgcggtcaccaggaaggcgccgagcagcaggttgtagtcgcgctgcagcagcgcgtcgaacatcaggcggccgatgccgggccaggcgaacacggtttcggtcagcaccgcgccgccgatcattccgccggcctggatgcccgcgagcgtgaccaccggcagcagcgcgttgcgcagcacgtgcgcgcgcaggatgcggccgggcttcacgcccttggcgcgcgcggtcttcacgaagtccatctgcgccacctcgagcatggcggcgcgcgtcatgcgggcatacaccgccatgtagaagagcgcgagcgtcagcgccggcagcaccaggtgaccggcgatgtcccaggccagcgcgaggccggtggccccggagcccacggtgctgaagccgaagcccggcagccagtcgagctgcaccgtgaacaccagcaccgccatcagcgcgagccaatagagcggcgtggcatagaagatgagcgccaccaccgtgatcgagctgtcgacccaggtgccggcgcgccgcgcggccagcgcgccgagcgtgatgccgaacagcagcgacagcgcgaaggccgtgcccgtgagcagcagcgtggccggcagccggtccatgatgagcttcagcaccggctgctgttgccggtacgaaaagcccaggtcgagctgcaccaccttgccgacgtaggtggccagctgcgtcgtgatcggctggtcgagcccgaactgcgcgcgcagctgcgccacgaactgcggatcggacgcgcccgcctcgcccgccagcaccgacaccggatcgcccggcgccgcgcgcaccagcatgaagttgaccgtggcaatcagcaggatcgccagcaggccctgcatcacgcgacccagcatgaactgcgtacgtttcatcggcagcctccatggctgcgtggttgcggcgccgccatcatcatgcgaccgtcgccgtgcccaggctgtcgttcagtccgattcccgatgtgatcaggttgccaagcttcgtgcggtacagcgtcggaaagttgagctcatgcagccaggccacgggcacttcgtcgagcaggatcttctgcacctgcaggtagatggccttgcgcttttccgggtcggcctccttggcgccggcatcgaacagctcgtcgaccttcggattcgaatagccctcgacgttgttgaacggcgagcccttggcgatgttgctggtggtgtagttgcgcgccacgcccagcgcggggtcgccgtactggtacacgtaagtaaaggcgaggtcgtagtcccactcgttgagcttctggttccagcccgcgacgtcggtggccaccagttcaaccttgatgcccgcctgcgccaggttctggcgcaggatttcggccgagcgcgtccacgtctcgccgtagggcaagggcagcaggcgcagcgtctcgcccttgtagccggcttcttccagcagcttcttggcggtggcgacgttgcgcgggtacttggcaacgtcggtgctgtggaacttgatgttgctgttgaacggcccggtggcgggcttggcgaagccttgccatgcgatcttggccatcgcctcgcggtcgatggcgaacatcaccgcctggcggaacttgacgttgtccatcggcgccttgcggttgttgagccacaaccacgaatgcggcgcgaagaactcccagcccttggtggtgaccgcgacgccgggcagcttggacagccgcagcacgtcgaagtattcgaccgccccgcccggcaccaggtcgaccttgcccgactcgaacgctgccgcacgcgaggccgcatcgggaatgacgtggaagtacacgctctccaccagcggcacgtccttgacgtggtacttgtcgttggccacgagctggatgtacgagcccttgacccattccttgaacttgaacgggcccgtgccgatgggcgtggcgttggcggggttggtcgcgaagtcggtgccttcgtagatgtgcttcggcagcatcggcatgctgccgacctcgaagatgccgatgaacgggccgaaggggtacttgagcttgaactcgaccgtgagcggatcgagggccttgatgctttccaccgacgccaggttggcgcgcaggcgcgcatgcgtcttgcgcaggaacacgtcagccgaaaacaccacgtcggccgaggtgaagggcttgccgtcgtgccaggtgacgccgggcttgagcttgaaggtgtagagcgtgccttccttgttgacggtccacgaggtggccagcgagggtagcgggttgatcttctcgtcgtagcgcagcaggccctcatagatgttgcccgagatcatctgcgtggggccgttctgcgtgatgcccagcatgagccccggcggctcgggctggacgacggcgttgatcacgccgcctttcttgcccgcggcgagcaggtgcaagggaacgcctgccagcgtcaggccggcggtggcagcggcactcatctggatgaggttgcgacgtttcatgtgcggaaactccttgtggctctgtcgagcgggtgggtcgaaaagaaacgggaacggaagaacaccggcgccgcggcgccgcaatcagtcgcggtacgacgtggcgggaagcggatcgatgcgctgcagcagcgcgcgccattcgcgcgcgttcgggtcgggctggcccggctcgcgcacggtgtcgccgctttcgtactgctgcgcggtcttttcgcagacctcgggcggcaccggatacacaggctgcccgctcgaggcgatggccacctgcacacggcaggcgcgctccaggttcagcatcaggatgaaggcctccgacacggtgcgccccagtgtgaccaggccgtggttgcgcaggatcagtgcgcgcgcgctcgggcccaggtcggccaccaggcgctcgcgctcgtcggcgtcgagcgcaatgccttcgaagtcgtgatagaccacgcggttgtagaactgcagcgcccattggttgcacggctgcaggccgcccgccagcgacgacaccgccacgccggccaccgtgtgcgtatgcagcacgcaggccgcgtcgtggcgcgccgaatgcacggcgctgtggatggtgaagccggccgggttcacgtcgtagggcgagtcgtcgaggatgcggccggccaggtcgatcttgaccagcgacgaggccgtgatgtcccggaacagcgtgccgaaggggttgatcaggaactggtcttcggcccccggcacacgcgcggagatgtgcgtgtagatgctgtcgtccatgccgtagtgcgccaccaggcggtaggccgcggccaggtcttcacggacctggcgctcggcatcggaaacgggtgaggccttgcggcccactgcctgcaattgcatgtcgctttcctcttttcaggccgggcggaaatccccggcgctttttggggtccatcggatcgacagtgcaaactgtcgacagtcaacccgcgacagtcttaagcaatatgcaggcccgcgtgatggggtaagcccttggtgaggggcgttgacgggcggaaaacggcgccggcaaagggccggcgcacaaaaacgaacgccgcgggcaccgggtgaagtgcgcgcggcggtgacgccggatgggctggtcgtgcgccatcaaggcgccgggtgcaccagggtgcaccgggaaaatgcacctccctcagcccaggcgcccttcctcgcgcagccgcgccccgatgcgccggatctcggcctcgccctggtcgagcgccgccttgctggtgtgcaccgaatagcggcccatcaccagctcgtgcgggtgcctcgcggccgagcccagcacgaaggccgtgtcgccgtgggccacgaagtcgatggccgcgccggattcctcgaacaccgcgagttcaccggtggcgatcggctcgccgctgccgtcgccggcgtcgagccgcccggcgctgactgcgacccagcccaccgtgtggccggcgggcggcgtgtagcgccagtgctcgccgtccttcaactgcacggccaggtagttgatgggcgcgggcgccggaatggggctttgcgccgcgccgtagcgaccgagcagcacgcgcgccgggccttcgcgcggcacctgcgagggtgccaggtagatgctttgggccggcgcgttttcttccgcggccggcagggccacccacaactggaagccctgcacgcgcttcgtgtccggtgcgggcgcaccgtcgtgccacacgccgttgccggcgcgcatccactcgacgccgccggccggcagcacgcccttttcgccggtcgtgtcctcgtacaccgtgtcgccttcgatcagccacgtcagcgtggcgatgcccgagtgcgggtgaatgccgaaccccttgcggccgccgctggtgtcgaagccgaacaggtcgaggaacacgaagggcttcagaaattcgcccaggtcgcccgggctcatgagccggatgatcggcccgtgctgcgagccacgtgtgcggtagacgatggggcgggcggcttcggtggtggcgacggtggcggatgcggcggtcatgcggcctccctcgcggtcttcagcgccttggtccaccacgcgaggtcgtccagcatgccggtggcggcctgcgccaggtgcggaaagtcttcgaagctcttgccctgctgccagatgccgagaaactcgaccatgccgatgtgcacggcgttgcgcaccggcgccatctgcatctcgaccgcgaccagccgcagctgctccacggcacgcgccgcgcccacgccgccgtatcccacgaagccaatcggcttgcggacgaactccttgtaggcccagtcgatcgcgttcttcagcaccgcgctcagaccgtggttgtattcgggcgtgacgacgatgagcccgtcgaaggtgtccagcttggcggcccagcgccgtgcagcctcgttcttcaccgagccccaggccggcgcgcccgcctcgttgaagaagggcagcggatggtcgcgcaggtcgatcagttcgaacgcgagatccgtgcgctgcgtcgcgagctgatggatccagtacgccggcttgtcgccgaagcggccttcgcgggtcgagccgatgatgatgccgatgcggggttgtggcgaagtcatggggtgctcctgaattgggggacgagaagaagaaaaagggagttcaggccgtggtggccgccagccgcggcacgggccgcaggcgccaggtcacgaacgccgaaagcagtgcgagcacgatggctggagcggggctgccgccgatcagcaccaggtgcgtgaccacggcaaaggccatggtcacggccatcagcaagccgccgaggaaaccggccgccggcacgagcagcagcaccgcgccgccgacctcgaccacgcccgtcacatagcggaaccactggccaaaaccgatggcgtcgaacacctggaccatctgcggcgcgccggacagcttggcgatgccggccgcaccgaaagccagcgccagaagaatccgaaggccccagacgatgcggcgctgggtgggagatgaagaagttgaagaagtcatgggtccaaggttaggaccgcacccattgatcgactagacggcagaatcggattgcactcgtccaccgaaagaaggaattgccgccatgctcgacctcaacgacatcgccatgtttgtgcaggtggtgcgccacggcagctttgccgaagcggcgcgccggctcggcctgccgcccaacaccgtgagccggcgcgtccagcagttggaaacgcagctgggcacgcgcctgatgcagcgctccacccgcaagctcacgctcaccagcgcgggcgaggcttttcatgagcgctgcgcgggcgcggtcgacgggctggtcgaggccggacaggaactgatcaccggcagccgcgaacccagcggcctggtgcgcgtggcggcgacggccgactttttcgatttcttcccgatggaatgggttgccgacttcctggccgcgcatccgctggtgcgcatcgacttcgtgctcagcgacgccaaggccgacctgatcgccgaacgcatcgacatcgcattccgcggcggcgcactgcccgactcaggctacgtgggccgcaagctcatgagcgcgcggaccgatggcatggtcgcgagccccgcgtacatcgccgcgcgcggtgcgcccgccaccttgcaagacctggcggcgaaccacgactgcatcacctcgccccatcccagcggccgcaccccgtggcgcctggccggtcccgacggcgaggaagaagaagtacaggtgacgggccgcttcaccggcaacaccgcgcaggcgctgcgcaaggccgcgctcgccggcctgggcgtcgcgctgctgccgcccaccatggcccggcccgacctcgaagccgggcggctcgtgcgagtgctgccgcagtaccagcgcacggggcaggggttgagcgtgctgtacccgagccggaagcacctgccgctggcggtgtcggcgttcatcgggatggtgatggagaagctgagtggggtggaggggttgccggagatgttgcggggggcgaaggcgtagccccaccggccagccgatttgcacagaaaatgccctccatgaaaatcgaaaaagacaccgtcgtcaccctcaagtacaaggtcgccgacgcccagggcaagctcatcgaggccagccccgagccgatggcctatctgcatggcgggtacgagaacacgctgcccaagatcgaggaagcgctcgatggcaaggaaaagggctaccagaccacgctgcatctggcgccggaagacgccttcggcctgcgcgacgagtcgctggtgcgcagcattcccaaggccgactttccgccgggcgtgaaggtcggcgggcagctggaggggcgactcgacgacggacgcgagcacctgtttaccgtgatgaagatcaagggccctgtcgttctgctcgacggcaaccatccgtgggcgggcaaggcgctgcgcttcagtctccaggtgacggacgtgcgcgcggcgctgccggtggagatcgagcatcggcatgtgcatggggcgcacgggcaccatcactgatcgttgggtttcagtcgcctagttctgctttttcttcttccagaaccgcggcgccttcacgatctcgccaagcgccttgcggcaggcctttgcgcccgccgcgtggcgagcgctgaaccagccgacggcgaaccaggcgcgggcatcgcgcgcggtggcctcgcggtagagggcctgtgcgacagcttcgtcgttgaactcgcccagcgcgtcttgcgccgggcgcagacgtttcaggtagcgctcggcggctgatttttcttctttatcgtccgcatcggcgaacaacggcatcacgaactcggcgaggtagcgcaggcgcttgagccttttgcgcgtgcgatgctggtcttcggagttcagcgactcgaagcgccggccatcgcgcacgatctgtccatgcaggcgctgcaagcgcttgcgcagatagcggcgcgcatcgccggcatccagcggcccggatggcgagggggcttgttcgggtgcttcggcatcgcctttgggcgcgtcttccactgccgccgttgccgccgcggtgaacccaatcagcgaaaccagcaccgattgaaaagccggcgcgcgcacgacgtcaccgggcgaaggcgcgtgggccgctgcggcatcgtcgccggccagcggatcgaactccggcgcgcccgcgtctcgcagttgcggctgcgccagcttcacgacctgctcgcggtcgcgcagcacaccaagcgcgcgaaaggcctcgaccagcggcggctcccatgcggcgccgttgaaaagatccgtacgctcgtcgagtcccgccagttcgcggatcgcggtgcgcaggcgccggatgccgatgcgcagttgatggatctgctcttcgtcggcgctgcccgccgcgatttcgctggcgttgggcagtatctgcgccaggcaggacgcgacgacggcttgctggatggctcggccgccgagcttgcctttctcttcgggaaagcaaggcgtctcggccttcaccgccggaaccacgtcgagctttgccaacaagcgcgcgccacgctcggccttggaaacggtgctgaaccacaggccgtgctgctgcgaccagcggcgtgcgagcgcggccaggccctgcacgtcgccgcgcttgagttcgagctccagctcgcacaccggcgattcgcgttcgtcgggcgtgcccgcctgggcgacgaccttgccgacgtcgagcgccagctcgaccacggcgccgccggctgccgtggtgcgcacgtcgcgcgtgagccgcacgatgtcggtcgactggcgctcgaccagcggcgcgccgctcgcggccagcaccttggcgagccggtcgcccacgggcgtgccctggtggcgctgcgggtcgatggccggcaccgcgctgccggccgctgcggcgcccaggtcgacgttgtgttcgagccggtgcagcgcgttgtcgcccgtggccttggcggtctgcacccagcgcgggccctccttgcgcagccgcagcacgatgccttgtgcggccagcgcctggtcggcagtgtcgaaatagcgcgcctgcaggcgggtgcgcaccacggtaccgcgccgcagggcggtctcgacggctttcaggtgccccgagggaatatgaaacttgaactcgatttccatggcggccatgatgctccgttcgagcactcctgaacacgccgccgaagcgagaaaggtctccatgcgcacgacatcacccgaccccaccgccttgctggcagcgggcgccgcacggtcagccaaggcactggttgccaaagaggcgagtgccgtggaattgtgcgaagccgccatcgcccgcatcgaagcgctcgatggcgcgctcaacgcggtggtggtgcgcgatttcggccgtgcacgccgccaggccgccgacgccgacgcggcccttgcgcgcggcgagcgccggccgctgctcggcgtgccgatgacggtgaaggaagccttcaacgtcgcgggcctgccgacctgctggggtctgccgccgttccgcgatttcgttccgccgcatgacgccgtcgccgtgcagcgtctgaaggcggcaggcgcggtgattctgggcaagacgaacgtgccgccgggtctggccgactggcaatgcgacaacccggtgtacggccgcacagtgcacccgctcgatcctttgcgcacgccgggcggctcgtcgggcggcggcgccgtggcggtggccacgggcatggtagcgctggagctgggcagcgacctggcgggttcgctgcgtgttcccgcgagcttttgcggcgtgtacgcgcacaagccgagcgagggcttgctgccgacgcgcggctttgcgtttccgggcaccgaggaggcgctcgccgggctgccttcggtgatcgggccgatcggccattgcgccgacgacctgttgctggcgctgcaggtgctggccgggcccgacgcagcccatgtggctgatggttgcttcgcgctgcccccgccgcgccacgcagccgcgaaggattggcgcgtgctcgtggtcacggcgcatccgcaggccgccgtggcagcggaggtgcgcgccgccgtcgaaggcgccggccggcggctggcgaaggcgggcgccgtggtggccgaggcctccgatctgctgcccgatctgagcgagatcggcaacacctacgaccagatcgtgcagaccgtgctcgcacacgccgagccgggcggcgggtcgccgatgtcgctgcacgcctggttcgacctgctggccacgcgcacgcgcatccgggcgcagctgcgggcgctgttcacgcgattcgacgcggcgctgtgcccggcggtcggctgcgcggccttcgagcatgtggccgagacggatttcagaaagcgaatactcactatcgacggcgttgcgacgccttatgacgcgctgggcgcctgggccgcgttggcgagccttggcggactgccggccacggtcgctcccgcgggcttcgcgaagggcggattgccgctgggcgtgcagatcgtcggtccatatttcgaggaccgcagcaccatcgccttggcccgattgctgactgaggacagcagcgtttgaaaaataatgtggacaccgtccattttctttgatatcttttgtggacggtgtacacaactcaccggcaaacacctccatcaacctttcaccgaaacaggaagacaaccatggccaacaagcaaatcttcgtgaacctcgccgtcaagaacctcgaaaagtccaaggctttctttgccgcgctgggctataccttcaacgagaaattcaccgacgccaacgccgcctgcatggtgatccaggagggcagcatccacgccatgctgctggtcgaagacttcttcaagaccttcacgagcaagagcctgacggatacgagcaagagcaccgaggtgctgctgtgcctctcgtgcgaaagccgggccgaggtcgacgagatggtcgccaaggccgtggccgcgggcggcacggtgccgcgcgaaccgcaggactatggcttcatgtacggccacggcttccaggacatcgacggccacctgtgggagctgatgtacatggacccgaacgccgaagtgccccaccagaacccgtgatgccgcggcgctgaaaagaacgagcgcgatgcccatcgttccatatgcgcttctcactgttgcgcgaaagggccctttcttaaagcgcgcgagccccgatattccaaggaacagcgccgccgtacgttcggcggcgcacccaacggaaaggaataccgaggtgtccagcaacaacattgatgaagaagaagcccgcagccccgtcctgcaggtgagcccgctcggctttccgtggcagacgatcgacccgttcctgttctgcgtctatcacgacgacgcctatcccaaggccaacgcgcggatggggcccgaagccccgctggcgggccgtcagatcggccaggacttcagccgcaaggacggctggagcatgtaccacggcgagacggtgccgggcttcccttcgcacccgcaccgggggttcgaaacggtgaccatcgttcgcaaggggctggttgaccattccgattcgctgggcgccaccgcgcgcttcggtggcggcgacgtgcagtggctcacggccggcaagggcatcgtgcattcggagatgtttccgctgctcgatgcgaacgcgcccaacccgctggagctgttccagatctggctcaatctgcccgcccgcagcaagatggccgagccgcacttcacgatgttctggtccgaagcgattcctcgcttcgcatcggacgacgcgaagggcggccgcaccgaggtcgcggtcatcgcgggccggttcggcgacgctgcaggcaacggcgaggcaccagccgcgcccattgcaccgctcgcgccgccgcccgattcatgggcggcaaaggccgatgccgacgtggcgatctggacgctcaagatgacgccgggtgcccaatggacgctgccggcagctgccggcgaaggcacgcagcgcatgctgtatttcttcaagggcgccgtcgcgcacatcgcgggccggcgcgtggaaggcccggccgccatcgagctgcgtgccgacgcgtccgtggaactgctcaatggcgacggcgaagcaagcgagtttctgctgctgcagggccgcccgatcgctgagccggtggtgcagtacggcccgttcgtgatgaacacgcaggccgagatcggccagaccctggacgactaccgccgcacgcagttcggcggctggccctgggacgatacggcaccggtgcacagccggggcgccgcgcgctttgcgcggcaccctggcggccgcgaggaaacgccggaagcctgaagcgcgcagcctcgaggccgcgtcaaacggtcttgaggatctcggtggcgggggcggtcatgctcggcacgaactcgatcacttcggtggtcgccacgccgttctgcacgaacggatcgcgtgccagcaccgcctcgagcgcggcccgttcgccggaccgcgcgaagatcacgccgcccttgcgcggcacctggcggccggaggccaggaagagtccgctttcatagtgttttcgaagccaggtcatgtgtgcgtccatcaatacatcgagctcttcgaggggacgaatgtaggtcagggtgacgatgaacatggcaaaggcggcaagtggatcgagctccgatcgtatggccttgcctttccatttcgtgacaccagaagtaacggagtgatccagtttttacgggtttctgctaccgtcttttctaccgttcccaccgctcgaggagagttgctcatgccgcttcggtcgccgccccttttgccacccagcttcgtaccgccgtacctgctggaccggctggcggaacgtgccagcgcgcatgccagcgcacgggcggctcagacgctgatgatcgaccgcgaacaccgcggccttcgcgaagcggtggcttcgaaaggcgtgtcgtcgggcccggcgccgcgctaccttcggcgcggctcgcccgcgcgcgccatccacgacgcggggcacacgatgagcctgcccggcaagctggtgcgcgccgaagggcaggccgccaccggcgacatcgcagccgacgaggcctacgactacctgggcgccacctaccgcctgtaccacgacatctacgagcgcgactccatcgacgacgcgggcatgccgctgaccggcagcgtgcactacggcaacgactacgacaacgcgttctggaacggcaagcagatggtgttcggcgacggcgacggcgaagtgatgaaccgctttaccattgcggtggacatcatcggacacgagttgacgcacggcgtcatcgatcatgaatcaggcctggtctaccagggccagccgggtgcgctcaacgaatcgatctgcgacgtgttcggtgtcctggtcaagcagcacctcctgaagcagacggcacagcaggccgactggctggtgggcgcggggcttttcaccgccaaggtggaggcgcgcgcgctgcgctcgatggccgagcccggcacggcctacgacgacccggtgctgggcaaagaccctcagcccgcccatatgaaagactttgtcgtcacacggcaggacaatggcggcgtgcacatcaattccggcattccgaaccgcgctttctacctcgccgccacggccatccccggcgcggcatgggagaccacgggccgcgtctggtacgacacggtgtgcgaccggcggctgcgccaggacgccgatttcgaggccttcgcgcaactgagcgtggagaatgcggccaggcgcttcggcgccgacagcgcggtgcacaaggccgtcggcgcggcatggaacaccgtgggagtcacgccatcatgattcagcttccacccctggaccaggcttccgtcgtgcgggtgacgcgcgagggcggcgttgcctacttgccggggctttcgcgcccgcgcagctaccagttggggaattgcagcgaagaattgcgccagcagatcggcgaggcattgcaaagcgctgccccgcatgcggagcagggcggcggacccggctcgcagggcggcgaccagcgcttctaccgtgtcgaagtgctggtggaaagcgccaccgcccgttcgggttcggtcagcttcgaagtgcccgagtccgaggcgcccgaagcgctggtgcacctctggaaagacgccgccgaccgctgaacccttgcctcgaaagagcatgcgcgcgatgacagggtcgcgtgcgggaccagcgccgaagcggcgaatcttttagattcggcgactgccatccacaaccacaccggagctctttttccatgatccacgtcgtcgccgtcatcaccgccaagccgggccaacgcgccaagctgctcgaagcctttgccgccaaccgcgcggcggtgctggccgaagagggctgcatcgaatacggggccaccatcgacgcgcaaggcgttccgacatcgaaagccagcttcgggcccgagaccttcgtggtcatcgagaagtgggaaacgctggcgcacctgcaagcccatgcggtggcaccgcacatggcggcgcacggcgccaggacgaaggagctggtcgagagcaagctgatccacgtgctcgaaccggtctgagaggtccgccagcgggccttcgcgcgcggcgcaatgcctgctaccctcgcgccgggagcaggcatctcgaggagggatacaaggcatggcgatcttcttcagaccgcatggtttgcgcttgcgcgctttcatcgcaacgctcggcacgctggccgcggggttcctggtgtccggctgcgcgcagcttgcagcaccgccctacgcggccgactacgaagtgctggaccggctcgaagccgcgcgccccggcatggtggccgtggcgaaggtgcagccgaccgatccgaacgacggcatcaacacgctcggcttgcgccgcgcgaaactggtatcgcccagcggcaccttcgcgcaatacctggaagacgcgctgatgcgcgacctgggagagatatcggcctacgaccccaaggcgccgacccgcgtcgcggcgcgcatcctggtcaacgaactcgaccttggcgtgatcaacggcagcggccgcatggacgtggaagtggtcgtgacgcgtgcggccgcacagcggttgcgcaagacctaccgcggcgagatcgccttcgattcgagctacgcgaacatcgtggccgtgcccgccgggcaggccgcctacccgcggctggtgcgcgcgctgctgcgccagatgtatgccgacccgcagttcgtcgcggccatcgcgccctagaaccggagaaagccgcaccatgccgtttcttcattcttcggccactcgcctgctggccgctgtcgccctgaccatcgcggtggccggttgctcccatccgatcacgatgatcacgcagacggcgccgccgcgcgcaacggcccatctccttccgaagaaggtggcctacgtgatgaccgacgcccagcgcgaccagcaggtgaccaccgccggcggcagcggcgaccgcgtgagctactacccgtaccgcgatctggaaaaatcgattcgcgatgcgctgcgcgcggtgtaccgcgacgtggtcgtgctgcgtaccgccggcgatgccaaggccaacgagaccgcgggcgtgtcgctggtgttcacgccgcagatcaagaccgattcgagctcgtcctcctggatcacctggccacccacgtcgttcaccgccgaggtgagctgcgtggtgagcgatgccgcgggcgccgaggtcacgcgcgtgcgcgcggtcggcaacggcacggcggaattcggcgagttcaacggcgactacggactggccgcccggcgcgcggcgacgcggatgacgtcgcagctcagcagcgagatccggcggaacgagaagctgcgctgaggcgattcgctcctctgcgagcccaataaaaaacgcgcccgagggcgcgttttttattggagcttcgaaggcttacttcgaaaccaccttcaccatttcgaggcacttgttcgagtagccccattcgttgtcgtaccagctcacgagcttcacgaaggtgccgtccagggcaatgccggcttcggcgtcgaagatcgaggtgcgcgggtcgccgcggaaatcggtggccaccaccttgtcttcggtgtagcccagcacgcccttgagcgcgccttcgctctgcgacttcatttcagcgcagatttccttgtaggtggcttccttttccagctcgaccgtcaggtcgaccaccgacacgtcggaggtcggcacgcggaagctcatgccggtgagcttcttgttgagctcggggatcaccacgcccacggccttggcggcgccggtgctcgagggaatgatgttttccaggatgccgcggccgccgcgccagtccttgttgctcgggccgtcgacggtcttctgcgtggcggtggcggcgtgcacggtggtcatcaggccgcgcttgatgccccacttgtcgttcagcaccttggcgagcggtgccaggcagttggtggtgcagctggcgttgctgacgatggcttcgccggcgtacttcttgtcgttcacgccgtagacgaacatgggggtgtcgtccttcgacggggccgacatgatcaccttcttggcgcctgcctcgagatgcttctggcaggtttccttggtgaggaagaggccggtcgattcgagcacgatgtcggcgccgacttcgttccacttcagctgcgccgggtcgcgctcttgcgtcaggcggatcttcttgccgttgacgatcagcgtgttgccttcaaccgtgacttcgcccttgaagcggccgtgcaccgagtcgtactggagcatgtaggccaggtagtcgggctcgagcaagtcgttgatggcaacgatttcgatctcgttcttgaagttctgcaccgctgcgcgcagcacgttgcgaccgatgcgaccgaagccgttgataccgagtttgatagccatctgatttgctcctaaggttgaaaaactttttgatcgaacagaaagaaagaatgcgcctggccgggctcagtcgcgcagggcggcttcgaccgtggcggcaacgttctctgccgtgaacccgaaatgcttgaacagcgccgatgccggtgccgactcgccgtagctgtcgatgccgacgacagccgcgcagccgtacttccaccagccgccggtgcaacccatttcgacggcgatgcgcggcagcttcttgggcagcacgttcttcttgtaggccacgtcctggcggtcgaaggtggtggtcgagggcatcgacaccacgcgcaccgcaattttcttctcggccagcaatttctgcgcggcgagggccaattgcacttcggaaccggtggcaatgatgaccgcggcggtcttcttgctcttgaggccgacgacctcgggttccgacagcacgtaggcaccgcggctgatgtcgccgaggtcgcccttcggcgcataggcgatgttctggcggctcagcagcagcgccgtcgggcgcgactggttctgcagcgccacggcccaggccacggccgtttcggcggtgtcgcccggacgccagacgtcgaggttggggatcaggcgcagcgacgcggcgtgctcgatcgactggtgcgtggggccgtcttcgccaaggccgatggagtcgtgcgtgaacacgtgcaccacgcggcgcttcatgagcgcggccatgcggatggcgttgcggctgtagtcgctgaaggtcaggaacgtgccgccgtagggaatgaagccgccatgcagcgagacaccgttcatgatgccggccatgccgaactcgcgcacgccgtagttgatgtggcggccgatcacgccatggggcggctcggcgttgtcggcggtgctctcgggtgcggcttcgtcttcggcgccctggttgggctgctggaccggcacgtccatgaccacggtgccggtcttcgcgtcgaagcgcagggcggccgtgctcttggtgttggtgaggttggagccggtgaggtcggcgctgccgccgagcatttcaggcagcgcggcggtgaaggcctcgagcgcgagctggctggccttgcggctggccacggtttcgcccttggtatgggcggccaccacggtgtcgaacgccacttggtggaagttcttgggcagctcgccccgcatgcggcgggtgaactcggcggcgagttcgggaaaagccttggcgtaggcgtcgaacttgtcgttccaggcggcttcggccttggcgccctcggccttgtggtcccagtcgtcgctggcttccgccggcacctcgaaggccgcgtacggccagttcagcgcagcgcgggtgagggtgatttcctcggcgcccagcggctccccgtgggccttggcggtgttggcgcggttcgggctgcccttgccgatctgcgtcttgcagatgatgagggtgggcttcgaatcttccttcttcgccttggcgatggccttggacacgtccttggcgtcgttgccgtcgatcgggccgatcacgttccagccgtaggccttgaagcgttcttcggtgttgtcgatgaaccagggcttgacctggccgtcgatgctgatgccgttgtcgtcgtacagcgcaatcagcttgttcaggtgccaggcgccggccagtgcgcaggcttcgtggctgacgccttccatcatgcagccgtcgcccaggaaggcgtaggtgtggtggtcgacgatcgcgtggtgcttgcggttgaactcggacgcgagcagcttctcggccaatgcaaagcccaccgcgttggtgatgccctggcccagcgggccggtggtggtttccacgccgggggtcacgtcgacttcggggtggcccgcggtcttgctgtgcagctggcggaagttcttgagctcgctgatcggcaggtcgtagccggtgaggtgcagcaccgcgtacagcagcatcgaggcgtggccgttcgacagcacgaagcggtcgcggtcgaaccagtgcgggttcgcggggttgtagcgcaggtgctcgccccagagtgcgacggccatgtcggccatgcccatcggtgcgcccggatgtccggagtttgcttgttggacggcatccatggccagcgcgcgaatcgcgttggccatcagggcttggtttgccatgggcggaggactttcggggaatgtggattggggggaacccgcgattttaccgggctcgctccgacccccttcaatacgccttcgacacccggccgatgttcattggcagcgcccggactgctagagttgccacccatgcatgggctgcacctcaccgccgatctccacgactgccaatgcgggatgcaatggctgaccgacaaggaggcgctgggcgccgtctgcctcaaggcggtcaccgccgccgggctgcagccggtgggccagctggtccacggatttccggccacgccagagggaccgggcggcgtgacggccacggtgctgctggccgaatcgcacctgtgcatccacacctggcccgaacagcgcggcgccacgctcgatgtgtatgtgtgcaacttcggcggcgaccattcggccaaggcgcatgcgctgatggaatgcctggtttccctgttcaagcccggccacagcgaacgcaacgagttgctgcgcggcaaggtggcggcttgagcacccgggcttccgttcgggcgatgatccttgccgcaggccgcggcgagcgcatgcggccactgaccgacaccacgccgaaaccgctgctcgaagtgcgcggcaagccgctgatgcaatggccgatggaggcgctggccgccggcggcttcaccgaactggtggtcaacaccgactggctcggcgagaagatttccagccgattcggcgccaagcccttgctgaatgggcgcagcgcgctatcaatttcatattccgacgaaggccgcgactttggtggagcgctggaaacggccggcggcatcgtgcgtgcgctgccccggctgggcgaggttttctgggtcgcggccggcgatgtgttcgccccggatttcgccttcacgcaggctgcggtcgaccgcttcgcggccagcggcaagctcgcccacctgtggctggtgccgaacccggcgcacaacccgaagggcgatttcgggctgtccgccgatggcctggcgctcaattcggcggccgaaaaatacaccttctcgaccatcggcctgtaccgcgccgcgctctttgcgccgccttactgcgacattccccccggcaacccggcaggcaccaaagccccgctcgcacccattctgcgcgccgcgatggacaatgaactcgtgagcgccgagctctacaccgggccctggaccgatgtgggaacgcccgaacggcttcttcaactgaacacgccaagatgacctcagaacacgacaagatctacgccgagcgccgcgcgcgcctcgcctcgcaattgggcaaggacggcatcgccatcgtgccgaccgcgcccgagcggcagcgcaaccgcgacaccgatttcctgttccggcacgacagctacttctattacctgaccggctttaccgagcccaacgcctggctggtgctggcgggcgacggccgcgccacgctgttctgcgcgcccaaggacctggagcgcgagatctgggacggataccgcctgggccccgacgccgcccccgcagcgcttggcgtgaacgagggcttctcgatcaacgacctcgacgccaagctgccgaagctgctcgagaacaggtcgaccgtgtggtttccgttcgcgattcacaagggcctggaaacccgcatcgacggctggctgcaatcggtgcgcgcgcgcgtgcgctacggcgcgctgtgccccgaagagcagcgcgacctgtgcgggccgctcgatgaaatgcgcctggtcaaggacgcgcacgagcaggacatcatgcggcgcgccgcacagatcagcgcgcgcgcccacatccgcgcgatgcagttgtcggcccgcatgctgcgcgaaggcaaggacgtgcgcgagtaccacctcgacgccgagctgctgcacgagttccgcctgggcggctcgcagtgcccggcctacggctccatcgtggcggcaggcgccaatgcctgcgtgctgcactaccgcgcggacgcggcgccggtgcgaagcggcgagttggtgctgatcgacgcaggctgcgagctcgacagctatgcgagcgacatcacgcgcacctttccggccaacggcaagttcagcgggccgcagcgcgcgctgtacgacctggtgctggccagccaggacgcatccgccgcggccaccaaggccggcaaccgcttcaacgatccgcacgatgccgccgtgaaggtgctggcgcagggcatgctggacctgggcctgctcaatgccaacaaggtgggcagcgcggaagacgtgatcgacagccgcgcctacttccagttctacatgcaccgcaccggccactggctcggcatggacgtgcacgactgcggcagctacgtcgagcccacgcaggtgggcgaagtgagcgagcgcaaggatccgctgtcgaacgaagtcatcaagaaccggccgagccgcatcctgcatcccggcatggtgctgacgctggagcccggcatctacgtgcggcctggcgagggcgtgcccgagcagttccacaacatcggcatccgcatcgaggacgacgcgatcgtcactactacgggttgcgagctgatttcgcgcggcgtgccggtgaaggcggacgagatcgaggcgctgatgcgggcgtgatcgcccccgctgcgacgccgatggcatcgcagcggctttattacttcgcctgcagcagcgcgcccgcttccagcagcaccagttcgttgtcgtcggccttgttcggctcgcggctgctggagaacggcaggttgttgtcgttgcccaccacgatgtgcgtggcatccaccacgtcgacgttctcgatggtgaagaacgggaacttgagcacaccgtcgttgagtggcttgcgcgcgagcttggccgggtcgacgatgttcagcagatcgatgtagccgatcttgcgcaccgcagcgcccacgttggcgtcgttcagctccaccttgtagacgcgcttgaacttcgcgatgtcgtggaagcagtcggtgcgcttctggccttcggggcaggccttgtcgctcgtgccttcgccgttgtcgcgctcgatgatcaagccagtggtggcgtcgatcatgttgaagtcgccgatggcgttgccgttggcttcgagcgggtacttccaatggcggcccgtccacttttcagacgccacgtcgaactccagcacgcgcagcgcttccttgccgtccagcttctcgtagtccttcgtctcggcattccacaccgggccttcgagcagcgcgtagagcttgctgccgtccttcgacgaggccatgccttcaaagcccttggagcgcttgacctggaagtcgaccgcaccgcccggcgcgcccggcgtggtgaccgcgggatggtcgggcgagcgcacggccttgccgtcgacctgcgtgtcgaacaccgcgagcaccctgcctttcaggtcggccttgatcaggaaggggccgaactcctcgccgatccacagcgcgccgccggcgaactggaagctctcggggtcgaagtcggagccggtcaggtagcgctgtttcgtgccttcgtgaacgatgcgaaaaggcaccttcttgtcgggatcgtgcaggaagaccgtgtcgagacggttgaacttgccgctcttgaagtccaccttgtagtggttcaggtagagcatgaagtcgggcgaattggccttggcgccggcgccgttgtcggtgaggatccagaacgaaccgtcgtccatcttcttgatgcccgagtggccttgcaggggctggcccttgaagggcagcgaaacgcccgtgccgcggccggccgaaaggccttcgaccgtgcccagcgcctccacgcgcttgcccgaggtgaacttgccgctcgcctgcaagtcggcaggtgcgtccttgggcgcggccacgaagctctgtgcaggcagcacggcgtggccggtgagcgttgcggggaaggcggtctgtgcggcggcactgctgcaggcgagcgcggcggcaagggcaatgaaggagagagaagcgaggcgcgtcatgggcaagaagaaagggttcagtcgaaacgcgagaccatgccgattgcgcgtgacgcggccatgacatgcagccgggtcagggtgcgatgtcgacagtgacctcgcgcgattcggcgcgcccctggtcatcgaccgcgcgcagcacgtagcgccggcccgtctccgcgaggtcgggcatccaggtgatgccctcgccgggtgcggcgcggccgatcagtgcatcgtccgcgaaccagtagatcgtctgcgtgcccgccgccgcttcggcgcgcagcaccagcggctcgggcttcttcacccgcagcgtgtgccgcacgccgcgcaatggcgaggtgatgagcggcgcggtctccgaagacgcgttgcctttctcgcagccatcggccggcaggctcgcgcgcggcagcccggcctggcggaacagtcggcgcatgtcgctgccccattgctcgaccacctgctgccgcgcgttcggctgcgggccgcacaccaccttgccggtcgtttcgtcgacccacaccgcgcgatgcaggttgctgacctggatcggcgacttgccggcgatgaaccacgtggtgctgcgcaccgggcacagcgcatccggcaggccgcccgtcgcggtgcagacctcgacctggcgcaggtccgccggctgccgcgttgcgacctcgccgggatcgagccgctcggcgcgcaatgcgtcgaccatgcgcaggaacaagggggcggccgcgtcgacgcccaccagcgcagggttgctcgttccgtcgaaattgccgacccacaccacgagcacatggcggccgaacacgcccgcggtccatgcatcgcggaagccccaggaggtgcccgtcttccatgcgatggccgggcgagcaggcagggtggtgtcgggccgcggcgtgtggcgcagcatgtcgagcgtgatgaacgaagcctcttcgctcaacaggcgcagcggctgggtcggccgctcgtcgggcgcgggttgcgtgtagcgcagcggctgcgagacgccgccgttggccagcgtggcatagaggcccgcgagctcctcgggcgtgacctcgccgccgcccaggaccagcgccaggccgtagtgcgattcgctctgcagcttcgacacgcccgccaaccgcatgaagtcgtagagccccggcttcgagagcttcgcggccaccgccaccgcggggatgttgcggctgcggatcagcgcctcctgcgcggacaacgggccggcgaagcggtggtcgaagttctccggcgtgtagggcccgaacgatgtcggcgcatccttcagcatcgtcttgggatgcagcaagccctggtcgagcgccagtgcatagatgaagggcttgagcgtggagcccggcgagcgcttggcctgcgtgccgttgacctggcccgcgatggcgtcgttgtgccagtcggccgagccgatcagcgcgcgcacctgcatggtcgaggcatcgagcagcagcgcgctcgcgttggtcattcccacgtcggcatgcgtgcgcaagtactggcccatcacgcgttcgagcgtggcctgcatgcgcaggtcgatggtggtgcgtatctcctgcaccccacgctcctgcgcgagcagcatgtcggtggcgtgcggtgcgagaaagggcaggctgccgcgcgactgcgccgagagcgcgagctgcgcgtcgggcgcgtgctgcttcgcggtcgggtcgcgctcggcccacagcgcccacagccgttcgcgcgccgactgcagctcggcattgcggccgcgctcggcaatgcgcttgacggggttctgcgggatcaccgcgagcgtcagagcttcgggcaggctgagcttggcggcgtccttccgaaagtagatgaggcttgcggcctgcacgccttcgatgttgccgccgtagggggcggtgttgaggtacgcctcgaggatctcgcgcttgctgaagcgcgcctccagccacagcgccgccccgatctgcgcgaccttgcccatggccgtgcggctgtcgatgccgtagatgcgccgtgcaagctgcatcgtgagcgtcgagccgccctgcctgcgctcgccgctggcaatgcgccaggcgctgcgcaccagcgcggcggggttgacgccggggtgtgcgtagaagcgccggtcttcatagagcagcaccgcatcgatcagtgtgggcgagatgcggtcgagcggcacccagaggcggtactgctcatcgcttgcgagcgtgaggcgcaagagctcgccgccttgggcgtacacggcgcgcgagctgccgacggtttcgctgaggggggcgtggggccagaagcgcagcagggcgagcagcaaggcaacagccacgaaggcgaccagggtcttcctccctctccctctgggagagggttggggtgagggcagcggcggtggatcgggcagcgtggtcatggtggcgccgagccctcaccctagccctctcccggagggagaggggacaagaccggggaatgccatggtcaattcgccaccacctggaagcgcgccccggccgagcgcgaatacacgcgccggtcgtacattgcctcgccatacgccgccggcaccacgaagtcgcccacgttggtggcgcgcgccttgtaggtcacttcgagcaggtccttgccgacaccgccatagaacaccacgcggtcttcgcggatgtcggcgtactgcaccttccaggaaccgctgccgcccaggcgcttcttccagatcggcgcgtcggcattggcttcctcgtcgtcgcccacggcctgcagtaccggctcgagcccgccgggcagcacgtcgaccagcgccacgtcgttcagctgcgcgcgctccaggctgcgcacgcgcacccgcaccgtgacctcttcgccgagcttggccttggtgaccgggttgcccttggcatcgagcacttcatggaagatctcgaggccctggttcaccggcgtggcaggcacgttgcgttcaaagccctgttcggcccagctgtagtagaggttgaagtcgctgtcgttcgacagcttgagctttgcggtaccggcgggcaccgccgcgcgcgtgatcgggttcaccgcgcccagcgcgagcgccgcggcctggccttgcgcgttgacggtctgcgccgtgagcttgccctcggcgttctgcgccaccgcttcgaaataggcatcgacggcaagcagcatcgaggccgacgacaggctgttgtaccagccgtcgcgcaccatcgcgcccatgcgctcccacaccgcgggcttgagcgtcttgaggcggctcgggaagtgccgcgccaccaggtgcagcgtcatgctgtcgtgcaccagcgggtcgtagtaggcgccccagacattgcggcgcgtgttcttctcggtgcgcgcgagcaggtcggaccacaccgggccgagcagctcgttggccacctgttcctgcttcacgagctggtagctcgcggccaggtacacggcgccgagatcgtcgctccagccttgggcctgccgcgtctgctgggtacgccaggcttcgcgcaggttggccagtgcggccggcgcgatgatgccctgccgcgtcagcaggtaggccgcctgagtgcgctggcgccagccgtcgagcgaggtgtcgccgctgccgagccagccctgcaggtaggtgttggccttctgcagcaggtcttgcggcacgggcagcttgtggtccttggcttcgaccagcaggtgcaccgcgtagagcgtggcgaaggcatcggtgccggcgccaggccacagcgagaagccgccgtcggccgtctgccgcgcgcgcagctgcacgaggtagcgctcgaaggtcttgcgggcctcgggcatcgggccctgctcggcggtgcggccgcgagccatttccttcaccagctcggggcggccggacagcagcacggccggaaaggtctggctcgtgatctgctcggtgcagccgtgcggataggcttccaggtactgcatgaggccggtggcaaaggcccacggtgcggcagacaccgccacgtcgctcttgcggaagttgggatacaggtcggccttgctcgacagctcgcccgcgcgctggaagctgccggcctgcaccagcgtgacgaacggcgatgcaggccgcacgctcacctcggtcgagagacgcgcgttgaaggtcttgtgcgtggaggtgaacaccagcgccgatgaccccagcaccgcctgctcgcccggcttggcacgcacgttgaacttggtgctggattcgccgcgttcattgaccttgagcgtctgcgtggcgtcgcccaccacctcgagcccgcccgatgcggtgagcgtgagcgcgatgggcgcctccttgcccgaacccgcgatgttgttggcgaggcccacgcccacttcgaccgtgtcgccgggcgccatggcgagcggtgcgttcggcaggatcaccatgtcgccgcgcaccacggtgcgggtgctcttggcggcggtggtctcgtcgttcaccgcgacggccatcacgcgcaggctgccgttgaagctttcgggcacggtgtagctgaactcgcggctgccgttcacgtcgaccagccccgaccagtaggccaccggcttgtcgcgcttgcgcttgaacgggttcaggtgcttgccgagctcgccttcgccgtcaccgccgggtgctgcgccctgcatgagtttcttgaactcgggcaggatcaggtcgagcgtctgcagcgtgccaacctcgagcgcgcgcttctggaagaagtgcttgagcgggtcgggcgtcttgtagcgcgccacctgcaggatgccttcgtccaccgcgaacagcacggcgcgcgtgggcttgtcgctggtgagcttcatcttcacggtctggccgggtttgacgagctcgctgctggtgagctgcaggttggcggtgcgcttggccaggctggtggcgaagggcgcgacgccgtacgacagcgggctcatgtagacctcgtcggaggctggatcgcgcacgaagtgcacgttgacatagccggtgccttcgaactccttgggcagcgtgatcttctgcaccgaagcggtcttgtcggtcttgaaccacgcgtgggcgtagaccttgtcgcgctcgatcgtgatcagcccggcgcccacgtagggcgcgcggatgctgacctcgatctcctggcccggctcgtagtccttgcggtcgagcgtgagttgcagttcggcattgcggtcgagcgagcgcgagacgttcgcgttgcccgccacgctgtactccacgcggttgagttccaggccgccggcgttgcgcaccacgtacgcgaagttgccgggcgtggaggtgttcagcacaacggtgttgccggccgcaacgatcgccagcggcttctcgtcgagcacgatttccttcctgcgcgactcgtaacggtagagcccgctgtcctgcttgacgagcaccgacagcaccttgcgctcgacgcgctcgatcttcaggtcggccacggcggtcttcttcgcctgcgggtcgatcgcgatcacggtggcattgcgcgcggcgcccttgctcacgtagctggtgtcgccgtcgaccttcacgcccacgaggtagggcatgtcgctcaccagcgtctgcgcctcggccgagacgctgcgcccgccctcgggttcgaaggccttggcaagcacgtgcacctggtaggtggcggcatcgaagcgcgagagacgcaggtcgaactcggccttgccctcggtgctggtctgcacgctgcccaggtcgtcgacctgcttctcggtggcgcgctgcggatcgaagaaggcgtagtcggcgaacgcacggaacaccgggaaggccgggctcagcgtgagcgtgccctcgaccttgcgatcgggcgcgggcgtgccgaagaggttctgcacatcgatcagcgccttcaggtccttgggcttgacccagccctcggcgagctcgctgctgagcttggcgacgaccttggtgcggtcgggcagaaactcctgcaccttcaccgtggtgctgccgatgagcaggccctgcacctcggggttgccgggcgaggactcgcgcggcaggtagaggttgacggtgtagttgccggtgggcgacgtgtcctgcgtggcgtgggcgatttccgccgcgccgccggggccgagcttgagcttttcgcgccgcacgctgaggccgcgcgcgtcgatgatctcggcttcgagcggcagatcgcgcagcgacgtgccccagttgccggccttgaccatcatggcgatgtgcatggtgtcgcccgggcggtagatgccgcggtcgctgaacacataggccgtcatctggttgggcacgccggccgcgcgcaggccgccgacgtcgaagcgcgagatgtcgagcgtgcggtcgctgcggttgaagggcaggaagctcaggtcgccgtccttgcgcaccaccagtaccacgggtgccttctcgcgctggtagccggcgaggttgggcagcttggcggtgccggtggcgccggtcgcctgcgacgcgatgatcatgccgttgcggccccacacctcgaccagcgcaccggccacgggctggccattggcaatgctctgcacgaacacgtcccgcgtgccgtcgagcgacttcttgacgacgatgcccaggtcggtgacgagcaccaggcgctggtccttctggtcttcggggttgccgctttcggggtcgctctcgccctcggacgactgttcctgttgctcttcttccggctgcgcctgcgcggcgtcgccttcggccttcttcttggccttcgggtcgtagccctgcaccttgagcaggaacacgccgcggcgatccgccacgtcgctgcgcaggtactcggcgaagtcgacggtttcgtagtgcgccttgccggcgggaatgctgagcggaatctccttctggaaacggtcgacgaggttgtccgactgcaggccgccgttgaattgcggatgcgcgaaatcgccgttggtctgggtgaccaggtgctgcagctgctgcggcagcaggcggccgatttccaggcggatgcccggcaggtcgcgcaccaggatcggcagtttgcgctcgcccgacagcgcgagcagcgagccctggctcatgatggtgagctcgggcgcgaaggtcttgagcagttgaatctcctgccgcgcggcgccgagctggtagccgcccggcgtcttgaggcccttggccacgcgcaccagcaggtagcggccgccttcggcctgtggcatgcggaagctgaccatctcggtcacttcgcgttcactcgcgatgggctgcaaggcgagcttcttcgcgcggcgcagcacggcatcggtgatcttcgagggctcggcggaccagtcgaacttctcgtccgggtcgcccttggcttcttccgtggcgggcagcagccaggcctgcaccacgcgtgccatctcgcgctcgtgcaccggcatcgacgcggtgatgtgcatcacatgctcgggttcgccgctctcgccggtgacgatggtgggctcgacgcttgcaatgtcgaggctgaagagtccggggatgtcgacggcgcgcgagacgtcgttgcgctggccggggccgcccttctgtgcgaccgcgccggccgcaaggctgagcaccacgggacgcgtcttctcggggatgggcagcggctcggactgcagggtagcagcgaggcgcagcttgtcgtagctgaccgtgaacttctcgccggtgcatttgcccacgccgaagaacgaggtgccgcaggcctggtcataggtgagcaccagtcgcttctcgaactcggccgtgttcacgggatgcgagaaactcacgcggaagagggcgcggcgcacgttcgcctgcacggggtcctgatagaactcggcgcccgcgatgcgcgcgctgaactcgggcgaggtgaactcgtacttgcgcagtgccatctcgatgtgcggcgccagcgcgctgttcgcaagctgcaccttgtacggctggcccaccggccagtcctgcgccggcaggaactccagtttcttctggctgctccacgtccagcgcccggcaatggcgggctcgatggtgataccggtcgcctcctggccgatgcgcgcaatcggcgcgaccgaggccgagaagttgataacgagcgggttcggtcccttgtcgttctcgatctgcgtgcgcggcggcggcacgatctgcgcggtggcgaccacgggttcgacgcggtcgggcgtgaggccgtgccaccatttcaggacgtgcgggcttgccatccagccggccagcacgagcagtgcaagcaccaccagccaggccagccgttgctgcagccactgcagtccgaagagaagaaacgcacccacgatgcgcagccagcccggaggtcgccaggaaccgatgagtccgcgcgtgagcggacgcagaaagccgagcgcgcggcccagcccggtgaagagcacgtcgctgagcgacgcgagttttcgattcgcaacctgaagcatggaagctcccccgatgtttttgttggcgcctggcagtctgccggcgatctgtgaagagacggcgctgtgtgtgaagtctgcgtgaaaaccgcacaggcccgcgctggggccacttcagtgatggatggtgcgttgtgcgttgggttgctgttgttcagggcgctgttgttcagggcgcgtgcgcaggccaccgggtactcccctccgcgaatgtcccccgccttcggctcctcctttatttcgctgcggggagcacccggcgccctgggcacaccgggcgctgtcgttgttccgctcgatcaacaaccgctctgcccaacgatcccgtcgatggggtgccttgcgcagcgaaataaaggaggaggccgcaggccgggggacattcgcggagcaaggtaccccgtcggcgggagcgcgccctgaacaacctgcttcaaacaaagttctcatctcagaatgaaagttgcggcttattcaccatcagccagaacacgacgaccatggccgcaggcgtcatgaaatggccgatgcctcgtcgatcacatcggtcaccatgccccagcgcgcgaactcgggctcgaactccgcaagcgtgggcaagccggcgcaggcgtgcgcgccgatgggcaacgcatcgcctcgtgcgagacggcgggccagcaggatggcggccatgcagggaatctcggggccgtggttgtcgtcggcggcaatgtgccaggcgcggcgcgcttccatgccgcgcgcatcgatgccttcgacgcgcaccaccatgccgcccagcgccgtgccgaaggcatcgaacacgcggcccgccgaatgcagcagcggcgcaagccttgcgggcgacggcagcaggccgatgcggcgcatgaatgccatgaaggcaaacgcatgctgcgccaggccaacctcgagcgccgcacgaaacatgacgaattgcacgccggcatagcgcgccggaaaaagctcgagatcggggatgtcgcacagcgcaccgcggcgcggtttcatgcgcgcgaaccgcactgcggtggggttggcccatcctggttggtcggtccatcctccgtcgcgccagacccggatcggctcgccgcagtaggccagcacgcccgcaagcgtggcttcgccgcgcggcgcgccttgggccggcgcaatgcaggtgtcgatgcttcggacgccgcgccatcctgcggtgagatggtcgaccaccgccgacgacagtgccggcacggtgctggcgccggcaacggccgtgcggcccgcgctgcgaaaggccgcgtcgagcgcagcgggaaagtcgcagacgaagcgccgcccgtcggccaggtcgatgtaatgcgcgccggctgccgccacagcatgcggcacgcgatagtcctggttctggaaagggcccgcggtgtggatgacgagttcgacgccgaggccgcgcaggttttcgacaaggtcgccggcctggacgtcgatgcgcacgccgcgcgccgcaccgcccagcgactgcgcgaaaacggtggcgcgctgcagatcgcggccgccgatcatcagttcgatgccggcatcccgtgccaacgcgcggcagatgcgcgcgccgaagttgccgtagccgccgagcaccaggattttcatgagacgcccatgcccgcgacgtggccgcgcgtgaaggcttcttcgaagatcgaatagccggaccagtccgcatgtgcgaacgagagacggccggcggcaacgcggccgcggtgcgccgggtcgggcgcggcgccgatccgcgccagcaggcccggcgcgggaatggccatggcgtggccatagcgggtgatctcgatgcgcgtggccagcgccggcaggtcggggtgcggcaccgagagctcggcgagcaggtcgtcgcgccatccggtccaggggcggtcctgcagcaggcggcggccgtcagcggcgtcgtagcggctcgggccgagcgggcggtaccagctgatgacggtgccgcgtggcgtggggtcgagcgcctggtggcgcgcatcgacgtaccccagtccgcgtgtgccatacacgacgttgtcccagctcgatgctgcgccggggcggtcggcgaacggtccgctcaggtgcacgttggcgaccagccagggcgcatagcgcaggtgcgcggcggcgtttttcaaaacctccggcgcgttctcgaccacgcgcgctgcgatgaacaccggcagcgcgacgatgcaacgctctgctttccagcgcaccagcgatttcgtttcggcgtcccacgcgtcgacctcgacaccggcgcgcagatcggcaatgcgcgtgacgacttgccccgtgtgcagccggtcgccgagcggctcggccatgcgcttcgtgagccagccgttgccttcgggccaggtgagcacaccatcgcgctcggggttcgaatcggcgccgctgcccgatgaacccggggcgtgaaatccgtgccggcttgcgaagtagtggatgccggcccaggccgaaacttgctcgatgccagcgccgtagtcatcgcggcagcagtagtcgaggtaccagcgcagctgcggatcgctgaagccttcgctgtcgagccagcgctcgaacggaagggcgtcgagcacgagcaactcgggcgtcgcggctaccttgagcgtgggaatggcgaagtgcgccgcatgctgcagcgcgtcgatccgctgcgcgaacttgcggtactgcgcatgggtgctttcgccgacgtcgtgcacgggcaggaggccgtcctgccactcgccgcgaaagaacaggcgctcctgcgggctgtggcaaaggttgcgctcgtcgtattcccagcggcccgccacgcggcggcgcaggccgagttcctccagcaggtcttgcacttcgcgcgcgtcgtcgttgggcacgggcaggtagtgcgccccgagcggacaggcaatgccgttgacgataccgccgcgcgcgttgccgccgggcgtgtcttcgagttcgagcagggcgaaatcctcgatgcccgaaaggcgcagtgcgcgcgcagcggcaagaccggctacgccgcctccggcgatcaccacgcgcgtgcgcttcaaggctacgggcacctggctcttgagcgcgccatcgcgcatcgcatggccgcgtgccacgtcgatgccggtaaagccgccttcgatggggggcagcgaagcctcgcagccggcgagcgcaagagcgcccgccgcacccgctacgccgaggaaattgcgcctttgcatggcgacgctagtgcgcaaccactttgccccactcctgctcataagtggtgacgagggtctggttcgagaggcggttcacttccgccggcacgcgcgccatgtcgagcggaaagtcgaacatcagcggcaacgtcgacggcgcgaggaaacgcaggcccgagggcagcgcatcgggcatgcgatagggcctgcggctcgcgatgatgtagccccattcgccgaagctcggcacatgcgcgtggtacggcgtgaccctcaggccgaccgattcgatggtggtcgccacggtccagtagctcttgcgcgccaccagcggcgaggtggtctggatcgccgcgtagccgcttgcagaaaggcgcttttcgagcagcgaatagaagctgttggtgtagagcttgccgatcgcgaaattggtgggatcggggaagtccaccacgatgacgtcgaacatatctcctggttgctgcagccactggaaggcatctgtattgacaactttcaccttcggcgaagacagcgaatgcccgttgagcgcggccagcgtttcgtgttcggtgaagagcttcgtcatgttcggatcgagctccaccagcgtgatcgactcgaccgacgggtacttgagaatctcgcgcacggccatgccgtcgccgccgccgagcaccgccactttcttcggcgcgccctgcgcggccatgaccggatgaaccagcgcctcgtggtagcggtattcgtcgcgctcggcgaactgcaggttgccgttcagaaagaggcgatggccgagctgcccgcgcgtgaccacgatgcgctggtagggcgaggtggcgctgaagacgatgcggtcctggtagaacttgtcttcggccagcgtggtgatgtgatcggcccacacaaaagcaccaagcagcgcggccagcgcaagaaagcatgcgaacgcgtgggcgccgatgcggcgcagctcatgccgaaacagccacagcgcccacaccgccacggccgcgttcatgaagccgaacaagagcccggtgcggatcatgccgagttgcggcacaagaatgagcggaaaggccaccgacaccgcaagcgcgccaagatagtcgaaggtgaggacctgcgacaccaggttcttgagctggatgttgcgcttgaggatgcgcatcaccagcggaatctcgagccccaccagcgtgccgaccaccagcacgagcccgtagagcagcagccggaacgcgccgggcacgtaggcattcgcgagaaagagaatggccggcagggcaccgccgacgagcgccacgagcagctcgatgcgcaggaagtgcgccggaagctggcgctcgaagtagcgcgagagccaggagcccacgcccatggcgaacaggtaggtgccgatgatggtgctgaactgcagcaccgaatcgccgagcaggtaggagctcagcgcggccgcggtcagctcgtagaccaggccgcaggcggccaccacgaacacactggcgagcagcgcgatctcgacgggctgcggcccgcgcgcatcggcggaatgcgcggacacggccgcctccccgctcaatggatcgcggctgcgacgatgacgcagatgcccaggctcatggcggccacgaccagcccgagcgccacgttctgcttctcgacgatctcgccccacaggtcatagggcgtgagcttgtcgatgatgaggaagcagagccagaagatcagcacgccaagcagcgcatacacgagcgatccgaggaccacgcccggtttcagccattcaaatcccatggggacctccagtcgtagtagcagtattagatgacatcaatgcgaagccgcctgtttttcatttgtggccgccgccgctcgagtagccgccgtacgatccgcccgagctgcgcgatccactggacgagctgctgcaggtgctcaggatgaccagcagcacgatgatgatgaccacgatgaagatgatggtgccgcaacccaggcccgaggcggcactgaccggcgatgcatcgccgcgcacgaacatgtctttcttgtcgtcgagcttgaacgccgcggacaccacgccgctgtcgagcttgccgcccgaggaccaggtcagctcgttggccgagcgctccatcgagagcagcgcattgccgttggcgaagtcgcggttgaaggttttctgcccgcgctccacctgccagtagaactcgcccgccacgtaggtggtctcggcgttgtaggcgtactgctgggtgtagcgcttgccgagataagtggcgctgctgccgttctccgccatcaccggcgcgccggtggtcggcttgaccatgctccagccgtcttcggcatcgaccaggaagctgaagccgcgcttcttgttgtacagcaggtactcgttccagccgaagtgctcgtcgtcgccgggctctgcgcccatgcggtgctgaaagcccaccacctgccattgcgcgccctgcagctggcccatgctgccgatggcgatgagcgggcgaacgggttcgttctgctccgcgtgcttcagctcgccgccaatgccttgcgacaggtcgatgatgctgttgcacgagccgcaggtgatgctcttgctgtcggccaggttgaccgtgatgggcgcgccgcaatgggggcagttgaaggcgcggcctttttcgtccttggcggattcgtcgcgcaggcccgtgagctgcagatcttccagctgcacggaacggcccaggtacgcgctcggcggctccgtgccgtagtcgatgctgagcaccaggcccttgtcgctgcgcagctcgaccatgggaaaggcgcggcccagctcgggcaggtgcggcagttcgccctgggcggaaagcagcgccacctgttcgttcgacgaaacggtgtagctctggccgttgaacgcggtggtggcgcccacgcgcagctcggccggcggtggcgcggcgcgctgcagctcgaatggcagcgcgaagacataggcgccgttgtcctcgctgaggatgccggtgcggtcgccgtcgagcgcggcgatccattcggtccagcgcccgcccgggttgctgtattgcagccggccgacgatggtgaacggctggttctggatgcggccggcggcaaacagctgcagcgggctgaagtcgtcgaacagctcggccatcttgccgatgcgcgcgagcgtctcgccctggcggacgacggtgctctggcaatacgggcaaacggcaaaggccgattgtgcggacctgaattcgaccggcgcgccgcagccagggcagggcgcgcgataggcgcgctcggcgcctggttgctcagccatcgccggtgcttagaccagcttcttgagcagctccgccttcttggcgtcgaactcttcctgcgtgaggatgcccttggtcttgagctcgccgagcttctcgagcgtggtcatcacgtcggccgggctcaccaccgccacggccggctgctgctgggtcgccgcggcctgggccgctgcgctcgggctcaggccctgcgcgaggttctgcgccagcacctggccgagcgccacgccggcgcccaggcccatggcatcgccggcaatgccgctgccgccgcccgcgccttcggcgaacttgggaatggcctgcgctgtctggtactgcatgaacttgcccatgtcgttgccgaccatgcccatgccgatcttctggtcgaggatcttctgcagctcttcgggcagcgagacattctggaccgtgatgttctcgagcttgatgccgatcttctcgaactcgggcaccagctgcgccgcaagcgcctgcgcaaactggatctgattggccgcaaggtcgaggaagggcacgccgctggaagcgatggcgttgctgatgttctgcagcaccaggccgcgcagctggccgtcgagatcggccacgctgtagatgtcgcgcgtgccggaaatttcggtgtggaagcgcttggcatcgccgatgcggaagctgtagttgccgaaggcgcgcaggcgaaccgcgccaaagtccttgtcgcggatggtgatgggctgcggcgtgccccacttctggtcgacctgctggcgggtgctgaagaagtagacgtcgctcttgaacggagactcgaagagcttgtcccagttcttcaggtacgtgagcacgggcagcgtctgcgtcgtgagcttgtacatgccggggccgaacacgtcggccacctggccttcgttgacgaacaccgccacctgcgactcgcgcacggtgagcgaggcgccgttctggatttccatctcggccatcgggaaccgccaggccagcgtgccgtcgccagtctcggtccactggatgatgtcgatgaactgtttcttgatgaaatccatcagggccatggccgctcctcgtctatttttttccggaacgtacatattgccacatcgtcttgacgggccgtcgtgcttttggcaggggcggatctccgccatgcggcctatggcgcccttggccgaggtctacaatcggcgcccccagaagaagcgccaccaggagcaacggcccatgtctgattcgacgacctcatcgacccccacgcccgaagacaagcgcgccgaactgcggcgcgccgccctcgagtaccacgagtttccggtgccgggcaagattgccatcgccgcaaccaagcagatggtcaaccagcgcgacctgtcgctggcctattcgcccggcgtggccgcgccctgcgaggaaatcgtcaaggatccggccaacgccttcaagtacacggcgcggggcaacctggtggcggtgatcaccaacggcaccgccgtgctcggcctgggcgacatcggcccgctggccgccaagccggtgatggagggcaagggcgtgctgttcaagaagttcgccggcgtcgacgtgttcgacatcgagatcgacgagaaggacccggccaggctggtcgaggtgatcgccgcgctggagccgaccttcggcgccatcaacctcgaggacatcaaggcccccgactgcttctacgtcgagcgcgagctgcgcaagcgcatgaagatcccggtgttccacgacgaccagcacggcacggccatcaccgtggcggccgccatgctcaatggcctcaaggtggcgggcaaggacatcggcgaggtcaagctggtcacctcgggcgcgggcgccgcggcgctggcctgcctgaacctgctgctcaaggtgggcctgaagcgcgaaaacgtcttcgtgaccgacctggccggggtggtctacgaaggccgtgaagagctcatggacgacgacaagcgccagtacatgcagccaaccacggcccgcacgctggccgaggtgatcgagggtgccgacgtgttcctgggcctgtcggccggcggcgtgctcaagcccgccatggtggccaagatggcgccccgcccggtgatcttcgcgctggccaatccgaacccggaaatcgcccccgaagacgcccacgcggtgcgccccgacgtgatcatggccacgggccgcaccgactacccgaaccaggtcaacaacgtcctgtgcttcccgtacatcttccgcggcgcgctcgattcgggagccaccacgatcaccgacgagatggaaattgccgcggtgcgcgcgattgccgatcttgcccaggccgagcagagcgagcgcgttgctgccgcctacgtcggcgaaaagctgtctttcggccccgaatacctgattccgaagcccttcgatccgcgtttgatgatgaagatcgcgcccgcggtggccaaggccgccgaggaaagcggcgtggcctcgcgccccatcaaggacatggacgcctaccgcgaccgcctgcagagcttcgtctacgcctcgggcaccacgatgaagccgatcttcgacgccgccaagcgggcgcagaagaagcgcgtggcgtattgcgagggcgaagaagaacgcgtgctgcgcgccgcccagatcgtggtcgacgaaggcattgcccgcccgacgctgatcggccgcccggccatcatcgcgcagcgcatcgagaaattcggcctgcggctgaaggaagagctcgactacgacatcgtcaacgtcgagcaggaccaccgctaccgcgatttctggcagacctaccaccgcatgacggagcgcaagggccagacggtgcagaccgccaagatcgagatgcgccgccgcctgacgctgatcggcgccatgctgctgcacaaggacgaggtcgacggcatgatctgcggcacctggggcaccacactgatccacctgcactacatcgaccaggtgatcggcaagcgccccggcggctgcgagagcaccccgcaggacgtgccggtgtacgcctgcatgaacggccttttgctgcccgaccgccaagtgttcctggtcgacacgcacgtcaactacgacccctcgcccgaggaactggccgaaatcacgaccatggcggccgaggaaatgatgcgcttcggcctgaagcccaaggccgcgctgctgtcgcactccaacttcggcaccagcaacgagcccagcgcgatcaagatgcgcaagacgctggacctgctgcgcgttcaggcgccctggctcgaggtggacggcgaaatgcacggcgacgtggcgctcgacagcaagcagcgggcggtcgtcatgccgcacagcgcgctcgcgggcaatgccaatctgctggtattcccgaacatcgacgcagccaatatttcctacaacctgcttaaaactgcggcaggcggaaatatcgcgatcggcccggtgctgctcggcgcggccaaacctgtgcatattctcacggccagcgcaactgttcggcgcatcgtgaacatgacagccttgacagtcgctgacgcaaacgctgagcgataagcgatttttcgagagtggccgcccactttaggtgccactctccgtcccatgcactgctcaaactttgggcagtcgcttgctattttcgtcagcgtggtgcacactcgcgggcttgaatttgcgggttaaccccagggttgatcgccaattcggaaccccgctcttttcttgtggtgccccatggcggcttacgcctcgatcacgtcctcagtcactaagtttgcgctcaccggctttttgctggcggcgttggcgaccggggccgaggcccgccgcgattggtttggcaccggaaagcccgcccaggattcgattgcactgtccgaactgccggcacagggccggcgaacctacgaagccattttgagtggcggccccttccaatatgaaaaggacggcacggtatttggcaatcgcgagcgtctcctgccgccagcgcggcgcggtcattaccgcgagtacacggtggcaacgcctggctcgcgcgatcgcggggcgcggcgcattgtctgcggcggtgaacagcgcacgacacccgaggcctgctggtacacggcagaccactacgcgagtttcagacggattgcaccatgagcgatgacaacgacttgagcggcgccccgaagcgccccgaagaaatgatgatgactatggaaagaccagcggagatgacactatcccttcgtgccgtacgcccgaacatcgtgcagtcgattcgtgcgttccgcgtgaacgacctgcaggaagccgcgaacgccgcgggccagcatttcctgtacgccaacctgggcaacgcccagaccaagcaggacgttctcgacctgattgcccagcagttcacctttccggcgcacttcggcaagaattttgacgcgctgtacgactgcatgaccgacccgttgcataaatcgggcccgcagcccggctttgtcatcgtgctcgagcagatcccggccaacgccaagttcgacaaggaagcgcgcgagcaactgctcgacatcttccgcgacgcctccgattactggggggaccggaaagtcccgttccggtgcttctattcttttctgtagcccgttctgcacacaccagccaagcagaacgggcgaacgaggctcagccgaacggcgcagcactcgatggcatcgaaatcaacggcaataccgcaaccgcagcagccggcacggagccggaaggcgaaaaaatgccgaccgataaactggtcgacgtttcgccgctcgcattgcgcatgagcagccccttcaatgcgggatactggctggcggcagcgtaaagctctcgccccaggcgcaagaaaaaagcccgtttcgacgggcttttttattagggctcggggggaaccgcctgggccagggcgacgtattcggccacgggtacttcctcggcccggcgctgggcatcgaattggccagtgaagccatgctcgtcgagccacttgcccagggtatggcgcatgatcttgcggcgctggctgaaggcgacctgcacgatttcgccgaggcgggctgcatcgacggccggcggctgggccagcggcaccatccggaccaccgcgctgtcgacacgcggcgggggatcgaagctctcgggcggcacgaacagcacgttttccatttcgtagcgccattgcagcatcacgctcaggcggctgtagtcggacgtggcgggccgggcgaccatgcggtcgatcacttccttctgcagcatgaaatgctggtcggcaatcaggtgcgcaaaacccagcagatggaacaggatgggcgtggagatgttgtagggcaggttgccgaccacccgcagcggggccggaaatttggcggcgagctcggcgaagtcgaccttgagcacgtcggactcgatgacgtcgagctgcggatgatcgcgcagccgcttggccaggtcgcggtcgagttcgatgaccgtcaggcgcccaagccgctccaccaggggctgcgtgagcgccgccagcccgggaccgatctcgaccatggcgtcgccaggctgcggcgcgatctcgtgcacgatcgcatcgatgatgcccccgtcggacaggaagtgctgcccgaaccgtttcctggcgatatgggccatcaggactggggcggctcgcggtattcgacgtaggcgcgcgcgcgcacttcctgcacccaggtggtgaaggcctcttcgacccgctgctcgcgcagcacggcgcgcgcggcttcgcgctgctcagcctgggtgagcttggattcgcgccggccgaccacctggatcaggtggacgccgaagcgcgacaccacggggtcgctgatctggcccgccgcgagccggtccatggcttcctcgaactcgggcacgaactggcccggacgcgaccagcccaggtcgccgccctccttggcgctcgcgtcttgcgagttgtcgcgcgcaaggccggcgaaatcggccgtgccggcctgcacgcggcgcttgaattcggccagctgcgccacggcctgggcggtggtgcgcttgggatcgttgagcagcaggatgtggcgcacctgcgtctgcgtgacggtggcatcggtggcgccaagctgcgacttggccagcaccttcagcacgtggaaaccggcgcccgagcgaatgggccctgcaatgccgttgaccgccgtggattgcgtcgcttcgacgaacagcgagggatagcggtctgcagtgcgcatgccgactgcgccgccattggcgcggtcgggcgagtcggagttttcctgcaccagcttggcaaagtcttcgccggaacgggcgcgctgcgccaggctttgagcccgttgctgcaaggtggccacctgcgcgggggttgcgttctcgggcacggcgaccagcaggtgcgcgaggttgatgttctgcagcgccgcgtccttggtgggggaatttcgctggtcgcgcaggtattcgtcggcttcggagtcgctgatcttgaccttcgattcgacctcgcggtcgcgcaggcgcgtgagcagcagctggtcgcgcaggtcgttgcggaattcacgtggcgagatgccttcggccaccacgcggcggcgcagctcttcgaccgtgacctggttctgccgcgccacggtctgctcggcctggtcgatggccacgtcgtccaccttgatgccgttttccttggccagctggagctgggcgcgctcggagatcaggcgctcgagcaccaggcgggtgagctcagcgcggggaacacgctcggcctcggcgttttcgcggatcagccgcgtgacgcgcgtctgcacctcggtgttggtgatgggttcggagttgaccagcgcgacgatgtactcagccgagcgctgcaccggcgcggccgaaggcgcggggcgtgctaccggggccgcaaggcgcgggccggcacgcatgatgtccgtgatgccgccgccgccaccggggcgcaggccttgcgcgccggaggatgcggccagcgccgcgaggcagcccaaggtaaggatggaacggatgtgtttcatggcgttgctcaatcgtctcagtcgtaattggtgaagcggctcggcccttcggtgggctggcgaagaggctggtagcgctggatgttttgccgcagggcctgcatgggactcgatccgatgctggaaaatccgacgaattcgagctggaacatgatgcgggtgttggccgtcacctggccggtggtgacacgctgcagcaccacgcgtccgatccagcagcagccgtcgtactcgaagccgagcacgccgtccgtgagtttcttgtcctgcaggctgtagttgagccggccgaccgcgtaccaccgtccgcccccctggcccttgcccgggccgaggtccttgcccttgtcgccccacaggtcgttgagcggccactgccagcccacgtcgaacgacttgttgccgtcggtggcggtcggggtggtgggcgcctggtagcggaaggccgcactcaggttgtggtacggctcggggttgtagcgcgcgctgatggccgagcgctccgacttgcgcgtgtcggggttgtactggaccaccgtgtccaggctccacttgggcgtccagttgatctgcgcgcccagcagcaggtcgctcgcgcggtcggtcaccggcgtgccgcccggcagcgtgaccttctggtcgctgaagcgcagccgctgcgcaatgccgaagcgcgccgcctcgacgccggttgcggggtcgatcagtcgggaggtcacgcccagcgtgagcgtgttggtgtcggagatgcggtcgttgcccgagaaggcgttctcggtgtagatggtcgcaaagctgaaatcgttggcggccgaatcgtagttcggcagcatgctctggttgcggtacggcgtgtagacgtagtacgcgcgcggctccagcgtctggcggaaggcgcggccgaagtagctcgcgtcgcgctcgaagatcaagccgctgtcgaggctgaaggtcggcaccgtccggttgctcgaggtcgggaagaagtacagcgaattcgcgttgtagggcacgccattgacatatgtgatgccattgacggtgagcttcggaatgtccgactgcggcaggtagtagttgtacgacgccgtattcagctgcagcttgggaatgacgaaggaactcggcgtgatgaacggccggctgatcgtgccgatcgccaaggcgcgatcgccgtcgggctgcgactgctggttgatgtcgaagccaggctggccggccaggatggagttgacgcggaagcgcgtgtagtcgaggttcagcgaaacgtcgaagccgtgccagtcgtacttgttgtagttggccgtgatttgcggcatccggtcataggacggcacgatcggcgacaagttgtattgcagcgtctggtagcgcagcgcacgaatcccgccgctccagtcgcccttgccccagttgagcgccgcttcgttcggcagctggcgctgcgccaaggtgggcgtgcgcgtgaagtcgcgccagtagtcgtcgtcgctgacccggttgatgttgatgttggccgacagcgaatcgagccccagcgccttggcgttgaagtcctggtggtggttggcccagatgccccatcgcttgctgctgttgggcgcagcggtcaggtccttggcctggatttctccgttggccagttgctggagctgggtggcgcgcagctcgttgtagcgctgtcctaccaggcggtcgctgcccatcaggtccaggcggatgctgccgctgtagtctttctcgagatagcggaattccgagcccaggttgaggccccgcttgctcatcagcgttggcgtgaaagtggcgtcgcggttgggtgcgatgttccagtagtacggctgcgagatctccatgccgttggtgttgtcgaggccgatcgtgggcggcagcaggccgctcttgcgctggttcgacagcggaaagctcacgctcggaagcggcggcgtgctgatgcccatgaaactcagccgcgcatcggtggccacgcccacgttttcctcggtgtcggtggtcatcgtggctgcggtcagcagccaggccggcatccagcccggaaaatcttcgcggcgacaggtggtgtaggtggcattgcgggccaccgatatgttgctgtcgacgaaatcgatgcgctgcgcctcgccgtgcccgccgttgacgaggaaggagtagcgcacgttgttgaaaaagccctcgaaagtctcgagcttgagttcgagttcggggccttcgtacacattgccggcctggttgacccgcacgttgccgcgcgccttggcgcggtcgtcgggctggtagtactcgagccggtcggcggtgatggcgacctcgccgcgccgcagcgtcgcatggccttcgaccacggtttcgagatcctggcggcccgacagccggtcgccggtgatgaggctcggcagttggctgcgttcattcggcggcagcgtttcggtcagttgcggcgtgcgcttgagcgtgagcggaccgtcgaggccgcccgccggctgtgcggacgcgccgtgcgcatgcagcagcgccagcgacaacacggccaatggcaggggcgggccggaacgccgcaaggcaacgcgtcggctcatcaagccacccgccagggcattccggagaaggcccgcagtctcccctggaagggctgcgagtgcacaaggtgccaagcgtggaggctttggatcgtaggcatcggtcaggaacgaaggatcgtcgggaggacggcgcggcaggccggcaggttgcaggagccggcggcagccctgttcgaccggggaggaccgcaggagttgccgcgccaggcggatttgtagaatcgattatccatgacagcacccccgctcccggcttccgagcctaccccctccgccgaggccattccctggaccgatccgcagcgcgccgcgaccttccggcactggctggccggcatctccgccacgcaccgcctgctgcccgaaaccgtgcgccttgcgtccgccgacgcgagctttcggcgctacttccgggtcgacggtgcggaggattgcggcacccgcatcgtgatggacgcgccgccggacaaggaaaacagcgagcccttcgtgcaggtcgcccgcctgatggccgaagccggggtgaccgcgccgcaggtgctcgaatgggaccgggtgaacggcttcctgctgctcgacgacctgggccgcgagaccatgctcgacgtggtcgatccggcccggcccgacgcgagccgtccgctctatgaccaggccatcgacgcgctgatccgctggcagctggcgtccaggccgggcgtgctgccgccctacgaccgtgcgctgctcgagcgcgaactggcgctttttcccgagtggtacatcggccgccaccgcggcattgccgtcgagggcaagctcaaggagcggctggagcgcagcttcaagctcatcgtcgagagcaacctggcctccgcaagtgtctacgtgcaccgcgatttcatgccacgcaatctgatggtccgcgatggagcggatctgggcgtgctcgacttccaggacgcggtctacggtccgatcacctatgacatcgccagcctgatgcgcgatgccttcctgagctgggacgaggagttcgtgctcgacgtcacgatccgctactgggaggccgcccgcaaggccgggctgccggtcgacgccgatttcggcgctttctaccgctcggtcgagtggatggggctgcagcgccacctcaaggtcgccggcatcttcgcccgcctgaccctgcgggacggcaagcctcgctacctggccgacacgccccgattcatcgcttacatccgctccacggccagccgctacatggaactgacgccgctgctgcgcgtgatcgacgaaatcgaaggcagctcggcgctcaccggcttcgtctacggtcggccctagatgccgcgtttccattgcccggtgccgctgattgcgggtgccacgttcgaactgccccccggcgcggcgcgccacgtgcaggtgctgcggatgcaacccggcgacgcgctcacgctgttcgacggctcgggcggcgaatacgcggccacggtcgaacgcatggggcgcagcgacgtttcggtgacgcttggcgttcacgcggccacagagcgcgaagcagggcgcgcggtgcatctcgcggtcggcatgcccgccaacgagcgcatggactggctggtcgagaaagccaccgaactgggtgttgcaagcatccagccactggcaacggcccatggcgtgctgcgcctctcgggcgagcgcgccgaaaagaaaagggcgcattgggaggcgattgccattgcggcctgcgagcaatgcggccgcaaccgcgtgccggtgatccatccggtgcggccgttctcgagcccgtcggcctgggccgatgcgaacagcggcgccgccgcgctgcgccttgtcctgagcctcgccgaaggcacgcggggcgtggccgatgccacggcatcggcaccgggcgaccgcagcgtgctggtgctgagcggccccgaaggcggcctgagcggcgccgaggaaaaagaggccctggcgtgcggctttgcgccggtcactctcggaccgcgcgtgctgcgcgccgagacggcggcgctcgcggcattggtgtcgctcgccggcccctgattgtgttcccgtgaggcgagcgtgcctcacccattcgtcatgacagacagaaagaaggatcttcacgccatgcttcgttcaccgcgcgccctccggcttgctccccttgcgccccttgttctggccatgttctgcgccgtgcagggcgcccaagcccagaacaccgccgttgcgcccacgcccgcgcaggtcggccccgaggtggaaaaaacctttacccagctgatggcggcgcccacggtccagaagctgctcgatgcggtcaaggccgaccatgaccgcgcggtcgaagacctcaagatgctcaccgagatcgaggccccgccgttcaaggagcagaagcgcgccgaagccttccttgcgcgcatgaaggcactgggccttgccgatgcgaagatcgacgccgaaggcaacgtggtcggcctgcgcaagggcacgggcaacgggcccaagctgctgatctcggcccacctggacaccgtgtttcccgccggcaccgacgtgaaggtgaaggagcacgacggcaagctgcatgcgcccggcatagcggacgacacgcgcggcctctcggtgctgctgtcgtggctcaaggtgctcaacgacaacaaggtgcagacggtgggcgacctgctgttcgtcgccaatgtcggcgaggaagagctgggcaacctgcgcggcatgaaggccatctttcgcgaccacctggatatcgacggcatggtggggctggagccttcgcccgacggcaacgtgctgatcctcggcaccgcgagccaccgctacgaagtcacgttcaaaggcccgggaggccacagcttcgccgccttcggccaggtgcccagcgcgatccacggcatgggccgcgccattgccaagatctccgaggtgcgcacgccgagcttcccgaagaccacgttcacggtcggcaccgtgggcggcggcacctcggtcaacaccattgcgcccgacgcgcgcatggccgtcgacatccgctcggacgacatggcctcgctgctcgaaacggagaagaagatcctcgcggccatcgacgaggctgtggtcgaagagaacaagcgctggaacgtgacgacgctgagcgcaagcaacaagctgatcggcgaccggccgggcggccgcacgccctccgactcggtcatggtggaagcagccatccgctcgaacacggccttcggccacaagacgctgctgcgcggcggcagcaccgacgccaacgtgccgatgtcgtacggcattccggccatcatcatcggcgggggcggcaagtccaccggctttcacgccctgagcgaggcgatcgacgtgacagacgcatggaaaggcgcgcagaattcgctcgtcacggtgctcggcttggtgggcgtgcaaggggtcagccccgcattgctgcccaaacggccggcgcgtacccggtaatttgtcacacggcgcggcgatagtgggcgctaccactgtcggctcgcggtccgtttgcgttggaaaatgcgggcggttctgtcacacaccaaggaaatcgccatgggattgctcgattcggtactcggtcaggtgctcggaggcgcgggccaacagcagcagcaaccgcagggcggcgggatgggcgatctcggcggcctggccggcgcgctgggcgggctgctcgccaacaacggcagcgcagggggcctgggagggctagtctcgaagttcgagcaagccggcatgggcgacgtgatcggctcctggatcggcaagggagaaaaccagccggtctccggcggacaactgcaggacgcgctgggcaacgacaccattgccaacatcgcctccaggctcggcatcaatgcgcaaacgctgctgcccatgctggccaccttgctgccggttctcatcgaccggctcacgccgcagggcaaggtgccggagcagggcctcggcgaccagagcgatctcctggcttcgcttggcggcctgctgcagaacaagcagccctgagccattgctcatcgagaattccagcgcccgcgagggcgcttttttttggcctgcgcatctcggctggcgcaccgggagcgaatcgcgtagaacctcagcctccatgccgctgcgcgccttcgccacttttccatgaaccgcaacctttggctgctcgccatctgccagggcttgttcctgaccaacaacgtgaccttcatcgccatcaacgggctggtggggctgagcatcgcaccgcgcggctggatggccacgctgccggtcatgggctacgtggtgggcggcgcgctcaccaccgggctggtggcgcgcacgcagcagcgattcggccgccgcggctcgttccagatcgggctggcggtggcgctgggctcggccttgctgtgcgcgttcgcggctgtgtcgaagaatttctggctcttgtgccttgccacggtggtggccggctactacaacgccaatgcgggcctctatcgctttgccgccgccgaactcgcggcaccggcctggcgcgagaaggccgtgtcgctggtgatggccggcgggttgatcggcgcggtggcgggccccaacctggcggccgccacgcgcgaagtgtttgcggtgccgttcgcgggtgcctacatcgcgctggcagcggtggcactgctctcgatgggggtcatgcggttcatcgactttcccgccacgctgactcgccagcaggcgctgggcgggcggccgctctcggagatcatgcggcagccggtgttcatcgtggcggccgcggcgggggcactgggcttcggcgtcatgaacctgctgatggccgccacgcccatcgccatgcagatctgcagcctgccgttttccgatgccgccctggtgctcgaatggcatgtgatcggcatgttcgcgccgggcttcttcaccggacacctcatccgccgctttggcgcactgcccgtgatgggcgtggggctcgcgctcaacttcggctgcatcgccgttgcgctgtcgggcgtggaactgcagcacttcctggtggcgctctgcctcttgggcgtgggctggaattttctgttcaccggcagcacgacgctgtcgctgacggcctatacggccgaagagcgcgaccgggcgcagggcgcgctcaacttctgcgtgttcgcgacgctggcgctgacttcgttcgcctcgggcgtgctggtcacgacgcagggctggcaattgctgaactacggttcgctggtgccggtggtgctcacgggcgcggcactgctatggctcgcgcagacgcgccggcgcgctgctgctgccgccaacgcctgaagcgcccgttcagtcaggcggaaagcgcttgtcgagccagcgctgcagcgcggcgaacaccggcccggcatccagctcgttgaatatctcgtggtacagggattcgaagcaccgcgcttcgaccatgccgctgggcgcggccgcctcggcgaaggcacggctggcggccggcaccaccagacggtcgtcgcccgcgtagatcagcaaagtgggaaccggccaatgcgccgcggcctgctgcaccaaagccccttcgtgcgcgagaaagcgcgcaagccggccgccgatgcggtcgtgcgtgagcggatcgtcgcggtaggcctgcaccacggcgcgatcgtgcgaaagaaaattgtcatccagcccattgccgacgcgaagcctgggcgcaatgcgcggcagcaccgcgagcagcgccttctggaaaccattcaggccgggatcaagccccggcgaggacagcaccagcccgtcgaccggccgtacgccgcgcgccaccaggctggccgcgaccagcccgcccaggctgtggcccagcagcaccagcggcaggccggggttctcgcgccgcgcgtcgtcgatgaccagcgcaaggtcgtcgaccagccgcaactcgctcggcaggccgccgcgcgcgccggaggactcgccgtgcccgtgatggtcatgcgcccacacggcgaaaccccacccgtgcaggcgctcggccaatgcctgatagcggccggcatgctcgccgaggccatgcaccagcaccaccacggcgcgcgatgcggcggccgacgggaggcggcgcagcgacagcgtctcgccgtcgggcgtggacagcgaaacgcgctgctgttgcaaaggcggcaaagtcggcgcgggtccggtcaagcagcgaccggctccgcagccgcggcgcgatgcgcagccggcagggccgcaatcacctcggccacggcggccgtgagcttcttggcgtagggcacatgcaggaattcgttgggtccgtgcgcgttgctcttcgggccgagtacgccgcagaccatcatctgggccttcgggaagcctgcgctcagcatgttcatcagcggaatggtgccgccttggccaatgtagccgcaggaggcgccgaagtgcgcccgcgaggccttgttgagcgcgtcttcgaaccacggcgtgatcgtcggggcgttccagccggtggcaccgccaccgctttcgaaggtcacgcgggcctggtagggcgcgttgtcttcgagcagcgtcttgagctgctgcaccgcttcggccgcatcgaccagcgggggcaggcgcagcgagagcttgaaggcggtgtaggggcgcagcacgttgcctgcatccttcagcgccggaaagccttccgcgccggtgaccgacagcgtgggcttccaggtgcggttgagcagcgcctccaccgggtcggtggtggttggcaacgcgaacatggtcgagccgccgcagtcgtagtgcgcccacggaaagcgcttgtagacctcttcgccgaggatggcggcggtggccctggcctgcgccaggcggtcggccggcacttcgcaatggaagctcgcgggcagcaggcggccggtggcgctgtcttcgaggcggtcgagcacctgccgcatgatgcggaagctcgaaggcaccaggcccgacgcgtcgccggagtggatgccttcggtcagcacttcgaccttgagcgtgccgctggccatgccgcgcagcgacgtggtgagccatagctggtcgtagttgccggcgccggagtccaggcagatcaccagttcgacattgcccagccgcgggcgcagcgcgtccacatagggcagcaggtcgtaggagccgctttcctcgcaggtctcgatcaggcccacgatgcgcggatgcgccgcaccctggttcttgagcgcctgcagcgcggcgacgctggcgtagaccgcatagccgtcgtcggcaccgccgcggccgtagagcaggccgttctcgtacttgggcgtccaggggccgaggtcgttgcgccagccggtgaattcgggttgcttgtcgaggtggccgtacatcagcacggtctcgcccatgtcggtgccggtggctggcacttcgaagaacagcaccggcgtgcggccttccaggcgcacgatctccagcttcaggccctcgaccttctgcgcctcgacccaggcggccgcgttgcgcagcaccgtttcaaggtagccgtgggcggcccactcggcgtcgaagccgggcgacttggcaggaatggcgatgtagtcggtcagctgcctgacgatgtcgccgtcccatcgggcgctgacatcggacagggcgcgctcggcatcgagcgttccggcgggcatttcgcggtgcaggggggcgttcatcggggggttctccgcgggtgaggaaaaaacgcattttgcgcctgcgcgcgaccccgcgtagagtgcgggcgatctcaacccggagcgcaatgtgagcaaggcaacatcgactcggaacccggtggatatcagggtaggcatcggcggctggacctacgagccctggcgcgacaacttctatcccaaggggctcgcgcaggccaaggaactgcgctttgcgagccgccaggtgagcgccatcgagatcaacggcacctactacagcaccttcaagcccgagaccttccgcaagtggcacgacgaggtgccggaggacttcatgttctcgatgaaggcctcgcgcttcaccaccaaccgcaaggtgcttgcgaccgcaggcgactcgatcaagcgcttcatcgaaagcggcgtggtcgaattgggcgacaagctcggcccgatcgtgtggcagttcatgccctccaagcagttcgatgcggaggacttcgaggcttttctgcagttgctgccgaagaaagagggcagccgcgcactgcgccacgtgatggacgtgcggcatgagagcttcatcacgcccgcctaccaggcgctcgcgaaaaaatacaaggtatcgaccgtgttcaccgacgcggacaagttcccgtcgttcgacgagcccgaaggcgactttgcctatgcgcggctcatgatggccgacgccaagctcaagacaggctatgcgccgaaagcgctcgacagctgggccgagcgcgcgcggcaatgggccgaatcacccagcaagcgcgaggtgttcgtctacttcatcaacggcgccaaagaaaaagcaccggccgcggccggtgccttgctggagcgcctgggttggaagccgcctgctgaagaaacagcctgatcaggctgcggcttgcagcgacggcttggcgccgaagctgatttcgcccgacagctggccgccttcctcgatcacgatcttgccgtagcggatcttgccggtgaccttgccggtcgaatggatcacgagcttttcgcgcaccgtgaggttgccgtcgaacacgccgcggatttcggcgatgtcgatttcagccgagcccttgaactcgccctgttcggcgatctgcatcaggcgcgagtccatcgtggcctcgaccaggccttcgaccacgagcgtgtcgcaatcggtgatctcgacgcccttgagcttgatgttggggccgacggtgagcttgctgccgccttccttggcgggtgcggtcgctgcggtgaggccgccttgctgagcggtcagagaagaaggattgacgggcgaacccgagagattggtacccgaacccaccagcggcgcggggcgggaggtcaacgagtcggtgtcacgatcacgcttgccgaaaaagggggactgtgtagccaatggggagctcctcaacaaaggggctatcgtaagaaccccctcgcggcctgcggcacttcattgcgcaagaaacgtaactgaataaatcccacggccgcccgacaatggcactctcaagtggcccaggccttgcaaagatgacccgaacgaacaccgactctgccgcccggaccttcgcgatctcctcgaccatcgacgcgcgcttcgacaagccggcaagtggctggcgacgtcggctgttcacggtgatcttcgaggccgacacgcgcgcgggcctgctcttcgaccttgcgctgattgccgtcatcgtgaccagcgtgctggtggtcattctcgacagcgtgcagtcgatccgggaccaatggcggtcgctgttcaatgcgttcgaatggacattcaccattctgttcacgctcgaatacattgcgcggctcgcctgcgtgaacaagccgatgcgctacgcgctcagcttctatggcgtgatcgacctgcttgcgctcctgccgacctacctggtggcgttcgcacccgaactcgcctatctcatcgacgtgcgcgtcctgcggctcttgcgcgtgttccgcatcttcaagctgtcgcgctactcggtggaataccgcgcgctggtctcggccgtggctgcaagccgccgcaagatcacggtgttcgtcggcttcgtgatgctggtggtgctggtgatgggcacgctgatgtacgtggtggagggcccggtgcacggctcacggcttcaccagcattccgatcgcaatctactgggccatctcgaccatggccactgtgggcttcggcgacctcgtgcccaagacggatctcggccgtgccattacctcggtgatgatgctgctgggctggggcgtgctggccgtgccgacgggcatcgtcaccgccgagatggcgcggcgcggtcccaatgaggatgctgagcccctgccgatagcggggcgtggcgtgctggcaatggtgcctccctcggcccgggcggttcccgcgcgtcggctcacgcctgctgccagacggcgcgcccttgcgcagcatcgtcgaggcgggcgatgaagctgccggcgtcggactcgggcagcgtgaacgcgaagtccaccgcgtcgccatgccgcacctcgaccagcgcggcgcctgccgcggcggcgatctcgcgccgcaccagcccctcgagcgcatagggcacggcgcattgcagcagccgctggcgcaccagcggaaccagcgtcgccccgaggcaggcctgcgccacggcatcggtgtaggcccgcacgagcccgcccgcgcccagcttgatgccaccgaagtaccgcaccaccgtggccagcacgccttcgagctgctggtgccgcagcacctcgagcatcgggcgcccggcggtgccgcccggctcgccgtcgtcgttggctgccgattggccgcccgccatgagcgcccagcagacatgcgcggcggcggggtgttcgttgcgaagcgtcgccaccacggccagtgccgcggctcggtcggccaccggctgcacgcagccgatgaagcggctcttcttgaccagcagttcgctgtgcgccggttgcgagagcgtgaagctcatggggccgccgttgtctgccaggtcacggaatcgctcagcgctcccgttcgaacttgaacacggccgtgcccgcccgcgcattgggcagccagcgcacgctgcggccttcctgcacgccgaaggcatcgagcacgtgcaggctgttcttttgcgccagcacctcgaagtccttgaacgtgccgacccggatgttgggcgtgtcgtaccactggtagggcaggcggcgcgtcaccggcatgcggccgcgcgcaatgctgatgcggttgggccaatgcgcaaagttgggaaaggcgacgatgccgatgcggcccacgcgcgcggtttcgcgcagcatgacctcggcattgcgcaagtgctgcagcgtgtcgatctgcagcaccacgtcgaacgtggcgtcgtcgaacacggcaaggccttcgtccaggttcagctggatcacgtcgacgccgcggcggatgcactgcagcacgttgccgtcggcaatctcgacgccgtagccactgcagccgcgctcgcgctgcagcaggtcgagcatggcgccgtcgccgcagccgaggtcgagcacgcgcgagccttcgggcacgagattggcgagaaggcgctgggtttcgatgtcactcattgcgctgtcccttcagcctggatctcatgcgccacgcgctcgaaataggaccgcaccacacccatgtagcgcacgtcgtcgagcaggaaggcatcgtgcccgtgcggtgcgtcgatctcggcgtagctcacgttgcggcggttgtcgagcagcgccttcaccagctcgcggctgcgcgcgggcgagaagcgccaatcggtcttgaagctcacaagcaggaacttggcggtggcttgcgccaacgccacactgaggttgccgccgtgggcgcgcgccgggtcgaagtagtcgagcgcgcgcgtgatcaggaggtaggtgttggcgtcgaagtattcgctgaacttgtcgccctggtagcgcaggtagctctcgatctggaactcgatctcctgcgtggaatagcggtagtcccgccccgccgcctcgccttcgaccgcgctgcgcaggatgcgtccgaacttctcgttcatgacgtcgtcgctcaggtaggtgatgtggccgatcatgcgcgcgatgcgcaggccacgtttgggaatgacgccgtgctcgtagaagtggccgccatgaaaatcggggtcggtgacgatggcgcggcgcgccacttcgttgaaggcgatgttctcggccgtgaggttgggcgcgctggccaccaccacggcgtgccgcacgcggtcggggtactgcagcgtccacgacagtgcctgcatgccgccgagacttccgcccatcaccgccgcgagcgtgcggatgccgagcgcgtcgagcagcgcggcctgggcatcgacccagtcctcgaccgtgaccacgggaaagtcggcgccatagacgcggccggtggcggggttcacatgcatcggcccggtcgagccgaagcaggaaccgaggttgttcacgccgatcacgaagaagcggtcggtgtccaccggcttgcccggtcccaccatgttgtcccaccagccttcggacttggactgcccttcgtaggtgcccgcgacgtggtgcgaggcattgagcgcatggcacaccagcaccgcattgctgcgctcggcgttcagggtgccgtaggtttcgtaggcaagcgtgtagctgccgagcgatgagccgctgcgcagggccagcgggcccgcgaactgcatcgactgcacagagacgaccaaggaaggtgacgacgacatcaatgaaaaaacccggcctcgccaaaaacgagccgggttgtcgccaactgactgtctttagctgaatttataaagcgcccgcaagctgtagcaaatcggcgcaggagccagtatatcgcccgccgcactaccagccgacgatcatcacgatgccgagcacgaggaagatcgcggccgagatgccgtgcacgagcttgatcggcacgcgcttcacgatcttgtcgccgagccagaccaccggtgcgttggccagcatcatgccgagcgtggtgcccgcgaccacccagacgtaggcctgcgtgaagcgcgcggccagcatgacggtcgcgatctgggtcttgtcgcccatctcggccaggaagaacgcgaccagcgtggtgccgaagacgccgtagtgcgaagcggcgggcgcgtcgtcttcgtcgagcttgtcgggaatcagcatccacgcggccatggcgatgaacgagccgcccaggatccagcgcaggacctcggggccgagccaacgggtgatgtagttgccgaccgcgccggccaatgcatggttgacgatggtggcggcgaagatgccgagcacgatgggccagggttttctgaaacgagcggccagcaagagggccagcaactgggtcttgtcgcccatttcggcgagcgcaaccacgcccgttgcaacgagaaaagcttccatgagagcaggggttccttgggccgaaggacgcaattgaccgtgcaacaccttcggccatattcccgaagttgcacggtcaaaggtctcgccaggtgattcactgcacgcgccatgtcctgtgtggggcaggacaagtctgttgacgcgggcccttctcgcggtggaaggcggctactccccaatgacgctcgggattctacctaacccgccgaacgccctctgtcgacaggtaagcgggcgctagcttttcgtaatttttggagcccctgcaggaagcggcaaattcctgcttgcatttcacgtatttcacccataatgcacgagcctccctcttcattttgctgggaggaagttcggtgatcggtcagtttcgcgcgactcgacggctctcgtttgagtgatgcttcagggactccgtcgcttttcttgctatgtgtttataggagtcccttgatgggcaacaaactgtacgtcggcaacctgccttactcagtgcgcgacggtgatctcgaacaggcttttggacaattcggttcggtgaccagtgccaaggtcatgatggaacgcgacaccggccgctcgaagggctttggcttcgtcgagatgggcagcgacgcggaagcgcaggccgccatcaacggcatgaacggccagcccctgggcggccgcagcgtcgtcgtaaatgaagcacgtccgatggaagcacgtcccccgcgcagcggtggtggtggtggtggcggctacggcggcggcggtggtggttatggcggcggtggtggcggtggctacggcggcggtggtggcggctacggtggtggcggcgatcgcagcggtggtggcggtggccgctccggcggtggtggcggctacggcggcggtggtggtggccgcagtggcggtggcggcggtggtggcgacggcggtttccgcagcccctacggcgccggtcctcgcggcggtggtggcggtggtcgctccggcggtggtggcggcggctacggcggcggtggaaacagcggctactgagccctgcatcccggttcacacagacaaaaggctccctcgggagcctttttcattggaacggacgcaaagtggcggcgcccgaggaaggctcagctttcgccgctgcgcttcttgcgggcacggccttgcacggcacggtcgagcaaggcgttcggcagcatgcgcatcagcttggcgaccacgcccatctgccagggaatcactcggtagctggtgccggcctcgatggcgcgcagcgcctggtccgcaaagtcttcggccttcatgagaaagggcatgccgtagcggttgccctgcgtcagcggcgtgtcgatgtagcccgggcacagcgtgacgaccttgacgccgctgttgtgcagctcgccccgcaggctctcgcaatacgcgaccacacccgccttgctggcgcagtaggccccatgccccggcaagccgcggatggccgcaacgctcgcgatgccgaccagccggccgctgccgcgctgccgcatcgccgcaacgaaaggatggaaggtggccatcaggcccacgttgttggtggcgaaggtccgactcatcacctcgatgtcttcgcgctccgccgtgtcgatgcccacgctgatgccggcgttggcaatcaccacgtcgggcgggccctggcgttcgatgcaggcggcgccggcagccaggatgctgtccgtcagggccacgtcggcgctatatatctgatagcgggaggggtccagctggcaggcggcggcccaggattcgatttccccggtgcggcgggcgaccagcgccagccggtagccggcccaataaaagctcgcggcgagggcctggccgatgccgctcgacgcgccggtgatgaagacaagcggggatgggctcatgcgcgggctgtcttccgggttgcttttgttttgtcttcagcgcggtttgccggctgagggagcggccgatgggatcagcacgccgcgcacccggccggtcaggttggccacgccgctcaggttgtcgtagtcgaggttgtcggcggtgaactggtcgctgccgcggatgagcgtgacgggcttgttcgaggtcacacgctcggagtcgagaaaggcgtggaggaagtcgccgcggaactcgagccgcggcgtgcccttgccgccgggcgcgacgacggggtcgcggatgacgacggcattgccgaagagctggatctcgctgccatcggaattcgacaggccgcggttggccgtggcgtgggtggtgtagccctgcggcgagacggagcgcatgcgcacgtcgtcgacctcgacggtgtcggtgtccgggtagtgccggccttccttgccgtggagttcgctgcgcaggtcgccgttgggcaggaagttcttgatcacgaagccgcgcatgaaatagtcgggctcgtgcgtgggcgcggccttggcggtgggttcgagcagcttgggcgcgttgcgcaccagccagtaggtaccgagcgccaccgccgcggtcaggatgatgggcaggtagatggtggcgcggtcgagaacgtcgcgcagcaggttccaggcacccttcattgccggggaccccgggcggtgtcgagcaggcgccggtactggccgcaggccgtcagcagcaggtcgcagaattcgcgtgccgcgccttcgccgccgcgtgcgcgggtgacgtagttgaccgcttctcgcacttccacgtgcgcattggcgggggctgccgcaaagccggcgcgcgccagcaccggcaggtcgggccagtcgtcgccgatggcggccgcctggtgccaaccaaacccaagctgttggagcatggcttcggccgcgggcagcttgtcttcggtgccgtagcgcacatgctcgatgccgagcgcttcgagccgcacgcgcagcggcttcgaatcgcgcccggtgatcaccgcgggcgtgatgccggccaggcgcagcagcttgaggccgtaaccgtccaggatgctgaagcgcttgagggtttcgccgtgttcggtgaaatagacgccgccgtcggtcagcacgccgtcgatgtcgaagaacgcaatgcgcgcatcctgcgcggcaatcaaggtttctgcctggaagtcgagcggcatcagatgaccttcgcgcgcatcaggtcgttgatgctgagcgcgccgatcaaatgccccgcgggatcgacgatgagcacgctggtgatgcggtgttcttccatcagttcggccgcctcgaccgccagcgcatcggcgcgcagcgtgcgcggaccggggtgcatcacgtcggcggccgtgaggccgcgcaggtcgccgccggtctcgacctggcggcgcaggtcgccatcggtgaagatgccgatggcccggccttcggcgtcgaccacggccgtgacacccaggcccttggagctcatctcgcgcatcagttcgctgagcgtagcggtgggcgcgacacgcggcacttcgtcgcccgagcgcatcacgtcggccacgtgagtgagcagcttgcggcccagcgcgccgccggggtgcgagcgcgcgaagtcttcggagccgaagccgcgtgcatcgagcagcgccaccgccagcgcatcgcccatcgccatctgggcggtggtgctcgcggtgggggcgaggttgagcgggcaggcctccttggcaacgccggcgtcgatcacgatgtcggcgtggcgggccagggtggaatcgatgcggccggtcatggcgatgaggggcacgccctggcgcttgacgaccggcaggatcacggtgagctcgtcgacctcgccgctgttggagatggcgagcaccaggtcgaccgccttgatcatgccgagatcgccgtggctggcctcggccggatggacgaacatggccggcgtgcccgtggaggccagggtcgcggcgatcttgcggcccacgtggccgctcttgcccatgcccatgacgaccacgcggccgcgcacttcgaggatcttgcgcacggcgtcgacgaagctcgggcccacgcgcgacttgaggccgagtacggcgtcggactcgatgtcgaaggtggcgcgcgcgcgcgccaggatcgcgtcggcgtcgaccacggggggcaggggagctgaactcatcggcggattttacgggccggccgacttggccggtcagcgggcgaaaggggcacgcccggggcatggacattgctctagcatccgaccatgtcttcgttcgatctcacgctgatgtatttgctggccgcggtgatcggcgtcgtcgtctgccgttcgctgaaactgcctccgatgctcggctatctgacggccggcgtgctgatcgggccccatgcgctgggattggcgcacaactccgaagccatcctccacttgggcgagttcggcgtggtgttcctgatgttcgtgatcgggctggagttcagcctgcccaagctgcgcgccatgcgcaagcacgtgttcgggctcggcctcctgcaggtgctgctcacgatgaccatcgccaccgccggtgcgctcttgatcgcctcgcagctcccgccggcctggcggctcggctggcagacagcgctggcgctgtcgggcgcgttgaccatgagcagcaccgcgatcgtggtcaagctgatggccgagcggctcgagctcgagagcgaacacggcaggcgcgtgatgggcgtgctgctgttccaggacttggccgtggtgccgctgctggtgctgatacccgcgctcggcgcaccgccagaggcgctggccaaggccatcgggctggccatggtgaaggccaccttgctgatcggcctgctgcttttcggcggtccgcgcatcatgcgctggtggctcaccctggtggcccggcggcgcagcgaggaactcttcatcctgaacgtgctgctgatcacgctcggcctggcatggctcaccgacctggccggcctgagcctggcgctgggcgccttcatcgccggcatgctggtgtcggagaccgaatacaagcaccaggtcgagaccgacatccgcccgttccacgacgtgctgctgggccttttcttcatcaccgtgggcatgtctctcgactggcacatcgtggtggaccggtgggccctggtggccgtgctgctgatcctgccgctggccttcaagctcgcgctggtgacggtgctggcgcgggtgctgggcgccaccgcgggggtgtcgctgcgcaccggcctgtacctggcgcaggcgggcgaattcggcttcgtgctgctgacgctggcccaggagcgcagcctgctgccgccctggctcgccaacccggtgctggcctcgatggtgctgtcgatgctcgcgacgccgttcatcgtgatgtacgccaacgccatcgtgcgcaagctggtggcaagcgactggctccagcaatcgctgcagatgaccagcatcgcgcgcaagaccatcaacaccgcgcagcacgtgatcatctgcggctacggacgctgcggccagaacctggcgcgcatcctggagcacgagggcattccgtacatggcgctcgacctcgaccccgaccgcgtgcggcaggccgccgcggccggcgattcggtggtgttcggcgacgcggcgcggctgcaggcgctgatggcggccggcctggcccgcgccagcgccgtggtcgtcacttatctcgacgtgccgggcgcgatgaaggtgctggccaacacccgtgcccacgcgccgcaggtgcccgtgatcgtgcgcacgcaggacgaccacgaccttgaaaagctgcaggccgcgggcgcgaccgaagtggtgcccgaggccatcgagggttcgctgatgctcgcgagccatgcgctcgcattggtgggtgtgccgatgcggcgtgtgatccgcgtggtgcaggaccagcgcgatgcgcgctacaacctgctgcgcggctacttccacggcgccgacgacgacaacgccgacgagatcgaccatgagcggctcaacaccttcaccctcacccccggcgcccgtgcggtgggacagaccctggcgcgactggcgctggaatccttgggcgttcgcgtcgccagcctgcgccgccataacggccaggcccaggtactcaccgacgacacggtgctgagcgacggcgataccctcgtgctgtccggcaaaccggcagccctggcggtcgccatagagcggctgcaaaagggctaggaccctcccgcggcgccgagctagttgaccagcgtcgggttgcgcttttcttcttcgatgcgctgctgccggcgcacggcctcgcattgcgcgtgcggcttgtattcgggcttgaggcactgcgcggccatgcactgggccttcgcgatgaaattgcggtcgccgcaaatggccagcgggtcggtgggcgccgagggcgcctgggacggcgccggcgccgcggcggttgcagccggaacggactcgggcgctccggcctgcgacggtgccgcgggtgcgggcttgcgcgacttgctcacggctgcaggggctggcttgaggttggcggcaggggccgtggttgccgccgcatcgtgcggcagggtttccgcggccggcggctccgcaggcgcaggttcgggcactgccgccggtggctccatcgacggcacgggcggcacggcgggcgcagcgggtttggcgatttcgacttcttcgtccggctggtccgctccgtagccgcgccagcccgcagcgaccatgacgagccccgccgccagcaacagcaaccagagccagaagccgcgggagcgccacggctttcggggctcggcacggggcggccgcggcgtcctgggcttggaagacttccttgcccgaggttcccgcggcggcgacggcgggcgcctcaggcggcccaacgcggcaatgagggtcttctcatccgccagcgttgcggtgcccgcagacgacgccgtggatgcggccggcacgccggtctcgaagagcccgccggggatcgtgggtgcgcgcagttgcgcgggcgccgtggtggcccactcgcgctccgaccggctgcggggagcgggagacggcgaaatcggcatgggtgcggcgggcgccagcttgccgccgcagctcttgcagaaattcgcgccctcgcggttttccatgctgcagaccggacagatcaaggccatttcgactgacttctagggaacggggaacgattttctggaacggaccgcggcgtgctgccacggtttgcacttcatgcggaatggccggatggaggctcaggtgaccgcgacgcgcttggaccggtgtgccatgcgcttggcgatcaccgcgccaagacccatggcgatttcgagtgccaggttgggctgccgattcgacatttccaggaagcggaccgccgtgagccgccatacgcgccccgcaccggtgaccaccacgttggccgaatgcggttcgcgcgagaagaaagaaccttcgcccaccaccgaccccggcatgagcacggccagcttcatctgttccttgctgctcacgcggtgcacgctgatggcgccgctctcgagaaagtacaccgagcggtcgtgcgtgccctgctcgatgagaacgtcgccaacgccggtcgtgatgggctgcagatagcccgccagcgtttcccactgttgtacgttcagcgtcaacgcaaaggcgtcggtgctgttgttgtccgcgatggcgcggctcaggttctggatggacatgcttttctcaacccccgcatctgtgccggagtatccgcgaagggcgcggttttcggctacaactctttacggttttcggaggggctgtctctatttgccgatacagaagcgcgaaaagatgactcccagcaagtcgtcggcgccgaactcgccggtgatttcgttcagcgcgttctgcgccaggcgcagttcctcggccagcaggtcgagcagttgcgcctgcgctgccagatggatcgcggccagcgtcaggtgcgtttcgacccgggccagcgcctgcacgtggcgcgcacgcgccaggtagaccccctcgggcacggcctgccagccggccatggccagcagttgctcgcgcagcgcttcgatgccgaggccggtcttggcggacagggcgatgccctgggccgtactcgcacctgcactcgccataggcgcggcgtcctgcttgttccacacatcgagcaccggcacgctcgcgggcagcttctgccgcaggctgcgcaagatctcggcgtcggcggcgacgtagtcgggcaggccggcgcgcgtcaggtcgtgcaggaacagcaccgcgtcggcgctttcgatctggccccaggcgcgtgcaacgccgatctgttcgacctcgtcgctgctttcgcgcaggcccgccgtgtcggccacgtgcagcggcacgccgtggatctggatggtctgcgagaccacgtcgcgcgtggtgcccgccaccgcgctcacgatggccagttcggcacccgccaatgcattgagcagcgaacttttgcctgcattgggctggcccgcgatcaccaccttgatgccctcgcgcagcagtgccccctgcttggcgcgctgctgcaccgcagccaattgcacctggagtctcgcgagctgcccagccgcgtcggctttctggagaaagtcgatctcctcctcgggaaaatcgagagtggcttcgaccagcatgcgcagatggatcaatgcatcgcgcagcgtgtggatctcgcgcgagaacgcgcccgagagcgagcgcccggcgctgcgcgcggccgcctcggtgctggcgtcgatcaggtcggcaatggcctcggcctgggccaggtcgatcttgccgttcaggaaggcgcgctggctgaactcgcccggctcggccacgcgcaggccgggcaggcgcgggcggccggtgaccggatcggcctgggcggcggcttcgaggcaacgtgccagcaaaagctgcagcaccaccgttccgccgtgggcttgcagctcgagcacgtcttcgccggtgaacgaatggggcgagggaaagtggattgccaagccgtggtcgaccggttcaccggccgcgtcgcggaacgggagataggtggcttcgcgcggcttcagcggccggccgcagagggcctcgatcagcggcgcgagccgggcaccggacacgcgcacgatcccgacggccccgcgccccgaggcggtggcgacggcgacgatgggatcggtggtgcgggcgaaggtcatggaaacacgattctttcagcaaaaaggcaaagggccgcggatgcggccctttgcgtgggtggctaaggccgctgtgcttacttgcccagcacgcccagccgcttgttgatgaaccactgctgcgcaatcgacagcacgttgttggtgatccagtagagcaccaggccggccgggaagaagatgaacatcacgctgaacgcgagcggcatgatccacatcagcttggcctgcatcggatcgggcggcgtcgggttgagccaggtctggaacagcgaggtgagcgtcatcacgatcggcaggatgtaccagggatcgggtgccgacaggtcggtgatccagccgatccacggtgcgtggcgcatttcgaccgacgacagcagcacccagtagagcgcaatgaacaccgggatctggatcacgatcgggaagcagccgcccatcgggttgaccttttcggtcttgtagatgcgcatcatctcctgctgcatttcttgcggcttgtccttcagccgctcgcgcatttccatgatcttggggttgatggccttcatcttggccatgctggcgtaggccttggcgttgagccagtagaaggccgccttcagcagcaccaccagcgccacgatggcccagccccagttgcccagcatgccgtgcagctggttcagcagccagtacagcggcttggaaatgatcgcgaagatgccgtagtccttgaccaggtccaggcccggcgcaatggcttcgagcttcttttcttcttcagggcccgcgaacagcgcgctgttgaccacctgggtctggcccggggcgatcttcggcagcgtggccaccatggccacggtgaagaggttgccgcccagatccttcacgcggaattcgcgcttgagctgttcgctggccgggtcgcccttgagcagccaggccgacacgaagtaatgctgcaccatggcaatccagccgtcgttggcgggcggcggcggctcgatcttgcccttggcgatgtccgagaagtcgagcttgtggaacttcttctcgttggtgtacgcggccgggccggtgaaggtgttggtgccgaacatcgtgccggcggccaccgtgccgtggcgcagcagctgcatgtagagctgcgcgtcgcgcggctggtcgcttacgttgacgacctcgtggcgcacgccgatggtgtagtcgccgcgcttgaacacataggtcttgacgtacttcaagccgcccgagggcgcgctttcgaagctcacttcgagcgtgttctggccttcggccatttcgcgcggacccggcttcggcgccatcggcgtcaggtggttggggaagggttcaccggtctggctcagcaggccggtctgcgccacgtattgggtggcgggcgaatcgctctcgaacaggacgacgtgcttggtgcggtcggcttcttcgtacttcagcagctccaggtagttgaccgtggcgccttcgctgtcgatcactgccttgaagagatcggtggtcacgctgacccgctcgcgcggcgcggccggggcggcctgcgtgggcacggcgcccgcagtgccgccggtggcggacgcggcggctggcacgccgttgctggcggccggcgtgctgcccgctggcgcggaagccacggcagccggcttgctcgacggcaggaaggtcggcttgttgccgttgaagacctgccattggtcccacagcagcaccagcgagaaaccaaaaatcacccacaggatcgtgcggcgtatatcgttcatgacgaagacttcttgtcggaggagagaagagacgaaaacagcgagcctggcttgccagtgcgacgctgtgatttcggtggaaccggatcgtgcccgccctggcaccagggttggcagcgcgcgatgcggtgcagggtgaggtaactgcccttgagagcgccgtggacttcgagcgcctcgatcgaatagacggagcaggtcggctcgaagcggcacgactgcccgagccaggggctcagcagcaggcgatagcctttcacgaggccgatcagcaagcgcttcatgacgacggggcagaggagcgcgcggcccgcgccagcaggtgctggagttcggcgcgcacggcggccttgagcttgtccgaggaggcgctcacgaattccttgcggtcaaatcccgcgcgcagccgcaccacgtgcgccgcacggggcaggcccgcatcgggtgcggcgctcacggtatagatctgacgcttgatggcgttgcgcgtgaccgcgcggcgcgcccagcgcttgggcaccatggcgcccagccaaacatcgtcggacgcgaacaaaggctgcgcgctcgacgaatcgagcgcgcagcgatgcaatgcgaaatgagcagtgcgcgccacggtggcacctgcgaggacggcctggaactgcgcgcgggtcttgagccgctgcatggaagccgggccgcttgcgttgtcgctggtcgggccagaagtactggcggcgaaagctggcgctggcggctcggcggctggcaacggcagaactgccgtcagacggccaggcgcttgcggcccttggcgcggcgtgcgttgatgacggcacggccgccacgggtcttcatacggaccagaaagccgtgggtacgggcgcggcggactttggaagcttggtaagtgcgtttcatgatgagatttcctgctgattcccccgatatccgcgatgtcccctatgaagccatgaaggccatattggacatgcgagcgctgggagcgtttttcggatgacccccgaaagacgcaatgaggttttcagggaaacccgcaattatcgcaaacattcggcccaacaccaaacatcgagcaactttgcgggcctttgccgggtgcacccggggatgtggataaggttttgacaagttagaatgcgggccgccttgcagcggagcatatccacaacacatataccaaaaaatggccgcgggactcaccactttttcaagcacccatgtcgactgacggcatcggtgagagcctctggcaggcttgcgtcgaccagctcgcgcaggagctgtccgagcagcagttcaacacctggatcaaacccctgacggcgcaggtcgcggacgacctttcgcgcatgacggtgttcgttgccaaccgcttcaagctcgactggatccgggcccagtatgcgggcaagattgccgccatggccgagaagatgtacggccagccggttgcagttgagttagcgctcgctccgcgcgaagcacccgtgcgctctacacccgttgccgttctggccgaaaccgacgtgccgcgcgacgtggccgggccgggcgaggaaccggcggccgccggcttcaagaaccgcctcaattcgggcctgaccttcgacaccttggtggagggcacggccaaccgcatggcgcgcgccgcggccatgcacgtggccggcatgccgggccacctgtacaacccgctgttcatctacggcggcgtcggcctgggcaagacccacctgatgcacgctgtgggtaaccggctgctcgcagaccgtccggattccaaagttctctacatccatgccgagcagttcgtctcggatgtggtcaaggcctaccagcgcaagactttcgacgaattcaaggagcgctaccactcgctcgatctgctcttgatcgacgatgtgcagttctttgccaacaaggaccgcacgcaggaagaattcttcaacgcgttcgaagccctgctggccaagaagtcccacatcgtgatgaccagcgacacctatccgaagggcctggccgacatccacgagcgcctggtgtcgcgcttcgattcgggcctcaccgtcgccatcgagccacccgagctcgaaatgcgggtggccatcctgatcaacaaggcgcgcgccgaatcggccgaaatgccggaagaggtggccttcttcgtcgccaagaacgtgcgctcgaacgtgcgcgagctcgaaggcgcgctgcgcaagatcctggcgtactcgcgcttcaaccagaaggaaatctcgatcgccctggcgcgcgaggcgctgcgcgacctgctgtcgatccagaatcggcagatctcggtcgagaatatccagaagacggtggccgactattacaagatcaaggtcgccgacatgtacagcaagaagcgcccggccagcatcgcgcggccccggcagatcgcgatgtacctggccaaggagctcacgcaaaagagcctgcctgaaatcggcgagctgttcggcgggcgcgaccacaccacggtgctgcacgcggtgcgcaagatttcgggcgagcgccagcagctcaccgaactcaaccagcagttgcacgtgctcgagcaaacgctcaagggctgaccgcgaatgtcatcaagaatgcgcctcgcaacagcggagaatggcgtcttacaagcggattcaaagagataaagagaagaggaagaagacatgatcgttttgaaggcaacccaagacaaagtcctcgccgcgctgcaatcggtggcgggcatcgtggaacggcgccatacgctgccgatcctcgccaatgtgctgatccgcaagaccggcggtcagcttcagctgaccaccagcgatctcgagatccagatccgcaccacggccgaactcggcggcgatgaaggcaacttcaccaccaccatcggcgcgcgcaagctcatcgacatcctgcgcaccatgccggccgaccagaccgtgagcctcgaatcgagcgcgagcaagctggtgctcaagggcggcaagagccgcttcacgctgcagtcgctgccggccgaagactttccgctggtgcaggaagccgccaacttcggccccgtgttcagcgtgccgcaaaaaacgctgaaggacctgctctcgcaggtctcgtttgccatggccgtgcacgacatccgctattacctgaacggcatcctgttcgtggccgaaggcaagcaactgagcctggtggccaccgacgggcaccgcctggctttttcgtcggccacgctcgacgtcgaagtgccgcgccaggaagtcattcttccgcgcaagaccgtgcttgaaatgcagcgcctgctgtcggacgccgaaggcgccatcgagatgcagtttgccaacaaccaggccaagttcagcttcggtggcatggagttcgtcaccaagctggtcgagggcaagttccccgactacaaccgcgtgattcccaagaaccacaagaacagcgtcacgctcggccgcgcccccctcctggccagcctgcagcgcaccgccatcctgacaagcgagaagttcaagggcgtgcggctcaacatcgagcccggcaccctgcgcatcgcatcgaacaacgccgagcaggaagaagcgcaggacgaactcgacatcgactacggcggcgacgccatcgagatcggcttcaacgtcacctacctgatcgacgccctgtccaacatggaccaggacatggtcaagctggacctggccgactccaacagctccgcccttttaaccatccccgagaacgcatccttcaaatatgtcgtgatgccgatgcgaatctagaagacagaaaacacagcgccttgcgcagacagcccgcggccctccgcgggtttgcgctttcaagaggccggaaaaacaggctcccagagcccgaaaaatcccgtgaatgccgtgagagatagaggaatatccgaatgagtgcagaagagaacaagcccgaagtgccccacaccgaaccggtctacacccccgagatcgagagtgcggtgccgatcgagatcacgcccgccgacaccagctacggcgaaggctcgatcacgatcctcgaagggctcgaggcggtgcgcaagcgccccggcatgtacatcggcgacacctccgacggcacgggcctgcaccacctggtgttcgaagtggtcgacaactccatcgacgaagcactggctggccactgcgacgacatcgtcgtcaccatccacagcgacaactcgatctccgtcaccgacaacggccgcggcattccgaccggcgtgaagatggacgacaagcacgagcccaagcgctcggcggccgaaattgcgctcaccgaactgcacgcgggcggcaagttcaaccagaacagctacaaggtctcgggcggcctgcacggcgtgggcgtgagctgcgtgaacgcgctgagcgtgaagctgcgcctgatcgtgcgccgcgaaggcaagatccacgaactcgaattcagccgcggcttcgtgcagaaccgtttgctcgagaccgtgaacggcttcgaggtgtcgcccatgaaggtcatcggcgacaccgacaagcgcggcaccgaggtgcactttctgcccgacaccgagatcttcaaggaaaacgccgatttccactacgagatcctgagcaagcgcctgcgcgagctgagctttctgaacaacggcgtgcgcatccgtctgcacgacgaacgcaccggcaaggaagacgacttctcgggcgccggcggcgtgcgcggcttcgtggagttcatcaacaagggcaagaccgtcctgcatccgaactcgttctatgccgctggcgaaaagccggccgacacctacggcggcatcccgggcacgcacatcggcgttgaagtggccatgcagtggaacagcggctacaacgagcaagtcctctgtttcaccaacaacattccccagcgtgacggcggcacccacctcacgggcctgcgcgccgcgatgacccgcgtcatcaacaagtacatcgaagagaacgagttcgccaagaaggcgaaggtcgaagtcaccggcgacgacatgcgcgaaggcctgtgctgcgtgctgagcgtgaaggtgcccgagcccaagttctcgagccagaccaaggacaagctggtgtccagcgaagtgcgcgccccggtcgaagacatcgtcggccgcctgctcaccgactacctgcaggagcgcccgaacgacgccaagatcatctgcggcaagatcgtcgaggccgcccgcgcccgcgaagccgcacgcaaggcccgcgaaatgacgcgccgcaagggcgtgctcgacggcatgggcctgcccggcaagctggccgactgccaggaaaaagatcccgcactctgcgaggtctacctggtggagggcgactccgccggcggttccgccaagcagggccgcgaccggaagttccaggccatcctgccgctgcgcggcaagatcctgaacgtcgaaaaggcgcgctacgagaagctgctcaccagcaacgaaattctcaccatgatcaccgctttaggcaccggcatcggccgcgccggcgccaccagcgcgggcggcggggcggacgacttcaacgttgccaagctgcgctaccaccgcatcatcatcatgaccgacgccgacgtcgacggcgcccacatccgcacgctgctgctcacgttcttctaccggcagatgccagagctggtcgagcgcggccacatctacatcgcgcagccgccgctttacaaggtgaaggtcggcaaggaagagcagtacctgaaggacggccccgcgctcgacgccttcctgctcaaggtggccctgaaggacgcgagcatcgagaccggcggccccaactcgaccacgctcaccggcgataccctggccgaactggcgcgcaagcaccagctggccgaagccgtgattgcgcggctgcgcaacttcatggatgcggaggcgctgcgcgccattgccgacggcgtggcgctcgacctcgacaccacccccgcggccgaagcctcggccgtggcgctgcaggccaagctgcgcgaactcaacaccaccggtgtgccggccgaagtgagcagcgaattcgatgcccgcaccgacaagccgctgctgcgcatcagccgccgccaccacggcaacatcaagagcagcgtgctcacccaggacttcgtgcacggcgccgactacgccgcgctcgccgaagccgccaacaccttccgcaacctgctgagcagcgacggcgccaccgtccgccgcggcgaaggcgaacgcgccaaggaagaaaaagtggccgacttccgcatcgccatgaagtggctcatcggccaggccgaaaacgccacctcgcgccaacgctacaagggcctgggcgaaatgaaccccgcacagctgtgggaaaccaccatggacccgaccgtgcgccgcctgctgcgcgtgcagatcgacgacgccatcgaggccgaccgcgtgttcacgatgctgatgggcgacgaggtggagccgcggcgcgagttcattgagcagaacgcgctgcgggcggcgaatattgacgtttgattgattgattagcgatcagcggcagcccagccggaactgttggtcccgcgcttgctgcctctcgttgcgcagccggtcttgcgtagccatgccgtgcggctgccgccccatcgtgtcgagccacttgatgtgcgcttcgagtgcgctgcactcgcccgcctgcatgttgttgcccgcactctgagccacctggcgttcatacgattgctgctgctgcgccgcgagcgccgcattgctccggttcgacgcctcccgcgcctcgacgctcattccatccgccagattcagatcgcgccgcagccgcaccgtagtggcgaccgagcctgccgggcagaggccatccgaataggtagccttgcctgacgcactcacgcactttgcgacctcgacggtccccggcgcagcagaacgatccggttggaccgcggaagacggtggcgatgggacacgcccggtcgtcggcgatgggaccggcggagagggcagggcagaaggcgccttgggtctgagcgcggcgcgttgcgccaacagccattcagcgccgcaatagaccccgaacatcagcaagcccgacagcccgacccacatcagccagtggcgctcccgcgtggggcgcaagccgcgctcccattccgtcatcgcgttgcggctgtcgtgcagcgggtcgcgatggtcggaattcatgaaggccgagtatccccgcttcgctggctgtttcgccaacgaacggcccggcgcttcaccagtagcagccgatcaatgcaatgcgagactcagattgaccgatgcacgcgagtgccgctcctgccgccctgcatcattcgcgctgcgcgggccacgcgggccagcccgcccgtcccgctcgccgcgcggccgaccagcgcaccgcccgccgcgcctgccagcacacggcgcatcagcgagcggctgcttcccgccttcagcagcagcaagaggcctgctccgagcacagccaagtgctcgcccggaatcccgcggcgctgggcatccatcttcttgattgcgtcgatcttcgatccgatggtcatttgaaagctccttttctgtacgaacttcttcataaccaacgaggcggtgcaccgctgtaggcgccgatcacgtgcgccgcgtcggatcgggcgcacacagagggcgtctcagggttttcataggtaggacggtgcaaaaccgcgcagatacccgtcacacaatcgtcatgagctattaaaacaatagcgttcagcaggtcgccgaggatcgttcctcgtaaacgctatatctagcccgactcttgctaagcaaaatcctcgacggatttcacgtcacccatgatcgaggacatcgaagcaatgaaccttatgcgtctccggcagccgatggctgcgttggtactgggcggcacagcagcattcttcggggcgatgaccacatcggcccacgcgttctcgaacccgcccatccagatggcgcagggcgtcgaatacatgtgcgggggcacgagcaaggacgaagccgctttcatgcagatggtctcgccgcgctgggcggccacgctcgagttcggcgtcaacgacagcgcgcaaaagggcaatttccccgcgcgggctgcggtccaggtgcgcgaaaagtacacgggccgcccggtgatggaagcccagtcgcaagggccgtacatgctgacacggctcgacccgggcgcctacgacgtgaacgtcacgcttggcggcctcacgatcacgcagacgctgacggtgatcgccggcgtgccggcacgcgccgtgttcatgtggccgtcgaatttcgacatggcctcagtgctgccgcctgcagcgcagacccaggcgttcgcgcagacctccgccgcccgctgagcatcctccgcccttcggctggcgccggggcccggatcccttgttaagccttgtttaagccgtgcgccgcagagtggcgccgtggtgtctcgccacgcaggtacgcaagaaaaggaaaggatccagaccatgaccacccttcggatttcatcgcccagccggcccgccgcagcggccgccaccatgctgtgcggcgccgctcttcttttcttggcggcgctgacttcagcgcacgccacggtcaacccgccgatccgcatgacgcacggcatcgaatacatgagcggcggcatcggcagcgacgaggcccaactgatggaaacggtggcgccacgctggccggccacgttcgagtttgcgatcaaggaccacaagggcgccgatttcgcgtccgacgtccgcgtgaccgtgcgcgacagccgcggcacggtgctgctcgacaacgtggcgtcggagggcccgttcatggtggctcgcctcgaccccggcacttacgaagtggaggctcgcttgcgcggaaacacgctcaagcaaacgctgcaggtggcaccaggaacgcccgcccggatggcatttctgtggccagcaggcaccgacatggcttcggccggcacgcgcacggtgcagtaacaagcgagcctggtttcggacgccgggccccggacctccggttttcgagttcacatcacccgcggtgcctgctatccggggcccctgcgctatagaaaaaatagctactcgggcgccgcaaggcgccttgaatgcacggcatgcgccttgcagatgtcccatcccgggcaacgccctttcccattgccccaatgccgatacgtctcctgagcgttctcaccgcgctcctgcatgtctacatggcgctgcgcctgctgcccgcgctggccacgctcacgccagcctggccgctggcgctggccgcgctcgccatctcggccgtcacgatcccgctaccctttgtctcgcgccgcattgcgcccaacgcctcgctgggcgaaacgctcaagtgggtcggcctgatcagcatgggctggttctcgtcgatgttcgtcttgacgctggcgcgcgaggccggcttgctgcttatctggctggcgagcacgctgggcggcccgcaggtgcgctgggacgcgttgctgccgtggagcgcactggcggtgctggcaatggccacgggcactacgctgatcggcttcatcaatgcccgccgcaccgccagcgtgaagcacgtcgacattccgattcgcggcctgccgacggcgctcgacggcttcacgatcgcgcagctcagcgacatccacgtcggtccgacgatcaggagcgcctacatccagcgcatcgtcgatgcggtgaaccggctcggcgccgacgccattgcgatcacgggcgacttggtggacggcacggtggccgaactgcgcgagcacatcgcccccttggccggcctgactgcgcggcacggtactttcgtggtcacgggcaatcatgagtattacgccggggcccatgcatggatcgacgaactgcgtcggctcggcctgaaggtgctgctcaacgagcacgtggtgctgcaaacgcgcaacgtgcgcggcgcgcagaacgacgaagagctgttcgaaagccagctggtgctggccggcgtgaccgactacaccgcggggcatttcgatgccgcgcatgaaagcgacccccacctggcgctgttcgacgcgccgccgctggtgcacacgcgggtgctgcttgcgcaccagccgcgcagtgcgccgttggcggccaaggccggctaccagctgcagctgtcgggccacacgcacggcggccagttctttccgtggaacctcttcgtgccgatgcagcagcccttcacggcgggcctgcaccggctgcacgacatgtggatctacgtgagccgcggcaccggctattgggggccgcccaagcgctttggcgcgccttccgagatcacgctgctgaccctggtgcctgcgcgcaattaattaggcacgcgcccgctcagtcgcgcagctcggccaggcgccgggcgttcgaagtggcggcggcatggatcggcttcagcccctggcgcgcgatgcggaccgccgcacccgacagctggctggccgtgcccgccgcgcgcgcggcagccctgacgaaagcatcgctgcgcacggccgcctgcgccggcgtgacgctgcccgtcatcgagaggaaggcgcccgcgctctgaaaccattgctgcagcgcgcggttcgccagggcgacatggctgctgtgccactgcttggccatggccacccccgattcgcccgccgcggcgagcttttcattgcccatgagctggaactcggcaaggtctgccgcgctgggcgtgagtcccgccttggcaatgcgctcggtgcgcatctggatcacggagcctgaagacaacagcatctcgtgggtcttgagggccacatcgacccacagcatcagggggctggccagacgaacggcggaggtaagggacgacatgagggcgggtctatggaatggacgaacaccactataggcgccgacgaaggggatttgctgcactgcaacaaaatgcgcagccattttgttgaacaagtcgtgccttttgacacggaaacagccttccgccccggcagtgaacagaacggaagtaattatttacttccttcattgacaacggcccgtgcgcgccagcgcttggcgcgcagttccgcaacaaagtaagccagcgtggccacgcccaacggcaacaggtagtagaggccccggtagaccagcagtacgcccagcagccggccttggggcacctggtccgaaagcagcgcaatgaacaccgcttccagcacgccaagccccgccggcacgtgggtgatgacgcccgccaccgcggccacgagcagcaccgcaagcaccgagtggtaagccagctcaccctgcagcagcacccagatcacgccgcctatcagcgaccagttcaggcaggacatggccagctggagcagcgccatgcgcagcgacggaaccttgaacgaatggcggtgaatacgaaagacgtgtccgctggcgaaggcgcacagcaccaggtacgccgcggccaccagcagcagcacggcgccgaggatgcgcaggcccgcgttatcgatcttccagtcggccggcagcaccagcggccagacgcagaagaccgcgccagccaccaccaggtaaccgagccagttggtcagcatgctgaaacccagcacgcgggtgatggtgccgttggagagttccagccgcgagtagagccggtagcgaaacgccacgccgccaaccagcgaacccaggttgaggttgaaggcgtagctgatgaaggtcacccccatcacgatgccggcactcagcgggtgccgcgtgagatgccggcccaggaggtcataggtgctgtagagcgcaaaactgctggcggccagcgcgcccgccagcagcagcgtggccccgggaagcgcgcgcacggcgtcgaacacctcttgccagtcgatggcgcgcgcctggttcacgagcagccaggcgatcaggccgaaaaaagcccaggccgcgatccggcgcgcccagggccaccagggccggtgcgcaagccgtgcaatatgggtgctcatgccacttccgtcggcgtcacggcgtcgtcgccgtttttcttgtccgtctcgcgtcgttcgcgcctttcggccaggacaatggcctcggcgggcgtcaggcgcggcacctggcgcggcagccagccgagccaggagggataccagcgcaagaagtgaaagatgaagaagctgcgcaccagccgccagccgctccattcgttctcgaggtcggcggggccgatctgcttgcagctcttgcacatgagcgtgtccatgcgctcccacagcagctggttgaaagccttgtcgcgtgcgatcacgttggcttcgaggttgagcgacaggctcagcggatcgagattgctcgagcccactgtggtccaacggtcgtccatcagcgcgatcttcgcgtgcagcgggcgttcgcagtactcatagatgcgcacgcctgaatgcatcaggtggtggtagagcatgctcgcggccgtcttgacgatcggcatgtcgggctcgccctgcagaatgagccgcacgtccacgccgcgccgcgccgcgcggcgcagttccttgatgagccggtagcccggaaagaaatacgcattggcaatcacgatgcgctggcgcgcggcgcggatcgcgatcaggtactggcgctcgatgtcgccggtgtggcgccggttgtcgcgcgtgacgaacatcgcctccacttggccaaccgcttcccggtcggccggcggggcttgcttgaggcggcgccggaaccagcgcggccccttgtcgccgagcgcgatggcacgcagcacgaactgatggatctgcgccacgatgggcccacggagttccaccgcgtagtcctgcttggccttgggcccgaagtcgagcagatggtcggccgaatagttgatgcccccgacgaatgcaagctcgccgtccaccaccacgatcttgcggtgcatgcgccggaacacgttgagtcgctggccgaggatgcgcttgccgtgatcgaacacccgcgtcctcacgcccaccgaactcagcccttcgatgaattcgcgcgaaagatcgggcgagccgaatccgtcgaccagcatgtcgatcttgacgccgcgctgggccgcggcacgcatggcggcgtgcagcgccaggcccaccttgtcctcgaacaggatgaaggtctcgatgatgacttcgcgctttgcctcgcggatggcgtcgaacacgcgcgcaaagtactcctcgccgttttcgagcagcgcaatgcaattgccaccgatccagcggtcgccgttatccatggcagccaccttcagtgcccgccggggcgggcgatggaagtcgcggcgcgaaatgaactgcgcggagcatgggcgtagtccatcttcaaaggtcgatgttcgccaccagcggcgcatggtccgacaggtgcgaccagggcttgcgcggcagcaccaccggttcatgcacgcccgcattccgaacgtagatgcggtccagcggcagcagcggaaagcgcgacggaaaagtcttggcggccgcgccgttcgcatgcaggaacacctcgcgcagcgcggcgccttcttcgagcacccggtgcgcgcggccgcgccagtcgttgaagtcgcccgccacgatcagcggcgcgtcggccggcacctcgtcgcgcacgatgtggcagagcagctccagctgctgctgtcgatgcgtctcggccaggcccagatgggcacagatcgcatgcacgtcgaccgtgcggcccggcaggcgcaacacgcaatgaagcaagccgcgcttttcggggccggccaccgacacgtcgtggttgcggtaatgcacgatcggaaacttcgacaacagcgcgttgccgtgatgccccctcggatacaccgcgttgcgcccgtaggcgaactgcggccacatggtgtcggccaggaattcgtagtgcggcgcctccggccagttgttgaccttgcgcgagtggcgcgaatgagtgccgagcacctcctgcagaaagaccacgtcggcccccacggtgcgcaccgcgtcccgaagctccggaagaatgaacttgcggttgagcgcggtgaaccccttgtgggtgttcaccgtcatgaccttgagcgaggtcggcgccgctgcggggaggggaatcggggaagaagacatcgatgctgtggttgtacgttgccgcgccgccggcgcctgtaggaacgcgccaccttcttctccacctttcgcaacagggcggccggctcctacaggcaggcctgccgcaccccgacatggccggcatcccgggcctcctacggtgggatttcaggccgaagaaaacggcccgtccgtcaatcgttcaccgatctctcgagacaagcaaaggaaaccaccatgaagcaaggaatctttcacgccacgctgctggccggcctgatggccacggccggcgccgccatggcgcaagccacctcgatacccgcccagcccgacccgtccgtgggcggccaggccagcacgcagacaccctccggcgtgcctaacccgccgcagcgtccggacaccagcatgccggcttcgcgcgaagccgtgaaggccgaagcgcgcgcccacaaccgcaacaacatcaacaacccggtgccgaagggcgaggccagcaccaccgtgaacgcccaacccaacgccatgccgcaacccacgggcgagatgtcgcgtgccgaagtgagccagcaggcccgcaagaccaagccccggttcggccagccgggcgaacggccggacgtgccgacgaatccgacggaaaggaccggcacacctcaataaacccgcgtactaacccacgtacgtagaaaacgtaaaaagcccgcgatgcacgaggcatcgcgggctttttatcgtttgcgccgttcagcgcgccgttcgctcagctcttggtgggcgctgccgaatggtggccgtcgggaccaccgtggccatggtggccatggtggccgcgatgcccgtgcatgcccacatgcaccgtttccgcgtcgaaggtcttcttctgctcgggcgtcagcgccgcatagaaggtcttggtggcttcagcgcgcttggcgaaccttgcgctgcgttcggcctggcgggcctgcatgcgctccaggcgctcgggcgtggtcagcttggcaaattccgcgcggtccatgcgcggggggcgggcgccggccggcggctggctggccgatgcgaaagtgctccacgcgctttcctgtgcggcagtcagcttgagcttttccttcagtgcggcaaggcgcttggcgcgatgttcctgcatgcgctgcatgcgctcggccgggtccatgcgcttgttgtgctgcgccttgtttccggcggcaccatcggcctgggcgacggccgcgggcggggtcgaagaggtgctgggtgcggccggtgcctgggcgaaggcgcccgaagaggcgagggcggccgatccgagaaggctggcccagacgatgcgttggcgaagagagatcatgaaaagtgcttcctttcgaagaagcccgctgccaaggggcagcaggtgaagcgaagtgtggaagacctctgtatcgcccaggtgagccgacagtgagcgtgcgtaaagaatcatgaacagccagggctcgcgccgcccgcggcgtggcttatttcggccttggaggcttcagcccgcgatcgggtgcctgcagcttgcccgcccgcagctcgccgactgccagtgccactgcccgggccgcgttgcgcacttcttcctgcacgtcttcgtcggcgtcgaggctgtcgtggctgcttgcatagggctcgtagtagccgatgtagcggtcgagccgggcctgcgtgcccgcatcgatcaggcccatccagtcgagccagtccgacagattgcggcgcaggctctcgacgccggccacgtcgccgtgcaccaccacgccgtaaacccggccgctcaggtgcttggggtagccccagccttcgagctcgagggccttggcttcgtcaggcttcttgccgtgggtgctggtggggtcggggttgccgccatcggcgcacaccagccggtcggccatgagcttgagcgggctcgcggactggtaccagtgggtgggcgtgaacagcatcacgccgtgcgcggcaacccagcgctcgtagatctcgttcatccagtcgccggtctggcgcaacgaatgattgggatagcaactgcagggccagtggcacagcggcatggcggtggaaacgcaacccttgcagggatggatttgccggccgtattcggaggtgagcaggctcaggtcgagcacgtcgacgtcgatgccgcagccgtcgagcacctcgcgcgcaagctgcaccaagcgccaggtcttggaaatttcgccgggacaggtgccgtcgttgcgcggcgagccattgaccagcagcacgcgcgaccgcgtctgcgggttgccccaggcggcctctgccgcgtcgatgcgggccttggcctcgagccagtcaactgaaagttcgtactcgggatcggcatagccggggccggccttgcgcgtgaccggcgccttgcgcccttcctggtaagcctcccaggcaatgagctcgatgcgctgcaacgactctttctcggcctcgaaggccgggtcctggaacgactgcatgaagcgctcgtggaaccggtcgcgctgcaacgtttcgggcgcctgtcctttgcggacccggggcgctttggaggtgctggacgtgctggacgtgcgaaaaggcatggcgccaatctatgcgccgcattgccgcccgtgacctgcgcgcggcgccgattttcggtaggcctgcgactacatgccgaacttgccgttctggaaatcgtgcaccgcctgcttcacttcttcctgcgtgttcatcacgaaggggccgtactgcgcaatcggttcgcgcagcggcctgccggcaatcaacagcgcacgtgccgggctgtggttggtggcgcctgcgcgcagcaccacgccgtcgctgccgggctcgttcgcaagaatggccatgcggcgcgtcggcacctcgctgcccgagatccacaccgattcgcggaacacgtacaccagcgcgttgtgatcgtccggcaggggctgcgcaaactcggcgcccggcggcagggcgatgtcgagatacagcggctccgagtcctcgcgccgcaccgcgccctcgatgccgtggctggcgccggcgatcacgcgcacctgcacgcccgcggcggtggtgtattccggaatttcctcgctctggatgtcgcgataccagggctcgcgcatcttgtccttcgcggggaggttgagccagagctgaaagccttccatgaggccgtcttcctgttccggcagttcgctgtggatgagcccgcggccggccgtcatccactgcacgccgccgttttgcagcaagccctcgtggcccgcgctgtcgcggtggcgcatgcggcccgcgatcatgtaggtcacggtttcgaagccccggtgcggatggttgggaaagccgccgatgtagtcgcccgcgttgtcgctgccgaaggcatcgagcatcaggtaggggtcgagccttttctgcagcggctgctgcagcacacgggtgagtttgacgccgtcgccatcgctggtggatacaccggccacgatgtggtcgatgccgcgcggcgtggcgacgggatcggtggggtggttggcatgatgatttgcgttcgtcatgcagccatggtggcactaacgccgcaaccgcaccaccggtgggggtgtggctttcaggggtgtgtggctttcaggtgggcgccgtcaccgcggccactgctgccgctgccagtagcggtactgccactgggtggaaaaaccggcccgccggtagagcgcatgggccgcgaggttgtgcgcatcgacctgcaggaagacgcgctcgaagccgcgctcgagcgcggcctgcgccatgcccgcgagcactcgccccgccaggcccctgccacgctgcgactgctcggtgcgcatgccgtgcacgctggcccatccatggctgaaggccatggcgcccgcggccacggtgcgccggccttcgcgcacgctggcatagagcgaccccttggcacgcgacagggcccgcacgcgatgcgcgccatccaccggatcgaagccctcgccgagaaacagcgtcgcccaggcctcgtcgggcgcaaggtcgacctcggccagcgcggcgtcggccgctgccacctcgcgcatgcgctgcgcggagccgatctgtacgcaggtcggcgaatcgccgacgtagtgccgctgctccagctcggtttgcagcgcagcaaagcaaggaaggtcggcaagccggaaggcgggcacgaactgccggctgtcgtagcggtcttcgatgcggtcgatcgtgtggtcgctgacctcgccgcggtgcaacggcaccgccgacctggcgcgcttgacggtgccgtcgtcgaagggcagcagccagccgtcgagttcttcgacggcaaggggagacacggcggcgaccgtggcgcgctcgatggcctcgacatcgttcatggcgccgcctcgggcgccgtgaaccgggccgccgccacgctcttgagcaaggcctcgcgctggttgcggctgatgccgcgcacgctctcggccacccacttggttcggtcgggatcgatgcggccgtcgtgccgccattgctcgagcaccgcctgtggcttgtgcagcatggccgcgagccatacggcctgcgcgggttccaggttgcgcgccgggcgcttgaaatatcgccgcgcggcggcttcggcaccgcacaggctgccgccccagggcgcgttgtcgaggtaaagctgcaggatgcgcgccttgccgagcgtctgttccatttcgaccgcgtagagcagctcgcgcagcttgcgctcggcggttcggtcgctgccggtcaccagcatcttggcgagctgctgggtcagcgtgctggcgccgcgcttctgctggccgtccttctggttgttgtcgatcgacgcgacgatttcggtcaggtcgtagccggcgtgggtgaagaagcgctgatcctcggccgcgatgaccgcccgcgtcagccagctgtcgttggccagcttcgacggcgcgccgcagctggtgcgcgcgccgagcatggcttcggtgcccagcccttcgacggtgaactggctgacggtgggaatcacgacgaacgtggcttcgggcagcgccacctggccgcgcaacgccagcgtgccgccgatgcgggcgcgctgcagttcgggcaggttgggcgcgagcaccgcataccagcgggcgatgggcgcgtccttgatgtcggcgctgaggtgcatgcccttgggcgaaaggcgcccttcccattggccctggatcacggcggcggcatcggcagtgcggggcgtggccgcgagggtaccggacagcgtgttgccgtcgcgcctgacggtggcgatcaggccttcgacctggatcggctgcgtgccgagcgccgggacatccacgctgcagggtgcgcagcgcatctcgagcaggccctccgcgtccttccaggcgaaatggatcgtgccgaaacgcgtgtccagagcgtggccatgaagccgcggcgcaagccacgacgaagtggccaggcgcaccgccgtgggcacgccgacttgaaagctcagcgggccggccttgacggtggtgctccactcgcccgccgcgggtgcaagcgcgaacctggctatcagaaagatggccaggccggctgtcaccaccacggccgacagcgcatagatcacgaatctcagggtcttgttcacacaactctcacaagggtctcgccaccgtgacggcttgccacggaccgcgcgactgcccgctggctgccgcccagtaccaagctgaagtgtcggtgaaagcggcgccttcggcatcgacgatgcgctcgcaaacgcggaactttttcacaccgtgccgttgcgcaacaaagcagcgccacagacgtgcctgcgcgtcgcgttccaggcgcgcctgctcgatgcgaaaacccagcgcgcggtagcagtcggccgccggatgcagcatgcgcgtgggtgcgtccaccgcgcgcatcacgatcgtctgcgtgccgtcggtcatgcggccgatggcacccggaaaacggtcggcaaagcgctgctcgacctcgctcagcgccatcgggcgcagcggcgcgccatcccattcgcgcggccattcgtgcgacgccacggccgccaccggccccggcggcgaacgcagggccgcagcggtcgaccacagcagacacagcagcatcgcgagcgcgaacgccgccttgtggccgatgcgattgatgaagtggttagcgaaaaagttttcaaagaaccgtgtcgacatggcggcctccttgcgcggtgatcaggcccggaatgggctggtcggcaaatccgggcgccgtgcgcgccggcaccatcaggcgggcgatgccgccgcacaccacagccagcaccagcaggccgagcaggttgtgcgcccagggcgccagcggatggcccgcgccttcgaatgcaatcagcacgctgttgcgcaggatgttgcctgccagcaccagcagcccgaccatcggcagccggcgcagaaagccgccgtcgctgcggcgcgcccagagcgccaccgcgcacgcagtgaagtagccgagccacaccatctgcacgcccgagcacggcgcatcgacgatgaccagccggccatcgaccagcaggctgcttccctcgcgcgccacgctgaagcccggcgccagcagccagcggctcgcctcggccgtgaccacgcgcagcggatagcccgcatagaactgcagcgacgacaacagcggcaaggccagcaccgcaagccccacgaccggcaacgcggccacgcgccgcggcaggaaggcgagcaagccgcacgccagcgccagcaccgccaccaggcccgccgcgagcgggggcagggcgggcagcgccccaagccccgtgcgcagcagcgtggccagcaaggtgccggcccccgccagggccagccagcccagccgcggcgcggcgcgcaattcgcgccgccattgccacgccagcgcggccaacgcagccagcgccaggaggcccagcgggtcgtcggagccgtcgcgcatgcgccggaccatccaggcccaggtcggtgccagtgcggcgaattgcagcgcaagccagccggcggccggtgcgcggtcgatgcggatgccccaatccacgatgcgcggatggcgatgggcaagtacggccagtgacatttgtttttcctttttcttttgcgttcaggccgtgaagcggcgcgggtcgttgcgccgcgcgcggcggcgcagcatggcgagcatcgacagcaccacggcaatggcgcccagcgtttcgggctccggcgtgctcggcacctcggcgccgagtgcgagttcgctcacgccctgcggcaagggcagcggctggttcacgtccacgctgttctgcggcgcgaggttgcgcaccaccttgtccacggcgatgaagctggtgtactgcgtcagcaggctgtacttcaggccgagttcggtgatgcgctccttgaaagcgccgccgccctcgagcgtctcctggtcgcggaggctctcgatgcggtggcgtgcccacagcgtgcgcagcgcggcggtgtcctggcgcatctgcgggtcgatgcgcagctcctggcgatacgggccgttggcgccgtggccttcgacgatcacgcggcccctggcctttccttcggcatccgcgcgccacttgccgaacacgatcaccgggcgttcgccgagcacgtcgggcagggcttgcggctccacgtcgtatacgtcgaggccgccgaaagtgaccttcacgttggtgagcaccggcgactccaccatgcggcggaaacgcgcggcctgctcgggcgcctggatcgggtcggtgatgatgaagggctcgcccatgccggcgcgcgcaatgccttccatcaggctgcggttcaccgacgagccgatgccgaaggcgaacacgttggccttcgacaggttcttgcgcaccagctcgaaagcctcgcgctccacgctcacgtagccgtccgtcaccagcaccacggtgcgcgacacgttctcttccttcggctcggcatagacgcgcttgagcgcggggatcagctcggtgctgccgctgccgccgtagttctggatggtggcgagcgcctgctcgatgttggcgcgcgtggccggcaccgattggggcgagagcatcttgttgctgcccgagaacagcagcacgttgaaggtgtcgctcggacgcagcccgccgatcaggcgttcgagcacggtcttcgcggtgtcgagcggaaagccgtgcatcgatcccgagatgtcgaccacgaagatgtagtcgcgcggcgaaatggcgttggcggccacggccttgggcggctcgaccatcgcgagaaagaagttctccgtgctcccatcggtgttctggcccttgtagagcatcaggcccgattcgatcttttcgccagcaaggcgatagtcgagcacgaagtcgcggttgtccgcggggcggccgtcagccgcgagcaccacgtcggcatgccggtcttcatcgctcttcttcacgtcgatggcgtgggtgttcgagcgaacctccttcaggcccatgggcgtgtcgatgctggccttgagcctgaagctggtgccgggcgccacgcccgcgcgcagcgtgggctgggccacccacttggcctgggcgttttccgactgcgggctgttgtagcgcgggcccaccacggtgggaaacacgaacgcgtagttgcccgattgcggcaccaggagctcggtgtagcgcagttccaccctcacgtcgtcgcccggcaggatgttggcgacgttcatctggaacacgttgggcaggtgctgctcgagcagcgcggcggtcttgccttccttcttcgcggtgtcgtattcgatctgcgcctgctgcttctcgcggatctgcgcggtgatcaggcggtcggccaggcgcacgttgagaccgctgaccgcggccttggtcgagcccggaaaaacatacttcgcttcgatcgcgcgctggccctcgttgcggtaggtctgcgtgaccgtcacgtcggcaatgacgcccgagatcttcaccgccacctcggttcccttgagcggcaagcggtcgaccgaggggtcgtcgctcttcacgaagaagtaagggctctcggtcttcagccgcgggccgggtgcttcctgtgcatgcacggggttgaggctgagcgcgacgaagcccgcggtggccaggctcacggtggcgagccagagccagcggccgggacgggaggtggtgtgggcatccatggcggtggtgtcggtgtccgtgcgaacttgcacagccgcaactgtcaccgccgcgcgagaaggaaattggaaggctgcttgaagtccgcctgccggacgcagccttgtgtgaagcctgtgtgaagtccgccgccggccacgcttcacacggccttcggatcgcacggcgagcatcacggcttcgctatcgaagaggagaaaaaaacatgtttcagttgttcaaggccttgcagggttcgatgctggtcaaggtcgccggcctgctcatgctcacgctcctgctgtgcattccattggccgagatcaactcgatcaaccgcgagcgcggccacagccagcgcgaggcggccgaggagcttgccgccacctacgcgagcgggcagaccatggtgggcccgctgctgctggtgccctatgtggaacgctggatggagccgctgcgcaatgcgcaaggcaaggtgatcggccaggaggcgcgcagcaaggaaatggcccacgcggtgtttcccgacaagctgcacatcgaaggttcgatggcgccgcacgagcgctatcgcggcatcttcaggattccgttctacacgctcaacgccacgctcggcggcggttttgcggccttcgaccccaagtccgtggcgcacagcgaagccgattcccgcatcgagttcaaggcacctttcgtcgtcttctacgtgagcgatctgcgcgggctcgacggttcgccttccatcgcgatgaacggcgagggcctgcgtttcaagcagcgcgtgcccggcctggcggacagcagctggctggccgatggggtccacgcaccgctcaccggcgccgcgctcgccgcatgggaatccaaggcgccgctgcccttcgagatgaagctcggccttgtcggacaagacacgctctcgatggtgccgattgccgaagagaccaccgcccacctgagctcgccgtgggcgcatccgagtttcggcggccgctttctcgccgcgaagcgcgaagtgaccccgcagggtttcgatgcgcactggcgcgtgtcgtcgctggtgacctcggcgcgcgagcaagtgcgcgccggactgtcggaccgcgatgatcgcagcgctgctgccgccgccacggccgccgcagcaaccgtcggccatgcgccacgcaacctcggcccgctgcagaccttcgacgtgtcgctcgcccaaccgatcaacgtgtattcgatgagcacgcgcgccggcaagtacggcgcgctcttcatcggcctggtgatcatggcggccttcatgttcgagctgttccgcaggcagcgcatgcatccggtgcaatacgggctggtcggactttcgatcgcgctgttcttcctgctgctgctggccctgtccgagaagctggctttctggctggcctatgccagcgcggccgcagcgagcgtgctgctgctgggtatctacttcagcgctgttttgcaaagctggaaacgcggcgccggttttggggcctatgtcgcggtactctatggcgcgctctacggcctgctggcatcggaaagcaacgcgctcctgcttggcgccctgctgacattcggcatgctgacggttctgatgctcgccacgcgcaaggtcgactggtatgcgctgtcgggcgggaacccccgaacgcccgagccggtcttacccgagtcggccgcttccgtgtaacggacgctaccgactgttttcttacttactgatttccatggacgattcctctcattccaccgacccggcgcgctccgagcgatcgatgcggctgcggcgcattgcacggtggagcgccatcgtgctcggctccggggcggtggtgctgctggtcgccgccgtcgtggcggtggccgccatctatccgcgcttgcccgacatctcggaacttgccgactaccggcccaagctgccgctgcgtgtgtattcggtcgaaggcacgctcatcggcgagttcggcgaggagcgccgcaccctcacgccctttgccagcattcccaaggtcatgaaggacgccgtgctggccgtggaagacgcgcgcttctacgaccatggcggtgtcgactacaagggcttcgcgcgcgcggcggtggccagcctgaagggcggccggaagcagggcgcctcgaccatcaccatgcaggtggcccgcaatgtgtacctcagttcggagcgcacgctgagccgcaaggcctatgaaatattgctggcactgcggctggagcagcaactcaccaaggaccagatcctggagatctacctgaaccagatctatctgggcaaccgcgcgtatggttttgccgcggcctccgaggcgtacttcggcaagccgctgcacaacatcaccacggccgaagccgcaatgctggccggcctgccgaaggcgcccggcgcaaacaacccggtggccaacccccgccgtgcccgcgcgcgccagctctacgtgatcgaccgcatgcaggaaaccggcttcatcaccgccgagcaggcggccgaggccaagaaggaagaactccacctgcgcgatgccgccgacccgaaccggctgcatgccgaatacgtggccgagacggtgcgccagatgatgtatgcgcagtacggcgacagcatctacaccagcggcatgaaggtctacacctcgctggtcgcggccgaccaggcggcggcctacaggtcgcttcgcaagggcatcatggactacgagcggcgccagccttatcgcgggcccgagcgtttcgtcgatctgccgaccgatcaaaaggaagccgacgaggcggtggacgacgcactggccgaacaccccgacaacggcgacgtgatggcggccgtggtgctggaggccaacagcaaggaaatcaacgcggtgcgtgcgaacggcgaagccgtgcagatcaccggcgagggcctcaggcccgcgcaatcgggcctcgcggccaaggcaccggcgaacatcaagatccgtcgcggtgcggtgatccgcgtggcgaggacacccaagaacacctgggagatcacgcagctgccggaggtcgagggagcgttcatcagcatggacccgcgcaccggcgccatcaagtcgctggtgggcgggttcgatttcggcaagaacaagttcaaccacgtcacccaggcctggcgccagccggggtcgagcttcaagcccttcatctattcggccgcgctcgagaagggcttcacgccggccaccatcgtgaacgacgcgccgttgttcttcgagcccagcacgcccggcggccagccctgggaaccaaagaacttcgatggtggcttcgaaggtccgatgccgctgcgcacggccctgatgaagtcgaagaacctggtgacggtccggctgctgcagtccatcggcgcgccgtatgcgcaagactggatcaccaggttcggcttcgacaaggacaagcacccggcctacctgccgatggcgcttggcgcgggctcggtcacgccgatgcagatggccaccgcctattcggtgttcgccaatggcggctacaaggtcaatccctatctcgtcacgcgcgtgaccgacctgcgggacaaggtgctgctcgaaaccgagcccccggtgctcgacgaaacccgccgcgccattccccagcgcaacgccttcatcatggattcgctgctgcagagcgtggtgaagggcggcaccgcctcgcgcgcctaccaggcactcaagcgcgacgacctgttcggcaagaccggcaccaccaacgattcgttcgacacctggttcgcgggcttccagcccacgaacgtcggcattgcatggatcggctacgacacgccgcgccagctgggcgtgcgcggcgaaaccggcggcagcctgagcctgccgatctggatcggctacatgcaggcggcgctcaagggcgtgcccgtcagccagattccggagccgccgggcgtcatccacatcgacggcgagtggtacttcgacgatttcgcgccgggacgcggcgtcgcgagcctgggcgtcgagaacgccgagtcgccgccaccatcggccgaagaactctcgggcgtgccgctgggcccgccgccgcagccggaagagcgcaaccgcatcctcgatttcttccgctaggggcattgcgaaagcggaggcgggtctccggtgcctacactcggtgctgcccgccgctttcaccttcccttctccacgccctcatggaaattcttaccctggtgacgctgatcgtcatcggcgcctacatcctcaagtcacgggaccagcgccagcgcatcgcgctgctcgggagccatctcggcaagtaccagatcgaaaacctgatggagaccctcaccgagggctacctgcgctgcctcggcgaggacgacgccgcgcggcgccagcagatctggagcctgctcgattcgaccgaggaaaagctctcggcccagttcgacagctttgccgcggagttcgcgcgcgtcgatgcggcggaagcgcgcgtgagcaagctgccgctggccgttccgtttgcgcacaagctgtttccggccgccactttcgactttcgccaggcccttgccattcatgcgcgcggcattgccgaggtgatgcggaacgaatcgggccgcacccccaaggccaaggccttcacgatgtcggccgagctgttcctgatgcagcacacctgccactggttctgcaagtcgaaggctgtggcgtcggcgcggatgctggcgcggcacaagacctcgtacgagcaattgctcgatgccgtgagcccaggaacgcgcaaggcctacggcgccctcaccggatcttgagggtcgcatgcccgcaggtctcgatcaccatcgtgtccatgccgagcaagcagacttcgtcctcgaaggcgacgttcttttcgcccccggaaagtcgctctggttttcgggcatgggcggtgcggcgctgctcggcggtgggctgttcttccgctgggatgcactggcgcttttcgtcttcagcaccggtttcgtgctgctctttggccattccctgggcagtcatcggcaactgattcaccacagcttcaagtgccaccgatggttgcgctgcacgctggtttactgcggggttctggtcggccttgcggggccgcttggcatccttcgccagcacgaactgcgcgactatgcgcagcgccttacctcatgccatgactacctgcgccacggccgtggtttctggaccgacgcgtggtggcagctgcattgcgagttgcatttgcaccggcctccgctcatcgagatcgaggcgctcattgcgaacgaccgcttcctgaggtggctggaaaaaacctggatgctgcagcaactgccgcccgcacttcttttctacctgtggggcggctggtcgtttgtattctggggcgtctgcgcacgtgtcttcgccggtgtgctcgggcattggttgattggctggttcgcgcacaaccgcggcgcgatgaactacgaagtgcgcggggccgccgtgcaaggtcggaacatcccctggacctcgctgctgacgatgggcgagagctggcacaacaaccaccatgcctttccaggatctgcccggctgggcctggcgcctggtgaatgggaccccgggtggtggatgcttagattgctcgagcgctgcggcctggtgtgggaactgcgcttgccagattcgctcccgccgcgccccgaactcgcagtgctcaaggccgttcagtgatgcgacggcggcagcagcggcagcgtgagcgtggccaccgcgccgccgcgcgccgcattgccgagctcgatgcggccgcggtgcagcgcggcaatctctttcacgaaggccagcccgagcccggtgctcttcttctggctgtgcggccgcgccagcgaatagaacttctggaagactttttcctgtgcgtagtccggaatgcccgggccgcggtcgcgcacgctcacgcgcgcaagcttcgaggtggtctccagcgtcagcagcacctcgctgtcccgcggtgaaaaatcgatggcgttgtccagcaggttgctgatggctcggcgcagcaggaatgggtcgccctccgtgctggcctcggtgcggatgttcactttcacgccgatgttgcgtttggccgcggcgggctgcgcgctgatggcaatgtcctcgatcagcgaagccagcgccaccggttccgtgcggtcgaggccgcggcgggtttccagcgcggtgagttccatcatgcggtcgacgatttcctggatgcgctgcgtctcgcgttcgatgttcttcaggaagcgctcgcgctccgcgtgaggcatcgacggttcctgcagcagctcggctgcgccacgaatcgccgacagcgggctcttcacttcgtgcgtgaaagtctgcacgtagtcggccacgtagttgcggccggtgagcgcatctcgcatctcgctgaagccggtgcgcaccgcatcgactgcgcgccgcgccatgcgtgaaaggctcagggtgcgctgcgcgcgcacccaggtccagtagtccgaaatcaacccgaagggtcgcaccagccagaccgagacgatcaacgccagcagcagcagtgcgaggcccgaacccacgcccacccagagcgtgcgggcgcgcgcgtcttccacgaactgcccgaagctctgcaccggcttgccgacgctgaccatgccgacgatctcgttgttccagcgaatcggcgcacccacgtacatcaccgaggtgcgcgggtcgccgtccacgtcgcgcgaagtgcgcgcgccgtagatgcctgcaagcgtgcggttcacgtcgctccactgcgagtagtcggcgcccaggtgcctgccgagcgaatcgaacaccacgcggccgctgcggtcggtcacgtacacgcgcagctcgacgcggttcttgtgcaggttgtagatctgggccgagaactcgcgcgcatagaccgtgcggaacagcggctcgagccgcgcggtggtgatggcgcctgcgatcacgtcctgctcgaccaggctcgcgatgagctgcgaggtctcgaccagcgattcttcggccgattcgcggtagcgtggatcgatgtccgacaccacgcggtacagcaggaacgcgatgcccgccgtgtagatcagcaagatgccgatgaatatccgcgtgcgccggctcacggcacgctgtggggcagttcttcgttcaatgcgtagccggtgccacgcagcgtgcggatcggctccacgtcgggcgccacggccttgagcttggcgcgcagggttttcacgtgcgcatcgaccgtgcggtcgaagctgtcgctcgcatcgtcccagaccagttgcagcagttcgtcgcgcgtgaagacgcgtccgggtcgctgcaccaggagccggagcaggccgtattcgtagcgcgagagttcgagcaggcgaccgtagtagcggatctgcatgcgctcgttgtccagcgcaaacggcattgcggggggctgagagctcgctggagccgtcgcacccggaatttgagggggtaccccgttgttcgtgcccacgggccctccaggggccgctcgcgcgctgcgccggaggatggtgcgcacccgcgccaccagttcgcgcggcgaaaagggcttggcgatgtagtcgtcggcaccgagttccagccccaccacgcggtcgatctcgtcgcttctcgcggtgagaaacagcatcggcacctcggcgccgccctgcgactggttcagcgcgcgcaggcgcttgaagagctcgaaaccgttcaggtccggcaggcccacgtccaggatggccagcgccggcggctcctgcgcgaactccgcgatggcttcctcggcggtggcgcaccacaccggcgtgaagccgtcgctcttcaggacgtattggagggtgtcggcaatgcccgattcgtcttcggcgatcaggatccggggtttgaaactcatccccggatgttagcgagagggcgctgttcggcgaggctggttttcgtgcgtggcgccgcgaacacggcgcggccgttcgcggcctttttttcgggcgcggcgctggattcctatcttcttcttattcttcttattcaaattagtagtagtagataagggttgccccggtctgtggacatggcaatttttcccttgcgtgacagtcacttgtcatacctctgtcactgtgcgcagctgtgcttccgagctgtcgcgccaaaagggacaacattggccggccgctctgccctgtggataacaccctgcttgtgccggaactctccccagagttgtcctttgacaccgtcctctaaatctgcgaaaggcggttttcagcgcgagaaattcattgcctgatatttgggcagactgtagatttccatttcaaatcaacgacttggcgcacccttacaaggaagtgcgagtgttatccacagagttgcccaagctttgtggggagaacccgcggcggaaccttcgcgcgcgatgtcgaacgaactttgtccttcaaccttaggaaattcgaacgtgaccccttccgaaaccaaggccatcgtgacgctgagcttgctggccgccttcgtcgacggtgaaaaacacgagcgcgaacgcgccgagatcaagcgcattgccgagggcctgtcgcaagccgacggcgtgaacctccccacgctctaccaggacgtgctgatgaagcgcgtctcgatggcttccgtggcgggcgaactgcaaagcaccgattcgaagcagctggcctatgaaatggcggtatgcgtgtgcgatgccgacggcacccagtcggaagcggagcgcatgttcctgacggacctgcgcacgtcgctcgggctcgatgcctcggcggcgcagttttcgcgccaggcggaagacattgcggcggctgttcccgtggcggccaccggtgcagccgcggcatcgacggccgccgcggtgccatcccccgacagcgcggagctcgacaagtcgatcctcaacgcagccatcctcaatggcgcgctcgaactgctgcccgaaacgctgtcgaccatggcgatcattccgctgcagatgaaactggtctatcgcatcggcaaggcccatggctacgagctcgacagcggccatgtgaaagatttcctggccacggtcggtgtgggcctgacctcgcaatacctggaacaggccgggcgcaagctgctcggcggcctgctcggaaagatgggcggcggcttgctgcgcggccttggcaaccaggccgtgagctcgggcatgagcttcgcctcgacctatgcgctggggcacgtggccaagcgctactacgcgggcggccgcacgctctcgacgcagatgctcaaggacagcttctcgaacgtggtgcaggaaggaaagagcctgcagacgcagtacctgccggccatccaggaaaaggcccgcaccctcgatgccggcaaggtgctgtcgctggtcaggggcgcctgaggcagatcaggccgcggccaggtcgtcgagaatggggcagtcggggcgcgcatccccgtggcagcagtgcaccaggtgcgccagcgtgttgcgcatcgactgcatgtctgcaatgcgctgttccagttcatggagatgcttctgcgcgatgcgcttcacgttcgagctcgcacggcggcggttgtgccacagccccacgagctcggcaatttcttccatcgagaaaccgagatcgcgcgagcgcttgatgaagcgcagcgtgtggatgtcggcatcgccgtactggcggtaaccgctttcggtgcgcgccaccgcgggcagcaggccgagtccctcgtagtgccgcaccatgcgcgccgacacgcccgaaagccgcgccgcttcgccgatggtcacggtgccgaagctgctcattggaccctgtagccggcgttctcgatagcggcgacgatgtcttgccgaggttgcgcgctcaatacgtcgacatgccctgtttcgagatccaccgtcacctgcgcttccggatcgaccgtctggaccgcgttttgaaccgcgctcacgcagtggccgcagctcatccccgagacctggaatttctggctcatcgttgttgctcctgttgaatgaatgatgggagacacaagtttgaaccctctcacgatgtcaatgtccagcgcaggggcactcggcatcgaggcttgaccttgccatgatgtgaggctttagcctcgcggcatggaaaatctgctgcactctccgcaccacccaatgagcaccctggatctttctgttggcggcatgacctgcgcctcgtgcgtggcacgcgtggaacgcgcgctcaagagcgtaccgggcgtgcaggacgtcagcgtgaaccttgccaccgaatcggcgcgcgtggtggcggccgacggcgaagacatcgacgtacgcctgcgccgcgccgtgcgtgccgcgggctacgagccgcgcgttgcaagcgatgtggccgacgaggccgcggcactgtcgccgtggcagggattcgggccggtcggcatcggcctcttgctgtcgatccccttgctggcgccgatgctcggacaacccttcgggcaggactggatgctttcaccctgggtccagctgctgctggcggcaccggtgcagttctggctcggtgcgcgcttctaccgcgcgggctggcatgccgcgaaggcgcgcaccggcaacatggatctgctggtggcgctcggcaccagcgcggccttcgggttgtcgctctggctctggtggcgcgcggcaaccggcgagcacgcggggcacggcgcggtgccgcacctctacttcgaagcgtcggccgtggtcatcacgctggtgatgctcggaaagtggctggaggcgcgcgccaagcggcaagccacttcggccatccgcgcgctgcagcagttgcggcctgaaattgcgcacctggtgggcaagcgcagcgaaagcgatgtgcccatcggcgaggtgatggtcggcgacctgctcgcggttcgccccggcgaacgcgtgccggccgatgcgcgcgtggtcgagggagagtccgaagtcgatgaatcgatgctcaccggcgagccgctgccggtgcccaagagaccgggcgatgcactgacgggtggcgcagtcaatggcgacggccgcatggtcgtcgaggtgaaagcggttggcgccgaaagcgtgctggcgcgcatcatccgcctggtcgaggacgcgcaggcggccaaggcgccgatccagcggctggtcgaccaggtggcagctgtgttcgtgccggtggtgctggtgattgcgctggccgcgctggcgggctggctgctcgcgggcgccggtatcgaagttgccatgatccatgcggtggccgtgctggtcattgcctgcccctgtgcgctgggccttgcaacgccggtggcggtgatggccggcaccggtgtcgcggcgcgccgcggcatcctgatcaaggacgcacgtgcgctggaagtcgcgcaccgcgtcgacaccgtggccttcgacaagaccggtacgttgacactgggccggccggtgctcacggcgctcgtgcctcttgtgcttcttgcaaccaacgaagacgaagaccgattgcttgccacggctgccagcctgcaaggcggcagcgagcatccgctggcccgtgccgtgatggcggccgccgcacagcgcggcgtgcaggcgcagacgttgagtgccatgcaggcgatgccgggccgcggcgtgcgcggcgaggtgaacggcgaacgctgggccatcgcgagcctgcgctggtgcactgaactgggcgtggtgcccgatgccgcgcaggtcgagcgcctgcatgcgcagggcgccaccgtgtccgcgctgctgcgcttcgatgcggcagacgctgccgagatacaggcgttgctggcctttgccgacaagcccaagccagaggccgaagaagccattcgcaccttgcgtgcgcggggcttgcgcgtggtgatgatctcgggcgacaaccggcgctccgcagaggccatggcggcacggctcggcattgctgccgaagacgtgcgcgccgatgtgctgccggccgacaaggcggcgcaggtcagtgccttgaagaaagacggccacgtggtggcgatggtcggcgacggcgccaatgacgcgccggcactggccgcggccgacgtgggcattgccatggcaccttcgggcggcggcaccgacgtggccatggaagccgcgggcatcacgctgatgcgcggcgacctggcgctggtggccgaggccttcgagctttcggcgcgcacggttgccaagatccggcagaacctgttctgggcctttgcctacaacgtggccggcattccgctcgcggccttcggattgctgagccccgtggtggcgggtgcggccatggcgttgtcgagcgtcagcgtgatggccaatgcgctgctgctgcggcgctggaaaccctgagcctcatcgagttcagtcgatcagcagcgccagcaggtgatcgtcgatgtagtcggcttcgccagcgcgcttgtagaacttgcgcaaggtgccttcgcgttcgaagcccagcttttcatagaagcgcaagcccggcgcgttgtcgctctccacatagagctcgatgcgcttgacgccttcggccacgagcctggcgatgccatcgctcaccatcgcatgcgcgatgcccttgccgtgcagcgacggatcgaccgcgagcgtgccgaagcaggcgacgtggctcacgcggccggggtagcgcgtcgcacgatagaaacccgcgacgcgcccctcggcttcatagatgaagaagctgcggctctcgaccagctccctgtagatcggccgaaattcatcgagcggcatcgggtcgtagcccaggaagggcacgaccttctcatgcatgtagatggaaaagaccgcttcgatgtcttggggtgtggcaagcctgcgcatggatgacagcatagccagtcccgatccgccgctcgcggctgccgcactgcagccgtttctttcttcagtggttcgtggcgcggcccgcgatcagtacggcgttggtgccgccgaatgcgaacgaattggagagcacgtagcgcaggttccgggcttggcgcggttcgccgcgcacgaagtcgagatcgaagcccgcatcgggcagccgcaggttggccgtgggcggaagcatgccgtgcgcgagcgtgcgcagcgccgccaccagttcgatggcgccaccgccaccgagcacatggccgtggatggccttggtggcgctcacgggcacggcattgccgaacacctcgcgaatcgatgcagcctcggccgcatcgcccgccgtggtggcggtgccgtgcgcgttgatgtggccgatctgtccggcctcgagcccggcgtcgcgcagcgcggcacgcatggcgcggacctggccggcgggatcggggttggtgatgtgcgtggcgtcgcagttggtggcatagcctgcaagaaaaagcggcatcgcttcactcgcgccgcgcgcgcgtgcatgggcttccgattcgagcaccagcgcagccgcgccttcgcccagcgcaaagcccgctcggtcggccgagaaaggccggcaggcgttgcccggtgtattggccggaggaggcgccgtcacgcgcatcgcatgccagctggccatcacgccgggagtaagcatggcctcgtgtccgccgacgaccgccatgtcgatccagccgccgcgaatggcgcgcatggcctcgccgatggcgacggccgaagaggcacaggcacacgcgtaggcaatggccgcgccctgggcgccaaactgcaatgcgagctccgccaccgcggcgttgggcatgacggtgagcaccgtcgtcggccgcatacggcgcttctcgccgtagagcgcacgcgtggtgtcgtcgaaggcgcccgcgccggccaggccgctgccccagaagatgcccaggcgctcgggatcgacactgcccgcgtgaagcccggcctgcgccgcggcatcgcgtgcggcggccagcgccatggcggtgccccggtcgagcggcagccgcgagctgctgcgcacgccggccgaatcgaaatcacagggcgccacggcgagctcgatcgcatcgaggcccgcgatgccgagcgtctgtgcgcgcaccgcggaccttccgttgaagagcgcatcgtcgaaggactcggccgtgtggccgatcggggtgacgaagccgatgcccgtcacccgcaccggcgcggaagccgcatgcaaggcggaggcggcgagcgctgaatgagcggcgccgctgctcacgcgggcgcggccatcgcaggctcgacgtcgcaccggatctgcgcttcgatcgcctcgcacaagtgctggagcgtgatgccggcttcgcgcgggtcgagccggtcctcgggcagacggaggtggaacgcgtcttccaccgcgaagacgaactccatcagtgcgagcgaatcgagcccgagttcggacagcgcaacctgaggcgcgatggaagcgggtgcaacgtcgaagttgttcaccaggatggccgcgatgctgttgaagaccggcgtagaaaaggaagcggaggacatgcgtttttctttcaggcgggaacgagatgcagtggcaacacgccggaggtgccgcgcgcgccgatgccatgggccagggcgtcggcaaaagcgaccgtctcgcgtgccacctgctggcggtcgttgtcgatcgagatcatgtggtagctgttgtggagcaccctgctgcggaattcgcggcagcagcgaaggccgcgcgcgaggatgtcgaggttggccaggctggccacttcgtcctcgcgggcatgcagcgcgagcacgctgccgcactgcacctggtcaaggttgcgcttcacatggcggatcagccggtcatgctcgcgcagatggctgacgccgagcaccgaactgcccgcgcgcgacaccttgcggtggcgcagctcgcgctcgatccaggcgcgcacgcgttcgttcttcacgccgtagggcgggcattcccggtactgccagaagcgtccgagcggcgtgtagaacgcgagcggcagcagcatgcgcgtgcgtggaatggcccagccgtcgaagcgcagcgtggtcgacatcagcaccagcgcatcgacatcgctgccgcagcggatggccgcgccgagtgcgagcgacgagccggccgaaatgccgaccagcagcacgcgctcatgctgcgcgcgcagtgccttgacgcgcacctcgatggcgtcgagccagcgctcgtagggcagggcgtgctgcagcggcgcgccggcatcgaaggagtagccgtcgatcgccatcgggtgcaccggatagccgctgccgcgcaaggccgattgcacggtcaggagctcgtcaggtgtgctgcataaaccatgcagcagcacgacggccgtgcggcgcaccgcggggtgcaccacgctcagcaggtcggcgggatcgcgggcgctcatcgggtcgcaaggggctggaaaggggccctggccgcaggttgctgtcgtatgctcatggcgtgtttatcgtccgggtgtgctgaccggctgctgaccctccgtcgcgcaagaataggcactgaaacccaccacacaaacaccatgcgaatcctgcttgtcgaagacgacgccgtgctgcgcgacgtgatgctgcgcagccttgcggatgccggccaccgggtcgacgtgtcggccaatgtcgaggacgccgaccacctctggcgcgtgcagcccttcgatgccgtgctgctcgacctgaacctgccagccaccgcaagcccgacgagcggcctggcaagcggcctcaccgccttgcggcaggcgcgcgcgcgcggcgaccgcacgccggtgctggtgctgacggcgcgcggccggaccgaggaacgcatcgccggcctcgatgccggtgccgacgactacctgggaaaaccgttcgacctggccgaagtcgaggcccgtctgcgtgcgctggtgcggcgcgccaagggcaccgaggacatcgtgctgctcggccagctcaagctcgaccgcaaggcgcgccgcttttccaccgcgagcgggccgctcgacctgccggcgcgcgagttcgaggtgctgtgggagctgatgagtcccccgggccgcacggtcagcaagcgggcgctgtccgacaagctctcgagcttcgacgaatcgctgggcgacaacgcgctggaggctttcatctcgcggctgcgcaagaagctggccggttcgggcgcgagcatccgcacgctgcgcggcatcggttatctgctcgaagccgaagtgtgagcggcacgacaccggccgcgcttcggccgccgaaggcagcaccttcgctcacgcggcgcgtgctgcgcaacgtgctggtgccgctggcgctcacgtggatgctgggcgcggtcatcgccctcgtcatcgccaattatttttccgaacgggccttcgaccgcggcatgctcgacgacgcctatgcgctcgcggccaacgtgcaggccggcgaacgcggggtcgagctgctgctcacgccgcgcgaggtggccacggtgctgttcgaccaggtcgacaaggtctacttcgcggtgcagcggctcgacggcacgctgatctcggggcaggctggcctgaacgcattgctgccgccggaaggtgcgcgctaccgcttctcggacgtggccttcgacggcaaggcccttcgtgcggtggtgctccagcccatcgtggagccgggcctgccggtgccctatcgggtcgtgattgcgcagaccacgctgagccgcacggcactggtgcggcagctgctcggctttgcgctcgcaccgcaggtgctgctgctgatgctgctcgcggtgtggctctggtacggcattcgcagcgacctgcgcccgctcggcgagctgcaggaggcactggaccagcgcgatgtgtacgacctctcgccggtggcggtggtccgcacgtcgcgtgaagtgcagcgtctgggcaatgcggtcaacgcgctgttcgaccggctgaatcacagcgtgcgcgcgcagcgcgagttcgtgggcaacgtggcgcacgagctgcgcacgccgctggcgggcattcgcgcgctggccgagtacgggcttgcgcagcacgactccggggtgtggcgcgagcagctcgtgcgcgtggccgaacggcaggcccgtgcgagccacctcatcgaccagctgctggcgcttgcgctcgctgacgaggcccgcaccggccttgcgcgcgaaccggttcggctcgacgttcttgccgaggagaccgtgctgcggcacctggcacgcgccgactcgcgcggtgtcgacctgggtgcgcgcggcctcgacgagcgcaccacggtgctcgcgaacgaagcgctcgtcgaaggaattctcgacaacctgatcgacaacgcgctgcgctacggcgggcgcaccatcaccgtcgaactggcgggccggaccttgagcgtgatcgacgacggcgccggcattccgctggaggcgcagcgcgacctgatgcagcgctgggcgcaaggccccgcgggccagaagctcgggcagggctcgggcctgggcctgtcgatcgtggcgcgctacgcggaactgctgggcgccgagctgcggctcgatgcggcagaaccttcgggattgcgggtgagcgtggtgttcggcgacgtggcctgagtcggcatctgcagcggcgtgccttggtggaacgtgcgttgcacgggactatctcaatggcttgcgcaggaagacgcgggtgcgctccgcgagcgcgaggcgcttgtattcgacatagccgatgcgttcgtagagcgcgcggttttcggtcatcttctcgttggtgaagaggtagatcgaatcgtggccttgccgcagtgcctcgtcttcggccagccggagcagggcgcggcccacgccggtgccctgatgtcgcggctgcaccgcgatcacgtcgatgaggaagccttcgtcggtgacgtcgagcaccagcgcggcgatggtctcgccctgctgcgtggcgacccagacctgcgcattcgcgatggcctcgccgtagtccttggtcatcggaatcggcgtgagaccgaggcgcggaatgtagtgccggaaggcctcgacggcgcaggcggcaacggacgccgcatcgtccgcttcggcccgcctcagcacccacggggcgacgtggctcatgcgtcgaactccacctcggcctcgatgcgggtcatggcatttctctccttgaaggcggacacaaaagcgtccgccgcatcttgccatggccccggggctcaacccagtgccggatagtccgtgtagcccttggtgccgccgccgtacatcgtggccttgtccacggcattgagcggtgcgttctcgcgcaggcggcgcaccaggtcggggttggcgatgaaaggcttgccgaaggccacgaggtcgtcgccttccttgaccgcctcgtccgccagcggcttgtcgtacccgttgttgaccatccatgcgcccttgccgccggcctggcggtaggcggccttgagggcctcgtagtcgaagggacggtcctcgatctcgcgcgggccgccggtggcgccttcgatgatgtggatgtaggccaggccgagcggggcgagctgcttcaccacgtaggtgaagagcggctgcggatcggaatcgtgcacgtcgttggccggcgtgacgggcgacaggcggatgccggtcttgccgccgccgaccgcatcgaccactgcccgcgtggcttccagcagcaggcgggcgcggttctcgatgctgccgccgtagtcgtcggtgcgcttgttgctgccgtccttcaggaactggtcgagcaggtagccattggcgccgtggagttccacgccgtcgaagccggcggtttccaccgcgttgcgcgcggccgccgcataggcgtgaacgatgccgggcaactcttcggcatcgagcgcgcgtggctccgaggtctcgacgaaggtcggcacgccgtccttgatgagcacggtcttggtcttggcggtgatggccgagggcgcgacgggcttgccgccttcgggctgcagttcggtgtgcgacacgcggcccacgtgccagagctgcaccacgatcttgccgcccttggcatgcaccgcgtccgtcacgcgcttccaggcgtcgagctgttcggtgccgtagagcccgggcacgtcggcatagccctgtccctggtggctgatggcggtggcttcggtgatgagcaggcccgccgtggcgcgctgtgcgtagtaggtggctgcgatgtcctgcggaatggcgttgggcgagcggttgcgcgtgagcggcgccatcacgatgcggttggcgagcttcaagtcgccggcctgtacggggtcgaagagggaggacattgcgcggattgaaaagtaggggaagaggccgcgaggctaaacctgcgcggccaaccctgctgtcgcacggttgtctggttgctgctaggcgtttcccgtgccggttgccgccaggtccagcaaggctgcactcgcgcgcaccggcatcgcgagcaggatctgccccatgcccttgccgagcggatcgttgcgcagcgacgccatgccgccgccgccgagcgcctgttcgcagacgaagttgaaggccccgatgcccggcacttcgtagcgcgtgaccggccccttgacgagatgcgccagccattcggccactcgcgcttcggtgagctgttcgcgcagcagcggcagcaatgccggatggcgcgcgatgacgccgatgttcgaggtgtcgcccttgtcgccgctgcgggcccatgcgaggcggatgagcggcacttcgatgggatcggcagcgaaggattcgggaacgtccaccgcacccgttgcattcttcggtgaagaagaaggggcgctggcggccaccgcagactcggcatcagggtgcagctcgatgcgctgcccgtccatcgtcacgcgggcttcgaccttcgacttgtccagcaggaacgcgtattgccggatcgagggcgacacggatgagcgcccgccacccgcgcccgtggtgccgggtgcccacgaggtgccggccggcgccacctcgcgcgcgaagagttcgagcgcgtccttgcgcgcatgcgtcaccgcgagccggagcacggcttcgcgcgtctgcgtggcctgtgcatgcgggccgtagcaggactcggcgccgagtacctcgagttgcgtggcgctgtagggaccgaagccgtgctgcgcgaacagcgcgctggtgcgtgcaaggatggcttcgccggtgcggcgtgcctttgcgacggcatcgaagccgacgatggtgagctgtgccgcgcacttgaagccttccacgtaggtggcgcagaccttgtagctttcggtgggcgcgcggccgcgtgcgccgcgcacatgaacgcggtgttcgccggcctgttcgatgcgcacctgcgtgaagtcggccaccacgtcgggcagcaggtaggccgaggggtcgccgatctcgtacagcatctgctcgcccaccacggccggcgtgaccttgccgcccgtgcccgtcggcttggtgacgacgaagctgccgtcggcatggcactcgacgatggggtagccgatgttgggccaatcgggcaccgtgtcccagtcggtgtgcaggccgccggtggcctggcagccgcattcgatgatgtggcccgcgaggctcccggccgccagcaggtcgtggtcgccaggctgccagccgaacgcgtgcatcagcacgccgagcgtcacggccgagtcgacgcagcggccggtgatgaccacctgtgcgcccgcgtcgagcgcggcctggatcggccttgcgccgagataggcgttggccgtgagcacgcgccccggcaatggcgcgccgctttgcagctcgcgcaccgcgggatgctgctggcggagctgcggcagcaagggcgatacgtcgtcgccgctcaccacggcgatcttcagtgcaatgccttgctcggctgccagcgcggcgagcgcatcggcgcagccctcgggattgacgccacccgcgttgctcaccacgcggatgccttggcgcaccacgtcattcagcacggccttcatcgcgaccgagacgaagtcggtggcgtagccgagctccggtttcttgagccgtgcgcccgcaaggatcgacatcgtgagttcggccaggtagtcgaacacgagatagtcgatctgtccgctggccacgagctgcggcgcacccacgccgctgtcgccccagaagcccgaggcaccgccgatgcgcacgacgcgttccggctgttcgctgcggtcggcgctcatcggccgctccactgtggcttgcgcttttcgcggaaggcgagctggccttcggccgcgtcttccgtgagtgcgaagagcccgatctggctttcggtgaacgccatcgattcttcgaaggccatggcttcgatttttttcatggtgtacaggccgcggcgtatggcggcgggcgacttgtcgagcacgcggccgagcagccagtccacgctctcgtcgacgtcgtcgctcacgcgattcacgaggccgtgttcgagcgcctctgcagcggtgatggattcgccggtgatgcacatctcggccagcacgcggcgcggcagcaggttgccgagcacgctgagcacctgcgcggggaagaggccgaccttgacctcgggcaggccgaataccgcgtggctgccggccacggccatgtcgcacatgcccatgatccccatgccgcctgccatgcaggcgccgttgacgcgcgcgatcagcggaacggtcgattgccgggcctggcggaacaggttggcaaagccctggtagggctcggcatagtcgaacttgaaggaagcgccgctttgcaggtcggcgcccgcgcagaaggcgcgcgtgcccgcgccggtgatgaccacggcgcgcacggcgcgatcggtgtcggcacgggccagcgcctcggacagtgccgcaagcacgccggcgctgatggcgttgcggcgttcctggcggtcgatggtgagccacatcgcgggcccgcgcatctcctcgcgcagttcttggagggcaggggcttcggccatcggcgggtccttcgctttccagggtctgaagttcgacccgtagcgtgacccgaaaaaaaagccgcggcatgcggcttgtggctgaaaggggcccgggttttccccatgatgggccaggccgcctcgcagctgctgcgagcttgtgcgcgcttcttcttacttcagcaggccttcggccttcattgcgtcctgaaccgcagggcgggctgcaacgcgcgcatgccaggcctggagatgggggaagtccgaaatgtcgacgccggtgggcttggcccagttggtcacggtaaacaggtagccatcggccacgctgaagtgctcgcccatcaggtactgcttctcggccagctggccgtcgagccattggtagcgcgacttgagcttgtccttgaagatggtcttggcttcgtcgggcatggcggggttgaacagcgggctgtagcccttgtgcatctcggtgccgatgaaggtcagccactcctgcaggcgatagcgctgcaaggtgcctgcggccggggccaggttcttggtgggtgcgagatcggcgatgtactgcacgatggccgggccttcacgcaggcgggtgccgtcgtcgagctcgagcatcggcacgtacccgagcgggttgatgccgtagtagtcggtgccgtcctgcagcttgtggctcttggtgctggccatcacgggctcgaaggcaatgcctgcctcgtgcagcgcgatgtggggcgagagcgagcaggcaccgggcgagtaatacagcttcatgcgagaaatctccaaggttgaatatggatagcggaaatcgatccatggaccgaaggaatgctagcgggtttgcgcgccgcgcgtttgtcctacggccgctcgcgcgcgccgactatcggggccgcctcggcgcgtttctaagctgcgcgcacggtgggcgaggcccgccgaaaggagtgtccagatgttgaaatacgccatcgtgtttgcggtgatttcattgatcgccgggctgctgggcttcggcggcatcgccgcgggtgcggcgggtatcgccaagctgctgttcggcctgttcctggtgctggccgtgctgttcgtggtgttggcggcattgggcgtgggtgcggtgaaaaaggcgatcgattgatgcagcgcccaccaccgcactggccgcgcgtgcgtccgctcggcttgctgcttcagagcccggcgcaccgcgtcgtgcgggtgctgctcgtcacgcaatcgcattggcagcttccggagcaccgctcgcatcgccggcgggtctgaggcgcccatgcacatctcacacatcgaggcagaactgcgttacgaggtccgggcgcccgcgcacatgctgctcaacatcgaggcctcgcaagctggcgcgcaggccgtcatcagcgagatgctgaccatcgaaccgccgaccgaagtgcggctttactgcgacggttccagcggcaaccgctttgcgcgtttcgatgcgcagccggggccgctacggatcagctacagggcgagcgtgcagcgcaggcagatcgacgtaccactcgacctcgccgaggtgccggtcaaccaggtgccggatgaaatccttcactacatgttgccgtcgcgttactgcgagtcggacctgatgtcgcgttgcgcgcagcagctttttggcgatctgccgcccggcatcggccgggtgcaggcgatcgtcgactggattcacgagagcattgcctatgaaccgggcagcagcgattcgacgaccacggcgcgcgaggtgttcgtggaacgcgcgggtgtgtgccgcgaccttgcgcacctgggcatcaccttttgccgtgcgctcaacatcccggcccggctggtggtgggctacgtctggttcgacgagccgccgcaggattttcacgccgtgttcgaagcctggctcggcgggcaatgggtgttgttcgatccgacacgcatggccccggtcgaccggctggtgcgcgtgggcaccgggcgcgacgccaaggacgtggccttctgcacgatcttcggcgccgtgaccatgacgggcaaagacatcggggtgcgcgaagtgcaggacgaaagcgtggctcccgccgcggcaccgcagcctaccggcgcgatcatgggcatcgaaaaacccgtgcccgtggtggagctggcggcttcggctggctgaaagtaccgtcagtgctgaatagtttgctatgaataacgtagcattctattcaatttcatgggacgaatcggagggctggggtctttgatcccggttgcccttattcccggcgcaaaagggtacccccgattaaaattggtgccccctttgcgcagcgcacgcgtcagtgcgcccctctctcatgctgtatcccgaagaatttgatgtcatcgtcgtcggcggtggccatgccggcaccgaggccgcgctggcggctgcccgcatgggcgccaagacgctgctgctgtcccacaacatcgagacgctggggcagatgagctgcaacccgtcgatcggcggcatcggcaagggccatctggtgaaagaggtcgatgcgctgggcggcgccatggccatcgccaccgacgaggcgggcatccagtttcgcattctcaattcgagcaagggcccggccgtgcgcgcgacccgtgcgcaggccgaccgcgtgctgtacaaggccgcgatccgccgccggctggaaaaccagccaaacctcagcctgttccagcaagcggtcgacgacctgatggtggagggcgaccgggtggtgggcgccgtcactcaggtgggcatcgcctttcgggcccgcaccgtggtgctcacggccgggacttttctcgacggccgcatccatgtgggcctcgacaactaccaggccgggcgcgcgggcgatccgccggccatcagcctgtcggcacggctcaaggaattgaagctgccgcaagggcgcctgaagaccggcacgccgccgcgcctcgacggccggaccatcgatttctcgaagtgcaccgagcagccgggcgacggcatgccgggtggggcagggccgatgccggtgttcagcttcatgggccgggccgacatgcatccgcagcaaatggcctgctggatcacccacaccaatgcacgcacccacgacatcatccgctccggcttcgaccgcagcccgatgttcaccggcaagatcgacggcgttggtccgcgctactgcccgagcgtggaggacaagatcaaccgttttgccgacaaggaaagccaccagatctttctggagcccgaaggcctgacgaccaacgagtactaccccaacgggatctccaccagcctgccgttcgacattcagtaccagctggtgcgctcgatgcccgggctggagaacgcccacatcctgcggccgggctatgccatcgagtacgactacttcgatccacgcgagctcaagagcagcttcgagacccggtcggtcaaggggctgttctttgccgggcagatcaacggcaccaccggttacgaagaggcggcggcccagggcttgtttgccggcatcaacgctgcgctgcaatgccgaggcgaagaggcgtggttgccgcgccgagatgaagcctatctgggcgtgttggtcgacgacctgatcaccaagggcgtgaccgagccctaccgcatgttcaccagccgggccgagtttcgactgcagctgcgcgaggacaacgccgacatgcgcctgaccgaagcagggcgcaagctcggcctggtcgacgacgcgcggtgggatgctttcagccgaaagcgcgatgttgtttcacgtgaaacagaacgcctcaaatctatctgggtgaatccgcgcaatctgccggcggctgagtcggagcgggtgctcggcaaggccatcgagcacgaatacaacctcgccgacctgttgcgccggccggacgtgaactatcaaacactgatgtcgctggacggcggaaagtacagcgcggccattgcgctgaacgaaaccgaaatcgagcagatcgagatctcggccaagtactcgggttacatcgaacgccagcacgacgaagtcgagcgtgccgctcacttcgaaaacctgcgcatgccgcccgacttcgactacggccaggttaaggcactgagcttcgaggtccggcagaagctggacaagcaccggcccgaaacgctggggcttgcttcacgtatctcgggcgtgacgcccgcagccatttccttgctcatgattcatttgcgaaaaggcggtcacaaggctttcgaccgcgatgccaccgctgaagccccagtcgaaccgcaatccgcccaatgaacgcgcccatcgatacgctgcgccaaggcgcggcagccctgggcctcgccttgtccgatacccaggcggagcagttgctgtcatatggcacgctgatgctcaagtggaacaaggtctacaacctcacggcgctgcgcgacgccgcgagcgtgctcacgcatcatctgctcgacagtctggcggccgtaccgccgttgcagcgcgagtgggcggggaagggcaggctgctggacgtgggctcgggcggcggcctgccgggcgtggtgattgccatcatgcggccggatctccaggtcagctgcctcgatgcggtcgccaagaaagcagccttcgtgcagcaagtggcggccgaactcgagttgcccaacctgcgcggattgcacgcacgcgtcgaatcgctcgccggcagctatgaagtcatcagctcccgcgcctttgcttccttgccagatttcttcaatggatccgcccatctgctggcgcccggtggcgtctggctggccatgaaaggcaaagtgccgaccgaggaactggccgtgttacctgtcggtatcgcagtgtttcacgtggaacaattgactgttcctggcctggatgcggagcgctgcatcgtctgggcacgcgaagaagtcgcctgaccgggcaaaaaagaagcgcctacgccagcgaaagccggcggcagagggtgatcgcaggggccgcctcgcttagactcgacgcctccccctggctctcttttccgaggcaaatccatgttcggcatcgctgactacggcgcattcgtcgccgccatcgtcctctttctactgattcccggtccgggcaacctcgcgttgatcacctcgaccagcaaaggcgggattcgtggcggattggcagcaacgctgggcgtgatcatcggcgatcaatttctcatgtgggctgcggtggccggcgtggctgccatcctggctgcgtacccggcagcgttcaaggccgtgcaatggctgggcgcggcttaccttgcctggttgggcgccaagatgctgctggccaagcccggtgcaggcccgatcctcaacatccgccccagccatttcctgcgccaggcgctggcgatcaccttgctgaatcccaaggccatcgtgttctacatggcgttcttcccgctgttcgtcgacccggcacgccaccagggcgtggtcaccttcggcgccatggctgtgacgattgcagcgctgaccttcctgtacggcctgagctcgacgctgctgacgcactttctggcggaacgcattcgcgccaatccgcgcatttcgggcgtgctcgaaaagctcgcgggcgttttcctgattgccttcggcgtcaagctcgccatttcccgctgattcccgtatggccaagattttctgtattgccaaccaaaagggcggcgtcggcaagaccaccaccaccgtcaaccttgcagccggcctggccaaggtcggccagcgggtgctgatgatcgacctcgatccccagggcaatgccaccatgggttcgggcatcgacaagcgccagctggaactcacggtgtacgacgtgctgctcgagtcggcttccgtggccgaggcgcgcgtcaaggccgacaaactcgtggagggcggctgcggctatgacgtgctcggcgcaaaccgggaactggccggtgccgaggtcgaaatggtggcactcgaccgccgcgaaaagcgcctgcgcaccgcgctggctgcggtgggcgccgagtacgacttcgtgttgattgactgcccgccgagcctgagcctgctcacgctcaatggcctgtgcgccgcgcatggcgtgatcgtgccgatgcaatgcgagtacttcgcgctcgaggggctcacggacctggtcaacaccatcaagcaggtgcacgccaacctcaacaagaacctgcagatcatcggcctgctgcgcgtgatgttcgatccgcgcatcacgctgcagcagcaggtgagcgagcagctcaaggcccacttcggcgacaaggtgttcgacacggtcattccgcgcaatgtgcggctggccgaggcgccgagctacggcctgcctggcgtggtgttcgacccggccgcccgtggcagccaggccttcgttgcctttgccagggaactggtcgaaaagttgccgcccgccagcgcctttgcatcgaatgcggtcgcgccgccgattgcgccggtcgcggccggcgcgcccaacctggccattcccgaagacgtgctggccccggcggccgcacccgattccaccagcgaaaaaagcctctgacgcggtccatcatggacctgcgccaacaagtttccagcagatgacgacgacgactccccgcatcctcttgctgccgggctggcagaacagcggccccggccattggcagacgcggtgggaatccgcgtacggcgaccgccgcgtcgagcagcacgagtggatgcgcccgctgcggggtgactggtccgcacggctcgaggaagaagtgcttgccgcacccggcccggtcgtgtttgccgcgcacagcctgggctgcatcctcgtcgccgcctgggccgcgcattcgcgcaacacgcacagggtgcgcggcgccctgctggtcgcgcccggcgacctggagcgcgacgacctgcgccagctcattccgggctgggctcccatcgtgcggcagccattgccattcccggcggtgctgatcgccgccaacaacgatccctactgcgacgccgcgcgctcgcgccagctggcggccgactggcgcgcgcgcttcgtcgacgccggcccgggcggtcacctgaatgccgagtccggcctgggcgactggcccgagggccggaaactattgaacgaaatctcgaaagacaagcactgatggcgaccaagaaacccaagggcctcgggcgcggcctcgaagcactgctcggcccgacggccgggcattccgtcgacaacgcaggaacggaagagggcgccgccgcgcagaaccccaccacgctgatgctcgaccagatggtggcgggcgtttaccagccgcgcacccgcatggacgaaggcgcgctgtacgagctcgccgagagcatcaaggcgcagggcatcatgcagccgatcctggtgcgccggctcgatggcgaatcggccgaggccaagaacgccgagttcgaaatcatcgccggcgagcgccgcttccgcgccgcccgtctcgcgggcctcgaccgcgtgccggtgctggtgcgcgacgtgcccaacgaggccgcggcggccatgtcgctgatcgagaacatccagcgcgaagacttgaacccgcttgaagaagcccagggcttgcaacgcctggtttcggagtttgggctcactcacgaattggccgcgcaggcggtgggtcgttcgcgcagcgccgccagcaatctgctgcggctgttgaacctggcggagccggcgcagcagatgctgatggccggcgacatcgacatgggccacgcccgcgcgctgctgtcgctggaccgcggcacgcagattaccgctgccaaccagatcgccgccaagaagatgtcggtgcgcgaggccgaggcgctggtgaagcggctcgcggccgagttcacgctcacgccttcgcgccgcagcaacgatggcgagaagtcgcgcgacctgcagcgcgtggaagaagagctggccgacctgctcaccgccgaggtcgaggtccgcatcaagaagcgcagcaagcgcggcggcaaggtcgaggagagcggtgagctcgccatccacttcggctccatcgaggcactcaacggattgatcgaacgcatccgccgaacggcctagttgctgagctgtccctcggacgtttgcttgattgattcttgcaatcttttacgcgtatcctcgccgggcacatcaacccagatctcgaggagagggagtccgccatcatgaggttcactagtacaaggtttccattcgcggccgtggctgcgggtgcgctgctgctggccggctgcgccaccacggacatgcaaatgggcagccagtcggccaagaccatggccaccggcagcgcggcaggttcggccaccgccggcgaaagcagccagctcgagcgctgcgagtcgccgctcggcaccgtctcgctgatcgagaacgtgaattccggctggtacaccatcctcaccggcgaataccgcctgccgcccacggccaacctgctgcgcctgctggtgcagcaatcgaactgcttcgtggtggtcgagcgcggcgcggccggcatgaacgccatgacgcgcgagcgcgcgctgcagcagtcgggtgagatgcgcggcggcagcaacttcggccgcggccagatggtggcctccgattacggcctctcgcccgagatcgtgttcagcaacagcgatgccggcggcattggcggtgcgctgggcggcctggtgggcggcggtcgcggccgggccctggcggccgtcggtggcagcatgcagaccaaggaagccagcgcgctgctcacgctcatcgacaaccgctcgggcgtgcaggtcgcggcttcggaaggcagcgcctccaagaccgacttcggcgccttcggctcggtgtttggcagccgtgcggccggcgggctcggcggctacaccaacacggcgcaaggcaaggtgattgccgcggcgttcatggacgccttcaaccagatggttcgctcgctgcgcaactacaaggcgcaaaccgtgcgcggccagggccttggcggcggcggccggctgggcgtggacggcggcgcggccccgtcgcaaacctacgtgccgccggagcaggcacccgcccgccgtcgcaagtaagtaagcaagacgcgcgggccagccgcaaaaaagcccggggctctcgcgagcagccgggcttttcatcgggcccgaacgcgccggatcagagcgcgaagatcttgccgggattcatgatgttcttcgggtcgagcgcgcgcttgatcgtgcgcatcatgtcgatcgcgcccacgccggcttccgtcaccaggaagtccatcttgtgcagccccacgccgtgctcgccggtgcaggtgccctccagcgccagcgcgcggctcacgagcgcatggttcagctcctcggccttcacgcgctcttcgggaatgttcgggtccagcaggtagccgaagtggaaattgccgtcgcccacgtggccgaccaggaagtaggggatgccgctcgcatcggcctcggccaccgagtcgagcaggcaatcggccaggcgcgaaatgggcacgcaggtgtcggtcgagatcacccggcagccggggcgcgactgcacggccgcaaagtaggcgttgtgccgtgcggtccacaggcgcgtacgctcttccggcgtgctggcccattcgaaggcgttgccgccgtggccgctggcgagctcctgcaccgtctcggcctgctccttcacgccggcgggcgagccatggaattccatcagcagcagcggctcttcgcgcaggcccagcttggcgtaggcgttcaccatgcgcaccgtgttcacgtcgatcagttcgacccgcgcgatcggcacgccgagctggatggtctcgatggtggtgcgcaccgcggcctcgatgctcgggaacgagcagattgcggcggacaccgcctcgggcagcgggtagatgcgcagcgtgacctctgtgaccacgcccagcgtgccttcgctgcccaccatgaggcgcgtgaggtcgtagcccgcggacgattttttcgcgcgcgtgccggtgcggatgacttcgcccgcggcggtcacgacttcgagcgccagcacgttctcgcgcatggtgccgtagcgcacggcgttcgtgccgctcgcccgcgtggccgtcatgccgccgatggaggcgtcagcgcccgggtcgatggggaagaacaggcccgtgctcttgatgtcgtcgttgagctgcttgcgcgtgacgccgggctgcaccgtgaccgtgaggtcgtcggcattgaccgacagcaccttgttcatgcgcgacacgtcgatgctgatgccgccctgtacggcgagcagatggccttcgagcgatgagcccacgccgaagggaatgaccggtacgctgtgctcgctcgcgagcttcacggcgtcggccacgtcttgcgtgctctcggcaaagaccacggccgaagggggcggggcgtcgaacgaggactcgtcgcgcccatgctgcgtgcgcaccgccatggccgtggagcagttggcgccgaagcgtgctttcaggccctcgatcaggctgtcgggcacgtcgcgcagatgaagcgccggcatcaggtgcgaggtttgggtcggtgcgttcatcgggcgtctcctggagggggtgagggcggggctctgtgcggccattttacggagcgagcaccataatgcgcgtcagcagaaccatgaaccctacgaccctcaacacactcgcggcgtttccgtcgcaactcgccgcccactatgcggccattcccgttgcattccggcattgggcgcccccctcgtgggagggcgttccgagcgaggccttcacggccatcgagcagctctgccatgtgcgcgacatcgagatcgagggctatcacgtccgctttcgccgcacgctggaagagcgcaatcccacgttggcttcgatcgacagcgagccgctcgccattgcgcgcgcctacggcatggccgacgcggccaaggtgctggccgagttcaagatcgcgcgcgcgcagaccatggaaatcatctcgaagctgagcgatgcgcaacttgcgcgcaccgccgtgttcgagggctacggaccgctcaccatgcgcagcctcatccactacctctgcagccacgaccagcagcatctggcgggcctgcaatggctggccggcaagatcgacgcgtcgaccatcctgcgataaaacaggcacaacaggagcgcccatgggcaaccgactttcccagatcgccacccgcaccggcgacgacggcaccaccggcctgggcgacaacacgcgcgtgcccaaggaccacctgcgcgtgcacgccatgggcgacgtggacgagctcaactcgcagatcggcgtgctgctctgcgagcccatgccggagcccgtgcgcgagctgctcgtcgacgtgcagcaccagctcttcaacctgggcggcgagctttcaatgccaggctacacgctgctgaaggccgacgcgctgcttcaactggacaacgcgctggccgagcacaacgccgccttgccgcgcctggccgaattcatcctgcccgcgggcacgcgcgcggcctcgctcgcgcatgtgtgccgaacggtggcgcggcgggccgagcgcgcggtagtggctctcggcgccacggcggaactcaatgatgcgctgcggcaatatctcaaccggctcagcgatctgcttttcgtgcttgcgcgcgtgctcaaccggatgaacggcggcgacgacgtctactggaagagcgaacgcatggcgcgagttgccgcagaagcatcggatgccgaccagcctgacgacaaggaaggaagcccctcatgaccaagaagatgcctgctcattcattcgcgctggctgctgcgagcgccgcgctcctgctgctgtccgccactgccgttcacgcccagagcgccgacaacccacccaaggtccagcccgcgcacaccctcccgccgccgccgcgtgacagcaaggtcgtgaacagcgtgcagcgcggcaccaacgccgccggccggggcatcgaccgcgccgaagacgccacgcggcgcggtgtcaacaacgtttcggaaaaggccagtcggccggtgcgcagggtgggcgagtcctttggccgcaagctcgcgcccggctccagcggccgcactgcgccgccgccggtggggccgcaaggcaacgcgccctgatcgtcatcagggcgcgatcccgccgacggggtacctttctccgcgaatgtcccccggcctgcggcctcctcctttatttcgctgcgcaaggcaccccatcgacgggatcgttattcagaggggttgttgatcggcggtacaccagcagcgtgccctggtgcacagggcgccgggtactccccgcagcgaaacaaaggaggagctgcgggagcagaaggcgggggacattcgcggaggggagtacccggtggcctgcgcacgcgtcccgaacacaagcaagccacaacacgcagcgacagaccaaccgagatggcaagaaacatagagatcaaggcccgcatcgacagcgtggaacgcgtggcgctcatcgccgcgaaactggccgaatcgggcccgatcgaaatcgcgcaggacgacacgttctttcgctgcgagaacagcgccgatcgcctcaagctgcgcaccttcgcgcccgaccatgcggagctgatcttctaccgccgcgcgaacagcagcggcccgaaagagtcgttctatctgatctcacccaccaccacgcccgacaccctgcgcgagtcgctcacgctggcctggggccagaccggccgtgtgcgcaagcagcgtcggctcttcatcgtgggccgcacgcgcgtgcaccttgaccgcgtggaaggcctgggcgaattcctcgaactcgaggtgatgctgaaagagggcgagcccgccgaagagggcgtagccgaagcgcatgcgctcatggcgcagctgggcattgcgaccgaccagctggtgcagggcgcctacgtcgacctgctgcgcgccgccgttgctgctgctgcttgagtctcatcagcgccagcccgcggccttgagctggtccgcgagctgctgcgcaaccttggcatagcccttggcgttggcatggatgcggtcggagcgcagcgaggcgtccgacagcacgctcgaatacacattggcgacgagcagcgcctgccccgacttcgcgacctcgtcgtagaacggcgcatcgctgagcgatccgacagccgcgcgcatcgcatcgggcgagggcgtggccagcagcgcgacatggggcgtgtgcgcacgcgcctggctcacgagggccgcaaggttgtcgcgcgtggcagagggcgacacgccgcgcagcatgtcgttgccgccgatgccgatcaggatcgcgtcgtagctgcccgccgccagcagcgacggcaggcgctccagcgccccggccgaggtgtcgccattgatgcccgcgttgtcgatctgccagccggtgagttcgcccagtttcacgggccaggccgcctcgggcggcgcgccgtagccgaaggtcaggctgtcgcccagcgcgagcacgcgggcgtcggatttcaatgcggcggcggagggcttgcgcttgccacacgcggccagcgcggcggctgcggacatgccggccagcaggtggaaaaggtgtcgtcgcttcatgctgggcgcgagcttaaacgcattcaatgaagcaagcgccgggctcagcccttgcgcgcggcggcgtgcgtcttgcgcagctcggcctgcatctgcttccagagcaccggccctcctttttccatggcggccgcggccgctgcgctctcgcgcgtgaccggctggtgcttgcgcccccagatgccgatctgcgccaccaccggcagcaggtcgatgcccatcggtgtcaggctgtagatggccttctgcttgtgcgtggggtcgtcggccttgtggagcacgccgtgctccacgagcttgcccaggcgctcggtgaggatgttggaggagatgccttcgtcggattgcaggaattccctgaagtgccgcttgcccgcaaacatcatgtcgcgaacgatgagcaggctccagcggtcgccgaagacctcgagcgatagattgatcgggcacagggatctctgctggtttgccatcgtcgatattgctctcttattgaaactgcttgcattttcgtaccagtactccaatacttcaaccggttgcaaatcaagagcagttatccggcatgcaccggcgaaggagaaccgcatgagaaagctcgttctgcaaatgcagatgtcggtcgatggctgcgttgcagctgccaaccccggcctcgactggcagctttgggggtggggtgaccgttggggctgggacgacgcgctcaagcaatatttcaacgaggtcttcgaatcggtcgacaccattctgctgagccgcaagatcatcgaggagggctatctcgaccactggggccgggtcgcgagaagccaccccgccgattcgaactacgccttcgcgcggaaggtggtcgatgcacggaaggtcgtgctcaccggcaagctgaagacatcgcgatggccgcgcaccgacattgcgaaccgaagcatggccgacgaggtgaatgcgctcaagcagcaggcgggcgcgaacatcctctgcatcggcggcgccggctttgcatcgtcgctcgtcgccgaggggctcgtcgacgagtttcagttcttcgtgaatccgaccgccgttggcggcgggcgctcggtgtttcacgaccagcgcaacggccacaagttgcgcttgcttggctccagggcctacgaatgcggtgtcgtggtcaaccgctacgcgccaaattgaaggacaacgcgccgcgccgataccagcgcttacctgatttcacctgacggcgacctgatgtgctccgggcagacacaagcgccactgagaatggactcgtcatcaacacgaaggagttccagatgatcatcaattcaaagagcatggccgtcgctgctgcggcgctcgcgatgtgcatggcagcgggaagcgccttcgcgcaagaccgtggcggccatgatcgcgatcggggccatgaccgcggcaacgatcacggcaacggccgctacgaacaacaggaccgccgattcgaccggcacgacaaccggtatggcgaccggcatggcgaccgctacagccgcgaagactaccggcccggccgccagttcgatcgccgcggctacccccagccgcatgccgaatggcgccgcggcgggcgtgtgccccatgagtaccgtggccgcaactacgtggtgaacgactaccgcgcctaccagctacaggcgcctcctcgcggctatcagtgggtgggcgtgggcggcgactacgtgctcgccgccattgccaccggtctgatcgcgcagatcatcgtgggcaaccagtaaaggcaaagagcgcggcacgccgcgcgcacagcttcattcaagaccgtcgcagggcttcctgcggcggtctttgtttttttgagagggagtgaaaccctcaggctgctacggtgggcagcgactgggcgcaaacattgcgcccggtgatggtgagccgcaaaccaccgccgtgccattcgagccagttaaggctcacatacgcatcgatgtcggcgtcgtcgatgcggtccgcctggcggctttgcagcagttcgacggtggcgggcagtgcccgtctgagccgctcgcgccgttcggcggcgtcggcggccttctgggcggccttggtttgctgttgctgctgcggggtcgatgccattgctgatccgttccgggaagccaaggaattaatccgaatgtacgctccctgtgtgaagcagccagcttcttttttaaacctgtgtcggcaagcgttgaatccgttgcgccggcgctagatttcgtagtgcgagcccttcgcttcatcgcccagagccttttcgaccacgctgcgcgtcaaggtcggtgcaaacgactcgatgaacgagtagacgtacttgcgcaggtaattgccgcgccgtaccgccagcttggtcaggttgatgccgaacagccgacccgcgtcgagtgcgcgcagctgcgtgtcgcgctcagcctcgtaggccacaccggcgacgatgcccacgcccatgcccaattgcacgtaggtcttgatcacgtcggcgtccatggccgcgaggacgatgtgcggtatgagcccgcgctgcgcaaacgcctcgtcgatgcgcgagcggccggtaaagccggtgtcgtaagtgatgagcggatggcgcgtgagcgcctcgagcgtcagcggcgcatcgagcagcgcatggcccggcggcaccaccacagagtgcgtccagcggtagcagggcagggccaccagctgcggatagtcgcccagcgcctcggttgcaatgcctacgtcggcctcaccgtcgatcagcatctgcgcgatctgcttgggcgagccctggtgcaggtgcagcttcacgttgggaaactgcgcgcgaaattcctgcaccgccaccggcatggcgtagcgcgcctgcgaatgcgtggccgccaccgagagcagcccgctttgctgcgccacgaactcctgccccgcctgcctcaggttgctgctttccatcagcatgcgttcgatgatcggcagcacgtggccgcccggctcggtgagtccggtgagtcgcttgccggctcgcacgaaaagctcgatgccgagttcctcctccagctcgcggatctgccggctcacgcccggttgggaggtgtgcagggtatgagcgacctcggtcaggttgaagccgcaacgaacggcctcgcgtaccgagcgcagttgttggaagttcatctggcgcgaaggatcggaaggagaaggcccggactggccgagcggcgattctcggcacaagtgcttatgcggggaacgatgcgtttgttggtttcacatgagcaaatcatctgtgccgcaccgactggagtgcctctgccagtgcatttgaaatttcgcacgactgtgctaaagtctgaatcatggacgccaagacccagaaaagcgaactcacccgcaccgccatcgtcggcgcggcgatggacctcgcgctgaccgaaggcctggacgccatcacgctccaggccgtggccagccgcttggcgctctccaaaagcggcgtgttctcgcgcgtgggttcgcgcgaggcactgcagaaggccgtgatcgaagagtacggccgtcgcttcctggccgacgtgttcgtgccggccatgcaaaagcccaagggcctggcgcggctcaacgatatcgtcgaccgctggatagcgcgcacccgcgacatcgaagccgaaaccggctgcatctacatggccggcgccttcgagtatgacgaccgcgaaggcgagctgcgcgacctgctgctcgccgagatcacgcgctggcgcgccgccctgcgccgcaccgtgctgcaggccatcgagtccggcgagctgcgcgccgacaccgacgccgcgcaggtcgtcagcgaactcaacggcctcatcatgggcttgctgcatgacgcgcgctttttgcgcgacgcccaagccgccgaccgcgccaagcagacctggcagcggcttctttccagctaccgcgcctgagccacgggcgcacaggtttcattcgtctttctttgttctaatttcgcacagtcgtgcgataaaaaggagaagcaccatgctgatcattgccctctgccttgtcgtctacctgggcgccatcggcgccgaagccgctcgggaggcattgcgcagcctgccgcgcagcaatgaagactgggtctggtactgaatcgacggagccattgcatgccgagcagcaccaccacctccgcggccacgcacgccgcgcagtcgaactactaccgccccagccgtgtaatgcgcacactgcgtttcgccctgaccaccgcgcagcgcctgtggcctgcattgggagtgcgcgccgcgtaccggctcttcggcacgccgctgccgcccaagtggctctaccgcgggcaggcgcccggcaccgattggcgtcgcgaagcttgggccttcgagaacgcgagcctcggcctctatcaccttgccacgcaggattcgggcgcggaatcggcacccatcgtgctgctggtgcatggctggggcgggcatgccggtcagatgctggcgttggccaaggtgttggccgatgaaggccttcggcccgtgctgctcgagctgccggctcatggccgcagcgcgggtatcatgagcaactcgccgcagttcgcccgtgccatcgcctatgtggtggcaaggctcgcggccgacggttatgccctccgcgcagtggtggcgcattcgatgggcgccaacgccctcgggttggccgccgcgcagggcctccgcgccgagcggctggtgctgctcgcgccaccggcttcggcgcgcgaattcacgcgctacttcgcgcacacgttcgggctgagcgaagcgacgcggctcgcaatgcaacggctgttcgaagcgcgcgaaggcctcctgatggcgcagctggagccgccggctgtcggtccgcgcatcgtgcagccgacgttgatcgtgcatgaccgcgatgatcgcgtgaaccgctttgccgacgcggaggcctaccgcgatgcgatcaagggggcgcggctcgtggccacggaggggctggggcaccgccgcatcctcaaggaagaggccgtgctgcggcaggtggcgcgcttcgtggcgcagccttgagctgagccctgaactgaaacgggagggctgcgccgccccccgcgtgttcgatcagcgtgccggcgagggcgccgggtcgggcagttcgatcttgatgtcgagcacttcgaggtcgtcctgcttttccaggtgaaccttgatgtcctcggcattgatcttcacgtatttcgagatcaccgccatcagctcgcgctggaggtcgggcaggtagtcggggcgcttcttgccgctgaggctggaccgctcgtgcgcgaggatgatctgcagccgctccttggcgacgctggccgtcttcttcttttcgccgagcaggaacgagaaaaaggacatggcctacttgcctccgaaaattcgcttgaagaagccaggcttttccgcatcgacgaagcgcatcggcttgtcttcgcccaagaagcgcgccaccacgtcgctgtaggccttggccacgtcggtttccttgtcgtggatggcaggcacaccctggttggacgcctgcagcacgctttcggattcgggaatgacgccgatcagcttgatgcgcaggatgtcctggatgtcttccagcgagagcatctggccgccggccacgcggttggggttgtagcgggtgatcagcaggtgctccttgatggggtcgccgccttccttcgcccgcttggtcttgctgctcagcatgcccaggatgcggtcggagtcgcgcaccgaggatacctcggggttggtcaccacgagtgcctcatcggcaaagtgcatggccatcatcgcgccggtctcgatgcccgcgggcgaatcgcagacgatgtagtcgaagtccatcgcggccaggtcggtcagcaccttttcgacgccctcttgcgtcagggcttccttgtcgcgcgtttgcgaggccgccagcacgaacaggttgtcgcactgcttgtccttgatgagcgcctggctcaggttggcttcgccctggatcacgttgatcaggtcgtacaccacgcggcgttcgcagcccatgatgaggtcgaggttgcgcaggcccacgtcgaagtcgatcaccgccgtcttcttgccggcgagcgcaaggcccgacgcgaagctggcgctcgtcgtggtctttccgacgccgcccttgcctgaggtcaccaccacaattttggccattgccattccttcttgtttcgattcggttgttggtttttcggatgcgccgcggcgcatcagatcggatcgatcactaatttcttgccgtccaggcgtatctgcgccggcttgccgagcaccggatcgggcagcggcacttcgttggtgcggtagatgcccgcgatggccaccagctgcgcttccatgcaggtcgagaagatgcgcgcctcggtattgccgcgcgctccggcaatcgccttgccccgcagcggtgcgtacacatgcacgttgccgtcggcaatcacttcggcgccaaagctcaccactgccgtcaccaccacgtcgccgccgcgggcgtagacctgctggcccgaacgcagcggcttgtcgatcaacagcgtgccgttggccggcaccggcacttcgcgcacgatctgcggcgcttcgctggcgggtgctggcgaagcagcgggcggcgcgggggagcgcggcgcgggcgcgacgggcatggccgtgaccgagagaccggccgcgcgggccgccgcattctgggcgtcgttgcccccgcgcaccgcaatgggttgcgtctggtggcgcgccagcaggccgcgcagcgccgcgaagtcgagcgctgcgggctcctcgccgccttcttcttccggctgcagctgcgagaggtcgatgaccaccggctcctgctcgaagaaatcgggcgaatcggccaactgggcgtcgagcgcctcagccagcacggccaggtcggccgtcttgaggatcactgcgatcagcggcagcgtggcgctcttgaattcgaaaaccgccttggtgcgcgcggcggagacatcggccattggaaaacgtcggtgcgaaaagcgttgaagtctaacgggcgcgggcttccggccagtgaccgggccctgcttcaaccacttggcagaacatttattgcaaggcgtttcactttgaaagggcggaagcgttgcgcgttcgccccagaagtgcgtaaagaatgatcgcaccgaaagtcgcggttccaatgccgcccagcgcgaattggccgaacttcaaggtgaagtcgccggtgccgatgatcagcgtgatcgcggccacgatcaggttcttgttctgcgagaaatcgaccttgttgtcgacccagatcttggcgcccgcaatggcgatgaggccgaacaccacgatgctcacgccgcccatcaccggcagcggaatggcctggatcagcgcgccgaacttcgggctgaagcccagcaccagcgcgatgagcgcggccaccacgaacaccgccgtcgaatagatgcgcgtggccgccatcacgccgatgttctcggcataagtggtcacgcccgtgccgccggcggcgccgctcaccacggtggcaatgccgtcgccgatgaaggcgcggccgatgtacgggtcgaggttgcgccccgtcatggccgtgaccgccttcaggtggccgaggttttccgccaccaggatgatggccacgggtgcgatcagcagcatggcgttggtggtgaacaccggggcggtgaaggtgggcatgccgaaccacgccgcattggcgatgccgctcaggtcgaccggcttgcccatgccgaagaggttggtcagcagcgcatagaccgcagtagcaaggatgagcccgatcaggatcagcaggcgctggagcatgccgcgcgtgaacaccgccaccagccccacgcagagaaaggtgacggcctgcatccacgaatcgaaattgctggccgccatgttcttgatcggcacgctcgccaggttgagcccgatcaccgccaccaccgcgcccgtaaccaccggcggcatgaagcgttcgatccagccggtgccgatggcctgcaccagggcgccgatcaggatgtagatcgccccgcaggccacgatgccgcccagtgccacggcgatgttggcattgggccccttgcccgcatagccggtggccgcgatcaccacgccgatgaacgcgaagctcgagcccaggtagctgggcaccttgccgcccgtcaccaaaaagaagatcagcgtgccgatgccgctcatcaggatggcgatgttggggttgaagcccatcaggatgggcgccagcaccgtggcgccgaacatcgcgatcacgtgctgcacgcccatggcgccggtctgcagccagggcaggcgttcgtcgggcgcgaccacgcggccctcggtggcggcgacttcgcgccagctgaatagattgctcatgagtttgctttctcctcgtcttgtgtttttgaggggcttcttccggcccgctgccacccgtctgttggacgggattcttgcttgcctagcgcggcggcagcaccgccattgtgatgcgcgagacgcaggtcaattcgccggcgtcgttggtcaggtcgatctgccatacctgcgtggtgcgcccgcggtgcaccggccgtgcggtgcccgtgacccagccgctggtggccgagcggatgtggttggcgttgatgtccaggcccacggcccggtcgccctccggggccgagtagtgcgcgccgcaggagcccagcgtttcggccagcaccaccgacaccccgccgtgcaggatgccgtagggctgccgggtgcgctcgtccaccggcacgcgggcgcggatgaagtcgtcgcccacctccaaaaactccatgcccagcgtggagacggcggtgccgatgtggttgcgggtcagctcttcgaccgagatgtcttttttccagatgcgcatgaggttgtctccagtacggggttccggaaactatagcgatggcggctgacaaccgcagtcgcctttgcgtgctaagttggttcgatgaagcaccccgtccgacgctggctcatcggcattgccgtggtgttgctgctcggcaccggcgcgctggtgtgggttgcgagcacccgccttcccagcgacgaggaagtggccgcgcgcatttccgaagcgttcgaaaagcgctttggcgtcggcctgacgatcggcggcgcgcattgggcgctgtggcccagcccggtgctggtgctgtcccaggtggccaccgagcagccgcgcccgatcaccctgcgccgcatcacgctgcagctcaagctccggaagctgctgcaaagaatcgtcgccgtcgacgaggccgaaatcgaaagcctggtgctgccgcgcgaatcggtgcgcgccttccgcggcaagggccccaagccgaaggagggcgaccgcatcttcgcgctgcccgcgccctgggcgctggcgcccattccactcgaaaaggtgcgctggcatgacgtggtctggatcgaccggcgcggcatcgctctcgcctatgacggcgacatcgttttcgacacccactggcgcccgcgccaggcgcgcgtcgaacgcgccggcgcctcgcctcccgcccggctgcgcctggaccgcgaagccggctgggaccgatggcacacccgcatcgacgtgggcggcggcacgtggaacggcgtcacgcgcttcgagctgctgcccgatgacacgatgcgcgtgtcggccgaactcgagccccggcaggtcgacatcgaagggctggtgcaggccttcggccggcgcaccgccgtggcgggcaagttttcgggccagaccacgctggtggcgcaagccggcgagcttggcgcgctgatccgcagcctgcacacgcgcaccaccttcacggtgaagcccgccacgctcacccggctcgacctggccaaggccgtgagcaccgccggcatcagccgcggcggcaccacgccgctcgacgagctcacgggcaccctcgacacgcaaggcggcgaagacggcatcgtgatgcgctacacggggctcaaggcgcgctcgggcctgctcaccgccagcggcaacctgaagctcttcaaccgcaagctggacggcgaagtggcggtcgatcttgtcgacggcgtggtcggcgtgccgctcaaggtgagcggaagcatgagcgaacccgaggtgtcgctgacgggcggcgcgctggccggtgcggcggtcggtaccgcggtgctgccgggcgtgggcacggccatcggcgcgcgcgtggggcagcaggtggaaaagctgttcggcgcggaggagcccgcgaagaagaagacgccgccgcagccgcaaagatcgccgggcgtttcccgctgagcgccctcctggcgcggtggctcaactgcgcaactggatgatctgcaggtcgtggtgtgcgccggcgtgcaaccgcgcaacttcggccgcgcgccgcgtgagcaccgcgcgctggttgatgtagcccttgtcggtgatctcgcccgcgtcgaggctcggcggttcggtgagcaccagcgcgcgcgtcgggcattgcgaagaaccggcgccttcctcgcggagcgtgcgcagcacgtcggcgatgcgctcggccaacgcttgcggcgcggcctgcgggctgggaaacaccagcatgccgatttcgccgcggtcatggcccgtgagcaccacgtcctgcgcatgcggcgccagcatcgacaccagcttgacgcgcaaggtacccaccgacacccaggtgccgctcgaaagcttgaagtcctcggccacgcggccgtcgaagatcacgccgcgctcggcacgctcggggtcggcaaggtagcccgcatcgccgatgcggtagtagccctcttcgtcgaaggcctcggacgtttcgcgcggtgcatggcggtagcccgggaacaccgagacgcccttgacgcgcatctcgagcttctggccgttgggcacgaacttgagttcgagccctggcagcggcgagccgatgcagcccgcgccgtcgagcttccagtgcgccgaggtgatggcgggcgacgtttcggtcgcgccccatgaggtggtgagccacagcggccgctcgggccgcacgcgcttggccaccgcttcgagccgctgccaggtcgagggggcgagcgccgcggccgcgtagaaggcgagccgcaggcgcgagaacacttcggcggccagcgcatcgtcggcttcgagaaacggcagcagcatgtcgaagccgcgcggcacgttgaacagcagcgtgggcttcacctcgcgcaggttgcgcaccgtcttttcgatgagccctggcgcgggccggccctcgtcgatgtagagcgcaccgccgtggcatagcaccatgttcaggttgtggttggcgccgaaggtatggctccagggcagccagtcgaccagcacgggcttttcgtgctcgaggaagcgccaggtctgcgccatcatctgctggttggcgcacagcatgcggtgcgtgttgatcaccaccttgggcttgccggtggaacccgaggtcagcaggtatttggcgtgggtgtcgggcagcacggcttcgtgggcctgcatcacggccggcgtttcgctggcctgcagcagttgcgcaaagggcagggcgccggggtgggcatcggcgttgcggctgaacaccgccaccgcctccacgccggagcccgcgagcgcgccgccatacaccttggcatccgatgcgtagatcaacgccggctgcagcgcctgcagcatgccgtgcagccgcgacggatcttttgccatgcgcgaatacgcgctcgacagcgaacaggccgtgcggccgatgtgcattgccgcgagcatcagcacggcgtggtcgatggcgttgtccgagaggatcgcgatgggcttgcccgccggcaggtccaggtcgagcagcgcctgcgccaccgcacccacggcatggcgcagcgcgcggtagtcgagcttgcgccagccttcgccgctctcgtcgcgctcggcgaaggccagcgcatcgggcgtctcgcgcgcccagcgctcgatccattcgccgatgcagcgcgcgtagggcttgagcgccaccggcgaacgcagcgcaaaggagccgtcatcgaagtcgatgcgcaccgtgcgcggcggggcgatctggcgctcgtccaggaggaagtcgtggttgctcatttcaatcgagtctgccggtgtcggctttggcgcgaatcaggtttaacagcaggacgtcgcgcgcggcctcgaggtcagccacgcgccgcgcgcccagttcttcagccacgccctcggtcaccttggccttgagttcgtccgtcattgacggcgctccgaggtccttccaccagtcctcgatcggcccgcccaggtgcgcgagcacatgtgcgatgccgccggcgccgcccgagagatgcaggttcatgaagggccccatcaccgcccagcgcaggccggggccgtgcgcaatggcggtatcgatgtcggccacgctggccacgccttcattgaccaggtgaaaggcctcgcgccagagggcggcctgcagccggttcgcgatgtgccctttgacctcgcgcttcacgtggatcggccgcttgccgatggcggcatagaaggccatggtgcgatcgatggtctcggccgatgtgcgctcgccgcccaccacttccaccagcggaatcaggtgcggcggattgaacgggtggcccagcaccacgcgttccggatggcggcattcggcctgcaccgcgctgatggcgagccccgaagagctcgatgccaggatcgcgtgggcgggtgccgcctcgtccatgcggcggaacaggtcgaccttgaaatccagccgctcggggccgctctcctggacgaaatcggcttccgccaccgcgtcttcaagccgcgcatgaaagcgcagccggccggccgaggcaccctctgccagcccgaagcgttccagcgtcggccagtgcgcggccaccgccgcgcgcagccgcgcctcggcatcgggcgaggggtcggtggcgtccacgtcgaggccgcgcgccaggaagaaggcggcccaactggcgccgatgacgccggtggcgaccaccgccacgcgtttcggattcggttccatcggcatcgtttcaggattccgccgtgaagccgatcttctttaccagcggcccccagcgctcgccctcggccttttgcgagcgcgccatctcctcggccgtggagccctgggcgatcaggccgaccacggccaggctgtccgtcaccaccttttccttgatggccgcattgatcgcggcattggcggtggccaccacgctggccggcgttttggccggcgcgtagaagccgaaccactcctcggtggtcagttccgcaaagccctgttcggcaaaggtcggcacttccggtgagaacggcgagcgcgccttgcccgaggtggccagcagccgcagcttgccggccttgtggttggggatgaagtcgccgctgggggtgaccatggcggcgatctgcccgcccaccacgtcggtcacgccgggaatggagccgcggtagggcacgtgcttcagttcgaccccgttgttgaggcccagcagcgcgccgatgaagtgcggcgtcgaaccggccgccggcgagccgtagctggcctggttcgggttggccttggcccaggcgagaaagtctttcaccgtgcgcacctcggacggcaccagcgggccgaccgccaggccgtggtgcatgacggcggcaatcgacaccggcacgaaatccttgcttgggtcgtagctgagcttgctgtagatgtgcgggtagatcgacgtgcacgagaacggcgacagcgccagcacgctgccgtcggccggtgcgttcttgagggtttcgagcgcgatgcggccacccgcgcccggcttgttttcgaccacggccgcattgcgggtgtaggccgagcccgcgagcttttcgcccacgcggcgcgccacgctgtcgccggcgctgccggcgggaaagccgtagtagatcttgacctgttcgagcgcctgggcgaatgcagccagcggcgagagggtacccagcgcagtggctgcgcccagggtgtggaggaagtggcggcgggtgttcatgaaatgtctcctactaatatcttcagggcggtttctggcgggatgacggccgcttcaatgcggcgcgaattcggggcgcggcccgcctctgcgcggcagccccatcatctgccttgcctcggccggcgtggccacttccatgtcgagctcatggataacgcgcacgatgcgctcggtgagctgcacgttggtggcgagctcgccctggcggaaataaaggttgtcttccagtcccacacgggcatgcccgcccagcagcagcgccgccacgttggcctcgagctgcgaggggccgatgccgctcacgcagaagatgctgcccttgggtagggtgtcgaccatcatctgcaggaagcgcggcgaatagggcatcgcgttctggaagttgcggtgcacgttcatcaccaggttgatgaagtagggctcgtcgtcatggccttcttcgatcagcgtggtcgtgtcctgcaggatgtgcgtggggctgaacacctcccactcgggcttgatgccgcgcgccttcatgccggcggccagctcgcggccccgggtgatgggcgtgtccatcaggatctgcttgccctcgaagctcaggttcagcgtggtcgcatccagcgtgcacatctcggcgcccgcatccatgcccttgatgcgctcttcccacgcaatttcccagcggtcgccagccagcggcttcaccatgtcgccgtgcaccccgccgccggtggagttgttgatgacgatgtcgcagccgcccgcgcggatgcggctgttgatgtcgcggtacacgtcggcgttgcaggtggcaccgtcgtcgggccggcgcgcgtggatcgccaccacgctggcgccggcgttccagcagcgcagcacgtcggccgcaatttcggccggctgggtgggaaggtgggggttctgcgacttgtgcgccatgccgccggtgggggcgatggtcacgatcactttgcgcttcgacgacatgctccggagtctcctggtgtcttctttcatgaggggcgcgctattatttttggaggcgcaggcacactcagtcattgcgacgacatttggggtcagggtttacgcggcgcgggccgcgcccatgccatcaggagctttcttttcatgcctacgacgaagccggccatcaaggcggcatcgctgacggttgcgcagctgcttcagcgctcggcctggtttccgctgctcgacgaggcagcgcgcgagcgcgtgctcgatgaaatccgcgaggtcgaggtagcggccggcgccgccctgtgccggcgcggcgatacgccgctgcactggtacggcacgctcgaggggcttctgaagtggtcgatcacctcgagcgatggccgctcggtgaccttcggcgggctctcggtcggcagctggttcggcgaaggcacgctgctgcgcggcgctccgcgctcggccgacgtcattgcgctgcggccgagtcgcgtggcccagctgccggtagagactttcgagtggctgcaccgcacgcagcgcggcttcgaccattttttgctgcagcagctcaacgagcggctgcactggttcatgggcaactacgcggctcaccggctgctcgacgccgacagccaggtggcccgtgcgctggcggggctgttccacccgtggctgtatccgggcagcgagccgcatctgcagacctcgcaggaagagatcgccaacctgtcgggtgtttcgcgccagcgttgcaatgcggcgctgaaccggttgaaggaggcggggtttttgcggatcgagtacggcgggattaccgtgatcgacctggaagggctgcggcggttcatcgagtaggggaaagggctggcgcctttgggaagtccttgctgtaatgcgactggacgggtgtgtgtttcacgaaatgctcatagccctcggagatccaattcacggcaagcgcctcgaactttctcgcaacaggcccgtatggcttccccggaatcaattcatcgcctcctcgccgtcgcttcaagattgctggacagcgccgcttcagaaatacgggacgcgaagctggagcctgttcgcgagaacatctcgcagatcggtcacctcattgctggaatattcgagattcagcaagagatctacgtgctccgaccggatctgaaaccggcttacctgagcgaaccctcgccgtattccgcttccaacaagttgctcactcggttcatgggcgaggccttggagcatgaagacgcaggcgaaattgcaatggccgtcgagaagtacagggaatacctcggcctcgaagagtcgacctttcatcgcgaaattgcggaacgcgagctcagtcgtctcttgaacagaaacaactgatccgtccatttcacttcgctggcttcgccttgtccgccagccgcttgcggtactccgtcgtcgtcaggccgccgaagccccagtcgtcggtgtcgatctcctcgatcacgatgtgcgtccattcgggcggcttgttcagcacgcgttccagggtttccgtgaactcggcgatgacctgggttttctgttcgcgcgtgacgccgtcgcgggtgatcttcaggttgatgaaaggcatggtgtgctccttggaatggatgaggtgattaccacttgcccgtgctcatgccgccgtccaccggcagcaccacgcccgtcgtgaaatcggcgttcgtgagatagagcaccgcatcggcgatctcgcgcacggtcgcgatgcggccggcgggcgagaggccgttcaggaagccgtgctgctcgggcgtgtacagcggcgtgtcgacgatgccgggtgccaccgcattcaccttgacgttgtgcggcgcgagttcgagcgccagcgcgcgcgtcgcggcgttgatgccacccttgatcagcaccggcagcgcggccggcacctgctggttcggctgcagcgcaatgcttgcggtgatgttcacgatatggccctggcggcgcgccaccatgtgctttgccgcagcttgcgaggcgtagacgaaacccttgaggttcgtggccaccagctggtcgagttcttcctcggtgtattcgacaaaaggcttggcgttgaagatgcccgcgttgttgatgagcacgtcgacctggccgaagcgctccacggcgcggtcgatgagctgctgcgcggtgtcgcggcggccgatgtcgccggccacgccaagaaagcgcgtcgggttcccgagttgctttgccgcggccgcgaggcgttcatcggttcgcgcattggcgaccacgttgaagccacgttcgagataagcctgcgcgagtcccaggccgatgccgctcgaggcaccggtgatgacgaccgtggacggggtgttgagggtgtcttgcatgtcggtactccaaagagttgagggaatggatgaactgtattgatgacgccacaggagataaatcactagactcgtacttcaattgatacgtgaggtaatcaatccatgcagcggcagttcggcgacatccttctcggcagcatcgagctgttctgcctggcggcggaaacgggcggcttcacctcggccgcgctggccgcgggcgtcacgccggcggccgtcagccgctcgatctcgcggctcgaaaaacggctgggcttgcgactcttcgtgcgcaccacgcgcagcgtgcggttgaccgacgcgggccgctcttacttcgcgcaatgccgccaggcgctgacgcagttggccgaagccgagcgcgaggtcatgggccagcaggcgcagccctcgggcatgctgcgcatcagcgtgcccaccacctacggccaccaccgcttgctgccgctgctgccggtctttcgcgaacgctttcccgacatccggctgcacgtgcacctgagcaaccggaacatcgacttcgtggaagagggctacgacatggccgtgcgggtgcgcgcccagcccgactccacgctgatcgcgcggcatctcgaggatgcgcagctggtggtggtggccggccgcaagtatttgaagaaggccggcacgccgcgcacgctggacgatctctcggcgcacgagtgcatccagttcgagttgcccagcagcggccgccgcatctcatggctcttcaaggagaacggcaaggaccgcgagatcttcgcggacagcgcctacagctgctccgacgacgtgctgggcggcgtcacgctcgcgaaaagcgacgcaggactcttccaggcctaccgcttcgtggtggaaaaagagctggccgacggctcgctcgtcgaggtgctgcagcctttcgcgggccgctcgcggccctatacgctgctgtacccggacgggcggcacgtgccgctgcgcatgcgggtgttcatcgatttcctgatggcgcagcgggccgcctgaggcgccttacacacccagcaattcttcgagcgcctgaggctccgccagcaggtcggccgacgcaccgtgccgcacgatctgccccttctccatcaccaccgccaggtcggtgtgcgcgagcaccttgcggtagtcgcggtcgacgatgagcgtggcgatgccggtgctgcggatttcgccgatcacgcgccagatctcggccacgatcagcggcgcgaggccttcggtggcttcgtccaggatgagcaagcgcggattggtcatcagcgcgcggccgatggagagcatctgctgctcaccgcccgagagctgctggccgccatgcgagagccgctcggcgaggcgcggaaaggtggccatcacgcggtcgaaggtccaggcgcggtgcccgtcgatgccggcgcgctcgctcatcacgaggttctcacgcaccgagaggttggggaagatgccgcggccttcgggcacgtagccgatacccaggcgcgccatcttctccggcggccagccggtgaccgtgcggccatcgacctgcacttcgcccgaggcggggcgcacgtagcccatcatgctgcggatcagcgtggtcttgcccatgccgttgcgcccgagcaggccgaccgacgtggcggccggaatgccggcatgcacgccgcgcaggatgtggctgttgccgtagtaggtgttgagatcgcggacgacgagcatcagtggtcttctccaagataggcggtgcgcacttccgggttttcgcggatcgaggccgggtcgccggtggcgatgacggtgccgttcaccatcaccgtgatgcggtcggcaatgcggaacaccgcatccatgtcgtgctcgaccagcaggatcgcatgggtcgatttcagtcgtgcgagcagcgtgagcatgcggtccgtttcctcggcgcccatgcccgcgagcggttcgtcgagcagcagcacgcggggcttggtggccaggcacatcgccacttcgagctggcgctgcgcgccgtggctcagcgtgccggcaacgcgccgggcttcgttcgacaggcccgcggcctcgagcgccgcatcggccgccgcattgctggccgcgcagcgctgcgacgactgccacacggtccagggccgcgccgtggcggcctgcgccgcgagccggcagttctcgtgcacgctgaactccgggaagatggtcgtgcgctggtagctgcggcccacgccggcacgcgcgcgtcgccattgcgcgcgctgcgtgacgtcgatgccgtcgagcgcgatgcggccttcggaggcttcgatttcgcccgaaagcatgttgatgagcgtcgacttgcccgcgccgttggtgccgatcaccgcatgcacttcgccgacgtgcaggtcgagcgtgacggcgttcacggcggtgaggccgccgaagcggcgcgtgaggccatgaacggaaagaagagcggtggcgttcatggtttggctccttccccctttgggggaaggttgggatgggggcgggcagagcgctcggtggtggcgccgcgtgcccccaccccagccctcccccgggaggggagggagaaacacagggagcaggtcatgcggcctccttgggagacagccgcttgaccaggccgatcagacccttcggcaacagcgccacgaacacgatgatcgcaatgcccagcgtcagctgccagtggtccgcaagcggccccatcaccgcatgcgtcgagaagatttccttcagcagcgtgaacgcaatggcgccgatcaccgcgccgcgcaaatggccgaggccacccaggatcaccatcagcagcacctcgcccgagttgtgccatgccatgagctcggggttgaccacgccgtcgcgcgaggccagcagaaaacccgcgagcccggccagcgcgcccgccagcacgaaggccgcgagcttgtagccgtacaccgggaaacccgccgcgcgcatgcgctgctcgttcacgcggatgcccgccagcgccgcgccgaagcgcgagcggcgaaccaacgccaagaggccgtaggtgaacaccagcgacgcgagcaccacgtagaacagcaccatgcggttttccatgtcgagtttgccgatggcgggccgcacgtacatgtagatgccgtcgctgccgccgcccaccttggtgtcgtggaacacgaagaaggccatctgcgcgaaggccagcgtcaccatgatgaagtacacgccgcgcgtgcgcaggctcagcgcgcccacgaacaatgcatacagcgccgccgcgcccatggccgccggcagcagcagcgcgaggttgccgccctcgttgcccgaggccagcaccgtgacgtaggcgccgatgccgtagaacgccgcatggcccaggctcacgaggccggtcatgccgaccagcagttcgaggctcagcgcgaagatcgacaggatcatcaccttgacgacgaagtccgagacgtagttgcccatgagcgggccgagcacgccgatggcaatggcgcaggccaccggcacggcgaacgcgcccagccgcatggaggttgtgcgcatgggggtggtggcttcggtcatggccgcctccccatcagcccttcgggcttccatatcagcacgatggccatcaacaggtagatgccgatgccggcgaggtccgcgaagaacaccttgccgaaggtgtcgacgaagcccaccagcagcgaggccagcagcgcgccggtgatcgagccgatgccgccgatcaccaccagcacgaagcagatgatgagcacgctcgcgcccatgttcggatacaccgaggacatcggcgccgcgatcattccggccaatgccgccagcgccacgccggccgcaaacacgatccggtagagccgcttcacgtcgatgcccaggccacgcaccatgtcgcggttgctcgcgcccgcgcggatcatcatgccgagccgcgtgcggttgaccacccagtacagcccgaccgcgagcacgatgcacgcggccgaggcaaagagccggtaccacgggtagctcatgacgttgccgagcgcaaagctgccgtccagccatgccggcaccttcacgccgtgcacgtcgttgcccacgaggatggagcgcagctcctcgaacaccaggatgagcccgtaggtcatgagcacctgctgcaggtggtcgcgctggtacaggtagctgaagaaggcccattcgagcaggtagccgaagacggccgccagcaccacgccggccaccagcatcaacagaaactggtcaccgaacagcggcgcgagcgcgaacgccatgtacgcgccgatcatgtagaaactgccgtgcgccaggttgatcacgcccatgatcccgaagatcagcgtgagccccgaggccaccaggaagagaaggagtccgtactgaaccgagttcaggcactggacgaggaaggtgccgaaatccacgttggattcatccctgtgagatcgtgaggggagcgtggcgcgttagcgcccgcgatgttcgtgagacaccgcggatccggcttcgccggtccgctggtgtcgccccctcaaggggggagtcgagctacacgaagtgagcgagggacgggggtgggtcacattctgcagccacgggccgggtctgcgagccccttgatcgccgtgctcaccagcttgttctccttgccgtccaccttgcgcaggtagatgtcctgcaccgggttgtgcgacttgctcatggtgaacgagccgcgcgggctgtcgatcttggccttctcgatggcggccgtgaactccgccttcttgccgatgtcgcccttggtggcggcaaggcccacgcccagcatctgcgccgcgtcatagccctgcaccgcgtacacatcgggctgcagcttgaaggccttggcataggcgacgcggaaggcgttgtcgcgcgcggtgttgaggccgtcggcgtagtgcagcgtggtgagcatgccctgcgcggcctcgccctgcgcatcgagcgtgccgtcggtcaggaagcccgggccatagagcggaatggtcttgttgaggcccgccgcctggtagtccttgacgaacttcaccgcgccgccgcccgcgaagaaggcgtacaccgcatcgggcttggccgccgcgatctcggtcaggagcgcctggaactcgacgttgggaaacggcagcgtgagctgcttctcgaccttgccgccgttcttctcgaagccttccttgaagccgttgaccgactcctcgccggccgcgtacttccaggtgatggtcatgaccttcttcttgccctgctgcttggccgccacctcgcccatggcgtaggccggttgccagttgctgaacgagctgcggaagatgttgggtgcgcacatcgggcccgtgaccgcgtcggcgccggcgttcggcacgatcagcacggtgccgctttccttcgcggccttggccatggccatggcgacgccggagtgcacggtgcccacgatcacgtcgacgttgtcgcgcttgatcagcttgttgacgttgtcggtcgccttggcgggatcggactcgtcgtcgaccttgaagtattcgatctcacggccggcgagcttgccgccctgctcgtcgacgtagagcttgaagccgttctcgatggccacgcccagcgcggtgaaagtgccgctgtacggcagcatcaggccgaccttgagcttgccggtgccctgggcgccggcggcggatgccagtgcggcgaatgcgatcgccgtgagcgcgaggcgggcggtgcggatggtcatgatggctgtctcctgtttttaccaatgaaagaagtggtcgcgacgatgacacgatccggctgatcgcgatgcggggaatgcccgcattccgggatttccaccagttcgcagccgggcacgcgcgccgcgatgccgcggatttgcgcgagcgtgccgtattcgtcgtccgtgccctggatggcgagcaccgggcagcggatggtgtcgagttcggcctcgatgttccattcgcggaagggcgggtccagccagatgcggttccagccccagaaggcggagtcggcattgtcgtggtagcggccgagcttcttcggcaggtcggtgccgagataggcgctgcgcgcctgttcgatgttctcgaccgtcacgtcttccacgaagatgtgcggcgcgaggaccacgaggccttgcacgcggtccgaaaaacgcgaggcgtagagcagcgagatcgagccgccgtcgctgtggccgaagagccagggtttttcatcgtcgacgatcttcagcgcggcgaacagcgcgggcagcacctcgtgggcctggcggtgcatgaagtcgacgtcccagatctcgttttcttcgcgtggcgtggagcggccgtagccgggccgtgaaaacacgaggccgcgcgcgccggcggcttcgcagagctgcgcgggaaagtccttccacatggcgaccgagcccaggccttcgtggaggaagacgatgagccgggcatcggtgcgctcgggggcgatccaatggcattcgatgcggacggggcggccgcgccagtcgatggtggcgaagtcgggggtcatggctgttgccccctctgcctctgggagagggcgggggtgagggccagcggcgctggcaaaagctgtgcgccagcgaaggccgatgccctcaccctagccctctcccagagggagaggggacaaagcgggaatctcatgcctgcttctcccgctcacgcaacctgaaccgctggatcttccccgtcgccgtcttcggcagctcctgcacgaactccaggaaccgcgggtacttgtacggcgcgagccgctccttcacgaaagccttcagttcgtcgtccgtgatcgagtggccgtccttcagcacgacgaaagccttggtcttggtgaggccgtccgaatcttccttgccgatcaccgcggcctcgagcacggcggggtgctgcatcagcgtggcctcgacctcgaagggcgacacgtagatgccgctgaccttcagcatgtcgtcgctgcggccggcataggtgtagtagccgtcggcatcgcgcgtgtacttgtcgccgctcttggtccagccgccctggaaggtctcgcgcgacttctcgcggttgcaccagtacatcagcgccgagctcgggccgcggatgtagaggtcgcccacttcgccgtcgggcaccggccggccgtcttcgccgcgcagctcgacctcatagccttccaccggcttgccggtggtgccgtagcgcacgtcgccggggcggttggagatgaagatgtgcagcatctcggtggagccgatgccgtcgatgatctcgcagccgaagtgcgccttgaagcgctgcgcgatctcgccaggcagggcctcgccggcggaagagcacatgcgcaatgcgacggcttcgcgcggcggcagcttcggcgaggcgagcatgccggcaaagccggtgggcgcgccgaagaacacggtgggtttgtgctcgacccagcggcggaaggtggcgtcgggcgtgggccgctcggccatcagcaccaccgtggcgccgaccgaaagcggaaaggtcagcgcgttgccgagcccgtacgcaaagtacatcttcgcggccgagaagcagacgtcgtcttcggtgagcccgagcaccggcttgccgtagagctcggccgtccaccacaggttggcgtgcgtgtggaccgtgcccttgggcttgccggtcgagccggaggaatacagccagaagccgggatcgtccgaggccgtgggcgcgggcgatgccatcggctcggcagcggcgagcgcggcctcgaattcctgcgcgcccgcgggcagcgcagccgtcggctgcgaagcgatgagcgtgtgcacctcatgcgcgccgcggttcatcgcgtcttgcagcgtgggcagcagcgcgcccgacaccagcacggcctgcgcgcggctgtggtcgagcatgtaggcgtagtcgtcgggcgtgagcagcgtgttgacggcgacaggaacgacgccggcataaaggcagcccagaaaactcacgggccagtcgccgctgtcgagcatgagcagcagcacgcgttcttcgcggcgcacgccggcggccttcagcgcggcagccaggcggcgggcgcgctcttcgagctggccgtagctgagcgtgccgcggtcgtcgatgtaggcggtgcgatcggcgcggccgcggttgagggcgaacaggtgttcggcaaaattgaatcgtgcgggcgggctcgtcatggggtctccttgggccgtgttcttttttctagaggccgagctgcgcgagcacgccggggctcgcttgcacggcgctgcggcgatggtagaagtccagcgcgcgcagtccgccgagttcggcgccgccgccggcacggcccgggccgccgtgcagcgacatcggcatcacgttgccgtggccggtgtgggcctgtgccacttcgggcgtgaccacgtgcacgcggccgtggctcggcgcaacggccaatgcggcctgtgccaaggcagcgtcgtcgctgccgtagagcgaagtcaccagcgaaccctggccgcggtgcgccagcgcgatgccgtgcgcaaggtcgcggtagggcagcagcgtggcgaccgggccgaacacttccacgtcgtgcacgcgctctgccgcatcggcatcgcgcgcgcccagcaacacggggccgatgcaggccgccacggccgggttggcgtcgaccagcggcgtgctgcggccgtcgtacagcacggtggtctgcgccgacagcgcctccaggccttcgttcaccgcgtggagctgcgcgcggctcacgagcgaacccatgcgcacgctctcgttgcgcggattgccgaccgtcacgcccttgagcttggcgccgatggcttcggccgcggcgtcgtacacctcggccggcaccaggatgcggcggatggcggtgcacttctggcccgacttcaccgtcatctcgcgcaccacttcgcgcacgagcaggttgaaggcgtcgctgccgggcgcggcgccaggcatgagcagggcgctgttgaggctgtcggcctcgatgttcacgcgcaccgagcgctcggccacggccgggtgcgagcggatcaccgccgccgtttcggccgagcccgtaaaagagaccacgtcgaaaggctgcagcgcatccatcaagccggcggaactgccgcagacgaccgacagcgcaccggcgggcagcacgcccgcatcgaccacgtctttcaccatgcgctgcgtgagccaggcggtggccgtggcgggcttcacgatcacgggcacgcccgagagcagcgcgggcgcggccttttcccacagcccccacgaaggaaagttgaaggcgttgatgaacagcgccacgccctgcgtcggcagctggagatgctgcgactggaacaccggctccttgccgagcctggccgcgtcgccgtcgcgcagcgcgcgcacgtcgcccaggccgtcgccccacttggcgtactggccgagcgtgaagatcgcgccgtcgatgtcgacggccgagtcgttcttcaccgtgcccgaattggccgtggcaatctcgtaatacgcatcgcggttggcctgcagcaccttcacgacggcgccgagcaggcccgcgcgctggcggtaggtgagggcccgcagcgcgctgccgccctgttcgcgcgcaaaggcaaaggccgcgggcaggtcgaggccggtggcgtcgacgcgcacgagctcggtgcccagcaccgggtcgaacaagggcgtgccggcgcccgatccgctttgccagcggccggcgacgtggttgggtaggagctcggtcattgggtgaatttgatctgcccttcgggcaagagatagagaacgagcgcgcggccctgcgccacggttggtcggtgtgcggtgccggggccgtagacgcaccagcccgcgggtcgcccgtcgaaggtggcatcggcgctgccctcgagcggcatgatcaggtcgatctcgccgttgggatgggtgtgatgcggcccggcgatgtcctgcatgtcgaccacgtcgaccgagaaccggtgcagcgcgtcttcggccttgaacacgcggccatacttgatgccgccgccttcgcgctcgcacagccagccctcggccacgccgccgatgcaggcctggcgcagttgctcgaaacgcgggctgcccgcgccatgggtggcgttgagccactggtcgagttgttcgtcgagcggcctgccggcaatttcggcggtcaggccggcgatcaactggtgaaatgcttccttgctggacattggcgggcttcctttgggaggctggctggcagcgatggcgccacagcgaaacttacgatctaccttgcaggattggtgcgcgtgcagtatcttgcttgtgatcgaacaataagcaccgagacatcgggtgtcaagcaatatagtgcatatatggtgtttaccctgagcgcgcacaatcccggcctagaacgaggacttgcatgaacgagcatgtagacgcggtgctgcccgccgcgcgcgacggcaaccacgccagcaacgccacaccgccgggagaagccaggaatccattgctggccgctttgggcgaccgcgtgcgcaacctgcgcgcgcagcgcggcctcacgcgcaaggcggtggcggtgtcggccggcgtttcggagcggcatctcgccaacctcgaatacggcatcggcaatgcgtcgatcctggtgctgcagcaggtggccggcgcgctgcactgctcgctggccgaactggtcggcgacgtgaccaccagctcgcccgaatggctgctgattcgcgagctgctcgagcaccgcagcgaagccgacctgcgccgcgtgcgcgtggcgctgggcgagctgctgggcacggcctcggtcgatccggcgcggcaccgccgcatcgcgctcgtggggttgcgcggcgcgggcaagtcgacgctcgggcagatgctggccgaagacctcgacgtgcccttcatcgagctgagccgcgagatcgagacgctggcgggctgcagcgtgcgcgagatccacgacctctacggcaccaacgcctaccgccgctacgagcgccgcgcgctcgaggaaaccatccagatctacagcgaagtggtcattgccacgccgggcggcatcgtgtccgaccccgccaccttcaatgagctgctcgcgcactgcaccaccgtgtggctgcaggccgcgcccgaggaacacatgggccgcgtggccgcccagggcgacacccgcccgatggcggccagcaaggaagccatggaagacctgcgccgcatcctgaacggccgcgcggccttctattcgaaggccgacctgtcggtggacaccagcggcaggacccttgcgcaaagcttccaggcgctgcgcgccatcgcacaccaatccatgcgccccggcgcctgaaccgctgaattgaaaaaaagcgattcaggcattgacttgcctgttcgcatgcagcatgatgcatgtcatcggaaccagaagatgcattattcttccggtttgcatctggcccacaggagacttccgtatgaccgagaccacgacccttcaggcgcccccgcgcgtcgactaccgcatcgaacccgcgcaatacaagcattggaagctcagcttcgaaggctcggtggcgcgcctagtgctcgacattgcggaagacggcggcatccgccccggctacaagctcaagctcaacagctacgacctgggcgtggacatcgagctgaacgacgcgctgaaccgcgtgcgcttcgagcaccccgaagtgcgcagcgtgatcgtcaccagcggcaaggaccgcatcttctgctcgggcgccaacatcttcatgctgggcgtgtcgagccatgcatggaaggtgaacttctgcaagttcaccaacgagacgcgcaacggcatcgaagacacgtcgaagcactcgggcctgaagttcatcgcggccgtgaacggcgcctgcgccggcggcggctacgagctggcattggcctgcgacgaaatcctgctggtggacgaccgctcctcggccgtgtcgctgcccgaggtgccgctgctcggcgtgctgcccggcaccggcggcctcactcgcgtgaccgacaagcgccacgtgcgccatgacctcgccgacatcttctgcaccagcgtcgaaggcgtgcgcggccagcgcgcggtcgagtggcgcctggtcgatgcggtggccaagcccgcgcaatttgccgccgccgtgcaggagcgcgccgcgcagctcgccgccggcagcgaccgccccgcgaatggcaagggcgtggcgctgacccgcctcgaacgcgaggaaaccgccgacagcctcagctattcgcatgtcgacatccagatcgaccgcagcaagcgcaccgcgaccatcaccatcaaggcgcccaccggcacccagcccgcggacattgccgccatcgaagcggccggtgccgcctggtggccgctcgcgatgtgccgccaactcgacgacgccatcctcaacctgcgcaccaacgagctcgacatcggcacctggctgctcaagaccgaaggcgacgtacaggccgtgctcgcatcggacgccgtgatgctcgccaacaagaaccactggctggtgcgcgaaaccatcggcgcgctgcgccgcacgctggcgcgcctggacgtgtcatcgcgcagcctgttcgcgctggtcgaggcgggttcctgctttgccggcacgctggccgaggtcgcatttgcggccgaccggacctacatgctggcactgcccgacgacgccgcgcgcgcaccgaagctcgtgctcaatgaattcaacttcggcttcttcccgatggtgaacgaccagagccgcctgcagcgccgcttctatgaagaagccgcgccgctcgacgccgcccgcgccgcggccggcaagccgctcgatgccgacgaggcgctgaagctcggcctcgtgaccgccgcgcccgacgacatcgactgggaggacgagatccgcatcgccatcgaggagcgggccgccatgtcgcccgatgcgctcaccggcctcgaagccaacctgcgcttcgcaagccaggagaacatggccacccgcatcttcggccggctcaccgcctggcagaactggatcttcaaccgccccaacgccgtcggcgaaaagggcgcactgaaggtctatggcaccggcgagaaagccggcttcgatttgaaccgggtctgaacccgcagtccttcgcacaacccaaggaacaacgatgagcacgatcaactacagcgagaagatccccaacaacgtcaacctcggagaggaccgcacgctgcagcgcgcactcgaaggctggcagcccaacttcatcaactggtgggacgacgtgggccccgagggatcgaccaaccacgaggtgtacctgcgcacggcggtgagcgtcgatccgcagggctgggcgcagttcggccacgtgaagatgcgcgactaccgctggggcattttcctgaacccaggcgatgccaaccgcgagatccacttcggcgaccacaagggcgagaaggcctggcaggacgtgcccggcgaacaccgcgccaacctgcgccgcatcatcgtgacgcagggcgacaccgagcccgcatcggtcgagcagcagcgccacctgggcctgaccgcgccgagcatgtacgacctgcgcaacctgttccagatcaacgtggaagaaggccgccacctgtgggccatggtctacctgctgcacaagcacttcggccgcgacggccgcgaggaagccgaggcgctgttgcagcgcacctcgggcgacgtggacaacccgcgcatcctgggtgccttcaacgagaagacgcccgactggctcgcgttcttcatgttcacctacttcaccgaccgcgacggcaagttccagctggccgcgttggccgagagcgcgttcgatccgctcgcgcgcaccaccaagttcatgctgaccgaagaagcgcaccacatgttcgtgggcgagagcggcgtgtcgcgtgtcctggcgcgcactgcgcaggtcatgaacgagctcaagaccgacgacccgcagaaggtgcgtgccgccggcgccatcgacctgggcacgatccagcgctacctgaacttccactacagcgtgaccatcgacctgttcggcgccgatcagtcgagcaacgccgccatcttctacagctcgggcctgaagggccgctacgaagaaggcaagcgcggcgacgaccacgtgctcaagggccagacctacaaggtgctcgaggtgaaggacggccagctcctggagaaggaagtgccgatgctcaacgcgctgaacgaagtgctgcgcgacgacttcatcaaggactcggtggccggcgtgggccgttggaacaaggtgctcgagaaggccggcatcccgacccgcctgtcggtgccgcacaaggccttcaaccgccagatcggggcgctcgccggcatcaagatgtcgcccgaaggccgcgtggtgaacgaggtcgaatgggccgcgaagagggacgaatggctgccgagcgccgaagacttcgctttcgtggcatcgttgatgggccgcgtggtggagcccggcaagttcgccggctggatctcgccgccggtgatgggcatcaaccgccagccggtcgatttcgagtacgtgcgtttcggttgattggtatgactccctctcccctcggggagagggcaggggtgagggtaggcggcgtccccacgacaagctgccgccccctcaccctgaccctctccccaaggggcgagggaaaggagaaaaaacatggacatggccgttgaagccggagtgatcaagcagcacctgatcgaccccgagatctgcatccgctgcaatacctgcgaggccacctgccccgtcaacgcgatcacgcacgacgacaacaactacgtcgtgcgggccgacgtctgcaatggctgcatggcctgcatctcgccgtgccccacgggttcgatcgacaactggcgcacgatgccgctggtgcgcgcctactccatcgaggagcagctcacctgggaatcgctgcctgccgagctttctcccgaagagttcgaagccgcgggcgtatcggccgaagcagccggcgatgcggcagccgccgtgcccgcacagacccaggcgcaagcccaggccgcggtcgaatccgtcgagccggttttcaactcggcgcaatacggcgccactgtgcccccgtggtcggccgcgcacgcctacaccaacctgtttgcgcccaaggcgccgaccaccgccaccgtggtcggcaacttcaactgcaccgaggcgggcttcgacagcgagacccaccacatcgtgctcgactttggcgtggtgccgttcccggtgctcgaaggccagtcgatcggcatcgttccgccgggcgtcgatgccatcggcaagcgccaccacgcgcgccagtattcggtcgccagcccgcgcaacggcgagcggcccggctacaacaacgtgtcgctcaccgtgaagcgcgtgaccgaagaccaccagggcgacccggtgcgcggcgtgtgctccaactacgtgtgcgacctgaaggtgggcgacacggtgcaggtggtcgggcccttcggcacctcgttcctgatgccgaaccatcccaggtcgcacatcgtgatgatctgcaccggcaccggcagcgcaccgatgcgcgccatgaccgaatggcgccggcgcctgcgcaagagcggcaagttcgaaggcggcaagctcatgctgttcttcggcgcgcgcacccagcaggagctgccgtacttcggcccgctgcagtcgctgccgaaagacttcatcgacatcaacctcgcgttctcgcgcacgccgggacagcccaagcgctacgtgcaggacctgatgcgcgaacgcgccgccgacctggccgcgctgctgaaagacggcgcgagccacttctacgtgtgcggcctcaagagcatggaagaaggcgtggtgctcgccttgcgcgatgtcgccaaggaagccggactcgactgggacaccgtcggtgccgcattgaagcgcgaaggccgcctgcatctcgaaacctactaagctccggcgaatgaagttcgccgacttccaccccggccaggtcatcgaggccgggccctatgtcgtttctgaaaaggagctgatcgggttcgcgcaggcctacgacccgcagtggttccataccgatcccgtggccgcggcggacagcgcctttggcggactgatcgcgagcggctggcacacctgctccatcgcaatgcgcctcgtggtcgatgccgcacttgaaggctccgagtcgttcgcgtcgccggggctcgagcatgtgcgatggccgcacccggtgcggccgggcgatgccctgcggctggtggccgatgtcatcgaggcgcggcgttccgagaagcggcccacgctcggcatcctgcgctggcgctggcggctcttcaatcagcgcgaactcatggtgctcgatgtggaagtcacgagcctgttcaggctcgagccgcccgcctgattcgccaaacaaaaagaagcccgcaacgcgcgagcgctgcgggcttcatgggcgtttacggctccagcgtcttacttcgtgacgtcgacggcgcccgagcccttcgccttgccgctggccttcacgccggcgcccgaaggcttcaccgcgccgccggccgagcccacggcgccggtcgcgctgttcagcgtgccgcccacggtgttcgtgacgccgcctgccgcattggtggcgccgccgacggcgcccgtcgcaccgctcacagccccggtggcaccgccgaccgtatcggtcgctttgcccacggcacccgttgcaccgcccaccacgccgccgagcgtgttgcccaggccgcccgctgcaccgccggcatttccgccagtggaagtggaggtgccggccgttgcggcggttcccgcccctgcgcctgcactgccctgggccggtgcggtcttgacggcacccgaggtgttgacatcggcattcacgcccacgccgacacccacgccttgtgcctgtgcgaaaccgctcatggcaagcaggcctgcgagcaaggcgccgacgacgatggacttgtgttgttgttgctgcttcataggtgacttttcctttcgtttgaagatggccggtgatcggcccgaaccggcttggggccagttcggtcgctaccgtcgcgggccgctcctatgtcgccatgtgcgagatggccgctcgctggtgtgggacctctccgtcgtcggaaaccgggtctcgtgcgttagggccgcggctcttggtggtgttcgaaacccgaccgctcaaaacagccccaaaaatccctctataattcgactcctgaaatgcgggaatagctcagttggtagagcgcaaccttgccaaggttgaggtcgagagttcgagactcttttcccgctccacatttcatgcaaaaggccacctcaccggtggccttttcttttgggcgctgcgaattttttcagcctcttgcgggcagcaccgttccacggctttcgccgaagccgatgcgcgcatgccctggcttttcgcaccagccgcgcagcagcacggcatcgccgtcttcgaggaatccgcgctcttcgccattggccagcgtgacggggctttgcgcggcgcgcgtcaactcgatgatcgcgccggcctcgcccggccccggtcccgagatggttccgctcccgaacaggtcgcccggattcaggctgcagccacccaccgtgtggtgcgccaccatctgcgccacgctccagtactggtgcttgaagctcgtgcgcgacaggcgggaaggcccgcttctgtcgtcgcgcgccttctcgctttccagccacacctccaggcggatgtcgatggcgccgctgtcacggttcgccgggctttcaaggtagtcgagcggctggggctcattggcgggccgcgtccatgcctgccggtagggcgcaagcgcttccatcgtcacgatccacggcgagatggtggtcgcgaagttcttggcaagaaagggcccgagcggtgccatctcccagaactggatgtcgcgcgccgaccagtcgttgagcaggcagatgccgaagatgtgttcttccgcgcgcgcgagcggaatcggctcgccggcggcattgccctcgccgatccacacgcccagctccagctcgtagtcgagccgcgcacaggcgtggtacgtgggcgccttcgcgcccggcgccatcgtctggcccatcggccgatggaagcgctggccgctgacgccgatggtcgatacgcgtccatgataggccgtgggaatccagcggaagttgggcgtcacgtcgccctcgggattcatcaggcggctgatgttcagcgcgtgatcgatggaggtgtagaagtcggtgtagtcgccgatgcgtgcgggcaccgtgtattcgacctcggcctgcggcaccaggcactcgcgcacggcatacaccgtggcggcagctgcatcgctccgcagcaatgcaaacaccgcgtggcgcaacgcctgccaggcggcgccgccgagcgcgaagaaatcgttcagcgccggcagcgcggcggcacgcgccgcatcgagggcgagtccgtcgagcaattggcgtgcggagagcgccgccatgtcgagcacctggtcgccaatggccacgccgccgcgaaacggttccggactgcccgtgcgacgaaacaccgcatacggcaggttctggatcgggaagtcggttccttcgatattcgcggtgtcgacccagctcctgacgcgggcgtcgtgcgtgtggttgagcgcaatcatttatctctcgcctcccgcgttcagaccgacgccatcagcgcgtcgtcgaagatcgccaccgcgcgcgtccacccggccgacgctccgcggatcttgtgcggaaagcagctgatgaaaaagcccgtgggcggcagcacctcgaggttgtgcagcttctccaggtggcagtagccgatgtcgcggccggccttgtggccttcccagatcagcgaggcgtcctgcgtctcaccgtacttcttggcggtgtgcacgaagggcgcgtcccagctccatgcatcggtgcccgtgaggcgcacgccgcgctccagcaggtacatggtcgcttcgtagcccatgcccgcgccggccgagacgtagtcggggttgccgtagcgcgagcccgcgcgcgtgttcaccaccacgatctccagcgggctcagcgtgtggccgatgcgcttgagctcggcctccacgtcgtcggcggtcaccacgtagccatcggcgaaatgccggaagtcgagcttcacgccgggctggaagcaccattcgagcggcacctcgtgaatggcgatggcgggtttcttctcgcccagcgccttgtccatggtcgagtggaagtgatagggcgcatcgaggtgcgtgccgttgtgcgtggaaagctgcaccagctccacggcccagccttcgccatcgggcaggtcttccttcttcaagcccgggaagaagggctcgatctgctcgtaggtctgctcgtgcgtgaagtactggatcttcggcgcgaaggctggcggatcggagagcacatcgttttcgagaaagatcgagaggtcgacgaatttgcgtggcatgtgagctccttgtacggtgttggtatggacggggcgtgaagagttcagggctgctgccagcgcagcagccgcttctcggcaaaggccagcagcgcgttgctcacgaagccgatgagcccgagcagcacgatcccggcgaacaggtcgctggcgcgaaacgcgcgcgccgcgagaagaatggcctggcccaggccgctttgcgaggcgatcatttcgcccaccaccgcaacgatgagcgcaatggtcaacgcgagccgcatgccggccagaatgtcgggcatggcattgggcaggcccatcttccagacgaaagccgcgcgcgacatctgcaggcagcgcgccacctccgacagccgcggctccacggccgcgaagccgtgcacggtggccagcagcaccggccacatcgcgccgaaggccaccacgaacagcaccatgccggggttcagcccgaagatcgaaatggccagcggcagcagcgccgaggcgggcagggggcggatgaattcgagcgtcggctgcacccaggcgcgcaccgcgggcgacacgccgatggccgcacccagcagcacgccgaacagcgaggccagcaaccagccctgcaccatgcggccgaccgtggcctgagtgaaggcgagcagttcgccgttccccgaaccgcctgagagattgagcccttcgagcaggctcaccaaggtggcttgcggcgtcggcaggaacacgcggctcacccagcccgcattgcttgccgtccaccacagcgcaacgagtgcgcacagcacggcgaacgaaccgagccagttcatgcccacgaggcggcggtttccggcgttcatggctgcacccccatgcgccgcgcaaccacgcgctgcagcagcagcatgcccgcgttgaccgcaaagcccaccacgccgatccagcccagccacgcgagcatcagcgcgggatcgaagctctgctgcgcaatcatcatcgcgtagcccatgccgttggggttggccgcgatctccaccgtgaccgccaccaccagcgccaccgccacgcccagccgcagcgcaacgaacaggcgcggcacgatggccggcagcacgatcttgaaagcccgctctcgcgccgagaggcccagcacgcggctcacctcgagcagccgaggctcgatctgctgcaccgccgactgcaccagcaccaagagcggccagaaggtggcgaaggcgacgatggccagctccatgcgcacgccgaatccgaaggtcagcatcgcgagcggaatcagcgccaccgagggcacgggccgcagcacctcgatcgacatcgagcccaactgcgccgtgcggcgcgagaggccgagcaccagcccgagcgcgatgccgagcaccgcgcccagcagcaggccgagggcggccgtgcccagcgtgaagccggtggcttgccacagcgaaccgtcgagcgccgcaccgacgaaggccttggcggccgcactcggtggggcaagcgcatcgctgcccaacgccgccgcacgccgcgcataccactcgaacgcgccgacgagcagcgcaggaaacacccacggccgcacccaacgaagcaggcggctttcagtcatggccctgctcgatgaaggcgaacagctcgcgccgtagctgcagatactcgggatgctccttggtcgtgagctggtcgcgcggacgcggaatcttcacgtcgatcatccgcgcgagactgggccggcccggccccggattggcctgcagcgcgatcacgcggtcgccgaggtagatggcttcttccaggtcgtgcgtgacgaaaagcaccgtgagcccatcgtcgcgcaccagccgcgcgagttcgtcctgcaggctctggcgcgtgagcgcatcgagcgcgccgaagggttcgtccatcatcatgagctcgggcttctgcgccaggcagcgggcaatctgcgcgcgctgctgcatgccacccgaaagctgcaccggaaacttctgcgcatgtttcgcaaggcccaccttgcccagtacgtcggcaatgcgcggcgcgcgctcggcggcgggcacgccggccgcttcgagtgcgaggctcacgttgccttcgaccgtgcgccagggcaagagcgcgcggccgtagtcctggaacacgaaggccacttcgcgcgagggctccgtcatcttgacgccgttgcgccgcacctcgccggcactcgcggtcacgagcccgctggccgcgcgcagcagcgtggtcttgccgcagccgctcgggccgacgatgcagacgaactcgccgcgcgccacgtcgaacgaggtgggcgacaagatctcgcgcccgccgagccggatcgcaacgccgtcgaagcgaagaaagtcggcggcagcgctcacttggcgatcaacttcgcaacgtcgatgggcgtcttcagcatgtcctggtccttcatcaggccgacccagtagcccagctgcttctcgttcaccatggcgccgggcggcgagatctggatcttcgcgagcacctcgggcggcagcttgatgtacttgccgatggccgcgcgcaccttggcatcgttcttcggctgctgcatgaaggccgcggcctcgaccagcgactcgcggaatgcgcgcgcagcagcggggttcttcgtcacccattcgcgcttggccgcatgcacgatggtctggttgttctccggcaggaaggtggagtagtacgacgccacgtagcccgcgccgctctccgtgatgcggctcatgaacgggtcggccgacaccaccgcatcgaccgagccgccgcgcagcaaatcggcatgctgcggaaacgaggcctcgacgaagttgaccttgcggtagtccacgccgctgtccttgagccaggcgcggaaggtcacgtgcaggaacgcgccgagcccgggcacgccaatcttcttgcccacgcaatcctgcgggttcttgatgcccgagccggcgcgcgccaccaggccgaagcccgtgatggtcttcgacgtgagcccgccgccggccaccagcaccaggtcgagcccgccgtccaccgcctgcaggaacaccgaaggcgtgggcccgccgatctgcagcgagtcggactgcagcgccgcgggaatggtggagttgagcggaatgaatttcagctccacgtcgaggttgcgcttcttgaagtagccctcttcggcggccaggaagaccgaggcgaagtcggacacggccgtgtagccgaacacgatcttcgggttcgcttgcgcgcgcgaaggcagcgccgcggcggccgatgcggcggccagcgccgacagcagggtgcgtcttttcatcatgtcttttgtctcctggaggtggttttctttggcggtgccttgggccgcggcagcgcggcgcgcagcccgccgacgatgaagttcacgagcatcggcgccgccgccggatcactgcgccggttctcgccgtgcgagagccgttcgatgcggctgtcggtcaggtgatgcagcagcgccccgagcgagaactggtagcaccaggcggcctgcccgcgcgtggcatgcggcagtgcgacgtgcagcgcgtcgatgtaggcctcggccagcgggtcgaagtagccgcgcagcacacggtcggcttcctcggtggcgtggtagagctcgcgtgccaccaggagcgcgtagtactcgccctcggcgctcgcacgcagcgccagcaccggcccggtgaaggcctcgatgatgcgcggcagcgtgcgcgcgtcgtcggggtcgttgttcaccgccttgaggcccgcgagccgctcctcgatgctgtgactccagtgctcgaagatggcgtggaagagctcttgcttgggcccgaagtagtagcccaccagcgccagcggcacgcccgcttcctcggcgatctggcggatggtgaccgcgtggtagccgtgctgcgcaaagagcttttccgccgccagcaggatcgcgtggcgccggtcgggccgggccgcttcggcgctggtggccgcggcacggtgggcgcttcgtctggcgggcggggtacgggtgttcatcggagcgtattgaacatctgtacaaaactattgaacacacgtacaaaccctgaggtcaaccccgattgagcggcgcgtggcacggcattacgctcgacgcatgtccgcccccaacatcccccagatccgcctctaccaggactggctgcgcgaccagcgcggcctgtcgttcgacacctatgacgcactgtggcgttggtccgtgaccgacctcgacgcgttctggcagagcatctgggactacgtcggcatgcgctcgcccacgccgcacactgcggtgctggccgacgcgcgcatgcccggcgccaagtggttccccggtgcgcaggtcaactacgcacgcgaggtgctgcgccacgccgatgcggcccatgcggccggcatgcccgccatcgtgagcgacaacgaactcggcgaagtgcgcgagctgtcctggcccgagctgcgccgccaggtggcctcggtcgcgctcacgctgcgctcgctgggcgtgcagcgcggagaccgcgtggcggtctacatgcccaacgtgcccgaaaccatggtggcgtttctcgcgtgcacgagcatcggcgcggtgtggagcgtgtgcgcgcccgacatgggcacggccgcggtggtcgaccgcttccgacagatcgaacccaagctgctgatcgccgccgatggcgtgcactacggcaccaagcccatcgaccgcagcgccgtggtgcaggagctgcgcggcgcgttgcccagcgtgcagaagctgctgctgctccgcacgccgcatgccgcgcaacagctcgccgccgatgccgactggcacgacgccattgcacgcaacgacgccgaggtggcggccttcgaacccgagtggctgcccttcgaccatccgatctggatcgtctattcgagcggcaccaccggcctgcccaagcccatcgtgcacgggcagggcggcatcatcatgacgatgtatgcctgcggcctgcacaacgacgtcggcgcgagctacggcgccaacaacttcggcgaacgctttcactggtacagctcgaccggctgggtcatgtggaactgtcagctctcgggcctggcctttggcgccaccatcgtcatctacgacggccatccggccggcagcaaggagaagcccgactgggccgtgctgtggcgcttcgtcgcgaagcaccgcatcaccttcttcggcgccggcgcggcctacttcaccaactgcatgaaggccggcgtggtggcgtccgaatgcggcgacctgtcgcgcgtgcgcgcgctcggcagcaccggctcgccgctgtccgaagacgtgcagcgctggggcacggcgcaattgcaggccgccggcgccagcgacgtgtggtggtgcaatatttcggggggcacggatttttgcggcgccttcgtcggcggcaaccgcgagctgcccgaggtacccggccagatgcagtgccggcagatcggccacgctgtcgaggcatggaacgagaacggccagcccgtcatcggcgaagtgggtgagctggtctgcacgcggcccattccgtcgatgccgctgtacttctggggcgacgaaggcaacgcgcgctacctgtcgagctacttcgacacctaccccggcgtctggcgccacggcgactggatcaagatcggcgaagacggcggctgcatcatctacggccgcagcgacgccaccatcaatcgccagggcctgcgcatgggcaccagcgagatctacagcgccgtggaggctctgcccgaagtgctcgactcgatggtggtcgacctcgaatacctcggccgcgaaagctacatgccgctcttcgtggtgctgcgccccggcgtggcgctcgacgacgccatgcgcgcgaagatcaacggcgccatcaagacatcgctctcgccacgcttcctgcccaacgacatcttccaggtggacgagattccgcgcacgctctcgggcaagaagcaggagctgccgatcaagaagctgctgctgggccagccgctcgagaaggtggtcaatcgcgaggccatggccaaccccgcttcgctcgcctggtacgtggaattcgcggcgcggcgcgcggcgtcgtgaggccctagcgcgcgtcgtggaagatgatgcccagcgtatggcgacgccccgagcgcacgcggctcacgccatggcgcatcgtcacgcggtaggtgccgcgcgtgcctgccaccggccgctggttgaccgcgaagatcaccgcctcgccctgcgcgagcgccaccacttcggcgcgcgactgcatgcgcggccgctgctcggtgagcacgaattcgccgccggtgaaatcttcgcccggccggctcagcagcaccgtgagctgcaacggaaactgcaggtcgccatacaggtcctgatgcaggcagttgtagtcgccctcgccgtagcgcagcagcagcggcgtggggcgcagttgccccgccgcatggcagcgcgcgaggtaggcggcatggtccgccggataggcggcgggctggcccatcgcggcggcccaagcgttggcaagcggcgccaggcgctcgtacagcgcgctgcgccatgaggccacgaccggcggcagcgggttggcaaagtactggtactcgccttgcccgaagccgtgccgctgcatcaccacgcggctgcggaaacggtccggttcgtcatacagcgccgccagcgcgttgcattcctccgggctgaagatcacgcccgtggttgcagagccgcgcgtcgcgaggtcggtttcgatgcggggccaatcgagagcggcaacgaattttttggcagagatcggcatgccgccagtgtgcgactggcgcggctgcggcgctcgctgtttccggacatgggtgcagccctgcaggcccacaggcctacagccacttgccgctgcccgtcggcatctggatggtcgttgccggatcgccgctgttcaccagcgaatcgatcccgatgctcaggagcgaaatgaagatgctcgcgaagaacgccgtccagaagcccgagagcttgaacccgcgcaccatcgcggccaccagcatgatcatcagcgcgttgatcaccagcaggaacaggccgagggtcagaagcgtcagcggcagcgtgagcacgatcaggagcggcttgacgatggcattggcaaggcccagcagcagggccgagatcacgagcgccgaagtgctctcgaacttgatgccgcgaaagatcaggctggccacccacagcgacagcgcggtgatggcccagtgcacgagaaagggagcgaggttgttcagcatggtgtgaggggcggaagaagacggtccgcggggcgatgcggaccatcatatcggcagcttcttacggcgagccgcgccgtgcctcgcccagcagccagtcgctgaagaacttcagcagtggacgctggtcggcgcgctcgggtgtcacgaggtagtaattgcgctcgcccgacagcggccgcgcgcaggccaccaccagttcgccgcgcgcgagttcgtcggccaccagcatcgtgggcatcagcgccacgccgagcccgtgcgatgcggccgcggccaatatggaaaacagctcgtagcgcggcccgccgcgcgcattgggcgcatcgatctgctgcgcatcgaaccactggcgccagccttcgggccgcgtgctctgttgcagcagcggcatctgcgcgatgaccgccggcgccacggccttgccgcgcggcaacagcgaagggctgcacaccggcaccacgtcctcgtgcatcagcagcagcgcacgcgtgccggcccagttctcgacctgcgcgggtgtgccggcgtacagcgcggcgtcgaactccgcatcggcaaagagaaaggggcgcgtgcgcgtctcgatgtgcaccaccacgtcgggctgcaatgccgcgaagcccttcagccgcggcatcagccagcgggtggcaaaggtgggcacggccgccagcgagagcgagccgccttcgccctggtgcgccatggcgtcgagcgtgtcgcgctccatcgcttcgagccgcttggtgatctgccgcgcgtaggccgcgccgctggccgtgagcgccacgccgtggcgggtgcggcggaacagcgccacgcccaggaaggcttcgagcgtgccgatctggcgcgacaccgcgctttgcgtgagcgcgagttcctgcgcggcgcgggtgtagctctcgtggcgcgcggccgcgtcgaagcacacgagggtttgcaggggtgggatcttgcggcgcatgtatgccggtagtgtatgactggagaagtgccgctaccaatggaaacgtctttccatgcaggtgcgagatgtgcgctaagcgcatatctgggtgaggattcatcgtttgcgcccggccctccgcatggctaggatcgaccccattccccctctctttcgtttttcccccaataccggagacagccacatggccgccaaagcgcaattccactgggacgacccccttcttctcgaccagcaactgaccgatgaagaacgcatgatccgcgacgcggccaatgcctactgccaggagcgcctcgcgccccgcgtcatcgaaggcttccgcaccggggagaccgaccccgccatctttcgcgaaatgggcgcgctcggcctgctgggcccgaccattcccgagcagtacggcggccccggcctcaactacgtggcctacggcctgatcgcccgcgaagtcgaacgcgtggattcgggctaccgctcgatggccagcgtgcagagttcgctcgtgatggtgcccatcttcgaattcggcaccgaggcgcaaaagcagaagtacctgcccaagctcgccaccggcgaatggatcggctgcttcggcctgaccgagcccgaccacggctccgaccccggcagcatggtcacgcgtgccaagaaggtgccgggcggctattcgctcagcggcgccaagatgtggatcagcaactcgcccatcgccgacgtgttcgtggtgtgggccaaggaagtcagcgaaagcggcaccgtcggcccgatccgcggcttcgtgctcgagaagggcatgaagggcctttccgcccccgccattcacggcaaggtcggcctgcgcgccagcatcaccggcgaaatcgtgatggacggcgtgttctgccccgaagaaaacgcgttccctgaagtgcaaggcctgaagggtcccttcacctgcctcaacagcgcccgctacggcatctcgtggggcgcgatcggtgccgccgaagactgctggcaccgcgcccgccagtacacgctggaccgcaagcagttcggccgcccgctcgccgccaaccagctcatccagaagaagctggccgacatgcagaccgaaatcacgctgggcctgcagggcagcctgcgcctgggccgcatgaaggacgagggcacggcctcggtcgagatcacctcgatcatgaagcgcaacaactgcggcaaggccctggacatcgcccgcctggcgcgcgacatgatgggcggcaacggcatcagcgacgagttcggcgtggcgcgccacctcgtgaacctcgaagtggtgaacacctacgaaggcacgcacgacatccatgcgctgatcctgggtcgtgccatcacgggcatcgccgctttcgccaactgagccgagagcgcatgacagccaagcccgcagcactcgacggcatcaaggtcctcgatctgtcccgcgtgctcgcgggcccgtggtgcacgcagatcctcgcggacctgggcgccgacgtcatcaagatcgagcgccccggcgtgggcgacgacacgcgcacctggggcccgccgttcatcaaggacgcgaacggcaacgacaccgaccaggcgagctacttcaccgcgtgcaaccgcaacaagcgctcggtcacggtcgacatggccacggccgatgggcaagccttgctgaagcagatggcggcacaggccgacatcgtggtggagaacttcaagaccggcggcctcaagcaatacggcctcgaccacgaggccctgcgcgcggccaacccgcggctcatctactgcagcgtgaccggtttcggccatgacggcccgtacgcagagcgcgccggctacgacctgatgatccaggccatgaccggcatgatgagcatcaccggccgtccggacgacgtgcccggcggcggcccgctgcgcgtgggcgtggcgctcaccgacctgttcaccggcgtctatgcgagcaccgccatcctcgcggcgctgcaggtgcgtgaccgcacgggcgaaggccagcacatcgacatggcgctgctcgacgtgggcatggccatcctcgccaaccaggccagtgcgttcctcaacaccggcaaggcgcccgagcgccagggcaacacgcacccgagcctggcgccttatcaagactttccgacgctggacggctcgatgctgctggccatcggcaacaacggccagttcgcgcgcttctgcgaagcggctggccacgcggagtgggcggccgatgcgcgctttgccaccaacacgctgcgcgtgaagcaccgcggcgtgctcatcccgatgatggaagagctcacgcgcacgcgcaccaccgccgactgggtcacgctgctcgaagacaaggccgtgccctgcgggccgatcaacgacatcgcgcaggccttcgacgacgcacaggtcaagtcgcgcggcctggccatcacgctgccgcgccatgcgggcgacggcatcgaaagcatcaccggcgtggcgagcccgctgcgcctcacggccacgccgcccgtgctgcgccacgcgccgcccgcgctcgggcagcacacgcgcgaggtgctggccgagttcggcatcgacgccgcgcgcttcgatgcgctgcgctcggcaggcgtggtctgaagaagaggaaaaatggcagccatgaccagcccgatgcaccccccgttctcggtgctgcgcatcgaccacatcgtgctgcgcgtgaaggacgtggagcgcgccatcgccttctaccgcgacgtgctgggctgcgaaattgaaaagcgccgcgacgacctggggctcgttcacttgcgcgccggctcgaacctcatcgaccttgtcacgcacgatgggccgctcggccggcagggcggcgccctggccggcaaggaagggcgcaacgtcgatcacttctgcctgcgcatcgagcctttcgacgaagcagcgattcgcaccttgatggcacagcacggcgtgccggtgaatggcgacgtgcagaacaacttcggcgccgagggcaacggcccctcgatctacatcgccgacccggacggcaacggcgtggagctgaaagggccggcaggcagctactagcccgtctagccggcgcggcccaggatcgccacgccgaacaccgccacgccgagcgcgaggttcagggtcaccagcttgcggatcatgtcgagccggccggcggccacgggccacgcgctctcgtccaccgcgcgccgcagggccttgaacaccgaggcgcggatgtacacataaattccgaccatcacgatggcgatgctcatcatggcctcgacgcgccagtgcaccgtgcgaaaaccgcccgcgagcaggatcatcgccacgcccgtcacgaacagcagcgtgaccgccgcatccacgccgacgaagaagcgccgcagcgccgccgccatggtgcgcaggcgcagtggcggctctagcgtggcgacggcggcgggacgcacggcgaagtgcagggtggccatgccgccgacccagaaggcggcggcgagaagatggatgaaaagcaaaatggcgtgaggcatggggaccgatcagaacaccgaacggtgcgagcgcgcaatgtccgcggcgttgcgttaaaaacccatccttcgacgcaagaaagaaagacgaggctttcatgacccgcaccaccgcgcagaagcgcgccgatttccgcgccctccacgagcagggctgcttcgtcatccccaacccctgggacactggcagcgcgcgctacctgcaagggctgggcttcaaggcgctggcgaccaccagctcgggccatgcgtggtcgcagggcctggccgacggcgcccaatcgcgcgacgtcgtgctggcgcacctgcgcgacatcgtcgccgccaccgacctgcccgtgaacgcggacttcgaaaatggcttcggggccgatccgcaagccgtggcagagagcgtgcggctggcgctcgacaccggcgtggcggggctgtcgatcgaggactcgaccggcaatccggcgaatccgctcttcgagatcggcgttgcggtcgaacgcttgcgcgcggcacgcggcgccatcgatgcggccggcggggacacgctgctggtgggccgcgcagaaaatttcttcgtcggccggcccgacctcgacgacgccatcgcacgcctcaaggcctacgcggaggccggtgccgactgcctctacgcgcccggcatccgcacgcgcgagcagattgcggccgtggtcgccgcggtggcgcccaagcccgtcaacctgctgatcggctgggccagcgagctcaccatgcaggacattgcagagcttggcgtgcggcgggtcagcgtggggggcgcgctcgcacgcgcggcctggggcggcttcgaccgcgccgcgcgcgcactcgccgagcaggggcgcttcgatggcttcgcgggcgctgcggtgggtgcggacctcgacgggttcttcaggccgttctccgcaccctctgcgtcctccacgtagcgcattcgctggcgtcatggacgcgctcctcgcggaaatccgcaactgccgagcctgcgccgcgcacctgccgctcggcccgcggccggtcgtgcaggccagcgccagcgcgcgtctgctgatcgtcggccaggcgcccagcatgacggtgcacgccaccggcctgccgtgggacgacaagagcggcgagcaattgcgccgctggctcggcatcgatcgcgaggtgttctacgacgccacgcagatcgcgatcatgccgatgggctattgctacccgggccgcggcagcagcggcgacctgccgccgcgcagggaatgcgccgagctgtggcacgcgcgcctgctcgcgcagctgaagaacatcgagctgacgctcttgatcggccagtacgcgcagcgccatttcctgggggcggcgcgcaaggccggcgtgaccgaaaccgtcgaggcctttgcggagtacgcgccgcgcttcattccgctgccgcatccgtcgccgcgcaacaccggctggttcaagcaccacccgtggttcgaaagcgatgtgctgccggtgctgcgcgagcacgtgcggcaggcgctcgctcagccctatggcgccacggcgaccgaggtgcccgctgcatcgaaaggccgcgcggcatagaccacgcgcccgcccaccaccgtcatcagcgacaccgtcctgccgatgcgctccaccggcaccgcgaagaagtcctggtcgaggatcgcgaagtccgcgagcttgccgacctccagcgtgccgcgcttggcctcgtcgaagctgaaccatgcactgcccgccgtgtagagccgcagcgcctgttcgcgcgtcggtgtttcgtcggcgccgcgcatcggcttgtcgctcacggtcttgccgtcgagcatccattgcagcgcgacaaaggggttgtacgacgccacgcggtgcgcatctgtgccggcgcccacgttcacgcccgcgcgcaatgcgctgccgatcggtggcatgcggcgcgccgcctcgccgcgcaccgtgagcgcgcggtcgccctggaagtacatcgcgtcctgcatcgtccagccgatgcccagcgccttcatgcgcgccagcgtttcgggcgaggcgtcgtcgagatgtgcgatcgaccagcgcaggtccttgatcggcacctcggcgttgagcttttcgtactgcccgagcagatggtcgaccgatccgttctcctgccagtggatggtgacggccagcttgcgcagcgccgcccacttgatcagttcgtaaaacttttccttcgctgccgcatcgggaaaattgttgttgtacatcgcaagcgtcacgcgttcgccaagcccgttgaacttcagcatgtcgtcgccaaagcccatcggcagcatctgcgtcagctcgcgaaactcctgcagctcggcgccgggcttctgcgcgaacacgctgtaggccacccgcagcgtcagcgccttttcgcgccacagctcgaacagcgccgcgtattgcgacggcgcgatgctgaagccgcccgggtccaccaggccggtgatgccgaggcggttcagctcgctgaagaaggcgcgcgtgccggccacgttgtcggcgtaggtcggcttgggcagcttgtcgaacagggccgagatgccgacgatgtcgcccgtcatccagcccggcgcgccatcggccgcgggcttcatgccggccggcagcgcgcccgccgcaaccccgagcgcttcgagcgccttcggcgtcatcaccaccgcctcgtagaacagctgtacgtacaccggatgctccggcgcggcttcctgcagctccgccatggtgggacggcggcgctcggcaaactgctgctcgttccagccgcccgccacgatgagccagccgccgggccgcgcacgcgaggccgcggtgcggatgcgcgccatggcttcggcgatggtgccggcgccgatccagttgacctcggtcgagtagctcagcgccgcgcgcactgcgtgcatgtgcgagtcgatgagccccggaatcacggtgcgcccgccggcatccaccgtgcgcgtgcccgggcccgagaacgcgcgcatctcgccggcaccgccgaccgcaacgacgcggccttcgcgcacggcgagtgcctgcgcggtggtcgaggcggcgtcgagcgtcgcgatcttcgcgttggtgacgatgaagtcggccggctgtgcctgcgtgccgatcggcagcagcagtgcggtggccgcagccatcgccaggaaggtgcgcagcatgctcaatccaccttgatgctggctgccttgaccacctgctgcgccttggccgtttcgtcggcgatgaacttgttgaactgcgccgaaggcatggtgaagggctcggcgccgagcttgtcgaggcgctccttcagttcgggcgaagccatgatcttcgcgacctcggcctgcaggcggtccaccaccggctgcggcgtcttcgcgggtgcgaagagcccgacccagaacaaatactcggagcccggcacgccggcttccaccgtggtgggcgcgtcgggcagcgccggcgagcgcttggccgtacccaccgccagcgcctgcagcttgccgctcttgatgagcggaagggccgacaccatcggcgcgaagaaccagtcgacgcgcccggccatcacctcggtcatggcctcgggcgtgccgcggaagggcacgtgctgcgcgtcgaccccggccgcgaggcggaacacttcggcgttcatgtgcgtggccgagccgttgcccgcggagccatagttgaagctacccggcttggccttcgccttggcgaccaggtcttgcacgttcgtgaaatgcgaaggcgcggtgaccagcacgttgggcaggctcgccatcggcgtgatgcccgtgaagtccttgagggtgtcgtacgacaaacccttgtagatccacggattcacgaggtgccccgccgaatgcaccagcagcgtggtgccgtcggccggcgccttggccgtgatggccgcgccgagcgtgccgcccgcgccgggcttgttgtcgaccaccacgctggtgcccagcaccggcccgagcttctcggccaccaagcgcgcgacgatgtcggtgccgctgcccgccgtgaagggcaccaccagcttgatcggctgcgtgccgggccatgcgttctgcgcctgtgcgctgctgaatgcgcaagccgcgagcgcggcggccatcgcgagcgcctgccggcggctcgggttgaatgtcttcttcatgcgtcttgtctccgttgatttgtttgggtgagcgatgaatgaccgggaaagaggagggcgctaggcggcgggcggtgcgttcggcatcaccagcgccaccagcaccggccggttgcttcggttctcgagctggcgcttttcgccgggcgcgaagcggcagctgtcgtaggggtcgagcacttcttcctcatgcgcgccgtcgagctcgccgaccacgtggagctggccttcgagcacgaggtacaacttctccatcggcgagccgtccaggccggtgtggccgccgggcaggatctggctcatgcccatccacatctgcgtcgagggcccggcctccttgccctgcaggcgcaggcagcgcatgtcgaaatggttgggcgcttcgtagtgcggcgcttcgctgaaacgggtcacgtgcatggcggtggttcctatctgtgttcagggccgcagcacgacccggtcggtgctgcccgaaagcacgagccggtaggcgtccatggcttcgtcgagcgtgaagtgccgcgcgaccggaaagggtttcagcgtgccgcgctcgaagccttcgcgcatcgcgtcgagctgcgcggtggaggccacgcagtccatggcgagcgagtcgatgcccacgaaggtgtgcatgccgcggtagaacgcgaagatgtcgaagggcacggcacgctcgtgcgtggcgatgaagatctgcgtcgcgcccttggccatcgccttgttggcggcctcgaagtaggcgctgcccacggtgttgtagacgatgtgcgcgccgcgcccgtcggtgagttcgcgcacttgcgcacccacgtcggcatggtggcgtgcatcgatcacatcgaccggcccacttgcgaagccttcgaagggtccggcgcggcgctgcaccgcgatgacgcgcgcaccggcctgcgaggccagctgcaccgccgcctggccgaccttgccgttggcgccgagcaccagaacggtctgcccggcctgcggcatgccgctgcgccgaaagccttcatacgcggtgacgaagggcacgcccaccgcgccggcttcgtccatcgagatgccctggggcttggcatgcagcgccgcttcgggcagcgccaggtagcgtgcatgcgaaccgtcacgcgtgatgccgatgtcgccgcccgagccgtagacctcgcggccgatccattcggtgggaccgctcaccacggtgcccgcgaagtcgcgtcccggggtgcgcggccacacggcctgcggcatgaggcccagcgcggctttcacgtcgctcgggttcacagctgcggcggcgactcgcaccacggcatggccggggggcgctgttggttccggctgcggcgcggcttcgagttgcagcgcgtcgaggttcgcggccttttcgttcacgcgcagtgcgcgggaagtgtgggttgtgtgcatggcggcgatgctcatttcagtgttccaccgcggtgttgtgttgcgggttgcttgtgttcgggtgtcgttcgttcagggcgtgtgcacaggccaccgggtactcccctccgcgaatgtcccccgccttcggctcctcctttgtttcgctgcggggagcacccggcgccctgtgcacaccaagcgctgccgttgttccgctcgatcaacgacggctctgaacaacgatcccgtcgatggggtgccttgcgcagcgaaataaaggaggaggccgcaggccgggggacattcgcggagaaaggtaccccgtcggcgggagcgcgccctgaatcgcccacagccgtactaacagaagaacaagacgtcatctcctagctccccgcaccaggcaagcccagcatcgcgcgcgcctcgcgcgggttggcaatctcgccgcccaggctcagcaggatgtcgcgcgccttcgccacgagttgtgcgttgctttcggcgagcacgcctttctcgaggtagatgttgtcttccatgcccacgcgcacatggccgcccatgagccaggcctgcgcgacgatcggaaactccatgcggccgatgccgaacgcgctccagaaggcgccgcgcggcagcatgttgcgggcatagagcagcgtctcgggcgtgggcgcgaagccgtacttcacgccgagaacgaaggtccacatcgcggggccgtcgagcgtgccgtcgccgatcaggtcgagcgcgaggttgatgtcgcccgaatcgaagatctccagctcgggcttcacgcccgcctcgcgaatcacctttgccatgcggcgcacgttcttcggcgtgttcatcaccacgtcggggcccgagttcatggtgttgagatcgagcgagcacacgtctggcctgatgagcgcgatgtgttccacgcgcttctccggcggcagcagcgtggtgccgggcgcggcgatcttcggatcgtcctcgctcggtatgtagcgcccgccgggtccggtcgtgaggttgatgatcagctcgcggttttcgcggcggatgcggtcgaccacctcgcggtagagctccacttccatcgacggcttgccggtttcgggatggcgcacgtggatgtgcacctgcgccgcgccggcctccgcggcggccaggcattcgtcggcgatctgcaccggcgtgatcggcaggtgcggcgtctgctcgggcttcactaggttgccggtgacggcgcaggtgatgagggtcttgagggccttggtagtgctgctcacaggtggcgccctccgtcgaccacgatgcgcgtgccggtgacgaagcgcatcgtcgtcgcgagcgcctcgaccgcggcggccacgtcgtcgggcttgccgatgcgcccgagcggcgtggtgctcgccatcttgtcggcaaacgccgcgccgcggccgggcacgaagcccgactcgaccgcgcccggcgacaccgacaccacgcgcacggctggcgccagcgccttggccagcgcatcgcccaccacgtcgaggcccgccttggccgccacgtacgcaaggttgctgcccacgcccgtgaagcccgcgatcgaagagatgttggcgacgaggccgtcgccgctttgcttcagcatcggcgcgaaggcgcggatggtcgcgaacacgccgcggaagttggcgcgcagcagctcgtcgatgagctcgtcggtcagcgcgtcgaggtctgcggcgggaatgggctgcgtgtgccccgcgctgttgaccaggatgtcgcagcggccgtgcgtgactttcacctcggcggcggcggcctgcaggctcggcgtatcgacgatgtcggcgcggatcgcgctgtggcgctgcccgtgggcggatggcagggccgcggcgcgcgcggcggcatcgtcgcccttgcggtgcagcagcacgcaggtggcgccgagcgcggcgagccgcatggccgtggcatagccgatggcgccgaggccaccggtgatgacggccaccttgccgtcgagtcgggaaacaggatcgaagctcatgggatgaaagaagagtgggttcagggaatggggggacgagggaacttcatctcgccgggctcgagctggaagtcgtactgcagcgtggccgcctggccatcgggcgtcagcgcgaagcggccgatcagccgccgcgtcacgccgaaggtcgggtcgctctccaggttctcgtcgtcgtcggcaaacacctgggtgaccagtaccttgtgccccggcttgctcaccatgaagtgcaggtgcgccggccggttggggtggcgttgctgcgcgcgcagcaacacgccgcatggcccgtcggtcggaaccgggtagccagccggccgcacgctgcggaaatgaaagcgcccttgcgcatcggtcgtgaagcgaccgcgcaggttcatgtcttcctgcgccgggtcctggttttcatagagaccgatgggcgaggcctgccacacgtcgaccgtggcgcccgcgaccggttcgccccgcgcgttgcgcaccgtgcccgacaccgagagcggaacgcccggcgtgcccgagcgcgcgatgttgtcgccctgcgcgcaggccggcgagttcgcgcgccagaaaggcccgagcagcgcggccggcgattcgccgtgcgggtcctggttgttctgcagcgccaccaccgtggacacgccgaggatgtcggccgccagcaccacctcgttctttttttcgcccgtggcctggccgatggcgacgatgaattcgagcgcctgctcgaactcttcctccgtcagcttcacctcctggacgaaggcatgcaggtggcgcgtgagcgcatccatcacggtgcgcagccgtgggtcgggtgtgcgtgccatggcttcgagcgcgaagcccagcaccgaatcgggcgaggtggcaatgttcatggcagtctctgcaatcgtttgcacgatcttagtccaaaatcctggaaagtaaaatgaccctgttctgcaggttgggaatggtgagtaaccatttcagcgtgttcttccgccgacaatcgtttgcaccaatcagccccatgagcaccagtccgtcttcttcgcccgtcacgatccgcgacgttgcccgcgcggccggcgtgcatgtgtcgaccgtgtcgcgcgcgctcagcccggacaagcgctcattgatcagcgacgaggtgctgcgcgtggtcgaagaggcggcgcagcgcctgggctacaggcccaaccgcgcagcctcggccttgcgcaccggccgcacccacaccatcggcgtgctggtgcccgacatcacgaacgcggtgttcccgcccatcctgcagggcatcgaggccagcgcggcggcgcgcggctacttcgtgttcgtcaccaacgtggtcgaccctgcgctcgcgcggcctgtgctcgagcgcatgctggcccagcgcgtcgatggcgtgatcctggccacagccacgcgcgacgatccgcttgtcgatttcgtcaccaagaccggcatgaccgcggtgctggtcaaccgcgccgatgaaaccggccgcctgcccgccgtggtgagcgacgaccggctcgcgatgaagctcgcggtcgaccaccttgtgagcctgggccacaagcgcatcgcgcatctcgccggcccgcagaacatccccaccggcgtgggccgccgcttgggcgtggagcaggcgctgcgcgaccatcgcatgaagcccttccgcgtggtcgagtgcgcgagctacagccgcgaggccggcgcggtggcgatgcagcagatgctcgaagccggggccgcgccgcaagcggtggtgtgctgcaacgacctggtggcgctcggcgcctacgacgcgctgcgccaggccggcctgcgcgtgcccaaggacatttccatcaccggccacaacgacatgccgctggtcgacatggtcgatccgccgctcaccaccatccgcctgccgcatcgcgaactgggttggcgcgcggccgagatgctgttcgaggagatcgacgggcaggcgatgtctgcgtcgacggtggtgctgcggcccgaactggtggtgcgcaagtcgacgggtgcgccggcgacgcggtgatcagccgggccggggcacggctttcttgcgcgcggccggccgccgtggcggccgggtctccagcaccagctcggccggcaaggtgtcgttccaagactcggtgaaataggcacggtcgctcggcaccagctgcggcaatgcctcgcgcagcgactccagcgactgctcggccgccttcaggtcgcccgcaagcgccgcataccaggcgtgctcgaacagaaggctgcaatgctgcaggccggggtagcgccggcggccggcctggtggtcggccagccgggcctgcgccacctcgacccagcgtacgggccaatgcgcggcatcgaaggcatcggcgagcgggccggcgagtttcgagattgccgccgggtccagcggtttctgcgcgcggaattgcgcgagcgtgggttgcttctcgggctggcaatggccgcgcgcgatgcgcatcaggtagatcgcattccaggccgagcggccctggccgtcggtgtggccgcagagccattcgctgaaggcgatccactgtacggcgcggcgcatggtgtcggcgtgtccgtcgtgcgcgagcgctggcaggtccgagaggcccacgcggtcgaacagccacgcggccatgcccatgttggcggccacgtgctgcgccgcgtcgaaggagtgcgattcgaaggccgcggccaatgcctcgccgaagcgttgcagcgattcttcggcgagcgaggcggccgcgggcctgtcgtcggcggcgagcgccaatgcgcgcgagcggcacaccagggcccagaggttgcaccattcgaagcgcacgtcggggtggtgccgcagcacgagtccgcgcaccgcatcctcggccatgccggtaaggagcgactgcgcgagcggcaggtcgcgcgcggtgtaggcgcaccaggccgagacgacgcattccatcgcgcccaggtagtcgttgcccgccacgtggtgggcgaggcgttgctttttcagggcctgcagacggcggcgtgcctgctcgttgtcgccgaggcggcgccacagcatggcctcgttgagcgtgaccagtgcgcgttgaaagtcggtcgcggccaatgtgccggcgaggcggatcgactccaatgcgctggccggcgaaccggtcgcgctgccaccacctgccaccggtgccatgagcctgccttgccgcgccgcctgctgcgaggcgaccagctgcttccagaaggcggcgtcctgcaggtgcaccgcgtcgggcggcctcggcgagccgggagcagccgcactcgcccggcgcgagcgcagccccaggaaggaagcgacctcggccgccgtggccgcgcggccgcccaccagcatgcgcacacgcttcgcctcggcagccggcagccagaagggtccctggctgcgccgctcggcgttgagaaagcgcgcttcgcgctgcgtgtcctcgccccagccgacctcgatgtcccatgccttgaagtcgcggaacgcgcggctcaccaccatgcgcagcgtgcttgcatcggacacttcgccgcgcaggtcggccagccgcacgaggccgccttcggcatcgtgcgcgtgcttcatgcgtgcgagcagccagagcgactggaacgccgcgcgccggccgttgaccgattgcggcgaggtgagttcgatgaaaagcggggagggtgtagcaggcttgggcacgccccggattgaacctcaaatctcggagcgagggagagacggcgggcagggccgttttcttcagaacctgtcgcggtccagcaggccccgcacctggctgcggccgatgcccaggtcgcgcagctcgtggtcgctcatgccggccaggtgctgtgtgtccgcgcggctgcggcggcgctccgcgacgcggtggcgccagctgcgcagggcatgcatcaggcgttgatgaaagggcgagtgcgtcggcgctgtcacggtgggctccttgtgggggagcgctcatcttgcggcgatgcgtgctattgtggaagttgagattcctgacaccttcaatcagcattcctgatgcgacaactcaacctcgaccagctgcgcacccttatcgccattgccgacctgggcaccttctcggcggcggccaaggcgctgcatcttgcgcagccgaccgtgagcctgcacatcagcgaactcgaatcgcggctgggcgcgccgctggtggtacgcggcaaccgccgcgtgacgtccacggcggccggtgcggcgctggtcgagcgcgggcgcaagctgctgcgcgacaccgacgatgccgtcgaggcggtcaagcgccaggccgaaggccgcaccggccgcgtgcgcctgggcacttccactggcgtggtggtcgacctgctgccgcaagtgctcgaagcgctgggcgtccggcattcgggcatcgacgtggaggtgagcatcctgggctcgtacgaggcgatggcgcggctggccgccggcacgctcgacatcggcctggtggccgtcccgcagccgccgcagcgcgacatcgtcgtcacgccgtggcgcgaccaggccatgatggccttcgtgccccagcgctggaaggcgccccggcgtgtcacgccggcgtggctcgcggcgcagccgctgatcttcaacgacgccaccactcacatgtaccggctctcgatggagtggttcgcggcggccggcttcgcaccgcgtgcgcgcatcgagctcaactacgacgcggccatccgcagcctggtggcggccggttacggcgcggcgctgctgccgctgcagcagaccaccgatgcggcactgaacgagcgcatgcagatcctgccgatcacgcccaggctcacgcgacgcctgggcatcgcccaccgccagagggccatgctggatggcgccacgcaaagcgtgctgcaggtgctgacgacgtttcgccagctctgatttcagccctgggcgcttccgttcggaaggccctcgatcgggcattcggccgtgccgatggtgctgcgcgtgatcgactccaccttctcgcgcgtgccctcggggtcgttgatccactgggtatagaagtcgtaggggcagtccgccaggccgcggtcgccgtcgcccgagttgatgacgccggtgtagccgcggtgcagcagcttgaacaggtggttctgcgattggccgttcttgcgcgcatcgcggatcaggctgagggacatctcggcgtagttgatgcccatttcctcttcgccgcattcgcccagcgtgcggccgtcgaagccgatgagggcggagtgtccgaagtacgaatacacgccgtcgaagcccgccgcgttggccaccgccacgtaggtgttgttcatgaaggccatcgccttcgacaccaggatctgctgctccttggccgggtacatgtagccctggcagcggatgatgagctcggcgccgcgcatcgcgcagtcgcgccagatctcggggtagttgccgtcgtcgcagatgatgaggctgatcttcatgcccttggggccgtcgctcacgtaggtgcggtcgcccgggtaccagccttcgatcggcgtccacggcatgatcttgcggtacttctggacgatctcgccctggttgttcatgaggatcagcgtgttgtagggcgccttgtccggatgcgactcgtggcactcgccagtcagcgagaacacgccccacacgttggcgcggcggcaggcgtcggcaaagatcgcggtctcctcgccgggcacggtggcggcggtgtcgtacatctccttcgcgtcgtacatgatgccgtgcgtggagtactcgggaaagatcaccaggtccatgcccggcaggcccttcttcatgccgaccagcatctcgccgatcttgcgggcgttgtccagcacctcggccttggtgtgcaggcggggcatcttgtagttgacgactgcgacgccgacgccatcgctgctgctcgaaatatcaccatgtctcatgacgctgctcctggagggtggttgagagaaaagagagaaacaaaaaagcccgagccggtgttcaaccggttcgggcttgtctctggtgcggcagtggattcgtgtcgtcggagccgattgttctcaactcagctcaggctgcccatacgtcatttcgctgattgcggagcgcgttcagcggggccgcgcgtaatcggattcgatccaggcggttgcgctggcggcggagagccggaaggcgggcgaaacgttgacgctcgcgagctcggtgtcgtcggcatcgtcatgcgcggcaagcgtggccgaggggctgtcctcgtcgggcacgatggcaagcgacacgcgcacgcgctggtcgcccttggcggtgacggtcacgctcttgttgagcgtggcatgcagctgctgctcatggcggcgaatcacttcggcggcggtcttcaccagcgtggaaaacgcgggaccgtcgagcggcttcgggttcttcttgtcgcggcccatggtccaggggccgaccagcgcgggctcggggtcgccgtggcgggtcatctcgacggcccagccgtcgtcttcctcgttcttgatgacgcgtgcggtccattggccgtcgcgccagaggcggggttcctgcagggggagggtgtcggagtcggtggagtctgtggcttcggtcattcgggtgctcgggttcgtgctcggcccattttcgcctgcgcctccgggcagcccgctcagaagaccgacagcccggttcgcgcgacgaagagttcgagcgccttcattccgagcagcgagttgcccgtggcgtcgagcgcgggcgaccagacgcacagcgtgagccggtcgggcaccacggcgacgatgccgccgcccacgccgctcttgcagggcaggccgatcgagaacgccacgtcgcctgcggcatcgtaggttccgcaggtgagcatcagcgcgttgatgcggcgcgtctgccgctcgccggtcacctcggccgcgccgtcgattgggtgcgcgccgtcgcggcacaggaaggccgccgcgcgcgagagctggcggcagttcatccgcagcgcgcactggtgaaagtaggtgtcgagcaccgcggccacgtcgttgtcgatcttgccgaagctcttcatgaagttggcgagcgcgatgttgcggaagccggtcgcggcttcggagcgtgccacctcgtcgtcgaacgaaatcggctcgccgcacaggctgcccatcaacgcaagaatgtcggccttggcgctgccgccggcctgcagggcctgggtcaccaggcggtcggccacggcgatggcgcccgcattgatgaacgggttgcgcggcttgccgtgttcgttctccagctgcaccagcgagttgaacggattgcccgatggctcgcggccgatgcgctcccacagcgcgtcgcccatgcgctgcatggccagcgtcagcgtgaagagcttcgacacgctctggatcgagaacggcgtttcggcgtcgccggcgaaagcctcggtgccgtcgcaggtgcgcagcgcaatgccgagctggcgcgggtcgatgcaggccagcgcggggatgtagctggccacggtgccggcttggcccagcagcggccgcagggtgccgacgatgtcgtcgagcaccggctgaaaatccgtgtctttcatgggcgcgccctccgccggttgaccatcacgatgcccagcgccacgcccgccagcgcgagcatcagctgcagcgtgagcggttcgccgagcagcaccacgccgaacaccagcgcgaacagcggcgtcagaaagctgaacgacgacatctgcgtggcgggatagtgccgcagcagccacatccaggtgagatagctcgcgaaggcgccgaccacggtctgcaggccgatcgaggtccacgcccacaccgaatacgagaagccccacttctcgccgagcgccagcgacagcagcgggcacacggcggcggtcacgcctacttgatagaacaaggacttctcggcgctcgcggtggccaggcgcgtggtgcgcagcgccagggtggtcagtccccagagcatgccgcccgcgaggcccatggcatcgccgatcaactggcccgagcccgaatgcccgaagccttcgctgaacgcgaacagcacggccgcgaaggcgatggtgaggcccagccattgcaggccgcgcaggcgttcggcgggcacccagcgcggcagcagcagcgacacccagaacggcgcggtgtacaggaacaccgtgagccgcgaggccgaggtgtgctgcaggcccaggtagatgcaggcgaactcgcccgcgaacagcagccccaccaaaaggccgcccggcagcgtgccgtcgcgctcgaaaagcggcacgcggcgcgacacgcaccagagccacagcagcgcgacggcgccgaccatgcggatcgatgcctgccagagcggcggcacttcggccactgtggtcttgatgaggatctgctgcagcccccagaacgcgcagcatgcgatcaggaggccgatggcgagggagtcgaggtgggtcttgcgctggatcattcgtcgcgttgttgtcgtcgttgccgctgctcgtgcggctgctgtttgttcgttcatcggccggccacgggataagtcggcttgccccgcgtgcccaccatcaggtcgggcaccacggtttcgacatcgggcaccacgcgtgcggcgcgctcgagtttgcgggccagtgcggccgaaggcacgcagccttgcaggtagacccagcggcgctggatgaccacccacacgctgctcttttgcacgcccggcacggccagcagcgcggcgcgcaccttgggcgcgagcggcttgtcgtagcggtaggcgttgctgtcggtgcattggcccgcgagccagcagctggtgccgcgctccagccgcgaatgggtctgggcgcgcctttcctccgcggtatagaacgggccttcgggcatggcgcaggcgggcaggccggcggagatgcggaagaagggatcgtcgaaccagttctgcttgagcggtgccgcagcctcctgcgccgtggcggcctgcgcagccagcagcagcacggacccgagcgctgcggcacggctcacaagggatgttccgtgtagaagcgtccgccgtggaacagcagcggcgaggcgcccgcgttgtgcgtgcagcgctccacttcgccgacgaagatcacgtgatcgccttcgtcgtagcggctgcggttgaagcactcgaagcttgccgccgcgcccgccagcaccggcgcgccgcccaggccttcggtaaaggccacgtcggcccagcggtcgatgttcttggtggcgaagcgttcggccagctgcttctggttggccgcaaggatgttgatggcgtagtgcgagccggtgctgagcgccgccatcgaggcggccgcgcgtgccaggctccacagcaccagcgggggctcgagcgacaccgagttgaatgaattggccgtgaggccgaccagcacgccctcggccgagcgcgcggtgacgatggtcacaccggtggcgaacatgccgagcgcgctgcggaattcttcggtcgagaaggaaggcggttgcgcctgggcgggagcgttcacgagaaaagccagagagagagtgcgcagaatgacgccgctctattctggcccaaggccgcaatggccgccgccgccccttcgcgcggcctgtctgatcttgctggtgattagattaattggcgacaagccgccgtcgctatagcaaagaatgcatagggaaagctctcgtatttctttctcaacttgacactgataagattaaaacgcgccccgcgatcgacgggagcgatccagaaaaaggagacgacatgctcggacgacaactctctcggcgcatgctgcggtgggcgccgctcgccgcgctggcgctcttcggcgccgcggcttcagccgccggcgcctacccggaccggcccatccggctggtcgttccctatacggcggggggcatcagcgacgtgctggcgcggacactggccgagcgcatgcgcaaggaactcggccagcccgtgatcgtggacaacaagcccggcgccaacaccgccctgggcgcgcgcctggtggcctcggccgagcccgacggctacacggtgctatttgccaccggcgccactgcggtgctgaatccgctgctctatcccaagctgtcgtacaaccccgagaaggagctgcagcccgtggcccgcatcgcggtcactccgatcgtgatgttggtcggcaacaactcgccgcatcgcacgctgcgcgacttcgtcgccgatgccaaggcgaacccgggcaagctcaactacgcatccacgggcaccggcagctcgctgcacctggctgtcgagctgctgcaaaacgccactagcgtctcgctggtgcatgtgccctacaacggcagcgcgccggcccaggcggcattgatggccggcgacgtccagttctttgccgactccacgggcagcgccatgggcctggtgcgcggcggcaagctgcgaccgctcgcggtcaccacccgcgaacggctgccggcgctgcccgatgtgccgacggttgcggagagcggctaccccgactacgaggtcaccacctggttcggcctcatgctgccgcgcaacgcgccgcccgacgtggtgagccggctgaacgcctcggtggcgcaggcggtggcggaccgcagcttccgcgaacagttcgaggcgctcggcctggtggtgccgccggcactgacgccggccgagttcaacgcctacatcggccgcgagcgggagcgctgggcgccgctgatccgcgccaagaacatcgtcctcgagtaagtctcgcagcctcatcggaagccattgcatgttcgaagccaacctgctgcgcggcaagcgcatcctcgtgaccggaggcggctcgggccttggccgcgagatcgccgagcgctacctgcaactgggcgcggaggtccacatctgcggccgccgtcagccgatgctcgacgccaccgccgccgagctgaccgaacgccatggcggcgtggtgcgcgcgcatgcggtggacatccgccatgccgacgcggtcgatgccatggtcgagcgcatctgggccgagcacggcccgctcgacgggctggtgaacaacgcggccggcaacttcgtcagccgcacgcaggacgtgtcgccgcgcggcttcgacgcggttgccaacatcgtgctgcacggcacctactacgtcacccaccacgtcgggcggcgctggatcgcaaccggccacaagggctcggtgatctccatcgtcgtgacctgggtgcgcaccggcgcgcctttcgtggtgccgtcggccatgagcaaggccggtgtggacgtgatgaccaagtcgcttgccatcgagtggggccgctatggcatccggctgaacgccatcgcaccgggcatttttccgaccgaaggcgcgaacagccggctcagccccaaggccgcctgggaagatggcgcggtgcgcaacccgatgaaccggctgggccgcatgcccgagctgcagaacctggcggtgttcctgatggccgacggcgtcgagtggatcaccggcgagaccatcgccatcgacggcgcggggcaccggcagaacggcgcgtccttcacagagctggccgatctggacgacgaagcctggcgcggcatgcgcgaagcgatccgcgggcaggacgcacgcgaccgggcattgcgtgaagcggcttcggaatccaacgggccggacgccgcgccccgaggccattcatgaggatcgaccgcatcgtcgacgaagtggtcgcagcaagccgcggcgaccaccccgcgctggtgctggaggacgggcgcgcgctgtcgtatgcgcaactggccgcccgcatcgaagaagcggcagccgcgctcgccgaggccggcctcgcgccgggccagcgcatggtgctggtgggcgagaacagcgaggacatggtggtgctgctgctcggtgcgatccgcgccggcggctgggcggtgccgctcaatgcccgcatgtcgggcggcgagatcgacgcgatctgcgcgcacaacgagccgcggctcgtgtacttcgcggctggcgcctcgggcgaggcgatggcccatgccgaccgacatggcgccgccggcgtgctggcctgcgcgccgggcgggcgcttgcagcgctgcgagggctcgggcacggcggccgaagatgcgtccggcgacgtcgccctgatgatctacacctcgggcagcaccggcctgcccaaaggcgtgatgctgacccatggcaaccttgatttcgtcacgcgggcttcgatggcgcagcaggtgctgctgccggacgacgtgatctttcatgcgctgccgatctcgcattcgttcgggctgatctccgcgctgctgtgcggcctgcgcgcgggcaccacgctgcgcctggtgggccgcttctcggccgggttgctggccgaggcgatcaccgccggccaggttacggtgttccagggcgtgcctgcgatgtacgcgcggctgcacgaatggtcgcagcagcagggccgcccgcttacccccaaccggctgcgcatggcctacatcggcggctcgctggtcgacgccacgcgcaaggcgcagaccgaggcgctgctcggcctgccgctgcaccacggctacggcctgaccgaatcggcaccggcggcgactcgcaccttcggccatccgccgcccgcggacgtgaccgccggctggccgattcccggcgtggaggtggtgctcgcggatgcggacggccggccggtggcaggcggcgagcgcggcgaggtcctgatccgcggccccaacgtgatgaagggctactttcgcgacccggcgcagacgcgcgcggctgtcgatatggagggttggctgcacaccggcgacatcggcgtcttcggaccggcgggcgacctctccatcgtgggccgcagcaaggagatgatcatccgcggcggcttcaacgtgtacccggccgaggtcgagaaggcgattgccgcctttccggaggtcgcgcagtgcgcggtggtcgggcgcagcgtgccgggcgacgaggagatcgtcgccttcgtcgagccgctgcagggccgcagcatcgacaccgcgcggctctgtgccttcttgcgggaacgcctggcgccctacaaggtgccggccgaagtgcatgtgatggcgcaactgcccgccagccccaccggcaagctgctcaagtcgcaactgaaggcgctggcgcaggccgcaccggcggcggcgcgaccatcgctcgaacgcttgctggcgccgcgctccgtggcggtggtgggcgcatccgacaacccgcacaaggtcggtggccggccgatccgctacctgctggagcagggcttcggcggccgcatctatccggtccatccgcgcgccggcgaggtgcagggcctgcaggcctacgcggcgctcgaccagctgccggaggtgcccgatgcggtggtgctttgcatcggcgccgggcaggccgagcagcagcttgccgagtgcgcgcggctgggcgtcggccatgcgctgctgttcgcctcgggctatgcggaggtcggccccgagggccgcttgcggcaggaagccctggccggcatcgcccgtgcgggtggtgtccgcctggtggggccgaacagcatcggcgtcgccagcttcgacagcggcgcggtgctctccttcgcatcgatctacagcgaccatgcgccgctcgacggtccggtggcgatcgtctcgcaaagcggcgctttcggcgtgtccgcctatgcgctgctgcgcgaggctggatggggcgtgcgctgcgtggccgccaccggcaacgaggccgacgtggacactgccgacctcgtcgatgcgctggcgcggcagcccggcgtgcggctggtgctgctctacgtcgagcacgtgcccgacccggcgcgcatggccgcggcgctcgacacggcccgccagcgcggcgtggcggtgctggcggtgcgctccgggcgttccgcgcacggcaggcgctcggccgatctgcatacgggttcgggcggcgcggcgggtgacgagctcgatgccctgttcgaggcgcacggctgccgcaccgtgggcggcctggtcgaactggtcggcgccgtgccgctgtacctcgggccggcgatgggcgtcggcggccacggagggctgccgcggctcgcgctcgtcagcaactccggtgcgtcctgcgtgctggcggccgacgaagcgcaggctcgcgggctaccgctggcgcggctggcagcgcacgcggagcagcgcctggccgagctgctgcccaatttctcgctcaaccgcaatccggtcgacctgacggcgatgctgctggccgaaccggcattgctcggcgcggtgatgcaggtggtgctgcatgacgaggcagtggatgccgctaccctgggcctgctggccgtcggcggaccgagctacgacctgccgcgtttcgtgcgcgaatgccgggccgtggtggacgatgcgggcaagccgctggcggtctacagcccgcacgcccatgtgcgcgaggccttcgcccgtagtggcttcgccgtgttcccgggcgaggccgaagccatgcaggcgttgcaggccttcgcgttgcaccgcggccaatcggccggggcccgcgcggcgcttgcgctcgaccttccggaagcgagccgcgctctggcggaagtagtgccgggctagcttgccgccggctggtggtccagccccgcgatgaagatcgagaacacgtcgtggccgatcttcatcgggtccttgccgacgatgtcccaggcgttctggcggtcgaccatcacggtggccaggccgtggcaggcggtccatgcggccagcgccgcggggcgcacgcgggccagcgggacgttgcggtggctcaggtagtcgcccacgcaggtctccaggatgccgtaggagcgcgtggcggcttgctccaggtcggggaactgcagcttctgcggaatggccgggccgtacatcaactggaacagcgcgggccgctcgatcgagaactgcaggtgcgcgagcatcacgctcagcagccgttcgcgcggatcgctgaggctgcgcagcgcgcggatgcgctgctcgaacatcatgcgaaagccctgcgcggcaatggccgcgaggtagcccgacttgccctcgaaatggtgcagcggcgcggtctgcgacacgcccacgtcgcgcgccgcctggcgcaggctcagcgcggccaggccctgtgcatcgaggatttcgatgccgcgcatcaccagcgcatcgcgcaggttgccgtggtggtaggtcgagcgcttggcctccgcatcgggcaccggcgcatcagcgccgggtgccgccggaaccgtgcgcgatccggcatgcgacctggaggcggaggagcttttcttcatgggcctgcgagcttaaaccggcagcaccgcgcgctgccgctcatccgaagaaccagtagcagaccgcgatcgccgccaccacgcccgcgagttccgcggccagtgcacaagacaccgcatgccgcgcacgctggatgccgaccgcaccgaagtacacggccagcacgtagaaggtggtttcggtgctgccctggatggtggcggccgcgagcgcggggaagctgtctacgccctgagttttcatggtctcgatcagcatggcacgcgccgcgctgcccgagaagggcttgaccagcgcggtcggcatcgcgtcgacgaaacgcgaatcccagccgcccgcgtcgaccagccagcgcagcccgccgagcacgaagtcgagcgcgcccgaggcacgcagcacgccgaccgcgcacagcatcgccaccaggtagggcagcaggttcttcgcgatgtcgaagccttccttcgcgccctcgatgaagcattcgtagaccttgatgcgccggatcgcaccggccagcaggaacacgatgatcacgccgaacagcgccaggttgcccatgagcgaggagagcgacgcaatcgccgccgccgacaaggtgcccagaagggccatgaagccgcccagcagcagcgcgcccggcaccaggtaggccagtaccaccgggtcccacagccgcaggcgctgcgccacggccaccgtgagcaggcccaccagcgtcgatgcgctggtggccagcaggatcggcaaaaacaccatcgtcggatcgcttgcgccctgctgcgcgcggtacatgaagatggtcacgggcaacagcgtgagcgacgaggcgttgagcaccaggaacaggatctgcgcgttggtggccgtgaccgggtcggggttcagccgctgcagctcgcgcatggccttgaggccgatgggcgtggccgcgttgtcgagcccgagcgcattggccgcaaagttcatcgtgatgaggcccagcgccggatggcccgccggcacgcccggcatgagccgcctgaagagcgggccgagcagccgcgcgagccagccgaccagccccgctgcctcggcgatgcgcaggaagccgagccacagcgtgagcgtgccgaacagcagcaccatcacctcgaccgcgagccgcgccatcgcaaagaggctttcgacgatcgccgcaaaaacggccgggtcgccgcccacgagccagcgcccgagcgcggccagcatcgccattccgaagaaacctagccacaagccgttgagcacgcgtgttctttcctttttttgtgagcgcgatcatagggctccattcgcgcctgcctggagctacagtgcggcccatggcagcctctcccctgatccgcaggctcgcggccctggtgtgggccgccgtggcctcagcgtggctggcgggctgcgcgagcctgccgccgccgcaaccgcgtgctccgactgcggccatcaccgacgtggccggcaccgcgctgggccaactggtgaggccgggtgcgcccgatgaagccgcatcgctgtccggctttcggctgctcccggaagcggccttcgccttcgacgcccgcatctcgctcgcgcggcatgccgagaagtcgctcgacgtgcagtactacctgatcgagaaagacgatgtcggcctgctgctgctgcgcgaactgcgcgatgcggcggcgcggggcgtgcgggtgcgcctcctggtggacgatctctacacgggcggcgaggacgagctgttcggcacgctctcggcgtttcccaacgtcgaagtgcggctgttcaatccgctgccttcgcgggccgactcgctcgcgctgcgtctcctgctctcggttgcggatttcggccgcatcaaccaccgcatgcacaacaagctgctggtggccgacaacagctttgcagtctcgggcggccgcaacatcgccaacgaatacttcatgcgcggcacggcggccaatttcatcgacatggacgtgctctccagcgggccggtggtgcgcaagatgtccgaaggcttcgaccgctactggaacagcgagcatgcgtggcctatcgagcgcatcgcgccgctgcgcatgacggtggacgaggcgcagaagcgcttcgatgccatcgccagcacggcgcagcccgacgtgccgattcgccagcgcgacgtgatggacaagtcgccggtgggcgagcagctcaccaccggcaaggtcgatctgcgctgggcaccattcacgctgttcgtggacgaccccgcgaagatcacgcgctcgcccgaagcggcctatgcgggcagcgtgaacgagggcgcgctgggcgtcatcaattcgggcaagcgcgaggtcaagatcgcctcgccgtacttcattcccggcccgcccggcatggccatgatgaaggcggccatcgcgcgtggagggcgcatcaccgtggtgaccaactcgctgggcgccaccgacgagccgctcgcctacgcgggctacgagcgctaccgcgccgacatgctgaagatcggcgtcaccatctacgagatcgcaccgatgctcaccgggcgctcggggcacttcggcaacttcggccagtcgatcagccgcctgcacgccaaggtcgcggtgatcgacgacgagcgtttcttcatcggctcgatgaatctcgatcgccgctcggccgcggtcaacaccgagatgggcctcgtgatcgacagccctgaactggtggccgactacgaaaagctcatgggcggggagcgcgtgagcctgggctaccggctgcggcttgcgcccgacggccgccgcgtgcagtggctggaatacgacgatgcgggcggcgacgtcgtgcacgaggacgagcccggcgagtttctctggctgcgcttcaagaactggctgctgctgccgatcgtgggcgaagaactgctctagcgtcagggcacttcgatcagcagattcgggcgaaagccttcctgttcgcccttgcccttgtacccgagcggattggccaccacgcggcagccgtccttcacgtagtcgaaggggcagtgcaggtggccatgcagccacagccgggcgcggggcagcagcgcatcgagcgaattgcagaaacccgccgtgcccggcgtgaggccgtagcgcggatcggcgctggccaggctgggcgcgaaatgcgtgatggccaccgtggtgccgtcgaacggctcggccagcgccgcttcgagccaggcctggcatgccagcccctgctcccgcatcgcaccggccatgaagggctggccatggcgcacggtggcggctttttccaggtagaaatcggccgcccgcatggccttgccgcgcttcttgagcgcgtccgccaggccgtcggtgggcgttaccagcgcgtcgaagtcggcccagagggtggtgccgatgaagcggatgccgtcgatgactgttgtttcccgctcgagccagaggatgtcgagctccttgcagagcgcacgcaggcgctcgtgggtctggtcgaaatcggcgttgtcgtattcgtggttgcccggcacgtacatcaccggcacgggccagccgttgcggggcgagaagcggcccaggccgaagtcggtatcggtcaggcgggagccttcctggtaggacccgatgtcgcccgccagcaccagcatgtcggccccgggcgcgggctcggcctggaaccggggatgggactccaaatgcaggtcggagagcagttgcagcttcatcgtctactcagtctaggggaatcagcccatgcataaagcgcatgaagtggggctttcaatattagggataacccctattcttaggacatcaaccactccagcgcagccaaaagcagcgcactgtcatgttcagcctcattgcccaagtggcccgtttcttccgttcttccaatgacagcatcccggccagccatgccgcgacgctgatggaaaccgccgacgtccgtgccggcctcgacgcccaccacgcgcaggaactgcgcgttgcggcatcggcctggctttcggtcgttcgctaaaaaaaagcccaggtcagccgggcaccttctgcccgaggaccgaatccgcgaaagccgccgcggccgaacgcagcagcgccgtgcgcagccattcgtgcgcgtgcccatgctgcgcacgccgatgccagatggcgtcgacgtgcaccatcggctggtcgaagggcaggtcgcgcagcaccagctggtcatcgatgccggtgacggtgacgaaatgccgcggcagcaccgtgagcaggtccgaattcgcgaccacccggcccgcggtgaagaactggttcaccgtcaccacgatgcgccgctcgcgccccaaggcgcccagcgtctggtcgatgaagccgtacggccgccccgaaaagctcacgagcaggtgccgcgcggcgcagtagtcgtccagcgtgagcggcgcatccgcgagcgggtgtccgcgccgcatcacgcagacatactggcccagatagagccgctgcgtctcgaacgccacccccacgcccgattggccacgcgccgccaggctggcaatcacggccggaaagtagccgatcgccatgtcgacttcttcctgctccagcatgcgccgcggatcgcgtgtggtcagtggcagaacgcgcagcgagatagcgggcgcttccttctccacgattttcaccagccccgggatgagctcggcggccgtcgcatcggccatggccaggaggaaggtggtgtcggccgtcgctgcatcgaactcgcccggcgcgagcgtgtgctgcagctgcctgagcgcatcgcgcacggtgggccagagcgccagcgcgcgcggcgtgggctcgacgcctgcgcccgaccggctcaccagctcgtcgccgagcacttcgcgcaggcggcgcagcgcattgctcaccgcgggctgggtgatcgacaggttgcgcgcggcgcgcgtgaggttgcgctccgccatcacctcgtcgaagacgcgaagcaggttgaggtcgaaggtgcggaaattgacgtccatcagtgttgtgaatgataaacatcagaaagataaagtggataaacactagggcaaaccctaatatcactacatcggcactcagccattcatccctggagggattcatcatgaccagctttgtccacgtagaccaacccactgtgcaccctggcgtccagcgcgccgaggtgttgttcggccagatccaggccgcccgcgccggcgcgagcggttcgcgtccgctgattgtcctgctgatcgttgccgtggcttccgcggtgctggtggtggccgacacgctcgttgccaactgggacgaaggcgctttgctcgccgcctgggctgtgctctgcggcgccgctttcggcatcgccgccctgtttgccggctcgctgcgcaacgcggccgccaaggttgccggcgtgttgagtgcagccgcccagcgccgcgccgccgaccgtgccgacgagcgctttctggccactgcgcacagcgacccgcgcgtgatgcaggaactgcaagccgctgtctggcgccagcagtcggaaggcacggcttccattgccacggttgccaaggtcgacgcactggcccgccgccaggccgcacgtgccaacgacgtccgcatgcccacgctctacgaagccatgcgccgcatgaacagctcgcgctactactgatcgacccattcgattcttcagccgagtcatgaaaaagccgcccacgagggcggctttttcgttgctgcggcccggtggccgcacatggagaggcgtcaggccgccaggcgctgctcgatcgcggccttggtttccggcagttccttcggcaggtggtgcgccagctgctggaacagttcggcatgcagcttcagctcggcctgccaggcggccttgtcgatgctggtgacggtggcgaactgctcggcgctgaagtccaggccggtccagttgaggtcttcgtagcgcgggctcacgccgaagacatggtccacgccctgggccttgccttcgatgcggtcgatgatccacttgagcacgcgcatgttctcgccgtagccgggccagacgaacttgccgtccggacccttgcggaaccagttggtggtgtagatcttcggctgcttggcacccgaggcttcgagcttcttgcccaggtcgagccagtgctggaagtagtcgctcatgttgtagcccatgaaggccagcatggcgaacggatcgcggcgcaccacgcccacctggccgacgatggcggcggtggtttcagagcccatggtggcggccatgtagacgccctcggtccagttgcggccttcggtgaccagcggcaccgtcgtcgagcggcggccgccgaagatgaaggcgtcgatcggcacgcccgccgggtcgtcccaggccggatccaacgctggattgttgatggccgcgacggtgaagcgcgagttggggtgcgcggccttggcgccggtttccttggcgatctgcggcgtccagtccttgccctgccagtcgatcaggtgctcgggcagcttcttgccgggcacgtcgtcttccaggccttcccaccacacgtcgccgtcgtcggtgagccccacgttcgtgaagatcacgtcgcggtccaggctcttgaggcagttggggttggtcttgaggttggtaccgggggccacgccgaagtagcctgcctcggggttgatggcgtacatgcggccatccttgccgggcttgatccaggcgatgtcgtcgccgatggtcgtgaccttccagccgtcgaagccggccggcggcaccagcatcgagaagttggtcttgccgcaggcggaggggaaggcggccgctacgtggtacttcttgccttcgggcgaggtcacgcccaggatcagcatgtgctcggcgagccagccctcgtcgcggcccatggtggaagcgatgcgcagcgcaaagcacttcttgcccaggagcgcgttgccgccgtagcccgagccgtagctccagatctcgcgcgtctcggggtagtggacgatgtacttggtcttgttgcagggccaggccacgtccttctggccggcctcgaggggcgcgcccacggtgtgcacgcagggcacgaactcgccgtcggtgccgagcacctcgtacacggccttgcccatgcgtgtcatgatcttcatgttgaccgcaacgtaggggctgtcggaaagctcgatgccgatgtgcgcgatgggcgagccgagcgggcccatgctgaacggcaccacgtacatcgtgcggcccttcatgcagccgtcgaagagcggctgcagcgtggcgcgcatctcggccggggccatccagttgttggtggggccggcgtcttccttcttctcggagcagatgaaggtgcggtcttcgacgcgcgcgacgtcgctcgggtcggatgccgcgaggaaagagttgggacgcttggcggggttgagcttcttgaaggtgcccgcgtcgaccagtttctggcacaggcggtcgtactcttcctggcttccgtcgcaccagtagatggcctccggtttgcagagcgcggccatgtcggccacccaggccaccagttttgcgttcttgacgtatgagggcgcctgaatggcgaggccctgcatcgtgggtgcgttcatcggaaatctcctaagttgaaaaatcgtctttccgaacgggacgccgcgccggcatggcgcggaggtccgtttgagaaaacgtttctcttagagagactgcgtcaacgcgggccgcaaaacccgcggacgaagacgcaaatcgctgtcaggccaaatagacagcgatggacgcgagcagcagcatcagcacgccgccagccaacggcagcacgatcggcatcaggtgcacgaccgattcgacggcgtctttttcaacggcggcggcgtggtggggctcgacgggagtggggttggacattgaaattacctcgaatactcagattcaaaaactggggggcattttacgggtcgggcccgccggacgggtctagggggttgccagccccctcaatgctgctcttcggcctcgaagccggcgtcgtgcagcgcgcccagcacgctggccaggtgggcccgtccgcgggtctgcagcaccagctcgatgtcgacgttctgcgctgccagcatggtaaacgcacgttggtggtgaacctcatcgacgttagcgcccgcttctgccacagtggccgtgatctgggccaatgaccccggaacgtcgcgcgcgctcaccctcacgcgggccagccggccggcccgcaccatgccgcgttcgatgatggccgcaagcagcagcggatcgatgttgccgcccgaaagcaccagccccacgcgcttgcccttgaagcgctccggatgccggatcagcgccgccaggccggccgcgcccgcgccttcgaccagggttttttcgatttcgagcagcatcagcacgccctgctcgatgtcgccttcgtcgaccagcagcaggtcgtccacatgtttggcgatgatttcccgcgtcagcacgcccggcgtgccgaccgcgatgccttcggcgatggtgctcttgccctgcaggtgctgggtgcccttgacggcattgaccatgcccgggaagcgcgtggtctgcacgcccacgatctcgatgcccggcttccggtcgcgcgccgcaatggccatcccggcaatcagcccgccgccgccgaccgacaccaccagcatgtcgagatcgggcaccgcgtcgagcatttcgagcgccaccgtgccctggcccgcgatgatggcctcgtcgtcgtaggggtggacgaaagtcagtccttcgcgctcggccagctccagcgcatgcgcgcgggccgcgtccagcgtgtcgccgtgcagcaccacctcggcgccgaagccgcgcgtgcgctcgatcttcacgccgggcgtgaaccgcggcatcacgatgagcgcgcgcaggccgagccgctgcgcgtgataggccacaccctgggcatggttgccggccgacatggccaccacgccccgcgtggtttcctggccgtcgccgcgcggcccattctccgaaagatcgaccaatttgttgcacgcccctcgttccttgaacgaggaggtgaactgcaggttctcgaacttcaggaacacttgcgcgcccacgatttccgagagcgtgcgcgattcgacacagggcgtgttgagcacctgaccctgcagacgcgccgcggcgcgccggatttcttcgattccgaccatggcgggcattgtggccggaatcgcaccatcagggtttttaccgttccagcgtcttcccgaaggcaaaagtctgcgctatggtcgccccaggaagttcctcgcctggaggttgtctgatggtcaagcgtgcgggtgtcgatgtggtggctgctgcggtgcgcgggcaggcattgccgtcgcctgggctcaagggagcgccggtgctcgagctgatgtgctcgcacttcgtgctcacgctcgccgccaagcaggggccgcgcttcaacgtgcgccgcgacatcaacggcctgctctcgctcaccggccgccacctggtctggccggccgcggtgctgcatcgcctccgcgagttcctcggccgccgctgcgcgggcaacgaggcctggaagggcgtcgagaatttcgacggccgcacgctgctggagcgccacggcgtgtggcgcggcccgtacgaggaaggcacgctcttcttctatctggacgaatacgccaaggaccagcccaaggacctgctctcggtgctggccgtcacgcgcgactggctcacgcatgcgctgcgcaagcagtcgacgctggtcgagaaaaacatcgatgcgctcgcaggcctcttgcaactcaacaaggccgagcgcgcactgctgctctacggcacgctcgcgcgctaccagcgcgacctgcgttcgctgctggtcgagttcaaggtcaacaatgcgcccgaggcctacgcggccattgccgacatcgcgggcgtcaacgcgagcgaagtgggcgaggcgctgcgcgcgggctcgcggctggagcgcatcggcctggtcgagaacctgatctccgagcacaacattaccgacctggccgacctcatgaaggtcagcgaaaagctgccgccggtgctgatgcgcgaataccgcgaccacaacgaactgatggccgtgttcacgcggccctcggccaagagcgcgctcaccacgcaagacttttcctttgtcgaggaagacgcacagatgctcgtcacgctactgcgcgcggcagtggcgcgcaaggagccgggcgtcaacgtgctgctctacgggccgcccggcaccggcaagaccgaactcgccaaggtggtggcgcaggctgcggggctcgagctgttcgaggtcgaatatgccgaccgcgacggcaactcgctgagcggccgagaccgctaccgctcgctgcagattgcgcaggtgttcctcaagggcagtgcgcaggccgcgctgctgttcgacgaggtcgaggacgtgttcccgcccatcagcaccgaggccgcgcagttcatggcgcgcgccgagcagattccggcgcccaccagcggcagcgtgagcggcaaggcctgggtcaaccagatcctcgaagccaacccggtgcccacactgtgggtgaccaaccgcatcgagcagatcgaccccgcgttcaggcgccgctttgcctatcacctcgaactcaagtcgccgccccccggcgcgcgcgagcagctggtgaagaaaacgctcgaaggcatcgtggtgtccgaagccttcaccgccaagctggccgagcgcaagggcctcacgcccgcgcagatccgcaccgcggtgcgttttgcagggctggcgcagacggaggatggcgcctcgatggaggcgctgatcgagcggcagctcaagaacgccgacctcgcgctgggcaccctcgacaccggcccgggcgagcgccgcagcgtgaccacctacgacctggacatgctcaacgtcgagacccgcttcgaaattccgcgcatcgtggtggcgctcaaggcgcgcggccacggcacgctgtgcttctacggcgcgcccggcaccggcaagaccgcgctggccgagcacatcgccaaggccatcggccggccgctgatcatcaagcaggccagcgacctcatgagcaagtacgtcggcgaaaccgagcagaacatggccgccatgttcaaggaggcggaggccgaaaaagccgtgctgttgctcgacgaggccgacagcttcctgcaggaccggcgcggcgcccagcggacctacgaagtgaccgaggtcaacgagatgctgcagggcatggagcgcttcaacggcatcttcatctgtaccaccaacctgctcgaccggctcgaccaggcggcgcttcggcgcttcaccttcaagatcaagttcatgccgctcaccgcgccgcagcgcgagcgcatgttcgtgaccgaggcgctggcgggcgatgccgcgctgctcaccggagagatcaaggcccgcctcgcgcaattgcgccagctgtgcccgggggatttcgcggccgtgaagcggcagacggacattctggcggtcgatttctcggccgccgaattcctcgaccagctcgaggccgagcaccgcatcaagcccgaggtgcgcgagtcgcgcggcatgggtttcgtgcagtaggtagacgccggaagcggccgcaacaggtccgccggaacacggcaaacaaaaagcaaccgtccgtcgcagcggacacgaggagggttcgatgaactttggcaacgcgagcgcgcgggagatgccgcgctccaccgtatcggccgcggccgcattcgtgctggcctgcgcggccctcgtcctcgcgggctgtgggggcgggggtggcggcggaggaggagggggcgtcgcgttcccgatcgttgcgccccccacggccatcgcaccgccgcccggcggcgacgacgatgccattcttgcctcgtccaccgtggcgggcctgtgcgccgcgccgcgcggcggcatcaaccccgaaaccggggtggcctaccccgacaaggccggcaccctgaccgacgagaagcgctgggtgcgcggctggatcgacgaaacctatctctggtacggcgaggtgccgaccacgctcaaggcggccgactacgccacgccggtggcttatttcaacgtgctcaagaccccgctcgtcaccgcgtcgggccgcgcgaaggaccgctttcattacgtgtacgacaccgagcgctaccggcagttgtcgcagaacggcgtggcgccgggctacggcatggagttcgcgttcgtgcgcaactcgcgcccgcgcgacctgcgcattgcgttcatcgagcccggctcgcccgcggccggggccggcattgcgcgcggcgccaaggtgctcgaggtggacggcatcgacgtgatcaacggcaccaacaccaccgtcatcaaccgcggcctctcgccgacgacgatcggcgagtcgcacaccttcaagctgcaggaaggcagcgcgacgcgcaccgtgacgctggcggccgcgagcgtcacgcgcacgccggtgcagaacgtgaagagcatcgacaccggcagcggccgcgtgggctatctgctcttcaacgaccacatcacgacctcggagccgcagctcatcgatgccttcaaccagttcaggcaggacggtatccaggacctggtgctcgacatgcgctacaacggcggcgggcagctcaacatcgcgagccggctcgccaccatggtgtcttcgtccaccgcttcctcaggcaaggctttcgagcgcctcgtcttcaacgacaagaacccgttccgcctgacgccggcgcagtcgatcattccgttctacggcaccagccgcaccggcgcgccgctgcccaggctcggcctttcgcaggtgacggtgctggtcgggcccgacacctgctcggccagcgaatcggtcgtcaacagcctgcgcggcatcgacgtcagggtcaacctcgtgggcggcgccacctgcggcaagccctacggcttctcgccgcaggacaactgcggcaccagctacttcgcgatccagttccagggcgtcaacgccaagggcttcggcgactatggcgacggcttcgtgcccgactgcaccgtggccgacgatttcgaccatgcgctcggcgacccggccgaggcacggctcgcggccgcgcttgccatgcgcggcggcggcgcatgcccggcatcggcttcggccaaggcattgccggggctggaaaaatccgaagcgatcgaggagcagccctacctgcttcatcgcaccccgctgcgcgaaatgcgcctgctcgaagccgcgcccgcgccgggctgagccggctcggcggcgtggtcgttaccctttgaaaccttgccctttgccacgcccacggcttgcgctttagagtgcaagcaaacgtttgcgcaaacgtttggcatttagttctacatcgccaacaacaccaccactcgagaaggagccgggatgaagattcggattcagcgacgcaaatggatggcggcggctttgctcgccacggcgctttcggcctgcggtggtggcggtggcggtggcgacggcaacagcggcatcgggctggccccggggtttggcgcggccccgccgccggcgcagaagatcatcatcgacagcgactacaacaccatgagcgacgacggccagctcggcgtcatggccgcgcagctgcaggcgtcgggcaaggtgcaggtcatgggcatcagcgtggtgtcgggcaaccagtggctcaagcagggcgtggccgatgcgctgaagtcagtggagcggctgggcgtgggcgaccgcatcggcatttatgcgggtgcgaactacgcgttcaaccacgactacgcgaccatcgaggccgagatggcggccggctccggcggcgacggctacctgggcgcctggagttcgcccgagcccaagagcgatgccgacctgaagccctcgcccgacggctttgccacgcatacgccggtgcagggcaagagcgcggtcgatttcatcgtcgacaccgtgaaggccaaccccaacgagatcaccatcctggccatcggcccgctcaccaacatcgcgctcgcggtcaagcggaaccccgagatcgtgccgctgatcaagaagatcatctacatgggcggcgccatcgacgtggcgggcaacaccaccaagtttgccgagttcaactggtggttcgatcccgaggccgcgcagttcgtggtgcggctgccgattccgcaggtggtggtgccgctggacgtgaccgacaccgtgttcctgaccaagcccatctacgaccgcgtcgcgcacaccgccaagccgacggccgtgaccgaggtgttcgggcaactcaacggctatggcttcagcggcaccaatggcttcgagaacaaccccagctacacgcagaacatctgggacacgctcacgctcgcctacctcatcgatccgagctatgccacgcaaacggtggagcgttatgtcgacgtggtcgccaaaccgggcgccgccgacaacggccgctccatcggctacagctcgcagcccgcggggcccacgctgcagaagatgacggtggtgaagaagttcgacaacgcgcgattcttcgagctgtatgtcgacctgcttacgcggcccgtgccgatcacgctgcctgccgccacgaactgagcgtcataagccgcgcttatccaaacgcaaccaggagacgcattcccaacaggttttgccttgcggatactcgcccacgttcgctcccgaacgcacaacgattccgaccgagacaaacgccgtgcctcctgccgccatcacagccatcgacagccatgcccatgtgttcgcgcatggcctgcccttggcggcggcgcgccggcatgcgcccgactacgaggccacgctggccgaatacctggcgctgctcgacacgcacggcgtttcgcatggcgtgctggtgcagcccagctttctgggcctggacaacagcttcctgctcggcgcgctgcgcgcctgccccgagcggctgcggggcgtggcggtggtcgacccgaccgcggacgacgccatgctgtattccatggccgaggccggtatctgcggcatccgcctcaacctcgtgggcctgccgctccccgatttctccaggcccgagtggcaccggctcttcgtccgcgcgcgggcgctcggctggcatgtggaactgcaccgcgaatcccgcgacctggcactcgcagcgcaggccgtgctcgatgccggatgcgcgctggtggtggaccatttcggccggcctgcgtcggcgcccgccatcgccgatgaaggctttgcctggctgctcggcaccgcagccagcgggcgcatctgggtcaagctgtcggccgcctaccggaactggcccgcggcaacggccggcacagccgcgcgcgatgccgcccgcgcgctgctgaaagccttcggccccggacgcctggtgtggggcagcgactggccgcacacccagcaccgcgaggtcgcgaactacgccgccgcgcaggcggcgctggccgactgggtgcccgacgaaacggcacgccggcgcatccaggtcgacacgcccgcgcaattgttcaagttcaaaaccggagacatcgatgacgaccaatgagctctcgcgcgcacgcctgctgcgcgccattccccgtgcccttgcgggcgcggccctgctgctcgccgggctttcagcgcatgccggcgcgtggccggaaaagcccgtgaggctggtcgtgagctatccgccgggcggcaccgtcgatgcggtggcgcgcatcatcgcgcccaagctctcggcgaagctcggccagccggtagtgatcgataaccgcggcggcgccggcggtgccatcggcggcgacctggtcgccaagagcgcgcccgacggctacaccgtgatgctcgatgcttccaaccacgcccagaaccctgcgctgcgcaagatgcccttcgacacgttgcgcgacctggcgccggtgtcgctgctggtgaaggtgcccaacgtgctggtggtgaatccgtcggcgccgatgaagagcgtcgccgacctgatcgcccaggccaaggcgaagccgggcggcatcaactacgcctcgtcgggcaatgggtcggcgcagcatctggccggcgaattgttcgcctcgatggccggcgtccagatcacgcacgtggcctacaagggcggcggtccggcgctcaccgacgtgatgtcgggacatgtccccgtgttcttcgccagcctggcatccagcctgcccttcatccagggcggcaagctgcgtgcgctggccgtgaccggcaagacgcattcgcccgcattgccgcagctgcccaccgtggccgaggccggcctgcccggctacgaggtctacgaatggaatgcggtgttcgtgccggccggcacccccgcgcccgtggtggagcggctgtcgaaagagttcgccgccacgctcagggaccccgaggtgcgcacccggctcgaagcgctcggcgccgaggtgatcggctccagcccggccgagctcgacagcttccgccgtgccgagatcgccaagtggacccggctcgcgaaggacaacaagatccaggtggactaggccggcgccgggctgctcgcaagcagggcggcgaaagcgtcggcgaacgtcgggcgcgagcgcgccagccacagcgccgacaactcgaaggccggcagtcctgcgccgtcgcgtacctcggcataacgcacgccctcgtgccgcagcgcgcgcaccgagcgcggcagcagcgaccagcccaggcccgccgccacgcaggccagcaccgtcagcgtgcggttggcgtcctgcaccacccgcgtctcgtggcccgcgcggcgcagcgcgccgagcagctgggcgcgcagggcgggaatctgttcttccggaaaccacaccagtccgtgccgggcgatctcggcgagcgacacgcatccatcgtcggccagcggccagtcggccggcagcgcggcgaccatcgcctcctcgcccagccgcaattcgtgcacccgggcggtaaccgacaccggcggatgcagcagcgcgatgtcgatgcggccgccctccagcgccgccacctgctcggcattgctcatctcgcgcagcaccacgtcgagctgcggatgttcggcgcgcagccggcgcaacgcgtttggcagcacctcgtagaccgcatgcgtcacgaaacccacggtcagccggcccgcacgcccggcgcccatggcccgcgcgcgttcggccgccgtgtcgctgtaggcgaggctggcgcgcaggtcgtcgatgaccgcgaggccggcctccgtgagcgtggcgccgcggcgcgtgcgggtgaacaggcgcgtgccgatctcctgctccagccggttcagcgtttgcgtgagcgccggctgtgccaggccgagccgctccgccgcccgcgtgagactgcccgcctcggcgaccgcgacaatgcagcgcatctggcgggtgtccatggctgcgcccgtgtcagaacgccttgcagacccgcagcacctcggcgccgtaggcctcgagcttcttggtgccgatgccgctgatgccctgcaggtcttcgagcgtcgccggtgcgcgctcggcaatcgacgccagcgtggcgtcgtggaagatcacataggccggcaggttgtgctcctttgccacctcggcgcgccaggctttgagcgcctcgaagcgcttcttgccggtgtcgtcgagcttggcagcggccggcgacggcgcacccttggcgactttctcgcggcggggcttgcgctccgcgggcgacgagatggattcgcgcagcgtcacgttcgattcgcctttgagcaccgcgcgagagccttcggtgagcttcaacgtgttgaaggcttccgcgtccaccgccagcgcgcccgtggcgatgagctggcgcagcacgccgcgcagctgcacctcgctgaactccgcgcccagcccgaaggtgctgatgcgctcgtgcccgaactgcttcaccttctcggtttccttgccgcgcaggatgtccatgatgtggcccgcgccaaagctgatgccgctcagctgctgtacgcggtagatggtggagagcagcttgcgcgcggcatcggtgccgtcccacacctgcggtgggttcaaacagttgtcgcagttgccgcagggcgtgctcttctcgccgaagtagcccaggaggcgcacgcgccggcagtcgctcgcctcggccagcgacagcagcgcatcgagcttgccgcgcatcacctgcttgaattcttcgccggcggggctctcgtcgatcatgcggcgctggttcaccacgtcctgcaggccgtaggtcatccaggcgtccgccggcgcgccgtcgcggcccgcgcggccggtttcctggtagtagccctcgatgttcttgggcatgtccaggtggccgacaaagcgcacgtcgggcttgtcgatgcccatgccgaaggcgatggtcgccaccatcacgatgccttcctcgcgcaggaaccggtcctggtgcctctggcgcaccgccgcatccaggcccgcgtgatagggcagcgcgttgatgccggcgccctgcagcatcaccgccacgtcttccacgcgtttgcgcgactggcaatagaccacgcccgcatcgccctcgtgctcgcgctcgatgaagcgcagcagctgcgtggtcgcgtccttcttctcgacgatggtgtagcggatgttcggccggtcgaagctggagacgaactggcgcgcctcttcgagctgcagccgctcgacgatgtcggcgcgcgtgagcgcatcggcggtggcggtgagcgcaatgcgcggcacgcccgggtagcgctcgtgcagcaccgtgagtgcgcggtactcgggccggaagtcgtggccccactggctcacgcaatgcgcctcgtcgatcgcgaacagcgagagcttgccgcgctctttcagcgaatcgagctgcgacagaaagcgcggcgtgttgacgcgctcgggcgccgcgtacagcagcgtgatctcgccgcgcagcatgcggcgctccacgtcctgcgtctgttcccagtcgagcgtcgaattgagaaaggccgcgttcacgccggcctcgtgcagcgcgccgacctgatcgtgcatcagcgcgatcagcggcgacaccaccaccgagacgccgcgccccgcgcgttgccgcgcaatggccgggatctggtagcacagcgacttgccgccgcccgtgggcatcagcaccagcgcgtcgccgccgcccaccacgtggtcgacgatgtcctgctgcggcccgcggaactgcgaatagccgaagacttcgtgaaggatgtcggcgggtgcgctgctgctgccgggggcgtcgagggggaggggggcgagcgaggacacaggcagcgggtgcgaagggcgggatgggcagggaaaggagggaggcgtcgattgtcccccagcggcatcgacatgactgtggcatgaggtttgcaaaggtgaagcccgtcccgccacccttcctgtatagacagcaatctggtgcattttcctgaaggatgcaccggaattgatcctttcgggttatcctgtatatacaagttggggcgcttggcaacaatgcgaggttcgtgcagcccgagtccgggtgcaccgccgagcctttttccagagaacagaaccaggagtacccatggtcaaaccggtaattgtgaaagtcgcgtccctgctggcagcaggcgcatgtgcagcgggcatggctggaacggccgccgcgcaggaaacaaaaattgcgctcggcatgtccggctggaccggcttcgcgccgctctcactggccgacaaggccggcatcttcaagaagaacggcctggacgtcgaactcaagatgattccgcagaaggaccggcacctggcgctggcctcgggcgccatccagtgcgcggccaccacggtggaaacgcacgtggcctggaatgccaacggcgtgcccatcgtgcagatcttccagatggacaagtcctacggcgccgacggcctcgcggtgcgcaacgacgtgaagggcttcgccgacctcaagggcaagaccatcggcgtgagcgcccccggcaccgcgccttacttcggcctggcctggatgctcaacaagaacggcatgacgctgaaggacgtgaagctggtctcgctcgagccgcagcccgccgcccaagccttcgtggccggccagaacgacgcggccatgacctacgagccctacctgtcgaccgtgcgcgccaaccccaccgccggcaagatcctggccaccacgctcgactacccgatggtgatggacaccgtgggctgcgcgcccacctggctcaaggccaacgccaaggctgcgcaggcgctcacgcagtcgtacttcgaggcgctcgacatgatcaaggccgacccggccaaggccaacgagctcatgggctcggccgtgaagcagagcggcgagcagttcgccaagtcgtcggcttacctgcgctggcaggacaaggccgccaaccagaagttctttgcgggcgaactcaccagcttcatgaaggaagccacggccatcctgctggaggccggcgtgatccgcaaggcacctgaagactatgcagcaaccttcgatgcaagcttcgtcaagtaaggccctgccgcaggtgcagccgctggctgcatcagcgcctgccgtttcatccaagaccgtggcgaacacgcggcgccgcgtgttcgcgccgctcgaacccatcggtgcgcgctcgcgcgtgctgctggggctcggcttcttcgtcgtgttcgtgctggcgtgggccatggccacgctcggcggtttcgtgtcgccgaccttcctcgccagcccgccgaccatggtcaaggaaggctggctgctcttcaccgagtacggcttcatcggcgatatcggcatgaccgtgtggcgcgtgttcggcggcttcctgctggccgcggtgttcgccgtgccgctgggcattgcgatgggcacgtggaaaacggtcgaggccttcttcgagcccttcgtctcgttctgccgctacctgccggcgtccgcgttcattccgctgctcatcctgtgggcgggcctgggcgaaatgcagaagctgctggtgatcttcatcggctcgttcttccagatcgtgctgatggtggccgtgaccgtgggcggcgcgcggcgcgacctcgtcgaggcggcctacacgctgggcgccaagagccgcggcatcgtggcgcgcgtgctcattccgggtgccgcgcccggcattgccgaaacgctgcggctggtgctcggctgggcctggacctacgtgatcgtggcggagctcatcggttcctcgtcgggcatcggccacatgatcaccgacagccaggcgctcctgaacaccgggcagatcatcttcgggatcatcgtgatcggcgtcatcggcctcgtgtccgacttcgctttcaaggcgctcaaccgccgcctctttgcatgggcggccctgtgatgacgaacaacaaccagctgtccattcaaggcgtctcgcgcgtcttcaccggcaccaagggacagagcacgcaggcgctgctgcccatcgacttcgaggtgaaggagaacgacttcgtcaccatcctcggcccctcgggctgcggcaagtcgacgctgctgcgcatcgtcgcggggctcgactttccgaccaccggccaggtgctgctcgacggcgagcgcatcgatggcccgggcgccgaccgcggcgtggtgttccagagctacacgctctttccgtggctcacggtggcgcagaacatccgcttcggcctgcgcgagcgcggcatgagcgaggccgaccagaaggagcgcagccagttcttcattgccaaggtgggcctgcgcggcttcgagaaccacttcccgaagcagctatcgggcggcatgcagcagcgcaccgcgattgcgcgcgcgctcgccaacgaccccaagatgctgctgctggacgagcccttcggcgcgctggacaaccagacccgcgtgctgatgcaggagctgctgctcggcatctgggaatcggcgcgcaagacggtgctgttcgtcacgcacgacatcgacgaggcgatcttcatggccaaccgcgtggcggtgttcagcgcgcggcccggccgcatcaagaccgagatcgcagtcgactttccgcatccgcgcagctacaccatcaagacctcgccggaattcatggacatcaaggcgcggttgacggaagagattcgcgcggagtcgatggctgctgtggagcactaggatgaaggccgggttttcaattcatcgcgggttgcgtttggcgcgttgttcggagcgctgctgttcagggcgcgcacccgccgacggggtaccttgctccgcgaatgtcccccggcctgcggcctcctcctttatttcgctgcgcaaggcaccccatcagcgggagcgttatacggagcagtcgttgatcggcggaacactcagagcgtgccccagtgcacagggcatcgggtgctccccgcagcgaaataaaggaggaggcgaagccgggggacattcgcggaggggagtacccggtggcctgtgcacacgcccagaacaacagcgcccagaacaacagcgcccagaacaaaagcaccatcgcgttggaaacctgacatgaaacgcgacctgcccaccctcgccctctacgcgcaagtcaaggatcacatctcccgcaagatccaggacggcacctggccgcccggccaccgcctgccttccgagagtgagctggtcacgcaattcggcatttcgcggatgacggtgaaccgcgcgctgcgcgagctcatggagcagggccgcatcgtgcgcacggccggcgtcggcagcttcgtggccgagaacaaaccgcagtccacgctgctgcagattgccaacatcgcgagcgaaatccgccaacgcgggcacgactaccgctgcgagatgctcgcggtcgaacgactgtccgcctcgcccgacgtcgcggcctggctcgacatgcgcgcgggcacctcggtgttccacagcgtctgcctgcacctggagaacgacacgccggtgcagctggaagagcgctacgtcaatccgcaggttgtgcccgactacctcgagcaggactttgccgccgtgccgcccagcgagtacctggtgcgcaacgtgcccttcgaccagatcgaacacgtcgtcgatgccgtgctgcccaccgccgaacaggcgagccggctcgcgatggaacccaccgacccgtgcctgctgctcacgcgccgcacctggacacgcaacacgccggtcacctgggtgcgctgcctgcatccggcgtcgcgctacagcctgggcagccgcttcaaagccgacggcaacccgtccttcggttgatttttttgacacggaaaccgaaggttttctctcgcaaccacttgtatagacaggttcacatgccaagcaatcacacaaccgccacactgaccctcacgcccggcaaggtggacctcgcgatgctgcgccgcatccaggccggtggcgtgcagctggcgctcgacccctcggtgcaagatggcatggcccgcgccgaagcggcggtgcgccacatcgtcgacaacgaccaggtggtgtacggcatcaacaccggcttcggcaagcttgcgagcacgcgcatcggcaacgaccatttggccgagctgcagcgcaacctcgtgctctcgcacagcgtgggcaccggcgaggcgctgcccgcgcccgtcgtgcgcatggtgctggccaccaaggccgtgagcctggcgcgcggccactcgggcgtgcggcccgcgctggtcgatgcgctgctggctttgttcaatgcgggcgtcatgccgcgcattccgtgcaagggctcggtcggcgcttcgggcgaccttgcgccgcttgcccacatggcctgcgtgctgatcggcgagggcgaagcgaccacggccgacggcacggtggtcagcggcgccgaggccatgcgcctcgtcggcctggagccattcgtgctcggtcctaaagagggcttggcgctgctcaacggcacacaggtgtcgaccgcgctcgcgctcgcagggctgttcggcgccgaggatgtgttcgcctcggccttgatgtcgggtgcgctctcgctcgaagccatccagggttcgatcaagcctttcgatgcgcgcattcacgcggcacgcggccagccgggacagatcgcggtggccggtgccgtgcgcacgctgctcgaaggcagcgagatcgtgccgtcgcatgccgactgcggccgcgtgcaagacccatattcggtgcgctgcatcccgcaggtgatgggcgcctgcctcgacaacctcgcgcatgccgcacgcgtgctggtgatcgaagccaacgccgcgtcggacaacccgctggtgttctgcgacaccggcgaggtgatttcgggcggcaacttccacgccgagccggtcgccttcgcggccgacatcatcgcgctggccgtgagcgaagtcggcgccatcgccgagcgccgcatcgcgctcctgctcgacaccggcctctcgggactgccgccgttcctggtgcacgacggtggcctcaactcgggcttcatgatcgcgcaggtcacggccgcggcgcttgcgtcggaaaacaaatcgctcgcgcatcccgccagcgtcgacagcctgccgacctcggccaaccaggaagaccatgtgtcgatggccaccttcgcggcgcgccgcctgggcgacatggtcaacaacacggcggtcgtcgtcggcatcgaagccatggccgccgcgcagggcatcgaattgaagcgtggcctcaagagctcgccgctggtcgaagccgaattcgccgccatccgccggaaggtcgcttttctcgaacgcgaccgctacctcgcgcccgacatcgaagccatgcgccagtgggcgctgaaggccgaactgccggccgcgctgctgaacatcctgcccagccattcgtaagaaccgacatcccgattgaggagaaccacgccatgaacgctccggaaaaattcgccgccctgaacagccctgatgccgccgatccgcgccacgaccccacgcgcgtgatccgcgctccgcgcggcagcacgctcaactgcaagagctggctcaccgaggcgccgttccgcatgctgcagaacaacctcgacgccgaggtggccgagcgcccgcaagacctcgtggtgtacggcggcatcggccgtgccgcgcgcaactgggcctgctacgaccagatccttgcgtcgctgaaggaactcaacgacgacgagaccctgctcattcaatcgggcaagccggtgggcgtgttcaagacgcacgagaacgcgccgcgcgtgctgcttgccaattcgaacctcgtaccgaaatgggccaactgggagcacttcaacgagctcgaccgccagggcctcttcatgtatggccagatgacggctggcagctggatctacatcggcagccaaggcatcgtgcagggcaccttcgagacttttgtcgaagccgggcgccagcactacggcaacagcctcgcgggcaagtggatcctcacggccggccttggcggcatgggcggcgcgcagccgctcgcggccacgctcgcgggcgcggtgtcgctcaacatcgagtgccagcagaccagcatcgactttcgcctgcgcacgcgctatgtcgacaagcaggcacgcgacatcgaccatgcgctcgaactcatccagcagcactgcgacgcgaaggaagccgtgtcgatcgcgttgctcggcaatgcagccgacatcctgcccgaactcgtgaagcgcgcgaaggccggcggcatcaagcccgacctcgtgaccgaccagacttccgcgcacgacctgatcaacggctacctgccctcgggctggaccgtgccgcaatggcaggccgcgatgaaggatgcctcgcagcacgacgcgctgaaggccgccgccgccaagtcgtgcgccgtgcacgtgcaggccatgctcgacttccaggccatgggcattcccacggtcgactacggcaacaacatccgccaggtcgctttcgacgagggcgtgaagaacgcgttcgactttccgggcttcgtgccggcctacatccgcccgctgttctgcgaaggcaagggcccgttccgctgggtggcgctgtcgggtgaccccgaagacatctacaagaccgacgccaagatcaaggagctgttccccgagaacacccacacgcaccgctggctcgacatggcgcgtgagcgcattgcctttcagggcctgcccgcgcgcatctgctggctcggcctgggcgagcgccacatcgccggcctggccttcaacgagatggtgaagaacggcgaactcaaggcgccgatcgtcatcggccgcgaccacttggacaccggctcggtcgccagccccaaccgcgagaccgaagccatgaaggacggcaccgatgccgtcagcgactggccgctgctcaacgcgctgctcaacaccgcgggcggcgccacctgggtgagcctgcaccatggcggcggggtcggcatgggctactcgcagcactcgggcgtggtcatcgtctgcgacggcaccgatgccgccgccaaacgcatcgagcgcgtgctgtggaacgacccggccaccggcgtcatgcgccatgccgatgcgggctacgacattgccgtggccaccgcgaagaagcaggggctgaatctgccgatggtgcgctgactgactgaccgtccgctgaagcggtaagacgaaggtagaaagaaaaagcgcgctcattcccactcagtgggaatcaaggcttggacgtgggaacggcgggcaagatactgcaggccgcatccactttcgacacccgcgattgcccccgatgacgacgccgacgcccgaagcttccgcctacaacgaccgtgccttgctggtgctgtcggtgctggcgcaaagcaaggtggcaatgtcggcggcggagctgatgcaggccacggggctctcgcagagcacgctgtaccggcagatcgcgatgctgcggcgctggggcttcgtgatggagtccgacgggcgctattcgcccggcccggtgagcgtgcagctcgcgagcggcttcgacggcaactccgacctcgtgatggcggcgcgcgccgacatgcgcgcgctcgcacagcagagccatgaaagcgtggcgctggtcacagccgtgaacgaccgcgtggtgtgcctcgagatgatcgacagcgagcagtcgctgcgctgttcgttcgaccggggccgcagcgtgccggcgcgcgacggcgccagcgccaagtgcctgctggcccacatgccgaccgaccagcgcgatgccttgctcggcgccttcggcgaaagccccgggcggcgcgccgaacgtgccgccgagctcgatgccatccgcgaagccggccatgccgtgacgcatggccaggtcgatgccggcgtctggggcgccagcgcaccggtgctggccgcgggccggcgcctgcgcggcgcgatcacgctcatggcgccgctcacgcgcgtcgaaggcatggaagctgcattgctccacatgaccgtcgtcacggcggcccgcatttcccgcgctctgcagtaggcatcgctgcacctttctttttcaacccacgaaagccttcgcatgaacacccgccgcaccctcatcgccgccgcactctcgagcctcgccttcttcggctttgccaccaccgcgcaagcccagggcgagccgctgcgcgtggccaccgatgccacctttccgccgatggaatacgtggagaacggcaagcgcacgggcttcgacgtggaactggtggaggccatcggcaagacgctgggccgcaagatcgagtggatcgacatcgacttcaagggcctcgtgccgggccttatctccaagcgcttcgacatggccgtgtcggccatctacatcaccgacgagcgcaagaaggtcgtcgacttcaccgtgccgtactatgcgggcggcctggtcgtgatggtgaaggacggcaacacggccatcaagacgccggccgacatcaacggcaagaaggtcagcgtgcaggtgggcaccaagtcggtcgcctacaccaaggaaaaattcccgcaggtgcagctgatggaggtcgagaagaaccaggagatgttcaacctcgtcgacatcggccgcgccgacgccgccgtgaccggcaagcccgcggcctaccagtacgtgcgcacgcgcggcggcctcaaggtcctgccggagcagatcaccaccgaggaatacggcatggccattcgcaaggacacgcccgaactcaccaaggccgtgaatggcgccatcgagaagctcaaggccgacggcacctacgcgcagatcgtcgccaagtggttcaagtaatgtcggccccccggcttttcacgcgctgcgcgcgtgtaactccaccccccatgggggaggcgcggccggcttggggcggcccggcgctcggccgccgaagaggttgacccatggatttcgacttctcgccggtctggcagggctggcctgacctgctgcgcggtgcgctcgtcacggtggaaatcaccgcctgcgcgctcgcgctcggctgcgtgctgggcctcttggtcggcatcggccggctcaacccgaagcggcgctggctctatggcgtgtgcacggcctacgtggcggcgattcgcggcacgccgctgctggtgcaattgttcatcctgttcttcggcctgccgcatttcggcatcctgctgccggccttcttgtgcggtgtgctggggctgggcgtttactcgggcgcctacgtgtcggagatcgtgcgcggcgcgatccagtcgatcgacaagggccagaccatggccgcgcagtcgctgggcatgacgcccggcacggcgatgcgcgagatcgtgctgccgcaggcggtggtgcgcatgattccgccgctgggcaacgagttcatcgcgctcatcaagaactcggcgctggtgtcgctgctcacgatccatgacgtgatgcacgaggggcagaagatcatcagcgtgtcgtaccgttcgctggaggtctacctggccattgcgctcgtgtacttcgtgctcacggggacgatgacgctggttctcaggcacttcgagcagaagctgcggcagggcgggttgatgcgatgagcggcgccgctgcgtttgaatttctccctcccctcccgggggagggtcggggtgggggcacgacggcctcgagccttgctcggcgctcattggacgctgcccccatcccagccttcccccagagggggaaggagcaagaggatctctcatgaaccacgtgcatcgcttctcgcgtgccgcgctgccggccaccccctggaagaacggcggcggcaccacgcaggaaatcgtcagctggccccgaggcgcggggctcgaaagcttcggctggcgcgcgagcattgcgaccatcgcggcggccggcccgttctcggtgttcgcgggcgtcgaccgcagcatcatgctgctagaaggcgacggcgtgcggctctacacgcaagacgggcgagtggaccacgcgctcgacgtgccgcatcggccgttcgcgttcagcggcgacgacgcgatcgactgtgcgctgctgggcggcgcatcgtcgaacgacttcaacatcatgacgcggcgcggcgaatggcgcgccgacgtgcgggtgctcgcgcacgcatcggccatcgagcccgcgccgcacggcgtgctgcttgcgcttcgcggcgcatggcggctgaacggcgaggcctgcgccgagggtgaaggcctctgctggaccgacggcgcgcaggcgtggcaggccgtgcccgagggtgaaggcgctcggctggctgcggttcgcatcgtgccggcgtaagctgtggaaaccggaaaacgaaccatgacatccgcacactcatttccatcggccgacggcctctggaccggcctgcgcctggcgcccggtgccgcgcccgacgccgcattgccagccgatgccgaagccgcgatcgcggtcacggagggcgcgatccgctgggtcggcgcccgcaatgcgctgcccgccgagttcgcttctctcgcgccgcacgacggcggcggcgcgctcgtcacgccgggcctggtcgattgccacacgcacctggtctacggcggtcagcgcgccaacgagttcgcgatgcggcttgccggcgccacctacgaagaagtggcaaaagccggcggcggcatcgtctcgtcggtgcgcgccacgcgtgaagccgacgaagacacgctcttcagagaggccgcgccgcgcctcgaacagctgctggccgatggcgtgtgcgccatcgagatcaagtcgggctacggcctttcgctcgaacacgaacgcaagcagctgcgcgtggcgcggcgcctgggcaaggcctatggcgtcaccgagcgcaccaccttcctcggcgcgcatgcgctgccacccgaatacgcgggccgcagcggcgactacatcgacctcgtctgcaaccagatgctgcccgcgctcgcggccgaagggctggtcgatgcagtggacgtgttctgcgaacgcatcgccttttcgctcgaggaaaccgagcaggtcttcaaggccgcgaagtcgctcggcctgccggtcaagctgcatgcggagcagctttccgacatgggcggcgccgcgctggccgcgcgctacggcgcgctctcgtgcgaccacatcgagcacctgtcggccgaaggcatcgaggccatgcgccagtcgggcaccgtggccgtgctgctgcccggcgcctactacacgctgcgcgacacgcacctgccgcccatcgaggcgctgcgcgccgccggcgtgccgatggccgtgtcgaccgatcacaaccccggcacctcgccggcgctgagcctgctcttgatgatgaacatggcgtgcacgctgttccgcctcaccgtgcccgaggcgctggccggcgtcacggtgcatgcggcgcgcgcgctgggcctgtcctccacgcatggcgtgatcgccgaaggcatgcccgccaacttcgtgctctggaatgtgcgcgatgcggccgagctcgcctactggttcggccagcggcccgtgcgcagcgtcgtgcggcggggccgcatcgccgtcggagccgccgaatgacgcaaacgcttttcgcggccgatgcattgctgcccgatggctgggcgaagaacgtcctgctgtcttggaacgacgctggccagctcacgcaggtgcagtccgcggtgcagcctgccgccggcgcgcaagcggcgaacggccccgtgattcccggcatgcccaacctgcattcgcacgctttccagcgcgcctttgcgggcctcacggaacatcgcgcggagcagcaagacagtttctggagctggcgcacgctgatgtaccgctttgccgcacgcctcggcccgcagcacatggaggccatcgccacctggctctatgccgagatgctcgaggcgggctacaccagcgtgtgcgagttccagtacgtgcaccacgatgccgacggccgcccctatgccgacgatgcgaccttgagcctcgcgctgctgcgcgccgcgcaaaatgtgggcatcggcttcacgctgctgcccgtgctctaccagaccagcggcttcggcggcctgccgccgaatgaagggcagcgccgcttcatccgctcgaccgattcgatgctgcgcctgctcgacacgctgaagcccgcgtgcgatgcggcgggcgcgcggctcggcctggcgccgcactcgctgcgcgccgtgccgcccgatgcgctgcgcgaggctgtcgcggggcttgaagccatcgaccgcagcgcgcccattcacatccacattgccgagcagaccaaggaagtcgacgactgcgtggcctggagcgggcagcgtccggtggcctggctgctggaccacgcgccggtcgatgcgcgctggtgcctggtgcatgccacgcacatggatgcggccgaatacgcacgcggcgcgaagagcggcgcggtcgccggcctgtgcccgaccactgaagcgaatcttggcgacggcatcttcgatttcccggcatggcgccaccatggcggggcctggggcgtggggtccgacagccatgccacggtcaacgcggcggaagagttgctgatgctcgaatacagccagcgcctgggcaagcggcagcgcaacgtcggcgccagcgcggcagagccgcacgtggccaccgcgctcacgctcgaagcggtgcgcggcggcgcgcaggcatcgggccgggccatcggcggcctggccgcggggcagcaggccgacttcgtcgtgctcgatgccgcgcagcttgcgctgcagggcctcggcgcgcccgacatgctgtcgtcgcacgtcttcgccagccaccgcacgtcggccatcgatgcggtctgggtgtccggccggccgcgcgtcgcggcgggccgccacgcattgcaccaagaggccgccgccgctttcgtcgccgcgcgcagccagcttcttctggaaaattgagcccatgagtttcaccaccaccgaacctgcattccgctttcgccagggcacccgtcccttgctgatctcgatgccgcatgtcggcacccatgtgccgcccgcgctcgccgcccgcttcacggaagaggcgcgccacgtgcccgacaccgactggcacctcgagcggctctacgactttgccgacgaactcggcgcctcggtgctcgttgccacgcattcgcgctacgtgatcgacctgaaccgcccgccggacggcgcgagcctctacccgggccagagcgtcaccggcctgtgcccggtcgacactttcgacgacacgcccgtctacgcatccagcgacgacctgccgaacgacgcagaagtcgccgcgcgacgcgacgcgatctggcggccctaccaccagcagctgcaggccgaactcgaccgcctgaaggccgcgcacggcaccatcgcgctgtgggacgcgcactcgatccgctcggtgctgccgcgcttcttcgagggcaagctgcccgacctgaacctgggcaccggcaacggcacgagctgcgacccggcgctggctgccacgctgctcagcattgccgaatcggccgctggctacaccggcgtgctcaacggccgcttcaagggcggccacatcacgcgccagtacggcaacccccccgccggcgtgcatgcggtgcagctggagatgacgcagtcgagctacatgcaggagacgctgcccttcgactacctgcctgatgtggcggccggcgtgcagccgcatgtgcggcgcatgatcgaagcggtgctggccttcgtcgaaagccgttaaagcaccgacggcggccagggacagcacccgcttcctacaatcaggggctatgaagcccgtcatctacacccgcggccaggcactcgccggcatcctcgaaaagcgcatcgccatcctcgacggtgcgatgggcacgatgatccagcgcttcaagctcaccgaagagcagtaccgcggcgagcgcttcaaggacttcgagcgcgacgtgaagggcaacaacgagctgctgtcgctcacgcggcccgacgtgatccgcgacatccacgagggctacctcgcagccggcgcagacctgatcgagaccaacaccttcggcgcgaccaccatcgcgcaggaggactacaagatggcgcatcttgcgcgcgagatgaacctcgaatcggccaagctcgcacgcgcggcctgcgacaagttcagcacgccggacaagccgcgcttcgtggccggcgccctgggcccgacgcccaagaccgcgagcatcagccccgacgtgaacgacccgggtgcgcgcaacgtcgatttcgagcagctgcgcgcggcctactacgaccagaccgaggcgctggtcgaaggcggtgccgacgtgatcctggtcgagacgatcttcgacacgctcaacgccaaggccgcgctgttcgcggtggacgagtatttcgacaacagcggccagcgcctgccgctgatcatcagcggcaccgtgaccgacgcgtccggccgcatcctgagcggccagacagtgaccgccttctggcacagcgtgcgccatgcgcagccgctggccattggccttaactgcgcgctgggcgcggcgctgatgcgcccgtacatccaggagctggcgaaggtggcgggcgacaccttcatcagctgctacccgaacgccggcctgcccaatccgatgagcgagaccggcttcgacgagacgcccgacgtcacctcgcggctgctgcacgagttcgcggccgaagggctggtgaacatcgtcggtggctgctgcggcaccacgccggaccacatcgcggccatcggcaaggccgtggcgccggtgccgggacggctgttgaacagcaacgctcgcttctaccgcgaagcagcgtaactggctcgcccccagtcttcgcgcacttcgtgtcgctacgccaaccccctgccgggggcaacaccagcggcccggcggagccggttccgcggtgtttcacgaaggggacactggcgctgtcgcgccctcggctgattgacggcattcgggctgccgcctaggctggctgcgcaaaggaagcccatcatgaacaacaaactccccatgcgctggatcggcatcggcgccatcgccttggccttgccgcttgcggcctcggcgcagcaggccctcacgcgcggcgccgtcaacctgcgggccggcccctctggcgactatccgctggtggcgcggctggcgccgggccagccgctcgacgtgatcggctgcaccgggggctacagctggtgcgacgtggtgctgcccgacggcggacgtggctgggtctgggccaggagcctcgactacgcctaccaggagcggcgcgtaccgctggcgacctatggcgcggtgatcggcgtgccgatcgtgaccttcgtgatcggcagctactgggcggactactaccgcgaccggccctggtatggcgaaaggcgctggtggggcggccggccgccgcctccgccggtgcccggttggcagccgccgccgcccgtgcgtccggcctggcagcccaagccgtggccgggaccgggcttcaaaccccagccggcgcccggcgtccggccgcaacccggtcccggctaccgcgcgccgcatccgggcccaggctaccgtccgcctgcggaccccggcttcaagccgccccggccccagccggcaatccggcccggaccaccgcccggccaaccgcaaatgcatcagggcggcgggcggcctgatggcggcggaggcgggcgcaagcagcgcggcgatgaaggcggcggcaagggtggcggccatgggggaggccacggtggcggcggaggcaagggcggcggccacggccatcgcgactagctaaccaggagccgcaaggcccgccgcggcctggcgatcgcgcgcaatcagcgccacgaagcgctgcgcccccaggcccagcggccgctcccgcgaccacaccacgtcgacccacaggtccagcccgttgctgaggttctcgaacgggatctcgaccagcgcgccggcggccacgtggggcttggcaaagttgcgcggcagccagccccagcccaggccggcggtgatcaggctcagcgcggccagcgcgttgtcggtgcgccagacatggcgcgcgaacacgaagcgcgggtcgctcgtcgcaaggtcgcgccctgccaccacgatctgccgggtgttcgtgaggtgctcttcgcgcaggcgctcgccggcggccgccagcagcacggggtggttgggcgccatcacggccaccatggtgtcgctgcccacttcctggaaaccttcgcggccgtcgaggctcgggcgctcgaacaccagcgccagctgcgcgcggccgctgtgcagcagcgccagcgcatcggcctggggggcggccagcacctcgacctgcagcagcggatattcctcggccaatgcggccagcggtccgctccagggtgcggccagcagctcgggcgcaatcgccagcgtgaggcggttttcgagcccctgggtaagcgccagggcctgaacctgcaattgcttgagctgggccgccaggagccgcgcctgcggctccagcgaacgggcggcggcggtcggctgcggctcgcggccactgcggtcgaacaggggcagggccagttcggcctcgaggttggcaatggccatgctcacggccgacggcaccttgcgcagcgcgcgcgccgcggccgaaaaggagccgtggtcgatcacggccaggaagacttcgacgttgtcgctggagaaggccatgagcgcccaatctatcaataaaactgaaacaagttaactttttatatcagtaaacagcaaataaagtccagccattgccttttgaaccgccggagaacagagccatgcaggggtttcagcgtcgagtcgtttacatcaccctttacgaagggatcgccatcgtggccgccagtgccggcctggcgctgatgacggacgccgggctcgggcattccggtgtgctggcggtggccgcctcggtcatcgcggtgatctggaacctagttttcaatgccttgttcgagcgctgggagtcgcgccaggcggtgggcgggcgcagcgtgcgccggcgcgttgcgcatgccatcggcttcgagggcgggctgatcgccttcctggtgccgctctttgcctggggcttgggcgtgtcgctctggcaggcgctggtgatggacctgggactggtggtgttcttcctggtctacaccttcgtcttcaactgggccttcgaccgggtgttcgggctgccggcttcggccgcgccccggaggccagcgtccgtggccgggcagggggcctgaacatccctcagggccgcggcccttgccgcagccggtaaaattgcgctcccttccaaggagcgttgcagcggcggcccaagtcaacaggcccgccgtcaggcttggaaggcgccccgtccgccggggcgcaagccgcaaacgacgctcacctgacgttttttcctgcacaggtgagccccccaatgagcgatgttcccacgccctccgttccaccgatgaagctgtccggcctcgagccggtggccatcgatgccggatcgctgttcgtcaacatcggcgagcgcaccaacgtcaccggttccaaggctttcgcgcgaatgatcctgaacggccagttcgaagaggccctggccgtggcgcgccagcaggtcgagaacggcgcgcaggtgatcgacatcaacatggacgaggccatgctcgacagcaaggccgcgatggtccgcttcctgaacctgattgcgagcgagcccgacatcgcgcgcgtgccggtgatggtcgacagctccaagtgggaggtcatcgaggcgggcctgcgctgcatccagggcaagggcatcgtcaactccatctccatgaaggagggggtcgacaagttcaagcacgaggccaagctcgtgaggcgctatggcgccgccgcggtggtcatggccttcgacgagaagggccaggccgacacctacgagcgcaagatcgagatctgcgagcgggcctaccgcatcctggtggacgaggtgggctttccgcccgaggacatcatcttcgaccccaacatcttcgcgattgccaccggcatcgaggagcacgacaactacgcggtcgacttcatcaacgcggtgcgctggatcaagcagaacctgccgggcgccaaggtgtcgggcggcgtgagcaacgtgagcttcagcttccgcggcaacgacccggtgcgcgaagccatccacaccgtgtttctgtaccacgcgatcaaggcgggcatggacatgggcatcgtcaacgccggcatggtcggcgtgtatgacgacctcgagccgaccctgcgcgagcgcgtcgaagacgtggtgctcaaccgccgctccgatgctggcgagcgcctcgtcgaagtggccgaaaccgccaagagcggcgccaaggacgacagcaagaagctcgaatggcgcggcacgccggagcatccggtgcacgtcaaccagcgcctgtcgcacgccatggtgcacggcatcaccgacttcatcgtcgaagacaccgaagaggcctaccagcagatccttgccaagggcggccgtccgctgcacgtgatcgaaggaccgctgatggacggcatgaacatcgtgggcgacctgttcggccagggcaagatgttcctgccgcaggtggtgaagtcggcgcgcgtgatgaagtcggccgtggcccacctcattccctacatcgaggaagaaaagcgccaggacgaggccgcgggccgcgacgtgcgcaccaagggcaagatcatcatcgccaccgtgaagggcgacgtgcacgacatcggcaagaacatcgtcaccgtggtgctccagtgcaacaacttcgaagtggtgaacatgggcgtgatggtcccgtgccacgagatcctcgcccgggcgaaggtcgagggcgcggacatcgtgggcctctcgggcctcatcacgccgagcctggaagaaatgcagtacgtggccggcgagatgcagaaggacgaccacttccgcatcaagaagattccgctcctgatcggcggcgccaccaccagccgcgtgcacaccgccgtgaagattgcgccgcactacgaaggcccggtggtctacgtgcccgatgcttcccgcagcgtgagcgtggcgcagtcgctgctgtcggagcaggccaccgcgtacatcgacgagatcaacgccgactacgagaaggtgcgcacgcagcacgccaacaagaagcaggtgccgatgtggccgctggccaaggtgcgcgccaacaagacgccgatcgactggacaaactacacgccgcccgtgcccaagttcatcggccgccgcgtgttcaagaacttcgatttgaccgagctcgccaagtacatcgactggggccccttcttccagacctgggacctcgcgggcccgttcccagccatcctgaaggacgaggtcgtcggcaccgaggccgtgcgcgtgtatgcagacggccagcgcatgctcaagcgcctgatcgaaggccgctggctcagcgccagcggcatcgtcggcttctggcccgccaacacggtgaacgacgacgacatcgagctctacaccgacgagacgcgcagcgaggtcgccatgacctggtacggcatgcgccagcagaccgagaagcaggtgatcgacggcgtgatgcggcccagccgctgcctcgccgatttcgtcgcgccgaaggacagcgggctgaaagactacgtgggcgtgttcgcggtcacggcgggactgggggtcgagaagaaggagaagtacttcatcgacgacctcgacgactactccgccatcatgctcaaggccctggccgaccggctggccgaggcctttgccgagtcgctgcaccaccgcgcgcgcaccgacctctggggctatgcgccggaagagggcctgagcaacgaggagatgattgccgagaaataccgcggcatccgccccgcgcccggctaccccgcctgccccgaccacagcgtgaagcgcccgatgttcgaccttctgggttgcgcggacattggcatgacgctgaccgaaagcctcgctatgatgcccgccgccagcgtgagcggcttctacctgagccatcccgagtcgacgtacttcaatgtcggcaagatcgggcacgatcaattgcaggaccaggcggcgcggcgcaaggagagcgaatccgacctcgagcgcctgctggcgccgaatctttgaacctgccggccggcatggccgaccggcgccgggagttgttattcagaagttgatgtttgccgccgcgcactacgcggcattggctgtctttgtccttgcctgctggggtttcgggcgcgcgctgctggcgcgcctttcgccgccgacccggcgtgacgcctggctcgaagcggcgatggccgcgaccctgggcgtcggcctcttcatctgcgccttccaggtgctggcgatcttcggcgcgttcaagaccggtgcgacggtggcgctgatcgttgccggcgtggtggccgccgccctgcagttgcggccctggtggcgcgacgtccgcacggttcgcgctctggccgtggcgcccgccgcgccatggacccgcgccgacaagatcgcggccatcgcgctgggcctggtggcgctgcccgcgctggttgcgccgctcgcgccacccgccgccttcgacgagctgatgtaccacctgccctatgcgcgacaggtggcgcagcagggctccctgggcatccacgagtggctgcgctacccctggtttccgtacaactacaacctgctctatgccgccgcgctgcaggtgggcgacgacgtgctgccgcattttctcaatgcgctggcgggtgtgctttcgtcggtcatggtcttgcgcctcggcatcaagaacaccaaccggctcacggccttgatcggcacggccatctggatcggcatcggcgactattcgaatgcgctgatcgacatgggcgtggcgctcttcgtgctcggcgcctgcgtggcgctgtggtggtggcgcgaatcgcagccggtgcagggcggcatgcgctggctcggcctggcggcgttctgcctcggcgtggccgcgggttcgaagtaccaggcactcacctttttgccgctggtggcgctgttcgtcgtctggcatgagcgccggcccaaggcctgggcgctggcgctcctctgctttctggttccgtgcgtgtactggtacgcgcgcaacgcggtcatgaccggcgatccgttcaacccgatcggtgcgcgcgtgttcggtttcacggagtggattccggccgactacgtgcagcaggtggccgacgtgcgcgaccatgcggcgcgacccaacgcgctgatctgggccgtgtttttggcgcccttcagcgtgctgtggaagcgctcggccgccgtgcgcgcggcgggctggttctgcttctattcggtggccgtgtggcttctgacctcgcgctacccgcgctatctcacggcgtcgtttccgctgctcgcgctgatggcggccatcggctggcaagtgctgttcggctgggtcgccaccggcgtgcgccgcgtgttcggtggcaagggtgcagcagcggccgcggtcgatgcaggcgccgaggcacctgccgccgcagcacctgccgggcgcctgggccttgccggcgactggatcgtcgtgctgctggtggccgccctggccgcggtgtcgctgaagcagaccgccgtcaaggtggcgatgatttcgcccacgcccgaatcgcgcgaagccttcttgcgccagcacgtgccaggctatgccgccatggactatctgcgccagcatgccaacgggcgcgtctaccaaattgcgctgaacgaggcgatctattacggccccaatccgatctggggcgacacgctcggcccgtggcgctaccgcgatttcctgctgctgcctccgggcgacatggcggtcaagctcgcacagcggggtttcacggccatcgtcatgcccacgtcgatggtgcccacgctcgccacccggcctggcttcgaccagcatttcgccctgctgtacgaaaaagacggcggccgggcctatcgcattctttcgaccgcaccatgaccgacgacaaccaatccgccgcagcccgtgcacccctgcgcatcgcagcggtgatcccctgctacaacgaggcgctgtcgatcgcgcaggtggtcgcgcaattccgcgcggcgctgccggaggccgagatccacgtcttcgacaacaactcgagcgacgacaccgccgccatcgcgcgcgcaagcggcgcattcgtgacgcacgtggcggcggccggcaagggcaacgtcgtgcggcgcatgttcgccgacgtcgaggccgacgtgtacgtcacggtcgacggcgatgccacctacgacgtggccagtgcaccgcggctggtggaaacgctggtgcagggcaacctcgacatggtagtgggctgccgcgtcgacgacgggcggaacgcgctcacctaccgcgccggccaccgcttcggcaaccggatgctcaccggcgccgtggcgcagctttttggcggcggcctgaccgacatgctgtcgggctaccgcgtgttttcgcgccgctatgccaagtcgtttccggccctctcgcacggcttcgagatcgagaccgagctcacggtgcacgcgctcgagctgcgcatgccccatgccgagctcgacaccgcctacagcacgcggcccgagggttcgcacagcaagctctcgacctaccgcgacggctggcgcatcctgcggaccatctgcaagctgttcatcagcgagcggccgctgcagttcttcacgatccttgcggcgctgctcgcggtgggcgcgatcgcgctggtcattccgctgctgatcacctacctgcacaccggcctggtgccccggctccccacggcggtgctggcgaccggcgccatgctggccgcgatgctgtcgatggtctgcggcgtcgtgatgcacgccatccggctcggccgccgcgaggccaagcggctgcgctacctcgcgattcccggcgtgcgccacttcgccggcaaatgaagcttggccgtcagttcctgtcgttcgcggtggtgggcgcgatcggcttcgtggtcgacgtggccgtgctgtacctgatggcgccgctgctgggctggtacggggcgcgggtgctgtcgtttcttgcggcggcaacggccacgtgggcgttgaaccggcgctacaccttccggcgttccgaagcttcggtgctgcgcgagtacctcggctatctggtgacgatgctgggcggtgcagtcgtcaactacggcgcgtatgtgctcgtgctgcattggttcacggggccctgggcgcccgcggccggcgtggcgctgggcagttgcgcggggctggtcgtgaacttcctgtcggcgcgctacctggtgtttcgggcgcggtagatgtggcatgcggcggcgctgcatgtgcgccgctggccctcaccctaaccctctcccggagggagaggggacaacgcggggagctcgttcagtgcgcggccgacaccaccaccggaatttcggtcgccggcggcgtgttgcggctgcggccgcagcgcacgatgccgtcgatcatcaccatgcccacgcccggaatgtcgccgagctgcacgctctccagcaggcctggcgcgggcgaatgctgcgcacggtccatgaagacgaagtcggcgtcgcggcccacctcgatcagcccgcagttgagcttgcggatcttcgcggtgttgccggtggcaaagcagaacaccagctccgccgggatgttggcgatggacgacagcatggccaccatgcgcaggatgcccagcggctgcacgcccgagccggccgggccgtcggtgccgaggatcacgcggtgcgggcacttgagttcgagcgcggccttggctgccgcgatggcgaccttctcgttgccgttgtgcacgatctcgatggcgcgcgagctcttctcgcacagctcgcacacatgcgcctcgggcagcgaagtgtggccgccgttgatgtggccgatgatgtcggcgtcggcttccagcaccacgtccttgtcgatcaggccggagcccggaatcgaaggcccaccggtgtggatggtgctctggatgccgtacttgcgcgcccaggcgaccatttccttggcttcgtagccggccttcaccgagcccaggcccacttcgccgagcaggcccacgccggcttcggcgagttccttgaagtcgctctcgaccatgcccttctcgatgaccggtgcgcccgccagcaccttcacgccgccggggcggaagttgtcgaacgcgcgctgcgcggtgatggccaacgccttcaggcccacgatgtccttcggccggcccggcaggtgcacttcgcccgcggaaatcatggtggtcacgccgccgtgcatggtggagtcgatccagccgatctggccctggcgcggcgtccagtcgccgaacaccgggtgcacgtggctgtcgatcaggcccggcgccacgcaggtctgcttcgcgtcgatgacggtcttcgcgccttcgaggtcgcagtctttttccttgccgaccgcaacgatcaggccgtcgttcaccacgatggtgtcggcgtcgaggatgggcttgtcgatgttgcccgagagcaagagcccgatgttctttatgacgactttgcccgacttgccgccggctgcgatttctgccatttcgtgtggtcctggtcgtgggggagggtgttgttgtcttgcggctcgtctgcgcgcacggtgcgcagcacggtctcgatcacgaagtcttcccagtgcgtgatcgcctcgggcgattccagcggctcgccgagaaaggccgtgagcgtgtgccggttcgaggtgtagaagtagccggtggacgcaatcagcaggtagatgtcgcgcgcgatcagttcgcggcggaacaggccctgcgccgcgccgctcgccaggatctcggcaatgatggccaccgcccgcgacgagtattcacgcgcccgcagcgacttggagatgtggcggcccttgtgcaggttctcggtgttcaggagcgtgacgaactcggggttcttgcggtagtagcccagcacgaagcggatgacctcggtgagcgcctccacgggccgcgaggcgtcgagcgcaatggcggcctcggcgtcgtccatgcgcttgtagatgccttcgagcaccgcgatgaagaggccttccttgctgccgaagtagtagtagatcatccggtcgtacgacttggccgccttggagatcttctccacgctgccgccgtcgtagccgtacttggcgaacaccttggtcgccgacttcaggatgctgtcgcgcgtggcctgcgccgcggcctcgcgcacgccggtgcggcgctggggcttggttgcagcaggcttgcgttccattaccggcggtcgccgccgggccgccccaaggcggaccgcgcctccccctcggggggtggagttacacgagcgaagcgagtgaaaagccggggggcgaacattacttttccgcgaacgcgcgttcgaccacgaaatcgcctggcgtgctcgtgttgccttccttgaagccgcgcccttcgaggatgtgcttcaggtccaccagcaggccggggctgccgcacagcatcacgcggtcttccaccgggttgatcggaggcaggccgaggtcgtccgtgagcttgttggtcgagatcaggtcggtgatgcggccctggttgcggaactcctcgcgcgtgaccgtcgggtagtagagcagctgcttctcgaccatctcgccgaggaattcgtgcttgggcaggtggtcggtcacgaggtcgtgataggccagctcgtcgacctggcgcacgccgtgcaccaggatgacctgctcgaacttctcgtaggtgtccgggtcgcggatgatgctcatgaacggtgcgagccccgtgcccgtgccgaacaggtacaggcgcttgcccggcagcgtgtagtcgatcagcagcgtgccggtgggcttgcggcccacgatgatggtgtcgcctacctggatgtgttgcagcttcgaggtgagcgggccttcttccaccttgatgctcaggaactcgagatgctcctcgtagttcgggctcacgatgctgtaggcgcgcaacaggggcttgttgttgaccttcaggccgatcatcgtgaaatgaccgttggagaagcgcagcgccgggtcgcgcgtggtggtgaaggtgaacaggcggtcggtccagtggtggacgctcaggacgcgttcttcgctgaatgcactcatacggaactcaagagttggttgaacagtgggaagctggctgggccgaaatgcacgcccctggggcacgagccttcggacggctgcgaaccctccattgtcgttggtcggaaaaacccccgatggataccgcgagaaaacaccattgcaagcatcgggcctgtttgctacattgaccgcgaatgtagtgaacgcaacatgaaagtgtagggaatgctacacaaacggaaggcggtgcacaagcgggcagacggcacgtttgttgcaacccttcgcagaccgagattcccgacgccgacccgcaaccacacgcccacgagaccgccccgatgacagaacacaccaagacagacggactgcccggcatggacatgccgctggttgcagatgccggcggcagcgccttcggcaaggcgccgccgcgcaacgagcgcatgagcaccgccaaggtcgagtgcaacgcctgtccggtgctgtgccagatctccgacggccgcaccggtgcctgcgaccgctatgccaacagggagggcgtgctggtgcgcgtcgatcccgtgatcctgctgcgccgcgagattgcgagcgaggccccggtgctggtgcccttcgaccggccggccgcggagaaggccgaagccggcgcgcccgactggagcggcgacctgctgcacgccgacgaagtcttcgtgaccggcgtgggctcgtccaccacctaccccgactacaagccggccccattcatcgtggcgtcgaaagcccagggcgtcgacatggtcaccgtcgtcaccgaaggcatcttcagctactgcagcttcaaggtgaagatcgacaccgaccgcttcctcggctccgagcaggccaacgtgcgctaccgcggcgaagtggtcggccacgtcaccacggccgagtacggctcgcagatgctctcgctcggcggcgtgcaccacctcaccggtggcagcaagaaggaaggccgcatgacggccgagctgatgcagctcctgggcaacaagaaggcggtggagtgcaccatcgacggcggctccaccctcgtcatccaggccggcaaggcacccatcgtcaatggcgtggaagagcagcgcatgcgcgtgggctgcggctcggcggcggtgggcatcttcgcgcgccagttcgcgggcgtggccgacgaagtggtggtggtcgacgaccacatcaccggcgtgctcaccgagcaccaggccgggcgctgcctcgacatggcaccttcgggcatccagatgctggggcgcaagtccacgccggggcgctacttccaggtggcgaacccgggcaacggctggggcggcaccgacatcgccgatccgctctcgatcatcgagggctgggaagaaggcgtggcgcgccccggcctgcgcctcctgatgacatcgaccaccggcgagcacgcgcagtggtatgtgctcgatgacgcattgaagcccgtggagcaacctatgcccgccgaagtgcgccgcatcgtcgagcgcatcggcgagaactgcgaaccgtcactgtgcaccgtgctgttcctcggcggtgcgggcgggtccttgcgcgccggcgtgaccgaaaaccccgtgctgctgacgcgcgccatcaagcgcgcgctcgtcaacgtgacctgcggcggcgcgccggcctatgtgtggcccggcggcggcatcaccgtgatggccgacgtcatgcgcatgcccgacaacagctttggcaccgtgcccacgccggccatcgtggcgcccatcgagttcagcatgcggcgcgatgactacgaggcgctcggcggccacatggaacacgtcttctcgctcgagcaggcgcttgcgcgcggcgcgtggcaggaagacggcgctcccttggcgcgccagtgggtcgtcatggacgatgccaatccgtggccgctcggccacccacccatgctgggctgaaccatgaccgcccaacgcgccgcgctcgacaagaaccgctggcacttcaaccacggcccgatcgacatcgtggccgaggcgcatggcgacccgtacgccgttgccgccgcgcacgacgcggcatgggcgcgcttcggccatgtgctggtcgaactggtgcgagagttgccgctgctgcgcctgcccgccagcgacaacatgcgcccgcgcggcgttgtcggccggcgcatgtgggacgcctgcgccgcgttttcgccgatgttcatcacgcccatggcggccgtggccggttcggtggcgcaggagctgatcgcgttctacgatcgccccggcatcgagcgcgcctggatcaacaacggcggtgacattgcgctgcacctcgcgccggggcagtcggcgcgcgtgggtgtctatgccgacctggcgcgcttcgactggcagggcaccggcattctcacgaccgacggccagttcgaaatcagggccgagcagccggtgcgcggcgttgccaccagcggctggcgcggccgcagtttctcgcttggcattgccgacagcgtgaccgtgctcgcagccaccgcggcagcagccgacgccgccgccacggtgattgccaatgccgttgacgtggacgatgctgccatccagcggcgcccggccagcgagtgcaaggacgacagcgacctgggcgacatcctggtcacggtcgacgtgccgtcgctggcaccttcgcaggtgaaaagcgcgctcgacaccggcgccgtttgcgccaaggtgctgcagaaaggggggctcgtctgggctgccttgctcgtttgccagggtcagtggcgacttgttgaacccttatgctcgaaggcgctgccaaaatcgccatccggtgcagttggttcagtatttgcttaacgaaagcaaggttctttttcatgatcgatatacgtcgcgtcttcacccatgtcgagcacatccaccacgagttcgggccgcgcgccaagactccgctggtgcgcggtgccatcggcgcggtgctgaccaatccgttcgcgggccgctatgaacccgacatcctgccgatgatggcgctgctcgaccccgtgggcgtcgacatggcgcacaagctgcacgccgccatggacgtgccgctcgagcagatcgccacctacggcaagggcgccatcgtgggcgccgccggcgagctcgagcatggcgcgctctggcatgtgcccggcggttacgccatgcgcgaactgctcggttggaagggcgaccgcgcggcctacaccgcgggcaaggccgaggaaaaaaccggccagcccggcaatgcgctgtccatcgtgccctcgaccaagaaggtcgggccgcccggcgccgcgctcgacgtgccgctcaccaacatcaacgccagctacgtgcgcggccagttcgacgccatcgaagtgcgggtgcccggcgcaccagcagccgacgagatcgtcttcatcctggcgatgagcacgggctaccgcatccatgaccgcgtcggcggtcttcgcgccgaaaacatcagcaagtgggacggcctgcgctgagccgcccgcaccgagacaagaaggaatacaagacatgaccgccaacatccgcaagctcgtcgtgcaggtcgacgagacccgcaaggaaatgggacaggacatcgatccgcccacgcgccgcgccgtcgccatcgcggtgatcgagaacccctatgcgggccgcttcagcgagaacctcgacgagctgatcgccatcggcgaagagcttggcgcgctcctgggccagaaggccgtgaaggcgctgggcatcgagcccggccaggcgcagagctatggcaaggccgccatcgtcggcgagagcggcgagctcgagcatgcggctgccatcctgcatcccaagcttggcgcgccgctgcgcgtggcggttgaaaagggcgcggcactcgtgccctcggccaagaagcgcggcaccctgggcacggccatcgacgtgccgctcggccacaaggatgcggctttcgttcgcagccacttcgacgccgtcgaggcgcgcgtgtccgacgcgccgcgcgccaacgagatcgtggtggcggttgccgtcaccgacagcggccgtccgctgccccgcatcggcgggctgcaggccagcgagatcaagggcgaagacgggctgcgctgagccgtccacccttcacgcgcatccacgttcccgcgatttcttttttctttctttctctttctgtttcgatcccaaggagcttccccatgaacccattgcgtcacgtcttcagcgccgcggcagttgccacgctggccacggccctcgttcctgcccatgcccagggcgtgatcaagatcggcgaggtcaacagctacaaggcccagcccgccttcctcgagccctacaagaagggcatggagctggccgtggaagagatcaacgccaagggcggcgtcaacggccgcaaggtcgaactcatcacccgtgacgacaacgccaaccccggcgatgcggtgcgcgtggccgaggagctggtcgcgcgcgagaagatcgacgtgctcaccggcaccttcctgtcgaacaccggcctggccgtggccgacttcgccaagcagaaaaaaatcttcttcctggccggtgaaccgctgaccgacaagatgacctggcagggcggcaacgaatacaccttccgcctgcgccccggcacctacatgcaggccgcgatgctggtgcccgaagcggccaagctcaagaagaagcgctgggccatcgtgtaccccaactacgaatacggccagtcggccgtggccgcattcaagacgctcttgaaggccgcgcagcccgatgtcgagttcgtcgccgaacaggcgccgccgctcggcaaggtcgatgcgggcgccgtggtgcaggcgttggccgacgccaagcccgacgcgatcttcaacgtgctgttcggcgccgacctttccaagttcgtgcgcgaaggcaacacccgcggcctcttcaaggaccgcacggtggtgagcgtgctcaccggcgagcccgagtacctcgacccgctgaaggacgaaacgcccaacggctggatcgtgaccggctatccctggtacggcatccagacgcccgagcacaaggccttcttccttgcgtaccacggcaagtacaaggactacccgcgcctgggctcggtggttggctacaccatgatcaagtcggtggcggccggcatcgaaaaagccaagagcaccgagacgcccaagctcattgccgccttcaagggcctgcaggttgactcgcccttcggcaagatcagctatcgcgccgaagaccaccagtcgaccatgggtgctttcgtcggcaagacgaagaacgacaacggcaagggcgtgatggtcgactacacgtatttcgatggcgccaagttccagccgagcgcggccgacgtgaagaaatcgcgcgccgcagactgatccttttttcttcccggaacgcttgcacccatgagcctctcgtccctgctgcttcagttcctgaccgggctgtcgtctgcttcgtcgctgttcctcgtgggggccggcctttcgttgatcttcggtgtcacgcgcatcgtcaactttgcgcatggctccttcttcatggtgggcatctacctcgcctacacgctggtcgacaaactcggcacgctcggcttctggccggccgtgctgatcgccgccctcgcggtgggcgtgatcggcgcgctgatcgagatggtgctgctgcgccgcatctacaagtcgcccgagctgttccagctgctggccacttttgcactggtgctcgtcatcaaggatgcggtgctctatgtctgggggccggacgaattgctcggcccgcgcgcaccgggcctgtcgggttcggtcgacatcctggggcggcagttcccgacctatgacctgttcctgatcgtcgtcggaccggtggtgctgggtctcatgtggctgctgctcacgcgaacccgctggggcacgctggtgcgcgccgccacgcaagaccgcgagatggtcagcgcgctgggcgtgaaccaggcctggctgttcaccgcggtgttcgcgctcggcgccacgctcgcggcactcggcggtgcgctgcagctgccgcgcgagccggccacgctggccatggacctcaacaccatcggcgcggccttcgtggtggtggtggtgggtggcatgggctcgattcccggcgcctatgtggcggcgctgctgctgtccgaaatcaaggcggtgtgcatctggctcggcgtggtcgagatcttcggctacagcgtgtcgttctccaagctcacgctggtggtcgacttcatcgtgatggccatcgtgctggtgtggcgcccctggggcctgctgggccgcccgcaggcgccgagccgctacgtgggcatgcaggaagagccactgcggcgcgcgagcaagggctacctgtggctcgtcgccgcgctcggcctcgcgctcatggccatgccgctgctcaccgcagattcaccctacaccacggtgctgatgatcgacctgctgattgcggcgctctttgcggccagtctgcacttcatcatgggcccggcgggcatgcactcgttcggccatgcggcgtacttcggcctcggtgcctacggcgccgctctgctggtgcgtgcgagcggcatgccgatggaactcgccctcgtcgtcgcgccgctggtggccgccatcggcgctttcgtctacggctggttcgcggtgcggctctcgggcgtgtaccttgcgatgctcacgctcgcttttgcgcagatcacctgggccgtggtctaccagtgggattcgttcaccggcggcagcaacgggctcaccggcgtctggccttcggagtggctgtcggacaagcgcacctactactggctcacgctggtgctcgtggcggccggcatcctgatgctgcgccgcgtgctgttctcgccgttcggctatgcgctgcgcgcggggcgcgattcggtgctgcgcgccgatgccatcggtatcgacgtcaagcgcatgcaatggaccgcttttgtcatcgcgggggccgcggctggactggccgggtcgctctatgctttttccaagggcagcatttcgcctgaaagcctgagtgtggacaagtcggtggatgggctggtgatggtgctgcttgggggtatccagacgctggcggggccggtggtgggggctgtgactttcagctggctgcatgacacggtggcgcgcaataccgattactggcgggctacgttgggggcgatcatcttgctgttggtgttgctgtttccgcaggggattgctgggtttgccaaacagcttagcgatcgtttgatgcgggggcgtcgccgtccggaggtggatgttgctttgaaggagaagcggacttgaggggcggttgttcgtctgttgcgctttctttttggttccgaggccgggtctcgccccggcgggcgactcactttctttgcttcgccaaagaaggtaagcaaagaaaggcgacccctactgtctgcgtcccttcgctgcgctacgggcaacctgcggtgctcgactccggcgggggtccgcagaactcgcttcgctcaaacagctgcggccctgatcccgcctccatctgcgctcctcgacgcatacagaaggggtgggagcgggcagccttcgctctcgctcggccccaagaccaacagccaataccgaagtacgcgccaataccaaccaccgcggcgcgcagcgccgcggtggcctggtggccgagcgaagcaaaggcccgttcggtctccaagcccctctgtatgcgccgaggagcgcagggtttcgcggatcagggctcgcagctgtttgagcgaagcgagttctgcgagaccccgcgaaacccgagcaccgcaggttgccccgtagcgaagcgcaggggtcgcagacagtggggtcgccttttctttgcttactttcttttggcgaagcaaaagaaagtgagtcgcccgccggggcgacacccggcctcgggaagcaaacgatcggcactgatcgaaatatcggcagcgatagaaaggccgctcgccctcaccccaaccctctcccaaagggagagggagtaaatccaaatgacccttctcaaagtagacaacctcggcaaatcgttcggcggcgtcaaggccgtggacggcatcagcttcgagctcaaagcaggcgagctgctcgccctcatcggcccgaatggcgccggcaagtccaccaccttcaacatggtgaacggccagctcaaggccgaccagggctcgatcgtgttcgacggccatgaactcgtggggcagaagccgcgcgacatctggcgcctgggcgtgggccgcaccttccagatcgccgaaacctttgcatcgctcaccgtcgccgagaacgtgcagatggccatgctctcgcacgacggcaagctgttctcgatgtggcgccgcgcggcggaccacaagcgcgacgaggcgctggcgctgctcgaccaggtcggcatgaaggcacaggccgaccggccctgcagcgagcttgcctacggcgacgtcaagcgcgtggagcttgcgatcgcgatggccaatgcgcccaagctgctgctgatggacgagcccaccgctggcatggcgccgaaggagcgcaactcgctgatggcgctgaccaaggagctggtggtccagcgcggcctggcggtgctgttcaccgaacacagcatggacgtggtgttcgcgtacgccgaccgcatgatcgtgctggcccgcggccgcctcattgcgcagggcaagccgctcgagatccgcgaccacccgaaggtgcaggaggtgtacttcggcagtggcaagaccttcgagaagattgcagaaaaagccgcggcagtgaacgcggccgtgggagcaacggtatgagcacgcacgaaaccctgttgaaggcgaactcgctgtgcgcctggtatggcgccgcacagatcctgtacgacgtggatcttgaagtgcgccgtggcgaggtcgtcgcgctcatggggcgcaatggcgcgggcaagtcgaccacgctcaagacgctgatcggcatgctcgccaagcgcaagggcaacgtcagcttcctcggccacgacatctcgaagagcgagcctcatcacgcggcgaagctcggcctcggtttcgtgcctgaagaccgccgcgtgttcaccgatctcacggtgatggagaatctcgaggtcggcaagcagccgccgcgccgctgggccgacggcgccgaggcgccgctgtggacgcctgagcggctgttcaagctctttcccaacctgggcgaaatgcccaaccgcccgggcggccgtatgagcggcggcgagcagcagatgctcaccgtggcgcgcacgctcatgggcaacccctacctggtgctgctggacgagccttcggaaggcgtggcgcccgtcatcgtcgaacagatggccaacatgatcctggagctcaaggcgcagggcgtgagcatcctgctgtcggaacagaacatgcatttcgccgagctggtgtccgaccgggcctacgtgctcgagaagggccagatccgctaccacgccaccatggcagagctcgcggccaacgaagaggtgcgccgcgcctacctgagcgtctagcccgcgggcgcccttcgttccctattcatcaaccaccggagcacacaccatgcacgactcgcaccgcagatcccttctgaagtccacggccgcattgagcttgctcggtgcgaccggaacgctgttcgcggcctcgaagctcaagcccaacgacaagtccgcgctgatcgtcatcgacgtgcagaactgtttcgtcgacggcggcacgctgcccgtcaagggcggcgccgaggtggtgccggtgatcaacaagctggccgaatcgttcgagaacatcgtggtcacgcaagactggcacacgcaaggccatgcgtcgttcgcgagcgcgcatgccggccagaagccgttcagcagcatcaagctctcgtacggcaaccaagtgctctggcccgaccactgcgtgcagggcaccgacgacgccgcgctgcacaaggacctgaagctgcccaccgcgcaagtcatcatccgcaagggcttccacaagggcgtggacagttattccgccttcgaggaggctgaccgcaagaccgccaccggcctgggcggctacctcaagcagcgcggcatcaagacggtctacgtggccgggctggccaccgacttctgcgtggcatggaccgcgctcgatgcgcgcaaggccggcttcgaggtctacgtgatcgaagatgccacgcgcgccatcgacctcaatggctcgctcgccgcggcatggaagcagatgacggccaagggcgtcaagcgcatccagtcctcggacatccaggcggcctgagcaccttctctgccgccacaatcaccaccttcgcaaccacaacgacagcaaagagcttgacgacgcatgacgatttcgatttcaaggcgcgccctggtggcgggcggcgcagccctggcaatgggtcctggtcttctacgttcggcgcgcgccgataacggcgtcaccgacagcctcatccgcatcggccagtcggccgtgttcagcggtccggccaaggacttcggcgtcgattaccgcgcgggtatcaagctctatttcgaccggaccaacaaatccggtggcatcaacggccgcaagatcgaactcgtctcgtacgacgatgcctacgaccccgcgaagacggccctcaacacggccaagctgatcgacgaggacaaggtcttcgcgctcgcgggcttcgtagccaccggcaacctcgcggcggcgatgccgctggccgagaaggcgggcgttcccatgttcgcgccgctggtgggcaccagctcgtttcgcgccaaggtcaaccgcctgctgtttcacgtacgtgccggctacgacctcgagctgcgcaagatcatcagccatctttcgaccatcagcctctcgtcgattgccgtggtctaccaggacagcgccttcggcaagtcgaacctcgccacctgcgagaagctcgccgccgaatacaaggtgcaggtcgtgaaatcgctgccgctggccattaccgccgaagacgccaagcaggtcgtcgccggactggccgaagccaagcctggcgcggtcgtgatgatcatggcggggcgcatggtcgaggtcttcatgcgcgactaccgtgcgaacggcggcgcggcgccgctctacacgctgtcggtcggcatcaccgatgcgacgggttccgccaagcgtctcgaaggcaagctcgcgggcctggtcacggccagcatcgtgccgccgccggaagcactgcgcgtgcccatcgtggccgactaccagcgcgaccgcgccgagttcggcgagaagatcgacggctacacggcgctcgaaggctacatcgcctcgcgcgtgatggtcgaaggcctgcgccgcgcgggcaagacgctcacgcgcgacagcttcatcgcggggctcgaaagcatcggcaacacgcgcttcggcgatttcccggtcgagtacagcgcgaagaaccacaacggctcgaccttcgtggacctggagatgtacacccgtgacggacagctgcggcgctgagccgctgcaattgcaggtcaacggccaggcctgttcgattccgggcgtgccgcgcgaggccacgctgctgcacctgctgcgcaacgacctcggcctgaacgggccaaagtacggttgcggcctcggccagtgcggcgcctgcaccgtgcatgtcgatggcgtggcggctcgtgcctgcgtgattcccgcgcatggcgtggcgggccgcgcggtcactacgcttgaaggtcttggcacgcgcggccactggcatccagtacaggctgcctttgaagacgcccaggctgcgcagtgcggctattgcctcaacggcatggtgatgcaggccgcggcgctgctcgcgcgcgatccgcatgcgagcgaggcgcgcatccgcagcgaactctcgggcaacctgtgccgctgcggaacgcatatcgaaattctggatgcggtgcagcgggccgcggtacgtatgcgcgaaatggtgcgtccatgagccgcttgtcttgtcccctctccctccgggagagggctagggtgagggcggcggccttcgcacaagcacggctccagccatcgccgccggccctcaccccagccctctcccagagggagagggagcaagacagggagagggagcaagacagggagagggggcagaaaccgtgactcgacgcgccgatctcccgcagacgcgcgcggagtttctctcggccaacggcgtgctgctggtggtgcgcgagacgccgcccgcaccaccccccgccaagggccagcccacggccgtcgcggggaaccccatcgagggcgacgaaatcctgcttgcggtgtgggacgacggcagcgcgtcggcgctcaacggccacgtcgatctgggcaccggcatccagaccgcgttggcgcagatcgtggccgaagagctcgacctcggcatgccctgcgtgcgcatgatgctcggcgataccgcacgcgcgcccaaccagggcgcaaccatcgcaagcgcctcgatccagatccattcgcagccgctgcgcctggccgccgcgcaggcgcgtgcatggctgcttgcgcgcgcggccgagcggctcggcatgccggtggacgcgctgcaggtgcgcaacggcgtggtgcgcgtggccgatgagcccgatcgccacgtcgactatgccgagctgatcgcggggcagcgcaccgtgctgcggctcgaccccgccgccgagctcaagcacccgtccgactaccgcatcgtcggcacgcgccaggcgcgcgtggacattcccgccaagctcgcgggcgagagcgtcttcgtgcacgacatgcgggtgcccggcatgctgcacggccgggtggtgcgaccaccatatgccggtgcggaccatggcgacttcatcggcaacacgctcgaagcggtggacgaatcgtcgattgcgcacattcccggcatccgcgcggtggtggtgatccgcgacttcgtcggcatcgtggccgagcgcgaagagcacgccgagcaggcgctgcgccaactgcgcgtcacgtggaaaagctggcccggcatgccggacctttccgacctggcgcaggccctgcgcgacaacccctcgacgcagcgcctgctggtcgatgaaggcgacgtcgatggtgcgatcgccgcggccgcgcagccgatgcatcgcacctacgtgtggccctaccagatgcacgcgtccatcggaccttcgtgcgcgctcgccgaatggcaaccgcaggatggcggcggcgtcggttccgccgccgggccgctcccaaggcggaacgcgcccccttcggggggcagcgacccacacgcagtgggggagcgtgggggcattgtcctgcgctgctgggccggctcgcagaatccccacgtgctgcgcgccgatcttgcaaagctcatgggtgtggacgacgtgcaggtcgacgtcatccgcatggaagccgcgggctgctacggccgcaatggtgccgacgacgtggcggccgacgccgcactgcttgcccgcgccgtgggcgcgccggtgcgcgtgcagctcacgcgcgaacaggagcacgcctgggagcccaagggcgccgcgcaactgatggaagtggatggcggcctcatggccgatgggcgcatcgcggcctacgatttcgagacctcgtacccgtcgaacggtgcgcccacgctcgcgctgctactcacgcgcaccatcgaaccggcggcgcaggccttcgagatgggcgaccgcacggcgcgtccaccctacagcgtcgacaacctgcgcgtgaaggtcaacgacatggcgccgatcgtgcgcgcctcgtggctgcgcggcgtgtcggcgttgccgagttcgttcgcgcacgagtcgtacatcgacgagctggccaccgcggctggcgtcgatccggtgcagttccgcctgcgccacctggatgatccgcgcgccgtcgagctcgtgcaggccaccgcgcagaaagccggctggcgcatgcgcaccggcccagaggagaacgccgacggcgggctgggcgagggcggcgacattctcttcggccaaggctttgcctatgcgcgctacatccacagcaagtggcccggcttcggcgccgcctgggctgcatgggtggccgacgtcgaggtcaaccgcaagactggcgaagtgcacgtgcgccgcgtggtggtggggcacgacgcggggctcgtgatcaaccccgcgggcgtcgagcaccaggtacacggcaacgtgatccagaccaccagccgcgcgctcaaggaagaggtgcagttcgcgccgcagcagggcgctgcaaagggtggtccgcaactgcccggcgtgctgccctcgggcgtggtcgcgagccgcgaatggggcagttatccgatcatcaacttccgcgacgtgccggtggtcgagatcatgcatatgccaaggcctggcgagccttcgctgggggcgggcgagtcgtcttcggtgccgggaacggcggccattgcaaatgcgatcttcgatgcgacgggggtgcggtttcgggagccgccgttcacgccggagaaggtgctggctgcgctcagtcccttgaccgcggatttgccccctctccctccgggagagggttggggtgagggcgagcggcctttgaacggggacgccgtcgcaccctcatcccaaccttctcccagagggagaaggagcaatgcagcctggccgcagcgcaagggcctcctcgccaccggcgccgccctcttcatcggcggcatcggcctcgtcgccggcctgctcggctggcgctcttccatcgcccccgtctcgctcagcgccccggtctacagcgaagccaccatcgaacgcggccgcgtgctggccgcgctcggcgactgcgccgtgtgccacaccgcaccgggcggcacacctaacgcgggcggccgcgcgatggagacgcccttcggcacgctctacaccaccaacctcacgcccgatgccgacaccggtctgggccgctggtcgttcagcgctttccagcgcgcgatgcgcgaaggtgtctcgcgcgacggccatcacctgtacccggcatttccgtacacggcattcgccaagaccagcgacgacgacctgcaggcgctctacgcctacttcatgtcgatgcccgcggtgcgcgccgaaacgccgaaggccgagctgaagtttccgttcagcatgcgtccgttgatggccggatggaacgcgctcttccacgatacggcgcccttgcagccggtggccacgcaaagcgcggaatggaaccgcggcgcctacctcgtcaacggcctcggccactgcggcgcgtgccacacgccgcgcaacgcgctcggcgcggagcagggcggcagcgcattcttgtcgggcgccatggtcgacggttgggaggcaccggcgctcaccggcctttcgaagtcggccgtgccatgggacgccgacgagttgtaccgctacctgcgccaaggccatacgcagcgccatggcatggccggcggccccatggcggaggtggtgcgtgaactcgcagaggtgccagatgccgacgtgcgcgccatggccacctacctcgcgtctttcaatccggcgccggcagccgagccgcaggccgtggcacagcaggtggtcgacaccgccgcgcgcacgcagggcaagctgctcggccccgcgccgcgcatgttcgacagtgcctgcgcctcgtgccatcacgacggcgacggccccacgctgctcggcgtgaacacgccgctcgcgctcaacagcaacctcacgagcgcgcggcccgacaacctgctgcgcaccattctcgatggcgtgcgcgagcccgcgagccagggtatcggcttcatgccggcgttccgcgatgcgctcgacgaccgccagattgccgaactcgtgggctacatgcgcgcgcgcttcgcaccgcaggagccggcgtggaagaacctgccggccgaagtggcgcgcgtgcgcgcggcccgcggccatggcgccgaatagcgcaccagtctccggcccggcagcggcaaggcagacattcattcagaatgtccgttccctgaaccacaagcgcctccggagacaacatgcccctcgatctttccaccgccaccagccttccccgcgacgccgagcgcgccacactcgtcggccgcatctggcagcccggcgtgggccccgttctcgtggcggtgcatgagggcggcttgcacgatctctcccggctggcgccgaccatgagcgacttgctcgaacgcgccgagtctccttcggccagcgtgcgcgatgcggtgactgccggcaaggccccgcgcatcgccgagctggccgccgtgctcgccaacagcgacgcgactgcgcgcgacgaagcgaagccatggctgctcgcgccctgcgacctgcaggccgtcaaggccagcggcgtgacctttgtcgagagcctgctcgagcgcgtgatcgaagagcaggcgcgcggcgatgcatcgcgcgccgaggccacgcgcgcggcgctcagcggcgtgctcggcgacaaccttgcgggcatcgtgcccggctcggccgaagccgcgaaggtcaaggaggtcttgatcgggcagggcgcatggtcgcagtacctcgaagtcggcatcgggcccgacgccgagatcttcaccaaggcgccggttctctcggccgtgggcaccggtgccgacgtgggcattcatgccgcatcggtgtggaacaaccccgagcccgaggtcgtgctcgcggtcaacagccgcggcgagacactcggcgccgcgcttggcaacgacgtcaacctgcgcgacttcgaaggccgcagcgcgttgctgctcggcaaggccaaggacaacaacgcctcctgcgccatcggtccgttcatccgtttgttcgatgcgcatttcggcatcgacgatgtgcgccgcatcacggtggcactcgaagtgacggggcccgaaggcttcacgctcgagggctcgagctcgctcgcaaagatcagccgcgatccgctcgacctggtctcgcaagccatcggcgcgcaccatgactatcccgacggcttcatgcttttcctcggcacgatgttcgcgccgacacaagaccgtcatggtcctgggcaaggattcacgcacgtcgtcggcgaccgcgtgcgcatcgcagcaccggaactcggcgcactcgtgaaccgcgtggtccattcggataaagcaccacggtggacttttggcctcagtgcgctgatgcgcaatcttgcgagccgcggactgctgtaaacgttctttctacgctttaaaaggagttgtactcctttgtgattcataggcggcacgtagcaatgtgttgctgttgaccgcgcttcgcgttcccctcaagataaccattgttgatggttattaataaaagggagatggggttgtcgccgagcgagatagaactattgcagtcgcctgttgaaggcccgctaccgtgcggcgaagacctcgaatacgaccccgacttcatggcgctgcagcaggctgcgacaggaaagcgggagcagcagttcggctccaccatcattcccgcggagccacccgactgggcccgtgtcgagcgcattgcaaagcagctgtgccaacgcacgctcgacgtacgcgtgctggttctgctgacgctggcgtggaccgagagccgcggccttcccggctatgtcgatgggttgcgcgtggtggacggcatcctgcaaaagtattgggacgacgtgcatccgcgcgtggtcgatggcgatttcgaagacccgctgccgcgcatgaatgcgctggctgcattggccgaagccgagggactcggacgcagcgtgcgcgacgcacgtctgctcgaggatggcgcatcgatgagcctgcggcaggtcgaggcactgcttgattcaagcaaggccgaccagatcgattacccgggcggcatcggccggctgcgggaagtggcgcgccgcgcgcaggaaaaaacggcagcgccggtgatggcattgcatgcggcgctggagttgctgcagcggattcgcgagacctcggaacgcgcgctggggcaaagctgggcgcctgacttctcgcgtctcgaacgctcgctgcgcaccgtggtccagctgctgcccgagcaggcgcagccggcgccggccgaagcattgaaggccgagagcggcagcgagccggcgcaagcgacggcatcggcgggacagggcatcgcgggctccccgagcggcgcgtccggccagcgggtagcaagcattaaagatattgaaatatcgaatcgtgatgatgtgcaggtgttgctggaaaaggcgtgccaatacatggaacgcaccgagcccagccacccggcaccgatgctcatccgaagagcgcaaagactgctggacctcaacttcttccagatcatcgaagaactcgtacccgagggcttgcagaagatagagagcctggcgggacgttcgctcggcagcagcaccgccgaatagcgaggcaggcggcagcgcaagaacacaaggacagacagtcagggcaggtccgacccacacgcacagagattcaagaggaagcttatggcagacaaccgtgtcagaaacagtggtcagaagttcatcgcgcgcaaccgggcgccgcgcgtgcagatcgagtacgacgtcgagatctacggcagcgaacgcaagatccagctgcccttcgtgatgggcgtgatcgccgatctcgcgggcaagcaggtcgacccgatgcccgatctcgccgatcgcgatttcatggccgtggacatcgacaacttcgacgaccgcatgaagtcgatcaagccgcgcgtggccttccaggtgcccaacacgctcacgggcgagggccagatgaatgtcgacatcaccttcgacagcatggacgacttctcgcccgcgcgcattgcacgccaggtgggcgcgctgcagcacttgctcgaagcacgcaccgagctttccaacctgctgtcctacatggacggcaagaacggcgccgagcagctgattgcccaggcgctgcagaacccggagctgctcaagtcgctcgcctccgcacccaatcccgccgtggccaaggcggtggaagcggcgaacgagaagtcgggcgctcccggcaattcttccgagtaagccgacaggacctccaccatgagcaccgcatccaaacagacagcagcgcgcgcgcagaccgccaccatcgaggcgctcgagcccaacgagttctccgacctgctgcagcgagagttcaagcccaagaccgaccaggcccgcgaggcggtgcagagcgccgtcaagacgctggcggtgcaggcgctcgaaagcaccgtcaccatctccaacgacgcctaccggaccgtgcaggcgatcatcaccgagatcgaccgcaagctctcggagcagatcaaccagatcctccatcacgacgacttccagcagctcgaaggcgcatggcgcggcctgcactacctggtcaacaacaccgagaccgacgagcagctcaagatccgcgtgatgtgcgcgtcgaagcgcgaagtggcgcgctcgctcaagcgccacaagggcatcggctgggaccagagcccgctgttcaagaagatctacgagcacgagtacggccagttcggcggcgagcccttcggcgcgctgatcggcgacttccacttcgaccacagcccgcccgatgtcgagatgctcggcgaaatggcgaagatcgccgcggccgcgcactgccccttcattgccggcgcatcgcccaccgtgatgcagatggactcgtggcaggaactctcgaacccgcgcgacctgaccaagatcttccagaacaccgagcacaccgcatggcggtcgctgcgcgagtcggaagacgcgcgctacatcggcctggccatgccgcgcttcctggcacgcctgccgtacggcgcgcgcaccaacccggtcgacgagttcgagttcgaggaagaaaccgactcggccctgcacaaccgctacacctgggccaactcggcctacgccatgggcgtgaacatcaaccgctcgttcaagcagtacggctggtgcacctccattcgcggcgtggagtcgggcggcgcggtcgagaacctgcccacgcacaccttcccgaccgacgacggcggcgtggacatgaagtgcccgaccgagatcgccatcagcgaccgacgcgaggccgagctggccaagaacggattcatgccgctggtgcaccgcaagaactccgacttcgcggccttcatcggcgcgcagtcgctgcagcagccggccgagtactacgacgccgacgccacggccaacgccaacctggcggcgcgcctgccgtacctgtttgcatgctgccgcttcgcgcactacctgaagtgcatcgtgcgcgacaagatcggttcgttccgcgagcgcgaggacatggagcgctggctcaacgactggatcatgaattacgtggacggcagcccaggcacgtcgtcccaggacacgaaggcaatgaagccgctggcggcggcggaggtccaggtggaagccatcgaggacaacccgggctactacgccgccaagttttttctccggccgcactatcagctcgaagggctgacggtgtcgttgcggctggtttcgaagctgccatccaacaagaaggacagcagctagttcaacggtgtcccgcaatcgggcatatataactttgggggttaatcatggcagtagacatgttcatgcgcgtcgagggcgcaaacggcgaatccaaggactcgaaccataaggactggacggatatcaagtcgtttgcatggggagcgacgcagcctggaaacatggtcagcggcggtggcggcggtgtgggcaaggcgagcttcaatgacctgcaggttcttgcgcgcatcgacaaggcggccccgtccgtcatgaagaactgcgccagcggcaagcacctgagcaaggtcgaggtgtcgttgtgcaaggccggtggctcgcagatcgaatacacgcgcgtcacgctggaagaagtgctggtgacctcggtgcagtacacggctgagcagagtggcgatgcggtgctggtgcagttcgcgttccaggccgccaaggtgaagcagcagtactgggaacagacggacaagggcggcaagggcgccgaaaccgtgctggcctggaacatcaaggaaaaccgggaatcctgatttcccgcgatcccggctgacctgcgcgcgccgctttttttgcggcgcgccgcaggccggtcacccgcagatattcaccggcggcctcgggccgtgcgcgagtcaatgaggaagtttcatgggcgatgggtttgcagtgctgggcgagcgctccgtggccgagcacaccgaatgggtacagcggcagattcgcgcgagtccccagaacgccagcctgcggcttgccctcggccactttcttgcgctccggggcgagtggcagcgggctgaagaccagctcaagctggccgcgaagatcgatccttcttttgctcccgccagcgccacctgcgcgatggcactggcaggcgagcgccaccgaaccgatttctggaatggcggccgtgcgcccgccatcattgccggcgaggccgactgggtcgcggggctggtggccgccgcggcgctgccgttcgagcgcgccatcgaagcggctgacctgcgcgaaggcgcgcggctggctgcgcccggattgcaaggcaccttgagctgcgtcgaccggtccgatgtgcgtaccgcgcaggccatcgatggcgagcctgtggaaagcatcgagttcggctggctgtgcgacggcgacgtgcgcattggcgcggtgctcgaacttctcacgccttcgggctatgcatggctgccgctgccggcggtgcggcgcctcaagttttcccgcccgcagcatctggtcgacctgctctgggcgccggccgagatcgtgctgcaggacggccgcggactcaacggcctggtgccggtccgctacccgggcgcgctcgatgcgctcgacgatgaaaccatgctgggccgacgcaccgactggcagccgctggccggcgaagaacagtacgccggcatcggccagcgcacattgatcagcgaagccggcgaccattcgctgctcgatatccggctcgtggagttcgctcctgcagagagtgccgcgcagtgagttccgtactgcccgccagccgcccggccatggaggccgacggcgaccagcaagagagcgttgcacgagaccgcctgcaaccggtgctgctcgaccgcctgaccgacaagcagccgcaaagccgccaggagcgcgcgggcgcgttcctgatgagcggcaagctgctgcgcgattcggtgctgcgcgatctgcagtggctgctcaacaccaccaactttggcgccggccacaccatcaacgccatgccgcgtgcgcggcgctcggtcgtcaactacggcgtgcgcggctgggccggcgggcgcatgtcggaggtcgacttcgcggatgtggaggctgccatccgcaccgccatcatcgacttcgagccgcgcatcatgaaggacagcatcgacgtgcgctgcgtcaccgatgccaccgacctggagcaccacaacctgctcgcgctcgagatccgcggcacgctgtggtcggtgccctatcccatcgaattcatcctgcgctccgagctcgatctcgagagcggccacatggtcctgcgccccacgggaggactttgatgcgccaactcaaggtgctgtccccgatttgctccctctccccctgggagagggttggggtgagggcgaccgcccctaaaacgagccaagacgcctgcaaggccgaacccctcaccctggccctctcccagagggagagggaacaacaaggaggccggggccactgatggacgcacggttactcgactactacaaccgcgagctcacctacatgcacgagctcggtgccgagttcgcgcagcgctacccgaagatcgcgggccggctgggcatgcgcggcatcgaggtcagcgacccgtacgtggagcgcctgctcgaaggcttcagctttctcacggcgcgcatccagctcaagatggacgcggagtttccgcgcttctcccagcggctgctcgaggtggtgtacccgaactttctcgcgccgctgccggccatgggcgtggtgcagatcgacggcaacctcaatgagggttcgctgaaggccggctacgaactgccgcgccacaccatcctgcgcggccgcatgatcaagggcgagcagacggcctgcgaatttcgcaccgggcatgcggtcacgctgtggcccatcaagatcaccgaggcgagcatcggccccgtgccggcggaaatcgcgcatgcgatgccggccgttgcgcggcaggccaagagcgcgatcaccatcaagctcgaagccgtgggcggcgccaggtttgcggagatgccgctcgaccggctcgaattctttctttcgggcgccgagctgcacgcgctgcgcgtgctcgaactggcggtgcaccacaacgttggcaccgtgtgccgcagcggccccggcagcaccgcgcgtatcgtgccgctcggcgacgaggccattcgccacgaaggcttcgatcccgagcaatcgctgctgccctacgacgcgcgttcgttccagggctaccggctgctgcacgagtacttcgcctttccggaccgctacctgttcttcagcgtgaagaacctgcgcgcggcggccgcggccatgagcggcaccacgatggaaatcgtgatcctgctcgaccgtgccgacggcgacctggagcggctcgtcgatgcacggcatttctcgctcttctgcacgcccatcatcaatctggtgccgcgccgcagcgaccgcattccggtcggtcccgggcagcacgagcaccatgcggtgatcgaccgcacgcgtccgcgcgatttcgaaatcttcactgtcgagcgcgtcacgggccacatgagcagcggctcggaagagcgcgagttcaggcccttcctggggtcgttcgcggccgacgacggcgacttcggttcgtacttctcgctgcgccgcgagccgcgcctggtgtccgaccgcgcccgtgcgcagggcacccgcaccagctacaccggcagcgaggtgtacgtgtcgctggtcgaccagcacgacgcgcccttcccgcacagcctgcggcacatcacgatcgatgcgctgtgcaccaaccgcgacctgccgctcttgctgcccacggggctggagtccgacttcaccttgcgcgtgtccgcacccgtgcgcgccgtgcgcatcttgcgcgggccgtcgcggccgtatcccgcgctggcggaaggcgcgctcacctggcgcctcatcagccatctggggctcaactacctgagcctgaccgacgtcgatgcgacgcagggcgcggctgcactgcgcgagatgctcgacctgtacggcaacctggccgacccggcggtgcgccggcagatccagggcgtgcgctcgatggcgctggcgcccgtgttccgccgcctgcccgaacccgggcccatcgtgttcgggcgcggcgtggaaattgcgctgaagatcgacgaggtcgccttctcgggttcgagcccctatcttttcggtgccgtgctggagcagtttttcagccggcatgtgtcgctcaacgcgttcaccgaattcgcgctctccagcctgcagcgcggagaaatcgcgcgctggatgccgcgcatcggacgccgccccgccgtatgagcgcaatcgatgtcaccggcgattcgccggcgctgcaagcggtgccggatgtgccggccgcaatcaaggcctccgcccggcgcggcgttccagaggccgaccccgtcttgtgggcgggcttggtcgaccagcctttcgagcatgacctgttcatgctgctgcggcggctcgatgcgcagggcggccacccgttgctgggccgcgcgccgcgcccgctcgacgagccgctgcgcctcgggcaggagccctcgatggcgtttgcgccgtcgaatgtttcgggtgtgaatgtcgacggcgacggaccgccgcgcatctccatctacggcttcggcctgttcggccccaacgggccgctgccgctgcacctgaccgagtacgcgcgcgagcgcaagcggcatcacggcgacgacacgctgagcgtattcgccgacctgttccaccaccggctcatcctgttgttctaccgggcctgggccgacgcgcagtcggtcaacagcctggaccggcccgacggccaccgcttcgtcgactatgtggcgagcctcatgaacatggggcagccgggcctcaaggagcgcgaccgcatcgcggaccacgcgcgcaccttcatggccgggcacctggtgcgccagacgcgcaaccccgagggcctgatccagatcctcaagctgtacttcgacgtgcccgtgcgtgtcgaggaattcgtgagcgactgggtgacgatcgatgagcggcaggtgagccgcatcggcctcttcgggcgcaaccaccggctgggtggcggcgccaccatcggcctggccgtgcgcgatgcgcagagcaagttccggctcgagctggggccgctctcgcagagccagttccgcgatttcctgccgggcagcaagcggctccagcaggtgctcgattgggtgcgccagtacgtcggcatcgagtttgcctgggagctccggctcgtgctgaagaagcaggaagcccgcggcatgcaactgggcagcgaccaccgcctgggctggggcagctggctcggcacgcgcctctcggacaccgacgccggcgacatggtgttccaacccgaagcattgttttcccgttccgcatcggcagcttccgtggcggatgaagtttcttccatggccctatgaccgatattcgccgcgtctctcttttctcgaaactgaacccgatgctctacaaggcattggaaaccgccaccgcgttcgccaagctgcgcggcaatgcctatgtagagctggtgcactggctgcaccagatattgcagttgcaggacagcgacctgctgcgcatcgtcaagcgcgcgggcctcaacctcgatgcggtcgagcaggacctagtgcgcgcactcgaccgcctgccgcacggcgccacctcgatcagcgacatctccgagcatgtcgacaacgccgtcgaacgcgcctgggtctatgcaagcctgcgcttcgaggccacctcgatccgcggcgcctacctcttcgccggcatcgtgaagacgccgggtctgcggcaggtgctctcgggcatctcgcgcgagttcgacaagatcgtgcctgacgttctcatcgcccagctgcccgcgtggaccgaaggttcgcccgaggacgacttcgatgccgcgccgcagggccatgccggcggcggccacgcgcccgcagcggcgcaccagggcgatggcgccgcagctggcggctccgcgctggccaagtacgcgagcgacctgacagccaaggcgcgcgcgggcgagctcgatccggtctatgggcgcgacgacgagatccgccagatcatcgacatcctgatgcggcgccggcagaacaatccgctgctcaccggcgaggcgggcgtgggcaagacggccgtggtcgagggcctggcttcgcggctcgccgcgggcgacgtgccgccctcgctcaaggacgtatctctgtgggtgctcgaccccacgttgctgcaggccggcgcgggcgtgaagggcgagttcgagcagcgcctgcgccaggtgatcgacgaggtcgagaagagccccaagcccatcgtgctgttcgtcgacgaggtgcacacgctggtcggcgcgggaggcaccgccggcacgggtgatgcggccaacctgctgaagccggctcttgcgcgcgggcggctgcgcaccatcggcgccaccacctggtcggagtacaagaagtacatcgagaaggacccggcgctcacgcggcgcttccagaccatccaggtgcacgagcccaccgagcccaaggccgtgatcatgctgcgcggcatttcggccgagctggaaaaacaccacggcgtgctcattctcgatgccgcgctcgaagcggccgtgagcctgtcgcatcgctacattcccgcgcggcagttgcccgacaaggccgtgagcctgctcgacacggcatgcgcgcgcgtggccctgagccagcatgcgctgcccgccgccatcgaagacctgcagcgccgcatcgaggtgctgggcatcgagtcgggcattgccgggcgggaggccgcgatcggcgtgggtgagcacaagcgcgtggaagacatcgcggcccaggtggccgcggcgcaggccgaactcgatctgctggaaaagcgacgcgtagaagaggctgcgctggtcgagcgcatcgtcgcgctgcgcaagctgctgtcgcccgccgcggtgcccgtgcaggccgtggttgaagatgacggcgacgaaggggcggcagacgcagcgccgtccgccatcgacaccgacccggacgcacccgagcgaacgcccgcagagattcgcgccgaactcgatgaggcacaggacaagctcgcgcagctgcagggcgaatcgccgctcatccttgccgccgtcgatgcgcaggctattgccaccgtggtggccgactggactggcattcccatcggccgcatggtgcgcgacgacgcgcaatcggtgctgcggctcggcgagattctctcggcccgcgtggtggcccagcccgatgcgctggagaccatttcgcggcgcatccgcaccgcacgcgcgaggctcgacaacccgaacaagccggtgggcgtgttcctgctgtgcggcccttcgggcgtgggcaagacggagaccgcgctggcgctctcagaagcgctctatggcggcgaacagaacctggtcaccatcaacatgagcgagttccaggagtcgcacactgtctccacactcaagggcgcgccgcccggctacgtgggctacggcgaaggcggggtgctgaccgaggcggtgcgccgcaggccctacagcgtggtgctgctcgacgagatcgagaaggcccataccgacgtgcacgagatcttcttccaggtgttcgacaagggctggatggaagacggcgaaggccggcacatcgacttccgcaacaccgtgatcatcatgacttccaacgtcggcaccgacctggtcatgcaattgtgcgaagacccgaccctgcggcccgaccccgaaccgctggcggccgcattgcgcgaaccgctcctcaaggtgttcgcaccggcgctgctcggccggctggttgtagtgccttattacccgttgcaagccgatgcgttgcatcgcatcattcgccttcagctcgaccgcattgccgctcgcctcgaggcgaaccatggcatcgccctggactacgacgacagcgccgtcgaactggtggcgcgccgttgcaccgccatcgagtccggcggacggatgatcgacgcgatcctcacgcacaccattcttccgcggctgagcgaagaggtcatcggcgccacggtcagcgcgcgcaagctcgccggcgtgcgattgcgcgctgcggacgacgactttcactacgaattttctgaacgctgagcgaagaaagggagtaagccatggccaccagagtcgtcaaagcccacacgccactgccagaagaccagctgatgttccgctcgatgcacggcaccgagggcttgtcgcagctcttcgagttcgaggtggatctggtgagcccgagcgtgtcgctcgacatgaagtcggtgctgggaaaaccgctctcgctcgaaatactgacgtccggcgagcctcgcttcctcaatgggcagatcgtccgtttcacgatggtcggcaaggaggggggcacttcgcgctacgtgctgtaccgcgccaccgtgcggccctggctgtggtatctgacgcgcaccagcgactgcaagatcttccagaacaagtcggtcgtggacatcctcgaggaagtgtttgccgactacaactttgcgttcgagaagaagctcagcggaacctaccgccagtgggaatactgcgtgcagtaccaggagaccgatttcgctttcgtgagccggttgatggagcacgagggcatttactactacttcaagcacgacaagaaccagcacacgctggtgctcgccgatgacatcggcgcacatgaaaccctgccggcctacccgaagatcagctatctcgcggccgaccgcgaccccgatccgttccaggaggtgatcgaccagtggcaggtgaccgaggaaatccgccccggcacctacgtggtggacgactacgacttcaagaagtcgaaggccgacctcatgggcatgcgcagccagccgcgtggaaatcctcacgatacctacgagatctacgaatggctgggcggcttcagcgaggccgagcagggcgagcactactcgcgcatccggctcgaagaagcgcagtcgcaggccgagcgtgacatcggccattgcagcgtgcgcggaatggcgccgggctatcgcttcacgatgcagaactgtccacggcaggacgacaaccgcgaatacctgatcgtctcggtggcctacgcgctgcgcgaaggcggctacgagagcggtgcggccgacagccagtacagcttcagctttgcggtgcagccgacctcgtatgcgttccgcccgccgcgcgtgacgccgatgaccaaaaccaacggaccgcagaccgccaccgtcgtgggcaaggcgggccaggagtattgggtcgaccaatatggtcgcgtgaaggtgcagttccgttgggaccgctatggcaagagcgacgagaacagctcctgttgggtgcgcgtctccagtgcctgggcaggctcgaactacggcgccgtcaatcatccgcgcaagggccaggaagtgatcgtcgacttcatcggcggccatcccgaccggcccatcatcatcggccgcgtctacaactccgaccagatgccgccgctggagttgccggcgaaggtgaccgtgagcggtttcgtgagccgcagccaggacggcacgccggcgaatgccaacgagttcatcctggacgatgcgccgggttgcgagctggtgcggattcacgccgagaaggatttcgaactcgatgtggaagcggacgagagggacactatcgccggcgatcgcaccacagtgatcgagggcgccgacgactacacgaccaacacctcgctcaccgagacgatcaacggcccgcataccgtgacggtcaacgagggtggaccgcagaacatcaccgtcaatggcgggccgcagaacgtcaagatcaaaggtggcaaccaggatgtctacgtcgatggcgaccagatcattcacgtgaccggtagtcgcacagacacggtggacagcggcgagacccggacgataaccggcggtttgaccgaagacataacgggacgtcagaaaacgacgatttccgcagcatatgaagaaacctcaggaaccaaaaatgtttcggtcagcaaaggaaacgaagactattgggtgagtggagacagcgttcggattgttggaggcaagtcaaatctgtattcggtcgggacggttcaggtcgacaccgtcggcggcatcaatctctttgcgaactcaggcgacgtcaacgtaacgacgccgaaccagttcaacgtcaatgccaacacgatcagcttgcactccgaccacaaggacgtcagctacacgaactcgctgcacacgcacgcgggcagcacgatcacgaccgaggccgacctttcgatcacctcgaagacgctcttctcgttcgccatcagctacgtgaactccttcacttacgcgtcgctgtccgaaaccgtcaacgccgtcagcctcaacgtcggcggcgccgccttcgactggaaggtatacaggctgtcgaaccaggcgctcaaccacggtaatggcgccaagatcaagatcgggccgttcaaggtcatgatcaagggcttgttcctctgcacatgaccggcgccgcatcgctgtccctgctgatgaaatggttgggggcggtcctgttcgctgtgggcgtcgtgccgatggtggtgttcgccggcggcatgagcgtgcgccagatgggagtgtgcatcgccctgatgctggtcgggtccttcctcctgtgcggtggatgggacctctttcagctctcgcgccgcgaggcggcgagtaacacgctcgacggacgggcggacggtgtgatcgtggcgagcgagatgggcggcagctacagcgatcgcagtcccctgatcacgttcaccgtggcgttccgggatgcggccggcgtccagcacagcgcacgactgcacaaggtcgtgccactcaacgagctcaccctgtacggcatcggttgcacggtcgatgtccgctatgcgccggaccgtccgtcacaaaccgccgtgatctttccggccgccgcatcccgttcctcttcttcttcctgatcgatcaccgccgttgaaaatcgtcaagccattccgactcagcctgctgacgcgcccctaccgctggaagggcagcaaccatctgggcatcgcctcgctcgccctggtcagcctgaaggcagacccgcaactgcagcctgaacaggagctctggcagatggtgagcgaggtgctcgaccccggcagtgtgctggacctgggcatgcccaaggccgaggccgaggtgctggccagcggctttgcctacacctgccaccaggcggagaagtcgcagtgcgcggtgcgcttgcgggtggaaacgctcgagaagtcgctgctggtgtccggcgatcgctactggcttgacgggcgatcgacggcccccgtgcccttcgagcagatgccgctggactggcggcacacctacggcgggcccgggttcgcgcagaacccattgggcatcggtgcgcaggacgaggtcgtcaacggcgtgcacacgcgccggctgcccaacgtcgaacaggcctcccatcgcctcaccgaccgcgagcggcgcggcgcgccggcggcgctctgtgcctatctgccggactggccgcagcgcatggcgcacatgggccgccagtacgacaacgcatggctggagaacggctaccctggtttcgccgacgacatggactggcgcttcttcaattcggcgccggaggaccagcgctggcccggactcagcacgctgccgccgggcgcggcatacgaactgtggaacatgcatccgcaaattcctgtcatgcaggggcatcttcccgactggagcgcggcctgccacgtcagcttctcggacgatgtccagacgctcagggcggtgccgctgcacttgagcaccgcatggttcttccccgatcgcgagcgcgtgatcctgatctggcacggttcgacaggcgtgcgcgaggacgacgccgccgacgtcaagcacatcatgccggtgctcgagctgcgggacgcgccgcggccgccagcgcactaccgcgaggttcttctcaagcgcatcgacccggaaaaagccgcggtgcatgtgctgcgcgacagcgacctcgtgccccggtcaatcctcggagactggcggcagatgcaactggccgacacgatggccgagccactgccgcgcaacatgcgcgccggcctgttgcgcgaccacgaagcgcgccgtgcggacctgctggcgcgggggctcgaccccgcccagtacctggaggcgccctgggagcccgaaccggttccggacttcgacgatctgcccgaatacctcgagcgcgccgaagcctcggcggtggagacacgggatcggctacagaaggagtccgagcgcatcgaggccgagcgggacgccttgccggacggtgctgccgggtcggcggcgcgcgcgcagccagtggtgcccgatccgcaacagatccagcgcgagatgaagccgggtgaccgctacgaccagacgagcccgggcaacagcgaccctgaaaccgaagccgacagcgccgacgagacggacgcaccggcggtgcccgccgatccgttgatgcgcctcggatacctgcactcggcacatttcggcggcgcggcacccgcaatgccgagcttccgaagtgccaagctgcgccggcggctgtcggtggccgaacccgggcagcgcacgttcgcgcacatgagcctgatcggcgccgatctgtccggcatggacctgcggggcgccgatttctcgcaagccatgttgacggacgcgaacctgagcggcgcgcagctcgacgactgcaatttttcgcaggcggttcttgcgcgtgccaacttcacggatgcgagcctcgcccgcgccaggctggacgaggccaacatcggcggtgcccgcttcgatcgtgccaaccttgagggcgcgagcttgcgggaggtgcatgccgaccaggcgcagttcgtggactgccgcatggctggcatccgcatggaccaggtgcaactgcacgaagcgtcgttcgcgcgctgcgacttccgcggctcgcaatggcgccagatggccctgctgcagatgacgctcgaagatctgcacttcgaccaggccgagatgctgcaggtagtctggatcgaatgccagctgcgccgcgtgtcctttgccggtgcgaagctgtcgcgctgcggatttgtggcggtcgcgttcgacagcgcggcggatttttccgatgcgacgctggacgcctgcagcgtggtgcaaggcagctcgctgtctggtgtgcggttcaacggtgcaaggttgaagcaatgcggcatgcgcggcatgccgctggtggcggcggacctgagcggggcgcgcctagagacctgcgatttttccgagtgcgacttcagcgacgcgaagctcgatggcctttcggccggcgagagcctgttcgtgcgcgccgacttcacgcgcgcctccttgcgcgccgccagcttcatcgatgcgaacctgtcgaaggctgtgctcacccattgcgatctgcgcggtgcgaatctcttccgcaccgatgtctcgcaggccctcatcgacggcaccacgctgctggacggcgcttacacccggcatgccaaggtatggccggcgcgccccgcggacacaccggcaccatgacgcgcgacgaactgctcgaccatgtgcgacacggcgtccaggtccggggcgtcgagtgccgcggctgggatcttcgcggcctcgatctgtcgggcgcgctctgggacaacgtcgacttcacgggcgccaacttccagggcgcgcacttggcaggcagcgtgatctcgcattgccggatgggcgaatgcgatttctcggacggcatcgccggcaaggcgcagttctaccggtgccggttcgagcgagccgatttctctcgggtcacgctcgaagaggcatcgttcgtcgaatcgcacctgcagcgggccgatctgtccggcgccaacctcgaccgcgcgaccttcttccgctcggaccttacgcagacccggctcgccatgctgcgcatggaccgggccacggtggctgagtcaaagctcgcgcaaactgatttcaccggcgctgtgctgagcttcgtcaccatgtacaaactcgacctcacgaccgcggccttcgccgatatgcaggccgacagcgtggtgtttctggagtgcgacctcacgcgccaggtcttcgcgggcctgacgctgcagcgatgccagtttaccgacagcaggctggatggggccgacttccgcaatgccacgctgacgcagagcaacttcaagggcgcgtcgctgcgtaatgcggacttctctggcgtggcggcggcgcagacgatctttgccgaagctgatctgggcgaagcgaactgcaggcgcggccgtttcgagcagtcgatctgggtcgatgcgaagctgcaggacacggcgttcgaggatgcctttctgccgctgagcgtgttccatcgcgcgcgcgcgaaccgagcggtcttccgtcgtgccgagttgcaggatgccgatttttcgtacgcggacctcagcgatgctgacatgagtggcgcgcacttttttcgtacgcgctttcatcgagccattcagcaggggacccgcttttccgcacgcggtggcatcattgaaaacgaccccgaactgcacaaggcgcaagcctggtccggcgactccgcgtgagtggcagggctctgcgcaaccgatcaacgccaagaagggaatcatcatgaaagtcgttccactccgctcggccccggccgaatcgacgccggtccatttcatcggacggctgacggcccacatgcccgatgggcagttgggggtcgaagacgacgagggtgtcgtgtggatgtgccggcgcgcggcgagctgcctgctcaagccggagcagggcgacacggtgctcctgtcggggccggaccggttccgggtctacctgatcgcggtgatcgaacaggccgaccctgccacgagccgcattgatgcaccgggcgacatcacgctcggcagccccaggggcacggtgtcgatcgagagcgcgggcaatctcagcctgcgaagcggcgcgactctggaaatgaaaagcacgcaatgggccgtgcaagccgacgaaggaaattgccgcgtggaccagttgcatgtcacggcccagtccgtggatgcgacggtgggccggacgcgactggtcggcaaggtgctggagaccgtcaccgaccgtatcgtgcagatggcgcgcaatgcgttgcgtctggtggaggaagtcgaccagtcccgtgtcggccacctggactgcaaggccacgcagacggtgcgcatccacggccagcacacgatggtgaccggcaaggaactggtgaaggtcgacgcctcgcagatccacatgggctgatacggagtcaacgatgtttgcaaactgccaactgatgggcatggacctggccttcccggatgtctgccgcactccggtgcctattccctttccaaacatggccctcgggccgatggccgtaccgaacgcctggaatatcctcttcatggcgatgccggcccacaacatggcgaccaccacgcccatcacgctgggcgaccagcccggggcgttgggcggtgtggtgtcgcagaccttcatgcagcaatcgcgtcacctcaccggtgcgttcacagtgctgctcaagggcacgccggccacccgggtgaccagcatcacgctgcagaaccgctgcaacatggtgggcatgcgcatcgtgccgagccagttcaaggtgctgatgctcgcagcttgaaaaagcctagctccggcgcaggccggagtcaggcggatgggcgcggcacagccgtccccgccagcgtcacctgctgcggaaaccccacccacaccgccagcgccgagtagttgtcgcgcgattcgtcggccttggcttcggccgcgcggcgcagcagcgcgagccactcttcggcgctgtcggccagctgcagcgatcgctccatcacctgctgcgagatgagctgccagaggccgtcggtgcacagcaggaatgcatcgccgtcggcgagccgttgaggcgtcgccacggtggtctccgccgtggcgcgcgcgccgagggcgcggtacagcaggttggtttttaccaggcgctcgcccccgttggcaccgttgcccagcgcggcttcgccggagcgctccgacaggctgtggtcttcggtgcgctgcatcagcgcgccgcggcggaaccagtagaggcggctgtcgcccacgtgggcccagcaggcctggccgctggtgcggtccacgaacagcgagacgatggtcgcgctcatccggctctggtcggcgagctcccgctgcttggcaagaatggcgtcgttggcggccttcacggcctgctggatgtcgtgttgcgccaccgacgggttgtcgacgaaggtgttgagcgcggtatcgaccgcgatgcgcgcggccagctcgccgcccgcgttgccgccgacgccgtcgctcacgacgaagcaggcgttgtattcgtccaggtggtagccgatggcgtcctggttgccgctgcgttcgcccacgcaggagaactgcgacgtcgaaatgggaaccgcgaaagcacgggtggtttcaagcacggcgtgcctccttcaagcggtccatctccttgtcgtaggcctgttggaaggcccggccaaagacggcctgaaaatcgtcctcgaccgcggccgtcgtttccgcatgcagcttctgcagctggcgccacaaacgcgcctcgcggccgccgggcagcagcttctcgcccagtccgccgtcgtgcggcgtggcggtgttcagcgccgtgggatcgaagcgcttcagcaccgtgagcagcgccgcgcgcatgccggccaccatgccgagctgatgcgactgcaggtcggcgagcgcgtcgtgcacggcggcttcgggcgacaggaagccgggcatgcgcgcgccgaacatctgcatcagcacggcgcggccgttgggaagaatcttgaacgggttgttttcctcgtcgacgatcatcgtgatctcggcgcgcacttcgcgcttgagcatggcgcgcgacgagagcagttcgatggtgccgtcggtgaacgcgcgcatgagccggccgaggcgccgcatggcctcggtgtccagcggctgatggccggccacgtcgggaacgccggcgccttcgagaaaagccttgaagagctcgtccggcgaggcgtccgatgatgatggcgacgcagatggcgccacggtggcaagcggcggggccgcggcaggcttgggtgccggtgcggccggttcaggcgccgtgggcttcgcaggcggtgcggtctccatgcgaacgtccgtggccggcgccaaggcgggagggctcacgggctcgacaggcgccgatgctgctggtggcggtggcggtggcggtggcggtggcggtggcggtggcgccgccggttctggcggcgcgggcacctctgccttcaccggcttcgcaacagccggcggatcgaaggccacgggggtcggcggcctgaactgcgccgacacttcgcgcgcatggttcgcatggctgggcccttgctgcacggccggcttggcgagcaggtcgagtgcgggatgcacgttaccgagcgggtcttcgtgggtcagcgcggtgggacgcggatccgaaagcggcgaaggtgcgttgctgtcggcggcaaagaaagagagcgggtccacgccacgcttcagcgtcacgtcggacatgtcgttggctgcccgcgggttcagttcggccagcggatcgaccggattcctgcgcgcctgcgatggcagctcgaaaggctcgtgcgccatcgggtcgggcatgggctcggccgcgctctgttcgcggcgcggcgcgttcgcgaggatggcgtcccaatcggcggcggagggaatctgcgaagccgccggacgaacgctggccggcgatggcgatggcgatggcgatggcgatggcaccggtgctggcggcggagcgaacacgggcttcgcaacgggcggtggttccgatgctggcggcggcatggccacggtggcgggctgtgcctcgccgatgggcagcgcgcccgcgccgaagagatcggagaacacatcggacaccggcgcggccggcagcaacgtgtccatggacgctggtgccgtcgcattcgcgggtacgggaacatcgcgcacgggcgcgatgggcggtggtggcgccgcggccggcatcggcactgcggccgcaacgcgatgcccgcttgccgcttccagcacgtagcttccgatggtcacgcggtcgccgtcggccaccggcgattcctgctcgtgctgcagcgtgcgtccgttgacgccgatgggaagcaccgcgctcatgttgcgcagcaccgccacacccttgtcgtcgaagcgcacggtggcctgcaggcgcgagatctggcgctgctcgtcgggcagcaccaggtggttgtcggggctgcgtccgatcgttccgccgggcgccgcgagaagggccgaaggccccgaggccaccggcctgccggcatgttcgatcaccgtccaacgcatggcatctccgtgttcatgtcgagccgcggctcaccgcctgcggcgttcaacgcttcattcgcttggctgcctcgaacgccgggccccagaccgggtgcttgcgctcggcaacgctcaggtcgaagttgggaaacgcatcgagaagcttgcgaaattgcgtgcggcattcgggcacctggttggccacgcaatagctgaacgcctcgagcttcatggcgtcgagccgcgtgccaggctctgctgcgtcgaataccgacacgccgccgctcttgagcgtggtgacggccttggcgtaatcgccttcgtcataggcctgctgcgcgcgttcgagcgtggtgcgcgccacttgctggctcaatcgttcgggttgcggcggctcgggcgggggcgtggtcgtgcaaccagccaccaaaaataacgtgaacgccaaagcaggcagacatgatttcaatcttctctcctacctcgcaaaaggcaatgcttgagatagtgtgccgctgtcattgcgacaggcacacgatgcgacgcggttcgtgcgcacgacttcgataatataggccgcgaacctctggggaagatctcatgcatcgacgaaccttgcttcaaggcgcacttgcaaccgtaccgttgtttggtggcctcagtggatgcgcatcgacagcgaagtcattgcccacaccttacgccgtcaccattcgcatcgacgatggcgtcaaccccgacggacgcggccagccggcgccgattctcgtcaaggtcttcgagctgaaatcttccggtaacttcgagacggcagactactttgcactacaggaccgcgatcgcgaaacgctttcgacggaactcgtgaacgccgaccaggccatcatgcgcagcggcgaagagcgcgtcttcaagcgagaggcggggctcgactcgcgcgccatcggcatcatcgccggctaccgcaagctcgaggcctcgcgctggcgcatcgtgctgccgctcaaggaaccgaagcaaaccaacctgtacaaggtgtggcagttttcgccgagcgaacaaggcgtgcgcatcgccattcgaaagacaggcatcgagttactaccaactcgttaactttcatgcttttagtaatgcttaagtgcgagtagtcgcgaacgaaattcggtgcaaaacgtaagaggcgccgtgtagcatcaagagaaaaaaatcgatcaatcgggagacgtcgaaagacgcatctcgccgcttcagtgtgggcactccccaggaggttctttggtgacagttcgcaatccgggcgccggcaggcagggcgtccatccgcaggcgttggcgaatcgcgtggtgtggtccgaaggcatgtacctgcggccccagcatttccagcagctggagcgctatgtcgagcagtacgtcacgcgccgtaccgcgggcctgcaaggcgcctactggggatggcttcacctggacatcgaccgcgatgcctacgcactcggccgcgtgtcgctgctcggcggcgcgggcgtgctgcccgatggcacgccgttctcgttcggcgccgaagatgcgccgccgccttatgaagtgccgagcgacctgaccgacgaactcatcgtgctcgcgctgccgctgcgccgcaccggcagcgaagaaatcatcttctcggacgacgaaggctcggccgcgcgttttggcgtgatcgagcgcgaggtggccgatggcaacgcagtggcgctcggccccgcggtgctgcagcttgcgaagccgcgcctgcgcctggcgcgtgcgtcgtctctcacggcggagtggcaggcgattggcgcggtgcgcgtgatcgagcgccgcaccgaccacaagctggtgatcgacgccaactacattccgccggtgctcgatgcgtcggcgcacgccatgctgcgcagcatgatcgccgagctgcacgggctgctcacgcagcgttcggaggcgctggcctcgcgcctctcgcagcccgggcgcggcggcgtgagcgaggtctccgactttcttctgctcgaactggtgaaccgctatctcgcaaccacgtggcatgcccagcaggcggtgcaggtgcatccggaacatctgttcgtcgactggctcaagctcgcctgccatctcgccacgcacacctcgcccacgcggcggcccgtggtgtggccggtgtacgaccacgacaacctcaacgagagcatccgcccgctgatggaagaactgcggcgatcgctctcggcggtgctcgagcagagcgccatcgccattgagctcgaagagcgcagccacggcgtgcgcgtgggacgcatgcccgatccggtgctggtgcgcaatgcgggcttcgtgctggcggtgcatgccgacctgccggccgacgcgatccagcagcgctttccgacgcaggtcaagatcggctcggtcgagcgcattcgcgacctggtgcaactgcagctgcccggcgtgacggtgcggccgctgccggtggcgccgcggcagattccatacaacgcgggctatcactatttcgaactcgacaagagcggcgacatgtggcgccagctcgaaaaatcgggcggcgttgcaatgcacctggccggcgacttcccggggctggccatggagttctgggcaattcgtccgtgagggaccctatgaacggtgtcaacgacatggccgtcggtccgggaggcttcgtgccgccgaacccgggcggcagcggcaacagcgatcacgcgggcgtaccgccggcgtcgcgcggcctcggccagcaaccccagtcattcaccgcatggcacgacgcgcgccgtccgcatgcgggcgacacggcgctggcgggcaacaacccgctggttgccgcggccaacccgctgctcgacctgatcccgcagatccgcgccaccggccaccacgatgcgcccgcgcaattgcgcgagcacctggtcgacgaggtgaggcgcttcgaaacgcgcgcgcagcaaagcggcattgcgcccgaggtgatcatcggcgcgcgctactgcctgtgcaccgcggtcgatgaagccgccgcgctcacgccctggggcggcagcatctggtcgtcgcagagcctgctcgtgatgttccacaacgagacctggggcggcgagaaattcttccagctgctgtcgcgcctggtgcagaacccgcagcagcatctgcagctcatcgagctcatctatttctgcctggcgatgggtttcgaagggcgcttccgggtcatcgacaacggccgcacgcagctcgaaacgctcaagcagcggctgctgcagatcatccgccagacgcgcggagaaattgccgtgccgctgtcgccgcactggcaggacgcgagtgcgccggtgcgccgcacgcgcaactggctgccgctgtgggccgtgggcgcggtggcggcggtgctgctggtgctggtgttcggcgtgctcacgttcagcctggccggccgctcggatggtgcgttcgcggccgtgaatgcggtgcgcctgccgcagaccgcgcgcgccgtggcgcaacccgcgccgcagccgcggctgcagcgctttctcgaacccgaaatccgcgacggcctgctgacggtgcgcgacgaggccgaccgcagcgtggtggtgctgcgcggcgacggcctgttcgcatcgggctctgaccgcgtgctcgaccgctatgcgcccgtgctcgcgcgcgtggccgatgcgctcaacgccgtggaaggcaacgtgctggtcagcggcttcagcgacgaccagccgattcgcagcgtgcgcttcccgtccaactggcagctctcgcaggcgcgcgccgatgcggtcaagaaaatgatcgccacgcgcgtcacacggcccgagcgcctgcgcgccgaaggccgcggcgatgccgaccccctggcgcccaacgattcaccggccaaccgcgcgcgcaaccggcgggtcgaggtgacgctgctggtggcacccgtggccggcgccgcagccgcagcgccgcagggaggagcccgctgatgctgcgcgcgattttccgtttcctcgtgagccgcgacctgtgggtttttctcggcctcttggccgtcgcgttcctgatctgggtcatcggtcccgtcatcgcggtgggccgctaccggccgttcgaaagcgagttcgtccgcatcgtcgtgatcgcgctgatgttcgcgatctggatcgcgcgggtgctctaccgcaaatggcgcgagcggcgcctcaatgcccaactgctcaaccagctgcgcacgccgtccgcgaaggagaaggccgccaagcccgaagacgcgcccgagatcaaggagctgcaaagcggcttcaccgacgccaccgccatcctgaagaacatgcgattcggtacgggcgccgaaggcaaggccgcgggccgcttcgcggtgttcgaccggcagtacctgtaccagctgccctggtacatcttcatcggtgcgccgggctcgggcaagaccacggcgctggtcaactccgacctcgactttccgctggccgaccaactcggcaaggccgcggtgcgcggcatcggcggcacgcgcaactgcgactggtggtttaccaacgaggcggtgctgatcgacaccgcggggcgctacaccacgcacgagagcaaccgcgaaaccgacgagagcgagtggaagggctttctcgacctcttgaagaagttcaggccgcgccagccgatcaacggcgcgatcctcaccatcagcattgccgacctgccgctggccgacgacgcacagcgcgcgcgccacgccatggcgctgcgcaagcggctgctcgaactgcgcaacggcctgggcatcaactttccggtgtacgtgctggtcaccaagaccgacttgctggccggtttcaacgagtacttcggctcgctgggccgcgccgagcgctcgcaggtctggggctttacctttccgatcgacgccaacccggcggacccggccaaggccgacctgcgcgagcgcttccaccaggaatacaagctgctgcaccagcgcctggacgagcgcctgcccgagctgctggcggccgagcccgaccagatgcgccgcgcgcaggcctacctgctgccgcagcagttcgcgagcttcgaggacatcctcggcaccttcctggccgacgtgttcaacccctcgaagttcgaggtggcgcccatgctgcggggcgtgtacttcacgagcggcacgcaggagggcacggccttcgatcgcgtgatgggcgccatcaagcgctacctgcaggtcaacgcgccgcccgcgccgccgccgggcccgggcaagagctacttcctcaaggagctgctgcagcaggtgatcttccgcgacgcgggcgtggccggcaccaacctgcgctggtaccggcgcaagcgggccatcgacctggcgggctacagcctcatcggactgctgctggtggtgctgctgggtgccggcatcaacagctggcgcaacaaccgcgactacgtggccgaggtcgacaacaacgccaaggccttcaacaaggccgcggcgcgcggcgagctgccgacggtggtcgattcgaacagcgacatcgcgacctccttgccggtgctcgaccgcctgcgcgacctgcccaagtcgggccagttcgacatcggcgatccgcccgtcggctaccgcttcgggctctaccagggcgagaagctccaggccgcgaccgatggcgtctaccagcgcgcgctcgagagcgtgctgctgccgcaggccgcgcagcgcgtggagcaggcgctgcgcgaggcctcgaagaccgatgccgaatacagctacgaggcgctcaaggcctacctcatgctgtatgacgcggagcgctacgacgccgacttcctgcaggcctggctgctcaccgacgtggaccgcaagatcggcgcctcgctcacgcgcgagcagcgtaccaacctcgagacgcacctgcaggcgctgttcgcggggcgcgtggtgacctcgccgtttgccaaggacgaccggctcgtgaccgagacgcgcggccggctggccggcgtgccgttggcgcagcgctcctatgcgcggctgcggcgcatcctgctgcagaccagcccgcccaacgccttcagcattgcggaggcggcgggggccgagtccgcgctggtcatcaagcgcgccagcggcaagccgctgaccgacggcattccgacgctgttcacctaccgcggctactgggatatcttcgacaagcgcatggcggaaaccacgctcgcgctcgagcaggaagaccgctgggtgctgcagatccgcgcgccgggcatcaccgacatcacctcgcgcgagctgctgctgcgcgaggtgcggcggctctatctcaccgactacatccgcatctgggacgagtacctgaccgacgttcgcctggccgacagccgctcgctgctgcagagcatccagatgacgcgcgtgctctcgacctcggagtcgccgatgtcgcgcctcattcgcggcgccgcgcgcgagaccgacctgctgcgcaaccacgacgaggccgcgcgcagcctgctcgaccaggcgcagaaccgtgtggccagcacgcgcgagcgcatcgagcagctcatcggccagcccgacggcagccagcgccgcaacaccgcgccggaccggcccgagtcgctggtggacaaccactttgcgccgcttcgccgcatggtcaccgcgcccaaggccggcgggcaggcacccatcgacgccacggccgcgctcatcaacgagctctacacctttctcacggccaccgacacggcactgcgcagcggcaacatcccgccttcgagcgatgcggtgaccaaggtgcaggccgaggcgggccgtctgccggtgccgttccagggcatgctgaacgacctctcggccaccgcgtcgtccaaggcagcggccgtgacgcggcagaacatcgggcagagtgcggccgccaccatcgggcagttctgcaaccaggccatcgcggggcgctatccgttctcccgcggctccaaccgcgacgtggcggccggcgactttgcgcagctgttcgcaccgggcggcatgatggacgacttcttccagaagaacctggcctcgcaggtcgacacctccgtcaacccgtgggccttcaagcgcagcgtcgacggcagctcgcagggccgctcggcctacctcgattcgttccagaaggcgcaggcaatccgcgacgtgttcttcatgggcatggcgggcggccgcacgccgtcgttcagcatcgacatccggcccgaggacatggacgccgccatcagccagttcacgctcgacatcgacggccagacggtgcgctatgcgcacggcccgcaggcgcccagcaccgtcaagtggcccggcccgcgcaacagcaaccaggtgcggctgcaggtcaccaccgccaatggcacaccggccggtggcatcgtgaccgaagggccgtgggcgctgcaccggctgttcgacaaggcgtctgtctcggcgggcaactcgcccgaatcgttcaacgccaccttcgacctgcagggcaagaaggtggtgctggcggtgactgcgaacagcgtctacaacccgctgcgcctgtcgcagatgaatggcttctcttgtcccggaaagtcctgacatgaacagcggcattcctttgccccgtgtgtgggtgccggccgacgagcagatcggctggtacggcaagctgccggcggccggcgactttctctatcggcgcatgccgcgcgagctccaggcctggtgggaccgctggatgcagaacggccttggcgccttcaagcgctggcccgacgccatgacgcggcactacgtcgtcgcgccggtctggaactttgccattcccgcaacgcagggcgtggacgcggtgcagttcggctgcattgcgcccagttgcgaccgcgtggggcgctactaccccgtgtgcgtgacgctgcaggtggcggcatccaactaccgcccgtccatgctggagggttccgccgcgtggtactggcagtgcggcacggccttgctgcaggcgattcgccacagcgttccgcccgaccagttcgaccaccaggtgctggccgcggcccatggcggcttccagactgcgagcggcggctcggacgacatcctttcgatcctcgggcccgcggccggaggcgtcggcgcgggcgcgcagcagcgcctcggctggcccgagcttccgctgtgcttcgatgccttcggaagcaccagctactggtggaccaaccaggcggacggctcgccgctgcgaaccgccgcgcacggcggaggcctcaacacaccattgttttcgaagttgttttcacaggggcatgtgccatgggcatgaataacgccagcagcagcaacaccagcagcagcgcgccggccgatccgcaggagcggccccatccgctggcggcgggccatcggctggacgagttcgaactgctcgaggtgatcggcgaaggcggcttcggcatcgtctaccgggcctacgaccactcgctgcagcgcgaggtggccatcaaggaatacatgccgtcgatgctcgcgcgccgcgtgggcgacgacagcgtgcacgtgcgctccgaccggctcacggccaccttccaggcgggcctgcgcagcttcatcaacgaggcgcgcacgctcgcgcagttcagccatccggcactggtgcgggtgcatcgcttctgggaggcgaactccaccgcctacatggcgattcagctttatcgcggccgcacgctgcggcgccttgccgaggaagagccgtcgaagatttccgaggcctggctgctcggcatgctgggcccgctgctcggcgcgctggaaacgctgcaccgcagccagtgcttccaccgcgacatcgcgcccgacaacatcttcatccagcaggacgacatgccggtgctgctggacttcggcgcggcgcgcaagtcgattgccgacctcgtcgacgaagtggcggtgatggtgaagtcgggctattcgccgatcgagcagtacgccgacgacaacacgctgctgcagggcgcgtggaccgacctctatgcactgggcgccgtgctgtatcgcgcggtcaccgggcatccaccgccctcggccgtggtacgcagcgtgcaggacgcctatgtgccgctgtcttcgctcggccgcggcgacctgagcccgggcttctgcgcggcggtcgaccacacgctggcggtgcacagcaaggaccgcacgcagaccgtggccgcattcgcggccgagctgggcctggccaaacttggcgacacctacgtgagcgggctgccggcgccgacggtcatcgttccgccgccttcgaaggcggcgccagcagtggtgcctccgccgcagcaagcgccggccgcgcccgccaagcccgccgcggcaccggaagccgccgcatcggccggggtcgtgcaagccaaggccgcggtgcccgaaccggtcgaggccaagtcagagcccgagcccgaggccgaggtcgtcgccacggccaagccggctccggcgccttcgtccaaggccgccgcgccgcgcgaggtcgcagtgccggcacgcgccccgtcggcagcggccaagccgctgccaccgttgtcgtccgccaagaaaaaatcgtcgcgcccgccgtggctgctggtcggcgcgctgttgatcgcactggtggccgtgggcagctggatcggacttcgcctgggttcgtggaagcaggagacttcgaccgcgatggcgccggtgcctccgccttcgggcccgatgtccgccaacgcgccgcctcccgccgccgtgccgccgggcgatggcggcacggcgcccgcaggaggcaacgtggccgcagcccctggcggcgccacgccttccgcgccggcggccagtgcgccggccggttcgttgacgccgctggacagcgtgccggtcattgccccggcgccggcagcgcaggccaacgcggcaacaccggcgacgccagcgacgtcgccaacggcaccgacagccgccacgccggccacaccggccatctcgccggaggccgcccttgccaccagcgaggtcgaagactggaacctggcacaggccgagaacacgcgcgagggctacgaggcctacctgcgccgctaccggcgcggcctgcatgcgcgcgaggcccgcaatgcgcttgccgagctgaaccggctctcgaccaccgtgccggcggcgcccggcaccacgccgacgaacgccgttcccaccgtggtggcgggcggcgccacgccgccggccacagcacagccggccgccccccccggcatgggacgcgtggtgctcaacatacggccctggggccaggtcctggtcgacggcgccgagcgcggcgtgagcccgccgctcaagtcactgtcgctgcgcccgggcatctacaacatcgaagtgcgcaacggcgacctcgacgtgtaccggcagcgcgtgacggtgcaggacagccgctcggcgcccgtggtgagccacgagttcaagtagcggcgtcggcgggagcccggcgccagcgctgcgcggcgaccagcgccagcaccgcgacgacgctggccgccagcagcacccagaggccgggcgtgtagccggcgtccggctgccacatcacgccgagcatcagcggcgccagcgcgcgggcgatggcgctcggcaggcccagcgcgccgttgagcgtggccacgtgctcgcggctcacgtactgcgcgatggcggtgcccttcacgatcgtgagcatgccgttgcccatgccgtagaagaacacgaacagcagcgcggcgcccggatgggccgcacccgcaagcagcgccagcaggccgagcggaatcaggcagggaatcagccggttcgcaagatgcaggtcgaaatggtgctcgaagaaatacagcagcgcccgtcccagcacctgcaccagcccgatgctcgcgggcagggcgatggcccacgactcggcgagcccggcaccccgcagcaggctcaccatgtgcggcggcagcgcggccgtgaccgccatcagcagcacggtgaacacgcccacgaacaggaaaggcgcgctgcgcatgtggtgactcgcggaacgcccgacgggtgcggcgccggccacgctgccggcacgtatggccacgggcgtgggagccggggcatgccgcagcacgcgggcatgcagcggcgcacagatgaacagatggatggccgccagcacccagagcgcgtgccgccaaccgagttcggcaatcagccaggccaccagcgggatgaacaccgtgctggccagcccaccgagaaaagtcagcgtgatgatcgcgcggcgaaagtcgtgggggaagcgacgcgtgacgatggagaacgcggggttgtagagcgtggccgccagccccgccccgagcagcgtccaggccaggtagaagccgagggcgccgtgcaccacgctgtgcagcaacaggccggccgcgatgaccagcgagccgcccgccatcaccgcgcgctcgtgcccgcggtcgatccagcgtccgaccggccatgccagcgcgccttcggccagcagcgcaaggctgaaggccagcgacgactgcgcccggcccaggcccagctcgcgttcgaccggctccatcagcagcgcaaaggcgtagaacacgctgccccaggtgatgagctggccgacagacagccagccgaccaggcggcggttgtagagcgtgggagcgggtgggttcaccgcggatcagtgtcgcaaagcccggcggtactgcaccgcctccgccacgtgctccgctcgcaccgactcggcgcccgccaggtcggccaccgtgcgtgccaccttgagcgcgcggtgcgtgctgcgcgccgaccagccgagcttggcggcggcattcaccatgaacttgcgcgccgcatcgtccagcgccgcatgctggtcgatggcgccggcctgcagcgcctggttggggctgccctggcgctgcagcgcgaattcgcgcgcggcgaccacgcgggtgcggatgctgccggtcgattccccggcgggcgcgccgagcagttgctgcgccgagaccgcgggcacttcgatgtgcaggtcgatgcggtcgagcagcgggccgctgagcttgccctggtagcgcaagatctggtcgggcgtgcagcggcaagccttcagcgtcgagcccaggtagccgcaagggcaggggttcatggccgcaatgagctggaagcgggccggaaactcggcgcgccgggcggcccgcgcgatggtgatggtgccggtctcgagcggctcgcgcagcgcctcgagcgcggatcgcgcgaactcgggaaattcgtccaaaaacagcacgccgtggtgcgcctgcgagatctcgcccggccgcgggggcgagccgcctgtaagcgacgtcgaaaaatgcgaatggccctggatctactgccgccaaatgcgaatggaccggtcccggacggtgactggtggttgcaagctgcacttcggcacacccgatgcgcttgcgccctaccgatccgccgggcctgccggcccttctgcagagacattttccagaatcgccacagcctggcgcgcatggaccagcgctcgctcgacgcccccatcggaggccacgttcgtgccatggcgtgctgctattgcacgcaggcagaagttcagcacgctggtcggcgctcccagtttctcgctctcgtaccggctcaggcaggtacggtcgaccccgagcaccttggcgaagtcggtcttcgtgagggggccgcgggcggcctgaatcagttcgctttgagatgcaggaaagggcattgggttgtgcttctattgcacagattgtgtgataatagcacgcgaaatgtatctacgatcaaccccaaagggcagtccaagttgagctggcagagctaatcacagcgcaatatccttaacagcacctcgcggtgcatggtggcgtccgaacgactcctaaccgcatctggaacaacctatgaacgcagaaatcctcaagcgagtggtccgggccatcgcagacggttctcaggaagacttggagcggcttgcgggcaagatcgttgagtccgagcgcaagactgggcatgtcaagctcgcggcccagctcgaggcgatcctgaagcaggccaagccggcacgcgcgcctaccgtgcaggaaagcccggaagttggtcgccccttggcggcactgccgataagccgccgccatggcgagtctttggcaacgctcatcgcgaccgatgcgctcgagcatcacatggtcttgcctgaggagatcgagcaccggttcgcgcgcgtcgaatccgaatatgccgcgcgagacaggttgcgaatttttggcctcaagcccagaaagacgatcctcttgtacggacctccaggctgcggaaagtcgctcggtgccaaacggctcgcatgggccacgggcctgccactgatgaaggtccgcttcgatgcgctggtgtcttcctatttcggtgagtccgcgtccaacctgcgctcgatcttcgacgctgcgcgcgggcgtccctgcgtgctgctcttggacgaatgcgacttcatcgcccgctctcgtacgaactcacgggatgtcggtgaagcttcgcgcatcgtgaattcattgcttcagctgatggaagattacgacgccccgggcctgctcgtggcgacgacgaacatcgaggagtcgctggactcggcgctcttccgtcgcttcgacgacgtgttcatgatcccattgccaggcgcggttgaaatcgaaaggctgctgagggagacgctggcctcggtccagttcgtggagcccatcgactggaaaagtctcgtcgagcaattacacggagcgtcggcagcgatggtcgtgaaggctgcgcaggatgccgcaaaggccgcggtgctgggcggcgggcatctactaacccaagcgcacttgcgacaagctatcctcgagcaacggagacacgagaactccgctcgaggagagtagggattgccaggtaaccataactttgagcatctttctttggttcgacgttttgagggcgaggcgaagcttcgtggtaacggcaagccatcgcctcagacgcttgcgaataagcaatttcgtgccgcacataccgctacgctgacgcaagcggcggaccgcctggctgcaaattggcaggcgcgtctggagagtcgaagtcgtgcaggcgatgctgttccgccggtaccagctgggtttccgatcctgctcaagattgatccggacctcgaaatcgaccagctgcgatccgccttagggctggagatagtttgtgagcaggaagacggctatgtgatcgtggcttccgaatccatcgatctggccgtgctccgccgaaagatcaaggacttcggtgtcagcattcacgggtccgccaccgtcgcaagcgtgcacatgctgttcgacgatcctgatcagcaggagcggctgggtcggatcctttcggatcagttgatggaggcgtggggagcgatcgacgacgtccagaactatgtcatcgacattggcgtcgcctgtgtcggcaccatcgaaatcccgtcgaagcccacacgcggggaaaccacccctgacgataagtgggacgcgcgaatgcgcgtgtggacaagacggcgagatgaggcttatgacgcgtgggatgtgctcaaaagcagccgtgaaagcgcgctgaacacgtttgtccaagcctatggcggaacgatcctgcgcattcgggatgcaatggatttcgagtcgggcgtcctttccgacagcttctcggttcggttgcgcatttcggggcagggcttgcgcgacctgatcctgaatttccctttcatcttcgaggtcgccgagcctgaagacatcgaattccctcgaggcgcaacgggcaccgctggcgccgctggcgtaggggtagcgccgataccgcccgatgcgggcgcgccagcagtctgcatcatcgacagtggtatccaggaaggacatgtcctgctgcgacctgccattgacactgcggcttcgtacaacttcatgccgggcacgcagccgaccgatgttgccgactatgtctcgggtggagggcatggcacgcgagtcgccggcgcggttctgtacggtgagaacatccccttaactggcactcctcagttgcccttctggatccagaatgcccgcgtgctcgaccagcacaaccagatgcctcaggggctgttccctgcagatgccattcgggcggccgtagagcggtttcgcagcagcgccagagcgacacgcatcttcaaccactccatcaacgcttatgggtactgtcgtctgcggcatatgtcttcatgggccgcggagattgacgctgtgagtgcccaatacgacgtcctcgtggtccagagtgcgggcaacctctcgcccaccggcccgcagcgtcatcccggcatcgaggatcatttgaacgccggtcgcgaatatcccgcgtatctctgcgagccggcctcgcgcatctcgagtcccgcgcagagtctgcaggccctcaccgtcggctctgtgggctacggcgcatactcggggactgactggagaagctttgtgcctgccggcgatcatccggctgcattctctcgctcgggcccgggcatctgggatgttctcaagcccgaagtggtcgagtacggaggtgacttcgttcgctcaaccagcggtgcgcacgatgtccgcggaagtgagggcgtggcatgcccgccactcgtcaggtccacgatgtatccgccagggccggcagccgaccgggacgctgcagggacttccttcgccgcaccgaaggtcgctcgtattgccgccagggttcagcaggtgctgccggcgcatagcgcacttctttaccgggcgctcgttgttcagtctgcccaatggccggcgtgggcaggagctgtccatgccagacttcagaacctgcgggcttgcaagagcaagcctgccaaggtgaagcaagaattggccgcgctgcaacaggacgctgcagcgattctgcgcaccattggattcggcataccgaatgaaagccgggcaacggaaaacgatgtgcaccgcacgacactgatcaccgacgaggtcggattgatcaaggcgggggagtgccacgtgtatcaggtgccgatcccgaattccatgcggcggccgggcgacgagtacgaggtgcgggtcgatgtgacgctctcgtacgcagcgcagcctcgtcggactcgccgccgtttgaatcggtacctttccacgtgggtggattggacgacgaacaagcttggccagggcatgaacgatttcttaagcaaagcgacgaaggatcacgtcggaacgatggaagaccttgaaggccaagttttaccttggacgctgcatgaggctactcatgcgggtgtcatgcatggcgtccggcgaaatagcgggaccgttcaaaaggactgggcggtagtgaagtccaacacactgccggaccatttttgcatcgcggttcgtggccacaaaggctggagtcaggaccctgattcgacggcgaaatatgcgctggccgtcactttcgagatcgtaggtaaggaaattgagatctacgatgccttgcgagtcgaggtcaacgaactgcgtgcatccatagagagcgagatcgagagcgagctcgaataacggggtgggtgatcgtggttattgtgtggcgtggtagtgcgccatctcgccggcatctgcaaactatcggcggcggtttctagcctatcggcgcggtcccggcgccagtgatgagcgctttcagcgggcgcttcaatgggtcgagctcatcggcgacgtccaatgcaaggcggatccagtcttcgaactgaggattcccttcaggccccaactctggatgagtcgaaagcacaccaaccatctctcgaatatccagcgcggctctgtgttgctggcccaggtcgatgatgcgctcccgaaccttccttcggttcgctgcgatcgcttccacgcgttcagcttccctggcacgctcttcggcttctcgcttctttgcgatctcgacgcgccgcttgaccctttgctcgtacgcgaactgtgcaaagtcccgcatggccagttcggctcgctcgagcagtgtgcggatgatggccggcagttggctctccagcttttcgcccggcttgtccgcccattcaataacgccaagcgaactcgattcagtcccgaccctgagcgtcgtcgcatcgactttcttggagttctgtgctttcctctgatggaccgaggtgtcaggctcgatgatcaagagttcgagccggcatcccccaaaatggagactcattttcaggaaatggagggttccaatcccctggacccattcgtcgtaattgagaacttccaggccagccgtcacaggcgtcaacgcacgggcaacgctgttgaagatcctcaactggcgttggtgctgcggcccatcaaagtgcggcttgtcaaaggtccattcgcgttccagagacttttgacggcgcctggcctcggcgtcgagtacgcgcttcagtgcaccatgagggctcgacagatctcgacatgcggtcaccttgccgatgatcctgatcgccgcggtcacctgctcgtctatctgctctgcgaactccggagcggcaatggcctcggtcagatcttcatccattgaccaactgctatagccgcgatctccgaaggtgatttcaactgactggcctgggaggcgtatcggcaacggaggacggcgcccagccttgccaaccgccttcctcgcccaatagccttgcggtggccccgggatgtgagaccggacgcagagctttccgatcgcaacatcggatatccccaggtccttggcgagggtcgaacggggatgggtccaaacaagttcgtagagctcggttcgagtcagcgtcttcgtcatgactgttgtgtcaacatctgggcagtttggtttgcggcatattgttccaacaggaggaccgccttggcaaatacagattccactcggctggcagttctgatcgatgcggacaacgcatcttcctcggttgtgcaggaactgcttgaagaagtagccaagtacgggacggcgacggtcaagcgcgcatacggcgactggacgaccaccaatctgaccggctggaagacgcacctgcatcgccatgccattcagccaatccagcagtttgcatacacgcaaggcaagaactccacggattcggccttcatcatcgatgcgatggacctgctgtatgccggcaacgtcgatggcttctgcatcgtctcgagtgacagcgatttcacccggctggcaacgcgcatgcgggaggccgggaaggtagtctatggactcggtgaacgtaagacgcccgagccgttcattgccgcatgcgacaagttcatattttttgaggttttgaaaaagccattggaatcagcggcgcctgttcaggttgcggacgtcccggatctcaaggtgcttctcgtaggggcagtcaaggaaaccacacgtgatgccggctgggcttcgctggcggcagtgggcgggtatgtcggcaagaacaatacctcgttcgatgctcgcaactacgggttccggaggctcagcgacctcgtgcgcaatcaggaatacctcgaggtgaaggagctgcctgatgcttcaggctctatacatctgctcgtcaagctgaaatagggaatgttgcactcaagcagccgtgaactattgcgtgcctacgcgcgccgcaatctcgcgtgccccgagatctcgcaccgccgcaaggttttcgagttgtgccgctcgcggacgagccttgccttgctcccagtgatagatcgtctgcccggatacaccaaccagttgtccatagatcgctgcggacagcccaaccttggcgcgatgtgccgctaacctggttgcgctgaatcggcgcttcgttcccgctgaagcctcgccgtccgaatccggggccttggcggggcgcgtcaccccttttgcaatccgacgcagttccttctcgagcgcatccacttggcgacgtagttccgcaattgatgcgcgatgggcgacggatgtctttttgagtgtttcgatctcagcgcgcacttctttgcgagcaacgcgggagatctcggctttgaggatcgaggcgatatttggcataggggaattgtgccgctgcattcccgccttgccagtaggcggatttccttagagcagatgttcccacgaatccacgatcctctcgtaaacgtttaaggaactcggatatccgcagctatccagttagactgaggcgcataggcatgtgtttcccaataactgtgggaaagcagcgccgtcctgtgtgtcacccccgatcaaaatccaaacggagagggagaagcatgactggaagtaagagccgggcacgcacccggccacgcgttgaggctggcgcgacgagctcccccgcgaacacgggctcgggaagtggcggggcgcccggtggcaaagctgcttctggggcctgtaccgaactcgcagaaatcgtgatccttatgtccccagaccctacggtgctggtggacgtcaagccagatgaccagctagttgtggcgcgccagggcaggtccgttgtagtcctctatcaagggcgcatcgcaggttcgatagtcgcgactgatctcattcgactcattagctgtttggaacacggattcaagttcacctttaccgtactcacagtttccggcggtcggtgcgagggagctcttcgatgcgtcggacgatgatgaagatcgtcggtggcttctatggggaacggatgatgcatcctcatcatgaggcctcgttcggctccggactccgtgcggcggccgctctcgccaaattcagtgatggcatcgaactcttcacgtacgcaaccgacgcacagcgtccggaactggaggccatcgcgaacaccttcaatgtctccgcgcacgtcagtgagcgtgctcaagcaattgagttcgactacctgcacggttgcgtgtctccgagcctctatcccgacttgcgcaagattgaaaaggcggagccaatcgcagtcgagggtgaaatcgtcgtgcggtacggcatgctcgaaggctcaggaaccgtagacgccaaatgggcggtgtacgacccgcaatcggaggtggagccagagccgttcgggctgaatggctcgagggccaagcatctggcgctggtcctcaatacgtcggaggccttcgcactttcaaggacctcagatctagagtcggcagcgaaagtcctgctgaccggccctggagcagcgacagtcgtcgtaatcaaggccggcgtgcgcggcgcatacgtctgcaccaagaaaaagcgctcatgggttgcgccccgcaagacgccctctgtcttcgcgctcggttcaggagatgtattcactgccgctttcgcgttcaagtgggctcacgaacgacaaccccctgtcgaagcagccgagtttgcgtcgctggcaaccgcatactactgcgccaatcaatatctacccctccctgtcaatttcgagcaagaggcgagtcgcagctacaagcgtctgcagccgcgcgggacgcctgggtccgtctatctggcagctccgttcttctcgctaggtgagcgctgggtcgttgagcaactccgaaatgccctttgtgaccaaggcttccaggttttttcaccgctgcacgacgtgggcatcggcccgccagagcacgttgcgcctgcggatttgaagggacttcgcgacgcgagcgtcgtgctggcttgcgtcgacggggcagacccgggcactgtattcgagattggttacgcccgcgcgaaaagcatccccgtggtcgcactctccactgcaccagggaacgacgaagatctcacgatgattgctgggagcaagtgcgtcgtggtgcgcgatatcgcttcggcgatctatcgcacggcttggattctggctgaaagacgcaagtgaacgcggtgctcctgctttcaggagggatggattccgctgcactcgcctattggcagcgtccggcgcatgcgttgacgattgactatggccaggttgccgcggaaggggagtttcgtgcagccgtccagatagcgcgacagctcggaatcacgcatcacgtcttaacgctcgatctacgtacgcttggtctgggccggatggcgggacaacgccccgactcaggcgctcctacgcccgagtggtggccattccgaaatcagttgctgatcacgctggccgcggcaaaagctgccaccctcggtgttgatgctgtcatgatcggtacgctcaagaccgatggccttcacgcggatggtcgtcccgagttcgtggccggactgaatgacctgctgatgctgcaggagcggcacatcaggctgatcgcccctgcgctgaagctggacgcggtcgaacttgcaaggcgtgcccgagtcccagcgagtgtgtacggttggactcactcatgccacgtagccaaccacgcatgcggtctttgcaggggatgtcagaagcatctccagacacttgcgcagcttcagttggaaagcggccagtcgaagagttgatgctgcttgaccaatggtgctgttgcattgggagcgggtttgaacgaactcggtgttgagggctgcttcacgggggcgtattcctcgatgatttgtgggctgagctggcgcatcccatcccacatgactgcatccagccaagacgccttgacgttgagtgcgcgcgcaaagcggatgaacttctgttcgagctcgcaatagtggcgactgacatctgcagcagcttcgaaaaggccaaatgcctgacaggcccgcacgacgtgaatatcgaggatggcgacatcgtcgcttccgagccagttgcgagtgatgaaagacgacgtcttggggcccacccccggcagacggcgaaaccatgcccggaaagaggtggcatcttgttcatcaggcctgccttcccgtagtgctttcaagcctgcgctgagatggcgggatttcgtgcggtagaaccggtacctgattttccgcccatcgacatccagaggcttttccagcagttgtgtaattgcatcttcagaagagtcgctggtgccatccaataccccggactccctgagtcggcaggcagctgccatgccgatttcagcggatatgccatagccggccaaaacgcaggttgcatactcttcttcaagcgtatcgcccatgcgaaaacggtgcgaatcgatcgagtccatctgcgcgttgcattgaaaggcccaggatgcaggggtgagcatctcgtcgacgcgcccccaagcgacaccttccacgaccagctgatcgggttcgggaaggtctagcgacctgagctcgtcgttcaagcggaaaaatgcggtttgggtcatgtggcccccgttcgatcggcaactcgttcggaaagccatgcggccaagcatgcgcgctccacatccggcagacgttcaatacgcgcctgaagattcgcgactctgcgcctgatggcctcccgctcgcggaaatttgatccgaggcacgagtagtcgtgcagttgcgcaggcgcgtcgaaattcatccacaaggtctcaatgcggacgccggcgtgagttttggaccggaaagttactgtgcgccagtcgcacagaagctcatcgtagagatcacttgcataacccgagaggatcactgggccgggtagtttgcgcagcacggtgagaaggtcgatgtgctgttgctcggacatttcatgtcgatacacacgctcactgcgcctcgtcgagcgaaggtacggggggtcgcaatagacaagttcatcccccttgaagcgctgctgttgcaaccaggtcgtcgcgttggaacagattaactggcatggctggtcgagatcttcacgccgcgcagcgatgacctgggggtcgatgtcgatgccgatggactctttggcgggcctctttcggcgcatgactgctccccctcccaaatgcgtctcgacgtagacgcgatgagggggcatgcaattgatgacgtgagggaaggtcttgccttttccaccgggatagcgcatgcgaaatcatcgcgaaatccggtgatgatgtccagtgatttctagcgcgcccgttgatcgcgccggatcctggaaagctgtattgcggcacgacagagacggcgctgcacgccatccaaagcaacgtgggcgagcaccgacatcccggggaagcgatgcaaatgcatcgaggatgcccattcgtctaccggagctgttgccccggggctatgctgagcgcgggctacacactacaatcaaatgccgtatcgaggagtgtgttatgaaaacagctgaacttgccgttgtggccaatgctcgacgtgccgcacacagccgttttgatcactacaacgctgtcatgaatgcgtcgaagccatctggaacatcgacactgccagcaaaaaaagagaccgggaaaccagttccagtcccaggtaaaccatcgaagaagtaaaagcaggccacccgcgggtggcttttttttggagacgagggagatgctctacgacaaggctcgcgacttcaagcgtgcaaagctcgagaaggaagaagacgatgttggccgctcagccttccgtcgtgactatgggcgactgctgcactcgccgagcttccgacgtcttcaggggaagactcagttgttccctgggcatgagtcggacttctttcgcaatcgactcactcactcactggaggttgcgcagattgcaaagggaattgcgcaactcctcaattccaaggaacccgcattcaagcgtgatcccattaatgtcgatcttgtcgagttcgcaggcattgcacatgatttagggcatccaccgttcggacataacggagagcatgctctcgacgactgcatgaagaagaatgggggatttgagggcaatgctcaaactcttcgaattctcgcgcgcgtcgaaaagaaggcacttcgagctaccgaggacaaggacgtctgcggcatttctgtagatggtagtgatcgacgactaggtctgaacctcacctatcgcagcctcgctgccgtgctcaagtatgacaacccgattccactgcgacgcaacaaaggggcgtctctcgagaaggggtactacgccagcgagaagcagttggtcgaaagcatcaaagagcatgtgggagtaccgtcatcgggtggaccattcaagaccatcgagtgtcagatcatggatatagcagacgacattgcttactccacctacgacctggaggatgcgatgaagggcgggtttgcgcacccgcttcagctgcgtgcgaaggttcttggcagccctgaccttattgcgaaattgctcgcgaagatcgcgccagaggttccgaatgtcgaagaggccgaggtctttggcgcaatcgacgatctgctgaatcttgatgaagtcgactcccatggagcaagcagcagcctcggaagctacgagacgtccaaactggttgcgtcggatgggatgacgcgatgcgagttctcttcggaactcgtgggacgcttcatgcgcggagtgcgcgtggagatgctgaagggcaaggagatccgattctcaaagatagttgtcgatcgtgatatccgcatcaagatcgagacgctcaaacacctgaacttcctgctgaccatcatgtctccccgtctgaaggtggtggagtaccggggctatgaagttgtgagaaccatattcgatacgctggactcggaagagggccatctgttgcttccggatgacctccagctcatgtatggacggctgactgatactgactcaaagcggcgcttgatctgcgactttgttgcaggcatgacggatcgatatgccgttgagttctactcccgattgcgtgagtcaggcgcaaccatcttcaagccgttgtaagggccggaactccccgcttaggctgagcaggaggtactgtggattttcttctatcgcttccgaaaacgctactggacctggcggttggtctcctgaagatcaagaaggatgaccgcacgcgtcagcgacttgcggatctacttgcgtctgtagctgattgcgcatcaggaatcgctgacgcgatcgagaaaaacgaacatccaaccaagctctgcgcagagctggacgtgtacgtcttgaatctcgaaaaatttgtccttgagcagacaaatcaagaggtcgcgtcgaaactcactctgtggttgaggcatatcgccgatgtcccggggatcgcgaagattgatctcgcgaggctcgtcgagagcgagtcaaagccaaagtggactgcggtgcaaagatttcagcaggctgagaccgtccgacacattgctggcttgattgcagggacggctaacttggtgcgggtatgaagcgctatgaggtcggaggatcaggtccagttgttcttagtgtgattctcgcgacagtcgctccgcaatctcacgcgcaccgagcgcgatgacgcgtcgctccattgatcgcggcctctgtgtagttcggttcattgatgccccttgtccaccgcgattcagacggggatcaccaattcaggattgaaatccttgttctcgatcctgccgctccagttcacatagccgcgcggattgcacacgacctggcaagaacgggtttgataattgaacgactgatgtgtgtggccgtgaacccagagtacgggtacatcgaagaaggtttcagggagctcggtgacgaaggcgcccgaggaccagtcatcggcgtaacgctgcgccagtgagccgcgatgaggcgcgtggtgtgtcacgaccactgtcggtccggcgaacggttgtgaaagcctgtctcgcagccacgcgcgctgcgcctgatgaatccgaagcgtgtccgccgcctggagctttcttccttgcttgtagcgccaggtatcaggctccgccgcctcgtcgaacgtgcggatcagcgcgtagtcgttcagcagattggtcgccatcttcatggcgcgcccgacatcgctgaccggcccttcaggcgtctcgatggcgagcgcgaaatcggtccacagcgtggcgccgaggaagcgcacgccgtcgatcaccagttcgtcaccgtcgagcaaatggacattgctgccttcggcttcgcgacgtgcttcagccagtgtcgtgtcgaggcgcccatcgtagtactcgtggtttccgggcaggtaaaccacggacttgccacggaagcgatccgccgcccactggacggcgcgcttcgctggcgaatgaatgtcgccggcgaggatgacagcatcgaactcgagatcaggcaccggatcgaagggtgcgaactcgagatgaaggtcggaaagaatcagcactttcatcgggacacctcgtcaaagcgcgcgcgaagcccggcactcactttctagtcgaagccggtgaacgaaccacacaccaccaagtggtccttgcagtggtcgaactgccaataggcatcgtcgagtgcgacccaaggttcgtcgaccgcatcgtggatctggagccaggcaaggatttctccttcacgcttcccgtatggcggtggaaggccaaaacccgaatgtggcgtggcccccagaatccgggcccggatgtcgctggagaacggcttcagcagagtctcatagagaagctgctcacgccaggatgaactgatcacaatcatcacgtgcgggaactcgcgcagcaacgcctccaggcgtggcaggaagcagaagtcagcgccgccgttgagggcgtgatcttccccctccggatgcagcacgccgtcgaagtcgagaaacaggatcatcctgaatctcctagcccatatccatcggccctcatacgacaccgccgtgttgaatcgcgatcaggatcgatcgcactctgtcagcgccgcccccgacagcaaatgccgccggcgtttgaccgtcgagcagctcgtgcggcttgtcaagccaggcttgggccgctgcgccgaatacctgagtagcgagatcgagcacgtcttgtagaggccctcccggcccaggctcatcgcgcggccacgccaggtgtgagcccatgtcgaccccgacggcgcgaaacggtgccgcgttggtctgcattccctctgcgagatagtcgatgttttgatgatggtgaccgtggaccaccagttggacaccgagcgtctcggcgagctcgtcgatcactcgccaaccgtgcgggtgaaccgcaggcgcttcatgcgtcaccaggatgtcggcagattggtgcctgagcagttgttggaagtcggccgggaagatggaggaccggtgcttgcgggcgatgccgtcgcgccaccgttcctggcgcttcatggtgcggcgcatggcgtcgcttgactggaacgccgcctcctcgatcggtcgccgcggatcccagatcttgctacggaagatgccgcccaggcccgcgaccttgaacccggcaatctcgacaacctgcgcgtgcaggttgcgggtggcgaggtccgatcccaacaggttgtcgtagtcggcgtcggagtctgtgtcgtggttcccgtggatgaaccagatctcggtgagatccaggatcggcctcagctcgacgtgcagaggccggcgcgcctggatgtcgcccagcagcacgatcgcctcaggctgaaagcgctcgaccgcggcaatcaccggatcgagatcgccgtgcgggtcgccgaagaacatgagcttgggcttcgactggttgtgctcggatcgcgcatggaggtccgacgagatgagcggtttcatttcatatgccgaacggcggttcatcggccagccgcgaaccgaaggaagtgcgagcgcagttcctggaagctgtcctgatcgaatgcccgcgcgggatccgtgagcacgagccgcgcgaagcccgcttcgaagttcgagggccaatcgtcaagcgcaacccactctgcatcactacggccgttcccgtcgagccaggcctggatctccagctgacgacgatggtggatcgccacatgaggagcaatctgaggcgtcgcgccgatgatccgatgccgaatgtcagcgctgaaataccgctgcaactgctcgatgctctcggccagtcgccaatccgacgagatgatgacgtcgacagactcgaactctcgaagaagcgcttccagccgcggcaaatggctgaagaacctgctgctgaacgagtagtccacgccgacaggatgaagaacaccatcgatatccaggaacagcaaatcgttggaatcgcccgtgtagccggtggcatcatgggtcagcgtcacttctgccatgggtagacggcaagcaaagggcttcatcatccaataaacccggcctggaaggactcaaggagattgagcacgtcggcagctcgcccttcggctaccagcgactcggcggtcctgttgtcaaacagcgcgagtggctcgttcctgtaccagagaatggccgcctcgaggtccccacccgagaccgcagtcgcggcagccagcacttgctggatcgtgtgggtagatgactggatgtcactcatagatcgaccacgagttcggggttgaactgcttgttctccaggccgcggtcatgccgcaagtacccacggggattgcacaccacccggcagttgcccacttgatagtcaaagctctcgtggatgtggccatgcacccagagtgacggcacttcgaagaaggaacttgggagctcgctcacaaaagatgcggacagccagtcggactgatagtgccgcgcgagagagtttcgatgcggggcgtggtgggtcacaaccaccgttggcccgtcgaagggctcggccagcttctgcgccagccaggcgcggtcactctggtggagcgccagtgtgtcctcggggaccaggcggcgctttcttgacttggctgctaccacgggtgcgtcggaggattcctgcgcctcggcccaccggatcgatgagtagtcgttgagacggaccttggccgccttcgtggcccgttcggtgtctaccagcgaccctgtcttggtctggatcggcagttcgaagtctgtccacagcgtgcagcccagaaagcggacgccggcgatcacggcctcgccgggcgccaggagatgcacgttgcacgaactcgcggtgagcgccatttccttgagcgaggtctggaggacaccttcgtagaactcatggttgccgggcacgaacacgatgggggctgtctccccaaagttccccgcccgccgggcccagcgcatggccttggaaccggggacgaaaatgtccccagcaaggatcactgcgtcgtagtcgaccttcgggacgagaaaggtcccgaactcgaggtgaaggtccgaaaggatgagcagcttcacatcggtaggtccattgcttcagcagcgcattcagggcatcaggatcgagagcttggcgttccatgcctcgccgtcggacctggagggcacggcgacgcggatcgtcgggcgatcgaagtccctggtctcgaagaggaagtgcacgtgctgaaagcgaagcactgggttcctgggatattcggtccacttgagctgccaggtgttgaagtactcgaaatcgacggttcgggctttctttccaccgctgacgatgcaggccttgcgcgcatccggatcgaacaggatgcaggtttcatcccaatcgcccagcatgcggcggggatcgactgggaaaaaggtcgcgccagatgcctggccttgtgctcgaagcaattgctcgcgcccagcctgaatcgaccgaggcgatgcaatccaggcccagtagaagagaaccagtgcgactgcgagcatcagcagcagtgggagtgtcatggtcggatattcctgttgtgggggcggccccgcatccatcgcaatgaatcttccggtgagtctgcgcgcctcaacgcctcggcccggaagcggtggtaaaaatcatatcaaaaagatacttatagtccgcgttctaaaagtccgcgtacctattggccgtagtgctttagaccgcgtactccgaacatcgcgacatgactacgaagacgcgagcggccgctcagaatcccctggaggtttttggtgccggggtgcgtgccgaacgcaaagccaggggctattcgcaggaggcatttgccgaccacatcggcattgaccggagttacatggggggtgttgagcgaggtgaacgcaacctgtcgcttacgaacatcatgcggatcgtcaccggactggaaatgaagccatccgagttcttcaagcacttggacggatcggtacgcgccaagtaagggcgcgcgccgatcggtcgcggacacggggcgaactcgttccgctggctgacggtcacgctgcgcctcaatgccaaaacgcggatgctgtgatgcaagcgacctaccggtgaagtcgtaggcagaggcttcggcacgccaggtacatgaagcaaatccttacagatgcgcatgtcgccaacctagcggactgagctctcgatttgcgatcctttcacgaggtctcaactcaacacagttcgtcatgcaaccaccccagccatcgcggcgtattcccgtgtccgaaatcagcatgacggggaagttgaatgggcaagggtacgagtctgcgcttgaacgcgacttcctgatgcgcatggcctgggagtccgaggtcgaatggttcgtcacccagccgttgacgctggagtacgaggtcgcgccgagtatctggattccctatacaccggacgtgctgacctcgttcgtttcgcgtaatggcgtgcctgtacgtcgcccccttctgtgcgagatcaagtatcgagaggaactgacgacggaatggcggcggctgcgacgcaagttccgggccgcgaagtcgtactgcgattcccgcggatgggattggttggtactggatgagcatgcaatccgtggtccagagctggacaacatccgctttctttggtcgtaccggcacgcggcgatgtacgagcacgaggtcgcgccggtccttgacgcccttgctcactttccgagcgcctccttgaccacggtcaccgaccacctccgtccgacggcttcgcgacgaagcgaaatcatctggacctggtggtgcctcgtggccggcaagcgcattcagttcgatatcacgcaggccattcgcctggacaccctgttctggctgccagacgcgcaggcctgacatgagtgccgtcgctgagtttcgaacgccacccgggacaccggtcctcctcgggcaggatgtcctcgaggtggtcgactacgtcgacctcgagcacctggtgctcaggaacgcgcaaggcgactttgtcaccaagcatctgaacgaggtgcgccctgtgcggcacgtcgggcgcgagcgcaagatcgatctcgccagaatcgacccgtctaaatggatgcgggcggaagagatctaccgcaatatcaaatatctgttggaactgcccgaggccgaacgcacgctcaaagaggtgcagaagatcgctacggtggtggggcggcaccattcgacgatctatcgctgggtcgagaagtacaagaagtcgcaaaggctgtcatgcttgcttcggccggaacgcgaggatgcaggcaagagccgactcgaagccgaggtccttgaggtgatggacgagtgcatcgacaagcactacctcaccgaaaaccgcaagtccatggcgacggtttcgcgcgaggtcaagatggtctgccaggcgcgggggctgcacgtgccgcacatttcatctctgcgcacgcgcatcgggcaactcgatccggaggtggtggaggcacgccgttacggaaaaaagcgcgcagaggagaagtttctccctttgatcggatccttccccaatgcggattatccgctggcagtggtgcagatggaccacacgccgatggacgcaatcctcgttgacgatgaagagcgaaagccgatcggccgtgcatatctcactatcgctattgacgtctgtaccaagatgatcgtcggctttgcgatctcgctggaccatcccggttcccatgcgacagggcagtgtctgctcctgtccattctgccgaaggaagactggcttaaggagaagaacatccccgaggagttcacctggccgtgtcgcggattcatgcgcaagatccataccgacaacgcggcggagttccgaggccagatgctgagatacgcctgtggcgagcacaacatcgtgccggagctccgacccaagggaaaggcacgctacggagggactgtcgagcgagcttttcgcaccttcatgaagaagatccatgaggaggtgccaggcacgaccttctccagcgtgcatgacaaggtgaactacgactcggagggccacgcggttatgactctcggagagttggagcggtggttcaccctgtatgtgctgggcatctaccaccagcatgagcaccggggcaacgagaacaagatgtctccccactataagtgggagaagttccatctcgaaggcatgaacggacttcctccgctgggacttccgccagcgatcgagaatgttgagaggctgcggttggacctgcttccctttttcgaggccacagttcagcgatacggcatccgcaactggagcatcgactggttctcccctcgaattcgcgcgctcatcggaaccaagggggatcatggtaatgcgcggaagttcatctgccgcttcaacccacgcgacctgagcaagatctggctctacgacgaccggcacaaggtctacatcgaagttccctatcgcgacatcacgcgtccgccagtcaccctgtggcaggtcaaggccgccaagcggcgtctgcgggatgaaggaaaacccacgacgaacgagccactgatcttcaaggccgtcgagtacatgcgcaagatcgtactcgaggcgcagaaatctaggactgccacaaggcgggctgcacagaggatccgcaatgccgaggccgaacggaaaagggataccgcaaaggccagtgcgccggcgtcggatcggccgcgcacggaagtcaccgagcctccggtttccgcggtgccggagtacgtgccggaaatcgacattcttgaggaactagggggcgcatatgactgaacctgaaaggaaactcgcgccggaggcgaggcaactgctcgatgcaaccgatgaaattcgcatcaatcacatctacaaaacgtctttcttcgaacccgcacgtgtcaaggcgattctggaagagatggaagacctgatgacacgtccgaaggtatatcgtccacccaatctcctgatcattggtgcgaccgattcggggaagaccgaaattcttcaaaagttccgaaggttgcatccggcgagcgcccgtcccgatggtgatgcgatccatgtgcccactttctatctgcaggcgccaccaggaccgttcgaagaaattctgctcaacaaggctctgctccagttgggaatcattcctcgcaacagcatgacctcggcggcgaaaatcccgtgcttggtcgacgctctcgagaaggtcgagaccagagtcctcatgatcgacgaggttcaccagatgctggcgggcgcctccaagaagacgtcgtacatcatgaatctcattaagtacatcagcaacgagagccagatctcgttggtgcttgccggcacggccgccgcacgacaggccttatctactgacgaggaactgatcggacgatttcctgagcgaccgctgccgccttgggagaatgacgctccgtacaagaaattgctggcgttattcgaggccacgctgccgttgcgttgcccttcgaatctctatcgatcggatctggccgcccttatctatggcgagagcgagcggcagattggtggtactgcgaccgtgatccgtgaatgtgcggtccaggccatccggtgcaaggccgaggctattaccgaggggattctcaggaagtggatcgcggacaagcgcgcgcgggaggcggagtgcaagagcatcgtgtagtacgtcgctcctcgggggagtgctattcggtggaggggcgccttactggagcggagccggcgccgttgatgattgtgtcgagagcacgcctcagaggcggagttcatcggcgatgctcagcaccaagcttgcccgcccgtcttcgattcgatgtatcgaagctttggcgaagcattcgggtcaaggtgagggccgccaaatggaaggtcaattgcaccgcgaacgaaagtcgcgccgtgcatacttccttgaaacccttttggcgttaacgcttgggcgaagggggcgctcgacagaatgaatagtctggaactcttgcggatcagtgcgcgactgcccgaactgcatgatgccgagcgggtgaccaggaggccgtcgatctgtcccgccatgcccatctgggagggcaggggtatctggtgaactagtcaccgcggctgagcagttgcagccagcatgagtcgttgccccccgtgcagttctcgaggcctgattctccgtgaagctgccctatgatttcctcgtgcgtgtcgaagtcaagctgccaggaggaaacgaatcggtatgtcgaacaacccgcaagtgagcattgcaacgcagctgcaggcaagtgatgcatttgatgcaacccctaggccctatttccctcgcaggctcagggcgttgggcgagcccaatatggatgtgatccaggacgccgagctgctcgagatcgagcggcctatcgtcattcttggtgaacctggcatgggcaagtcggaaatgattcgccatctgagcgaaagggccggcgcctcacccatatcggcctcgcggttcatgaacagcatgaatcccggcttcttcgtcaacggcaaggatccactttttatcgatgcactcgatgaagccatggcccgttcggcaggcgatgccgttgacaaggtcctcgcgcgtctggaaggtgcgggctgtcctcgattcatcctttcgtgtcgtgcgcgcgaatggcaatccagaaccgagtgcgatctgaaggagatatatggggccagtccactcgtcgtatccatcgaggaactaagccgggacgaggcacgcaccttttggacaatgcgcggtttcgcgagcgatgcagatcccgtgttgaatcggatggacgagcagaacctttcagccctctacaagaaccctctgacgctaggcttgcttggttctgtcgccgatagtggccgggggctgcccactacccgtgccgatctgttccggcatgtctgcgagttgagttggtcagagtctgacgaatcaagacagagcgagccactcgccaagctcactcaggcggaagcactttcggccgctggcgcgatgatggcatcgtcgatatttgcaggggcggaggcgatcagccttgccggtgcaggcgttgctttgaatgaggacattccgattgccgagctcgaggggcttccaggaggtgagaaggcccgtgttgtcatctcttcgaagctgttcaggagtgtgggggcgaaccgggcagccccgattcatcgcgtcgtcgcagagtttctgggtgctaaatggttggctgatcaggcagccacgagccgagctcgtcggcggctcatagtgcagtttcaaggggccggtgcggtgccatcgagccttcgtgggctacacgcctggttggcgtttcacagcccgccgctggctgcggcggtcatctcggccgatccgttcgggctactgcgttacggggaaagtgccgcgcttgacgtggcgcaagcttccgcgctgcttgaatcccttgaagcactcgctcgcgatgacccccattttcgggcgcaggactgggacgcgcgcacagcgttgagcttggcgcagcctgcactcgcgtctcggatcgagtcggcgatcggcgattccacgagcaacgttcacttgcgctcgctcctcctggaatcggtcaaggggtcacctattgtcgagggactttcgcgggagttggaacgcatcgtccttgcggcggatcgttactactcggaacgccgtctggctattgcagctctgttgacgcttcgcggtcgcacattctggcaagggatcattgaaaaattgcttgaggagcgtgccgacgactctgcccgcctggccagaagcttagctgacgacatccagtacgacctgtcggacgaactcttggcaagaactttgttggcggagattggccctatcgatttgcctgcatcgaagacgagaagccggcggccgattcgactccacagattcgaccaactcgctgctgccctcagccccgcacgagccaaagctgtcttgcattggctcttctcgactgtcgcaagcgcctctcccggcaatgttgaggagcatcgcgatttttccaaactcacttccttgctgctacttcgtgcgcttcgaggtggacagatatcgacgagagacgcccctgccttgtggagatggcttgaagcggcaagcaaggaagacctctacgccagaaaagccgaagcgcctctggtctcagagatacgtgcgcgcgatgaattgaggcgcgcggtgcagcgctatggaatctggcgagtgaatcgtagaaaacgactccggcatgtggagtatcagttaagcaggagggcaatttcgatcgctgcggatccacgtgacgtggctttctttctgcaagaaatttccgagcagccgcggatcagccgacggcagcgcaacgactggcaggatcttgtcgacctgagcgttcgccccggtgccgacaatgcactggtcattgacgcagccctcaagttccccaacctgtcgagtagacagcgggtgcatctgagtgcaaagctgcgtccacgcaagcacggatggcagatcgagcaggaagtctatgcagcccagagagcgatggaactgacgacgcaacgcgacgaaaacaatcgcgcttacgaagccaacatcgaagcgatcgggcgaggcgaccttcaggaagtatttgagccggcggaggtctatctgggccgcagggcgtgggatgacggcaacttcgagaagccgctggaagcacgcttgcctgccttcttcaatgagcgcttggcaaaggagttcatggcaggattcgaagccgttctccatcgagcagaccttccgtcgcttgccgatctggcagcgagctacgcggaggggaaggtattcaattactcatacccactcatcgcaggtttgctcgcgcgcgagaagggtggccgtggtttcggagacctctctcatcaagtactccgttcgggccttttgctatgcatggatcgacggtacttgttcggcggcgacgaggatgacctcattgccctccggtcgtcaattgagcgtgttgtagctccgtctatcgacgaaaaaaggcagtttttgcgcacatggattgagccgcttctggctgcgcgccgccaggccgagagcgacattcagttcatggcgcagttgcccggttggtcggaggctgggtgctcgcttgccagggattggctatcgcgctttcgcgatattccgctggccacagaaatggcgatcgtcgcgttgctagccagtatgcgagggggcgaagaacaaatcatcgacgcttcccgtgagcgcgatcatgggatctttcgggacgatgagcaggccttggcctggcttgcgatcgatgtcgtacacagattcgatgaggtgcgggcgcatctcgctggtatcggagacgaaaattccgaattcatctgggagctccgcgacagggtccagtcgcgcaggcgaggttcggccgtggatattgcacctgcgattgcgaagtggatcgtgtcggagttccgacgcccctgtcccttcacaacactcatagatgtttcgtccggcaccaagaacggcttcgatgcaaccgatttcctgcaagcgctcatcgtgcgaattgccgacgacacaagcgatgaatcagtcggtctattgcgcgaactcgccgaggcaccgacggatacgtataccgatgaaatacttcacaggctggctgaacagcgccagaagcgcgccgaagaagctttcaagccaatcgcgccacacgagttgggagctattttgaccagcgggccacccgcaaacatcgatgacctgagggccttgatcgtcgaggaacttcatgaggtacagcgcaagctcttgggcgacgaactggacccagttcgtgacttctggggagacaatggcaagccctacgacgagaatcgatgccgagaccgcttggctggtatcgtcgatacgcgtttgtccgatatgtattcggtcaagcgcatgaccgaagcggacatgccgagggacaagcgggctgatttggctttcgccgtgggatcgacgatgcaattgccgattgaagtaaaaggtcaatggcacgacaaggtttgggatgcggcgaactcccagctcgaatcccagtacctgattgactggcggagtgaggggcgtggcatctattgcgtcttctggtttggcaaacttgccgccgcaacgcgcaagcgtctcagggcccatcctgacggactgcccgcgccatctagcagtgccgagatgcgatcgatgctcattgatcgcattccacttgcacggcgtcctttcatcgatgtgatcgtcctcgaccttgttacgggtcgcaagtagcgaacctgattcggtcaaggcgtccgcgtcgttacagatcaatgccggcgtggactcgtccgcatgaatggtcggccgggttcggcgcagttgcttggtggagactacggctctgcctggctcgctcaagtgcagttgacacgtgaatgcaagggcgcccgatcctctacagtcccggcagattgagcgccccttctgaacgcgatgagatcaggaatctccgccgtgagaaaagcctccgcaacggcgtcatgaaagcgcttccacaatgcatttcctcccagtggcttagcagtcgtgggagagacgaccaggcgatctgtaatctgcgctccgggaatgttcggccgaatcgtttcgatgaaccaccacgagtgtgagcagacggcggcgatatcacgaggctccgttgtgaaatccactggggagtcttcttgtggccgaggcagcaatgttcccaactcgtcgaccgtcagccggcagattagcctggcaggccaccccatcacgcgcatcaacgcgaagaccatcttgtcctgcaagagcgccatccgctcttgcggcttgtgttcctgggagattctgtggtcaacactcgccatcagcaactcataggcatcgtcgctgacgaaatgacgcaagctatccgcgcgctcgtcgtccacattcaccccgaacttcaggcatatctgcgtctgtgtcagtggtgcgccggtcaggttgcgggcgacgcgggcgatctcggtgacttcttcctttgatcgcttggggtgttgtacgcgcatgatcgggatcagtgcctcggtcaaccagaatggtgccgattcccgcgggtgcaggacatcgctgatattgatgccgtgcgtgcgggcataggcctgcagcccttcgggtccttgcgcgatggcggtcaccacatggatcatcgtctcgcgtcgttgtgcgacggtaaggaagtcgaaatttctcgtcggcgagccgtttccttcggcatgtaccacccgttttctgatcgcggtgaccagcatgcgcaagccgttgaagaacaggatcgagtgcacgccctcgcgtgcgccccagccgatgtagccgtcgcgactggcagcgagaagccgtgacgtccactccgtcagcagcggctgggcagcgctggatgccgtcttgcgcagatcgtgtccgcaggcggggcaatagacgatccggtctggtccaggcacgaagccgttgggtccgatgtccacgcgatgtggcgcgagcggagccgagcattcggggcaggcgtccaacaactccaccccatggcgagggcagaccgtcgcgaaggataggcgccaagtgcggcgaaaatacggaatgctatcgctggctaagcatgcggggcagtagctcaggcctggactcttccgagtccggtggtagatgtgaaggggcacgacccagcagctgccgccttgcgcgttgaagtagtcggagatgtatccttcgaaggagtgcaggctcaccgcatccagttgggcatcggtgatgccggtcactcgtttgagtgcatccctcaggagcggggactgaaacttgtcgacgtccgagttccacagccggcgaccgcggccgagcagcatggtgcacagctgctccaccttgtagccatgcgcgtgcgcaaggcggatgagccagatgctcagcagctcgtcttcaagtggtttgaagtgaaatggccagagcgaaatctgctcttcgatctccgacatgtcgacattggcccccgcccgttctgactgcggctcgggccgcactctcgttggctccctgaggggtgatcagccggcgatggtgttctcctcggggccgtttgtccaaccaggctgtccagctcggtcaatgcggcgtccgcttcagcgacatcgcgcgtcccgaacgttggcctggcgtctagccccttgatgcgctcgagatctcggaggcggcccgcaggagccggatgagcgcatcggcgtggcgctcggtgccgtcccagacgtcagcaatggtctgctgcaacctctcgctcgcagtcgaagccggggtgtctacttttagcgggatatttgcatatttgcatagacgcctgtgcgtatccgtgagccggcgtggggagcgcaatgcccggctgagcgtcggctgaggaatgccagtccttcgagaaagctcaatctgagtgagattgtgctcagtcatgtagttctcgatttgtcggagtgcaacattgacggtcatgcaaatattattgcatagtgcatgaatgaactacctctgctcttcgtacatgggtctgccgctggatacgtggtccgtcgcctcggactgccagttgcgggcgctcttgaagcgaagtgggctgatcgccgccgatgctttggtcgtcgacgagttctgcctaccaggcaacacggttcgagcggaccttgctgcggctggagaagagctcgtgggctacgagatcaaggctggcgctgaccgcctgacgcgcctgcctcgccaaatcgctggctatggcaaggtattcgccagggtgaacatcctcacagtgcctgctcacttcgatgctgtgctcgagttggtgccggcgtggtggggcgtcatgctcccgacgggccgtcgcactgatctgcagttgcatcaggctcgagccgcggggctcaatcctcatcgcagcgctcatgccatgtgttctctgctttgccgcgaggagctggcggcgaagctcaaacaagggggcgcggcgcgcgggctgagcggctggagcaaggcgacgatgctcgaggctgtcgtcagcatgctctccgtggaggaggcggattcctatctgtgcgcctgcctaagggcgcgtactcgcctcgttgcaaagcccgagcctcgggagccaagcatcgactggaacctcgctcgcaagaacttcgggcttgcgctatgccctgcgccctgaacaaggcgcgcagttgggagcgctaaccatgtcgcagaaagtgatgtccatctacgacttgctctggaatcgatgtcatgtctggtagacgaaaatagatcatgtgccgtacaaaatcgggctgttgatgcgctcgcatgccatggtatgtccgatggtccaatacgaccacggtccctggagggccggtaatttcgagcggctcgccgttgatgccctcttggctaaggatcgcctcccgcacattcttgcgagtcaccggtctctcaaggccatcgaagcgagattgagttacgcggtgtgattccggccagacgagaagcgctccattgtcctcgccagacttcacctctacgagcaggatgccgaccaacagtccgaaccacgaaagttcgtccgcataggcaccatcgacatggcggttgagccccacaggcgtgtagccgtcagccaggctcgatagctgtgcaacgttgggaagaatcctgagttcttccttaagtaactctgtaaggagctcctggagtcgggtgtcccgcggcatttccacctgaaactcgccattgttgatgtgccacccaggcgttcccgttttcttgcgtggttcgttctgggcccttcgaagaaccgacctggcccagtccttcatggagtccgacggttccaatgttgtgaaaccctgttgaatgaactgagtagcttcgggggaggtcatcttgtcggcctacatatcggcatgttgtctcggcggtcagaatttaccgtagacaagtcgcaggtgatcaggagcaagtagcttggccgcgcaatggccttgtgtcgaggacggggggcggcgctaccatctccgctccaaagaggatgagcgagggacgggatgagtgctttcgatgaactggcgcgcgaagacggcgtcgcgcttcgcatcgattggtttggcaacgtcggcaactcactgcagttcgggcccgagcaacgcacactgaaagtgtcatgctcgctctggcgtcccggtctgggatggatgctgcggagtagcgacgagcgccaggagatcgaaatcccgatcgcggtcctaccgcacattcgtctcggggaggtctggaaggatggagctcgtgtcgagtcggcgccgttgacgcgcatgctcttcaaggaaatggccgtcgacgaacaaacctccgaggtcctgccttcgggtctcccgtattcgcctgcgggaggttcgacctcgtacctccttcccttcaatgtgttcaatgcgcacaacgaacacacgcgctcatgggtcacccgtgttcaggttgacgtacgcaccgtgctggtcgtgccaagcctggagctgtttcgcttctactttggcgcgacaggatcggtgctcgagggcgtcatggcaggcggggacgccgagcagaggctatatcacgctgcgtacatcagccgggtcagcaatgcggcgaacgtcgttctgggtatggggatgcccgcggcggccgcaccgacggtcgcgcgcatcgctctggatgacgaagccaagaaggcattcttttccctggtcaaagggggacgcatcgccgggctgaacaagaccgactggcagcctcggatgggctttcccttcacgggtaagacgaacctcacggtcgatggtctgtggctggatacgcctgggcagcgaaccttcgtcgcgctgcgcctgatcaggtgcacctaccctcatccgttcgagcgactcaactacagcatcgatgatggtcagctgaggactcggccaccggtgtcgggggggcgcaaggagcgcgggccaggtgagaagaaggagaggaagccgaagatcgtgaaccaatgggcggacagaagccaagtggcgctcgaggtgtacagcgacgacgacgacggggatccctttccgtatctcaagaaaacctcgattcatcgaacgtcgcatgcgccttttcgcgccaatcgaaccgatgccgaagatgaggatgcatgtttgtacgcgatcggtccctcggacgccgcaggattgccgccggcggagatcatggggagccagaatgactacgatgaacgcagacttgagccgtcattcttggccgacctgcgccaagcgttgccggcttgcctgcccgggtgggagttctgtccgctcgaggacggtgaggtggcccgtcgcatggcagtgcctgcaccggccggtgtcgcgtcgtggtctgacctttgggtttggctttccacgatcgtcgaatatggggcgacgggaggcgcaatgcgatgcgcggctctgggagtcgccgagttcccggagggacagatcagcgtggaagtggtggcgcaactcttgggggcgggtgagccaaccatggagcagattgggcaaatgttgttcgagccctgctggacgtctaccgtgccgtccgaggtgaaccgggacgctggggcaacgattgcttggacgacggacgaactgaacgcgctggccgacgaattgagccctcaggagattgccgcctgggttttgagcgagttcaaacggcgcgtcttggcggagtaaggcggcccgcagattcgcttccaacaaaacctacgcacaacagaagggcaactccagtgctactactctcatgctttgaacttggcgatctcctgccgtcctcgggatggcgatctgtacgagtcccagattcgttgcaggatttcaatgctttcacccacgtcgccctggctcacttcacctcttcagccttcttggaggccatccgttcggaggggctgaagccgcgcaatgctggcatccagcccatcctcgacaaccttgtgacgagcctggacgacgtgtacctagccgcacgtgcagaccggttctattctgagcgtgcaacgcgtgcatttgggggtgtcgggattgcggtcttggtccatgtccccttggccaatctgtctgtggacgaaaacgtgttcgcaccgaacgattcttctcatccagtcgataaaaaatcagccttgcaccgatcactcttggtcgggtattgcaagcatcaaggacttatcgcgcctgaatctatccgcgggatctatcacatggatggtcggccaatttgatggcggatgcgcgcacgatccgcattgacaagcccgagaccggtccgaagacgagcgtgacctcttgcgccacgcgctcctgcactccgactttccccgcgagaactggcgagagtgggcagggcatggatggcatcgaaacggagcgacccgcggacaacgtgccagcttgagttgcgcaggtcagccgtacatgctggggcggccgactcctccgaaaccctcccttgggtgtttcggcaggaagacctcgaagcctggcaccggtactttgggatcaaaagcggctgtccatttctcattggccggatcggtccccgaatgcagggtgcttgccgcccactgcgcaaagttcaatacgacatcgagcggctcagctttgaagaagtcgattacaccgccggcgcgcatgagctcggcatagaacttcacattgacgatcgcttgcacgtcgtccttggaaatttggacctgccggacatgagctatgcgatttcgaatcgagcccagcgcgcccagtccgggcttcatagtgcccagcagagtgctgctgcccgggagcatgcccaccttctgctcgtaccgcagccgaagccggtctagatcgagcgttgggtgcatgtgcttcaggtattcagtcaagaagtactcgacgacgagatgcgcgtggaggacgcggcccagaacggcggaatcccgatcccacactgccatgaactcggaccggcgctgctcgctggccctgactaccgcgtcgactccaccgaacagcgctgcgacgcgcgccatagcgatttcggatggcatttcgagttcagcttcgggttcgggtgttggtgcggtcatgggtcaagcgtagcaaatagcccccctataggggtaggtgcatgcccgatggctcgcgaccattgccacgtcaacgggtagcggccacgacaaccaacccagagccctgtgttctggcatctgacctccgcgacgaggcgtccgcggcaccggccgtacgcgagagcagcccgacattccccgcgcgagcagatgagggagccagcggcatggacggcatcgagacgacgcactaccgacaacgcgccagcgtgggcgacgtgacggtctaccggtctaccggtctacggagacaccttaatcagttctccgaataggctcacgagcccggcgcctgccaagccgattgcggaggtcacggcaatgccgatcagtgcctggccgaaccaatgaaggctacgcgtcggcctgaaaaatttgatgttgggagccattgcgccaattgctcggcccgcaatgttgtggaggaattgccagattggcagatagaaaaagaataagacgataaaaccgaccagcgcggggttgtccacgtttaagcgaggcgcgagtttcacggcctgccagaggctgaatgccagaacaagcaacgtgccgacgacctgaatcagcagcggcgtccatggagttcgaactatcccactgtggttgttgcacttcttcaggcaatcgtccaccgcggaaaatgacccgtccatccagtctttgctctcggatgaggacacgagccagcaggcattgtcatcaccagcatcgagcttcaattccaagaaagagcccgtcgcgcgattggtcctgatgctctgcaacgattcggttgtcagaaccaatctttcgactttggcggcctgtttccaataggcaattacgtcgtctgccgtgtacaccttatatccgcggttgtcgaagcggatgacgaacaccgcagccttcacttcctcggtctgattcaccgtcagggttgggatgcccacccttgcccagaagatgtcacacagctcgcgcacggtgtcttcggtcatggtgaccgagcggattttcttgtccctcaggaagtgcgccattcgtcttaactctccaaatattctggcgaagcatacgtgaggccatctaatgagtcatggctcgtgcggaaagcgcctgactcacctcttccaagaacattcgcccgtaacggggttagaacggtgaagcttggcggacggtcgatcagcctgccctcggatcatgctttggccggttcaaggagcccgatccgttgacaccagtggcgccctcgaaatgttgcatgggcctcatacaggagcgcacgtaagcgggctgattcaatgccgagtttctggagcaacaacaggtggtaaataaaccctagtacttcggacaattcctgagcttccatcgtgagtgattcgctatcagcatcgcgacgccctccgaagtgagagatcaaattgcgcacgtcggcgcatcgttttgcaaacgttctgatcttctcttcctgcacgtccataggcaaaagaagagaactaaaaaggtcaaaaagacgctcttcgagcgacggctctccggcaaacgcgaggcgccccctcaaccaccgcttatcccttggctggacagcttcaagaatccgcgcaatcttttcgtcgagcgcggtgcgttgatctgccttgctcctacgatggagtgactccagcccccacaccaagctcgcgaagcggtgctcaacgtagaaggtcatccctcgtcgagttgcgagataaagaaagatgcctggaccgatgtctctgcgcatttctatgaagcattgatagagttcgccgaacttcggagctagctgttcgaagaatgtgaaaagttggtgtatgcctggcggctcggacttcccgccgatccgatggaagtaggccgtcgcagggtggcgcgtcgtgccgagcgtgactgtgggccactcgagcgttcgatccgagccggtcagcagaatcagcaagtcctgcagagcccgataccgctcaatcgcggccaccaacgtcattggctttcgaggagcccaagatacagagtgcagcgttttgagttcgacgctatggcgtctaatctgcggaattgccggaccgagtatgtcggatcgaaattccaaggccccatcgtcgagcttatagcgtgtcggcttagtggttgtgtgtttaacgctgagggtacgacgagtcttcgttggctgcagttcaccacgactgatccagttttcaaacccagccaaatcgacttcaagctcccgaacgtcgttcccaatgtcgctgtctggaaacggaccgcccgcgactaggcatgcttcaacgacgtagatcacataggagatcccgcgcgatcgagcggagccgccatttttcagcagaccattcagcctgacgtattggctgttctttttcagcagcccccaacagactcggtccttgagagcatcgtgctggtcctcgaggatgaccttccagggatgcccgctctcggcgaacattccgtcgagttcgagctgaattcccccgtcagtgtcgattgtgagtaggccagggaccgccgtagcggggacctcgcccgccgccaaggcctcttccgaggtccaaaaaaagcctcggtcttccagctgaatcgttttcattggattgacaggtgagcagcaagcacggagcgcggagtttgccctaccagtgctgcaccagaacgagttccgggttgaaccccctgtagggtttcgccattgtctcccgtctcttgaaactgcccctcaagcaccgcgcgcgagccttggggtgacgtcacggcggcaacgccgtggattcaaggcagatggcgcgggcccatgtggctcgcactggattgctggcccctttgcggccacggcgatatgtggccggacaggcatgacgacatccaacgactttttccagaacaacgaaatcaccggtgcactgacgccgcagcaggccgcgccgctcctcgagctcgcggcatcgggcgatagcacccaactgcgtcaagcatgtgttgtcttgttgctcactgatgcgtgcccgaaggcgcctacgacggcgcgggcagggacttcgtctttgcctgccatctctccatgacgaaggcgacgagagtatgagctgcgttcactgcgagcctggcctccgagacgtcaatcggcggcgggttcactccacgaccatgagccgatccaatgtgcgtccgataggccccgacgccgtccaccaccgaggctaggccttgaaggattcgcttttgatcgtcgcttaggatctgattcatgttcaagcccaagtgcggctgaaccgcgcgccacagcggcacgacggtttgggatgttggaagctccacaccaagcgtgtcgaggcatgtcttgcaaattgcctcaatgatcgagcaagcagcagtgatggcggcgtgcggatctcgatccaactgtccgagcgcacggtcaaactctgcgtcaatcgacgcgtagtctccggcccgcaggtagtcggccaacgtgcgagcggccgggcttgcaccagccaacgagatatatccgttgaaccgatacccaagctgattccgcgccagggcatcccgaattcgctgttggccgacgacgacctccggatggcaatccgcctcgggaatatccatgaaaggctggatgatgcgacccagcacggttaacgcgtcgacgtctggggcttcgttgcagctgcgcagccaagtcgagcacttggactcgcagttcccgcccgggacatcccccggcgctccggcttcgaggaagagcgagtcgagctttgaatgcgagtagtagtgagctgcgatgaccgacgacacggcgccgatcaccgagttggggatctggttgggcattgtgatgagttcctctcgggagtcggatcctagtccggtgcagcctccgttattcttcggccagacgcttgccgtggagtggctgggacctggaatttcgaactcggcgacggtcgaacatggtcggttctgtcaactcgccgctcgtagaacctgccattgatcgcactcgacctggaatcatgatgaccgaacaagcattgccgacacccgctgaagcagccccagtgacgcactgtgctctttgtctaaaacgtcgagtactagttgtctctcatattattccgaacgcgtacttccgcgcgatgaagcgtccatccaacgggaagctcgtcgcgatggatactgatccaaatacacgggcgacgtacagccaagacagcctgtcggaaccccttctttgctctgactgcgaaggacattttggaaagtgggaaacatcgtggattcggaagctgcgcttgaccgcaaagctattcacagatggagtggaaagcgtcgcagtcccctcgttcgagtacgagtcgtttcgatgcttcctcatttcaatcgtatggcgcgcggctgtctgttcccggcaggagttctcacttgtgaaattccctgaggatgggctcgaaaagattcgtgtcgacctatgcgccgggaaagccccaactgaaacagttatcggaaatcgagttcgtaagctggtcgacccatccgggcaactgaagctcactgacctggaaaatttcatgttcactccgatgccgctatcagagggaggccttcaaggctatcgactattttttgcaggatacgtcgttgacttcattacctcaaaggtcacgcgtcgggtatcgaacgtaccagggtttgtgcgtgacacactcgccctcaaaattcctgccgtgtcggtctttcaggtgcgggatttcatgagaatggggatgtacatggtggagaagcacgttcgcgggcaaaccgccttcggctcgggagcttagaagtaggagcctcacacaagggggcttcagctcagcgcggcgacttcaaccggtcgatgcgaaaaattcgttgaacatctcagctggcgtctggaagccgagcctcttcatcgaagacccagcatcaacgtgtgttcgctgtccctatatcaagggtgatctcgttcatcccaccgcaagcgccctgtcgcaaggctcgacgcgcgcccgctcaccgattcaaccagatagtcataggtgtgaatcttgatgttcagctcgcgagccatctggtgccgcctctgctcgacgccaggcggaagcgctgaacgccgaccaataaggatcaagccaggaaggtctgcgcgaacgcttgtgagcccgaggccgctatcccgtcgcagccggctcgcgtagttctggttggcatgcagccagattcgccagtcctggatctgcctgatggcgtggatcaggtagctggacgggtcgccgctcttgttgaacatcggtcgtaatgggctctcgagctcgacagcctgccattcgaagccgaaggaatgcttctcgccaataagaaaatcggtcacatggtccgcgcccagtcgctgtttgggaattacccatcgaccatggcctccgccgaggtgttgaatcagcagcttcgggttctgctgcagatactgctgaacatcttcttcacgcgtagcacgttcaagaacggcaagcagtgcggatgcatcttccggcaggatgtcatcccaccatacttgaaattccgccagaggatcatctctgagcgtttgagcattaatctcggcaactgtcgtgagcttcatcgcgcttactgagagcagctagtcctttgggtgccagctcgtttcgacgacaatcttgcccgtggcatcgcgctgctccacgcgctcagtaaccttgaagcctttgactgcgatgtgtttctcgtagacaacgcgtcctacgactgcgcccgcagcgtccactacgtcgtaagtgtccacatctgtttcacccatgaagcccttctctctggagctcacgtgtttcaaggtctggccatcgggcaggagcagttggtcttggaatttcatcggtccctcgggaatccaaatagcagttccattctcgctcggatgctgatttggggcgaaattgaccaacacgtcttagcctaatcgggtgcgcgggctcgtacaaacctgtccaagcacgcaccgtcaattcttccagtacggcatcgccttcagcgtcgaaaccgctgtcttgaaaacgccggccgtcaagacttggcgggttggcctgaagtcctggccacactctcatttaaataccgacgaaagcgcagattcgcatttatttaaatgcgttcgtgtttctcgaccgcgcttacaccgccgcccaccagcgcgacggcgctcgacgtatggtgcggcgctgaagtcggccgggtcatccagcgcgcggtcgagaagctgccgcccaggctggcgaccgccgcgctttcgagcgcctcgtccacgctcatgggcggcagcagcccggcaaagcgctgcgcgagcatggacttgcccgagccgggctccccgaccatcagcaggctgtgcccacccgcggccgcgatctcgagggcgcgcctggcgcctgcatgccccttcacgtcggccaggtcggcatacagcggcatggccgcggcggccgcgacgtggacccgggcccagccgtccgcggcgggcggctcggcctgctgcagcgccgcgtcctcggccatgaagcgccgcaccacgtccagcaggtgcctggcgccgtacacctcgccgccgggcaccagcgcggcttcctgcgcgctctcggtgggcagcaccaggcgcgtggcgatgccgcgggtgtgcagggccagcgccatggccagcgcgccgcgcacgggccgcaactcgcccgaaagagagagttcgccggcaaattcgtggcccgcgaggcgggcggcctggatctgctcgctggcggcgaggatgcccagcgcaataggcaggtcgaaacggccggaatccttgggcaggtcggccggggcgagattgaccgtcagggcagatgtactcttgtaaatgatcaaggaagcctgaagccagagctggcagcggctcctgcgcttacccgtacgtacatcacaccaggtaatcatggatatccaaaccgttgccacacgatatgccaaccgcaaattgaaatccaaaactattgacttggaagagattggcgcaacgatcgatacttggttgctggatttattgcgaacagtctcaaaaaaaagcttcgttaaccccatccaaagtaacgaactcgaaatcatattaaaaggcttaagactgctgtctacgaatcactcttggaagatgttaattcgacaacaccctcgagagctccgagttgatgatctgctcgatacgtatcaggaactggaagtagcgatcgccctgctaaaactttcagctaactcgtcccggcaaatgtttgacggaatccggcggcacgttaaaacctatctcgaacaacgtggcgactgcccgcaagtgtcaatgttgcgatcgttttatccgcataccaagttcagtttttcaaaagctcgtcagttgatcagcgatcagagctttcctggtcacaaagaagatcgggagccggtaggggcgctccgtcattctacggttagagaactcaaggccaaaattgaaaagaggctcgatggcgaccttagaaaaattcaagatgcatgcaccaaggaaatccgagatcagtttggcgtcttcgattggcttgaaagaatctcaaatgagcctagaaatctggcgttgaaagaaaaatgggacgagctagcaggtcgtcatggtgatgtatggcgtaaaagcgtgcgccagttctccgagcgcgatttgctccgagaatttttactaaggcacgcacttgctcccgcctttcgtcccagcttattcgcggcctatgtcgatcaggggcggatcttagagtacgtggcaaaggagaccggagtagccaccgcaaagcgactggcctcactggtccgttcgccacatctcctaacctcgaatttgctcgtgtatttcctaattttgcttcagattcattcctgctggaatgtctcttctgttcttgagctgaccatggattgcatcaaaaaagaaggggcaggatttttgattcaaggattcaaatctcgaacaaatagccaaactccaaaggtgtggatatttccgcgagatgggattatctttgattgcgtcgaaatgcttctttcgcgcgtgatgtacctaaaaaacctaggccgaattgcgtcagatgagaatcggatttggatggcttcccgtcgatccaatagcctaaacacgcaaatattaagcggcttttcgtcgtctctaaaaaatttaatagacaagcacagcttgcccatattttcgtttgagcaaatcagagtgcaatgcctggcgagaatttatgtgagcgaaggaggtttagaagcagcaaggcgctctggggggcatgcaagcattcgaacaacggcgcactatcttgatcaactcttgttaaatcgactaaattgcgcgattaatttggagtttcagcgaaggctagaggaaaatgtgcgctatcgcattgccagcgtaggtggggcccgtgcctcatgtttcgatgaagagatgctttaccccgtcggagatggaacaatgtgttcccaaccggctgagccgcccaacgcaagttggctccaagatggggtatgtaaagccgagaactgtcacattgatggcggctgtcctaacagcaagttgacgcttgacgctcctcgcatcgaagaaatcgcattgacgatgcggttttacgagaacaactggcagcgactcgccagccagaacattgatgcgttccgtgggaagcatcttcccgcgatgttgttcaatatggcgctccacggttttgtgtcgaaaggaccatacggtcatctattgcgccgcgtcgaagcgggaggccccaatgcatagcgcgaggcgcaaggagcggccaaccggcccatgtcctaccgaagtcccttgggatcttgggatcggagggaagcatcgattgcttgtctctcccgaaggggagatcgcagttcaccgtccctgggcgccatcaccgcatttggaatacagcaggttcgatttgcgcgaggcgcggttggcgccaacgccgtttgttccctacggcacgtccgtggcagatcggccggaccttcgcgaggcggttattcagggcctaaatgcttcattgcgtgtcactcggcctagcaaatcacagcaccgtaccctgatcctcagggccagatgcttggttaaaaccattgaattcggctggctgacggggatatatcggatgtccgattggactgtcaaagcctacgaaacactcgctaccaagctcgccagcggaggctggatcgaggcacttgatgttcatgcgcgcgtcgatcgacttctagatgacatgtcggcaggcgatatccacgcgctatggcttccttcgcactcaagtcagtacagacttgatgggcggaagctggcgcgcttgatgcactgcaatattggattgcacgaagtgtatcggctgcaagagtacgttgctcgacggttgggtgctccaacgcaaccgaaaataaccaaaccacagccagtcgatcgagagcctgtcgcctggtctagaacggcgctgaggtccgagctagcgatcatcaatctctttgccgatggatcgaatgcatcgctttcgttccgcccctttcctcgcgttgagaccttcgtgaagcgcttcgcgtcgtcacaagagacgcgcacgccgtccctggggccagacgatgcagccgcactgctcaaaggagcagtgcgatggattgaatcgatagcaccgcttcttcaggacgtactgctggaatttttcgaaaaatacaagctgctaccaaaaccgcacatcagcgctaaggccagatccgcgatgttcttaacatgcaggtcgcttccagccttagaagaggccttggcctgcaaggtaacgcaggttgataagcttcgagatccagttgcactcgacggagtgaccagcttgcactcggtggtgaagctgctttatgcagcttgtttcatcgtgatcgcccttttcaacgcacggcgaaaggacgaagtacagcacccggtcatcggactgcaaaccggaagcctgtccgtcgtggacaaacaacttgggctgtacatctgttcgttctacatcgaaaaaaaccgttcggggctgtgtcccgttctacgttggccagctcaccgctaccgccgtggacaccttaactagtttctccaatattgcgcgagaccttgccgctctcaatcaagatggccgcgccaatccgaatggtggcgcccctcagtctgttttcgcgatgcctagcttccctacaacggtaggaaacaatataccaaggtcgttcgattttcattcgatgcgcagaatggatcgaggtctggagaggctccaacgtgattggctgttccagtcactgcgaccacacatgttgaggcgcgcatacgctttgatctttcactatcgatacgaaaacgcgacccttcaggcgctgtcccagcagttgcagcatcaagacatcgagaacacgcgtgtctacgtatccgactccgctgggacagcggtggccgacaccggcgtatcgctttatggtcgcctgacccctgcacaaaggaaccaaattgagaccgatcgggattcgctcgatgtcgatctcaaggacgtggccaacgagaagctgatgctttttgtccagagcgtggtcggggggcgtgcgactttctcaggaggatacgcgcgccttgttcagcggtttcaccaacaattgggcagaagcatctcgtactcggcgctggatctgcgggaacgagcgaagcagttgggcaaaacgctcatctctcgtggacatgaaccacggcctatggcgcacggtacatgcatggcgggaacaagtgtttcgcggctgcgtggtcattgctttgatattgattctggggccctagatcgttcaaacgcaaaccccacgaaatgcgcacgctgtccctatcacgtggttacgcaacagcatctttgtgcgctccaggcagagtacgaccaggcggagttggagcttcgcaaaaacagtgatcaaccgtcgcttcaacgggtccgcagaatcgctgatcttgctttacttcgcaagcttatagagcttcacgctcggcggcttgctcaactaagttacgtcaatgaagcagattcatcctctaaaaactcgcagtgtcaaaccggcgatcgctgatctaaacgcagccgaagctgaggcgaatattcggcggaaactcacgatcctcaccgaagcgctaatgcagtcgactcgaccgaagcacgtccgcagtgcgtgggctcccgatatggccgttgccatcgagagtggtgcactgccaacaacgattcggcaatttaatctgtgggatacagaagccgtgccgcaagacctgaagggaaaattgccctccttccgtcgcaacgccggcgtcactttgaaacgtcaccgccaactgatgacaaatgtcgaagacgtgatcacggccttgcgcaaagctctcttgacgccaaccgtggagtcgcggcgagagcatagtgtggcctcgttgcgaaggcggattgagggggccaagacaatgcggcaaatcgccgagcgcgaactcgttgcaagtcgtcaagaagtacagcggctgaaggatttactcgcgctggagacgagtcgcagggaagcgactgagcgcgaatcaaaagagatggtgaaaaaactccacgcgcagttggcgcaagctcgcgcacagaaaaatccgtccaccgtgagccctactaaactcacgctcgctccaccatcgacggcgaatgaataaacactttgctctttcgccggttcgaatccgggatcgctggtttgtcatcgcgtatgacttggctcggggatcgactatcgcggaactgactgactattctcttcatgcttcaactgacctgcaactatcccgactaacgctggagaagaggatcggccaactcttaaacttctgggcgtttctaaaacgcgagaatatcctcgttgaagagatatccgatgcagtgctagtgcaatttcgcgatgatgagcttcaaagggttctgaagagaaagacttcgcgcggcaatgagctcaaggcgaagcgaaccgtcaacgataaacttggcgccgtctatgcatggctcggatggatggtcggatcaggacgactgccacactgcggcgccacacgaccaattcggcgcactgtcctccatggcaagacaccggctatcgcgactgcagtgggccgcgggacggtttcatttcgccgcaccggctccggatcaaaaactcggtccggctatgtcgcaacggcagagacgcatgacgcgatcacagataagttcttcgcggggcagagtttgtatgcggcgcaccgcaacgctctgatcctagcgattgcggatgcagtcggatttcgccgaggatccattgcgtccttatgtactaaacaattcgaccgtgctgaactcgagcgagagttgcaagcagtcgtcttggttcgcccgccgtctcaaaaattttcttatgagcacgattttccatttccggtatggctcgctctacgcatttgcgatttctgcgaagcatatcgagcaccgttggtggaacaaaaaaaggtgacgccgacacagactcaggatcgcatttttctctcttctcgtgatgcgcatcccctttcggaaagagcaatcacgcaaatattcagcaaggcaatgcgtgccgtaggtgctcctaagggggccgctttgcatgcctttcgcgccaaattcgcaaacgatcagatcgagcaagagctagatgttcgcactaggagcggcatggatacaagcagcagcgcggtcgccgcagcggtcgcaatgaagcttggccagaaaagctttgactcgatctactcgtacgttgtcgccgcccagacctctgcggccttgcgagaaagaacggatgcggcggcacatgtagatcgattgactgcgcgggtgcgcgagctacaaatggaaaacaaaaggctacgaaaatcttccgagcaatagctcgggcatccgagtctggctacggcaacaaaagagtacccaaagggccatcctgaagaccgtgccagcatcactgcgagcttgtgttacctctgctccagcgcatttcgaactggcgaagtcgaagcgcacctagtaaacctaggcctggcttaagtgctgccaggaggatccggcggcaaggatggcgcgcgacgcctagagcggcccctggtgggctctaacttccgtagcggcggcatttccgggggacgcgccaaaagatacagatcggcgtggctcacccctcgctcgcgcaggactcttatgcagtcatcaaggcgcgcccacgtgcgcaccctcaatgcgcttcgagcctcacacaccgcgagccatcctcgtccggactggtggaagtccaccgtgtagtaccagcgaggcgccacattctttgacgcagcgccgctcgtcactgaggccagagccgcctcgccttcaaagtctcgatgcgcgctgacgcgcacttgcatttgtcgattgatcatgcattgagccttcaagtactcgagtgtgggcggtggagcaccgtatggcatggttcattttccgacaaacgtatatgtttgtaccagaaatcaggaaggtcaaaagggtaagtactaggtcgcgatcttgtgacacaacaacaaaaaggaatatcacatcatgagattcattgaaatcttgaacttcgtactcgccctagttgatctactcatctggatatacgacaacctcttctaagcaatcggccggactcatccggccttttttctgcgccttcccgacgcgaaatgccggaaacagctaggaagactggcgccgcaggagccaatcgaacaaacatgcagatgtttgactgtttgcatggccgcccctgtccttcttgcagacaacaataggcctgccattcagaaagtgaccggggaaatggccatgggtgcgtgggcttcagccagatgctgcccgacgagagggcaacagcgcccgcgcgttcctgctggcagcgctgcctactgcaagaacttcggcgtcaaggtccagcaggtgatgcccgacaacggctaagccgacgagtccttcgcaggccgctgcgtcgatgggcatcaaacacatccgcacccgaccctacacgcccaggaccaatggcaagcccgagcggttcatccaggccttgttgcgcgaatgactactcaggcgcgaggccccacaagaatcagccagtgaacataggcgttgataggccgcgtctcattgccgccttcgaagttactttgacggggttcattgtgatgatcgccgcttcttcgagtcgtactgtcgacaccatcgacattgttgtcaccgatcatctgtataactccgtgcgaatgtgcgcgaaatgcgtcagtttgcacagatccgacagcattgcctggcaggcctcctggattggctgcgaacctttgattggcatcagggtcacgggcagcgccgtcatccacacctcgcaggaaccgccccctatagtcgggtaggttgaacgtcgagactgcgtccccacggccgtgtatgtcaccgatggtcgcgtacaaggccttgtacgccacgcgactaatcgctgcaccgtcgcagacaagccatcctgcgtctgccaagattcttcggctcgcctcgtccacttgacccgcataggggatcacactgccaagaggaaactgcacttgaatcgcctggggtaaaagtgttgtcatgtaattcgcccgccgtgaaggacattgaggatttggcgagcgaatagatctcaagcgccgcctgatttcatagatcagtcaactcgcggacggaagcctagatcgcagctggcagctctgacatcccatgaacgggggggggcggatcgtcgcccagcagttttcacgggcccagggccaaatcagcgcatctggcgcgtcccatctcggcatctctcgactgtcagtcttcctccgacgatggcatgtcgaaactccaatccgggcgattcgggggaagaggatcgctgttcactggacttcagaagatattttcatcgttcgggctccgacggcgccatgcatgttcagcctactgatggttcggctaagaaacggtgcgcaaccattgccggaaatccgggggaaggcgaacattgagtgcgggctctgctgcaagaagagtcccagcaatggctgcaaggccttcttgttggagcgcagccgtcactgcaggaagagtcgcattcgggttcttgaaggcaaatcgagcgcttaacgcggccttccaccgctgctgagcccattcgactacttgcggttcgatcgcgtgccgaaagttggagacgcttaaagcctgaataaaccgaagcgtcgccgcaaaaagttgatcatgagacagcgtgcgtccactggccacgtcgcgcaccgccgacaagatataggccgcttgcgttctatcgggtgaatccgcctttgcctcgaacatcagattcagcagtggcgcgacttcccctgtcgcgtttcccacttcggcccggaggctactcaatgcctcgctgtgtccgccgacggcagccctcaccgcgaagcacaggacagcatctcgcgcgtgctcagatagcctgcggtccttcagctgttcctccgaaactttgggcagatctccttctaccggagcggctggggaattgttgtgcatttcttcgctatggctgtacagccgcgcgcatgcggcaagccacgatgagatcagcagcgcgaagtcaacagactccagtcgtcgaatcgagctttccacgaagctcacacgagtcatgaactccaggctcggatagacgcgtccatcaagccttctgtccaaattcccccgcgccttcttgctgcccagatggagggactcgatcgctgcgatgaggtgccatgcggtgaccttgctcgctcgaggttgatctcgaatagcctcgggaggctcgggattgctgcacattcctgcctccatgtgaggaggtcggccgtcaacttcgatgccgccgcgaccgccaaaagcctgcgaatacatccagagaatgccatggtgaatcactcgatggcagtaaatggcctgcgtcgacgtgtccttttcgatctcacccaatagcaccagaacttccgccatctcggatagcgcaaacgcgtggtcgcctgtcttgtaggcgcacagtgcgttatcggctctcagaccgatcaacatgggcctcaggctctcgctttggagttcagacgctgcagtcagcgctgcgctcagccaagtgccacacttgatccagtctccaacgttcgcagcgctgattgcagtctcacggcacacaaaaaggcgctccagtggatcgtgcttgttcagatcggagcgggcgtattcaatggtggagagtgcatccgcgtagcgtcgatttctgaagtggatctttgcccgcgccctcgagaggagcggatccgcccccagcaaatcttcaacttccgccaagacctcgagcgcacgttcgggttggctaccgtattcatcaagcatgacgcagcgcgctacgtgaaaagacagcgcaaggtctcggcactcccaggcggcagcgagcgtcgcaagttcctggaacgcatccgccgcggctgcccaatcaagggtctgggccttcgcttcagcgagccaggcggcattgacgatggtgcgcagcccacctggtgatttgcgtggtccgtcgaggtatctggtgcgagaggccttgttgatctttcccaattcaacaaacagcgatcgctgccttgacacagttggtaccgccatcgcctgggtgacaaagagaagaccgggaagactaaacgacgtaccgtcggcggacagtctttgttcttgaagatcggactccagcgcgatgaatcgaggatcagatcgcgtcaactcctggtggcgttccaacagctccacgggattgggaaatacttgcgcgagaccaggcaatatcaggaccttgctgagcaccatgtactcaagcaggtccgctgctttgcttcctcgaagttcgagtatctcgcggcaaagagtgttccacgctgaaagcctgcgcggggcatcctcaagcgctgaaagcagaaggacctgagcgaatctcaaggtcgacgagacataggcgttccgagggcagatgagccgctgaaaagattccccgcaaaggctgggcatccaatccgcaatcatcttgagcttgtgggagttcgctctcacgattgcaaggcccgccttcagaagcatgtagtccacttcgcctttgagagaatggacgtacaaggcttcggcattgcttacgtccaatgcatcgccttgcccaaggacttgggctgcgcggtgatgcaccgccttctgttcggctgtgcccaaggcctcttcacccgctccgtccatcaacggggatatgcgcagacggtttgcacccaattcgtcgatccatgggccgatgagctgttcgaggttttcaccagcaagagcgatgggtggcgcaacatccgccatctgtagagcaagtgacctgtcaaaccgacctatcagcagagtcattctgtaaaggagggttcgggtgcttgtgtcgaacttcgcgagaagagtttggcggagacggcgctgctcggactggaggtctgagcgaatgtccttcgtgaccggcacgggatcgctttccagcgtcgcccaacctacgcgccgtgcgatcgagatgaacgctcggacaagctgaggatgtccgcgtccgctgtacaggaaggcgagtacagcggatctttctgatgccccgccagcttgctggacgagatctctgacttcttcgaagccaagtgtctcaacaggagccatctccaaagaagtctgtcccagacgatctgctaccgcggtggatggctgccggtagctggtgacgatgcaaacggcatcatgacgcttgattgcggcaacgaccctcgccatttggtgacttacacccggatcttcgagctcattgagatcgtcaaagatgatcccatctgcctggctgattgcgatctgagcgaaaaccaccgccaggcgtcgttgcgcttccgagatcgaaacatcccggaagtcgacgatgagccatcgcccgccgtactccgtcgcggtcaagcgcgcggcaagagttttgcccaacccgcttccgccgacgagaaatagaagcccttgctggcgcagctgtgccagcgccttcgcgatcagttgtcgtcgaggggcgatgctcgccggaagcggtacttcttctatggactccagcagcggcgcgaaccggagatccgtcgtagattgagtcggcagttgcgcggcaagttgcagacgggccagcgttgaggtcgagatagctgtcttcgagtgcgcttcgcatacccttagcaggtcggcgagcaccagtcttcgccgagatccaggcttgacgattgcctcgagaacctcggcgacgacgacttgggcaagaccggcacagtctgtcggcgagagctgcagcctctccgatgcgaattcgatcagggatgattcgagctgagcagccacttccgtcaggccgctttgcttgtagtcccaatggatgcgtttgagaagctcctctctcaattgagtgtcctcgcgagcttcgatgaacctacggaccgcctccgagattggcgccttgagcaaagcctgcctcaggggtcctatgtcgcagcccgctgcggcttgcctccaatactcgaggacgccttcgtcgcccacgcggtcagcgcgatcgcgctctcggcccagacttgcggttgtcagaaaacgaagacttaccttggtatctggatttcgatggactagatcgacgtagctgttcagtgcatcaagggcatcttggttgttgatggtcagcgcaccggactcggcagtgtcctttacttggacaccgttaagtgcgtcggccgcgaccactgcatagtcctcggcgacctcgagaaaaagttgttgcccagtcttcagtccgatccaggccagcgcgctgacgtgcagctggtatgcatagccgcggagcgaggcaactgcttgccgtcggggatcaccaatcggttcggcatctaaccttggacccgcggaaaaaatgctcatgagttctagatgtgctgcgcatcaatcagaggaatcaatcagtgttgattcaaccgatcaagcactgaaagatgcgcttccttaacaatcgtgatgttctctgggtttcccacctgaacatatttcattgcatccgtcaaagcgaaattttcagagatatcagtgtgcagcgcctcgacggaccaagagcattgcttcgaaagctctttaagaaatgcttcgtaccagtcagaacgtcgtgcattgatcgccatgtttgcttcgagttgggctttgtctcgcccagcacgatccagggacaggcgcttctgcatgctgaagaggatgtccgtgcagtggctcatgcgcagcattccggatacaacttctcgccatgtgagtcgaggggaaatttcgattgcggcggggagaaactcttcgagccgataaagaaatcgggcgttgaacatggcagcttttcttccgtcgatcggaaacagcgtggcaagcgccgtatgggctcctagcgtgaacaccgcatttgcgaccgagctatggcttccgtcaatcggcagggtatcgcatgcgctgaacatgatgatcggtggcaaagtgcacttcgctctgagtgcccacatatcgagaggttcgccgcccaccaccagtgagcccattccaagctcggcgtcgtaggtgccatggccgtcgaaaaccatcattgctccctcgaagtgccgaaccgcatctgcaaactcgttcggcgtcgagacgtcaacgaagcggtaactcacccgtttactctcgcttgcgctcgcgacaagcgatatcgccgattccaacagcgtcttcaaatggtcagttggctcgaaagagcgcacgaccaagatctcgtcgaatgcggcgaatgggagtgtgattggtggtcgaagacaatgctggatgaagaggtttcctggcatcggtggggtgcgcgaaacatcaaagcgcagactcactggtagccccctcgttgggagaagttcaagcggcaagtctgcaatgagtttcagtccttcgatgcggccatgcttggattcgcggtccaggcgttcgaggaagtctggggcgatcagacttcgcatttttttccctaaggcacggagcagcctcgactctttccaaccttggtgatgacgcggttccatgcgaacgcagtgtgcgagcagcttcacttctccccgaatcttgttgagctttggttctattcgcagtattggcgtcaacgtttgacatgcgactgctgacagcccagctgtaaagctctgcatgtcgcgactccgcatcatcatcgtgctcatatggaacctagccgcttcaggctcatcctttttcatctgaactggagcatcaaaatacgtctctgcatgaagaaacgccgtgagcgactgccgaaacatcgcacgatctgcaggggtggacttctgtataaatgtgcgccagttttgatggaacccccagtagaccccaggcaggaccagcgcgaacctgtagtcgatcaaatcagggtgtaggtcaaacgtcagtgaacggcgttcttcggccactgcatcggcagcgaggcatatccggctgatatagcgttgcggatccctttcttgcttctcgatcccctcgctaatttgatcgatctttttgaattttcgaccgaacgcgacgagtgcgagttcgttcggaatgacaacgttgtgggctccttggcggagggaaatgaagttttgtcgacgccgctgtgttccattaatggcttctcgcgcctggcgcgcaaacaaggcgttcttcggatcgttcgaaagtgcttccagaacgtcccgaacaaacctatccaagcggggtggatcggcgcctgccattgaaacacgatgggatccggaaacttccgagatgtgcagccgtggaattggtgaacctacgatcagcgcatcgacagccgccgccacctcggccgtgttggtcaagaaaacttgaaatggactcggcagtatcggtagcgaaagggagagcgcatcgagctcgagtggaataatcgacggccagatcagtttgaatagacgcatgcgcagcacgacgtccaagccggagtagggttcgcgtatgtcggcgggcagtgttgctgccaatcgcaacggccctgcagccttgtgcaacccatctgtatacatcccgaaaggactggcttcggccaagtcttgctccccgtgggggatgatgtagagaatcttaaaccgctgatctgcgaccgctaggccggcgtaggccttttgatgcttcgggagcagcgcttcgaaggtcgtcgcttttcccttttctgtggcactctgatggcggttctggggttcttctttcaaactctttcgcctagttgattgagtacagagagaatcgggctcagcacgcgaggcgataaggatactcagggatgcctcgaaatcctcttgctgcactgaaataatttagtccagcagaggcgcaaccaacatggaaagaagccaaccaaaaaggtccagacgtcggatcttggcagcgcctgtgtcgtcaattagctgcgttggatcgatagccagcgcgtagcattccgcgatcgacggctttcagaacggtatgtcgtcattgtccggttcgatccccattggagggggcgcgctccgcgcagctggggcggtggaaggcgccctggccgcgttgacctctgcgggcttggctgccgcagcgctgccctgcatcgttgcgcctacgcctgcaccgtccagcgcggccttcagcgcggcttcgaccgcatcaatgcgctcttggcacaccttgtaggcatcgaccgattccgtgacgattgtcagcagatcatcgatattcggttcggcctgatcacgcagcgtctcggcatgtttctgcaacaccccgtaggcgtctttgaaggttctctgggtcatgactactgtccttctttgcagggcttggtccgaacttcggtcgaaccatccctgaactgaatggtgagcatctgcgattcttgggcctggatgttagacgtcaccgtcttgccttcgtcggtgcgcacgatcgcgaaaccacgacccagcgtcttctcggggccttgtccggtgatctcgcgcatcagggcctgggcactgctgcgggcctgctgcacaacgccaccggcccgctccgccacgcgctgtatgcggttggccagcgcctgtgctgtcgtgcgcgtcgccgctgctgtgcgatcaacgacggtgttgagtgccacgctggtctccgatcttcccgcgctcaagctcgccagcgcatcgatgcggatcgaggtcatcaggacgggcagctcctgctttgccgtcgctaccgcccgtattgcattggtccgcacctcgttcagcagcgccaggctttgccgggaggcgtcatgaacgcgccgcacggaacccaccgcgatcgtgctcaggcttgccgtgctgtcttgcttggcgcgggccaggtgatcgcgggcatcggctctaatccccgcttcgtgacgttcgatggtcagtcggacggtgcgagcgctttgcgtcccggcggcaaggatggtgtcccaggctgaccgcgcttcgcgcacgcggcgcaagatctgttgttcaatgccaccgatgaccttgctgggcgtgtcgaagcgggcatgggccacctcatcaggcaacgtactatcgcgttcatggccgatgccagtcagcaccgggacgtcctgaacgcagatgaagcgtgcaagctcgtagtcgttcagccatgcgaggtcgttcaccgcgccgccgccgcgaatgatgacgatggcgtccggccgctcgccgtcccccaactcgcgaagtgccgtcgaggcggccgcgaccacctcgcgggccgcgccctcgccctgaaaacggctgtgcgcgtagacgaagcggcagataccgaaccgctccagtcgttcggcttccttcctgaaatcgcccaagccagccgcttcccgcggcgcgacgaccaagacgacgccgtagtcccagggcggcgggagtcggcgattgcggtcgaacacgccttcctgctgcagccgggtacgaatttccttcttgcgcgcttccaggtcgcccagggtgtactcggagtcgatggcatcgatctcgaggctgagtccgtaccgcgccttgaaaacaggcttcgcccgcaccaacagcttgatgccggcgccaatcaccgccccagtggcattctcgaaatcgggaaggatccgggaggcggtgccggcccagatcatggcgcgcgccctggcgatcggctggccggcgccgtcgcgctccgaaagctccaggtagacatgcccgttgcgcacactggcttcattgacctcgaccaaggtccagacgccgctggcaaacgcctgtgtcaccgcggccgcgacgccgttgagcaggcgggagagcgggatgcccttcttgatggtggccaggccggtagtcgccgtgtccgtgagcgccacgcccatggaactgctggcatcgggcgtgatgcccgggggcagccaggcgctgaacgcaaccaggtcgacgccggcttcgacgtaccagcgcttgaccgcgccatcgaaacgcgcgcccaaggccttggccgcatccttggaacggtaggggacgtcgaggtactggcgggacatggcggtgctcagattgctgtttcgcgcaacggacggccgatcttgctgacgtgatcaaagctgtagacgtgctcgcgcgccgaacgtctgcaacgacccacgatccgccctgggaagtctttgccaccatcgaacagttcgacgctagcattgcaggcagggcacgaagacgaatagcgagcgaacatcagtccgccgacgccgccgtcggccgatcgccgaagttccagcgtcacgttgtccttcgataggggaatcaacaatgtgggcgccatcacgatcctcagctcgaaaagctcgccgaagaagcgaaacagtgagacgacgcccagtcccagcagcagaacgctagccacgctcgtcaggtcggccggactgagagggcgagagatccgaacgccgacatagagcaacagccaagccaggagcaggacgctgatcaatgccgacatgatgacaatcatgatcgaccaccggatcggagcggaccagcgaacaaagccggtccgcagcgccttgctaagaaatgcgcctggcgccgcgacggcttctgtcgtgtagtagatgccgccttcggggatcgccggcaccggctccggcgccgcatcgtgggggaccggatcagcttggattcggtagaccgaagggctgccttggaccttttcgagccgcgggatgtactgcaaccccttgcgtcgagcagcctcgatcatgccctcggtccagcctttttcctctttgaccaggcgtgcccagtgagggctcagccatgcgctggcttcctttgcggcctcaggtgcaacaccgctcttgagattcagtgtcgtgatatcggtcgatttgccttcctgcacacgcgcgatggtctggattgccagttctctgaggacctcgaacgccttgtgccgaagcggcaactgcgtgttcgtgaggtaagcgagcactaccgttgcagcctgcgcctgtgggtcaagcacgacctccggagagggtcccgggagggtttcggactgcatagcgatcgtcatggtgccgagcataaggccctccagcacctcaaggatttctcatggcatcgcgaatcttcagacattcacgccaacggcaccgggcacggcgcacgcagcaaaatccccgcccacgtgatccgcgtggtaccccgcacgagcgcgcgatccaacgtcttgcaatggagttgaaggcgcgcgaaggattgatgggtctgttccatgccggggtcacgtggcgagcctttgcctgtcttgtgaatctgagcactgcggttgccgtggagaccgagaagtctctcaggatcggaagcagccggttcgtgcccgaccttgtcgtgagatgcatgcgcacccatcggatcctgctggtggtcgagatatggcatacccacacagtcagcgcgaaaaagaaggcggcctttcatgcggcgggattcccttgggtcgaagtgcgctcttggcacgtgatctcgcgaacccgccgccagccgctgccggtcctcgactgggccgggccaggtctcccgcagtcacccgagcagcattcgctttttcactcggagggggattggacagtgggtgacagacgtgagctcgcgggcgaccaccttgcctctggccatgtcgctgaactgccaccggggttgagaatccagtcgatattcagtaccgactcaaggctggcttcttgatacagctgtcagccgcgcaatgaagcggcccaagtgtcttcatgcacgatgaacaggggcacgccggcttccttgtgctgaatggctttctcgatcttggtgccgaagctaccgtgcttccattccgcactgccgaggccaccgaccacaaggtagtgcagcttcttgctgacgcctgcaatcgtcccgccgcgcgtctcgatggcctgctcacagagcttgcgcggcccgaaaacgaagtcgccggtaaagcaaaaaagcttgttgggaacctcgatcccttccaagcgatcgattggcaactcggtcacgaagcccgcatccgcaatctcgtccagcttgccgccgacaagctgacgcaaggtctcggcgagatggctgcgttcttcctcggtcacaagcccgtccgccaggatgctttcgacctgggctttgatcaccgtgcctggccacgtcagggcaactgtttccgcgccgctaagccatgacttgaggaactcgatttccgcatcgttgagatgtccgtcagacatgatgccctggacgatgccgaccagcgccgcacatgaggtgcgcatctcgtttcggaaggctgtcgcctggcgctgatagatgttgatcactcgatgcccccgggttcgcttgctgccttccagattacagaggtatcgccagtgaatgtgaccgccatcccggtcaaggtgcatgtgcgcgtgtctccagcaacaagatcgatggaaaggtcctcgccacgtagcccttgccacatggccaggtagtgcagcgtccctacacgcttgcccgccttgatggcttttcctccgcctacccacgggaggcttggcaattcaccacgcgaagcctgtgcggccatttcgggagattcgttcgccttctcgattcccctgagccatgagcaaatgaggcctttgtcggggccgttccatcgttccgcccaagactcgccctgaggtaaggcagcattgcaactgcattcaacgatcatgctggctccattcgagaggcgtacgaggaatatgcagggcgcatcctaacgctcgactcgcaggcaatcatgcgcgtgaaccctcagatgcccccgggtccatttgaacgagacatatgcgacgccgaggctgcgagtatgaggcatgcacaatgccggcatgccaaatattgcgaccatcctcaaagccgaaatctcgcgcgttgcccggaaagaagttcgcgcggaaatcgaagcactcaagaaggcctcagcgaactatcgctcgtcaatcgccgcgttgcgtcgacgggtggaggcactggagaaagaattgcgactcaccgtcaaaggctctgcgtggcgcgctttgaaaaaagaggtcatcgaggagtctgcagcccccatagcgcgtcggttcagcgccgggcgtttagccacccaccggagcaggctcgggctatcggcagcaatctacggcaagctggtgggagtctcggggcagacgatctatcactgggagcaagggaaggcccgcccgcgtgcagcacaacttgagagccttgcgtctgtgcgagaactgaaagctagggaagtctctgagaggctcgaaggcttatagaaggcaagcattctcgaagccaatgcggggccatgcgctcaacggcttcctatcgaagcggagggagtgagatgttcaaaggcattaagaggatcaagcggctaggagtttttggcgattattcccagccctcggggactgctgacttcggggttaaaaacatcatctacggatggaactactccggcaagacgacactgtcgcgcgtgttctctcacttagagcggggcgactttccgcttgatctcggcggttatgcattcggcgtcgacactgatgtcgggcaagtcaccgaaaccaacgcgaagacgagtggcctcgtcgttcgagtttttaactcggacttcgtccacgacaatctaaatttcggcggctcgatggcccgccctatcctgcttctgggggccgagtctgaagaggctcagaaaaagatcgtcgatctggccgagttgcggaagcgggtccatcaggcgactgcaaagcaggagaacaaggccgcggcggacgacaaggcattggccgacttgaagaagaaagccgcggcggtgaccaaggaggtgctgcagctcacggagatctacacggcgacgcaactcgaacgggatctggcagtagtaaacctcggcatcgactgcaaactgtcgaacgagcagttggaggccgacacgaagcttgtccggacttcggagcacgacgcattgcctgagctggccattctcgacgcgaagagcatgttgcctgaactgtggaaggaagcaggagagctgctcgcgcagaagccggagatggccaacgctatcgaatatctgacgcagcatccagcgattgctcgctggatcgagacggggcttccttttcatgagcacaagcagaactgcgagttctgcggcaacccgttggatcccgcgcgagtaaaggtgcttcgggatcacttctccaaggaccaggcggacttcaaaagcaaactcgagtcgctcatgctgcgggtttccgagcagcgggttgcgtttgcgccgcctagttccctggctctcaatgctcagttccgcgatcgttacgcggcggcggtcgatgcggcccttgcagcaagcgaagaccacgacaagctcgccgctcgacttgtacaagaacttcaagaaaagatctcggcgctcttcgtgtcccgcgaacacgcggcgcttgaccaaaccgccgtggaggcttggatcaacgcgggcgcatcactagatgagattatccacgagcacaaccaactcgcgagtcatttcccggaggagaagcgcaacgcaatcaagcgcgccaggctgcattacgcgcaggtactccacgagaaagaaagtctggaagaccgggcgaggaagcgagcgcgcttcgacgcacgcgcgcgaaagctgaaagcatttggcgaagcggtggaaaagcaaaagcaagagctcgaagccacgattagtcaatcgcagaaaggccgggaggagatcaacagacgcatcgataacctgctgggctcggacagcgtgcagatcaaggtcatagagctccaaggcgaggagcggtttcagctcgtgcgtcgcgacggcagcgtcgccaagcatctgagcgagggggaaaagacggccatcgccttttcgttcttcctcaccaagctccaagaactcaaggacttcgacaaggcgatcgtctacatcgacgatccgatctcaagcttggacagcaaccacatcttccaggtggctgccacgatacgggaggtgttcttcgagcaggctggaggccccggcggggagtggaagacaaagtgccgacaggtcttcttttcgacccacaactttgagttcttcggactacttcgcgagctaccaatcaatccaaagaaaacgtcgaactatctggtcaagcggatctcgcccgatgcgtcgacctttgagaacatgcctgtttcaatgtccaagtatgcgtccgaatatcacttcttgttctccgttctcgacgaattcaggaacgcgacggacaagtcggactacaaggtgctgatgcacattcccaacgccgtgcggcgcttcgtggagctctatacctattccaagtatcccgacggcatcggtggaaccgtggatcaacgagccgagaagctattcggaatcgagaaagccaagcgcattttgaaagtgctgcactacttctcgcatgccaacaacattgagcgcatcgcgaccaacacggacttgatctgcgacatcgaggccgcggttgacgagctaatatcgctaatcgaatcgaaagacccgctgcacttcgaagccctgaaagctgcgctgtaggcatggcacattccacgacaatggccgactcaggtcacggttgcgagtttcattgctgctgcaacaaccgctagatttttgaggaggacgaggtggctagttccgggagcgaagggcgattcagtgttgtcttcagtggcaggccggatgacgacggccctgcctactctatttccatagttccaagtcagcaggaatggaacgactttgggcaccagtctcacgtcaccatcaccattcggggcaaaaagggctctgcgaaagcggtcgtggcgggttttgttgggtttctcagcggtgcagcgagtggggcggataccctcaaagacctacttgctcgcacgccgcgcttggtcgttcccgcagaccctgacaagcatcgattcttcaccatgcttcgagacagtcaagcctatcggaccgtcgttcagacctttggtccagaagatggctcggaggccttgcgagctgtaagagatctagtggcgatcggggagttcgatccaaccgcacagatccttgagttggccgccgcaactgaagtgttcgcaatctcgtttgttcgagacgccgaatcattcttcgctttcaagaatgcgggctccattcttcgaggcttggaagctgaaacactggggcggctgtcagaggagttattcgtgcgattccagttgcctgggcatgaaaatgagcatcaattggagttcagtttcgaccatagcggagtattgccgaagcgcatggctgttgtaatcggaaagaacggcgttggaaagagccaaacgttaggacgtcttgctcgcgcggcgttgaagggcggacctgaactcacagagaaaaatggagggcgacccactgttagtcgcttgcttgctttcgcgccgacgaatgaggcagagtcggtgtttccctctgaccgtctgaagcacgcgaggattcagtaccaacgcttttcgctcaatcgatccagacgatcaaggcgaaacgaatacgccggcgatctcgtgattcaactcgcccgctccgatgagtccataaagggcttcgaccggtggatgatctttctcgactcactcaaggcgttggcgaagcctgaggaaatctgcttgcctacacgcagcggagaacaaccctttgaacccgtctctggattccgcaacgggaacgagtcaacggtcttgaggcgtttcgcgtccatcgacccacgcaaggagccggtgcgcttgatcggcgcgaaaggcctgccgctcagcagcggcgagatatcgttcataaagtttgcagctcaagtcagtctccacattgagaacggatcgctgatcctgcttgacgagccggaaacgcatctgcacccaaacttcataagccgatttgtgaagctgctcgacgggttgttggagcggacagggtcggcggcaatcatcgctactcactcagcgtatttcgttcgtgaagtgttcgcggagcaggtcactgtgcttagggttgacgagagccgattcgtcaccgcggagaagccgaggcttcggacgtttggtgccgatgtcggcgagatctcagtcttcgtcttcggtgaagaagaccaatcagatcatgccgcggacctgcgagaacggctgctctcgcagaacatgcagtggcaggagatctacgaacgctaccgcaacgaactctcttcggagttcctgaacgttctcagggcgacgaacgaagagcgaggtggttcgtgaattctgtacctctaccagcagtagacgatttcggtgccttgacggccgtggcaaacaacacccaggtaaagagctatcctgagctcctaccggcgctaccagcactccttgctgcgtatgcacagtatgaggctgtgtcgggcaatgcccactttgtccagcagattggtctcacgaatcagcagaaggactttttgcgcgcgcactacaagagcccgccaacggcgcttggatttatcaagacgctgagagctgagaattcccacaaaatctgtccgatgtgcgggtcgacacatcgcggcactctagatcacttgcttccaaaggacggttctccagagttcgctgtcttttcgcgcaatctggttcctgcttgcaactgcaatacgaagcgcgctacgaacacggttggtcctctcgcggggcagcgtgtactacatccctattacgacaagtgcttggcatcacggttgatagcggcgcgatttgatgatttgggccgtgtgccaaaagtgacggttaggctgcgcttgccagtggccagacccgagcacgccgcggtagcctttcacttggagacagtgatcagcaagacggacatacagggcttcttggcgacccgatggaccaagatgtgccgacgtcccgcatcgatcatccgagatttcagagtgcgcccgccttctccgaaggctttgcgtaggacacttgtcctcgaactgcgcgagcttgatgaagagcatgagggacgcaacaactggaaatcagtgttcgttgctggattgcttgacagtcatgtgatcgcatggctttacacggcattgaatcgacccgggcggctagtctctgggcctctgatcgatgcgtaaacccatcgtcaatgggaggatctgcggtgattcttttcattcgccagaacgggaatcgtcgtgccttttgcaagtactccatccggtagtccgcgcgtgatcctcccaaatctcaagttcttatcgcgtgaaaatgcgctagccctgctgcctgttccttcaactagcgtcgagaaaattgatgctgcgcttcataggctcaaccaaggtgagaatggaggaatcgccgggtcgattgaaagactgacgcgcatcaacaaggcgactcgcttcaatacaaagtcgtggggtcgattgaagcagggcgcgtccgtgaaaactgctgtttcctattcgttcataactttcgatgaagaagcagaccccgcagaccacgtggtctcattttgcgctttctgtcacacgtccacgcaggctccaatgctgttggttagctttgaccgctgctcgggcgcacgaccaacgagcttggccgaaccgggaaacacctatgtgctctcccgtcgcgttatctccctaccgctgcagtgtgtgctgaagcattggggtgatccaacgaaggggcacatgatttatgaacatgacatatcaccgatggaccacgcaggttcagaactacgtgagaggttcaagtctgcgagatacattggtctaacttcacgaaactggcaaacccgttatcgagagcatcaacgtgacgctttgacaggaagtgagttgctctttcacaccacgttggcatctgtctttcccgagggaggcatcgcccaggcgggcatgggatcgtttgaaattgtccgatgcgggttgtgccttacttccgagcttgagtatgtaaatctgacatacggggaagccatgcaggttgaagagcaacttgtcgagcggacactcaatcctgcgggactgaacatgatcccaggagggtttgcgggcatcaagttgcttcacaaactcggcttcttaaagcgatctacggcaaccgctgaggagagaaaccttgcagcgacgaattacgtccttcagaaaaagcggataagcagcccggcaccttggatctctgaccgatggcaaacggatgagtactacgagagggttgtgctcaatcgatcaaaaactctcagtcgagaacagatccttagcattcgccaatacggccttaactggaacggagctcccgaggtgatcgctagtctgtcgggtgcaagcgcacgacaagttcgagacatcttgcgcggaaagtactattcccgcgtgaagtagtcaccattgatgttgatgcccggttgctaaagtcttttcagcggcgggcggagattcggcatgtaattaccccgatctaccttcatgcttggctgattgattgctcatgaactttctgtccgcaatcgcgcgtgaagctaggattgctgcatggccacccatgtcaaccatcattacattccagattttcttctcaagacttggctcagcggccccgacaagaagttaagcgtcttcaaaatcttgcctgatgggcgtcttcgacatgatcggcttggctcaagggcagtggcacacgaagcgcatctttactccttgcgccgttccgagagcgaccctgatacgaggatcgaaaatgagtttttggcgaaattggttgatggcccggcagccattgcacatgctcagatgctgaagagcggtctggcatccctaactgcagagcagcgtgacgactgggcgagattcttggtggccggactggttcgcataccttggatgatcgagcagttccgtgacatcggacgtcgtgaattgttgactcagtttgagagcatggccactcacgcaggtcgacctgaagctgccaaaacgatgctgcaaccgcgcttcaaggatgtgcttgatgaccacggaatggaaacattcgtcaaagcaattcggtcggagaaatacgttcggtgggttaacgaggcagcctggtcgcttgttaccctgcctgcgaaagttgagagcaccatcattggcgatgcacccgtctcctacttcggtgagctgatggaaaacgcatttgccctagtcgcacccatatctccaaggcatcttttttcctgcaccagcaacgcccattaccactcgctcctcgaagggatgacgccaaaggcactcctcaaggcgacgaacaagaggatggtgcagcacgcggccgattatgtgtacgccgtcgatcaagctcataggccactaattgaaaggcatctggggagagggcgtcgacttctgaatgaacaacactctaagggagcgggtttgtcttaaagagttagacgcttggagcaacgcgacataggctgggcgccgtgtgccgcatgggcaccagtcgatcgagggagggtcgctgacccgcggctgatcgaaaccctcgagggcacgagcagccccccaagttctccagctcaaggcattgatcgagagcatgctggtcgaccgccatcgttgcattgccgctcccgcgaaactcaatcttggccagcctgcgcacttcgtggacttccacgactgtcaagcgcgccgcggcaagatcatcgccatgaggggcatgcaggcgacggcgctggaagaaggcatcccctggctggcgctgcagggctatcaccgtgcggaacagcacgatgagcaagcttcctatgagccgccaccaggacccgcccgggcgataacccatacgcgcgagctgcaacgcggaggcaccgtgacgttcacgaccgagatagtcacaactggcgtgacgtgatcgtgtggcataaaccaacgcccggccaactcggcacaggcgatggcgcaacttgtcggataccgttctatgcgctgcgccatgtgcttgacgtctgagcgccatcgatcttttcaagccgttcgtgtcaggagggccttgaggccgcgcttatcttgcaatggggaagatcgccgcggcgattccggagcgtggcggcggcgaaccgtgggttcacccttggtgagggcccgtgccatcaatcagtctgtgatggatttgataccggatctggtgcaatatcaccccgatcatcaagcggaggatgcaatgggagctttggtcgccagtaaatatccgacaaggttgttcctgaaagctgcagatcacacctatgtcgagtgcggggcgggcgcaacggggtggtcctgttggggggggaaagcaggaggaacccctttcaataccggaacaggcagtaccaagcgcgctgatgcgattgccgaacccaatgagcgagcaggcattacaacttacctagtgaatggtgtctgccatcaagcggcaaaccgcatcctattccctgcaaaaattcaagtgagcaatgcccgaggctactttctgtctcgatcgatcttcggctcctacggaaaaccttcgctattcaaccaccatgcccacgtaagtggggatctgccggcgtgcctcggggtcccgcagaagggtggtcaatctggcggactgtctgcagctcaagcgatgagcaaacaggacatcttgctgttgaaaaacaccagcaggagccatgatcgcctcagtccttcacaacgtccggctgaccctgttgctgtgctggattggatgaaagccaatgtccggctctttgaacgagaggtttcgcttcagtttagagaaaaattagattctgggacgatggctaagttaaaggctgcgaaagtggaagttgagatggaccactatcagatgtcgcgggcgttcttgcgcggcctgctcaaagcgcatgacttcgtccttgcgttcaacgagatgaccatgaggtttcaggataactgcgcgaacacgttaagcgagggcgcctatgaaactatgtttgccgtccgacgtgatgagcgcctagtacttgcggacccagacgctgtcgacgcagcatttggcgtgggtaccgcagcgaaagtctatgggactcgctgagttctttggtagaaagttgtgcatggcaggggaacatggcccatatggccggcgtctcacacagcgacagtacgaattggctgtggtggatctgcacagccgtgcgcgacttgagggggggacgttggatgaagaggtgatcgagcgccgagagttggatctcacaatcgactaccgtttggggatcgagtttccgaaggagcgccgcgagcagctatggcgggtgcagcggcaggtcgagaagcgtaggttgaagttcctcgtcggacggattgcgggcaaactcgctccgagctggctgtatggccaaacgaactggttggctcgcttcgtcattagcgaatatggcaggatcttgacacctcgcgaactagcggcgtactttggtgatgaacaaacaaacgggtcgccaaagccgccgaaataacctgtcgctcgagtctcttccctggaggcttcccgaagatcggcgcgcagcttcggtgcaaattgcgttttgatcactgcgtgatgcttcgtgagggtaactctgcagcccctgacgtgcggaatgatcgttctgctggaacgttggtgccggatagtagcgaacgcgtgttgacgtcgaagcgcccagtcttcagctgcctggcgcccagcgatggggcagcagctcgccgagtcgcgccaggtgtgttggcagcgatctgtagcttctcgtcggaaaacggtgtgtgggaggcgagagtttcgcccttagttaggcagccttcatttgccacggcttgaaccggcagaatcaaatgcggggaggtttgcgcgaagccgcagcagattgaattcctcgatgaccgccgcctcgatctcctgttttgtggtcggctcatcgtcaaacatgaaattcagcgaagcgcggtgcccgtcgaacgtcgcaattgcgtactcaagccagttgtcatatccccctggtggaggcggaagtgttttgctcgtgcgtgggggcatgactgttcctgctagttgttatcagccacggtgtacccgaccatgccgatagctatcgccaacaccgcgaaaacgaccagcctgcacaaggcaacaaggtaaaggcacattggacttgtggtgtgaaagaacgtccgtgggctgatcgtactcagggtggaaccattttgtccacgtccagtcaccccaacacagaggttcgtcgatagagatgcggcccgcgtagaggtgctgaacgcttgcagcccttgcttctcacgttggtggagcgggagccgtggaactccatgctccttcggctgaaacggatcaccgcaggcaacaaagctgggtgcggccgtgcgatagacagcaggtcgcgctgctcgtactattctctgcagaatgacaggaggggcaacgatggctgcgactcaacgaaaacttctgcaggcgctcgactacgtcaccatggggagcggcccacagatcgagacgttgggttcggttcgcgcgtcgcacttcaggaaggtcaatcacgccgccgaagacgacaacgtcgtcgccatcggcattagcgagaagttcgtcgagaaccgcgcatccggagagctcacgctttgcttctacgtgaagaagaagcaaccgcccagtcgggtctctgtcgacaaggctattcctggcgtcatcaacatgcctggcgacgaagctgtgttcacagatgtcaaggaactcggcgaggtggtgccggagatggcgcttccccaaagaaaaaaaaagccgatccagagcggtttcagtgttggccatttcaagatcaccgcaggcaccgtgggcgccatcgtgcgcaagggcggcaggtaccacattctgagcaactcgcacgtgctcgccgatagcggcaaaggctccgccggcgacgcggtcctatatccaggccccgatgacggcggaacactcgcccacagccaagtggcacggcttgcggagtttttcccgttcgacaagagcggcagctacgggaatcagatggacgctgcgctcgccgagatcgatgaagcgcaggtaccgaatcttgacctcgcgatccatcgcgcggcctaccctctgaagatggcggtcgccaaacgcggaatgacggtagtcaagtcaggacgaacaacgggtaagtccgaaggaaatgtgatcgacgtcaacttccgcgtgctgctgacgtatccgggcgtaggcaagatcggcttcctcgatcaggttctgtgtacccggtacacgggcgggggcgactccggatcgcttgtcgtggacaaggacacgggaaagatcgtcggcctgcacttcgcgggtgcgaacaatggaagcgtgttcaaccccatcggtgtcgtgaagaaggcactggggttccgattcgtagctccgatctgatggctaccgagaaggctgccaacaaggcgcgcgagcagttcgctcaagaactcttcgaccagggcgtgcatgcgctgcaggtcgacgcgctggagggtggcaaggccttctgcctcatcgctcacgttccgcagaagttcggaaaaagcttgcccaaccagctgaaggtcagtctgggcaccaaggaagtagaagtaccgctcgtcgtccgggagtcagaacccttcaagccggagtgacgctttttacccgccaatggcaggaagaggatgaacatgcccgcattcgtagaacgcaagctcccgcaagatggcccccaggccgtgagggccgcggagttcgaactggaactggtgccgcgcaactgcaggttgtcgcagtacgagcggctcgcaaacatacgcccggtgaacgtcaccgacgaagtcatcgcgtacgcttccccggactccacatacgcggtgacgaagaagttcttcgacgctgctaagaagtcgatccgcatcggcatctacgacttttcgtcgacgtacatgaaaaagctggtgctcgacgccctgggacgtggcgtggaggtcacgctcatgctggacctggacggccagaaggaagagcgagttgtgcaatccctggaggaaatgggcgctgagtgtgtgcccgcacccgcctgctccagccagcggtccaagtatttctcgtcgtgtcaccagaaattcatagtgatcgatgacgtctggacgctcgtgcaaagcggcaattactccgaccacagcattcctctcaatgagctcgacggcggagacccggacaacttccgcactggtaaccgagatacgggcttggccatcaagtcacgcaagctcgccactttcttcacgaaggtgctgcgctcggacatcgagctcgagctgagtggcccggaagccctaggcgcggtccgtgcggaggagccgatgttcctcgttgaggccgcgcccacgaagatccccaaggacctgttcaagagcaagagtttccagttcagcgcggataagcccctgccgatccttcccgtgctcagtcccgacaactacatggacgtgatgccggacgtcctgcgcacagccaggaaatccatcctcatcgagcagcagtacatccgcggcgcgcaggccgacatcaccatcctgctggacgccgtggccgaggctgtcgaggccaatcctgacctcgacatccgcatcgtgctgggcaagctgttcgacgccaaagacgtgcccaaggagaagttgaatctcaagcacctgaaagacacgtataacttgatgctcggcgccaacatccggtttatcaacgaggaccggttcgtccactgccacaacaagatgatcatcgtcgatggcgccaccgtgctcgtgagctcgcagaactggtcggattcggcagtaagcaagaaccgagaggccggaatcttgcttaccaacaagccgatcgcgaactatttcaccaagatctttgagtccgactgggcgaccgccgcgtccaaggtgccgtctccaggcgcgaagaccatcggtccggagacggtgcgcaagggcggctacatccaggtcgccgctgccgactatcgcgaagtctgagctttctacaggtatcgctcaggagcctgtcctgaactggttctgcgacagccaaggagaccgactccagcttcaaacgctggattgcgctcacgcgcctttccacgcacccctgaacagccgcatcggggcggtacagccagccggatccgattggtctcgatggaggatggaatcggtttggccatgttcgggcgatccgttcggcatgtgccgaggcgcattgaggggtggtcgctcagccctcgctctaaagcactctcagcttccgcgaaaattcttgctacagttgcccgcatggggacactcgtggccgaccaaatcactttcggaaaaccgccggtcaatgaagttgtgctcggaaggcacttcctccagcggcctgacttcgtcgcgccctactttggaacgttctggagcaagatccgtgatcgattcccgaaagttgagcaaacccaaccggtgttctcgccccaagagattgttttcctggacccaggcaccgtgcagccacgggtttggtatgtgtcggccgaccaggcgatgctggttcagctccaacaaaatcgcttctattacaactggcggcaacggccggccggagtgcaatatggccgatttccggccttgcttcgtgagagtttggacatctgggagctgttgaatgaggtcgccgtcgagctcacgggtcgtcctttccagacgacgggtggtgaaatcacgtatgtcaatttcatcgaaataaaggaagcttcgccaacggaaattgcgcaacaatcgttgtgtgacttcttctggaataaaaacgaacgttttttgcctccgccgagtggcttttccaggatgctgaattttcctctgccagaggcaaagggggtacttgatgtccaactgggaatcgcgaaaaacgtgcaaacgggcaatgatgccatcaggctggagctgactgcccacgcggcgttggtcgaaggtgagtcgtacgaagactggatcaatgtggcccatgatttcttggttgctgcgttcaaggacctgacatccagtcaaatgcataagatttgggaactccaggagtagaaatgacatacgaagcggtgctccccaaccctgcctcacgtggcctctccaattttggacagccctttcaagatcctcgcgcgttcggcgtgccgccatcgggtgccgtgatcggaaatggtttggaggagttggatcgattccaagcggtcgaacggaagctgcttgccctggattacgcgttcttcgaggactattcaaagtcgctgaatgatttctccagagaggcattttcagtattcatgcgccaccagccatgggccagtctcccgttgctgggcgccgaatccgatggaagtttgatcgccacctgggaaagggatggtgcatgtttgaccattcgctttgctaaccggtacgaaatagactttgcgatctccgttggtactggtgaaggtgcacagaggcattggggaaagagccagattgctttcttcattgcggagcatacgcaggcagcaagaatcatctcgcgctgaagtgccgttgccactcactgattcggtcgctcgcacatgccgtgcagctcaggttgatgggggaaggccgactccggcggcattcgaattgcgctacacagaggcgggccacgaagcctatgtttctgtgaactggcttgaattccttcatcagggggctgccgactaccagaccaagctgcaagtgcttcgggaatggttgctggctcggccgaagggcgaagtgattgccccttcaaagaatggtgtgctggccgtccttcctgtccaagccgtccaaggaatgccactatccgcggccaacggcagtcttgactgcgcgcacgagcctcgtcacgaaggcgatccccacagtggaattcggcctcagcctggtgttgaaacgtggccccgccaagaagatgcgccgggccgacttgccgttcagcagttcctctttcaggccgtttgccatttcgaggctggtcgctagcaaagaccagaacgggctctactggcaggatgccggtcgcgcctgaggaagaagtgcgcgtcatcgatgacgtgccgttgcgcggcgggtttcgcagatcactgaatcggtgccctctcaaagcaaggcgttgactggcgaagaggggccgccttccaccggtatcctgtcaccgaccgccgcggcgctgaagtggcttgaagtccgtgacagtcccaaaggagtccggttcgcgggccggaaaagcacacgtggtcattcttgcgagaccgcatcgccaagcgacaggacgctggttgactgtggccgctttttcccaccagaggccaggactgcggaagctatgccgttcgccccggatttctcgcgggcgctgatggtgactaacgcatgggagatcacgtttctctaattcaagagctaaggcgcccggctgaccgcggttgttctacagcccggcttctgcggccagttctgccacggaaatcccgattccggcagcaatgcgaaccacaaccatgacgccggggttctgagtccctcgctcaatgctgctcatgtaagacctatcgaccttgctcctatgagctaactcctcctgcgtgagtccgcgcgcttggcgggtcgcgcgaatagccattcccagcgccaccagcgcaggatccagcgcgtgttggggcgaaggggtcggcatggacaaaatcgtccgcgaatgcatacgatcgcaccacggacgatcttccacataagggcctcccaatgtttcgtgtcgacagtcgttttgagatccacattcctccgtttcctggggatcaaggtcagaaggtgcagcagtttcatttcgtcgagcagtgcttcaatgtgccgttgtggcatatccaagtacttccaagggcggtcggcgaggatgacttccagcgatggaactgctatttggcgacgcgcgccagcgacgcgctgggtatcttgctgggacagcgatgggagagcagcaagctccatgttgtcctaccgcaatacctgatccgcacggactcgatcgccctggctaggtgcagcgcgctttgggagtgcagggttaacggtcagagcaactcagctgctctgatgttcgatacaagcctggggtcattcgtcgacccggagttcgaggtgatcgaaacggccaacgtgcagagaaccgcagttagatggagggattcggagattgccggcgtggatttacatgcgcaaagcaagcgcgcctaggtcaagagttatccacattcgattggccaagtttttccgtaccccaaaacgggagggaaagcgtagtcacgacgctaccttgctcagctgagaaaaaaagcgcttgactacatctgatgcgcttgttgttcggaaattcgaggccggcattctggatggccgaccgcacgcgctcgcgggcttccttgacttcggtttccgccagcccgacgagcgtgaagctcggcaggccgttggccaaatgcacctcaaccgtgacactggccgcttccagcccaagcaaagcacggctttgcaccaaagacaggctcatttttattactctccccattgtggtgctcccattttgggttgggctcgtgcaccgccggggcctggaagccccgcacatgaaacgtttgtaatttttcatcggggtttgtggatcggcgggccacaggcgcttcgaagggtgaacgagcactttggcacgctccctgctacgaaacggtgtccccccaacttccaaccaaccccgaggagtctcgatgatgcaccgtaaattcgcccaggcaatggccgtggccgcccttgccgccctgccgatgctggcgagcgcccaacttacgggcaacgtggccctgaccagcaactacaagttccgcgggcaggaccaggacatgatcgggaagaacgattacgcgaagaccaagggcttcaagcccgccatccagggcggcttcgactacgcgttcggcgaaagcggcttctacgtcggcaactggaactccagcgtcaactggctgcagggcaacagcatcgagagcgacctctacggcggctacaagttcaaggccggcccgttcgacctggacgtgggcgcactcacctacatctacccgggcaactccatcggcaacaccaccgagctgtacggcgcgggcacctgggccgacgaagccgtcggctcgttcaccctgaagtactcgcacacggtgtcgaaggactacttcggctacgccggctacaagtcgggttcgggcctgaagggccgcaacaccggctacctgaacctggcctacagcaaggaaatcgtgcccaagctcacgctgaaggccgccgtgggctacacccgcatgtccagcgacatccgcagcctgggctacaagagctacgtggactacaacgtgggcgtgtcgtatgacttcggcaacggcctggcactggccggctcggtgcagggcgccaacaagaagagctcctacctggcggtgagcaacccgggcgtcgacttcggcttcggcaccttcggccagcagacctactcgccgaacaaggcgcgcttcatcgtcacgctcagcaagacgctgtaaacaagcacaagaacaaggtgcggcccaagctgccgcaccattcattccatccaagaaggagaaagtcatgaagctggtcacagccatcatcaaaccgttcaagctcgacgaggtgcgcgaagcactgtcggccatcggcgtgcaaggcatcacggtcacggaagtcaagggttttggccgccagaagggccacaccgagctgtaccgtggcgccgagtacgtggtcgacttcctgcccaaggtcaagatcgaagcggcggtgtccgacgacctcgtcgaccgcgtgatcgaagccgtcgagggtgcggcgcgcaccggcaagatcggcgatggaaagatttttgtctacaacctcgagcaggtcgtgcgcatccgcaccggcgaaacgggccgcgaagccctctgaccagcccaggctcgaaagaacaacgactatgaaaaaactgcttgtctctcttgcgctcggcttgagcgtgctcactgccgctttcgcacaggcgcccgcgcccgccgcggaagcgccggctgcatcggcaccggctgccgctgctccggcacccgcggccgcgcctgctgctgccgccccggctgcagcagcccctgccgccgccgaggcagcgcccgccgcggctcccgctccttctttcaacaagggtgacaccagctggatgatgctgtccacgctgctcgtcatcatgatgaccgtccccggcctggccctgttctacggcggcctggtgcgcagcaagaacatgctgtcggtgctcatgcaggtgatggtcaccttctcgatgatcgtggtgctgtggctcatctatggctacagccttgcgttcaccgaggggaatgccttcttcggcggattcgaccggctcttcatgaaggggatcttcgatccggccactggcgtgttcgcgcccgccgccaccttcagcaagggcgtctacatccccgagctgctgttcgccgccttccaggccaccttcgccggcatcacctgctgcctgatcgtgggtgctttcgccgagcgcgccaagttctcggccgtgctgctgttcatggtgatctggttcaccttcagctatgcgccgctcgcgcacatggtctggttctggatgggcccggacgcctacaccgccgccaacgtggtggatgcacagaacgccaaggccggcctgatctggcaatggggcgctctcgacttcgcaggcggtaccgtggtgcacatcaacgccgctgtcgccggcctggtcggtgcctttgtgatcggcaagcgcgtcggctacggcaaggaagccttcacgccgcattcgctcacgctcaccatggtcggcgcttcgctgctgtgggttggctggttcggcttcaatgcaggttcggccctcgaagccggcaccagcgccgtactcgccttcatgaacaccttcaccgccaccgcagccgcggtgctcgcatggtgcatcggtgaagcactgatgcgcggcaaggcctcgatgctgggtgccgcttcgggcgccgttgcaggcctcgtggccatcaccccggccgccggcaacgtcggcctgatgggcgccatcatcatcggcttcatcgccggcttcgcctgcctctggggcgtcaacggcctcaagaagctgctgggcgcggacgactcgctcgacgtgttcggcgtgcacggtgtcggcggtatcgtcggcgcgctgctcaccggcgtgttcaacacccaggctctcggcggccccggcctcgtgggcgactgggtcacggccagcgtggtgtccaacggcatcggcgcgcaggtctggatccagctcaagggcgtgctgctgaccatcgtctggtctggcgtggtggcgttcatcgccttcaagatcgccgacctcaccatcggtctgcgtgtgtcggaagaagaagagcgcgaaggcctcgacatctcctcgcacggcgagaccgcatacaacaggtaaccccaagcaataggcaaccccccagtcttcgcgcacttcgtgtcgcttcgccaacccccctgctgggggcaacaccagaggcccggcaaagccggttcctcggtgttccacgaagaaggcatacgacgcaaaggctggttataagaaccacaagaagcaatcctttttcagcaaggtctcctttggatgttcagcccgcgagcgcttcggcgccagcgggcttttttttgtcttcggggcagcggatgcacaatccggagatcatgtggaccaccctcgaagacagcctctgcgaactcggcgaatcgccgttctggcacccgcacgaacgcgcgctttactggctcgatatcccggggcgcgcggtgctgcgcacgcgcggcgacatcggcacgccgtcggccagggtggagcgctggggcttggccaccgaacccggctgcatggcgccggccaggagcggcggcctcgtgatcgcgctgcgcgacggcatctaccgggcccgcgaatggggcggtgagctggtcgcgatggcgcgtgtcgaacacgacgtgcgcaccatgcgcttcaacgacggcaaatgcgatgcgctgggccgtttctggggcggttcgctcaacgaggccaaggaccgcgccaacgccgcgctctattgcttcgatgcccgtaccgacaccggcgtggcccccacattgacgcagatggccaacgaggccaccaccgccaacgggctcgcgttctcgcccgatgcccgcaccctctactgggccgacaccgccgcgcacgtggtgtgcgcctggaactgggacgccgaggccaattcgctctcgcatgcgcgcgtgttccaccagttcgaggccaagcccgaaagctggacgcctgaatcgcccgtgcgctatgaaggccggcccgatggcgccaccgtcgatgcggagggccactactgggttgcgatgttcgaaggcgcacagctgctgcgcttcgcgccgtcgggcgagatcgtcgcctcggtgcccgtccccgttcagtgtccgaccatgccctgcttcggcggcgacgacctgaagacgctcttcgtcaccagcgggcgcaagggtcggcctgccagcgagatcgagcggctcccggcctcgggcagagtgatatcgacgcgcgtcgcaacgcccgggttacctgtcaacttcttcgaggactaggttgaaaccttgtctttctgcctgttgcgttggggatgattcgtggggcgctcccgccgacggggtaccttgctccgcgaatgtcccccggcctgcggcctcctcctttatttcgctgcgcaaggcaccccgccagcgggagcgttggtcagagcggtggttgatcagccagcacaacggcagcgcccggtgtgcacagggcgccgggtgctccccgcagcgaaataaaggaggagccgaaggcgggggacattcgcggaggggagtacccggtggcctgtgcacgcgccctgaacaacagcgccctgaacaacagcgccaagaacaacagcgccaagaacaagacagaagagggtaaagacatggccctccagcacatcccacccatccagtgcctcctgaccttcgaagccgtggcccggctgcgcaatgcaagccgcgccgcggacgaactgtgtgtcacgcccagcgccgtgagccaccgcatccgccagctcgaatcgcatgtgggcttcaagctctttggacgcagcgacttcagtctcactgccgacggcgcggcctaccttgccaacgtgcgcaccggccttgcagcgctgcaggccacgcccggaggcaacgcggcgaagcagcagcgcgcgacacgcctgcgcatcgccgtcacgcccaccttcagccgcgtgttcctgatgcctcggctcgaattgttccgcaacatctaccccgacatcgaactggtgctgcaggtgtcgatcccgctgctcgacgtcacggccgagcaagccgatctcgaagtgcgctatggcagcggcgcgtacgccgactgcgaacaccgcctgctgctcgaggaagaagtggtgcccgcctgcagcccgagctacctcaacgagttcggcccgttcaatggtttccgcaccgcggccgagattgcgagcgcacggctgatccgcagcccgctcgagccctggggcacctggttctcgagctgcggcatcgaccagcccgagccgcacgtcggctcccagttcaacgatcttggccttgtctacgacgcagccgcgagcggcttcggcgtggcgctggtgcgcctgaagatgggcgccgcctggtttgaatcgggccgcctggtgccgctctccgaccggcccgtgccttcgccacaccgccacaccatctgctggcagcccggcacgctcgatcggtgggagtgcgccgcctttgtcgactggctggcgcagagcctgcgctgagaagaaggtgtgggcccgtgccgcacggcgaagttctctcaagcccgacgcgaaaaagcttcaacccggcgccgtcgcatttgcgtagagtgcgaagcaccacgagacatacaacacatgaacgcgccgctcaccgccgtccagcacgactcgccgcagaaaagcgatcgccagtcgcagatcgtgcgcgccctgcaggcccacctgccggcgcatgcgctcatctggcatgccgaggacaccacgccctatgaatgcgacggcctcaccgcctaccggcagcggccgctggtggtggcgctgcccgaaaccgaggcccaggtggcggcggtgctcaagacctgccacgggctcggcgtgcccgtggtggcgcgcggcgcgggcaccgggctctcgggcggcgcgatgccgcacgcgctgggcgtgacgctctcgctcgccaagttcaaccgcatcttgaagatcgaccccgtgggccgcacggccgttgtgcagtgcggcgtgcgcaacctcgccatcagcgaagcggccgcgcccttcaacctctactacgcacccgatccgtcgagccagatcgcctgcaccatcggcggcaacgtggccgagaactcgggcggcgtgcactgcctcaagtacggcctcacgctgcacaacgtgctgcgcgtgcgcggcttcacagccgagggcgagcccgtcgaattcggcggcgaggcgctcgacgccccggggctcgacctgctcgcgctggtcatcggcagcgaaggcatgctggccgtgaccaccgaggtcaccgtcaagctcgtgcccaagccgcagctcgcgcgctgcatcatggccagcttcgacgacgtgcgcaaagccggcgacgcggtggccgcggtgattgcggccggcatcatcccggcgggcctggagatgatggacaagcccatgaccgccgcggtcgaagacttcgtgcgcgctggctacgacctcgatgcggccgcgatcctgctgtgcgaatccgacggcacggccgaagaagtcgaagaagaaatcggccgcatgactgccgtgctgcgctcctccggcgccaccgccattgcggtgagcaccagcgaagacgagcgcatgaagttctggagcggccgcaagaacgcctttccggcatcgggccgcatcagccccgactacatgtgcctggactccaccattccgcgcaagcgcctggccgacatcctgctggccatccaggagatggaaaaaaaatacaagctgcgctgctgcaacgtgttccatgccggtgacggcaacctgcacccgctggtgctgttcgatgccaacgaccccgacgagctgcatcgctgcgagctcttcggcgccgacattctggagaccagcgtggccatgggcggcaccgtgtcgggcgagcacggcgtgggcgtggaaaagctcaacagcatgtgcgtgcagttcaccgcggccgagaacgagcagatgttcggcgtcaagcgcgccttcgatccggccgggctgctgaaccccggcaaggcgattcccacgctgcagcgctgcgccgaatacggcaagcaggtggtgcgcggcggcaggctgccgcaccccgatctgccgcgcttctgagcaaaaaaagacatggaacccgcactcagccagatcgtcgagcgcattcgcgccgcggccgccgatgccacggcgcttcgcatccgcggcggcggcaccaaggatttttacggcgagccgccgcagggcgaggctttgagcactgccgggctcaccggcatcacgagctatgaaccgagcgaactggtcatcaccgcgcgtgccggcacgccgctcgccgaactcgaggccgcactggccgggaaagggcaatgcctgtctttcgagccgccgcatttcggcgcggctggtggcgcaggcaccgtgggcggcatggtggcggccggtctcagcggccccgcgcgcgccagcgtgggcgcggtgcgcgactacgtgctgggcgccacgctggtcaacggccgcggcgaggtgctcggcttcggcggccaggtgatgaagaacgtggcgggctacgacgtctcgcgcgtgctcgcgggctcgctcggcacgctgggcgtgattgccgaagtgagtctcaaggtgctccccgttgcgcccgccgaggccacgctggccttttcctgcagccaggccgatgcgctgcgcctgctcaacgagtggggcggccggccgttgccattgaatgcgagctgctggttcgaggatgcgcgcagcggcacgttgtggctgcgcctgcgtggcgccgccgcggcggtggaagccgcctgcgcgcaactgggcggcgagcgcgtggacaacgccgccgccgctgccgggtggcaatcgctgcgcgaccagcagcatccctggttcactgccgatgacgcaggcgccgcgctctggcgcctgtcggtgccgcagaccgcgccagtgctcgccctgggcaatggcggcgcgcccctgatcgaatggcacggcggacagcgctggtacaaggccccgcccgaacaggcttcgctcatccgcgaagcggcgcatgcggcaggtgggcatgcgacgctgttcaggatgccccctgcttccgtcgcggcagctagcgccggcgcccggcgcttcgacgccttgagcgcccccatcgcgcgcatccaccatgccctgatgcgtgagttcgatccccacggcctcttcgaccgcgcccggcttctcgcggacgcctgagccccagcgactcgacacctcatttctcgccatgcaaaccgagctcgcccccgaattccgcgacaccgacgacggccgcgaggccgaagccatcctgcgcaagtgcgtgcactgcggcttctgcaccgccacctgtcccacctaccagctgctcggcgacgagctcgatgggccgcgtggccgcatctacctgatcaagcaggtgctcgaaggcaaggcgccgacgcgcagcacccagctgcacctggaccgctgcctgacctgccgcaactgcgaaagcacctgcccgagcggcgtgcagtacgggcacctggtcgacatcggccgcaagatcgtcgacgagaaagtgccgcgcccggccatggaatcggccacccgctggttgctgaaggaagggctgccgtcgccgctcttcggccccgcgatggcgctcggccaatcggtgcgcgggctgttgcccgaggcgctcaaggccaaggtgcccgcgaagcaggaggccggcgcctggcccaccgccacacatgcgcgcaaggtgctgatgctcgcgggctgcgtgcagccgtcgatgatgcccaacatcaacagcgcgaccgcgcgcgtgctcgatgcggcaggcatccagacggtgatcgcgaaggaggccggctgctgcggcgccgtgaagttccacctcaacgaccaggagggcggcaaggcgcagatgcgcgccaacatcgacgcctggtggccggaggtcgagcgcggcccggaaggcggcggcgtcgaagccatcgtgatgaacgcctcgggctgcggcgtcacggtgcgcgagtacggccacatcctccggcacgacccggcctacgccgccaaggcggcgcgcatcagcgagatgacgcgcgatttgagcgaactgctgcccgacctcgttcctgcgctgaaggctcgcgtgcgtgcgccggccggcgtggtggcctaccatccgccgtgcacgctgcagcacggccagaagctgcgcggcggggtcgagacgcatctgcgcgcgctgggcttcgacgtgcgcgtggccatgaacgaatcgcacctgtgctgcggctcggccggcacctactcggtgttgcagcccgaactggcctacccgctgcgcgaccgcaagctcgggcatctgaagcaactgcagccgagcgtcatcgcttcggccaacatcggctgcatcacgcatctgcaaagcggcagccaggagacgcctgtgcgccactgggtcgaattgctggacgctgcgctgctggcgacggcctgatcgcacaccgaagagcgccctggtccgactcgcgcgggggccgctcgcacggcatcatggctgcaccgtttttcccaggagtcagccccatgtcttccgttcaagctttcatcgtttcgaagaacttgcggcgtgccttgctggcctgcgcctgcgcggccggcgccttcggggcacaggcacagtcggccatgccgcagtggaagggcgagggtgcggtgcgctatgtctgcggcggtatcggctcggacgaatcgaacgccattcgcgccgccatgaaggaccatccgctggcactgcttttcgcgcgcgccgacggcgcctatctggcggacgtgcaggtcgacatcaagggtgccgacggtgcgccttcattgacctggcgcgccagcgggccggtctgcctggtcgacattccggccggccgctacaccatcagcgccaccacgaccggcggcgacgccaagagccaatcggtgacggtgggcggcggctccaagaccgccagcttccgcttctgagcgagcgtctcagccggccgccagcgcggcctcgatgtcccgcgtgagcgaggcgggcgtgtcgagcggcgcatagcgccggagcacctgcccgtcgcgcccgaccaggaacttggtgaagttccacttgatggcggtgctgcccaggagcccgggcttctccttggtgagccactggtagagcggcgtggcattgctgccgttgacgtcgatcttttccatcatcggaaaactcacgccgtagttggtggtgcagaaggcgccgatttcctcgttggtgcccgggtcctgcgagccgaactggttcgacggaaagcccagcaccacgagccccttgtcggcgtacttttcgtgcagttcctcgagccccgcgaactgcggcgtgaagccgcattggctggccgtgttgacgatcagcagcaccttgcccttgaaggcggaaagcttcacgttcttgccgtcgatacggttggcttcgaagtcgtagatgctggccatggaagtacctcaagtgggagacgaaaggcgatcatcgccctctgccggcgttcgcgcaaacgccgaccacacggccgccagcacgatcagtgcgccgccggccaggatgcgcggatccatctgggccgcgccgagcgccacggaagagacgctggcgaacagcacctccgacagcatgatcaccgccgtggcgctggccgccagccgggccgcgccgtattgcaggcagacattggccaccacgaagccgacgcccagcaaggcggcccacgcgatccagcccggcgtggccgacaggggcgaggcgaaggcaccgagcagggtgccgctcgccgcggcgatgcccgccaccagcgcgcagccgcagaacatcgccagcgcacgcgattcgccgggcgcgccgtgcaagtggcgcagcaggatgttggtcacggcaaagctgaagccggccgccacgcccagccagtccggcaggctcgaaggcaccggccagtcgacacccggcgccttcagcaccacgaccacgccggtgagcgccagcgccacccgcgcgagcgcacccgccgtgggccgctcgcccagcaccgcccagcccagcagcacgctccacagcggcatcaggtagaacagcagcaccacgcgcaccacgtcgccctgcgtcacggcccagttgaaaccgaggttggtgaaacccgccgccaggcccagcgccaccagcatcggaaacgccgcgaagccgcgccaggcatgccggcgaaagaaccccatcacgagcgagatcgccacgtagatcaggcaagtggtccacacgggatgcagcccgtggctttcgatgtgccggaacgggaaccaggaaacgccccagacaaaggcattaaaaatcagtgctaaagcaggcatgggaggcggacttttcgtggaacaccgtggaaccggctttgccgggccaccggtgttgcccccggtgagggggtgggcgaagcgacacgaagtgcgcgcagcctgggggaggtcaatgatgcttgtcgctacgggcgatggcgagcaggtgctcgacttcttcggggtacttgcgcaggttgtgatgatgccagcgctggatgagccacatgcagccggccaccacgccgccgaaggcgccgatggccgtgaaggccgacaggcccaggccggtgcaggcgctgtagaagccgccgagcagcaggatgcaggcctgctcgttgaagttctgcacggcaatcgagcggcccgcgcccatcaggttgtggccgcggtgctgcagcagcgcgttcatcggcaccaccaggaagccgcccagcccgcccagaaggatgaggaagggcacggcgatccagacattgctgatcaggttcatgctgatcaccagcaggcccatgccgatgcccatggggatcacgcgcgtggccatgtccagccgcatgcgcatcgaggcgacgatggcgcccaccgccatgccgatggtgaccacgccggtgagcgccgtggcctgcgtggtgttgtagttgagcgcgagcgcggcccaggccagcacgatgtacttgagattggcgcccgcgccccagaaaagcgtggtggtggacagcgagatctggcccagcttgtcgcgccacaggcgcgcgttgcagtgccagaaatcgggcagcagcgagagcatgttgcgccccaggccgtgcgccggatcggcccgcagcggccgcatctcgacgccggtgtgcggaatgcgcgtgttgaaccaggccgccagtgcatagacgaagatcagcaccgagatggccgcctcggccggcgaatcgaccccggtgttgatcagcggcaggtcgatggacagcagctgggtcgagaccgcatggcccaccagcgaaccgccgagcacgatgcccaggagaatcgaagcgatcgtcaggccttcgatccagccgttggcttttaccaactgcgaagccggcagcagctcggtcaggatgccgtacttggcgggcgaataggccgcggcgccaagccccacgatcgaataggccagaagcggatgcgagccaaacagcatcatcaggcagccgacaaccttgatcgcgttgctgatgaacatcacccgccccttgggcaaggcgtctgcgaacgcgcccaccagcggcgccagcaccacgtagaagacagcgaagatcggcaccagcgccgcgcgctgccattcggccgctcccgtgcttcgcatgagctcgacagccacgacgaagatcgcgttgtcggccagcgacgaaaagaactgggccgacatgatcgtgtagaaaccgcgcttcatcgatgggctggctggccaggaaggttgctggcagtagtgagaaagtgttgcgacgtttggcgaatgggcggttatagcatgggggtacgacggcgaaatcagcgttgccaacctggacagccctgcttgcgaagatgctaaaaccccgtcttcaccatccgacatttgccatgccgcgtcccattctcgccactgttcacaccgcagcgcttcgccacaacctcgatcgggcacgccgcgccgcgctcgatgcccgcgtctgggccgtggtcaaggccaatgcctacggccatggcatcgagcgcgtctacgagggcctgcgcggtgccgacggctttgccctgctcgacctggccgaggccgaacgggtgcgcgcacttggctggcgcggcccggtgctgctgctcgagggcgtgttcgatgcgcgcgacctggagctgtgctcgcggctggacctgtggcacaccgtgcactgcgacgagcagatcgacatgctcgcggcccacaagacgctcaagccgcagcgcgtgttcctcaagatgaactccggcatgaaccgcctgggcttcgcgcccgagcgcttcggttccgcctggacgcgcctgaacgcactgccgcaagtcgacgagatttcgctgatgacgcatttcagcgacgccgacggcgcgcgcggcatcgcacaccagctggcggtgttcgagcgcgtcacgcacgacctgccgggcgagcgctccattgccaacagcgccgccaccctccgccacgccgaacagacccggggcgactgggtgcgccccggcatcctgctgtatggcagcgcgcccgactttcctcagcacgacagcgcgcactggcagctgcagcccaccatgacgctgtcgaccaaattgatcggcgtgcagacgctccaggccggcgacaccatcggctacggctccaacttcacggccgacgggccgctttccatcggcgtggccgcggtcggctatgccgacggctatccgcgccactgcaacaccggcacaccggtgctggtgaacggcgttcgcacccgcatgctgggccgcgtgagcatggacatggtcaccgtcgacctcacgcccgtgcccgacgcgaagttcggcgccgaggtcacgctgtggggccgctcggccgtgaccggcgcggtgctgcccatcgacgaggtcgcgcaggcggccggcaccatcggctacgaactcatgtgcgcggtggcgccgcgcgtgcccttcgctcccgccgaccacgaatgaaggtgctctccaactggcgctcggtgcgcctgtgggagacgcagctcgagcgcgacctgcaccgcaactacagcctgcgcacgcatggcatcctcatcggcagcttcacgctgctgctgatgtggggtgcctctgcattgcagatgcatgtgctcgacgtgcagtcgctggcggtgcgctatttcctcacgctgggcgtgggatacctcggctacctgctggtgctgcgctggtgggccaggcgtctggtcgagaaccggtccgacttcaacgtcgacgggggcgacatcgccgatgcggctgacttcgcgctcgatgcgggcggcagcagcccggcaagcagcgccgagggaagcgcgctgtccgacgccgccagcggcgcactcgacatcgcgggcggcgccgacgaaggcgcggtcatcgtggtgccggtggttgccatcttcctgatctgcaccgccatcgtgctcggcgccggctcgctcgtgctgctttacttcagctgggacgcgctgctggccgtggccgtcgaagtggcgttctcgtacgtgtcggcccgcgccgcggtgcgcgtggcgcgcgagggctggctgatggccgccgtgcggctgacctggaagccgctgctcggcgcggtggtctgcgccgtggctctgggcgccgcgctcgaccacttcatgccccaggtcaactccttgcccgaggccgtgcgggccctgctgaagaagcactgagcttcttccggccgccgtcctgggcagccagcgcatccagcagatggtcgatcagcacccggcacttgggcacggtgaagcggctgggcggatagaggatgtaggcgtgcccgcggtagttgccctggaactcccagccggccagcacccgcacgacgcggccgtcctccaaggcctcctgtgccatgaaggccggcacgcaggccacgcccagtcccgcgagcgcggcttcgagccgcacctcgctgtggttggagacatagcggccccgcaccaccacctcggcttcgtcttcgtcgcccttcctgaagcgccaatggttgtcgcgctcgtgctcgccgagcgagaggcagctgtgcgcgagcaggtcgcgcgggtgttcgatggcgttgccctctgccaggtagcgcggcgaggcgcacaggatgtgcgcgaccggcatcagctgccgtgccaccagcccttcgggtggcttcgtcgtcaaccgcaccaccaggtccacgccttcgcggattggatcgatgtcgcggtcgtccacgatgagctgcacgtcgacctcgggatggcgctgcaggaagtcgaggatgtgcggatgcagcacgcgccgcgcgaaggccttcggcgcgctgacgcgcaccagcccgctcggcttcttcgagaactgctgcgcaatgtccatcgtgccttgcgccgccagcaccagttcgcggcaccgcgcgaaggcctcgacgccgggctcggtcagccgcagctggcgcgtggtgcgctggatcagctgcacgccgatttccttttccaggcgcttcacctgccggctcgcggcagagggcgtcatgcccagcagatcagccgccgcggagaagctgcccagctcggcgacccgcaggaaggtcaccatctccggcagcactttgagaaatgaattcgttcccacggcgcaagggtcctgttccggccgaaggctgttcggcccgtgtgatgcccggaacaattctttctttagttgttcaggacggtgggccgacagtatggattcaaagcaggtgtgcggcatcgccccggtcgcgtggggcgagagaaagtgggccggcatcggcgccgccgagatcatgctgctgctcgtggcggccgtgtggggtggcagctatgcggtggccaagcaggccacgcagcagctgcccgtgctggagttcatcgcgctgcgcttcgggttgaccttcgtcgtgctgctgccggcgctcaagccgctcttcaacgtgcaatggcggcaaggcgttgcggtgggcggtctgctcggcgccaacctgctggcgatcttcgtctgcgagacgttcggcgtgtcgctcaccacggcgagcaacgccgcgttcctgatcagcctgtgcgtggcgctcacgcctttggtcgaatggtggctgctcgggcagcggccggaacagcgcgtgttctgggcagcgggcctgtcggcggcaggcgccgcaatgctgtcggccacctcgcccgcggacatctcggtggggtggggcgacggcctgatggtgatcgccgctttcctgcgcgccgtgatggtctgcatgacgcgacggctcgccggccgccattcgatgccagcgctgacgctgacggcagtgcagtcgggcgtgatggcgctcggcgcggcggtgctgtcgctcgccgtgtcgaagggcgcgtggcacgtaccgcctgccacggcctccttctggtggggcatggcctacctcgtgctgctgtgcacggtcttcgcgttcttcgcgcagaaccatgcggcctcgcgttcgagcccgagccgggtgtcgctgctgatggggagcgagccggtgttcggggcattgatcgcggtgtatgggttcggggagacggtcggggcctggggctggatcggcgggttgctgatcgtggtggcggcctggtgggtgacgatgccgcgaaaacctgtgatgggttgaggttggacgtgaagcgcccaatcaatacaggccaagctgccgcagcttcaagcgggcaaggcccagcagcgcgtcggtgaacggcgtggccaccccggtcagctcgcccagctcgcgcaccacggtcaccagcgcatcgagctccaccgatcgcccggcttccacgtcctgcagcatcgaggtcttgaacgcgccgagcttcatcgtcaccgcatgccggtcttccgggctctgcgtgatctcgatgccgatgcgccgtccgatgtccttcgcctccagcatcacggccgagatgaagccgcgcacgtagtcgtcgcccatgatcaggtcggtggtggcgccggtcagcgcgctgatcgggttcaccgtcatgttgccccagagcttgaaccacacgtccttctggatctgcggcgacagcgtggtgtcgaagccggcgctcttgagcagctcgacgagcttttgcacacgcggcgtggcctcgcctgaaggctcgcccacgatcagcccgttgccgaagtgatgccgtatcacgccgggcccgtcgagcgagcagctggcgtgcaccacgcagccgatcacgttgcgggtgggaatggccctggcgatcgcgccatcggggtccaccgccgccagccgatggccggtgatggcgccgccgaagccgccttcgaggaaccaccacggcacgccgttcattgcgaccagcacgagggtgtcgggcccgatcagcggcccgatgcgctcggccacgccggccagcgcaggcgccttcacggcaatgaccacgaggtcctgcacgcccagcgactcgggctcggcctgcgcgttgacgggcacgcgcgtgcgtacgtcgccgcgcatgagcgaaaggccatcgcgctgcagcgcgtcgagcgtggcgccgcgcgccaccacgttgaggcgttcaccggcccgcgcaaggccggcgccgatccaaccgccgatggcaccggcgccgtagatgcaaattttcatgaaagaggctgcctcagttgcaataactcggatcgatgcggtccacctggcgcaccagggcatcgaacacatcctgccccgcgccatgctcggggctgaactgcagcgcatcgcgcgtgcagcgctctgcgatgtcctcgctcaccggaatggccgcacccatcgagaaggtcgccatctggatctcgcaggcgcgttgcagcgtccagagaatcgcgaaggtctgcggcagcgtctgtccccaggccagcaggccgtggttgcgcaggatcacggcgttgcggttgccgatgctcctgagcaggcgcgggccttcgtcggcatggatggtgatgccctcgaagtcgtggtacgccaccatgccgtgcagctgcgcggtgtagaaattggtctgctgcaggccgccctgcaggcaggccacggccacgccggccgtggtgtgcgtgtgcatcacgcagtgggcaccgggcaggccgtcgtgaatggccgcatgcacggtgaagccggccgggttcaccggatggctcgaaccgtcgagcaccttgccctgcaggtcgatcttcaccaggttgctggccgtgacctcgctgtagtgcagcccgaaagggttgatgaggaactgctttgctccacccgtcacgctgtcgggcagccgcagcgtgatgtggttgtagatcatctcggtccagccgagcatcgcgaacacgcggtagcaggccgcaagctgttcgcgcgcggcgcgctcgtccggatggatcgagggatggaccagcgccgatggcggcacgggagtggcgagtgtgttcattgcagttccttcatacggttagccttcagcggtgaagccgacttccttgacgatcggcgcccacttggcggtgtctttcttcagcagctcggtcagctccgcgggcgtggaagacatggcttccagcccgaaggtgccgagcccgtcgatcacgtccttctgcgcgagcgcgttcttcatcgcggtgttcagccgcgcgaccagttccggcgatgccttggcgggcaggaagaaggcgaaccattcgctgtgcgccatgtcgtggatgccctgctcgccgaaggtcggcacgtcgggtgcgaagcggctgcgcttggcgcccgaaacgcccaggatgcgcaccttgcccgaggccagatgctgcgtgatgtcgccgatggggcccgacacggccgagatgttgccgcccagcaggtcgagcatggccggctgcgtgccgcggtaggccgcgtgcttgagttcggcgccgcccttcttgcccagcagcgcgccgatgaggtgcggcgtggagcccgcggcgggcgaaccgaagttggcgccggccgggttggccttggcccaggccaggaactcgggcaccgtcttcacgctggccggcaccgagggcccgaccgcaaagccgaagtcgaagatgcacgcgatgctgaccggcgtgaggtcgaccatcgggtcgtacggcagcttcttgtagatgtgcgggtagatcgtgaggatcgaggtcggcgtctgcaggatggtggtgccatcggcgggacggcctttcacgtagctcacggcaatctgcccgcccgcgccggtgcggttttcgaccacggcggatttcgcgtactcggggctgagcttctgcgcgatgcgccggcaggtggtgtccgaggtgccgccggcggcaaagccggtgacgatggtggcggtttcgatgctggcttgcgcaaaggcgtgctggcccaggctcgcgagcagcgccgaggcgccggtggtctgcagcaactggcggcgggtgaaggtcatggtttgtctccgggtgttgatagtgatttcacggctatgactcgtcgcgcagccaggtgactgcgcccgaatgggtcactgcgccctggtaggcggggcgcacggtgagggcatatttttccagcaagccgcggtggggcgcccccgcgtttacctgacgttcggagagccggcgcgcgatgtcttccgccgtcagttccaccgaaatgctgcgcgcctcggcccgcgcgtcgatggcgacgatgtcgccatcgcgcagcgccgcaatcggtccgccgtcggctgcctcgggccccgcgtagccgatgcacaggccgcgcgtggcgcccgaaaaacgcccgtcggtcaggagtgccaccttgtcgcccatgccctggccgtagagcagggcggtgatgcccagcatctcgcgcatgccggggcttcccttcgggccttcgtttcggatcacgatcacgtcgccggcttcgtagcggcggttctgcacggccgcctgggcttcttcctcggactcgaagacgcgcgccgggccgcggtgcaccagcgtctggaggcctgcggtcttgagcagcgcgccgtccgggcagaggttgcccttgagcaccgccaggccgccgtcgcgcgtgatcgggttgccggccgcgcgcaccacgcggccgtcgggcgcggcggcaccggccagctcttcggccatcgtgcggccggtgaaggtgagcgcgtcgccatgcagaaaaccctgctccatcagcgtgcgaagaatgacgcccgcgccgccgatgtagaacacgtcgcgcgccagatactgcccgcccggccgcaggtcggcaatgagcggcgtgcgcgcgaagatctcggccacgtcgtccaggtggaacctgatgcccgcctcgtgcgcgatggccggcaggtgcagcgcggcgttggtcgagccgcccgtggccgacaccacggcgcaggcgttttcaagcgccttgcgcgtcacgatgtcgcgcggcaaggggctgtcgcccatcaccgccttcatgaggttcttcgcggcgcggcgcatcagcggcgcgcgttcgctgaacaccgcgggcaccatgctcgagccgatgggcgcaaggcccagtgcctccgacaccatgcccatggtgttggccgtgaactggcccgcgcaggcgccggcagtgggcaggcaggcgcggctcatggcgtcgagttcgtcgtgcgtggcggtgccggccagcaccttgccgatggtctcgtaggtgtcgaccacgttgaggtcgcgcccgtcgggaccgggcatctgccccggcagcgccgagccgccatgcacgaacacgctcggcacgttgcagcgcaccatgcccatcatcaaacccggcaggttcttgtcgcaggcgccgatggcaaagatgccatcccattggtggccgcgcgtcgaggcctcgacgctgtcggcaatcagctcgcgcgagatcagcgagaagcgcatgcccgaatgcgccatggtgagcccgtcgctcaccgacaccacggggcattcgtgcggcgtgccgcctccggcatagatgccggtcttggcgtgctgcgcctgctcccgcaggttgaggttgcaggggctcatctcgccgccggtgtggaacacgccgatgtgcggccgagcgatgtcctcgtcgtcctggcccagcgcatgcagaaagctgcgcgtggtcgcgcggatcgtgccttcgcggatggtggcggagcggaagcgcttgctgttcggatcggtcggggaggtcatgacgcggtgcgaaaagaatttcagtagccgttgggcgtgacggtgcccgcggcgttcttgtatttcgccgccagctgcttcgccgccgccgtgagcaggatggtgtcgacgcccaccgccacgaactgcgcgcccgccgcgagccatttgcgcgcctgctcctcggtggtcgagagaatgcccggcgccttgccggccttgcggatgcgtgcgatggcgtcggcgatcacggcctgcacctcggggtggttcggttggccgacgaaacccatcgacgccgacaggtcggccggcccgatgaacacgccgtccacacccggcgtggccgcgatggcatcgaggttcttcattgcttcgacggtctcggcctgcaccagcaggcaggtctgcgcattggcttcgtgcaggtagccgggataggcctgccagcgcgaggcgcgcgcgagagcgctgcccatgccgcggatgccttcgggcggatagcgcatgccctgcaccattcgcgccgcctgttcggcggtgtcgaccatcggcaccaggatggtctgcgcaccgatgtccaggtattgcttgagcagcgtggtgtcgcccaccggaacccgcaccacggggtgtgagcgctcggcctcgggctgtgccgaccatgcgctggagatgccctgcagctgcgcgagcaccgagcgcacgtcgttgggcgcgtgctcgccgtcgatcagcagccagtcgtagccggtgccggcaagaatctcggccacgtagccgtcggccaggccgacccagaggccgatcttctgctcgccggcctgcatggcctgcttgaaggtgttgagcggtgtttgcatggaaggtctttcagacaaaacggaaggcaatgctgccgagcgggccgtagtcggcatggaaggtgtcgcccggcagtgcggtagtcgggcgggtgaacgagccgccgagcaccacctcgccggcttcgaggtgttcgtcccacggcgcgagcttgttcgcgagccaggccacgccggtggcggggtggttgagcacggccgcggccacgcccgactcctcgatcacgccgttcttgtagagcagcgcgctcacccagcgcaggtcgaccgcgtcgggcttcaccggccggccgcccatcacgatgccggcgttggccgcgttgtcggcgatggtgtcgaacaccttgcgcggcgccttggtgtggcggtcgaactgttcgatgcgcgcatcgatgatttcgatggcgggcaccacgtagtcggtggcggccagcacgtcgaagatcgtcacgttcgggccctgtagcttcttgccgaggatgaaggccagctccacctcgatgcgcggcgcgatgaaacgcttgaacggaatgtcgctgccctgctcgaagaacatgtcgtcgagcaaggtgccgtagtcgggctcggtgatctggctggacaactgcatggcgcgcgaggtgaggccgatcttgtggcctttcacggtgcggccctcggcgatcttggccttgacccattcgcgcgagatggcatagccgtcttccagcgtcatctcgggaaagcgcttggaaaagtgctcgacctgcacgcgcgatttttcgctttcgtgcagctcggccgcgagcctggcaatggtgtcggcggtgagcatggtttctttactactgcttgttgaagaggggatgcaggttgctgtgcttgccgtcgtacacctggcccggactttcgtcgatctgcagcgtgatgccgatatggcgtttgctgaagatgggctcgaaatgtgcgcgcacgtccgccagcagttcgtcgccggcatttttcttcacggcctcggagcgtccggccgccatgcggatgttgaggtacacgaaggcgtagtcggccttgccgtcggccaccgcatggtgcgcggccgggtaggccagcacgcgtgtgccgccgacgggaaacaccggctgcccggcttcgtcgcgctgcctcagcatggtgtcggccagcgtgcggcaaagcgccgtcatgtcggtttcggcttcgatgttgggcgtgtagaggatcacgaggtgcggcatgtgcgtgttccgttcattcgatcgacatcgtcgcggcggtgcatgtcaccgcgaagatcggtatggccttcatgtgcaggatctcgcccttgccgcgcgcggccgcggccacgctcaggaaggtgcggatctcgaagccgccctggccggcttcacggtaggtggcttcgtcgttgtagtcggcttgcgagagcagcgcctcgcggtcgttggcgcaccagcggcgcatgaactccgcgtcccactcggcgttgaccttgcccgaatcaggcgtggccggccagtgcgagatgccgcccgtgcccaccagcgcaatgcgttcgggcgccttgtcgcaggcgcggcgcaatgcctcgccaaaggcccaggcgcggtgcagcggcgtgagcggcgggccctggcagttgatgttcacggggatgaccgtggtgtcgaacttcggcgtcaagaagtggagcggcaccatgatgccgtggtcgaatttccattcttccgcgtaggccacgtccacggtctgcatcacctcgcggatgaggcgctgcgaaagcgccgcatcaccgggcaccttcgtcttctcaatgccgagccacttcgggtcctcgatcgggccttcgtagctgtcggccatgcccattgcatacgccggcatgttgttcatgaagaagttcgcgaagtgctcggccgcgaccacgatcactgcatcgggcttcgtggcgcgcattgcttcgccgaagcgatggaactgcgcgtggaactcgtccttcaccgccggatcggccaggtgggcgcggccggtgatgccgggggcgtggctgcaaacgcctgcgaatacgagactcatacgcctgccaccttttcgtctgtgcccgttgtcatggcataaattcctgcacgcaccggaccgtacttgcgcacgccttcgcgcatggcttcgaggtagtcggcccatgcgatgccgagcagtggtgcgaagtgcatcagcagttgtccgttgcagcccagtacgtacagcttgccgatgtcgcccttgtcgatggcttcgcgctcttcgtcgttgaggtcataggcagccagcaactcgacacgtgtttcaccgccttcggcgtagcggcgctgcgcgttggcatcgcggttgagggcgaacagaaatttctgcatggcgtagaggctcattgcagtgaccttgtatctttgttcagggcgcgtgcaaaggccaccgggtactcccctccgcgaatgtcccccggcctgcggcctcctcctttatttcgctgcggggagcacccggcgccctgtgcccaccgggcgctgtcgttgtgctggctgatcaacgaccgctctgcccaacgatcccgtcgatggggtgccttgcgcagcgaaataaaggaggaggccgcaggccgggggacattcgcggagcaaggtaccccgtcggcgggagcgccccacgaacaaagcaccgaatccacagcgcgttgaacagaaaaccggggactcatctcacaccccccaatgcggaatgtgatgcgaacccatcgaaaccgcaacgtttttcggctcgcaaaacacttcgtagctccaagtgccgccttcgcgacctgtgcccgaggctttggtgccgccgaagggctgacgcaggtcccgcacgttctggctgttgacaaagcacatgccagcttccaccgcggccgccacgcggtgcgcgcggccgatgttctcggtccacacgtaactcgagaggccgtactcgatgtcgttcgcaaggcggatcgcatcggcctcgtccttgaacggaatcaggcaggccaccggaccgaagatttcctcttgtgcaatccgcatgcggttgtcgacatcggcgaacaccgtcggcatcacgtagttgccgcgccgaacgcgctcgggcaggttgcccggaacctcgagtccgccgcacagcagcgtggcgccttccttcgggcccagctcgatgtagctgcgcaccttggccaggtgcgcctgcgaaatcatcggcccgacgatggtcttctcgtcgagcggatcgcccaccgtgatgcgcttggcgcgctcggcgaacttcgctgcaaagtccgcgtagatcgactgctgcaccaggatgcgcgagccggcggtgcagcgctcgccgttgttgctgaagatcatgaacaccgccgcgtcgagcgcacggtccaggtcggcgtcgtcgaagatcacgaacggactcttgccgcccagttccatgctgaacttcttcaggcccgcgctcttcacgatgcggttgcccgtggcggtggagccggtgaacgagatcgcgcgcacgtcggggtgcgcaaccagcggctcgccggcctccttgccgtagccgtgcaccaggttcagcacgcccggcggaatgcccgcttcgagcgcgagctcgcccaggcgcgcggccgtgagcggcgagagctcgctcatcttcagcaccgcggtattgccgaaggcgaggcagggcgcgaccttccaggtggcagtcatgaagggcacgttccacgggctgatcagcgcgcacacgcccaccggatggaacagcgtgtagttcaggtgcgtgggcgtggggtaggtgtggccgtcgacgcgcgtgcacatctcggcgaagtaatagaagttgtcggctgcgcgcggaatcagctgcttgccggtctgcgcgatcacctggccgcagtcgtcggtctcggtccgcgcgatctcgggcaagtgcttcgcgatcagctcgccgagcttgcggaccagcttggcgcgttcggtcgcgggcatgccggcccacttgggaaaggcctccttggcggcggccacggccgcgttcacttcggcttcgccgccggaggccacctcggccagcacctcttgcgtggcggggttgacggtctcgaagtagtcggtaccggcgacgctcttgccgccgatgaggtgatgaatctgttgcatggggtcccctgagggtcagtcgagtttgatgtcgcgggccttgatcaaggcatgccacttcttgcgctccgcatcgacgaagcgcgtcatctccgcgccgtcggcggggcgtgcctcccagcccgcgtcgtagagcttctggcgcacgccggcatcggccatggtcttctgcaggtcggcgccgagccgggcctgcacctccttcggcgtggcagccggcaccacgagcccttgccaggtgtaggcctcgacgcccgcgtagcccagctccttcgcggtcggcacgttgggcagctgcgggatgcgttcggcgcccatggtcatgagcggcaccaccttgccggccttgaccgcgctcacgccgctgggcaggtcgagcatcatcagcggcacctgcccgcccatcaggtcttgcagcgcgggcgcgccacccttgtagggcacgtgcagcatcgagacgccggcttcgcgctggaacaattcgagcgccaggtgatgcgggctgccggtgcccggcgtggcgatgctgtacttgcccggcgatgccttcagggcggcgatcagtgccttggcgtcggccaggccggcgttgggtgcggccgtgatgacgagtgtcgagcggcccatcatgcccacggtcgcgaagtctttctccgcgtcgtagggcagcttcttgtagagcgcggggttgtacaccagcacgccgttgtcggccgagaacacggtgtagccgtcgccgggcgagcgcgccacgttctccgacgcgatgatggcgcccgcgccggggcggttgtccaccagcaccggctggcccagctgctgcgaaagctgcgcgccggcggtgcgcgcgagaaagtcggtgccgccgcccgcgggataaccgaccacccagcgcacgggcttggcggggaaggcctgggcctgtgcgtggggtgcgaaggtggcggtggcgaaagccaccagggccgccgcgagcgctagcttgttcctggtcgtcatggggtttgtctcttctgtcgttggtatggaaaagcagtgcggcgctaggtgccctcgatggtgttgaccagcgcgccgatgcgctcgatctcggtcaccaccacgtcgccgggccggcaatcgaccacgccatcgggggtgcccgtcaggatcaggtcgccgggcgacagcgtcatgaagcggctgaaatactcgatgagaaagggcgcgtcgaagatcatgtcgcgcgtgttgccctgctgcgtgacagtgccgttcaccgtggtcttgagcgcgagcgccatcgggtcgggcacatcggccgcgtcgacgaaccagggtccgagcggcgtgcaggtgtcgcggttcttcacgcgcaggttggggcggtaccagttctccaggtagtcgcgaatggcgtagtcgttggccacggtgtagccgccgatgaagtcgtaggcgtcatcgcgcttcacgcggcgcgccgtcttgccgacgacgatggcgagctcgcattcgtagtgcatgaactgcacgccggccgggcggtgcgtgcgctggcggtggccggtcagcgtgctctggcccttgacgaacgcgagcggttcctcgggcgccttgaactccagttccttggcgtggtcggcgtagttgaggccgagcgcgaggatggtgcgcggacgcacggtcggcgcgagcggcggcagccatgtgagctgctcctgcggcacgatgcggccgtcttccaggcgcacggcggcatcttgttcgccattgaattcgtgcgcgatgccggtgtgttcgcggccttcgtaaatgacacgtgcgtgcttcatgcggccacctcctgcaccagcgtgttggccagggtctcgaaccccggcgcggagatctcgatgcggtcgcccgcgcgggccagcggccggccggcgtcgcagcccagcatcagcacgtcgccgtgcgcgagcgtcatgaagtcgccgacgtcggccagcagctgctgcgccggacgcacgagctgcgaaaaatcgatcgactgcttcagcgtaccgttgatgcgcacctcgacgcgaaagcccgcggggtcggccacctcctgcgcgtcgcgcagcaccggaccgatgccgaggaacccgtccacgcacttgaacttcacgggagggcggaagaagctcgcatgcggaatcgagagatcgttcatcagcacgaagccttccacgtcgccctcggcgccgatcaccatgccgatgctggcgccgatctccacttcgggtacggacgaaggcacagcgatggcgctgccgtgcgggctccaggtgttggcggtcttcacgtagagcaccggcgctttcggcggcgccttgtagggcggctctgccatctgcggcgcgagcgcgtcgaactcggcgcgaaagttcagcagcgtgccgtacacggtgcctgtcggaaggtaatgcggggcgccgctgctcatgagggctgctccagtgcaatgagttcgtcgagcagcccgtagagctgcgtgagcttggccttgccgagcgacttttccatccagttgtagtgcgcctcgatgctggtcgacaggcgcttcaccagcttcatgccatgcgccgtggcttcgaccacggtgcggcgctggtcctcggggtcgcggctgcgcgtgatgagcttgtcgcgctccatgcgtgcgagcacgccggtgaggctggggccgaggatgaaggcctcgcgcgccacgtggccggtttcgaccgcgccgtgctcgccgagcacgcgcagcacgcgccattgctggtcggacagcgcgtgctcgcgcaggctgggccgcgtgtgggccatcacggcttcgcgggcctgcagcagcaggcgcggcagattgcggtgagtgaaggtggtgctcaaaagctgtgtctcgctgaattagttaacatgttaaatgatttggaatttctttcctagccgttttccatcagggtttgtgcggacacctaaactccccgcatggccaaggaaaaaacactatttgtctgcagcgaatgcggcggcaccagccccaagtggctcggcaaatgcccgagctgcggcgcttggaacacactcatcgagcaggtcgcgggcagcagcagcggcccggccaacaaccgcttcggcacgcaatacacctcgctcgcgggcgcgtccgaactcgccacgctgtcggaaatagaagcaaccgacatcgagcgcacgcccaccggcctggaagaactcgaccgcgtgctgggcggcggcatcgtgtcgggcggcgtcacgctcatcggcggcgatccgggcatcggcaagtcgaccttgctgctgcaggcggtcgatgcgctgcagcgcgcggggcagaacgcgctctacgtcaccggcgaggaaagcggcgcgcaggtggcgctgcgctcgcggcggctcggcctcgaccattcgcaggtgcaggtgctggccgagatccagctcgagaagatcatcgccacgctcgacgccacgcgaccggccatcgcggtgatcgattcgatccagacggtgtactccgaccagctcacctccgcaccgggctcggtggcgcaggtgcgcgaatgcgcggcccacctcacgcgctttgccaagaccagcggcacggccgtggtgctggtgggccacgtcacgaaagagggcgcgctcgccggcccgcgcgtgctcgagcacatggtcgacacggtgctgtacttcgagggcgacacgcattcgagcttccgcctcgtgcgcgccatcaagaatcgctttggcgccgtgaacgagatcggcgtgttcgccatgaccgagcgcggcctgaagggcgtggccaatccgagcgcgatcttcctgagccagcatgccgagccggtgcccggcagcgtggtgctggtgacgctcgaaggcacgcggccgatgctggtggaaatccaggcgctggtcgacaacggcggaccgagcccgcgccgcctctcggtggggctggaccgcgaccgccttgccatgctgctggccgtgctgcaccgccacgcgggcgtggcctgcatggaccaggacgtgttcgtcaacgccgtgggcggtgtgcgcatcagcgaaccggcggccgacctggccgtgatgctggccatcacctcgagcctgcgcggcaagccgctgcccaagggcttcatcgcattcggcgaagtgggcctggcgggcgaggtgcgccccgcgccgcgcgggcaggagcgcctgcgcgaagccgccaagctcggcttcagcgtggccgtggtgcccaaggccaatgcgccgcgcaagggatcgaaagagatcgagggcctgaccatccacgccgtcgaccgcatcgaagaggcgatggacgtggtccgccgcctcgattgaattcactgcgggaaaaaatgcccggcgcaccactggcgcgccgggccaccctccctaccccccgatgtgcatcgtgaacgccggtccgccgttgagcacgcattggccgctgcccaacgtggccgagttcatcgtgtactggcaactcaggttgccgccgcgattgccgctggcgttcgccaggccggcacctcgcgagcccgcaacccgggtcgcctctccctgatacagctccccaccgatctgcgcattgaaatggccgcggccgttcatgtcgttggtcaccgtgcccgagacggttccgtagcgcgccgcttcggcgttcgacggatacagccgcgcactgaagctctgcgccaccggacccggtgcaacggcgtaagcctgcgaggccggcgccgcgggtgcgggttgtccgagtggcaccacgtagcaaccgctgaggacggtggccgtgagcgtggcggcgagggtgagacgaatgaagctggcaggacgcggactattcatacgcttttcagtggcccgggcaaatgcccgtgcggtgaaatgtgccggctggcgtcaccgggccgcgtgcttttcgcaatgagtaccgcgccgcgcgcccggcggtagccacggccgctactgccgcctgccttgccggtgcggcaagaaaagcgccctcgatccggatgcgaactttcgaatgacgccggcgaggcgaggatcgccgggcggcgacaatgcgccccatgaattttcagaaactgctggtgcccgtgggcggcatcgttcttctcgggctcgcgtggcgtagctacggctgggccggcgtggcgctgactggcggcgcgatcgtgatgtttttgctgctgcacttcaaccgcgcgatgcaggtgctcaagcgggcggccgaccggcccgtgggttatgtcgccagcgcggtgatgctgaacgccaggctcaagaagggcgccaccttgatgcacgtcattgcgatgacgcgcgcgctcggcgagctgcgttcgcccaaggacgaacagcccgagctctaccgctggaccgatacgggcggctcgtatgtcgacgccgtgttcaacggcggcaagctgcagagctggacgctgacgcggcccgaggcggcgcccgaagaagaaacagaaacgccggcgagctgatcaggcaagccgggcggggcgccttccttcagaacggcgcgtcttcttcttcctcgacggcgtcggccggcgtcgaggtggtgggtgcggcggcggcaggtgctgccgccggcttcgcggtttcgtccgtcggagcgcccgagaatgccgcttcgccgcccagcgcgtcgagcagcgccggcaccagctggccgagttcgccggtggcaatggccacgtcggcgtcgaagttgtcttccttcttgccacccgaggcaccatcgcccgtgccttcgaggaacacgatcttgcggatcagcatgccgtgcgtcagctcgaaggacacgcggtcgtcccacgtgagcgccaggcgcgtggggcgcttgccgtcggtgatgtgcttttgcacttcctcgatgtcgagcgggtgcttggcgtagcgcaccacggccttggaatcgtccgaggccttgagctcgcactcgcggtcgatggtgaagccggccggtggctcctgcgtgagcagccagttggccatggccgcggccggttcgatctgcgtgttgatgagggccaccgcaaagccgtcgagcgacttcacgaggctggtgaccacttcgtcggcgcgggcggcattggcgctgttgatcacgaggcggcgctcggcctggtcgatccacacggccacgcgggcgctgcgcgtgaaggccattggcagcagctcgagggtgatgtcttccttgagctccttcttttccttcttgccgggcttgcggccggtggtggcctcgatttgcgcgcagcgctcgtcgagcttgcgacgcaccacggagccggggacggccttgctctcgatcatgtattcgaccagccactggccgccgatggattcggccagggggccgttggcctcgccgcggggctcgacccagccggcggacttttcctgcgaggggccgcagggctcgaagcgctgcttgccgagaccttcttccacctcggtcaatgtttgggaccaggcaggttcgatgcgatagacgatgacgttcttgaatacggacacggaaaccctttttccactggtttggacaaccggccattgtcgggcaccccgttccggggtcggccgtaaaatcgcaagcttttgcgacttcctctccgtcgcacccccacaccgcttcccaaacaaaggaatcaggaaatgagctcgatccccccctcgctggacgaccgtgacggcaagatctggatggacggcgaactcgtggactggcgcgacgccaagatccacgtgctgagccacacgctgcactacggctgcggcgccttcgagggcgtgcgcgcctacaagacggcagatggcggcacgtccatctttcgcctggccgagcacaccgagcgcctgttcaacagcgccaagatcctgcgcatgaagattcccttcacgccagaacagctgaatgaagcccagaagcaggtcgtgcgcgagaacaagctcgaaagctgctacctgcgcccgctgatctggatcggctccgaaaagctgggcgtgagccccaagggcaaccgggtccacgccatggtcgcggcctggtcctggggtgcctacctgggcgaagagggcatgcggcgcggcatccgcgtgaagacctccagctacacccgccaccacgtcaacatcaccatgacgcaggccaagtcggtgagcaactacaccaactccatcctcgccaacatggaagcgctggacgacggctacgacgaagcgctgctgctcgacgcgagcggcttcgtctccgaaggcgcgggcgagaacatcttcgtgatcaagggcggcgtggtctacacgcccgacctgtcggccggcgcgctcaacggcatcacgcgcaacaccatcctgcacgtgtgcaaggatctgggcatcgaactcgtgcaaaagcgcatcacgcgcgacgaggtctacatttccgacgaagccttcttcaccggcaccgccgccgaagtgacacccattcgcgaactcgaccgcgtcgagatcggcaaccgcggcgacggcggctcgcgcggcccgatcaccgagaagatccaggcggccttcttcgacatcgtgaacggcaagaatcccaagtacgcccactggctcacgaaagtctgagaaaacccatgcctaccaacgcagtcgtcgaactcctggccagggagctcaaccatcagggcggcgtgttctgccctagccccaaggcggacatgaagctctgggacacccaccccaaggtctacctggacgtggcacgcaccggtgaagccaagtgcccgtactgcggcaccgtctatcgcctgaaggcgggcgagacggtctcgtcccggcattgaccgttcgcggcctgctgggccgtttcggcgccggctaccggctgttgcgggtcgtccggcaattcgcggcggccgaagccaggcacagcagccgtcgttagctagctggcttgcggcggggcctcatcgagcgccgctgcgatgtggcggctcggccacaggtcgcgccagggctgggcatcccgcggttcctgcgcgagccgcaggtagaccatcgcgatccacagcagcgccaggccgatctgcgcgtcgcgcatcgccgagttcacgctcgacgcgatcagcgcgatcaacgtggcggcgagcgcgtagcggcccgcgatgtcgggccttttccatgcctgccagacggcgccgaccatgatgaccaacaggcttagcaaggccggcagccccccctgcgcgccgacccacaggaagtcgttgtgcggcatgttcgaatcggcgaagagcaccgggccgcgcttgtgccactggtcggtccagccgccgatgccccagccggtgagcggccggtcggcgatcatgaggccggtgtcgcggtacatgtagtagcggatgacccagctgcccttgaagatctcgccggcctgcgccttctcgatttcctcgacgccggtctcgaccttgtgctggagctgcggcaactgatagagcccggccgccagcaccacggcacccagcaacagcgcgctcaccagcatcttgaggtggctgcgccattggtggatgcacaccaccggaatcaccagcatcagggcgagcaccgaggtgcgcgaggtcagcggcagcgccaccaccaggcccagcccgagcaccagcatgaaggcggggacggcacgcagcggcctgtgcgcggcgatctgcgcaatgccccacacggcggccgtggacgccaccacgctgaaaagcagcgcgttgctgatcgacttgttgcccacttccatgaccaccgcgcgcagcggcgaccagatcggaaagccgaaggcgtagtgggccacgatcagcagcacgttcagcgctgcgatcagcaggaagccgcgcagcgcccagatcgcttcctcgcgggtgagcgccatggccatcaagatggtgaggccgatgcgcagcccgtggaacaggttcgagcccgtctcggggtagtgcgggccaatggccagcacgatgaaggtccaggccaggtacgccaccatcggccaccacagcgggttggcacgaagccgcgcatagcgttcacggtagccgccggccagccccatggtggcgagcagcagcagggccgcaaggtaggtgacgccgacgggcatgaacaccaccagcccccagaacatggccgcgggcctgacgatgtgcgatctctgcataggggcgggattttaggtgggccccgctggcccaacctgactgggcgcccgtcgcccggtcagctgccgctggccaccggcagccggatgacgaagctggcgccgccgcccggccgctcttcgcagcgcacgctgccgccgtggcgctcggcaatcgacttcaccagcgccagcccgaggccgacgccgccgttgcgctcgctggcgccgggcagccggtagaagggctcgaagatgcgttcgcgcaaggccgccggcacgccggggcctcggtcgttcacgcgcacggtggcaaagccgttggcgctgccgagctcgaccgagatttcgccggcgccatagcggcgtgcgttctcgagcaggttgcggatcgcgcggcgcagcaggcgcgagacgccgggcacggtgagcttggcgttgtcggtgccttccaccaggtcgagctcggcatccacctgcgagcactcctcggccgcgagcccggtgaggtcgaccgcctcgatggtgcccatgtcggcctcgctggcgtcgagccggctggccagcaggatctcgtcgatgagctggtccagctcgccgatgttgcgagagatctcgtcgcgcgctgcggggctcgggcgctcgcccatcagctccaggcccatgcggatgcgggtgagtggcgagcgcagctcgtgcgatgcgttggccagcaacgatttgtgcgagcgcaccagtttttcgatgcgttcggccgatgcgttgaaacgtttggagagatcagccacttcgtcctgcccttcttcggtcacgcgcaccgagagatcgccttccccccagcgttgcacgccgcgctgcaatgtttccagccgctgggtaagccgccgcacgatggggtacacgcccagggccacggcaatgcccacgagcgcgatcatccagcccagcccgaaaggcgtgcgccagggcgcgaacccgccggtgcccgaggggcggtcgcgcggcgccacgcgcagcgtgatggccttgccgtcggcgagcgtcacgtcgaactccaggccctggcccggcacccgcagggccttgccgctgccgatgggtcggtcctgcgcgtcgagcaccaccacgttgcgcggcaccggtgccaggcgctcgcgctcggcctccgccgcctcgcgcacgatccagttggccatcagcgtgaggatgacgacgccgcccaccaccgcgagccagatgcgcacgtagaggtggcgcgaatacaaattgcgaagcatcaaatcaatcttgctgcttggcgaagacgtagcccacgccgcgcacggtgaggatgcgcttcgggttcttggcgtcgacttcgatcgcggcgcggatgcggcccatgtgcacgtcgatcgagcggtcgaaggcttcgagctcgcggccgcgcaccgcttccatgatctggtcgcgcgtgagcacgcggcccgcgcgctcggccatggccaccagcaggtcgaactggtaggaggtgaggtcggccagcgcgccgcccaccgccacggtgcgtgcgttgcggtcgatctcgagcgtgccgaagcgcatcaccgtgctggcttcggtgtcggcgttgttctcgctgcgccggcgcagcaccgcgcggatgcgggccagcagctcacgcggctcgaagggcttgggcaggtagtcgtcggcgccgatttccaggccgatgatgcggtccatcgggtcgcccttggcggtgagcatcagcaccgacaccttcgaggcgggcgcgggcaacgaacggatgcggcggcagatctcgaggccgtcggtgtcgggcagcatcaggtcgaggatcaccaggtcgggcgcgtgctgctgcagctgctcgaggccgctggcgccgtcgccggcatgcgagaagaggaatcccgactgcgtcaggtattcgcccaccatgtgtgccaggcgggcgtcgtcttcgatcatcaggagttggggggtgctcatgcgcttcatggtcgtccacggggggcaacggggcttgaacgctccgtaaagttgggtaaaccaggcgtccggatgtcaacccggggtgccgcgaaaagcatggcgccgaccggtgcgtcggccggcggcgtggtcatgctttcttcgaggatggcgggaaggttgcagccggccagttccgcattgtccgcgcgcgcccgcgccaggatttcgccggccagctggtgcagctgaaaggtcgaagcccggatgcgcgccttgaaggcggcgtcatccaggcgctggtccttgaggctgcggttgagttcggcgaaccacggcatggcggcctgatcgagcatgaccggggcgttgcgccgggggctggcggcggaccatgcgcgcagcagttgctgcaccgccaggttcaggcgctggcagtgctgcaactcttccttcaggctgcccagcagcatcaggtcggtgagccgctgctgaaagaagatctgcgagagcacgccccagtagtaggcgtagtcccagatcactttcaccggcagcacctcggggtcgccgaacagcgggtactggtcctggtagagcgccagcgtgctttcgtagaaggagtggtagatctggtcgtagagctgcgcgcgcgcttcgagcgagcggcccgcgcggtcgtgcgccaccaggtcggtgatgtaggtgttgctgatcgcgatgaagtcgctgccgggcgaatagaaggggtcgagaaacagccccgcctcgcccgtcaacgcccaccgctggcccgagaacacctgcttgcagccgtgcgaaaagtgcttgaggaaggcaaagtcctgcaagaggtgccgcttgccgtcgagcgcgtcgtacagcctcggctggtaggtggcaaaccactgcatggctttttcgaaggtgtcgatggtgtcgagcggatgcagcttcgggtcggccacgatgcccaccgagtgcgagcccgaagccagcggaatcagccaggcccagtagccggcacccaccaggtggttggtcgaaagccagcgcgcctgagggtcgcagcgcccgcgccaggccgtgtcgtcgctccattcgtcgatggaaatgcgctcgccgatgcgaaaccacacggcgttcacctcgtgcgcgttggcctcggcgagcccgagcttgcgcttgagcaggccggcgcgcccgcaggcatcgatcagccagcgcgcctcggcgctgtgggtttcgttgccgcgcgaccactccaggcggtgcggcgcatcggcgccctgggccagatcgacgcggcgcaccagcgcggcatcgtcgaagcgcacgccgcgccgcacggcctcctgggcaaggtagttctcgaagatgccgcggtcgatctggtagctgggaacggccaggtagcggctggcgccgatctcggtcacctggtcgatgtcgcgccggccttcgctgaagaagaagcggaagccgaacttgcgcagctgcgcgctgtccatgtggggcttgaggcccagcaccgtgtcgaagtagtgcgcgccgatctccaccgacgattcgcccaccttgtgggccgcgtgcggcaccggatggctgcgccgttccagcaccagcacgtcgatgtcatcgaagcgctgcttcaactgcagggccagggtcagccccgcgagcccgccgcccatgatcactgcgtcatatcgttgcgcagtgccggtcatggagcttcagtcccggatcggccgcagttgcagccgcagtgaaagggtggaagaagacagcggcagttcgagcgccggcgggtcggcctccacgcgcgccagcgattcgaacaggccgagcgcatgggccatcggattgatgtgcaccagcgttttcgcggcatcggaagaaaggggcgccggcacagcggcgccgccgctttcctgcagcgaccaatcgagagccgccacggtgcgcgccgtgcgctcgggcgcgatcaccagcgccacggccaggaggccctggctgtcggtcaccgaggtcagcgcgcccacggtgggcgtgtcgtagcccaccagcagcaccggcgactggtcggccgcgcattgcaccgccgcttcgagcaggccggcggcaaagctgttttcgtaggccgagatggagttgctggccgccatgcagccggtgccgatggtccagtagcccacggccgcgttgtgcaccgagttgtgaaagcgcgtcggcgacagcaccgtggggtcggtggccagcgtgctgcacatgtagtcgttgatcgagagatccccatgcgccgacacgaacacgcagggcacgtcggcggcgttgcggcccgagccggccatcgatgcggcggccacctcgagcgcgagggccacggtgtcgggcgcgcggcggcgctcggccggcgccagcacctgcggcgacgggcgcttggcgggcgggtcggccagcgcgccttcgccacggaaggcggcgcgggcggcgtcccagcccggcagggtgggcgtccagaaggccgggccttcgatgtagagagtgggcggcttcggggcctggcgggtggcggtcatggggcggccttgccgaacaccagcgagcagttgttgccgccgaaaccgaaggaattggtcagcgcgtagcgcacctcgccatgcgcaggctgcagcctgatctgcggcccgaagcccgcgtcgagctggttggtgttcacggtgcccggcatcaggccgcgctcgatcgccagcaggctgatcaccgattcgacgatgcccgccgcgcccagcgtgtggcccatgaagcccttggtcgagctggcatgggtgcgcgccggaaagcgccgcgccaccagtgcgccttcgacctcgtcgttcttctggctcgccgtgccgtgcatgttgatgtagtcgatggcgtcgggcgccagtcccgcgcgcgccagcgcctcgtcgagcgcgcgttcggcgcccaggccttcgggatgcggcgtcgacatgtggtgcgcatcgctggcttcgccgtagccgagcagccgcaacggcgcgccggcctcgtcctgcacgcgctccaccagcgcaaagccggccgcctcgccgaggctgatgcccttgcggccggcgtcgaagggccggcacggttcgttcgagaccagctcgagcgagttgaagccgaacagcacgctgccgcacagcgtgtcgaccccgcccaccaccgcggcgtcggccagcccgaggcggatcagccgctcggccgaggcaaacaccttggcgctcgacgagcaggcggtggaaatcgtctcgctgggcccggtgagcccgagcacttgctgcacgaacatggccagcgaatgcggcgtatgcaccgccgcccggcgctggttctggggaaagaggccatcggcatcgagctgcgtataggccagctccgtttcgccgatgctggacgtcgaggtgcccaggatcagcgcgatgcgcgaggcgccgtacctggcccgcgcggcggccacggcttcgaggaacccgtccgcatgcaggcccagccaggcgagccggttgttgcggcagtcccaggaagccagcgcttccggcaggcggatgtcttcgagcccgtcgacgcggccgatccacgtgggcagcggcgcatcgccgaaatcgttggcgcgcaggccgctgcgcgagtgagcgagtgcctcggcgagcggctccttgccgacgccgacggccgaagtggccgtgaaggcgctgatctgaagaggagaaatgcggggcggcacgttgcttgtgggttggcaggcagaaggtgaaaacgcttttgtatcagcgaggcgaaaggtaaccggaaaggtaaacgaattgtgaaagcctaccagttgagcgggccgggccgcgtcagctcttttcctataaggcccgtgctctattgacgctcggcggggcctgtggtcgtggtgatgcgggcggccagcgccaccagcagcagcaccggcacgcccaggagggcggtggcggtgaagaactgggcgtagccgtaggcgtcgacaaacacgcccgagtagccggcaatgaacttcggcagcagcagcatcagcgagctgaacagggcgtactgcgtggccgagtagctgatgttcgtgaggctcgacaggtaggcgatgaacgctgccgaggcgatgccgcccgccaggttgtcggccgacaccaccgcgatcagcgccgtcaggtcatgcccgcgcgaggccagccaggcaaagagcaggttgctcgcggcgctgagcaccgcgcccagcatcagcacccgcatcacgcccaggcgcatcgacagcacgccgcccacgaaggcgcctgccagcgtcatgaccacgccgtagatcttgctgaccgtggccacttcgtccttggtgaagcccatgtccacgtagaacgggttggccatgatgcccatcaccacgtcgctgatgcggtagatcgcaatcagcgagaggatcagcgcggcctgccacttgtagcggcgaatgaaatcggcaaagggctctatcagcacgctttgcagccattcggtggcgttcttcgccttgggcagcacgcgccgcacgggctcgggcgacagcagcaccgtgagcacgccgaccgccatcgaggccgccatcaccaagtaggccgttttccaggcgccgttctggtaggccgccgcgccggtgacggccgcggccggagccacctcggcccaggccgcgacccacagcacgccggcgccggcccagatcatcgcgagccggtagccggtttgataggcagccgcgagcgcggcctgcttgcgggtttcggccgattcgatgcggaaagcgtcgagcgcgatgtcctgcgtggccgagccgaaggccaccagcagcgcgcaccagatcagcggcacgagaccctggcgcggatcgttcagcgccatgccgatcagccccgcgatcaccaccccctgcgccagcagcagccagccgcgccggcgcccgagcagcgtggtcagcggcggcagcggcagccggtcgaccagcggcgcccagacccacttgaagccgtaggccaggccgacccagctcaggtagccgatggtggtgcggtcgatacccgcctcgcgcaggcgaaaactcagcgtgcccagcaccagcagcagcggcagcccggcggaaaagccgagcgccagcatgcgcagcgtggcgggctcgaggtagaccttcagcgcgtcgcgccagggcagggagggggcggtggaagtttcggcgggctgggcagacatgagccccggattgtccatgagggtgcgcttggcgccgagcggtctttttgccgcgtttgttcctatgatccgcgcatgtgcacacgatgcgagtccttcgtttcttccgcggctttggcctcccgctcctcggcctggcagccgcggcgggcttttctgcttgcggcggccggcgcggtgctgaccggcccggcgctggcgcaggtgaacgtgggcaatgcgtcgatggcgcgcaacctggtgccggccgaccgcatcgaggccgccggcgtgcagcagtacggccagttgctcgaaaaggcgcgcgccaagggggcgctcgccggcgacggcaacgcgcagctgcagcggctgcgcaccatcgcgaaccgcctgattcccttcgccacgccgtggaacacgcgggcgcgccagtggaaatgggaggtcaacctcatcggcagcaagcagatcaacgccttctgcatgcccggcggcaagatcgctttcttcaccggcattctggagcagctcaagctcagcgaagacgaggttgcgatggtgatggggcatgaaatggcccatgcgctgcgcgagcatgcgcgtgcccgcctggccaagagcgccggcaccggcgccgcgctctccatcggtgcgcagctgctgggcctcggccagatgggcgatctggcggcccgtgccggcacgcagctgctcacgctgaagttcagccgcagcgacgagaccgaggccgatctcgtcggcctggagctcgcggcccgcgcgggctacgacccccagtcctcggtgtcgctctggaagaagatggccgcggcctccaagaaccagggcgggctgagtttcctgtccacccacccgagcggaccggaccgcatccagcagctcgaagccaatctgccgaaggtggaaaagctctaccgcgaagccaagcgaggctgaggtgtgagccccacctcttctggaagagggcgcggctgattgtctgactccctctccctctgggagagggctggggtgagggcggcggccgtcacatctgagccgcgcttcgtcggggcacggagccacggagccctcaccccaaccctctcccggagggagagggggcaaaaccccaaccacgacttgtgaaggacgatcccgatcctcctggcacattgcttgcatctcgacttgtacacaagtttggatgccttatgatggtgcatgaaaaaaacggatcggctgctgcggcgtggatcgcacgcttcgcgcaacccgtgcccggtgcggacaccggcagcggcccgctcgccggcctgcgctttgccgtcaaggacaacatcgacgtggccggcgtgcccaccacggcggcctgtccggccttcgaccgcaggccctcggcacacgcggcggcggtgcagaaactgctcgatgccggtgcatcgctgcttggcaagaccaacctcgaccagttcgcctgcggcctgaacggcacccgctctccctatggcgaagtgcccaatgccttcgatccgcgttatgtctcgggcggctccagctcgggttcggcctatgtggtggccgccggcgaggtcgatttcgcgctcggcaccgacaccgcaggctcgggccgggtgcccgccgggctcaacaacatcgtcggcatcaagccctcgcgcggcttgctgagcgcctttggcgtggtgcctgccgcccagagtgcggactgcgtgtcgatcttcgcgcgcaccgtggccctggccgtcgacgtgctcctggcggccgccgggcccgacgcgcgcgacccctattcgagggggcttgcgctgcgcagcgatccgttcccctcggccttccggttcggcgtgcccgacaccctgagcttcttcggcgacggcgtggccgaagaggcctttcgcgatgcacaggcccggctcgttgccctcggcggcacggccgtgacgatcccatatgcaccgctggccgaggccgccgcgctgctctacgaaagcgcgctggtggccgagcgctatgccgcggtgcgcgagttcttcgatgcgcacggctcccaggtgatcgaaccggtgcgcggcattctcgagagcggccgcggctacgacgccgccgacgtgttcgaggcgcaaacccggctgcgcgcgctcgcgcggcaggccgaaccgatgtggcgcggcatcgacgtgctgctggtgccgaccgcgcccacgcactacacgcgcgaacagatgcgcgccgacccggtcgtgctcaatcgcaacctgggcgcgtacaccaacttcgtcaatctgctcgactatgccgcgatctcggtgcccagcgccattcgcgccgacggcctgcccttcggcatcacgctgatcggcccttgcggcagcgatctcgcgctggccgatctgggccagcgctatcaccacgccaccggcctttcgcagggcgccacggggttgccgctgcctgagcccaagcccgtgcctggcctgggtgctccggcggcgcagaccatgccgatcgccgtcgtcggcgcgcatctttcgggcatgccgctcaacgcgcagctcaccgaacgcggcgccacgctgctgcgcgccaccaccacctcgccgcgctaccgcctgcatgccttgccgggcaccgtgccgcccaagccggggctgcaacgcagcgccggcggcggaacggccattgcgctcgaagtgtggtgcgttccgctcgcgcaggtcggcagcttcctggcgctgattccgccgccgctgggcctgggcagcgtcgagcttgccgacggcaactgggtgcacggcttcatctgcgaaggccacgcactggccgatgcggaagacgtgagccaccacggcggctggcgcgcctacatcgcgagccgcaccgcttcttcccaagccattccaacctgaccgatcgaggagtcttcatgagcacccctgagaaatcacccgccgccgcctcgcgccgccagttgttgcaggccggtgccgcggggctggccgtgctggccgcgcccgccatcgtgcgcgcgcaagccgcaccgaagatccgcatcggcttctggcccgtggccgccggcctgcccttctttgccgcgatcgaccgcggctacttcaaggaagcggggctcgacgtggagccgctcaaattcgcgggtgcgcagcaggtcatggaaggcatgctggcgggccgctgcgacggcagctccaacggcaccggctcggccaacctcgccatcggcgagatcgcgcagccggggctcttcaagatcttctgcaccaacccgagcaacgccaagttcgtgctcgacgaattcatcgtcgccaaggacagtccgatcaagaccatggccgagctggccggcaagaagatcgcgtccggccccggcatccagaacgtgactctctgcaagaccatgctcgaacgcgcgggcgccaagggcgcggtcgtgagcgaacttcccatcggccagcacgtggccgcgctggttgcgggccaggtcgatgcctgctacacgctggagccgaccggcaccgtcggccgcatgaacggcaccacgcgcgtcatcgaggccggcgtggtggccaagtacatcctcggcgacccgatggcgccgtggcacggcggtgcggccagcctcacgagcgagttcatcaagaagaaccccgaagtgacaaagaaatacatcgccgcctatgcacgcggcgtggagctggtgcgcaccaagccggacgatgcgcgccagcacatgaagggctacaccgccatcgaaggcagcctcacggccgaagtgccactcgcctcgtacatgctctacaacgagttcaagccgagcgacgtggcgtacttccagaagttctacgacctgttcaccgaaaaaggcatcttcgagaaaaaggtgctggtggacggcctgctctacaaggcttgatcatggccgacgcaagcacgaccacggccgcgccgtggacaccgccggccgccggcgccaatgcggcggcgcccaagccgccgctgcgcgaccggctgctgcccttcatcggacccgtggtgctgttcatcgtgtgggacgtggcggtgcggctcggcttcatcaagccgatcctgctgcccacccccgccgacaccgttgcggcgctcatcacggggctcgcgggcgggccgctgctcaccgacttcgcaatgaccgtgtggcgcacgctgcaggcctttgccattgcagcggtggtcggcgtgccgctgggcgtgctgctcggcagcaacgagaaagcctaccgcagcgtcgaattcctgatcgacttcttccgctccacgccatcgtccgcgctgattccgctgttcctcctgatcttcggcgtgtcggacgtcaacaaggtggccatcgcagctttcggcgcgctgctgatcgtggtgttcaacagcgcctacggcgtgatcaacgcacgcaagcagcgcgtgatggccgcgcgcgtcatgggcgcctcgcgctggcagatcttcaaggacgtgctggtgtgggaaagcctgcagcccagcttcgtgggcctgcgctcggcggtgtcgatggcactggtgatcgtcatcgtggccgagatgttcatcggctccgacaccggcctgggccaccgcatcatcgatgcgcagcaggtgctcaacgtgaaaagcatgtacgcggccattcttgcggcgggcgccctgggctatgcgctcaacatcctctttctcattgccgagcgccgcatcgtgcactggagcggaagatgaaagtgacgcccgacatcgtcgtcaacggcccggtgtatgccgacgtgcccaggcccgtcttcaagcccggcccggccggcacgcacatcaccattcgcgggctcaccaagtactttgcgggctggccgctgtacgagaacttcgacctcgacattcccaagcacaggatcgtctcggtgttcgggcccaacggctgcggcaagtccacgctcatcaacatgatcgcggggctggttcccatcgactcgggcgagatcctgttcgacggcaagcagcgcaaggacaccaagatcggctacgtgttccagaactaccgcgaggcgatgttcccgtggatgcgcaccatcgacaacatcgcctacccgctgaagctcgaaggacgcagcaaggccgaggtcgaccgccgcatggaagagctggtggcgtcgttcgacgtcaagttcgacctgaagcgatttccctacgagctttcgggcggccagcagcagaccgcatcgatcatgcgggcgctcgcgcccaaccccgaggtgctgtttctcgatgagccgttttcggcgctcgacttcgagatgacgctcttcatccgcgagaagctgcaggaggtgttcatgcagaccggcaccaccatgctcctggtgtcgcacgacctcgaagaggccgtgtacctggccgacgaggtgctgctcctgaccaagcggccgaccaaggtggccgagatcctgcgctacggcgatgcccggccgcgcaccctggagacgctgagcagcgacagcttcgtcgcgatgaagaagctcagcctggacatcttccagcgcgaggttcgccgatgaccccggagatcaacattcccgaggtgctcaccgaagtgacggccgtgttcgcgcgctacgaagaagcgctggtgacgaaccagcgcgccgtgctcgacgagttgttctggaacagcccgcacacgctgcgctacggcttctcggagacccactacggccacgccgacatcagcgccttccgcgcatcgttgccgctgcagagcccgccgcgcgagctgctgcgcaccgtcatcaccacctacggccgcgactttgcgaccgccaacgtcgagttccgccgcgaaggcagccgccagaccggccgccagagccagacctggctgcgtaccgccgacggctggcgcgtggtcgccgcgcacgtgagcctgatggactgaacacgcaggcacattttttgcaccccaacttgtatccaagatcggagaatgccatgaccagccccatcaaccgccgcgattccctcaaatccctggccgcgcttggcgctgccggcaccctggggggctggagcgcccttgccggtgcacaggccaagccgctgaccgtcggcgtgatctacgtcggtgcgcgcgacgactacggctacaaccaggcgcacgccatggccgcggccgaagtcaagaagctgcccggcgtcaaggtggtcgaagaagagaacgtgcccgagaccgccgccgtgcagaagaccatggccggcatgatctcgcaggacggtgccaagctgctcttccccacgtcgttcggctacttcgatccgcacatcctcgcggtggcgcccaagaaccccgacgtgcgcttctcgcattgcggcggcctctggaccgaaggcaagcaccccaagaacgccggcagcttcttcggctacatcgacgaatgccagtttttgaacggcgtgatcgcggcgcacatgaccaagagcaacaagatcgccttcgtcgccgccaagccgatcccgcaggtgctgcgaaacatcaatgccttcacgctcggcgcgcgctcggtcaagccgaacatcacctgcagcgtgatcttcacgggcgactggtcgatggccgtgaaggaagccgaagccaccaacagcctggccgatcagggctgcgacgtgttcaccatgcacgtcgacggccccaaggtggtggtcgaaacggcggccaagcgcggcaagatggtctgcggctaccacgcgagccaggccaagctggcgcccaacgcgtacctcaccggtgccgagtggaactggctcaccgcctacaagaccgccatcgaagccgcgcaaagcggcaagccgcaccccaacttcctgcgcggcggcctgaaggaaggctacgtgaagatgtccgcctacggccccatggtgccggacgccgcgaagaagcaggccgacgagatcaaggccaagatgatcgcgggcaccttcgacatcttcaaggacggcatcaaggacaacaagggcgccgtcgtggtgccggccggcaaggtgctcaagcagaccgacctcgagctggaaaagatgaactacctcgtcgaaggcgtcatcggttcggcctgattcgcgccgcttcatcgccatgcgccacgcgctcaaggaattcgccctgccggtgttcgccattgcggcggcgctgctgttgttcggcgtgctagtggcctttgccggggtcgatccggtggaggtctgggcgacgctgttcaagggcgcgttcggcgactggttctcgtggcagaacaccctgcagcgcgccgcgccgctgatgctcaccgccctgtgcgtggcgctgcccgcgcgcgcggggctcatcgtcatcggcggcgaaggcgcactggtgctgggcagcctggcctcggcggcgcttgcgcatgcggtgccgttgcccggcaacgtggtgggcacggcggtggtctgcctcgccggcgcactggccggcgcgctgtggatcgccttcgcgggctggctgcgccagtaccgcggcatcaacgaaaccatcagcagcctgctcctggcctacatcgcgatcggcatcttcaagcacctggtcgaagggccgctgcgcgatccggcgagcctcaacaaaccctctacctacgcgctggacgccggattgctgatcggcggtatcggcggctctgacgtgcactggggcctggccatcggcgtggtggcgtgcctgggactcgggtggtggctgcgcgccacggcctcgggcttttcagtgcgcgtggtgggcggcaatccgcgcaccgcgcagctcgtcggcctgccggccacgcggctcatcctcggcgcctgcggtttgggcggcgcctgcgcggggctcgcgggcgcggtcgaggtggcggcggtgcacaccaacgccaatgcctcgctgatcgcgggctacggctatgcgggcatcctcgtgtccttcatcgcgcggcacaacccggtggccatcgtgccggtcgccattctcttcggcggcttcggggccgccggcagcctgttgcagcgtcgtctcgggctgcccgatgcctcggtgctggtgctgcagggcatcgccttcgtgctcattctcgcgagcgaggggctgcgcatggtcgactggaaggcattgatgagccgcagggccgctcccaaggcggatgccgcagtgcgcagtgcggaggttgccccatgaccgcggaccagtggatcgccctggtcgccggcatcgtcggcggcgccttgcgcgtgggcgcgcccttcctgttcgtgagcctgggcgaatgcctcaccgaaaagtcgggccgcatcaacctcgggctcgaaggcgtgctggtgctctcggccatggcggccttcggcggcgcatatctcaccgattcggcctggctcggcgtgctgatcggcgcggtggcgggcgcgctgcttgcgctgctccacggactcctgtgctcgctcgaccgcgtgaacgacgtagcgaccggcatcgccttgatgctgctcggcacggggctcgcgttctacctcggcaagccgctcatccagccgcaggcgccgcagattcccgcgataccactgggcttctggagcgacaacccggtggtgcgttccgccttgcagctcaatgcgctggtgcccgtgggcgtggtgctggccgtgctgctctggtggggctttgcccgcacgcgcgccggcttgctggtgcgcatggccggcgattcggcgcaggccacgcgcgcgctcggctattcggtgtcgggcctgcgcatcgcggcgacgacggcgggcggcttcattgccgggctcggcggcgcgtcgctcacgctgttctatccgggcagctggaacgaaggcatctcgagcggccagggcctgattgcggtggcgctggtgatcttcgcgcgctggagcccgctgcgctgcatcggcgcggccttgctcttcggcggcgcgggcgccatcgggcccgcgctgcagtccatcggcgtcggctggggctaccacctgttcaacaccgtgccttacgtgctcacgctggtgatcctggtgctcacctgcaagccgggcacggcagccgccggaagccccggcgaactttcatcgacaaggagctgaatgccatgatcgcccgtcacattgccgccgagccttatgcctggccctacaacggcgcgctgcggcccgacaacaccgcgctcatcgtcatcgacatgcagaccgacttctgcggaaagggcggctacgtcgacgtgatgggctacgacctctcgctggtgcaggcaccgatccaaccgattgcgcgcacgctggctgcgctgcggccgctgggctatcacgtcattcacacgcgcgaaggccatcggccggacctggccgacctgcccgccaacaagcgctggcgctcgcggcagatcggtgccggcggcgtgggcatcggcgacgacgggccgtgcgggcgcatcctggtgcgaggcgagccgggctgggagatcattccggaactcgcgccgctgttcggcgaggtggtgatcgacaagcccggcaagggctcgttctacgcgacggacctggagctgatcctgcgcacgcgcggcatcgagaacctgattctcgcgggcatcaccaccgacgtatgcgtgcacacgacgatgcgcgatgccaacgaccgcggcttcgaatgcctgctgttgtccgactgcaccgccgccaccgaccatggcaaccacctggcggcgctgaagatgatcacgatgcagggtggcgtgttcggtgcgcatgccacctcgcaggcgctgttgagtgcgctgggctgatgcggccatgaccgcttcttccgccgccacccatgccccgcacgccccccacgccattggtgcgctgccgagcggcagcggcgcgctcgcgctcgacacctacgagctgaccaagcgcttcggcgccttcaccgcgatggaccgcgtgacgatgcgcgtggagcccggcacggtgcatgcgctgctcggcgagaacggcgcgggcaagagcacgctggtgaagtgcgtcgccggcttccagcgcgcggaagagggcagcatcctgatcgacggccgcgagcaggacattgccaaccccatcgtggcgcgcgcgctcggcatcggcatggtgtaccagcacttcacgctggcgccgggcatgacggtggccgagaacctgctgctcgcgggcggcaagacacccgcgctgatcgactggaaggcgaagcgggccgagctcaaggcctttctggcgaccacgcccttcagcctcgacctcgacgtgcggccctcggagcttgcggcgggcgaaaagcagaagctcgaactgctcaagcagctctacctgaagccgcgcctcctgatcctcgacgaaccgacctcggtgctcacgccgcaggaggccgacgaggtgctcggccacgtgcgcgagttcgcgaagagcggcctgtgcaccgtgctcatcatcacgcacaagttccgcgaggtgatggcctatgccgacagcgtgacggtgctgcgccgcggcaaggcggtgcaccattgccgcgtggcggacacgagccctgcgcggttggcaggggccatgatgggcggcgaggacgctgcggtttcggcaccggctgcatcacccgtcgccagaaagcccgtgcccgctgcggcgcccattgcattgaaggtcgaaggactcaaggcgcagggcgaccgcggcaccttggcgctgcacgacctggccctttccgtgcgcgcgggtgaaatcctcggcgtggcgggcgtctcgggcaacggtcagcgcgaactggtcgaggctctggtcgggcagcgtccgcggctcgccggcaaggtgagcgtcatgggccaagcgtacagcgcgcggcgcgcagagaaccgcagcctcaaggtgcgcagcctgcccgaggagccgctgcgcaatgcctgcgtgggcgacctcagtgtggcggagaacatggcgctgcgcgatttcgacagacccccgttgtcgcgcggcggggtgttgaattttccgttctggcgcagccgcgcgcgcgagtggattgccgaatacggcgtcaagacgcagggcgagggcgccgcgattcgcagcctctcgggcggcaacgtgcagcgcgcggtgctggcgcgggagctcgccggcgacatcaacgtgctgatcgcggccaatcccgtgttcggcctcgacttcgccgccgtggccgaaatccacgagcgcatcgtgcaggtgcgcgagaagggcggggcggtgcttctcatcagcgaagacctcgacgagctgctggaactggccgaccgcatcgtcgtgatgagcgagggacggatcgtgttcgagacctcggccgcgggcgccgaaaggcatgtgatcggggcgcacatgggcggtgggcaccacgagccactgaaggctgcggcatgagcggccctttgaattaaagagcaacaccatgcgcatagaagaagccacccccttcccctacgagctcgagatcaagaacaccgccctggtcctcatcgacatgcagcgcgacttcatcgaacccggcggcttcggcgaaacactgggcaacgacgtgtccttgctcgaagcgattgttcccgcgacaaagacggcgctgcaggcatggcgggaagcaggcggcctcgtggtgcacacccgggaggcgcacaagcccgacctctccgattgcccgcccgccaaacgcaaccgcggcaaccctgcgctgcgcatcggcgacgaaggcccgatgggccggattctcgtggccggcgaaccgggcaaccagatcatcgaggcgctcgcccccatcggcggcgagatcgtcatcgacaagcccggcaagggcgcgttctatgccaccggcttgcatgaactgctgcaacagcgcggcatcacgcacctgctgttcggcggcgtcaccaccgaagtctgcgtgcagacctcgatgcgcgaagccaacgaccgcggctacgactgcctcttgctcgaagactgcaccgagagctactttccggccttcaaggccgccacgctcgacatggtccgtgcccagggtggcatcgtcggctggaccgcgccgagcgccgcgctcttggcggcgcttcgcggcgggcaatgacagcgactactattccatacgtgcctaccgttcgttcccgctccgcctcacccgcatccgccgttcccgccgctggcgcgacaaccgtttttcgcacccgcgccgacgaggtctacgcgcagctcaagcgcgacgtggccgatttcatcctcgtgcccggcgaccgcttcaccgagaacgagatcagcgagcggctcggcgtctcgcgcacgcccgtgcggcaggcgctgttccgcctccagcaggaggggttcgtcgaagtgctgttccgcagcggctggcgcgtgctgcccttcgacttcgaccagttcgagcagctctacgacctgcgcatggtgctggagaccaccgccgtgcatcgcctctgcgaagccgaccgccgtgtcgaccgcagcctgctcgatgcgctggccgatatctggctcgtgccggtggcccagcgcagcagcgacaccgcgcaggtggcgcaatgggacgaggcttttcattgcgcgctcgtggccgccgcgggcaacgccgagatggcgcgcgtgcacagcgacgtgaccgaccgcatccgcatcatccgccggctcgacttcacccagcagccgcgcatcgacgccacctacgacgagcacgcgaagatcctgaaggccgttcgcgccaaccgcggagaccaggccgcgatgctgctgcgcgcgcacatcgagaccagccaggccgaggtgcgcaagatcacgctgcaccaggtgcacctggcgcggcatgccggcaagacggccgcgccgcgctgatccgtcagagcttgaagtcgtactcgaccgtgatgggcgcgtgatcgctgaacttgatggtcttgtagatctgctcggtgcgtgcgagggcgccgagcgctggcgtggccaggtggtagtcgagccgccaccccacgttgttggcgtaggcctggccgcggttgctccaccatgtgtaggcctcggccgtggtctcaggcttgagcatgcgatagacgtcgaccaggcccgcaccgtcggtgccggcgtcgagcagccgcgtcatccaggcacgctcctcgggcaggaagccgctgttcttctggttgccgcgccagttcttgaggtcgatctccttgtgcgcgatgttgatgtcgccgcagaggatgaattcgcgctttttcttgagcgccacgaggtgcgggaagaagcccttcaggaaccggaacttggcttcctgccgctcctcgcccgagcttccgctcggaaagtagcagctgatgatcgacagcttgcgccccggcgtgtcgaagcgcagttcgagataccggccttcggcgtcgaattcggcgtcgccccagcccacgaccacgtcgctgggcgcgtgtttcgtgtagatcgcggtgccggcgtagccttttttctcggcgaaatgaaagtggcccttgagccccgccatttcttcgaagcggccctcgatgtcgctcgcctggacccggatttcctgcatgcaaatacaatccggcgcaagttcggccacccagtccgccacccctttcgtggcggccgaacgcaggccattgagattgaggctggtcagtttgaacacaaggaaattccgatggctgtagatggtgtggaaagcagtgcggtggcacaggacttcgttcagtttgcactcgacgcgggcgtgctgcgctttggcgagttcaagaccaaggccggccggctgagcccctatttcttcaattcgggcctcttcgacgacggcgccaagatcgcgcggctcgccggattctatgcagaccgactgatcgagagcggtgtcgagttcgacatgatcttcggccccgcctacaagggcattccgctgggcgccacggtggccgccgaactggcccggcgcggccgcaactacccctttgcctacaaccgcaaggaagccaaggcgcacggcgaaggcggcaacctggtgggcgcgccgctcaagggccgggtgctgatcgtcgacgacgtgatgtcggccggcaccgcggtgcgcgaatcgatcgccgccatcgaggccgcgggcgccacgccgcacgccgtcgccattgcgctcgaccggcaggaaaaagccaccgagaacggcgtggacgtggaccacagcgcggtgcagtacgtgcgcaaccagctgggcctggcggtggtggccattgccacgctcgacgacctcctgaactacctgtcgggcagccatgccgccgccgacctgggtacgcaccgggagcgcgtgctcgcctaccgcgcgcgctacggcgcccgctgaggcccgcccccatgcctgtgcgcaagctcgagaaccagaccgtgcggccgcttgccgcagcggcgctgctgctgtcgatggcggcggtgctgctgatgttgcccgccgaagtgccggcgcagcctgcaacgcaggcacccgccagtatctatacctgcaccgacgcccgcggccgcaccctcacggccgaccgtccgattgccgaatgcaccgaccgggagcagcgcgaactgaatccgagcggcaccacgcgccggcgcgtcgagccgacatataccccccgcgagttggctgagcgcgaagaccgcgcccgcgaagcggcgctgcaggccgcgcgccagctcgacgagcgccggcgcgagcgcgcactgctggtgcgctatcccaatgccacggtgcatgaccgcgagcggggcgaggcgctggtgcagatcgatgcggtgatccaggcggccaggaagcgcctggaggagctcgccgaggaccgcaagaaggtcgaggaggagctcgagttctacaagcacgacgtcagcaaggcgccgggcgccgtgcgccgcaagctcgaggacaacacgcagagcgtggcggtgcagaaccgcttcatcggcgagcaggaagacgagaagaggcgcgtgaacgcgcgcttcgacgaggagcgcgcgcgcttaagacagatctggtccccccagaacggcggcggcaagtagctcgccgccggccgatcaggccagttttgccttcagaagttcggtgacttgggcggggttcgccttgccgccgctggccttcatgacctggcccacgaggccgttgagggccttttccttgccggcgcggtattcgtcgacgttcttctggttcttggcgatgacctcgtccaggatcttgtcgagcgcgccggtgtcgctcatcggcttcaggtccttggcttcgatgatggcgtccacctcgctgccttcgccggtccagagcgcctcgaacacctggcgcgcggcgttgttgggcagcgtgccgtcggcaatgcgcttcaccagctgggccagttgctgcgccgtgaccggcgcggcctcgatgccgatttcctgtgcgttcaggcggcgcgccatctcgccggtgatccagttgcttgcgagcttgggagtggcgcctgctttcaccgcatcgtcgaagtagcgtgcgagcgcggggctctgcgtgagctgcgccgcgtcgtattccgacatgccgtggtcgcgcacgtagcgctcggccatggcgcgcggcagttcgggcatggtggcgcgcacgcgctcgatccattcgggctcgatggccagcggcggcaggtccgggtcgggaaagtagcggtagtcggccgcgtcttccttggtgcgcatggtgcgcgtctcgccggtatcggggtcgaacagcacggtggcctgctcgatcttgcggccgtcttccagctcgttgatctgcgagttgatctcgtagtcgatggcctgctgcatgaacttgaagctgttcaggttcttgatctcgcgccgcgtgccgagcttttcgccgggcctgcgcaccgacacgttggcgtcgcagcggaagctgccttcctgcatgttgccgtcgcagatgccgatccaggtgacgatcttgtgcagctcgcgcgcataggccacggcctcggcggtggagcgcatgtcgggctcggtcacgatctccaagagcggcgtgccggcgcggttcaggtcgatgccgctctggccgatgaagtcttcgtgcagcgacttgcccgcgtcttcctcgaggtgggcacgcaccaggcgcacggtcttcttttcttcgcccagaaagaacgagaccgagccgccctgcacgaccgggatctcgtactggctgatctggtagcccttgggcaggtcggggtagaaatagttcttgcgcgcgaacacgctgcgcggcgcaatgtgcgagccgagcgccaggcccagcttgatggcgcgctcgacggcgcccttgttcatcaccggcagcgtgccgggcagcgccaggtccaccgcggaggcctgcgtgttgggctcggcgccaaaggcggtggaggcgcggctgaagatcttgctcgcggtcgacagttgcgcgtgcgtctcgaagccgatgatgacttcatagccgcgcaccagcgggccggtcgggcggccttgttgctgtgcttcgaaagtattcacgggttcgctcatcttaaaagccctccggcgtgcgcgtgtgccagtcggtggcctgctggaagcggtgggccgcgttcagcagcttcgcttcggcgaagtagttgccgatcaattgcaggcccacgggcatgcccgcatcgaagcccgcgggcacgctcatgccgggaaggccggccagcgacgcgggcagcgtgaagatgtcggcgagatagtcggccaccgggtcgccgccgtgttcgccgatcttccaggcagtggtcggcgcggcggggccggcgatcacgtcgcactgcttgaaggcctgctgaaaatcgtcggcaatgatgcggcgcaccttctgcgcctgcaggtagtacgcgtcgtagtagccgtgcgacagcacgtaggtgccgatcatgatgcggcgcttcacctcgtcgccgaagccttcggcgcgcgtgcgctcgtacatgtcggccagatccttgtactggctggcgcggtggccgaacttgacgccgtcgaagcggctcaggttgctcgaggcttcggccgcggccaggatgtaatacaccggaatcgacagctcggtgagcggcagcgtgacttcgacgcgcttcgcgccgagcttctcgtattgcgcgagcgccgcatcgatggcggcgcgcacgccgggcgcgacgccttcgccgaagaactccttcggcacgccgatgcgcaggccttcgagcgagtcgccgagcgagcggccgaagttctcggcgggcttgtcgagcgaggtcgaatcgcggtccaggtcggggccgcagaaggccgacagcagcagcgcgcagtcttcggccgagcgggccatcgggccggcctggtcgaggctcgatgcgaaggccaccatgccgtagcgcgaggcgcggccgtaggtgggcttgatgcccgtgacgccgcagaacgaggccggctggcggatcgagccgccggtgtcggtgccggtggccgctggcgcgaggcgcgccgccacggcggccgcgctggcgcccgaggagccgcccggaatgtgttcgcggttccaggggttctgcaccggcacggccttgtcgtggcccacggcgggcacggcgacgttctcgttggccgagcccatcgcgaattcgtcgcagctcagcttgccgagcgtgaccgcgccggcctcggccaggcggcgcaccacggtcgcgtcgaagggcgagcggtagcccgcgagcatcttcgagccggcggtggtggcgaaatcggtggtgacgaagatgtccttgtgcgcaatgggcacgccggccagcgcgggcgcgttgcccttggcgatccgggtgtcggcggcacgagcctgggccagcgtgacctcctcgttgacgtctacaaaagtacccagtgcttcgtgcgccttcatgcgtccgaggaaaacctgcgcggtctcgacggcggaaaccttgcgctcggccagggccttggcgagggcgaccacgcccaactggtgcaattcgccgctcattcgatcaccttcggcacgaggaacaggccggcttcgacggccggggcgctcttctggttggcttcgcggttgtcgggttcgctcaccacgtcgtcgcgcaggcgcagcgtgacatcctggacggccgccaccgggtgggccagcggctcgacgccggtggtgtcgacggagcgcatgcgctcgaccaggtcaaagaagccgttgatctggctgagcatgcgctcgctttcgtcgggagcaagctgcagccgtgccagcgaggcaatgcgtgcaatatctgaagcggaaagggacatggatgaaaccggccaaaaaaaccggaggtaatgcacgccggagggggtgctgacacgggattcagaggggattcaggtattatcccgcctttgccgcaacccccgcgaacgcgccggcttttgcgccaaaaacgatcaatacaccccgtcacacgacccaaaaacagagcgacgacctgccgacgcgcaggccgtgctccagaggattccgcacatgtttggagctttccgtcggtacttttccaccgaccttgcgatcgacctcggcaccgccaacacactgatatttgcccgcaacaagggcatcgtgctggacgaaccctcggtggtcgccatccgccacgaaggcggcccccacggcaagaaggtgatccaggccgtcggccgcgaggccaaggcaatgctgggcaaggtgcccggcaacatcgaggcgatccgcccgatgaaggacggcgtgattgccgacttcgtgatcaccgagcagatgatcaagcagttcatcaagatggtgcacccgcgcacgctgctcacgcccagcccgcgaatcatcatctgcgtgccttgcggctccacccaggtcgagcgtcgcgccattaaggacgcggccgaagcggccggtgctacttccgtctacctcatcgaagaacccatggccgcggccatcggcgccggcctgcccgtgagcgaggcttcgggctcgatggtggtcgacatcggcggcggcaccaccgaggtgggcgtcatcagcctgggcggcatggtctacaagggctccgtgcgcgtcggcggcgaccgcttcgacgaagccatcatcaactacatccgccgcaactacggcatgctgatcggcgagccgacggccgaagtcatcaagaagaacatcggctcggccttcccgggctccgaggtcaaggagatggaagtcaagggccgcaacctgtccgaaggcgtgccgcgcagcttcaccatcagcagcaacgaagtgctggaagccctgaccgatccgctcaacaacatcgtctcggccgtgaagaacgcgctggagcagacgccgcccgaactcggcgccgacatcgccgagcgcggcatgatgctgaccggcggcggcgccctgctgcgcgacctcgaccgcctgctggccgaggaaaccggactgccggtactggtggccgaagacccgctgacctgcgtggtgcgcggttgcggcattgccctcgagcgcatggaccgcttgggaagcattttcacgagcgagtgaatgcgtcaccgccatcatcggccggctctgcttgcgcaggccggcctttttgccatctgacgttgcacggccaggcttgaaccatgcccttgggcacgctcgatcgcacagccccgcccctgttcaaccaggggcagtcggcgctgagcaagctgatcttcttcggcgcgctggcgctgttcctgatggtggccgacgcgcgcttccatctcgtgcagccccttcgcgccgccgtcggcgcggtgctctacccggtgcaatggttggcgctcaagccggtgcagctggcgatcggcggcggccgctatctcgaagacctccagaccgcgcagcgcaacgagaacgaggcccgcaaggcgctcatgctgcaggccgagcgcgcgagccaggccgacacgctggcgcaggacaacgcgcggctgcgcgcgctgctcgaactgcgccagaccacccaggcgccgggccgcgcggccgaggtgctctatgacgcggccgatccgtacacgcgcaagatcgtcatcgaccaggggctcacgcagggcgtggcgcccggctcgcccgtgatcgacgcgcacggcgtgctcggccaggtgacgcaggtgctgcctttcaccagcgaaatcacgctggtgatcgaccgcgatctttccatcccggtgcagaacacccgcaccggcgtgcgcagcgtggccttcggcgacgcgtcggcgcacgggggcgggctcgagctgcgcttcatggccgccaatgccgatctgcaggagggcgacctgctctccaccagcggtgtcgacggcgtctatccgccgggcctgccggtggcgaagatcgagcgcatcgaacggcgcgccgactccgcctttgcacgcatctactgcgtgccgctggcccgcgtgacggccgcgcgctacgtgctggtgctggcgcccacgggcacgccctcggcaccgccccccgccgcgcccgccgccgcggtgcgcaagaagtcagaggccaagcccgccaaggcggacaacaagggcgacaaggccgagaagaaacccgcggagcacgcccgatgatcaagcgtcccggacaacagcagctcctgctgcccgtgagcccgctgttcatgtgggccagcctcgtggtggcgctgctcatcaacatgatcccgatcggccgggccgcgtggatgcccgatctgctggccctggccatcgtgttctggggcgtgcaccagccgatgcgcgtgggcattggcgcagccttcgtgttcggcctgtgcatggacgtgcaccaggcctccatgctgggccagcacgcgctgtcctacaccacgctgggcttcttcgcgatcaccatccaccggcgcctgctctggtatccggtggcgtcgcaggcgttgcaggtgctgccgctctttgcagtttcgcagctgatcgaggtcgtcacgcgcatgatcggcggcggtgtgtttccgggttggacggtgctcatctcgccggccatcgaagccgtgttgtggcccttggcgaccgccctgttgcttgcgccccagcgccgcacccccgaacccgacgagaaccgtcctctttaagccaaagctcgcatttgcctttggatttgccatcgcacttgcacgcgcctaagctcacgccgccatgaccgagatccgcaacgttgccgccgacctcgcgcgcttcaagcgccgcgtgatcgtgatcggcatggtggtgctcttcgccttcagcctgctcggcgcgcggctggtgtacctgcaggtggtgcggcatgaagacctggccgagcaggccgagagcaaccgcacggccatcgtgcccgtggtgcccaaccgcggcctcatcctcgaccgcaacggcatcgtgctggcctcgaactattcggcctacacgctggagatcacgccctccaaggtgggcgacgtcgaggagaccatcgagagcctgacgcaggtgctcgaggtctcgccgcgcgaccgccgccgcttcaagcggctgcgtgaagactcgcgcagcttcgactccattccgatccgcacccgcctgagcgacgaggaggtggcgcgtttcgcggcgcagcgctaccgcttcccgggcgtggagatcaaggcgcggctgttccgcaactacccgcatgccgagatcgcctcgcacgtgctcggctacatcggccgcatcaaccagcgcgagaagaccgcgatggaagactgggccgaggaagaccaggccaactacaagggcaccgactacatcggcaagctcggcatcgagcaaagctacgagaagacgctacacggccagaccggcgtcgagcagatggaaacctcggccggcggccgcgcgatacgccggcttgcgagccatccggccacccccggcaacaccgtgatgctgtcgctcgacatcaagctgcagaagctggtggaagacatgttcggcgatcgccgcggcgcgctggtggccatcgaccccaagaccggcgaggtgctggccttcgtgagcaagccgaccttcgaccccaacctgttcgtcgaaggcatcgacaccgaaagctggaaagagctcagcgaatcgctcgacaagccgctgctcaaccgcgccctgcgcggcacctacccgcccggctcgacctacaagcccttcatggcgctggcggcgctgcagactggcaagcgcggcccgaacgtggtggtgaacgaccccggctacttcaatttcggcgggcaccgcttcggcagccccgaaggaaacctgggcggcgtcgacatgcggcgctcgatccaggtgtcgagcaacatctattactactcgctggccaacgagatgggcgtggatttgatccacgacttcatgaaaccgatgggcttcgggcagatcaccggcatcgacctgggcggcgaagtgcgcggcgtgctgccgagcaccgaatggaagcgcaacgcctacaagcggccggagcagaagaaatggtatgcgggcgagaccatctcgctcggtatcggtcagggctacaacaccttcaccatgctgcaactggcgcaggccacggccatcgtggccgacggcggcatgaagcacaaaccgcatctggtgctggccacgcgcaacacggtgagcggggaagtggcgccagtgccccagccgccggccgagaacctcggctacaccgcagccaacgtcgcggtcattcgggagggcctcaccagcgtggtcaccagcggtacggcgcgcggcgtgttcgccggcgccagctaccaggcggccggcaagacgggcactgcgcaggccgtgacgcaggcgcagaacaccaagtacaacgcgcgcgcgctcgaggagcaccagcgcgaccacgccttgttcatggcttttgcgccggtcaacgatccgaagatcgccctggcggtgatcgtcgagaacgcaggctggggcgccggtgccgcggcacccatcgcgcgccgcgtgttcgactactggctgctggaccagtacccgagcgaagccgacatggccgccatcaaggtcggcaaggccgccgcccccatgggcaagccgcgcgtggccagcgaagtggcgtggccggctgcggccaccgctgtaaccgcaccctgatcttgctccctctccctctgggagagggttggggtgagggcactgtgccgccgataaagtgcggcgcccatacgacggccgcctgccctcaccctagccctctcccagagggagagggaacaacgcggggaggggatgaacctcagggcaccaccgtgccgctgacttcccccagcccgatgcgcactgcccccgcgcgctcgcagtagccgcgcatgaccagcgtgtcgccgtcttcgagaaaggtgcgcttctcgccgttgggcaaggtgattgcctgcttgccgcccagcgtgagctctatcagcgaaccagcctcgtcgggcttggggcccgagagcgtgcccgagcccagcaggtcgccgggctgcaggttgcagccgttcaccgtgtggtgcgcgacgagctgcgcggcggtccagtaggcggcctcggtggtgttgccgcgcgtgaggcgcatgggagcttcgcccgcggtgcgcatcttcgccgtctgcagcagcacttcgagcgtgatgtcgagcgcgccgctttcgcgattggacggcgcatcgagatacggcagcggctgcgggtctcccgcctggcgctcgaacctggcgcggaaaggcgccagcgcttccatcgtcacgatccacggcgagagcgtgctcgcgaagttcttcgagaggaacggcccgagcggctggtattcccaggcctgcaggtcgcgcgccgaccagtcgttgagcagggtcacaccgaacagatggtcctcagcctcgccgatcgcgatcggctcgccgagcgcattgccgcggccgacaaagaagccaagctccagttcgtagtcgagccgcttcgacgggccgaagctcggttctgccgcatccggcgccttggtctgcccctgcgggcgcttgaagacctgcccgctcacgccgatggacgaggcgcggccgtgatagccgatgggcacccacttgtagttgggcatcagcggctggtcgggacggaacagcttgccgatggtggtcgcgtgatggatgccggtgtagaagtcggtgtagtcgccgatgcggcagggcacggtcatttcggccctggcctgcggtagcagcgccttcgaccatgcggcctctttgccgttgccttcggcaaggccggccgagatggcggcgcgcagggcctggcggtccttcgcgctggcgctcatcagcgcgttcatgtcgtcggtgccggccaggcctgcggcccggaggtcgagcacctggtcgccgatggccacgccgatgcgaaagccttcgctgctgccggcagtgcggaagcgtccgaagggcaggttctggatcgggaagtcgcagccgggctcgttggccgaggcgacccagctgcgcagcttcgggtcgtgggtggcgttcaatgcgatggtcatgaatgtctttctgtaatgtcggttcgctcgaacaacgtcacgccttgaactgatcctggaggccggcccagcagtccgcgtagtcggagtcgagcgccgggctctggagcgcgaagttcgtcggaatgaagcgaaagcggctctcgaacatgaaggccagcgtgttgtccagcttgtgcggcttcaggtcggagtgcgcggccttgtcgaaggcttcctcgtcgggcccgtgcggcaccatgcagttgtgcaggctcgcgccgccgggcttgaagccgcccggcttggcgtcgtactcgcccagcaccaggcccatgaactcgctcatcaagttgcggtggaaccatggcggacggaaggtgttctccatcaccatccagcgcggcgggaagatcacgaagtcgcagttcgcggtgccgggcgtgtcggtgggcgaggtcagcacggtgaagatcgagggatcgggatggtcgaagctgatcgagccgatgaccatgaaattggccgtgtcgtacttcaccggcgccaggttgccgtgccatgcgaccacgttgaagggcgactgcttcgtcggcgccttccagaagcggccgccgaacttcttgacgagttcgtaggcgccgccgtcgtcctcgaaagccgccacgggcgcctggaagtcgcgcgcgttggccaggccgttggagccgatggggccgagttcgggcaggcggaaatgcgccccgtagttctcgcaggcatagccgcgggaaagcccatccggcagcgccaccttgaatgccatgccgcgcggcagcacggcgatttcgccgggcttcacgtcgagcacgccgagttcggtcgtgatcacgaggcggccctgctgcggcacgacgagcatctcgccgtcggcgttgacgaaggcgcggcgctccatcgagcggcccgccaggtacatgagcgagccgatgcccacctgcgcttcggcgtcgccgttggccgcgatcgtgtgcatgccgtcgatgaagtcggcctcggccgcgccgtcgagcggaagcggatgccagcgcagcggctcgggcggcagcgcgatctcgcggtcggcgccggtggtccagtgcgcctgcgcatacggctggtagcggcccgacaccaccgagggctggcggcggtagagccaggtgcggcggttttcgcggcgcggcgcggtaaaggccgtgcccgagagcagttcggtgtacaggtcgaacggcgcgcgctgcgggttgttgcggccctgcggcagggcgcccgcgacggcctcgctggcgtactcgttgccgaagccgctttgatagagccgttcggtggcgggggttgcggtggtcatggtgtccttcctcacgggatggcttgtggatggtcttgcttcgctgcgtcgagcgcttcgcgcagcacggcgagcgagccgacgtggttggccagcaccagcacgaggcgcgcgttgtaggcgtggctctcttcggtggaaagcccctggtgcgcctcgatcagcgcttcgtagaaatcgtcgggcgcgtcgaggttcggcgcggtgttcaggtggtgttgctgttgcatagtggtgctcaagcctttgccagtgcgtggtcgatggcggcgcggatgttctctgccgtgggatgccgccagcgcgcgcacacatgctggtcgggccgcagcagatagacggtgccgggctgcgcgtcgtaacgctgcgtggcaagttcgccttcgggcgacgcgccttgcacgcgcacgatgtgcagcggaaagtcgcaggccttcagcgcctgcaggctgcgttcggccgcctcgcccgtgccgaacaccagcgcggtgaaccgcaccgcatggcattcgcgcagcagccagccggtgctgccgtcggcccgcacgagcggcgcatcgaccgccgcggcgcccggcaccatcgcacccttgaacacatcggcatcgggcgtgttgagcggcgaatcgcgcagcacggcgggcaccgagagccgcccgctgttgaccagcgtgcgcgcgaaggcatggcgcttggtgagctccagcaccgcgtcgcggaacaggcggctcacttcgctcttgggcgtgatgaagtcggtggcgcgcgtggagttgcggatgttctcgtcggccgcgtgttcgcgctcgcttgcatagctgtcgagcagcgcatcgggcgcgtcgcccgcgagcacggccgcgagcttccaggcgaggttgtcggcgtcctgcacgcccgagttggcgccgcgcgcaccgaagggcgacacgccatgcgccgagtcgcccgcgaacagcacgcggccatggcggaagtgctccatgcgctggcatgcaaaggtgtagacgctggcccagccgatctggaactgcacgccctcgaagccgatgctgtcgagcagcgcgcgcacgcgcggcgtgatgttctcgggcttgcgttcttccaccggatcggcgtcccagccgagctggaagtcgacgcgccacatgccgtcggcctgcttgtgcagcagcacgctctggccggggtggaatgggggggcgaaccagaagcggcgctctgtaggcaggtccgcatccatcgtgatgtccgcgatcaggaagcggtcgcggaacacgcgccccttggcttcaaggcccatcagttgccgcaggttggagcgcgagccgtcgcaggcgccgacgtagtcggccgccagctggtagctgccctcgggcgtctccaccgtgagcatcgccgcgtcgccgccctgcgcgatgcccgtgaccttgttgttccagcgcaggtcgatcagcgccagcgccgcggcgcgctcgacgaggtagccctcgacgtaatactgctgcaggttgatgaaggccgggcgctcgtggccgggctcgggcagcaggtcgaagcggtagacctgctcgtcgtggaagaacaccttgcccacgtgccacgacacgcccttgtcgaccatgcggtcgccgcagccgaggcggtcgaacacctcgagcgtgcgcttggcaaagcagatggcgcgcgagccgctggacagggtgttgtcgttgtcgagcagcaccaccggaattttgcgcagcgcaaggtcgatggccagcgcgaggccgaccgggccggcgccgacgatcaccaccgggtgacgggcgggcgtggccgcgtcctggtcggcgtggcgcttgtagtcgaagcgcaggctttgatagtcgatcacgtgttgtctccgtgtctttgtcttgctccttccccctttgggggaaggctgggatgggggctcggcggcgttcgaaattggcgctctgcctgccccccaccccagccctcccccggagggggagggagcaaggccgatcagccttccagcgccttccacatctcgatgtcgcgctcggccgtccacacgcgcggatccgcatggcccgaggcttcgtcgtacgcgcggctcacgtcgaagggcatgcagtggtcgaagatcacccactggctgtacttgggcttgagcttcgcgtaggtgtccttgtagaccgtgttcaggtcgcggccggccttcacgccctcttgcacgctggcgtacacgtcggagatgaagtcgcgcgtgcccgtcaggccctcggccacttcggcgggcgtggtgagcgcggcgccgcggccgggcaccaacgcggcgggcttgagcgcggcgatgttgtccagcgtctgcggccagtcctggaagtaggcgtcgcccgcgtacggcgtggcgccgaattcgaccaggtcgcccgagagcagcgtgcgctcctcgggcagccacacgacggtgtcgcccttggtgtggccgcggcccagctggatcagttgcacctcgagcttgcccagccacagcgtcatcttgccggtgaaggtcatggtgggccaggtcaggcccggcggcacggtttcgacgttctggaacaggcgcggaaagcggccgatctcgctggccttgtctgcttcgccgcgctccacgatcaggtcgcgcgtgtcctggctggccaggatgtgttcggcaccgtagccggccgcgcccagcacccgcaccgcgtggtagtgcgtgagcaccacgtacttgatgggcttgtcggtcacttcgcggatgcggcgcaccacatcggccgccatggcgggcgtggcctgggtgtcggccaccagcacgcaatcgtcgccaatgacgatgccggtgttggggtcgccctcggcggtgtaggcccaggcgtgttccgagatctggctgaaggtgatcttcttttcttccatgtcagcctggctggcgaacttcttggcttggctcattggtgtgtctccgtcgggtggtgggatgaatttgaattcgtctaaagcaaatgaattcacggttaacgaatttccgaagtgtaagccccagatcggttaatgtctaatcccttcttcatgaacgaacaatcagacgccaaggcggccatgacagccagtgacaccgaccgcgccgcccagcgcggcatccagagcatcgaggtgggtggccagctgctgcgcgcgctggtgcaccacggccggccgatggcgctgaaagacctggcgcgggaagccgacatgacggccgccaaggctcatccctacatggtgagcttcgggcggctcggcctgatcgagcaggaccgcgccagcggccactatctgctcggcccgctggccttgcaactggggctcatcagcctgcagcaggccgacccggtgcacattgccacgccgctcattgccgaggtggcccagcgcatcggccacacggtggcgctggcggtctggggcgcgcgcggcgccaccatcgtgcgaacagccgaatcgccatcgccggtgcacgtgaacatgcggcacggcacggtgttctcactcaccaacacggcctcgggccgcatctttgccgcctatctcgctgccgacacggtcaggcagctgctcgatgccgagcgccagcggcagaagcagcgcaaggccggcgagcagccgccagaggccggcatgccgccgcagccgcccctgccctcgtggagcgagttcgagcgccaactcgaggaagtgcgggtgcacggcatcagccgctccgaaggcgaggtgatcgagggcgtgagcgccatggcggcgccggtgttcgaccacacgggcgccatcgtgctgtcggtcacggccatcggcccggccgccatcttcgacaccgcctgggacggcgaaatcgcacgcgcgctcaaggcctgcgcgggcacggtctccgggcggctgggggcaacgcctgccggaaaaaacggttccggaaaatcgggtccctgaccccgggctcgtcccgcgattcgggcgtcccgacccggatcagcggctcagcccttcttgccgcccagcagcaccagcgcgccgcccaccacgatggcggccacgctcgcccaggcggggaagttgacctgctgtttctccttcaccgagaactccagcgggcccagcttggcctggtgcgtttccttcgtgaagctgaagccgccgagcccgagccccgcgatgcctgcgacgacgagcaggatgccgatgatgcgtgttgcgttcatgtgggtctcctccggtgatgaaaattcgccttgccttgtgaaccgagcttacggccgcgcctgctggtccacccactgcacgacgtctgccacggccgcatcggtggccgcggccagcgccttgacgccgcctggcgcgtcggcgctcggcgccggacggcgcacggtgaaggtgcgctggcccaccacgcggtcgccgccgctgccgccgcggatcagcgtggcgcgcagccggaccaggccgacactgctgccggccgattcgaagtagtggctgaactcgtcgagcgagatgcgcagcgtgtcgggcaccttgccctcggcgcgcgcgagggttgcgctttcttccgggccgagcacggtgcgccgctcggcgagcgcatcgcgcagccgctggcgcagcagctgcgccggcggcaggctccagcgcgactggccgtaggggcgcagttcgttggcatcggcatagccgagccgataaagaatctgcgtgccgtcgagccgggtgttgctctcgatctcggccagcgcgagcgtgggcagtgcggccgcgggcggctgggcggcggtggccggcgcggcagcaccgggcccgaagtcgtacagcgtggcgcgcactggcttgtccggcagcgcgccgcagccggcaatcatcagcagcgccaggccggcggcggcaagcgccggagtgcgagtggcattgttcttcatggttgtcatcaccttcaggggcgtgccagggaattggtggccggcggcgccgagaagccaggctccccgggccccgcggcggtgccgccactgccgaacagcagcgattgcgggttgtcgttgatgccgtccgccgcgcggccgagccggcgcactgcgcgggaggtgtcgtcggccacgcggttcacgcgcggcagcgtggcggcattgaaggaatcgaccgcctgcgccagcgccttggtgccgtcgctcagccgctcgaccgggccgtccggcgcgttcaatcggccgacggtggtgttgaagttgttggccacgcgcgagacgtcgccggccgccttcttcaccgtggtcatcgtctctggaagcgctgccagcgcggggttcaacccggtcttcaccgtgttatcgagctgcttgatgagcgtgttggcgctggctgaggccgccgcgatgttttcgagcgcgtcggccgtccgcttctggttgtcgtctcccagcagggtgttggcgcgcctggtcacttcctcgacctggttgatgatcgattcgcctcggtcctgcagctgcgccagcatcgacggcttgagcggaatgcgcggcggatcgtcgttgttgggcttgagcgcgacgttcgattcgcccttgtcgtccagcgcgatgaaggccaggccggtcacgccctggtagctcagcgtggcaaagctcgaggtggtgagcggcacgcgctcgtcgacgctgatgcgcacgcgcacgttgcccttcaccttggggtcgaagtcgatcgacgccaccttgccgaccgcgatgccgcggtagcgcaccatggcctgcggctgcaggccgctgaccgcgtcgcgggtggagagttcgtagatgttgcgcacggtgttgtcgcgcgtgaaccagaccaccagccccacgagcacggcgatgaggccgagcacgaaggcaccggcggcaatggcatgggctttgttttccatgatgtggttacctttcagtggcccgcgccgacgggtggcggcggggctttggcgggtttgtcatgcagggcctccagggcacgctggccgcgccctcccagaaaatattcgtggatgaacggatgcggatacgtgatgacttcgcgtgccgatccgctggtgatcaccttgtggtcggccagcaccgcgatgcgggtgctcaggtcgaacagcgtgtccaggtcgtgcgtgaccatcaccaccgtcagccccagttcgcggtgcaggccgcgcagcaggtcgcagaagctgtcggaggattcggggtcgaggccggccgtgggttcgtcgagcagcagcagcggcggatccatgatgagcgcgcgcgccagcgccacgcgcttgatcatgccgcccgacaagtccgccgggctcatgttggcgtgccggggctccaggcccaccatctgcagcttgaccagcgctgcgttgcggatcagctcgtcgggcaaaagcttgagctcgcgcagcggaaaggcaatgttctcgagcacgctgaaggccgagaacagcgcgccatgctggaacagcatgcccacgttggccgcgcccttggcgctgagctcgccgggcgcccggcccagcacctcgaccgtgcccttcgatggcttttcgaggccgaggatctggcgcagcagcaccgtcttgccggtgcccgatccgccgaccagtgagagcacctcgccgcgctcgatgtgcaggtcgaggtcgcggtgcaccacgacctcgccgtcggcgttcttgaacaccgtccagagcttgcggatgtcgacaacgacagtggttgaggattcgctcattcgaatacctccgcgcttcgcactccggtgcgagcctccttcggagcggccgggcggcggctcatgcccggaaccccacgcccttgaacagcaccgcgaacagcgcgtcgaccaagatcaccgcggtgatcgaggtcacgaccgacgaggtggtgccgcgccccaggctttcggtgttgggcttcaccttcatgccgaagtagcagccgatcagcgcaatcagaatgccgaacaccgccgacttcgccagcgcgagccagaggttcgcgatcggcaccgcgcgcggcagcgccgacagaaagtacgaaggcgagatgtcgagtgcggcgtcggccgcgagcatgccgcccacgagcgccgccatcgaggtccagaggctgatcagcggcatggcgatggccagcgccatcacgcgcggcatcaccagcctgaagccgtgcggaatgcccatcacgcgcatggcgtccagctcttcggtcacgcgcatcaccccgatctgcgccgtgatggccgagcccgagcgcccggcgatcagcaccgccgcaagcaccggcccgagctcccggatcagcgacagcccgaggatgttgaccacgaaggcctcggcgccgtattggcgcagctgctgcgagatcaggtaggccagcaccacgccgatcaacaggcccaccagcgccgtgatgtgcagcgccgtggcgccgaactgatagagatgccccgaaaaatcccgccagggcgcgcggtgcggcgcgcgcacgagcgtgaaggtatccagcgcgagctggccgatcaacccgacgaaatcgcgcattacctccagcgcgcgcgggccggtgtgcgagaaatgccgcagccgctcggccagcgtgggcggcggctcgtcgggcgttcccacggtgtacagggccacctggtcgagcaccgccttgtgctgcggcgacatctcgagcgtggccggccagtcgtggtgccagtgctcccacagcagctgcgcgccgatgtggtcgagctgctcgatggggcgcaggtcccaggcgcggtcttcagccgggggcgcgtccgccaggtccttggtgagcgcctgccacgaggggcgcgacgacatggccagcgtggtccagcggccgctggccacggtccagcggcggccgtcctgctcgcgctcttcgacgcgcggcaacacgctgtcggcggctggtgcgtcggcagtcgaagttgctagggacatgatgcggcggtgcagggcgaagtaagaaaaagaggcggtctcgatgggcgcatcgtaaccggatgaatcggctttcttcgtgcattgcggctccggtttgcgtagggcggaacgccgtccgatggaacattcgcggcttttttgcggtcagtgccaggcccgtgccagcgcgttccatgcgctcgcgatcacgggctcgttgcgccgcgccgccagcgagacgaagcgcagcgcgcagtcgagctgaacgcggtcggccatcacgaggccgtgcgactggctctcgcggatggcgatcgagtcgcgcaagaggctcaggcccacgcccgacttcagcaggtcgagcatcgaggcttcctggtcgaccaacgccgcgcgtcgcggtgaaagcccgagcgggccgaacactttgtcgagcaaccgatggtgtgcggactcgggcggcgtggcgagccagggcagcgcggccagcgccttccagtcgcggcccagcacctgcgggccccagcccgcgggcgcgaccacgcggtaggtgaagcgcgtgagcgtgcgcgccgcgagcagcgctggcgcggcggcgtcgccttcgtccgtgtcgaggtgaaaccccacgtcgagctcgccgcgcagcacctgcgccagcaccgtgccgctcatgccgtggcgcagctcggtttcgatctgcggggccgattccaccagttcgcgcaagaacacgccgagacgggtgaactccggatcgaggatggtgccgatgcgcagcgccccgcgcaccgtgccctgcaggttgcgcgcggcctgctgcatgtctcccacggccgcgagcacgcgctcggcctgtggcagcaatgccgcgccgtcggccgtgagtgcgagcccgtgtggcgtgcgcgtgaagagttggagcccggtttcctcggccaggcgcttgagctgcaggctcaccgccggctgcgtgaggtgcagccgctcggccgcgcgcgacacgctgccttcgcgcgccgcgtgcacgaaggcgcgcaagatctggaggtccaagccggcggcagtcatataagaccaatttataagctacttgcgccgaaatcattggctttttaagcgtggcctggtgaaacttcggcctggggcgcctcatggcgccatgagtatcaaaaatatcgtcctcggagacaagcagccgccatgagcaacgacaacacattcgactacatcgtcatcggcggtggcacggcgggcgccctgatgtgcaaccggctgacccgcaaatcgcaacagcgcacgctgctgatcgaggccggccgcaaggacgactaccactggatccacattccggtgggctacctgtactgcatcggcaatccgcgcaccgactggctctacagcaccgagcccgacgcggggctcaatgggcgcacgctgcgctacccgcgcggaaagacgctgggcggctgctccagcatcaacggcatgatctacatgcgcggccagtcacgagactacgaccagtgggcgcagctcacgggcgacgacgcctggcgctgggaaaacgtgctgcccgatttcaagaagcacgaggactactaccttggcgccgacgagatgcacggtgccggcggcgaatggcgggtggagaagcagcggctgcgctgggacatcctcgaagcctttgccgaagccgctgtggaggccggcgtgccgcacagcaccgacttcaaccgcggcagcaacgaaggcgtcggctacttccaggtcaaccagaagaacggctggcgctggaacaccgccaaggccttcctgcggccggtctgctacggccggcccaacttcgagatgtgggtcaacgcgcatgtcaccaagctgatcatcgagacccagcccgacggcagccggcgctgcaccggcgtgcaggtgtgggacggccacgagatggtgacggcgcacgccacgcgcgaggtggtgctctgcgccggcagcatcggctcgccgcagatcctgcagctttcgggcattggcccggcagagttgctgcgccagcacggcatcgatgtggtgctcgatgcgcccggcgtcggcgccaacctgcaggaccacctgcagattcgcgcggtctacaagatcaacggcgcgcccacgctcaacgtgctggcttcgtccatgtacggcaaggcgaagatcgggctcgaatacctgatgaagcgcagcgggccgatgagcatggcgccctcgcaactcggcgccttcacgcgcagctcgcccgatcatgagtggcccaacctcgagtaccacgtgcagccgctgtcgctcgatgccttcggcgagccgctgcacagctttccggcctttaccgcgagcgtgtgcaacctcaaccccacgagccgcggcaccgtgcgcatcaagagcccgcgcttccaggatgcgcccgcgattgcgcccaactacctgagcaccgacgaagaccgcaaggtggcggccgattcgctgcgcgtgacacgccgcatcgcctcgcagcccgcgcttgccaagtacaagcccgaggaatggaagcccggcgtgcagtaccagagcgacgaagacctggcgcgcctggccggcgacatcgcgaccaccatcttccatccggtcggcactacccggatgggcgccgacggcgacccgatggcggtgctcgattcgaagctgcgtgtgcgcggggtgcagggcctgcgcgtggtcgacgcgggtgcgatgcccaccatcaccagcggcaacacgaacagcccgacgttgatgatggccgagaaggctgcggggtggattctggaagcgaatcgctgaggcgtttgttcggggctgttgctgtttcggggcgctgttgttcggggcgctgctgttcagggcgcgtgcaaaggccaccgggtactcccctccgcgaatgtcccccgccttcggctcctcctttatttcgctgcggggagcacccgatgccctgtgcactggggcacgctgccggtgttccgccgatcaacgaccgtcgcgcataacgctcacgtcgatggggtgccttgcgcagcgaaataaaggaggaggccgcaggccgggggacattcgcggagcaaggtaccccgtcggcgggagcgcgccccgaacgtccgaggccaatcacttctcgatcgtcttgttccaacgcgcattccaagcaggacggttcgcattgatgctgtcccagtcaatggtgaccgcggtcttcatccactggttgatgtcggccacctgcttcacgccatcgcccacggccggagccttggggttggtgggaatttgcgcgccgtactgcaacacattggcctgagccagcgggctcagcaggaactcggcgagcttctgcgacagctcgggctcgctgttgttcgcaatcacgcactggcccaccatcagcaccaccgcgccttccttcggcggcgcgtattccaccggtatgcccttggtcttcagcgcggccacggccgtaggcgtgagcgggaagatcgcggcttcgccggtctgcaccatttccgacagcttggccgaactcgggatgtactcgagcacgttcgggccaatgctggtgggccaggccttgaagccgggctccacgttcttgtcgttgccgccctggatgcggttgaacatcaggaagccatgcagcccgaacgacgatgaagacatcgactggaacaccaccttgcccttgtacttggggtcggccaggtccatccacgacgtgggcgcggcccagcccttttccttgaacatcttcgcgttgtaggccaggcccgtcatgcccaggctcacgccgctggccatgtcgtccttgaagcgcgcagccgggtagatttctgcgagcgacggattggaccgctgcttctggcacagacccatgccgatggcgcgcaccatgatgccgtcgtccaggaacatcacgtgcatctgcggccggtccttgttggcctgcgccttcgcgaggatgtcggacgaggtgcccggcaccaccaccaccttggcgccatggagcttctcgaaggctgggaacacgtactgcgtgtacgccttctccatggtgccgccgttcatgccgatgtagagcgtcttggtctgcgcgccggccgcgccgccggccgcgagcgcggcaaccgccgccgcaccgagcacggtccggcgaagagagaaaaaggtcttctggaaacggaacatggtgttttcctttcagggtggggtgggggtggttggttcttctgcaaagaagcgttcgatcgaaaaggcctggatcggcgtgctgctgcggccgtcgcgcaccagttcggccagcacttctccagccgcggggccgatctggaagcccgcgcccgaaaagccgaagccatggaacagcccgggcgtggtgcggctgggcccgagcaccggctcgcggtcgggcaggtagccttcggtgccgctccaggtgcggatgaagtgcgcgtggcgcagcgcgggcagcagctcgatggcctgtgccgcgagcgtggcgatggcgtcgctgccggcgcgggcgcggtcggcgtcgaccgcgatgcccgcgccgccgccgagcacgaggttgccgcgcgccacctgccggccgtagatgccgccgccctccacgccgaggctccagtccatgaaatgcggcatcggctcggtcaccaccatcacggggttgcccgagcgcagcggcacggtttcgtcgaatcgggtcgcgatcgggccggaccaggcgcccgcgcagttgagcagcacgggcgcgtgcacttcgagcgcattgcccgagcgcagcatgaacatcgcgccgtcgtgcgccacttcttcgaccgcgtggcgctcgaagacttgcgcgcccgcgtgctgcgccgcgagcgcgaaggccggcgacaccagccgcggattggcctgcccgtcttccacgcacagcgagccgccgacagcgcgcgcaccgagccacgggcagcgctcgcgcagtcgggcatcggagatcaattcgagcccgaggtcgaagtccaggctttgggagcggtagcgttcaagcgaggccatgtccgactcgctgcgcgcgatcttgaaatggcccgagcgcagatattcgccgtcggtgccgatcagcgaaggcaggccgccccagatttggtgcgcgcgttgcgcgagcggcaactggctcagcgggcgcccctggcgccgcacgccgccgaagttcacaccgctggagcgcgagccgcagaggtcgcgctccagcagcgccacgccgatgcccatctgccgcagcgcgagcgcggccgaagagccgacgatgccgccgccgacaatggccacgtcggtgcgcagggtcttgatcgaactcatgcgccagcgccttcagcggactcgcgcacggcgagctggatcggaatcggcttgatcggcgcctgcccgcgcagccgtccgacctgctgcaatggcagccccgtggcgtgcgcgaggatctcggccgcggccacgccgcacatgcggccctggcaacggcccatgccaacgcgcgacagggccttgaggcggttcatttcgtcggcgccgttgacggaaacggcctggcgcagcgtgccggccgtgatgttctcgcagcggcagaccaccagttcgtcgggcgcttgcgcggcccagtcgtgcggcaccgggaaggcgcgttccagcccctcgcgaaatccgccgagcttgtggagcttgcgttcgagcgtttcggcgcgcgcggggtcgacggcgacgccatggtcggccagcagcgcgagcgcggcgcgttcgccggcccattcggccgcatcggcacccatgatgccggcgccgtcgcccgcgaggtacacgccctgcacgctggaacggccggccgcatcgcgcaccggcaggtgggcgcggtgcagcggtgcaaattcgaagcggcagccgagcagatcggccagctgggtttcggagcgcagcgcatagccgaagccgacggcatcgcagggcagcgtgcgttcttcgcggccgtcgtgccacgccacgccggccacgcggctttcggcggcgtcgccgagcacgcgcaacggccgcacgccgccgtgcagcgccacgccatgcgcgcgcagccaggccacgtagtacacgccttttgcgaacaccgcgggttgacggagcatcgcgggcgtggcggccagctggtcggcgagccgcgccgtgtcgagcactgcggccaccttcgcgccggcctttgcgtactgataggccaccaggtaaagcaacgggccggtgcccatgaacaccacgcgctgcccgatggcgcagccctggaacttgagtgcgacctgcgcgccgcccagcgtgtagacgccgggcagtgtccagccgggcaccggcagcacgcggtcggtggcgccggtggcaacgatcagctggccgtagggcacgccggaggtgctgcgcgtcgggccgtgcagcacgtcgagccggccgccgtgcgcgttccacaccaggctgtcggggcggtagtcgatgcgatcccgcagcgcgtcgaaggccgcgtgcaccgcatcggcacggcgtgcctcgaacccgtagagtgcctgcgcgctgcgctgggccaggctcgcgggcgggcgccggtagatctggccgccggcgcgcgaagcttcgtcgatcaccgttggccgcacaccgtgggccaccagcgcctctgcggcgcgcacgcccgccgggcccgcgccgacgatcaccggccgcaatgcggaagaggaagccgtcatgcgccgctccttccggtgaccagcgccatgcccggcgcaatgaaggtggagcaggcgcgcaggcgctcgccttgctcggtggcgatccagcaatcctggcaggcgcccatcatgcagaagcccgcgcgcggtgcgccgctgaattcgttgcgccgcaactgggcggcctgcgtgagcacggccgtgagcaccgtgtcgcccgcgagcgcggaggcgggctcgccgtcgagcgtgaagagcaccgcggcgcggccggtctcggccacgcggtgcagcagcggttgatgaagaggcggaaggctcatctatcggcgccccaccagcacgcggtccagcccgtagacgcggtcgagcaccaccatcgcgatggccgtcaccgccaccatcagcgccgacaccgccgccatcagcggatcgatcgactccgtggcatacatgtacatgcgcaccggcagcgtcaccgtgctgggcgaggtgacgaagatcgacatcgtcacttcatcgaagctgttgatgaaggccagcagccagccgcccgtgacgcccggcaggatcatcggcagcgtgatgcgccggaacatcgtggcctggctcgcgcccagcgagagcgcggcctgctcggcgctgcggtcgaagcccacgagcgcggccaccacgaggcgcagcgtgtagggcgtgacgatcagcgcatgcgccatcaccagccagccgaagctgcccgtgccgcccaccagcgcaaagaggcgcagcagcgccacgcccagcaccaggtgcggaatgatcagcggcgagaggaacagtccgttgaggaagtcgcgccccgggaacgcgtagcgcgtgatcgccatgccggccggcaccgcgatcagcgtggcgatggtggccgaggccagcgcgagccacaggctgttccagaacgactgcatgaagtccgggtgcgcgaacaccgccttgaaccagcgcagcgagaagtgcgtggtcggaatggtcaatgtgttctcgggcgtgaacgcgacgatgcacaccaccacgagcggcgccagcatgaaggtgatgacgagcgcgttgaacgcgagggcgagggggccgttcttgctcatctgatcaccccagtgcctttttgtagcggccttcgacgaggcggttgtagctcagcatcacgacgagattcgctgccagcagaaccagcgcaacggcggcgccgaggggccagttgagttcgtgcaggtattcgtcgtaaacgacggtggcgaccatcttcaatcgacgcccgccgagcaaccccggaatcgcgaacgaactggcggccaggccgaacacgatcaggctgcccgagagaatgcccggcatcacctgcggcagcacgatgcgcctgagcgtggtgaagggcgaggccctgagcgacagcgccgcgttctccacgcccgcgtcgagcttctgcagcgaggtccagaccggaatcaccatgaagggcagcatcacgtgcaccagcgccacgatcaccgcgatctcggtgtagagcatcttcaccggcccgatgccgaccagccgcagcaggccgttcaccgcgccctcgggtccgagcagcatgctccaaccgaaggcgcgcaccaccaccgaaacgagcagcggcgccagcaccaccaagagcagcaccgagcgccacgggttgcgcatgcggctcagcacataggcctcgggcgcgccgaccagcacgcagatcagcgtgacgacgcccgagatccagaaggtgcgccagaagatgccgtggtagtacgagtcggtgaaaacctgcgcgtagtgctcgagcgtgaactcgccggctttcggcccggtggccgggtcgtagacgttgaacgacagcacggcggtgagcgcgagcggcaccagcagcagggccgcgaacagcagcagcgcggggcccgacagccaccacggcgtggccgccttgcgggtcgaaccgctcacgccgccaccgcctcgtcggccggcagcaggcgcgtgcaatgcgcgggccagtcgatgccggcgtcgctgccttcgtcgagcgcgtcgcggccgtcgttggggctcagcaccgtcaggtcgccggcgtgcgtgctcaggcgataaagccactggctgccgaggaagaagcgttcctgcaccgtgccgtcgagccggccgcggccggcctccaccagctgcagcttctcgggccgcacgctcatcagcacggccgcgcccgagctgtagccggtgtcgtccacctcgaccgcgagcgcgccgaccgcgacatggcagctgcgcgcgccgcaggccgtgacgcggccattcagcaggttggccttgcccacgaaggtggagatgaagcgcgtgctcgggtgctcgtacacgcggtgcggatggtcgatctgcgtggcgcagccgccttccatcaccaccacgcggtcgctgatggacatggcctcgctctggtcgtgcgtgaccatcaccgtggtggtgccgaccttgcgctggatctggcgcagctcgaactgcatctcttcgcgcagcttggcgtcgaggttggacagcggctcgtccagcagcagcaccggcggctcgatcaccagcgcgcgcgccagcgccacccgctggcgctgcccgcccgagagctcgcgcgggtagcgcgtggcgtgcgcttcgagatgaaccagcgccagcgcctgcttcacccgctcgatgcgttcggacttcggcatcttgcgcatctctaggccgaagctcacgttgtcggccacggtcatgtgcggaaagagggcgtaggtctggaacacgatgcccaggccgcgcgtgttggccttggcatgcgtgatgtccttgcccgccagctcgatgcgcccgctggagaccgcctcgaagcccgcgatcatctgcagcgtcgtggtcttgccgcagcccgaagggccgagcagcgagacgaactcgcccttctccaccgtgaggttcatggccgacacggcgcgcgtggcgccgtagaacttggtcacgtcggtgagccgtaggaatgacatggaagggcctttctgcgcggtcgtggatggcgtgcagcaccttggtgcacgccatggacaagagagaactttcaattcactctattgcaacgatcacgccagttcgcctcgggtattccattaatcagaatctttttcatatttattccgatgaatggaatatcatgaaaggaatagatctcaagaattccacaggagcaaggtatggaaaccccctcggcggccagcggcggcgtgccgcgtgtcttttcggtgatccgcgcgctcggtgcagtgcaggccgaaggcggccgcgtgacccagatcgcacgttctgtgggccttacccaggccaccacgcaccggctgctgcagtcgctcatggccgagggcatggtcgaacaggacgagcgcagcaagctctatcgcctgagcatcgatttcttcgcgctcgcggccagcgccggcaaccccggcgacctgcgctctatttgccgccccgtgctgctgcgcctgtgcgcgagcctgggcgacagcatctttctcttggcgcgcagcggcttcgacgcgatctgcctcgaccgcagcgaagggccgttccccatccgctcgttcaccggagacatcggtgggcgcattgcgctgggcgtggggcagggcgcgctcgcgatcctggcctttctgcccgaggccgagcgcgaggaagtgattcgcttcaacctctcgcgcgtgcgggagtacggcgtgtacgacgaggtttacctgcgcaccgagatcgagcgcgtgcgccaggccggctacgcggggcgcaacaccggcctgctcgaaggcatggccggcgtggcggtgcccgtcctcgaccgcgagggccgtgccgtggccgcgctgagcgtgggcaccatcgccgaccggctcaatgccgaccgcatgcccacggtggtggagctgctcaagcgcgaggcggcggccatcgggccgaagatcaatcccttcgacgcgaccttgcggcggccggcgcagagcctcgcgggttcgccggcagggcagcgcatcagcttgcccgaggcgccggggccctcggcctgagcctgtgttggtgcgctgcgagcatgaagggctgctgaggtccttcatgaaacgcaccaagtccttccgttttttcgctatgcaagcgcgcgggattcgcagatattgacctgttgccgcgtcccgtctcccttcgttctgttctttcttctccacccggagcgcccatgccagaagccaaatcctccctttccgtcgccgccgaaatcgagcagctgctgcagcgcctcggcgttcccggttccgcctgcaccggcggcgaactgacggtgcgctcgccggtcaccggcgaggtgattgcacaggtgccgcagaccagcgccgccgaagcggccgcggccatcggccaggcgcacgaggccttcaaggcgtggcgcaacgtgccggcgccgcgccgcggcgagctggtgcgcctgctgggcgaagagctgcgcgccgccaagggcgacctcggccggctcgtcacgctggaggccggcaagatcccgtccgaaggcgcgggcgaggtgcaggaaatgatcgacatctgcgacttcgcggtcggcctctcgcgccagctctacggcctcacgctcgccaccgagcgcgccgagcaccgcatgatggaaacttggcatccgctgggcgtgtgcggcgtgatctcggccttcaactttccggtggccgtgtggtcgtggaatgcggcgctggcgctggtgtgcggcgattcggtggtgtggaagccgtctgaaaagacgccgctcaccgcgctggccacgcacgccattgcgcagcgtgccatcgcgcgtttcggcgatgcgcccgaaggcctgctcggcctgttgctgggccagcgcgacatcggcgaggtgctggtcgacgaccaccgcgtgcccattctttcggccaccggttccaccgcgatgggccgccaggtggggccgaagctggccgcgcgctttgcccgcgccattctcgaactgggcggcaacaacgcggccatcgtcacgccttcggccgacctggacctcacgctgcgcgccatcgcgttctcggccatgggcacggccggccagcgctgcaccacgctgcgcaggctcttcgtgcacgacagcgtgtacgacgcgctggtgcccaagctcgccaaggtgtacggcaacgttcaggtgggcgatccgcgcgaggccggcacgttggtggggccgctgatcgaccgcgccgccttcgacggcatgcagaaggccttgggcgaatgccgcgagatcggcgccacggtgcatggcggccagcgggtcgacggcatcggcacgaaagacgcctattacgtgcgcccggcgctggtggaactgaagtcgcatgacggcccggtgctgcgcgagaccttcgcgcccattctctacgtggtgcgctacagcgcgctcgacgacgccatcgaatggcacaacgcggtgggcgcgggcctgtcgtcgtcgatcttcacgctcaacgtgcgcgaggccgagcgtttcctgtcgagcgccggctccgactgcggcattgccaacgtcaacatcggaccgagtggcgctgagatcggcggtgccttcggcggcgagaaggaaaccggcggtggccgcgaagccggctccgacagctggaaggcgtacatgcgccgcgcgaccaacaccatcaactactcgaccgcgttgccgctcgcgcaaggcgtgaccttcgagatcaacgactgatcgactccggccttctgttcttgccgcgcggcgtttcgccgcagcggcaagacagcggccgtgcgtgccccggaaaaacaaccaaggagacagagaagatgaagatgcaattgaagaccctcgccatcgccgcagcgctgctcgcgctcgcattcggcgcttcggcgcagcaggcccccaccggcggcacgctcgacaagatcaagagcagcggcaaggccgtgctcggcgtgcgcgaggcctcgccgcccatggcctacatgctgggcgcgaacgacaaatacgtgggctaccacgtcgagctctgcgagcgcgtgctgaaggacatcgcgccctctgcccggctcgaatacatggccgtgacggcgcagaacaccatcccgctggtgcagaacggcacgctcgacatcggctgcggccccaccaccaacaacaccgcgcgccagcagcaggttgcgtttgcgctcaccacctatgtgagcgaggtgcgcatggccacgcgcgtcgattcgggcatcagctcgctcgaccaattggcgggccgcaccgtgtcggcgtccaccggcaccactgccgtgcagctgctgcgcaagcgcgagcgcgcgcagaacaccaccatcaccacgatgctcggcaaggaccacctcgagagcttcctgctgatggagtcgggccgcgccgatgcctttgtgctcgacgacaacctgctcgccggcatcatcgccaacgcgaagaacccggccgcctaccgcatcgtcggcgatgcgctgggctccgagcccatcgcgctgttgttccgcaaggacgacccggccttcaagaccgcggtggacgatgcgctgcgccgtctcatgaagagcggcgagctcgagaagatctacaccaagtggttcgtcgcgcccattccgccgaagaacaccagcctcaacctgccgatgagcacggccttgaagcagctcatcgccgagcccaacgacaagccgctggaggcctacgcgaagtgacatccgccgttctcgattccgcgctttcttcgtcctccgcgttcgagcccgcacagcgtgtgcgcgccatcggcgtgtcggaaatcctgcgcatcaccgaccatgccaacgcactcaagcgcgccggccggccggtgatcgtgctgggcgcgggcgagccggacgtcgacacgcccgagcacattcgcgcggctgcggcccgcgcgatggagcgcggcgacacgcgctacaccgtgctcgacggcagcccggccatgaaggccgcggtgcagctcaagttcaagcgcgacaacgcgctggactttgcgttgaatgaaatcagcgtgggcgcgggcgccaagcaggtgatcttcaacgcgctgatggccagcctgaatccgggcgacgaggtgatcctgcccgcgccttactggacctcttacgcggacatcgtgcagatctgcggcggcgtgccggtgagcgtgccttgcagcgcagagcacggcttccggctggaggcagcgcagctcgaggcggccatcacgccgcgcacgcgctggctctttctgaactcgccgtcgaacccgagcggcgcagcctacagcgcggcgcagctcgcgccgctgtgcgaagtgctgctgcggcatcccaaggtgtgggtactggccgacgacatctacgaacacatcctctacgacggcctggctttcgccacgccggtggccgtggagccgcggctgcgggaacgcacgcttaccgtcaacggtgtttcgaaggcctatgcgatgaccggctggcgcctgggctacggtgccgggccgcgcgcgctgatcgcggccatggcggtggtgcagagccagtcgacctcgtgcccgtcgtcggtgagccaggccgccgcgatcgaggcgctgaccggtcctcaggacatcgtggccgagcggtgcgccgatttccaggcgcggcgcgatttcgtggtggccgcgttgaaccgagcgccggggctgcattgccgcgtgcccgaaggcgccttctatacctttgcgagctgcgccggcgtccttggtcggcgcacccgcggcggcgtgctgctgcagaccgacagcgacttctgcaactacctgctgcaggatttcgaagtggcggtggtgccgggcagcgtgttcgggctggcgccgtatttccgcatttcgtatgccacgtcgatggcgcagctcgaggaggcgtgtgcacgcattgccgcggcatgcgaagctctcacatgaatttctccctccccttccgggggagggcaggggtgggggcaggcggcgtgtctgtcaccgtcggcgtggttgacgccgtctgcccccatcccaaccttcccccagagggggaaggagcgaataccaagaccttcattgcattggacacagcatgacttcttcccgcaccggcggccagatcctggtcgaccagctcatcacccacggcgtcgagcagctcttctgcgtgcccggtgaaagtttcctggccgtgctcgacgcgctgcacgacgcatccatcgacgtgacggtgtgccgccaggaaggcggcgccacgatgatggccgaggcgcagggcaagctcacgggcaagccgggcgtgtgcttcgtcacgcgcggtccgggcgccaccaatgcggcggccggcgtgcacatcgcgcaccaggattcgacgccgctgctgctcttcgtgggccaggtcgcgcgcgaggcgctgggccgcgaagccttccaggagctggactacggtgcggtgttcggcaccatggccaagtgggtggtgcagatcgacgatcccgcgcgggtgcccgagctggtctcgcgcgccttccatgtcgccacgtcgggccggccggggccggtggtgatcgcgctgcccgaagacatgctgaccgaagccgccacggtggccgatgcgcagccctacgcggtggttgaaacccatcccggtgcggtgcagatcgccgagttgcaacagcgcttgtcagaggcgcagcggcccgtggtcatcctgggcggcagccgctggtccgaagccgcggccctgcagttcgccggtttcgccgaggctttctcgctgccggtgtactgctcgttccgccgccagatgctgctgtcggccgatcatccctgctacgcgggcgacctgggcctgggcgcgaatccgcgcatgctcgagcgcatccgcaatgccgacctggtgctgctggtgggcgggcgcctgtccgaagtgccgtcgcaaggttatgagctgctcgcgattccgcagcccaggcaggccctggtgcatgtgcacgccgatgccgacgagctcggcaagctctaccgcccggcgctgggcatccatgccacgccgcaggctttcgccgaagccgtgtccgcgctgcgcccggcttcagcgcccgtgtggcaggccgagacccaggccgcacgcgaagacttcctgcgctggagcgatccggcgcccatccgcattccgggcccgctgcagatgggtgaagtgatgcagcacctgcgcgaagtgctgccggccgacaccatcttctgcaacggcgcgggcaacttcgcgacctgggtgcaccgcttctggccgtttcgcgcgtttgcgagccagctggcgcccaccagcggatcgatgggctatggcctgccggcgggcgtgggcgccaagcggctgtggccgcagcgcgaggtggtggtgttcgcgggcgacggcgacttcatgatgcatggacaggagttcgccaccgccgtgcagtacgggcttccgatcatcgtggtgctgctcgacaacgccatgtacggcaccatccgcatgcaccaggaaaagcactatcccggccgcgtgagcgccacgcagctcaagaaccccgacttccgtggctacgccgaggtgttcggcggccatggcgagcgcgtggccagcaccgaggagttcggccccgcgctggcgcgggcgcgtgcgagcggcaagcccgcgatcctgcattgcctgctcgacccggaagccatcacgccggtcagcacgctgcagtcgatccgcaaggccgctctcgctgccggctgaaagaggaagaaggaatcagcccagtccgcccgcgtagcgcggcagcgggttcggcggattgccgtcgggcgcacgtgccgccagccgtgcggcgcgcgccaatggctccatggcctgctcgaggcgggtggcgagcagatagagatcctcgtccttggtctcggcggcatgtgcgcgcgtcatgcgcacgatctccgcggcgtactcggcgttggtggccatccattcggtgtcggtcacgcgtccatgctttcgccgcagcgcgacatgaaggcgcgcggcgagggcaatgcgatcgctttcggacatggacatggggcggtcctccaggaatggctcgtccgtttgcgtgcacaagtcgtgccacatcgtgggacgcacctcattaacgcgtggaaacacttttgtatgggaagaggcctgcggaggtaaggaaaagcgggttattcccaatgcactgagccggtgcaccccctaaagtctgcccactcgcgaacgggccaagctcgtactgccgagggtccgaggagacaaattcggtctacaacaaaaattcttcaaggcttccgttcgagaagccgtgcttgaacttgaaaggcgccgctggtcggcgccttttttatgcccgccgcatggcgccggccctggcgtttctctctggccaaagagagcgcctgcgcccgtcacacctttggatgaagctccctttttgatagcgctacgggtgcgacaatccagccatggaaatgctggtggtaacgggcgcctcgctgctcgcgggctttgtcgattcgatcgtaggcggtggcggactgatcctcgtgccggcgctttttgcggtcttcccgggcgcgccgccagccacgttgctgggcaccaacaaaagtgcttcgatttggggcacggcggccgcggcggcccaattcagccagcgggtccagatgcgctggggcgccctgtggccggctgcggtgctcggtttcgcgggatccatgctgggcgcctggggcgtgacggtgttccctggcgatttcttgcgccgggcgctgcccatcgtgctcgtcggagtgctgatctacacggtggtgcgcaaggacctggggcgcaatcatgtcccgcgtttcagcggccgagccgaaacgctggcggcctgcgccatcgggctgtcgatcggcttctatgacgggttcttcggccccggcgcgggcagctttctcgtcttcctgttcgtgcgctggatgggttatgacttcctgaacgcgtcggcctcggccaaggtcatcaacacgctcaccaatgccgcggccctgctgctgctggcgctcaaggggcatgtctggtggcactatgggctggtgatggcggtggccaacgtggccggcagcttgctgggtacgcgtgttgccctgaagcacggggcaggcttcgtgcgggtggtgttcatcgtcgtcgtgagcgcgctgatcttgaagaccgcctacgacgcattcctgaaatagcgaaaaaaaacgagaaagcctcatttcatggcattgccagagcccgccgtcgaaccacccgctcccgtcagcttctggcaggccttcggctactggctcaagctcggcttcatcagcttcggcggcccggccggacagattgcgttgatgcaccaggagctggtcgagcgccgacgctggatctcggagaagcgctttctgcatgcgctcaactactgcatgctgctgcccggccccgaagcccagcagctggcgacctacatcggctggctcatgcaccgcacctggggcggtattgcggcgggcgtgctcttcgtgctgccctcgctcttcatcctgattgcgctgtcgtgggcctacatggcctacggcaacgtgccggccgtggcgggcctgctctacggtgtgaagccagcggtgacggccatcgtgctgttcgccgcctggcgcatcggctcgcgggtgctcaagaacgcatggctctgggcgattgcggtggccgccttcgtggcgatctttgcgctacgcctgccatttccgctgatcgtgcttgccgccggagccgtcggctacttcggcagccggttcgcgccggcgtactttgcaccgggcggcggacacggagccgccgcggcatcgtccggcccggcgctgatcgatgacgacaccccgacgccgccgcacgcgcttttcggctggggccgattcgcgcgcgtgctggcggtgtttctcttgctgtggcttggcgccctgggcgcgctcacggcgctgtacggatggagcggcgcactcacgcagatggcctggttcttcaccaaggcggcactgctgaccttcggcggcgcctatgcggtgctgccctacgtgttccagggggcggtcgaccactaccactggctcagcgccacgcagatgatcgacggactggcgctcggagaaaccacgcccggcccattgatcatggtggtgtcgttcgtgggtttcgtcggtggctgggggcaggcgctgttcggcccgcatgcgctgttcgcggccggcgcggcagcggcggcggtggtgaccttcttcaccttcctgccgtcgttcctgttcattttgctgggcggccctttcatcgagtcgacccacggcaacctgaagttcaccgccccgctgaccgccatcaccgcggccgtggtcggcgtgatcgtcaacctggcggtcttcttcgcctaccacgtgctctggcccgcgggcttgtcaggccccttcgagattccctccgcggtcatcggcgtcattgcggccatcgcgcttttccgcttcaaggccggtgtgatcccggtggtgctcgcctccgcattggccggcatggcctggcaactgctcatgcgctgacgctcgcggagcctatcccttgacgaaaggcttctcttcgcgcccggctcgacgagcagccacgccgccaagcagcagcaccgctgcggaccggcggaaacgaaaaaagctcccgaaggagctttttttttcattcagagagccggggctctcttgatgagtgcgggaaagcgcgtgagggcttagtagccgccgcggccaccgccgccgccgccgtagccgccgccaccaccgctgcggccaccgccgccgccgccgccaccgtagccgccgccgccaccaccgccgtaaccaccaccaccgccgccgccgccgtagccgccgccaccaccggtacgggggggacgagcttccatcggacgtgcttcgttcacggtcagggcgcggccctggagcgaatggccgttcatggcttcaacggcagccagcgcttcagcgtcggtgcccatttccacgaaaccgaagcccttggagcggccggtgtcgcgttccatcatgaccttggcgctgacgatcgagccgaactcgccgaaagcctgttccaggtcgttatcacgcacggagtaggcgaggttgcctacgtagagtttcttgcccattgagggactcctaattcaaaccaacaatacaaagcgatggagtcccagaatcacaacaaacaaatgcgctgtggcgcgaaactgaccgatcaccgaattacgtgcacgggagcatgctcacagacacgtaggccggattatcaagccgaactggaaaaagcgtggcgaaatccgctgttattacgaaacatcacgtcctgacgggcggtttcgcaacggttggagcaggccggaaagcccgttgtggtctatttcatgcatcaaatggagcagccggccgatctcgcccgagggaaaaccctcgcgcgcaaaccaattcagataatttccgggcaaatcggcaatcaatgtgcccttgtgtttgccaaagggcatttcgagcgtgacgagacgctgcaggtcttcgggtttcatacgcttcagcctcccgcacgcttgaccgtgtggccctgcttcacaagggcggcgatcaccagttcacggtgatcgccctggatctcgatggtgccgtccttcacggtgccgcccgagccgcaggccgtcttgagctgcttgcccacggccgcgagcgcggccgcatcgagcgcgaggcccttgaccacggtcacgcccttgcctttgcggcccttggtctcgtgcgatacacgcacaatgccatcggtggccggaatgcgcgccttgttttccttgcagcggcactgcgccatcggcgcgcggcaatcggggcacatgcggccgcccgcctcggtggagtacaccagggcgctggcctgattgcttttcatcgttgccattcgatcgctctcttcttcaaatctgcttcacggcttccggtttcatctctctctgcctctccacatgccattcgactcactgggcctggcccccgcgctcgtgcaggccgccgccgaaagcggctatgccgcgccgaccgccatccaggctgcggccattcccgccattctgcaaggccgcgacgtccggggttcggcgcagaccggttccggcaagaccgccgcattttccctcccgctgctgcagcgcctggccgccgaacctgcgcaaacgccgcgtcgcgtgcgcgcgctggtgctcgtgcccacgcgcgaactcgcggcccaggtcggcgagacgatgcgcagcctggcgcagcacctgcccgagcggctcaagatcgccattgccttcggcggcgtgtcgatcaacccgcagatgatgagcctgcgcggcggcgccgacatcgtggtggccacgccgggccgcctgctcgacctggtggaccacaacgcgctgaagctcaacgccgtgtccgtgctcgtgctcgacgaggccgaccgcctgttcgacctcggctttgccgaggaactgggccgcatcctcgcgctgctgccgccgcggcgccagaacctgctgttctccgccaccttcccgcccgccatccaggcgctggccgacggcacgctgaaggaaccggcggtgatcgacgtgcagggcgagcccggcaccgagcccgccatcgtgcagcgcgtgatcgaggtcgacgccaaccgacgcacgcagctgctgcgccacctgctgaaagaaaacgagtggggccgcgtgctggtcttcgtcgccacgcagcatgcggcgcagaccgtggccgagaagctctacaagaacggcgtctacgccgtgcccttccacggcgacatcgcgcagggcacgcgcaccggcatcctcgcgcagttcaaggagagccggtgggacgtggtgattgccaccgacctggccgcacgcggcatcgacattgcgcagctcccggtggtgatcaactacgacctgccgcgttcgcccaccgactacatccaccgcatcggccgcactggccgcgctggcgagagcgggctggccatcagcttcgtgagcgcggccaccgaggcgcacttccgcctgatcgaaaagcgccagggcctgagtcttccgcgcgagcgcatcgaaggcttcgagccgaccgaggccgccgtgccgatggtcgatgcctcgggcactggcggcatcaagggcacgcggccgagcaagaaggacaagctgcgcgcggcgaacgcactggccgcgggccggccaggcgaaagcgagcagaacgactgaccccaggactagagccagcccagctgccgggcggccagctccttcatgatctcctcggcgccaccgccgatcatcatgaccttcacttcgcggtagatgcgctcgctcaccgtgccgcgcatgaagcccatgccgccgaggatctgcacggcctggtcggcgcagaactgcatggtctgcgtggcgtggttcttgagcatgcagacctttgcgacccactcgggcgcgttgaaacggcccgccgcctcgagtgcatcgccttcggccgacaccgcttcgagccaggcctcggtcgaggcgatgcgcatctgcatgtccaccagcttgtggcgcaccgcctggtgctcgatgagcgcagcgccgaaggtcttgcgctcgcgcgaccacgccagcgcctcgtcgaggcaggcctctgcgaagccgagcgcgccggccgcgaggccgatgcgctcgccgttgaagttgcccatgaccatgcgaaaacccgcgccttcttcgccgagcaggtagcgcgcgggcacgcgcacgttgtcgaaatgcagctgcgcggtgtcggagcaccaccagcccatcttcgcgaggcgcgtgcgcgtgaggccggccgcatcgccgggcaccagcagcatcgagatgccgcccgtaccgcgcccttcgccggtgcgcacggccaccgtgatccagtcggcgcgcatgcccgaggtgatgaaggtcttttcgccattcaccaagtagtgttctccgtcgcgtcttgccgtggtgcgcagcgccgccacgtcggagccgccgccgggctcggtgatggcaagcgccgagatcttctcgccgcgcagcacggccggcacgacctcggcgcgcacggcgtcgctcgcatgcagcaccaccggcggcaggccgatgttgtgcgagaacaggctcgcgagcacgccgccgcttttgccgtgccgcgcgagagcgatccacgccgggagcttgagcgcatacgaagctggcgtaccgccgaacgcttcgggatagccgagaccgagcagcccgagttccgcggcgcgcgcatagagcgcgcgcggaaattcgcccgcgtcgtcccaggcttcgacattcggcgcgatctcgttttcggcaaagcgccgcaccgtgtcggcgagcgccgcgcggtcggcttgcagttcggcgtccatcgcgcttcagccgcgcggcggccgcttggcgatgcccatggtcttcgcgaggatgccgagcatcacctcgtccgcaccgccgccgatggagcccagccggccgtcgcggtacaggcgcgagacgcggttctcgagcgtgaagcccatgccgccccagaactgcaggcaggtgtcggccacctggcgcgtgagccggccggtcttcagcttggccatcgacgccagctcgagcacgtcctcgccttgcacgtgcaggtcgcaggcgcggtaggtgagggcgcgcagcgcctccacttcggtcttgagctcggccagcttgaactgcacccactgctggtcggccagcgtggccccgaacatcttgcgctcctgcgcccatgcgatggtctgggcgatgcagtcctccatcggttcgagcgaactcgcggcggcccacaggcgctcttcctggaactgctgcatctggtagacgaagccctggccttcttcgccgatgcgatagcgctgcggcacgcgaacgttgtcgaagtagatgagccccgtgtcgctcgaatgcatgccgatcttgcggatcttcttcgccttctcgatgccggggctgtccatgggcaccatcacgagcgacttgttgcgatgcaccggtccgtcgccggtgttgaccagcatgcacatccagtcggcctgcaggctgttggtgatccacatcttctggccgctgatgaggtagtcgccgccgtccttgcgcgcatggctcttcaggcccgccacgtcgctgcccgcgccgggctcgctcacgccgatgcagccgaccgtgtcgcccgcgatggcgggcgccaggaactcgcgccgtagttcgtcgctgccgaagcgcgcgagtgcgggcgtgcacatgtcggtctgcacgccgatcgccatcggcacgccgccgcagctcacgtggcccagcgcctcggccatggccatcgcatacgaatagtccagccctgcgccgccgaattcctcgggcttgttgaggcccagcatgcccaggttgccgagcttcctgaagacctcgtgcgcgggaaagatctcggcctcttcccattcgtcgacgtgcggattgatctcgtcgtcgatgaagcggcgcagcgtcttctggatctcgagatgttcgtgggtgtactgcatgcggttgtctccaatcaatcgctcggtgattcgccgccgtcctggaacacgcgcggcgtctcggccaggtgaaagccgtcgaaaggacgcaccgccgcgcgctgccgcgcctgtgcgtcgggcagcgccatcggccagcccatgcgcacctgcggccgtgcgccgtccacgcgcagcacgctgccgctgatgaagctcgccgccgggctcagcaggaaggcgatggcggccgaggtctcggcctcgttgccgaagcggcccgcgggcacggtgttgcgcatcgcgcgcagcatgtcgccggcctcgggcgggtagtggtccatgccgctcgacgcgatgtagcccggcgccacggcgttcacgcgcacgccgctcgcggcccattcgagcgcggccgtttcggtgaagctcaccatgcccgcgcgcgcggcgccgctgtggcccatgttgggcatggagccccacatgtcggccacgatgttgacgatggcaccgccgtgcgcctgcatgctttgcacgaagcattcgcgcgcgacgaggaagccgcccgtgaggttggtgtggatcaccgcctcccagcccttggccgaaatggccgcgagcggcgtgatgtactggccgcccgcgttgttgacgagcccgtcgatgcggccatgcgtcgcaacgatgtcggcgaccgccgtgcgcaccgcctcttcctgccggatgtcgaaggcctggatgcctgccttgccacctgcctcggcgatctcggcctgcacctgctgcagcttttcggccttgcggccgaccagcaccacctctgcacccagcgatgcgagttcgtgtgccgtgcagcggccgatgcccgagccgccgccggtgacgacgatcacctgcccggcgaacagcccgggcgcgaacacggaacggtagcgggaagatgcattcattcgaaaggcttccggaaaaactggacaagcgcagtgtgcgccgtcatgcgtccgcaatctccgccaccacatggcgcgcggccacctgcgcgcccagcgccacgtgcagcgcggcaacgcggccggcgcgcggcgcgcaatgcacatgttccatcttcatcgcttcgagcgtgacgagcggctggccggcggcgacggcatcaccctcggccaccagcagcgcgatgacgcggccgttcatcgaggcgcgcagcaggccgtcgccggccgcggcatcggcgcggggcacggcgacatgcgtgaggtcctgcagttcgaaggcctggccgcgaaagtggaaccacaagcgatcggcggatgcgcgcactgccatagcctgctccgagacgccgccgcacgaaaagcgcacgctgccatcgccgggcagcgacagcaactcgatccgggccggcggcgctgcatcgagcgcgacatcgaaacggcccgaaccccgcggcgtcacccgcaccgcgtgcaccttgccgttgagcgaaaaacgcagggcgttgggcagcgtgtgcgcaatcggcgaaggccatccgcgctcgcccagctgaagcagcagcgcggccagccatacggcgcggtcttccgtggcggcatcaggcgcgagcaatgcatcggcgtgctcggcaatgaacgccgtcgtcgccttgccgtcggcaaacacagggtgcgacagggcgcgctgcaagagttgctggttggttgcgatgcccaatgccaccgtgtcctgcagccctgcgatcagccgccgtctcgcttcgtcgcgcgtgcggccgtgcgccacgagcttggcgatcatcgagtcgtagaaaggcggcaccgccgcgccatcacgcagcgcgtgctcgacgcgcagggccggcgaaggccgccatgcggcgagcgtgccgctttgcggcatgaagccctgctgcgggtcttcggcgcagagccgcacctcgatcgcatggccgctcatgcgcacgccgtcctgatcaaggggcagcggctcgccggccgcaacgcgcagctggagctcgaccaggtcgagccccgtcaccgcttcggtcaccgggtgttccacctgcagcctcgtgttcatttccatgaaccagtactggccctcggcgtcgagcaggaactcgagcgtgcccgcgccttcgtagccgatggccttggccgccgccacggccgtcgcacccatgcgttcgcgcaaggcagcggacacggccggcgagggcgattcctcgatcaccttctgatgccgccgctgcaccgagcagtcgcgctcgccgaaatggatggcgtggccgtgccggtcggcaaacacctggatctcgatatgccgcggtgcaacgattgcgcgctccaggatcacggttgcgtcgccgaaagcatggagtgcttcggactgcgcgctttgcagcagttcggcaaacgccgcagccgaaggcacgaaccgcatgccgcgtccgccgccccccgccgtcgccttgatcatcaccggccagccgatgcgtgccgcctccgcggcgagcgtggcggtgcgctggtcctcgccttgatagcccggaatgcacggcacgccggccgcctgcatcaggcgcttggcaccggccttgtcgcccatggcgcgaatggccgcgggcgaggggccgatgaagaccagccccgcatccaggcaggcctgcgcgaactccgcgttctcggccaggaagccgtagcccgggtgcaccgccttggcgccgctggcgtgcgcggcctcgatgatggcggcgatgttcaggtagctttgcgcgggcagcggctcgccgatgcacacggcctggtcggcttgccgcacatgctcggcttctgcgtccgcgctcgaatacacggccaccgtgtgatagcccatggcacgcgccgtgcgcatcacgcgcaccgcgatttcgccgcggttggcgatgaggatcttgttgaagctcatggccgcgccaccgaaaactgcattgcctgcggcacgcgcgcatcggcgtcgcggcagacagcaagcacttccgccagcaccgcgcgtgtgtcgcgcgggtcgatcacgccgtcgtcgagcagcagcgcgctggtggtgaacacgctggtctggcgctcgaagcgctcgacgatctgccgctgcatggcatcgatcttcgcgcggtcgaccgttcccttgcgagacattccggcttccatcacgatggccatggtctgtgcagcctgctcgccgcccatcaccgcggtgcgcgcgttgggccacgaaaagcagaagcgcggcgcaaagccgcggccgcacatgccgtagttgcctgcgccgtaagaggcgccgcaatgcagcgtgacctgcggcacggtggcgctggtcacggcctggatcatcttggcgccgtgcttgatgatgccggcctcttcatgcgcgcggcccaccatgtagccggtgatgttctgcaggtagacgatgggcgtgcgcgactggcagcaggcctggatgaagtgcgtggccttggtcgcaccatcggagtcgatgggcccgttgttggtgacgatgcccacggcgtggccttcgagccgcatgtgcccgcacaccgtggcgctgccatagtgcgcgctgaattcgaggaactcggagccgtcggcaatgcgcgcgatgacctcgcgcatgtccaccggccgccgtccatcgcccggcatgatgccgagcagttcttcggcctcgtacagcggcggcgcaaagcggcgcggcgcctcgtcgcgcgcccagtcgatgccgccgagaatcgagcgcgcgatgcggatcgcgtcgcggtcgtcctcggccaggtagtcgccaaggccggagacgtgggtatgcatcacggcgccgcccagctcttcctcggtcgcgatctcgccggtggcagccttgagcagcggcggccccgccaggaaggcgcgggtgcgatcccgcaccatcacgatgtagtctgaaagccccgtctggtaagcgccgcccgcggtggacgagccgtgcgtcaccgtcaccaccggcagccccgcggcggagagccgcgccaggttgcggaagatgccgccaccgcgcacgaagtcctgcacgcggtattgcatgagattggcacccgcgctttccaccagctggacatacggcagcttgttttcgagcgcgatctcctgcacgcgcaattgcttgtccaggcccatgggctgcagcgcgcccgcgtcgatgcccgagtcggacgcgctgaccatgcagcgcacgcccgagacccggccgatgcccgcgatcacgccgccaccgggcacgctcttgccgaggtcttcgttgtcgtggcccagccccgcgagcgaggccagcggcagaaagggcgcgccggtgtcgagcagcagcgcgagccgttcgcgcggcagcagctggccacgcctggcaaagcgctcggccgaggcattcgaggccgccaccgagcgggcctcgtgcgaccgcacctgcccgagcagcgcgagcatgccggcgcggtgggcctggaaggattcgctggccgtgtgcagccgggattcgatggcgggcatggaggagtcagtgcagaacgctttcgctctgcaccgactctagggcgccgatgcgcgcccggcttgcgccaattagctggtgcgggcccgctgcggcgcagcgggtgcgtccaggctggagcccgtgatcacccagtagatgaagatcagcaccgcaccggccgtgccgaacaccgtcaggcccatgtagttgccgccgatggccagtgcatcggtgggcgcggccgcgatgcagatcatgctggcggcgctcatgcccacgtagtgcatggtgcagacggcaacccccatcaccgcggcggcggcgatctggtggctcagccggcgcaggttgaaggccagccacagggccgcgccggccgcggtgatcgcaatggccaccgacagcgccacgatggtggggtcgaagtccatcgaagcgcgcatgttcattgcgaacatgcccatgtagtgcatcacgcagacgcccacgccggccagcaggctgccggccagccagccggtcttgctgaatttgcgccggccgcccgccaggtacagcgcaatgcccgagatcaggatggctgccacgagcgacaccacggtcagcggcacgttgtacgaaatgccgaccggcagccggtacgccagcatgccgatgaaatgcatcgaccagatgccaatgccccccagcgccaccgcggcgcacgccacgaccgcgagattgggtttgccgtcggcgccaaccatgcgccccgcacagatcagcgccaccagggaacctgcgaacgagatgaggaacgagagtgccaccagcccgagcgaatactcgggcgacagcagttggcctacgacgaggggagtcatgtttttatctccaaagagaacgactcgccgccgacggccggctggccaaaaggtgtaacgagacgcccgccgaggagtttgtaatacttgtttttaaaagtaaatcacttcttcatgccttgtcggcgcctcagtttttcgggcggatccgataaatcgcgttgttccggtcggctgacatgtagatggttccgtcgctgcccaccgcgacccctgtgaccacgtaaggcggcggcaagccggggctggcggccagcccgatcggcaggttttccgccaccgtgcggcgcgatccgttggcggggtcgatttccaccagccggcgcgccgcgctttcggccacgatgaagctgccccagggcgtttgcgccacgccctcgggcaaggccagaccctcggcaacggcgcgcagcggggcgctggcgtcaagcggaatgcgggtcagcttgccggccgcctcggtcacgtagagcgccccgtcccgcccgacgatcatctgcaccggcccgcccagtccgctggcgagcacttgcttctccgcgaagcgaaggcctcgcgcgcgggtgatggtgccggtggcaatctcggcatagatcacgctgccatcgggcatggggatcgcatcgaaaggcgccttcagtccgtggatggtttccacggtcctgagggtctggcgatcgaccaactgcaccgtgcccgtgaaccacgaggtcagcgcgaagagcgtgcccgagacgccgatcgcgaaggggtagtcgagctcgggatcgcgctgcatgcggaacacgtcgcgcacttcgccggtacgcacgttcacctggcggaagccgaacacgtccgccacccagagcgtgtggccgtcgatcttgaggccggccggcgccgcgagcttgccgctggtgagcgtgcgcagcgctccggtggcggggtcgaaggcctggatttcgttgttcgccatgttcgacacgtagatcgtgccgtcggacgcgatggcgaggttgtcgagggaggggcgcaactgcttggcgacggtcttccggccgctggccaggtcgacccgcaccagctcgccgctgcgcgcatcgaccacccagaggttgcccttgccgtcgaggttggcggccgcgggaatcttgaagccgtcggcgatcacggtcatgttgccgttggccgggtcgatcttcaccacctggcccttgaaccacagcgggccgtagagcatgccgtccgggccgacctcgaagccgttgaaaccgcccatgtccttcttgatgagccgcggcggcttctggcccatgcggtcgatctcccacagcgcatcgcccaaaaacacctgcgaggcgtagagcttgtggttgcggcggtcgaagtccagcgagttgaggccgggcaggtccttggcgagcacgcgcatcggcgcgccgtcgttctcgcggtagcgcagcatgcccatgaggtagttggtccacgccagctcgcccttgggaccgaccgcgatgtcgtcggcctggccttccggcgcgtcgaccaggaccttggcggcgccggtgttgcggtcgacttcccacagcgtattgccgagcaccgagcctgcgagcagccggcccttctggtcgatggtcagcccatgaacccctgcgaacgaggacggcggcaccagcgcttcgggctcggaccacgacgcgggcctggtgggcggcggcttcggtgcgaggcttccgcaggcgcccagcagcgcgaacatggcaatcagcgcggcggcgcaaaacgggcgacgggacatgtcttctccttctggtggatgcgcgagcagtctagaaggaggacggggaggcggcgcaatctctcccgggacatgcgcactttcgttcgctgcggattacccgcatccgcgcactgttcacccgcgcagcagctgcgtcaccgtgtgaatcaggagccccaccaagccgcccaccagcgtgccgttgatccggatgaactgcaggtcgcgcccgatgtggcgctccagctcgtcggtcatctcgctcgcgttccattcgccgacgcgctcctcgatgtagcggcggatgtcctcgcgatagcgctcgatggccagcggcgcggccgcttcgatctgctcgttgatccagtggcggatcgcctcgtcggcctgcagccgctggcccagtgcgcccgccatcgacgcgatgcgccggcggatcgtcgaatcgccgcggccgagatcgtcatgcagccaggccaggagctcgccccagattccatgcaggtagtcgcccagcgcggggtgcgccatcagctcggcgcggatctgctcgccgcgctgctggaactcggggtcgagcttgagccgcaccacgaagtcgtccacgaagtgatcgaagcgcttgcgcatggggtggtcgggctcggccgccagttcggcgatggtgcgcgccacggccgccacgatcttgcgcgtcgcgagcttggccgccacctggtccaggcccacgtagcgcagcgtcttgatctcgcgcgcaatggcctccgtgatgtgcgactgaacctcttctccatcgagcaggccggccacctgctgcagcacgtcgtcgagcagcgcctgatggcgtccgcccgccgtgagggcgtccagcgcctggcccatcaggcgagagaggtcgatcttcccgaggcctgccgcggcggcgcgtcccatgaaggcgcgcacgcgctcgtcgtcgaatgcggaaaggccgtagcgcgccgccgccacgccccattcgccgagcttctcgccgctggccgggcgcgcgagccagtcggccagccggccggccgcatcgaactgccgcagcttggcaagcacctgcgccgtgctcaggaagttgttgcagatgaagcccgccaacttggcgccgatgcgatccttgttgctcgggatgatcgcggtgtgcggaatcggcaagccgagcggatgccgaaacagcgccaccaccgcgaaccagtcggcaatggcgccgaccatcgcggcctcggcaaaggcggccacgtagccccaggccgggtgcagcccgtgcagcgcgctggccagcgcataaagcagcgcggcggcgcacagcaggccgagcgcgacgcgcttcatgcggtccgatgcgagcccgtgagcgccgccatcagccgatcttcggcgtcgaggcgaggcgctccatgaagagctcacagcgccccagctgctcgaggctcacgaactcgtcgggctggtgcgcctggttgatgctgcccgggccgcacaccacggtggggatgccggcgttcttgaacaggcccgcctcggtgccgaaagccaccagcgtggtgcgctcttcgcccgagaggcgctgcgcgagctgtgtgaccggatcgcccgccgcgccgaggaagctcggaatctcgcagatggtctcgaagcggaagcccgcatcgggcgccaccttcttcatcgacgcttcgaggctgccggcataggagacgacctcgtcctgcatcttctttgcgtcggccgtcggcaggtcgcggaattcatagcggaactcggcatcgcgcggcaccacgttgtcggcaatgccgccgtggaactggcccacgctcgcggtgctgaagggcacgtcgaagccctcgtagcgcggctcgctgcgctcgaagccttcggccatgtcgcgcaccttgccgaccacgcgcgccgccatctcgatggcattgactgagtgcggcgtgagcgacgaatgcgcctccttgccgcgcacgcagcagcggtagcggtacacgcccttgtgcgcgatggccggcaccatgctggtgggctcgcccacgatgcaggcgatgggcttgatgccggcgtcgcgcatgtcggcgatgagttccttcacgccgaagcagccgatctcttcttcatagctgaaggcgaagtgcaccgcgaagggcgaatcgctttccaggaaacgcccggcattggacagcgcaatcgcgatgaagctcttcatgtcggccgagccgcggccgtagaggcgctcgtccttcaccgtggcggagagtgggtcgacgctccagtcctgcccgtcccagggcaccgtgtccgtgtggcccgaaatgatgacgccggccggcttgccttcgccgagcgtggcaaacaggttggccttggtgcgttcggcgttgtaggtgatgcggctcttcacgcccagggcggccaggtggctttgcgcgaggtcgatcagctggaggttgctgtttgcgctgacggtgttcatgcgcaccagcgtctgggccagtgcgaggctttgaggggaaagcgtatggggcatgcaacagattgtccaagaagtcggtgccccgcgccgccgagcgcccttgctgtcatgcggagcgggtaccctgcgcctcttttggatggagaaaaagacgatgcgcactgttcagatcgccctcaccgcgaccgccgccctttgcctggcggcttgcagcaccaccggccccggctcgtccgggaagctgcagacgctcgacggccagccgccgctggtcatcgcgcatcgcggcgcttccggcttgctgccggagcagacgctcgaatcctatgcgcgcgccatcgaactcggcgccgacgtgatcgagatggacctggtctccaccaaggacggcgtgatcatcgcccgccatgaccccaacctggccatcagcaccgacgtggccaagcacccccgcttcgcctcgcgcaagaagaccatcaaggtcgacggcgaaacccagaccggctggttcagcaacgacttcacgctggccgagatcaagacgctgggcggcatctcgaccgacgccgagcggccgcaggagttcaatggcaagttcaaggtcgtgaccttccaggagatcatcgacttcgccaaggccaagtcgaaggaaaccggccgcaccatcgcgatctacccagagaccaagaacccgacctacttccgcgacctcgggctgccgatggaagacaaggtcatcgcggccatcaacgccgccggctggaacagcaagaccgcgcccatctacgtgcagtccttcgagccgggcagcctcaagtacatgaagagcaagggcctcaatacccggctgatccagctgatcgatggcgacagcgtcgacctgaagaccggcgccgtgacctttgccgtgccgagcgaccgcccctatgactggaccaaggccggcgacaagcgcaacttcgacgccatggtcacgcccgcgggcctggccgagatcaagacctatgccgacggcatcggcccctggaagcgctacatcgtgagcgtcaagggcaccatcggcgccgacggcaagccggtggacgtcaacaaggacggcaagatcaacgacgccgacgccacctccatcgcgcccaccacgctcattgccgatgcccacaaggcggggcttttcgtgcacccgtttaccttccgcaacgagtcgcgccggctcgcggccgactacaacaaggacggcaagaacgagtatggcgtgtattacaagctgggcgtggacggcgttttcaccgacttcaccgacaccgcgatcgccgcgcgcgccgagtatctgaagagcctcggtcgctgagtacggcctgggggtttgcccggcacggtctttgcggaggtctttgcaaagcctagactgtgcccccatgaaactcatcgattcgctcgtcacgcaggcggccggcatcgccgccgtccgacgtgacctccacgcccatcccgaactctgcttcgaagaagtccgcaccgccgacgtggtggcaggcaagctcaccgagtggggcattcccattcaccgcggcctgggcaccaccggtgtggttggcatcgtcaagaacggcaccagcagccgcgccgtcggcctgcgcgccgacatggacgcgctgcccgtcaccgagctcaacaccttcgcccacgccagcaagcaccacggcaagatgcacgcctgcgggcacgacggccataccgccatgctgctggccgcggcgcagcacctcgcaaagcaccgcaatttcgatggcacggtctacctgatcttccagccggccgaagagggcggcggcggtgcccgcgagatgatcaaggaagggctgttcgagcagttccccatggacgccgtgttcggcatgcacaactggcccggcatgaaggccggccagttcgcggtgagccccggaccggtgatggcctcgggcaacaagttctacgtcaacgtcatcggcaagggcggccatgccgcgctgccgcagaccggcatcgacccggtgccgatcgcctgcgagatcgtgcaggcgttccagaccattctcacgcgcaagatgaagccgaccgactcggccgtgatctcggtcaccaccatccatgcgggtgaaatcaacaacgtgatccccgacaactgcgagatgacgggcacggtgcgcaccttctcgatcgaagtgctcgacatgatcgaggcgcgcatgaagctgatcgccgagcacatctgcgccgcgcatggcgcgacctgcgacttccgcttcgagcgctactacccgcccaccatcaacaccgaggccgaagccaactttgcgcgccgcgtgatgggcgggatcgtgggggccgagaacgtgctgcggcaggaggccgccatgacctcggaagacttcgccttcatgctgcaggccaagcccggcgcctatgccttcatcggcaacggcgacggtgcgcaccgcgacgtgcaccacggcgaagggccgtgcacgctgcacaacgcgagctacgacttcaatgacgacctgattccgctgggcgccacctgctgggtgcaactggccgagcaattcctggaacccgggggagcagcgccttgatcggcatcggcgaggcgttttcgccccgctacgcgcaggcgcgccagaagttcctgcgggcctgcgtgagtgccggccttgcggtcgagccgcatgcgcatccgggcaaggggcaggacggcgaagagctctcgatggacgtggcgctcgacggcgctgccaatgccgagcgcctgctgatcgtctccagcgcctgccacggcgccgaaggccattgcggcagcggcgtgcaggtgtttgcgctgcacgacgccgaatggcgcgagaaggcgcgcgcccagggcgtggcggtgctctatgtgcacgcgctcaatccgcacggcttttcgttcgggcggcgcgtcacgcacgaaggcgtcgacctgaaccgcaatttcgtcgatttctcgaagccgctgcccgccaacgaagcctacgccaagctgcatccgctgctggtgcccgagacctggccgcccacgccggaaaaccaggcggccctggagaagtgggtcggcaagcacggcgtcgccgcattccaggccgccgtgagcggcgggcaataccagttcgacgacgggctcttctttggcggcaaggccgagacctggggcaacaagacgctgcgcaacgtgctgcgacgccatgcgggcggcgcccgccggctgggctggatcgacctgcacaccgggctcggcccgagcggcatcggcgagcgcatctttgccggcaaggacgacaaggcggcccatgcccgcgccaacgattggtggggcacgcccgcggcgccggtcacgtcgatctacgacggctcctccacctcggcgccgttgcgcggcctgatgtgcgaagcggtgtaccaggagtgcccggcggccgagtacaccggcattgcgctcgagtacggcacgctgccgctgctggatgtgatgaacgccctgcgcgccgaccactggctgcacaagcaccccgaggcgccggccgacctggccgacggcatccgcgcgcgcatgcacgaggccttctacaccgacaccgacgcctggcgcggccaggtcgtcagccaggcccgccaggccatgttccaggccgtggacggcctgggcgcctgaagccggcggggccggggatcaggtcctgacccggccgtcggccgtgatcatcgacagttcgacgaacttcgatgccacgtgattcttggccgagaaagacacctcgaagccgccgaactgctgccggtcgatgctttcgagccccgtgatgagactgtcgcgcgtggccttgcccggcgcgcggcgcaggccctcggtcagcaccttggcggcaaggtagccttccatgctcgagaaattggcgctggcgctggcaccggcttttttcaccgcgtcgctgaactcgcgcgtgatcgcgttggccgggttgtagggcgagggcaccacctgcgtcaccatgacgcccgcgccctccttgccaagttcgtcggccagcgcctgggtgcccacgaaggacacgttgaagaacgtgccgccgtagcccgccttgcgcgcctggcggatgaaggcggcgcatgccttgtaggcgcccacctggaccaccgcatcgggctttgcggccacgatgcttttcaccgccgccgccacgtcgaccgaattgcgctccaccgtggccagcgccaccggcttcaggtcctgctgcgaaagagccagggtcacgccgtcgagcccggccttgccgtaggcgtcgttctggtagaagaccgcgatcttcttcaggtggaggtgggtgagctgcttcacgatgagcgcggtctcgtcgttgtacgaggcgcgcaggtggaacacgttcttgtggaacggttcgcgcagcgacatcgcaccggtgaacggcgcgatgaagggcaccttgtccttcaccgccagcggcagcgcggccaggctggtgggcgtgccgatatagccgaagagcgcgaacacgtcctcttcgatcagcttctgcgtgttggcggcgcagcggtcgggctcgtagccgtcgtccaggttcttgatcaccaccgcgcgccggccggactgcgcgttgtactggtccaggaacagcttggcgccctggtgaaactggatgccgagctgcgcggccggcccggtgaacggggccgactggcccagcacgagcggcgtttcgccctgtgccctggccagctggaagccgcccagcgccgccgcgcccgcggcaacggaaaaatgtctgcgattcatcatggtgaaaacctcttttttgcgcgctggcgcgccaaacctggaaaactttagacttgccggatggtcgatgccccggtctccacaacagctgttctccccaccccaacttccgtggttctgggcgcgtgtccgcacgactgcccggatacctgcgcccttgtcaccaccgtccaggacggcgtggccgtgaagctgcagggcaatccggcccattcgcacacggctggcgttctttgcaccaaggtctcgcgctacatcgaacgcaacgagcatgccgagcggctcgttcagcccctgaaacggaccggccccaagggcagcggccagttcgagcccgtgagctgggaggccgcgcttgacgacatcgccgcgcatcttcgcgcattgcagacaaatccagacacaattgtgccgtacagttacgccggcaccatgggtttggtccagggcgagtcgatggaccgtcgttttttccacaagttgggcgcctcgctgctggatcgcaccatctgctccatggcgggcggcgaagcgatggtccacacgctgggcgccaaggtcggcatgcggatcgaattcttcgccgaggcgaagctgatcctgatctggggcagcaactccattgccagcaacctgcacttctggcgccatgcgcaggccgccaagcgcgccggcgcgcggctggtgtgcatcgatccgcgcaagaccgaaaccgccgacaagtgcgacgagcacatcgcattgctgcccggcaccgatgccgcgctggccttggcgctgatgcacgaactcatcgtgcacgactggctcgaccacgactacatcgccagccacacgctgggctgggagcagttgcgggagcgcgcactgcagtggccgcctgcgcgcgccgccgccgtgtgcggcgtgcccgaggcgcagatcgtggcgctggcagaggcctatggcaccaccaggccggccgcgatccgcctgaactacggcatgcagcgcgtgcgcggcggcggcaacgcggcgcgtgccatcgcctgcctgcccgcgctggtgggcgcttggcgcgaccgggccggcgggctcctgttgagcagttcgggccactttccggccgaccgcgccgcgctgcagcgccccgacctgctcgcgggccgccagccgcgcaccgtgaacatgagcaccatcggcgatgcgctgctcgacgaggccaggccggtgaaggccatcgtggtctacaacagcaacccggtcgcggtggcgcccgagtcgggcaaggtggtggcgggcttcgcgcgcgaagacctcttcacggtagtgctggagcagttccgcaccgacaccgccgactacgccgactacctgctccccgccaccacccagctcgagcactgggacatccactgcagctacggccacaccgacgtgctgctgaaccgtcccgcggtggcgccgcgcggcgaggcgcgcagcaacgcctgggtgtttcgcgaactcgcgcgccgcatgggcttcgacgagccctgcttctcggacgacgacgagacgctgtgccgcagcgcgtttgcgccgggcgtgatcgactacgggcagctgctggcgcagggcttcaccagcctgaagctgcctgaagcaccctttgccgacggcaagtttccgacaccttcgggccgctgcgaattcttcagcgagcggctccaggcgcaaggcatggacgggctgcccgaccacgtgcccaactacgaagcggcgggcagctccgccgagtttccgctggccatgatctcgccgccggcgcgcaatttcctcaattcgacgttcgtcaacgtgacgagcctgcgcgccatcgagggcgagccgctgctcgagatccacgaggccgacgccgccgcgcgcggcatcgagaacggcgccaccgtgcgcgtcttcaaccatcgcggcgagcaccgctgccgcgccgaagtctcgcgccgcgcgcggcccggcgtggtgcacggcatgggcatctggtggcgcaagctcggcatggacggcaccaacgtcaaccagctcaccagccagcgcctgaccgacatcggccgcggcccgaccttctacgactgcctggtgcaggtcgagcgtctcgttccttcgcccgcggggggcgggttggcgtgagggccgcgcccgcattcaccgcagccgccgccgcgctgttgctgctcggcggctgcgccgacctgggctactactggcaatcggccaacggtcacatcggcatcatgcgggtcgccaagccggtgcccgaatggctcgcggacccggccgtttccgagccgctcaaggccaagctcgaactcgcgcagcgcatccggcgctttgccgtgaccgagctgggcttgcccgacaaccccagctacaagtcgtacgccgacctgcgccgacccgcggccgtgtggaacgtggtggccgcgccgccgtattcgctcatgctcaagaactggtgcttcccggtggcgggttgcgtgggctaccgcggctactacgacgaggccgcggccagggccgaagccgacgcgcagcggggcaagggcatggaaacggcggtgtacccggtgcccgcgtattccacgctggggtggatgaactgggccggcggcgatccgctgctttccaccttcatcggctatcccgaaggcgaactggcccgcatcgtgtttcacgagctcgcgcaccaggtgctctacgtgcccggcgacacggtcttcaacgagtcgtatgccacggcagtggagcgcatcggcggtgcgatgtggctgcagcgcgaggccagcgagacggcgcgcagcgagtacgcgcgcttcgacgcccagcgccggcagtttcgcgcactggcgctcgatacgcgccgcgcgctgaaccaggcgtacgaatcgaaggaggccaaggcgggcgattgggcggcggtcgacgccatgaagaaagcggccatggacgatttccgcgagcgctacgcaaggcttcgcgcagaatggcagggcccgcgccaaggcgcctacgatggctgggtggcccgcgcgaacaatgccgcctttggagcccaggctgcctacgacgacctggttcccgccttcgaggcgctgttcgaacgcgagagccgcaactggccgcgcttctacaaggaggttcgccgcatcgccgcattgccgaccaccgatgagcggcggcacgcattgcaaacggccaccggaatccagcagacgaattcaagtcacgacaacaacggagaagatcacggtgcctgacatccttatcgaacgaaaccacgcgctgggcattgccagcgcccgcgaggtcgcgcgccagtggatccagcaggtggagcaggactacggcctggaatgcacctacaccgaaggcaaggaccgcgacctggcgcagttcagccgcgcgggcatcgacggcacggtggaggtcacggcccgcaccttcaagctggaggcgacgctgggttttctgttcgcgagcttcagccagcagatcgagcagaagatctcgcgcaacctcgatgcgctgctcgaagctcccaaaggcggcacgcgcttcgcgtgagcgggttcttcaggcgatggtctagccgccgatcatcgaagcgccacggttcgccaccagagcgaaggccggcggcggcacggcacactctggcgccatgacgaacacctcttctttccccgctgcgccgaccgccgcgggcccgctggccggactcaaggtgatcgaactcgggcaactgatcgccggccccttcgccgcgcgcacgctggccgacttcggcgccgaggtgatcaagatcgagccgcccggcgccggcgatccgctgcgcacatggcggctgctgaagaacggcacctcggtctggtggcaggtgcagtcgcgcaacaagcgttcgctcgcgctcgacctgcgccaggccgaagcgcaggccatcgtgcggcagctggcggccgaggccgacgtgctgatcgagaacttccgccccggcgcgatggaaggctggggcctcggccccgacgagctgctggccggcaatcccgcgctcgtgatgctgcgcatcagcggctatggccagaccggcccctaccgcgaccggccgggcttcggcgtggtggccgaggcgatgggcgggctgcgtcacctcacgggcgagcccggccgcgtgccggtgcgcgtgggcgtgtcgatcggcgacacgctggcatcgctgcacggcgtgatcggcgtgctgatggcaatgcagcaccgccatgccaccgtcagcgccgagcatccgaagggcaggggccaggtggtcgacgtggcgctctacgaggctgtcttcaactgcatggaaagcctgctgcccgaatacggggcgttcggtgcggtgcgcgaggcggccggcagcgcgctgcccggcattgcgcccaccaacgcctaccgctgcgccgacggcggctatgccatcgtggcgggcaacggcgacagcatctttcgccggctgatggaatgcatcggccggcccgacctcgccgccgatccggcgctggccggcaacacgggcagggtggcgcaggtggaaaggctcgacgccgccatcggcgactggaccgcgcagcgcacggtggacgaggtgctggccgcgctggccgcggcccaggtgccgggcgggcgcatctacaccatcgccgatattgccgccgacccgcactatgccgcgcgcggcatgctgcagcaggtgcagatggccgatggcagcgcgctcgcggtgcccggcttcgtgcccaagctgtcgctcacgccggccagccatcggcacaacgcgcccgcgctgggcgcggacaccgatgccgtgctgaaggagatcggcctcagcgccgagcagatcgccgcgctgcacgcgcgcgggatcgtcggctgagcggtcgaatgggtgggggtcagcctcgcagcgattcgatcaggtcgatgtatttctgcttggcttcgtcggcgccaaggcctttttgcgcggtccaggcgtcccacttggcgcgcgcgacgatgtcgctgaagctgggcttcttggcggtgttgtcgccttcggtggcctgtttgaagaggccgtagatcttgagcagcgtcgggttgtcggggcgctccgccagcagcttggaattggcctgggcagtttcgaattgggcgttgaggtcagacatggcggtgaaaaataggaattgaaaaagcgaacggccacatcttaaagtgcgcggtacccggcagtaccggtggcgcccgtcgaggggcggtgctcagtccgacagccccgcccgcgccagctccacgtcgagccgttccttggcgtccgcgggcagcagtgccgcggctttttcgtacagctgcgtggcctcgcccaggtaggcgtcgccgcgcagcatgagcagcgcgcggccgtactccatcagcgcgctggacgagtgggggtgcagctcgagcccgcgctcgaacagctcgaccgacatctcggcgcgcacgccgtacgtcatgcggccgaccagcgcgcccaccttgtcgatcacctcggcatggaaggcggccagcgcgatgtgcgcgtcggcatggtccggctgcagctcgatcacccgttcgagtgcgcccttgagcttgctgccgaggccctgcgccagcgcgcgcgccacgctgattccctggctgtagcggccgagcgcataggcctgccagtagagcgcgtggcagttgccgggatcggaggcaacctgcgcgccagcgcgctcgatcacctggcggaacatcgaaagccggaccgattcgcgcggctccaggtagttggcatagatggcggtggcctggttggccagcaccaggccttctgcgccgtgcagcaggccgagcgcggcggcgcgctggaactcaccgttgtggtacagcgcccagccttcggccagcgggtgtccctcggccggcggcggcacggcgtggccggcgtgcaggcggggccaatgcgcaagaaggttccgcgcgtcgtagcgcggcacgtcggcatagggcagcggcgtccaagggtccgctgtcgtggcaaccgggctggcggacatcagcgagagcggcttgaagtctggatggggcatggtctaggactgggctgccaaatcgactggcgcggccggaggcggcgcgctgtccgcatcatcgccgctgtaggcatggctcagtgtcagcaaatgccgccgctgttcagggccgaggtagggcgcgagcagctggagcgtgtgccggccgccgcgcatcagcgcaccctgggcatgcgcgggttccagtgcctcgcgcgggttgcgcacgtattcgtagctgagccagtaggtcagcaccaccaccatgctctgggcgagcgtgtcgacctcgtgggcgtcgatctccaggtggccggcccggctcaaacccgcgatgagcacgcggatggcgcgggccttgttcttgagcacgagctggaactgcgtttcgagatgccggttcttgctcagcaggtcgttcaggtcgcggtagagaaagcgatagcgccagatcagctcgaacaggctgtgcatgaagaaccaggcgtcttccacatcgtgcacgccttcgctggcgtgcaggagctcgttgagctcggcctcgtagccttcgtagagcttgttgatcagctcttccttggcgggatagtggtagtagagattgccggggctgatgttgagctcgcccgccaccagcgtggtggagacgttgggctcgccgaagcggttgaacagctcgagtgcggcttcgagaatgcgttgcgctgtgcggcgtggcgccttcttggccatgtcagtccccgtttgtcttttgaggacactctagcgtatgtgccccgcgccacaaactgggagggccatgtttttgcagcgccgccgttgtgcgccgccgcaaaaaggaagctcgaggcggcggtcagccggccttggtgctgcgccgaacggtcttcttggtggccgacgccggggatgccgcgctgcggccggccgtcttgcggctcgcggtgcgtgccggagcggcggtgcccttgccctgcatgcgctgcagttcgacctcgagggccgccacgcgcgcctgcagcgcggcatggtccgcggccgaaggcaggccgagcttctcgagggcgcgcgccacgcgctcttcgaagatgttctcgagcttgccccattggcccgcggccttggtgccgaattcgctcgcgaagccggccatgcgcgtttgcgcctgggtcagcgtttcttcggcggctgcctgggttttcttctgcatgccggcgccgtctttcaccagcgcctcgaaagccttgctgccttcctgctgcatcttggcgaaggcgccgagtcccgccagccagatctgctgcgcggaatccttgatccggtcggagcccttgttgccgtgatcgtcgtcctgggtagccatgcggatgttcctgtgaaaactatcgggctactctatccgctccacgcccttcccgttagagcttcatgtctacgaatcgagcctgatgggggctgcaagccgctaggcttttccagcagcgcggcttgcctcgaggtgggtcttggcccgttcggccagagccatttcacccggcgtgccgggcacgaagggctgcaccggtagggggcggccgtgcgaatcgaccgagacgaagacgatcaggcattcggtggtcttgtccatggtgccgcccttcatgtcgccgctgcgcacctcgaccgagatgttcatgctggtggtgccggtgtaggccagccgggcctcgacctcgaccaggtcgccgatcatgatcgggtggtgaaagcggatgctgccgatgaaggccgtcacgcaatagcgcttggcccaactggtggcgcaggcgtagcccgcttcgtcgatccatttcatgaccgtgccgccatggaccttgccgccgaagttgacggtgctgggctcggccagaaagcgaagggtgatggaagacatacgccgcctttttcgtgggctgatgggtgggaacctcaattatgcgagcgaccggcccctgggcggctcgccgccggtcgccatggcacgcacgttcagccgccgccgaacagttccgccagggtgagccggagccaggcgttgccggcgtcggcatggaagcgctcgtgccagtgctgcttgacggcgtaggccggcagctcgaagggcggctccagcagcttcaccggttcctgcgtggccagcaccttgccgaggatgctgggcacgatcacgatgagttcggtatgcgccacgatgcgcgccacgctcagaaagctcgacaggctggtcaccacgttgcgcttcagccccagccgggcgatggtcttgtcgacgatggcgtggccggtgcccgacgaagccaccaccgcgtgcgcctcggcctcgaagcgcttgcgcgtgagccgctggccaatgcgcggatggttgcgcgctgccaggcagacgaagttctgcatgaagagcgtctgctggtagaagcccgcgtccagctgcggcatgaagcccactgccaggtcgaccgcgccgtcctcgagccggcgcgcgctctcggtggaaatgatctcggtctcgatgcgcacccccggcgccgcatgccgcaggtggccgagcaggcccggcagcagcaccacctcgctgatgtcggtcatgcagatgcgaaagctgcgtgccgcggtggcggggtcgaagctggcgcgcccgcccttggcccggttcagccggtcgaggacgtcctgcattagcggctggatctgccgcgcgtagggcgtcggctccatgccgcgcgaggtgcgcacgaacagcttgtcgccgaaatgcgtgcgcagccgggccagggcggtgctggccaccgactgcgcaatgccgagccgcccggccgcactcgacacgttggcggtcttgtagacctcgtcgaacacccgcagccattcgagatcgagctgggccatgaaacaactcctttgccgccaccattatcaaaaaaccagatcgaggctatcgccttgtctcgattgcgccaatagtagtaccggtggaagatagccttttcccggagacaacggccacgcgagggccggaaccgccatgaatcccactgccaagaaacctgccgccacagcgcctgccaacgccgcggagcgccgcggctattacgagcgcatccgtccgctccacctcacgccgctgtgggagtcgctgcatgcgctggtgccgcgcgagcccgccacgccctgcgtgccggcgctctggcgctacgacgaaatccggccgttgctgatggagtcggcggacctcatcaccgccgaggaagcggtgcgccgcgtgctggtgctcgagaaccccgcgctgcccggcaattcgtcgatcacgcagtcgctctacgccggcctgcagctcatcatgccgggcgaggtggcgccctcgcaccgccacgtgcagtcggcactgcgcttcatcgtcgacggcaagggggcctacaccacggtgggcggcgagcgcaccaccatgtacccgggcgacttcatcatcacgccgtcgtgggcctggcacgaccacggcaacgagggcgtcggcggcacggtggagccggtggtctggctcgacgggctcgacattccgatgctgcgtttcttcgatgccggctttgccgagaacgacgacgccaaggtgcagcacgtggcgcgccccgagggcaacagcctcgcgcgcttcggacacaacatggtgccggtgcgtcacgaccacgtgtcggccacctcgccgatcttcaactacccctatgcccgcagccgcgaggcgctggccctgctgcagaagcaggaagcgcccgatgcctggctgggccacaagctgcgctacatcaacccgctgaccggcggcgcgccgatgcccaccatcggcacccagctgcaactgctgcccaagggctttgcgggcaagacgcaccgcgccaccgacggcaccgtctacagcgtggtcgaaggccgcggcagcgccgacatcgcgggccagcgcttcgagttcggcccgcgcgacaccttcgtcgtgccctcctgggcgccgctgcgcctctcggcatccggcgaagacgtggtgctcttcagcttctccgaccgtcccgtgcagcaggccatgggcatcttgcgcgaagccttcctcgacgaggcctgagagccggccggacctcattttttctttctttcttccgtccttgtcttgaccctgtgccgccgcgcggcaggagccttcatgtccttcgtcttcacgcctccttccatcgtcggcctgcccatcgccggttcgagcgacctgttcccggtgcgccgggtctactgcgtgggccgcaactacgcggcgcatgcgcgcgagatgggcttcgaccccgaccgcgagccgccgttcttcttctgcaagcccaacgacgacgcctccgtggtgcccgtggccgaaggtgaaaccggcgccattccatacccgccgctcacgagcaactaccactacgaagccgagctggtggtggccatcggcaagggcggcaaggacatcgcggtggagcaggcggccagccacatccacggctatgccgtgggcctggacatgacgcgccgcgacctgcagatgaagatgcgcgaacagggccgtccgtgggagatcggcaaggccttcgacttctcggcgcccatcgcgccgcttcgcacctttgccgacgtgggcgagatcaatgccggcgccatcacgctcgaggtcgacggccaggtgcgccagaacagcgacatcacgcacctgatctggtccgtcaacgaggtgatcgccaatctctcgacgctcttcacgctgcagcccggcgacctgatcttcacgggcacgcccgaaggcgtgggcgcggtgaagccgggccagatcctcaaggtgagcatcgacaagctccccttgctcaccgtgcgaatcgactgatcgagcattgcgcagaggcccaccatgagcacatctcccccgaagaatccccccaccgtgctgctcgtcggcggcggcatcggcggcatggccgcggcactgtcgctggcgcgcctcggtgtttccatcgacctgctggagcagagcgccaccatcggcgagatcggggccggcctgcagctcggtcccaatgccttcgccgctctcgacgcgctgggcgtgggcgaggcggtgcgccagagttcggtcttcaccgaccggctcgtgatgatggatgcggtcgattgcggcgaggtggcctcggtgcccgtgggcgaggcctttcgcgcgcgcttcaaaaatccgtacgcggtgagccaccgcgccgacctgcacggtgccatccacgaggcggtgaagcagcatcccctgatccgcttccacacctcggcacaggtcgaggccatcgacatcggccaaggcggaacgcaaggcgtggtcgtcaccacgcgcgacggccggcgtttcaaggccgacgccatcgtgggttgcgacggcgtgaaatcggtcgtgcgcgccagactcgtcggcgacgaggcacgcgcctcgggccatgtggtgtaccgcgcggtggtgccggtggccgacatgccggccgacctgcgctggaacgcacccgtggtctgggccggtcccaactgccacctggtgcactatccgttgcgccatggcgagcaatacaacctggtcgtcaccttccacagccgcgacaaggaagagtggggcgtttccgagggcagcagggaagaagttctctcctacttcgagggcgtgcatgcgcgcccgcgccagttgctcgaccggcccacgtcgtggcgccgctggagcacggccgaccgcgatccggtggagcgctggagcgacggcccggccacgctgcttggcgatgcggcccatccgatgatgcagtacctcgcgcagggcgcttgcatggcgctcgaagacgcggtgacactgggcgccgcggtgcaggcctgcgatttcgacatgccggccgccttcaagctttacgaggccgcgcgcattccacgcaccgcccgcgtggtgctttcggtgcgcgagatgggccggctctatcacgccaagggcgtggagcggctggtgcgcaacagcctctgggtaggccgtacgcccgaacgcttctacgatgcggtcgaatggctctatgcctggcggcccgagcattgcctggacgacgcgcgaccgggctgctcggccgcggtgatttcagcgcactgaatcgcacggatttcttccaccatcaccatttgaggccacaggcccaggagacaaaggaccatgaacaacaacatctcacgcgcactgtggacggggctcatcgccctttcggccagcggtgccgccctggcgcaggccagcgactttccgagcaagccggtaacgctggtcacgccctttgccgccggcagcgggcccgacgcggtgctgcggctggtgtccgacaagctctcgcgcctgtggaaccagcgcgtggtgatcgacaacaagcccggcggcggcggcttcatcgccatcgaccaggcgcggcgcgccgcgcccgatggctacacgctgctgcagctcgacagcgaacacatcgccgcgctgccgcatctgtacaagtcgcgcaacttcgtgacgctgcagcacttcgaccccgtggcctcgctgtttcgcacgccgtttttcgtggcggtgtccagcgagtcgaagtggaagaacatgagcgacctgatcgccgacgccaaggccaaccccgaagccatcgtctacggctcgtggggcgtgggcagcccgggccacctgggcgcgcagcagctggaggcgctcacgggcatccgcatgcggcatgcgccgtaccgcgaggtgtcgcagctgttctcgaacgtgggcacgggcgacgtgccgtggagctttgccagcattccgtcgagccagggcatctacaaggccggcaagctgcgctacctggccatcgcggcgcccaagcgcattccgcagctgcccgacgtgccgaccatggcggaagccggtggcccggcctcgctcgaggtgaattccttcgtctcgctgcttgcgcccaagggcgtgccggcggcggtcaaggccaagatcaacgccgacgtggccaaggtcattgcagaccccgaaatccgcgcccgcttcgacaccttcgcgttcgagccgctggcctggtcgcccgaggagatcgagcgcaacgccgaggccaagtccaaggtgtacggcgaactggtgcgccggggcaacatcagcctcgagtagcggcgcccatcagtaccattacgttttttcacagtcttctttttcaccttcttccatgcacgcatccaagagagccctcctgatcgcctgcggcctggcagccgccgccgcgctgccgctggcggcccaggcgcagaacaacgcctggccgaccaagccgattcgcctgctcgtgggttttccgggcggctccacgcccgacatcgccgcccgcaccatcgccgagccgctggccaaggcgctgggccagccggtcgtggtggacaacaagcccggcgcctcgggcaacatcgcggccgacatggtggccaaggccaccgacgaccacacgctgggcatcgtcatcaacggcaatctcacctcgtcgaagatgctgtacccgcggctgccctacgacccggcgaaagatttcacctacctctcgctgattgccacggcgccgctggtgctggtggcgcagaacaacctgccttcgggcgcggccttcctcgatgcggcacgcaagggcggcgacaagtggaactacggttcggtgggcgtgggctcggtcgggcacctgggcatggagctgctcaagagccgcgtggccggtttcaatcctgagcacgtgccctaccagggcaatcctcaggtcgtgaccgcgatgctcggcgaccaggtgcagatggccctcattcccccgggcgtggccatgccgcaggtgcgcgccggcaagctcaaggccatcggcctcacgggcggccgcagcgcgctggtgcccgagctgccgccgctggccgacgccggcgtgcgcgacttctcgctcgaagtgtgggtggcgctgctcggccccgccaacctctcgaagacggcgcaggcccgcatcagccgcgaactcgaagtgatcatgaagcagcccgaagtgcgccagaagctcttcgagcagggctggcaggcggtgggcacctcgcccgacggcatgcgcctgcgcgtcaaggaagaagcggcaatcatgagcaagatcatcgcgacccgcggcatcaagatccagtgatgacagccgtccagcacagcaagaccctgaccgagccggcgcgcgagctgccggtgttcggcgaatacgacgtggtggtggtcggcggcgggcccgccggcattgccgcggccgtcagcgcggcgcgccacggtgccagcacgctgctggtggagcgctacggctttctcggcgggatgggcaccgcgggcggcgtgaccaacttcgcgggcctgtacggcaagcgcgacggccagatgacgcagctggtgcgcggcgtgaccgacgacctgctggcgcgcatcgacgcgctgggtggcctcaacaagccgcaggacggcatgcagggccgcatccgcgtgcgctcctacgacacctcggcctacaagatcgcggcggaccagttgctgctcgatgccggcgtgcacctgctgttccacgcctgggcggcggcggtgattcgcgacggcgaccgcattgcggcgctggtggtcgagaccaagtcgggccggcaggcgattcgcgccaatgcctttgtcgatgccagcggcgacgccgacgtggcggcctttgcaggcgtgcctttcgaagtgggcgacggccatggcagcggcctcttcccgaccacgatgtttcgcgtcggccaggtggatgcgcagccggcgctcgcggccgtgggcgaattcaaggccatcaacgatctgatggagcgggtacaggcgcaaaagcccggcgcctacaagttcccgcgcgaaggcgcgatcctgcggcccaacatcgacccacgcgaatggcgtgccaacgtcacgcagatccgcaacgcggccggccgtgcgatgaacggcgtcgatgcgcgcgagctcaccgagggcgagctcgaaggccggcgccagattgccgaatacttcaagttcatgaaggccgaggtgccgggcttcgccgagtcggccatcgtggagatcgcgccgcaggtcggcattcgcgaaacgcgccgcatcgagggcctgtacgcactcacgggcgaagacatactgtcgtcggccagcttcgacgacagcatcggcatcaacgcctggccgatggaaatgcatgccgacggccgcatcgaatgggcctttccgcgcgacgacaaccgcacctacaaccagctgccctggcgcatgctggtgccgcgccggatcgacaacctgctggtggccggccgctgcgccgccatgacgcatgaaggccagtcggccgcgcgcgcgagcggcggctgctttgtcatggggcaggcagcgggtacggcagcggcttcgctgggcgacagctcgaagttcgcggacgtcgacatgcctgcgctgcaaaagaagctggtcgccgacggcgccgatctcgatcgctgatcctgcggcgtggtgttgaccgccccgcgacagcccgcgggcccggcctttgctatggttgagggttgcttcctctgcgttgaacgcgcctctcccgatgaccaccgatcccgccaccgccgcccgccttgtcgacgaactcgtcgcgctcatgcagctcgaaccccttgggggcgacaagttcctggcccagagcgaagacatcggcacgcccgccgtgttcggcggccaggtgctcggccagtcgctcgcggccgcaagcctcacggtcggcgccgaccggccggtgcattccatgcacgcctacttcctgctgccgggcgagcatgcgccgatcgaatacagcgtggaccgcgtgcgcgacggccgcagcttcaccacgcggcacgtggtggcgcgccagcaggagcgcatcatcttcgagatgtcggcctccttccagacggtggacgacggcgtcgagcaccagtccgccatgcccaccgtcgtgggccccgaggggctggtgagcgaactcgaccagcgccttgcgctcggcgaccgcctgcccgagcgctggcgcatcaagggcctggagccgcacggcatcgaataccgccgcgtcgaggccgacgacctgctgacgccggaggtgcgcccgtccgaaagcgccatctggatgcgcgccattgcgccgctgcccgacgacccggtcgtgcaccgtgcgctgctggcctacgcttccgaccacgggctgctgcgcgccgcgatgctgccgcacggcctgagcttcatgagcggccaggtgcgtcccgcgagcctcgaccacgcgatgtggttccaccgcgatttccgcatggacgattggctgctctacgtgctcgactcgccaagcgcgagcggtgcacgcggcctgtgccgcggcagcctgttcacgcgcgacgggcggctggtggcctccacggcgcaagaaggcatgctgcgcgtgaagcgctgaaaacaattcaaggacctgcatcgacatgaagatcttctactcgccggcttcccccttcgtgcgcaaatgcatggtcgtggcccacgaactgggcattgccgaccgcatcgaaaaactgccgagcgccgccggtccggtgaagcgcgatgccaccattcttccgaagaacccgctcggccaggtgccgacctttctgtgcgatgacgggcaggcactgttcgacagccgcgtgatctgcgagtacctcaacgccacgcagtcgggtgcgttgttcccggcggaaggcgccgagcgctgggcgcgcctgacggaactcgcgctggccgacggcatgaccgccgctgcattgctcgcgcgctatgaaacgatgctgcgcccggaggcgctacgctggaacgaatggaccgaggggcaactcgccaaggtgcgtaccggtgtcgaatggctcgaaacggccgcgccttcgtttggcgaccgcgtcgacatcggcaccatcgccttcggctgtgcgctggggtacatggacttccgttttccttcggtcgactggcgagcccaggcgctgaacacggcgaagtggttcgatgcgttcaaccggcgtgcttcgatgcaggcgactttgcctgcggtctagagttctagagttcttcagggcgcgctcccgccgacgggtgccttgctcctcgaatgtccccccgccttcagcgcatgtccagcgcgtcgcgaccgccgtggccgcgctgatgaaggcggtcgagcggctgcgcaaagtggatgccatcgggctcaaccaggccagccgcgacctgatcctgcggctggacgccgcgccggtgtaaggcgtgggttttaggtgattttccccatgagccgggtggtgccttggacctagcctttccggttcccgtcggatgtccgatggaccggaaaggctctcatgaaaattcccgctccggtgctgacgaacatgcgccgcaccgtccagtcctacgaagactccgcgcgcgaatacgacgcgatcgtggcggaccacccgccgcccgagatcgaggacgcgctgcgccggatgatggcgctcgtccccgccggcggcaccgtgctcgagatcggttccggcacggggcgggacgccgacttcgtcgagtccctgggcgggatcgtcaggcgcaccgatgcgacgcaggcctttctccatctgcaggcggagcgcggcaagaagggcgagctgctcaacgtcgtgacggatgcgctgggcgggccctacagcgccatcctcgcgatggccgtgctgatccatgtcgatcgcgcgcaggtcgcgccggtcctgcgcaaggtgtttgacgccctcgagcccggcggcgtcttcctcgtggccatgcgcatcggcgaaggtgagacgaatggcgactaccagaccgtgtactgggcgaaagaccggtttgccgaagagctcgcagcggccggcctgcgcacggaatgggacaggcagtggatcggccgcgagaacgtgacgtgggtcagcttcctcgcgtgccgtccacgggagcgcgtgcagacctacacgcccaggtagcgcgtccacagcgaacggtcggcgtccagcgcggccgagtcgccctgccacaccacgcgccctcgttcgaggatcacgtgacggtcggccagcggcagcaggcgctgcacgtacttgtcgaccaccaggatcgcttcgccctcggccttgagcgtggcaatgcaatgccagatctcttcgcggatcaccggggccaggccttcggtggcttcgtcgaggatcagaaggcgcggatgcgtcgacagcgcgcgcgcaatcgccagcatctgctgctcgccgcccgacagctggttgcccgcattggccttgcgttcggcaaggcgcggaaacaggccgtacagcgcctcgatcgtccagcgtggcgcgctgcccgggcgtggccgtgcaaaggcgcgcaggtgctcgtccacgctgaggttcgggaacacatgccggccttcgggcacgatggcgacgccgcgccgcgcgatggcgtcgggcttgtggccgccgatggcgtcgccgccgaaatgcacgctgccgcgcatcggcgcgagcatgccggtcagcaccttcagcagcgtgctcttgcccatgccgttgcggccgagcagcgcaagcacttcgccgggccggatatgaaggtcgatgccgaacagaacctggctggcgccgtagccggcctcgatggatttcgcatcgagcaatgtgatggtcgttgcgttcatgcgtgcccttctgcttccgttccgagatagaccgcctgcacgtcgggatgcccgcgcacttcgtcggccgtgccgctcatcagcacgcggccctgcaccagcaccgtgagccggtcggcgaggcggaacactgcgtccatgtcgtgctcgatcagcaggatggccatcgattcgcgcagcgattcgatcagctcgaccatgcgcgcggattcgtcggggcccatgccggccatcggctcgtcgagcagcagcagcttgggttcggccgcgagcgccagcgccacgtcgagcgcgcgctgtgcgccgtgcggcaaggtgcccgcgatgcggtggcgttcgccgcccagccccacgcggtcggccagcgccatcgcgcgttcgaccaggccgcgttcggtcgcgcgcggtgccatgaagcgcaggctgctgcccgcatgggcctgcgccgcaagcatgaggttgtcgtgcacggtttccttggcgaagacgcgcgtcacctggaagcagcgcgacatgccggctgccacgcgctggtggtccttgaggccggtgatgtccttctcgtcgagcaggatgcgcccggcgtcggccttgagcagcccggtgatcaggttcaccagcgtggtcttgcccgcgccgttcggcccgatgagcgcatgcacttcgcctcgctccaccgtgaggttcacatggtcggtcgcgagcaagccgccgaagcgcttgaccaacccttcgattctgaaaaggctcatgttgttgccttgctccctcgcccctgtggggagagggttggggtgaggggcaagcggcgtcgatagagagcagcaagccccttcggtgcccacaacgcgacagcaatcagcaacaggccgagcggcatgtgccaatgctccgtgtgctgcttcaggaactcttcgagcacgagccacacgacggcgcccacaggcccgccccagctgcgcccgagcccgccgatgacgaccatcaccagcagcgtggccgactgcgtccagtgcatcgtcgccgggctcacgaagccattgccacccgcgagcagcgcgcccgccagccctgcgatggcgccggcaatcgcaaaggccaccagctgcagcctgaacaccggatagcccagcgcccgcatgcgcgtctcgttgtcgcggatgcccatcagcgcatggccgaagcgcgattgcgtcgcgcggtgcagccaccagagcgcaagcgcgaccagcgccagcaccacccagtagaagttcgactcgttgcccaggtccagcccgggaagcagcgtgggccggctcatcagcgtgtagccgtcgtcgccgccatagcggcgcagcgacaccaccacgaagtacagcatctgcgcgaaggccagcgtggtcatgatgaagtagacgccgcgcgtgcgcagcgccaccgtgccgatcagcgccgcgacgaggccggcgacgagcgcggccgccggccacatcacccaggccgacaccacgcccgcgtcgctgagcgccaccaccgtgtaggcgcccatgccgatgaagcccgcatgcccgagcgcgaccatgccgccgaagccgaggatgaagttgaggctggcggcggccagtgccaccacgagcacgcgccgcacgaagccgatgtagaactcgagcccgaacacgggcgcgaccagcggaaaggccgcgagcagcagcaggagcagcccgagaccgatatagcgagaggaagacttcatgcgcgtgccgagaacagccctgaaggccggaagatcagaacaatcaccatcagcgcgtacatcgcaacttcggcgaacagcggccccaggtcggcggccgtggcgggcggcagcgtggcgcgcagcagcatcggcacgaaggcgcgcccgatggtgtcgaccacgcccaccagcagtgcggccacgaaggcgccgcgcaccgaaccgatgccgccgatcaccagcaccaccagcgcggggatcaagatggcctcgcccatgccgacctgcaccgcgacgatcggccccatgagcgcgccggccagcgcggccagcgccgcaccgagcaggaacacgccgttgaagatgcggcccacgcgcacgcccatcagctcggccatcggccggtcggaggcgcccgcgcgcactcgcatgccgatgcgcgtgtggttgaccagcaggtacagagcgagcgccaccagcattccgccgaccaggatgaccagccggtacgccgggtacggcaggccgtccatcaggttcaccggccccgaaagcgctgcgggtgtcggcgccatcacgggcgagggtccccaggccatcgtcacgatgtcgtccgccaccaggatcacgccgaaagtggcgagcacctgcgccagatggtcgcgtgtgtagaggcggcgcatcagcagcacttcgagcagcagcgccaccactaccgtgacggcgaccgcaatcacgatggccgccgtgaacgagccggtgcgcgtgtgcgcctcggccgccacgtaggcgcccgacatgaagagcgagccatgcgcgaggttcagcacgtccatgatgccgaacaccagcgtgagccccgccgccagcaggaacagcatcaacccatagccgaggccattgagcagctgctcgagaacgaggatgccgctcacttgagggggcacttgtcggcgtagctgtccccgtagttggtcagtacggtgttgatcagcttgttcgtgaccttgccctgcgcgtccttgccgatcacgcgcaggtagaagttctcgaccggatagtggttgttcgcgtacttgaagttgccgcgcgtcgaggcgtagttggccttcttcagtgcggccaccacggcttcgcggttctgcgcgttgccgccggcctgcttcacggcggcatccatcgcaaggagcgcgtcataggcctgcgccgcatacaccgacggatagcggccgttgtattccttgcggaacgcggccacgaaagccttgttggccgcgttgtccaggtcgtgcgcccagtgcgaggtgttgaacaaaccgagcatcggctcgcccacggcaccgatcacgtcctcgtcggccgagaagccgctggtcaccagcgtgatgtctttcgacaagcctgcgcccacgaactgcttgatgaagttgatgcccatcgcgccgggcaggaagaagtagatcgagtcgggcttggccgcgcgcagctgcgcgagttcggcggcgtagtcgatctggccgagcttggtgtagagctcgtcggccacctggcccttgaactggcgcttgaagccgccgagcgcgtccttgccggcgggatagttgggcgcaatgagcaccgtcttcttgaagccgcggtcttgtgcgaacttgccggcggcctcgtggaactggtcgttctggtaggcggtgccgaagaagtacgcattgcattgggcacctgcgaactggctcgggccggcattggccgagaggtacggcaccttggcgttgaacagcgtcgggcccacggccagcgccacgttggagccgatggggccgctgaagatgtcgatcttgtcgcgctggatcatgcggtcgaccagctgcttggcctggtcggggctgccggccatgtcggcctgcacgaactcgacgtcctgtccaccgagcttgccgcccagctgcttgatgccgagcgcaaaaccgtcgcgcgcctcggcgcccaaggccgcgaacgggcccgagatgtcgagcgccaggcccactttgacggaagcggccatggcggatgccccgccaccaagggctgcgccacagagcagcagcgaaagcagggtgcgcggcagcgcggacgacttcggggacggatggctcatggattctccgggcaaagaaagggtgaaacgacgccccggtgccgcgccatgcagcaccgaagacatcaaaccgttgatagctaaatactttaaccataaacaatttggtgtcaacggtgctagcacgaatggtgccaatgcctcgtgtcacttcctggtgcgcgggagccctttttccaagggcccgcgctggctcagccgaacggatttgcagtggcaaaccagaggccgatgcccgtcgcgatgatgaatgcgccgtcggtcacgcccgccaccaggaagaacttggtctgcagcgtgtcgaccagctcgggctggcgcgccgtgctctcgagaaacttctggccgaccagcccaatgcccaggcaggagccgagggcggcaacgcctatgagcagggcgactgcgaggggaaggatgttgaagccggtcatggtgttttctcctggtggttgatgtttgatcgatggaggtactttcccagagcgggtgcatgcggtccatgacgtgggaggtcatgggcggcacgaaaaaagccggccgtgaaaacggccggctctcgcgaagcatcgcgggcgctacggaagctgcgtccagttctggttgttgccgccgttgcaggtccacgtgatcaatgcggtgtcctgcgtggtggaaccgttgggtacgtcgaggcaggaacccgaggcgcggttgcggatcgatccgcccaccaggctccattgggtcgtgttgcccgccgtgcaggccagctgcaccaccggtgcattcgtcgtcgcggtgccgttctgcgccaggcacaggccgctgtgctcggccacgaactgcacatagccgccggtgaggctgttcaccgtgaacttctcgttgcttgcattgccgcacggccattgcaccgccgtcgcgccgctggcggtggacacgcccttgatgttcacgcacatcgtcggattcaggtccgagcggacgcgcgtgacgacggccggggccgtgtcctgcgaccgcacgtactcgcggatcgccacctggtcggccgcgggcaggctgttggcgttgccgtggccgctggtgagcacgtcctgcagcgtcgcggcctgtccgttgtggaagaaggccgtggtattccaggtgcccgacagcgtcggcgtgtcgaagcccacacccgccagcggttggttcatgcccttgcccgaagaggcctggatcgtgcccacgtcgtgccggatgccgtcgcgcaaggtgccgcccgagtggcaggtcacgcactgcgccgaggtgaacagcgcctggccccgcgccgcatcgacgctcaggctgccgtccgctgcacgcgccgggctgcgcatgtacttgttcagcgagctgaggtaggccgccatgtcgtcgagctgcgcgttcttgccggccttgggcgtgcccagtgggtcggacgtggccgcgaagtccgcattcgtcaggaagccggtgccgccgaactcgttgcggatgtcgttctcgaagtcctgcacttcgtcgaagttggccgtccagtgcagcttgccgtgccccaggccgcggcggcccatgaggctgatggtgcgccgcagcccctcgccgcgctgggtgaagtcccacaccatgccgtcgtcgccgccgtcggcgtggcagctcgcgcaggagaggtagttgtccttgctcatgcgccggtccgacgcgttgtagaacacctgtttgccgcgcagcgccgcggccgccatcggctcctgcgcgaccgtcaccacgttctgcaggaagatcggcgccgccgattccgatgacagcaccgaggccacgtcatgcaccgacaccgagcgcgcgaggaagttgttgacgaacaggcgcttgcgcaccgcgtccaggtacaggccgtgaggcgcgctgctggcgttgatctcgccccgcaccgcgcggctgtacggatcgacgatggccacgcggttgccttccatctgcgcgacgaagaggtagtcgcccgacggcgagaacagcgcggcgcgtgccggtgcgcggtcgtcgaagtcgatctgctcggcgaacacttccgcggccgtctgcaggttgacctgcgagaggatggagcgcaccgtctggtcgtgcgccaggttgttgccgtccctgaacttgccgcgcacgatgttgtccttcttcgaaggcagcaccgcccgcgcgccgtccggcgagatcaccacctggctcaggtagttggccacgccgcgcgcacggctctcggtgtccaccgtggtggtgtccaccggcagcgcgatggtggtcatggcgctcatgctctgcaggttcaccttgtgcagctggccgccggtcatcttcgacttgaagcgcgtgacgtaggccacctgtgcgtcggagctcaccgcgatgccgcgcaggttgccttcgagcgcgaccgcgccggtggtggcgccgttgctcgggtcgaagctcatcagcaccgccttgctctccagcgtcagcaggcccttggcgccgtcgggcgtgaaggccacgccgtaggggccgctgccgtaggcgagcggcacggtggccgagaggctgccgtcggccgcgctgagcgccaccagcttgtcctcgccctgcaccgtgacccagatgcggccgtcggggcccacggccagcgtcttcggctcgtcgccgacgcgcgtttcccagcgcttggccagggtctgggcgtcgatggcggcgaccgtgccgctgtcgggattcaccgcgtacaccgagttcgcatcgcccgcgatgttggtggtgtgcgtgggcgcccgcgccgtgaccggggcgatcaccgtgacgatgtaggtgtagaaggtctcgcggccgttcgcgtccttcaccgtcagcgtcaccgtgtagtggccggggcgcgtgtaggtgtaggtgtagttcggctggctcgcgtaggccgtctgcgtgccatcgccgaagttccagcggaactgcgcgccgctgctgcccagcgtggccgggttgaacaccagttggccgttgacgatcttcggcccgccgccgatgccggggtcgccgatgatggtctgcccgcgcagcgtgctcacctcggtgtcggagagcacgcggccgtagacgcgcacttccgccagcgtgcccttgaagagcgccgcgttgccctggatctgccccagcacgctgaacttgtttgtgaggcccttgttgcccgtgaggccggcggaggtggtcttcacgccgtcgacgtacaccgcctgcgcgccggaggccgcgtcgcgcgtcaacaccacgtggtgccagttgccgtcgttcactgccgccgtggaggtggtgccggcatggttgcccaccgacagcttgatgcgcccgctgttgtcgagccagccccagaacacatcgtccgcgccgcccgactggtcgcgcccgaagatgccgggcgcggtccacgagttcgccccgcccgcctgcgtggtcttcatgtagaaactcatcgatgcggtgccgccgagcacggtggccacggaatcgttcttcagcggcacaccggcggtgcggttcgcgaagttcatgccgatgctctcgaacgcgtcgcccgacgccggcgtgccgttgttgttgccgatctggtcggagaggttgccggccagcgtccagtagtgcatcaggttgatgtcggtcgcgttgccggtgttgaaggtcgacttgtagtccacgccgatggcgttgcccgcatagtccttcacgccgttggcgggcaggaacacttcatagctcgtgcccggcagcagcggctgctcggggtggaagttgacgatgcccaactgcacgctgtaggtgcccgccagcgtgttgccgcccaccgggcgcacgatgaaggtgttggagttcacgctctcgggccggatgctgtccgtcatgcccaggccgatgcgggacgtcagcgcctgctgcttcgcgccattggcgggcgagacctgcttcacttccggcttggtggtgtcggggtccaccgcatgcacgatgaagccgctgcccgagccgtggtcgttgcccacgaagacgagattgccgaacatcgcgacctggccgttgtccgaatgcgagaagttcggatcgtcctcacgcaggatgctgccgcggcccacctccacgtggttcagcggattgctcacgtcgaccttgtggatgcgggtctgggcgccctggatcacgtagttgtcctgcgtggcgcagtacagctgttcgtcgatgaccagccggttgtcctcggccacgaagcgcgaacggtcgctcaggtcgtagctgtacatcttggcgccgctgttgcgcgcggaggtatgcacgcttttgccgtcgaagcaggtcgcgtagtagaacggcgtggtgcccacgatggaatcgagcaccttggggttgagcgggtcggagatgtccaggctcgcgaaaccgccgttgctttccatggcggtcaacaccatgtggttgcccatcgtgaagatcgggccgacgcgaaagccgccgagttcgccggtgggcacagggttgggcttgccggcgccgcggttcgcaaccacggcgttcgcggggtccctcgcatcgacgatgaacatgccccggcccgccgatgccacatacaggtagggcgcctgccaccaaagctgccaggccacgttctcgtagtcgccggcgttgacgccgggcagtgccagcttcttcacctgcttgatgtcgttgatgtcggtgaagtcccagaactcgacgccgttgatgctcggcagcaccacgtaggtcttgccgccgatcttcgcggtgccgaaggagtgcgtttcgcggaactcctgggtgcggccttcgggctcgtagatcttcttgacgagctggatctggcgcgggttcgacacgtcgtacagcaggaagccgcccgggccgaggccgctgtccggcgcgaaggaggtgaggaagtagccgttgaccatgatgcccgcgttcatgccgtagtccttgcggcccgggtaagtggcgggtacctcgcgcgactcgtaggcgctgctgtgcgccggatcgagcgggtgcgcggcgctggtgatcatcgacaccggcttgaacagttccgccgaggtgtaggtgaggttgcccaggcccggcccctgcagcgggagcgggtccgcgacggcttcggaaaccgccgtcgccatgttgctcagggtcgtcatcggactgaccccggtgatcgccgcatgcgtcagcaatgtgacgagcggggccaggaacgccatcaggaaataccggatcttcatcgtcgcctccaggttgttagaagttcgcagggcaacccattcctcgaccgttctccgatgcgcgcgcaggacgcaccccggcaggcgacgggtccatcgcctgccgtgctgacttcttgttgtgttcttgcgccggcgcttttctttgtcttagttggcgccgctcgattcgtagagagcccaggccgcctcggcactcgcaccgcggtggatcatggccatcagcgcactcaccaccgccgaaggattcgcgtgctggtagacgttgcgcccgtacaccatgccgacggcgccctggtccatcagcacgcgcgaacgcgcgaacacctgctgcaggtcttcgcgccccccgccgcgcacgagcacggggcagcgcgcggcctgcaccacgcggtggaagtcggtggggtcgctggtcggatcggccttgacgatgtcggcgcccatctcgcgcgcgaggcgcaccagcgtgacgattttttcggcgtcgccgtcgacctggtagcggctgccgggggtgggcgattgcatcaccagcggctcgatcatcagcggcatgccatagcggtcgcagtcggcgcgcacgcgcgcgatgttctgcacgcactggcggaacagatcgggctcgttcggcagcatgaaaagattcacgacgacgcaggccgcgtcgcgctgcacggcgggcaacaccgggtcgtgctcgttctgcagcacggcccacatcacgcgatgcgcggtggcgttgtaggggttgcccatgtcgatgcgcatcacgagcgcgggcttgtcgcggccagggcgctgctgcagcaggtcggcctggccgtagttgagctggatggcatcggggccggcgggcacgagcttgtcgatgacctcgggcatgtcttccagcccgttgaggaacgagggctcgttgcacaccccgtggtcgagcgcaatgtccaggcagcggccgttgttcagcagccggttgagccgcgcgtctttgtccttcgacatttggaaagaactccttgttgggatcggaaatgacaggggtgtcaggcgagattgccgagatggcgctttgccgcggcgtcgatcagccgcagggcgtcgtctcccagctggacggcaccggcgccggcgttctcgatcgcctgctggcgcacgcgcgcgccgcacagcgccaccgagacggtgccgctggcgatggtccacgcgatcatcagttgaccgaacgagcaacccagctgcgtgcgcagcgggtcgagctcttcgaagaaacccttgagcctggagcggttggcttcgctgaagcgcgggttggccgcgcgctggtcgtcgcccttgaattcgcgtccgggatcgatcggaccggcgagcaggcccagcgccagcgacgaatagcccagcaccgccaccttgtattcgctgcacaggggagccagagtctcttcgatctcgcggtcgatcaggctgtagcgctcctgcgccgcatcgacagggccgtagcgcaggtattcggtgagcgtttcggggctgacgttgctcacgccgatggcgcggatctttccctgcttcttgagctcgagcagcgcgtccatggtctcggccacgggcgtggtgctgtcctgccagtgcgtgatgtagagatcgatgtagtcggtctgcaggcgcttgaggctctcttcgcattcatggaagatcgattcacggcctaggaagcggtgcaccgggtgaccgtcttcttcgaagaagtgcgtgccttgccgggtgtgccagaccaggccgcatttggtggcaatcacggcttcctggcggcgccccttgagtgcggtgcccacgatgctttcggagcggccgaggccgtaggccggtgcggtgtcgatcaggttcacgcccgcgtccagcgaggcctggatggcctccacggccgccgcgttgtcgccgccgccccacatccatccgcccatggcccaggtgcccaggccgatggccgagcattcgatgcccgacgggcccagcgttgtcttcttcatcatcatcatcgcgttgtctttctcgtgttcaggaggtggtcgatggtcacggccgcgagcaggatcaggcccttgatcacgtcctgccagtagggcgatacgtccagcaggatcagcgagctggtcaccaccgacagcagtgccaggcccagcaccgcgcccagcaccgtgccggagccgcccttgaggctcgcgccgccgatcaccgcggcggcaatcacgttgagttccatgcccatgccgaaggtgggcgtggccgcgccgaagcgggccgtgtagatcacgccggccaagcccgccgaagccgagcacagcaccgtgacccagaacttgacgcggcccacgcgaatgcccgaatacagcgcggccttctcgttgctgccggtgtagaacacgcgccgcagcaaggtcgatcggcgcagcacgaagtcgctcacgatgacgatcgccacgaagatcaggatcaccgctggaatgccgaacagcgtgccctgcccgatgaacttgaattcggccggcagcgagaacagcgactgcggcgtgccctgcgtgagcgcaaggcagagcccgcgcacgatcaccatgaaggccagcgaggcaatgaagtggttcaggccgatgcgcgtgacgcagccgccgatcatcgcgccgacgagcccgctcgcgccgatggccaccaggctcgcgagccacgggtccacgcccatcagaaagagcttgcccgttaccaccatcgcgaagcagaccaccgagcccaccgaaagatcgatgccgccgacgatcagcagaatggtcatgcccaccaccacgatgccttcgatggagaaggacagcagcatcgcgcggatgttgtcccaggtgaggaagtagggcgacgcgaagctcatcgccacgcacagcaccgcgatgatgagaagcagcccggcttcccgcatgctcgtgagcttgttggcgggcttcacggggccgccgcctgactggcgcggtggatggcccgcatcgagttctgccgggtagttcatgctgtttcctgttcgcagagtccggaggccagccgcagcagggcttcctccgtcatttcgttggaattcaattcgccggccagccggccgtcgcggatcaccagcgcgcggtcgcacaggccgatgatctcgggcagctccgaagagatcacgatcacgcccacaccctggttcgcgagctcgcgcaggatgtgatggatctcggacttggcacccacgtcgacaccgcgcgtgggctcgtccatcagcagcaccttggggttggtggccagcagcttggcaatggccaccttctgctggttgccgcccgacaggctcgacacctcgatggccacgccgtccgacttgaggttgagcttggcgcccagttcgcgcgccaggcggtgttcggccgagcgctgcagcaggccccagccggagctcacgcgccgcagcgccatcgacgagatgttctgtgcgatcggcaggtcgagatacacgcccgcagccttgcggtcttcgctgagataggcgatgccctcgcgcagcgcatcgctgtacttgcgaatagaaagcgccttgccgtgcaggcgcaccgtgccgcgcgtggcggcgcgcaggccgcacatggtctcggccagttcgctgcggccggcgcccatgagcccggcaatgccgaggatctcgccgcgcttcagcgcaaacgagatgccgtgcacgcgctcgccatcggcgatgtcgctcacctcgagcaccgggccggccgattcggcgggctcttgcttgggtgggtagtagttgccaagctcgcgtcccaccatgcggcgaaccagctcgtcggcggtcatgccggccagcgggccgcagtgcacgttgcggccatcgcgcagcacggtgacccggtcgccgtgcgtgaagatctccgccatgcggtggctgatgtagatgatgccgatgccctgcgccttcaggtcgtgcagcacgcggaagagggcggccgattcgttgtcggtcagcgcggccgtgggctcgtcgaggatcagcaccttgcagtccagcgtgagcgccttggcaatctccaccagctgctggctcgagatgctcagctcgcgcacgggcgcgctcgggtcgatgtcctgccccagccgcgccagcaccttggcggcgcgcgcgttcaggctggcgtagttcatccaggcctctttgccggcgttgatctccggcatgaagatgttctcggccacggtggcgtcggcgcacagcgcgatctcctggtgcaccaggccgatgcccaggcgcatggcgtgcgccgggccgtcgatgaccactttctcgccgttcagcacgatgtcgccttcgtcggggcgatggatgccgtcgatgatgttcatcagcgtcgacttgcccgcgccgttctcgccgcacagggcgtggatctcgccagcatgcagcgagaagtccacgcccgagagcgcgcgcgaagcgccgaagcgcttgctgatgccgcgaagttcgagcaaggtgctcactcgccgattcccttggtgccgcggcgggcgagatacttgtcccagtagaagtcgtcggcgttggccttgctgaccaccgacaggccgttgtccaggaagggcaccgacatgggattggtgccgttgcgcttggcgtcgttcatcgggtcgatgagcgaggggttcttggccagaaacagcatcatcatgcccatgtagccctgcatgccctggttggggttgatggcgccgaacacgtcgccggccttgatcatgtccaggatcttggcgttcacgtcgcagcacatcacgcggatgttcttcttcgattcgatcttggcctgcgcggcacccagggccgagttggcttcgggcatgaacagcgcgcccaggttcgggttggcctgcgccaggctcagcaccgcctggtaggccttgctcgggtcctggttgctggcggcgcggccgaccagcttcatgcccgcgtgcttggtcttcatgcggttgacgaaggccgcgatgcgccggtcgtggttgtcctggccggggttctcgaggacggcgtattcgcccttgccgcccagcgccgcggcaatcgcgtcggccgcctgcgtgccctcgcggtcgttgtccgaggtgacgaaggaggcgcgcttcgagttgggcgaatcggccgcgaaggtcacgaccggaatgcccatggccactgcccggttgatcggctcgatgaacgggtcggggttcatcgggtgcagcaggatgcccgcgggcttgcgcgccagctcctgctcgaacgaggccagctgtttgttgacgtcgtactcgggcgtgccggtgtagcgcgtgcgcacccccagcgtgcggccgagttgcttcatcatttcgtagaccggaaaccagtattcgacgccagacaccatcacgttcatcacgtagacgtcgctggcgttgccgcgcaatccggtggcggcggccgtgggggtggactgcgcaaatgcgctggtgccggccaggccgataccggcggctgcagcggacttcaggaaatttcgcctcatcttgtgtctcctcgcgttgactggcagagcttgcgacctgctttgcgggcagatcttcgggacctcattgtcacgacagttgttatgacaggtagaatgtaatcgcgggttgtttgccgcgataactaggggaaacgctactggcgagctgctttcaactcgccgaagctgttatgacatgaagccaaacatattgatcggcgtcgacatgggctcgagcagcctgaaggcgctggccctcgaagccggcagcggccgcaccattgccttgtcccgcatgcccctgccgcacgaccgcctgcccggtggcggctgcgaagtgggagcgacggcgatccgcgccgcgctgacccacgtgctgcgcgatgttgccaaccagctgggcccgcgcacggccgaggttcgtgccatggcctgcaccgggcacggcgccggcctctacgcgctagacgccaatgaccagctcgtgggcggccgtgccgtcgcctcgaccgaccagcgcgccgatgcccgtgcgcgcgccctggcggcgagccacggcgccaggctgttcgaagaggtgggctgcagtccctggcccgggcagcccacggtcattacggccgagctgctgggcgccgatgccgtgcagcgcggcgaactgcgccgcctgctgttcgccaaggactacctcggctttcttctgaccggcgagatcgccaccgatgccagcgatgcgagcaccgccggcctggtgtctctcgccaccggcacctggtcgcaggcggccttcgacgcgtcgggccttgccgagcttgggccgcatgctttcggtccgatcgtgcccagcggcagcgtgatcggaacgctgcggccttccgaggccgcgctgtgcggattgcctgccggcattccggtggcgatgggcgcgatcgacctgcttgcatcgatgaccgcgatctgcgcggaagggcgtggccgcgcggtgtcggtgttcggcacctggtgcgtgaacgcggtcatcgggcctgtgatggagcccaagccggccgtcgcctccatcgtgaattttggccgcacgcacgaacggctctacatggagaacagcccgtcctcgatggccaacatcgcgtggctggccggcgtgctcgcgctgcccgatgcgcgcgcggtggtcgacctggccatgacggtgccgctgggcgccagcggcctgcgcttcctgcctttcgtcaacggcggtggcggcgtgaccgcgggcttcgtggggctcaagagccaccacacgcgcgccgacatggcgcgcgccgtggtcgatgctgtggcggcgctgcatgcgcggcacatggcgcgccttgccgcagccggcctcgcggtgagcgagacgacggtgctcggcggcggcgcgggcgatgcgcgcctcgtgcgcctgctggcggcctttctcgggcgcccggtcgagcgctgcgccgacgacgagaccggcgcgcgcggcgccgcgctctacgccgccatgtcgcagggcttcgatgacgcagcgccgggcagtgccctgctcgcaccctgcgaggtgatcgaacccgacgcacgggacgccagcgcccatgcagatttcaacgccggtttcaacgaactgatcgacagcatgtcacttgtattcacccacatcgcgggcgacgtgaaatgagcgccgcccggccgcccgaaggcgctcgcaccgcagcgcgcagcgcggaggtttttctatgagcgcctggcaacttcccttcgtgcgtccggcttcgctggcggggcgccatttctcgaccgtcatcgtgggcgccggcatcaacggcgtcggcgtgttccgcgatctttcgctgcagcgcgtcgattgcctcatcgtcgacaagggcgacttcggcgccggcgccagcagcgcgccctcgcgcatgatccacggcggcctgcgctacctggagaacggcagcttctcgctcgtggccgaggccacgcgcgagcgcaacctgctgctgcgcaacgcgccgcacctggtgcgcccactcaagacggtggtgccgcttgcgaatttcttcggcggcctgatgagcagcgcgctcaagttcttcggccgcacgccgccgcagcgcacgcgcggcctgctggccgtggcgctgggcttgcggctctacgacctgctgggccgccgccagcgcgtgatgcctggccaccgcatcagccgcgtgccgtcggcggaccgcggcctgttccgcgcggccatccgctggaccgccaccttcttcgatgcctggatcagccatcccgagtggctcatcctcgaactgataggcgatggctgccgcgaccagccgcgctcggcggccgcgaactactgccgcgtgatgggctgcgccggcaacatcctcacgctgcgcgacgaaatcaccggcatgctcgttcgcgtcacggcagacaccgtggtgaacgccaccggcgcctggctcgaccgcagcgctgcggtgctcggcggcgcgggcccgcgcgtgatgggcaccaagggatcgcacctagtgctcgaccatcccgcgctgcgcgatgcgctcgatggccgcatggcctacttcgaggcggtcgacggccgcgtctgcatcgtctatccgtttctcgaccgcgtgctggttggctccaccgacatcccggtcgaagacccggatcagatcgtcaccgagccggccgaggtcgactatctgatcgacgtgctgcgcgaggtcttcccgaacatggccttcgggcgcggcgacgtggtctacacctatgtcggcgtgcggccgctcgcgcgttcggatgccgacaagccgggccagatttcgcgcgaccattcggtggtggtcgatccgccgaacgccacgcgggacattgccatcgtcggactcgtcggcggcaagtggaccacctttcgctcgctggccgaagaggctaccaacgaagtgctgcagctgctgggccgctcgcgcaccgcatcgacagagctgctgcccatcggcggcggcgccgagctgccggccgatgcggcggcgaccgagcgctttgccgacaagatggccgccgcctccggcatgagccgtgcacgcgcgctggccttgctgggccgctacggctccaaggcattgccgctcgcgcagcgcctcgcggcctcgggcgacgtgcccctgcaacacgcgccggactattcggccgccgagctctcgtacctgtgcctcgaaaccggcgtggtgcatctcgacgacctcgtggtccgccgcacgctgctggccattcgcggcctcgtgaccgatgccgcgctgtccgaaattgcggcagtggcggccgaggcgctgggctgggacgcggtgcgtgcgcacaacgaactctgcgcctgcgccaccgcgctgcgggaccggcacggcgtccggctccagccggcggcggccggcgaggaaccctctttcaatgcatcattgatggccagctcagtccttggccaggcttaaaaagtgaacagtcccaacgagatgtcgaccgtgctcgaccgcaattccgaatcaccgctgtgggcccagttccgcgatgccattcgcctgcagatactgcagggcgcgctgcccatcggcgccaagctgccctccgaggcggagctcggcgaacagttcggcatctcgcgcatcgtggtgcgggaagccctggccgacctggtgcgcaacaacctcatctacaagatcaagggccgtggcgccttcgtctcggcacgcgaacgcgacgaggatttcgtttccaccgtgctgggcttctccgacgaaatggaacgcaagggccgctcggtgcgcacgcagatcatcacccaggagttgcgcacccccaccgagcacgaggccgcatcgctaggcctggccgacgacacgcagcaggtggtggcgctcaagcgcctgcgcagtgtcgacggcgagctgcgcctgctggtcgagaccgtggtgccggccgacctggcgccgggcctgcaccgcgcgcggctggaagaccgctcgctctacgacgtgctgcgccggcaatacggcctgcgcctggtgcgcgccgaacgctggatcgacgccgtgctgcccgatgccgaaacctgcaagctgctcgacctgccgcagcccgagccgctgctgcgcatcgagtcgattgcctacggcgccaacggccggccgctggagcactaccgcgcgctgcaccgctgcaagaccagccgcctgcacgtgcagacgacgacctgagcttttcttcttcaggccttggcggagctgctacgcgaaggccacagcacggaggcgatggccaccatcatcagcgcgaccgccacccagtcctgccagtgcacgacttcgccgagccacacggcgccgctgaacacgccgagcacgggaatgaacatcacgctcaaggtcgaagccaccggcggcagcccgcgcgccaggtagaaccaggcggcgtgcgcaaagccgaagatcagcaccgcgttgtagaggatcgagccccaggtcaccgagcccggccaccgccactggccgcgctcgaacagcagcgtgagcaccgtcatcaccacggctgtcatcgccgtcatccagaacgagagcgtgagcgtcgcaagcccgatgcgcgagcggcgcagcagctgcgtgcccagcgcccatgtcgcagccgccaccaatgcgagcgccacatagccgggccggcccgcgaggtcggtgagctcgtgccacagcagcaacccgacgccgatggcgcaagcgcccacgccgatccaggagcgccgcgtgagcacggccgagaacagcaccgcgccgatgacggcggagaacaccggcatcgtgtagcccaggatggccgcgcgcccgcccgaaagcgccttcaccgcaaggatgatgcaggcgtgccagatgaacatgttggtggcgcccagccacaccagctcgggccatgcgcggcgcggcacgcggaacggcaccttcatgatcaccagcgcgaggcccagcaccggcacgccgagccagatcgagagcgcgcggaaggccagcggcggatagtccgccacgccgagcttcatcacgggccagttgagaccccatgcaagggtcaggagaacgagcaggacgaactggcgcggcgtaaaggaaggcatgggccgcgattgtggcgcggcccgcgcattcgtgcagaaggcgggccggctacagcagccgcttgaggtagcgccccgtgtggctcgcctcgttggccgcgatgtcttccggcgtgccttcgcccaccaccgtgccgccgccggcgccgccctcggggcccatgtcgatgagccagtcggccgtcttgatgacgtccaggttgtgctcgatcacgacgatggtgttgcccgcgtcgcgcagctggtgcagcaccttcagcagcagttcgatgtcggcaaagtgcaggcccgtggtcggctcgtcgaggatgtagagcgtgcgtccggtgtcgcgcttgctgagctccagcgcgagcttcacgcgctgcgcctcgccgcccgacagcgtggtggccgactggccgagcttgatgtaggagaggcccacgtcgagcagcgtgcggagcttgcgctcgatggtcggcacggccttcaaaaattcgtgcgcggtctcgaccgtcatctcgaggatctgggcgatgttcttgcccttgtacagcacctcgagcgtctcgcggttgtagcgctggccgtggcacacctcgcagggcacgtacacgtcgggcaggaagtgcatctcgaccttcaccacgccgtcgccctggcaggcctcgcagcgtccgccggccacgttgaagctgaagcgtcccgggccgtagccgcgctcgcgcgcggtgttggtctcggccatcagctcgcggatcggcgtaaagaggcccgtgtaggtggccgggttgctgcgcggcgtgcggccgatggggctctggtcgacgttgatgaccttgtcgaaatactcgatgccctcgaccgattcgtgcgccgccggttcctcgtgcgcgcggtagagcgtgcgcgccacggcggtgtagagcgtgtcgttcaccagcgtcgacttgcccgagcccgagacgcccgtgacgcaggtcaggaggccgaccggaaaggccacgctcacgttcttcaggttgttgccggtggcgcccaccacgcggatttcctgcaggtcggtctgcgaggccaggtgggccgcttcgcgcgcggcgcgccgttcggccgcggggctctgcggaaaacgcgaggccttcttgccttcgttgaaggcgggcttcttcaccacaggcagccaggcggtgcggcgcttgggcacttcgatcttcttcgcgcccgaaaggtactggccggtcagcgaatcggggttggccgccacctgggcatagctgccctgcgccatcacgcggccgccgtggatgcccgcgccggggcccatgtcgatcacgtggtcggcggcgtggatcatgtcctcgtcatgctcgaccacgatcacgctgttgccgatgtcgcgcaggtgcttcagcgtgccgatgagacggtcgttgtcgcgctggtgcaggccgatgctgggctcgtcgagcacgtacatcacgccggtgaggcccgagccgatctgcgacgccagccggatgcgctgcgcctcgccgcccgagagggtttcggcgctgcggtccaggctcaggtagttcaggcccacgtcgttcaggaacttgagccggaggccgatctcgcgcaccaccttgtcggcgatgtcggccttggcgccgcgcagcttgagcgtctggaaccaggcgagcgaatcgcgcaaggtgaggtggctgagctcgaagatcgccatgcgcggaggctcgccgccgtcggccgggcgagccgactcgtccaccaggaacacgttgcgcgcttcgggccggaggcgcgagccgccgcaatcggggcacggctgcaggttgcgaaagcgcgcgaggtcttcgcgcaccatcaccgaatcggtctcgcggtagcgccgcgccatgttcgggatgatgccctcgaagggatgcttcttcgtgagcttcttgcccgcgaagttgcccgactccatggtgtagttgaacttgatctcttcggccgccgagccctgcagcagcacctgctgcaccgaggcgggcaatgattcgaagggcgcgtcgacgtcgaacttgtagtgcttcgcaacgctctcgatcatgctgaagtagtagccgttgcggcggtcccagcccttgatggcgccgctcgcgagcgagagggtgggaaaggccaccacgcgcgccgggtcgaacacctcgcggtggccgaggccgtcgcagctcgggcaggcgcccacgggcgagttgaacgagaacaggcgcggctccaactccgacagcgagtagtggcagatcgggcaggcgaacttggcgttgaacaggtgctccttgtcggccgcaccttcggcgcccagctcgagcgcgatggcccggccttcggcgagccgcagcgcggcctcgaagctttcggccaagcgctgctgcatgtcgggccgcgcgcgcagccggtcgatcaccacgtcgatgtcgtgcttctcggtcttcttgagcttgggcaggtcgttgtattcgtacgtttgcccgtcgacgcggaagcgcacgtagccggccgcctgcatctcggcgaagagctcgaggaactcgcccttcttctcgcgcgccacgggcgcgaggatcatgaggcgcggctcgtcggggatggcgagcgtggcgtcgaccatctgcgacaccgtctgtgcctgcagcggcaggtgatggtcggggcagtagggcgtgccggcgcgcgcatacagaaggcgcaggtagtcgtggatctcggtcaccgtgcccacggtggagcgcgggttgtggctggtggccttctgctcgatgctgatggcgggcgacaggccctcgatcacgtccacgtcgggcttgtccatgagctgcaggaactgccgcgcataggccgagaggctttcgacgtagcgccgctgcccttcggcatacagcgtgtcgaaggccaggctcgacttgcccgagcccgacaggccggtgatcaccaccagcttgttgcgcggaatgtcgaggtcgacgttcttcaggttgtgcgtgcgcgcaccgcggatgctgatgcgctgctgcgcgagtacggcgccaagataggcgtcgcgttccgggtcttcagtggcgggggatttcaagggttcgatcgtccgagggcaaccgagcatgatagtccgcctgccttttcatggcgagggggcgggttgtggcggttttgacgggcggcgcctcgcgggtgcctgccggctccgcccggcgggtcggcatcgggcacaatctagggttctcttcctcctccttcatctacatatcaggggcagtgcatatggcatcggtcaataaagtcatcgtcgtgggcaacttgggtcgcgatcccgaaatgcgtaccttcccaagcggcgatcaggtcgcaaacgtcaccgtggccaccaccgatcgctggaaagacaagcaaagcggcgaaatgcgcgaagccaccgaatggcaccgcatcgttttcaacggccggctggccgaaatcgccggccagtacctgcgcaagggctcgcaggtgtatgtcgaaggcagcctgcgcacgcgcaagtggaccgacaaggacggcatcgaaaagtacaccaccgaaatccgcgccgaccagatgcagatgctgggcagccgccagggccagggcggcccctcgggcggtcccgaggacgacggcggctactcgcaaggtggtggcggaggcggtggttactcgcaaggcgcgggtggcggcggtggtggtggcggctacgctcctcgtgcaccggccgcggcaccccgcgctccggccgccgcgccgcgccaggcaccggccaaatcgtcgtcgggcttcgacgacatggacgacgatattccgttctgagttgaatcgacccatggctgaagctgttccatcgctgcttcagccgtgcggctcgccgaggacattcccgctcccgctggcgttttcctgaaccggatgcaggccgcgcgccaatgagttccacattcgcgcgtcggctgcacgcgcggctgctcgaacacttctccagctatcgcccggcttctttctgggcgagcggggtgcttcttgtttccgtggcgctgctggtggccatggtggccttctttgccgcgcccggcgtcggagaagagccctcggccatccacatgacgcatgccgactggcaggtggaagaggcaccgggcttccgcgaactgccgctcgccgtgcaaagcgatgccttgccggccacctggcaagccgtcgagctgcccctggctccgcccatcgccctgctgcgccaggccggcggcagcgcatcggcgggcccgacccgcatcacctggctgcggctttcgccgcgcgacttgcccggcacttcggcgccgctcgcgttgtatggcgcgcggatcaagacggacggcaccattgccgtctatgccaacgggcggttggttcatcgcgcccaggtgcggggtccgttgtggaacagcacccgcacgccgttgtggatcttgctgaacaaggcgcccgacggcgagccgctgcgcgagatcctccttcggatggagcacacgcgaggcgcgcaggtggcggtttcatcgctctggctggggcctgccgacgcgctcgaagggcgctatcgaatgcgccagtggctccagcaggacctgccggccatgctcagtacggccttcatggccgtgggcgtgttctcgctcttcgtgtggttcaggcgcagccatgagacgggctacctgctgttcttcaacctcgcgaccacgtccttccttcggggcctgcatttctatgtcgacgttccggttgccaacgactggttcgcctggctgacggtcaactccctgttctggctggtggcggtggtgcatttcgcgctgcggcagttgcatggccgtccgctcaggtggctgagcttcgcggtggtgggctggacggcgttgatcggccttttgacgctgccgggcctggccatattgagaaacacgccgcaggtgacgccgttgatctacatcggcgcggcatcgatgggcgtggccgtggcgctggtcggcggcgtcagcgcctggcgccgatccagcgaagggcggctggtggcggtcggcatcggcgtgtgcgtgctgctgggcgtgtccgactggctgctgcagaacaacttcatcagccccgaaggctggtaccttggcgcctacaccaatgcggccaccttcagcgtcttcggggtgctgatgtaccggcgctacgtcagcgccattgcagaggtggagcgcgtcaacgccagcctggcgcagcgtttgcaggcccgcgaggccgagctcgagctcagccaccagcggctgcgcgaggtcgaaaggctgcagaccatcagcgacgagcgccagcgcctgatgcaggacatgcacgacgggctcggctcctcgctgatcagcgccatccgctcggtggagggcggcggcatgagcggcgacagcgtttcgcagttgctcaagggctgtctcgacgacctgaagctgaccatcgattcgatggagcccctcgaagacgacctgctgctgctgctcgcgacgctgcgctatcggctcgggccgcgtctggagagttcgggtgtcgccttgcgctggaacgtgcaggagcttccggcactggactggctcgaccccacgagcgcgctgcagatcctgcgcatcgtccaggagagcatcgccaacgtgctgcgccatacccgtgccaccgagatccgggtgggcaccgtggcggaggcgtccggtgtgcgcgtgaccatcgaggacaacggccagggcttcgatgtcgacaaggccatgggcgccgccggcgggcggggcatgcagaaccagctgcggcgggcgcaggccatcagtggcgcggtctcgtggcgctcggggccggcgggcacgctgttcacgctgtggttgccgctcaagcgcgaggggcaggcggcgcgggcataggctcgcggctcagcccgcgaggcccacgaacacgttctgcacgtcgtcgttggcgtcgatggcggccaggaagacttcgacttcttccaggtgctcggcgctcaggctggccgggtcgaccgggttcttcggcttgtagcccagcttggccgacagcaccgtgaagccctgggccggcagcgcgcggctcacgaggtccaggtcggtggggtcggtcaggaacacggtggcgccgctttcgctggccggctcgaagtcttgcgcgcccgcctcgatggccgccacttcggcgtcggcatccgggcgcgagggctcggcttcgatcatgccgacgtggtcgaaatcccatgacaccgagcccgaggtgcccagttggcccttgcggaacagaacgcgcatttcaggcgcggtgcggtttacgttgtccgtcaggcattcgaccatcacaggcacctggtgcggcgcaaaaccttcgtagatcacgtgttcgaagtgcaccgcctcgccggtgagcccggcgcctttcttgatggcgcggtccagggtgtccttgggcatcgagaccttgcgggcctgctccacgaccagccgcaggcgcgcattcgaggccggatcggcaccgctgcgcgcggcgaccatgatttccttggccagttttccgaacaggcggcccttggcattggcggccaggtccttgtgttttgctttccactgtgcgcccatggcggatgttccttgtgttgggtatgcggtgtccagcctcgcttggcgccgggccgaagggctggatgaccggtttggggcagctactgtagccggagcgcatgcggacagcagttttttccaagtgctggaggcggggcgcctttacgcttggcttgtcttctcgttccgcaacgtatccaggtcacgcctatgacatctatcgaaacacgacaacagcaacatgcagaactcttccatcggctgcacgccggcccgcgccccttggtgctggtgaacgcctgggacgcggtcagcgcgcgcatcgtcgagcgcgcgggcgcgcaagccatcggcacgaccagcgccggcatcgcctggtcgatgggctatgcggatggcgagcgcatgccgttggacgaactgctcgcggcctgtgcgcgcatctgccgcgtggcgggcgttccggtcaccgtcgacatcgaacgcggttttggcgacagcacccaggccgtgtgcgatgtcgtgcgctcgctggtcgacatgggcgtggcgggcatcaacatcgaagacggcacgctgcctggcacgcgcgatctcgcgccgcccgaaatcctttgcgagcgcatccaggcactgcgcaagacggatgcgcggctgttcatcaatgcgcgcaccgacacctacttcgtcgccaacgacgatcccgcggcgcgctaccaagacacgctgcggcgcgcgcggctctacgcgtcggcgggcgccgacggcatcttcgtgccgggcatggcaagcctggaggagatcgccggccttgcggccgcggtgccgctgcccctgaacgtgtatgccggccacgccaaggcgccatcggtcgaggttctcgccagtgccggcgcgcggcgcatcagcctgggctgcgggcccctgcaggcagcgctcggcgtgctcggccgcattgccgctgaagcgttcgacagcggcggcaacaacagcaacggcgccggctttcgcaccatggccgccgagatgatcccggccggcgagatcaacgggctttttgcgggcgtgcgtcgctgaggcgcggcggccttcattcgcggcgaccgcggcaagggcggcgtttgcgcggtgcaggaacgggagattgtttccattccgtgaacgccgcggttctttttgatgagggtttttacttagatggcggcgcacaattcatctcacagaccggcccccaagccgatctgggtgaacagggccccgagcgaggtggccgccccccaagagggacggtgacccacccaagaccggttcgaaatcatccaaagtcaaaactgaactgaattgaaggaaatcaaaatgaccgtctcgaagatcctctccgccgttgctgttgctctcatggccgttgccggcgccgcccacgctgaaacctacgaaggcgtgcactcactgacggctgccgccagccgcgctgaagtggccagccaagccgtggttgccgcgcacagcgccaacccctatgccaccggcgccaatgcaggcccggcccaagtgttcgtttcgtcgaccagccgtgatgcggtccgcgccgatgccgtggccgctgcccgctccgccgacccgtacgccgaaggcgcttcggctcacgtcgcccccatcgtggccggcacggtggaccgcgccacggtgcgtgccgcagcccgcgctgcagctcgcggtgacgcactgccgctgtaatccgatcggccctggcgctctgcgagcgccaaccctcaagaaggccggccctgcgaaagcggggccggccttttatttgtccattgcccgtgcaggcagcaatcggaggcgcgcgacgaagaagggcacgccgtccccctccgccgggtcgtgcagctcgaccgaccactgcgccgatgcgtcctggctcgcatcgcccagtgcggcgtgcgcgcaaagctcgccggcaaagcgcacccggcctgcgcgtgcggtgtgatcgcaggtcatcacggtttcgtcgcagcattcgtccacccatgtccagccgccctcggggtcgctgcggaccgattgccgcatcagccgcgcgccgatacgttccggcgcggccgtgcgctcgccggcctgcggtgcgggcacggtccccagcagccgcagttcgagcggttcgccgacccgaaagccttcgccgcgctccagcgacaggtcttgcagcgcgatgcgcacccggcggcgctcgcgcagcgtcgtcacgacgaagaccaccgtcaataccgagaagatgccaaacaccggcaggcccaccgccagccagagccacttccatccgccggccagcgcccaggtgatggcgttgaacccgaagagcgcgaagaaagccagcacggccagcgcgaccagccatgcgatccagtcgccggccgaccggcgcacgcgttccgtgacggccggtgcgcccgaggtccattcggctggctgcacctcggccagcggagccgcgccggccatccgcgggtcgggccatggcgaccagaaatccgccggcgcgttgtcgagggaaatccgctggaaatcggtccaggcgggcaggtaggccgtggctgtttcctcgccttccacttccagcgtggtgccttcgaaaccgcgcgggtacacgccggtcgcccggtggtgccgccgctcctgcaggtcgacgatcaaggtgccgccgccgacttccgcggcctggtagcggccgtcggatgagacaaagccatagcccggcgagtgtccggacagatgggcgatcaatgcgacggacggatgaagccgggtcatgaagaagaggcgggaaaggcgccgagcatgccatgcgcggccgtctgataagctgccttcgcccctctccatcgacctgttccttccacccctgtccttgcgaacgcattgcgcatgtcgtccgaagaaaccctgcgccgctggcgcctgatcctcggccgctatgcggcgcaacccctggcgcaaacgcagttttcgtccggcgactggaagctcgaccaggccctcgaatatctctacggccgcgaatacgaaggccgcggcctcgccagatccagcggcggcccgggctcgctcgatcccagccagctgcgcgctgtcgactggctcaaccgttcgcgcaagctctttccgcaagaggtgttcgagcgcatgcagacgcaggccatcgaccgctaccagctcaccgatctgctcgccgacccggccgtgctgcgctcgctcgacgccacgcccgggcttgccaaggcactgctcggcatgcgtgggcggttgtcgggccagatgcgcgatgcggtgcgcgaggtgatccagaagaccgtcgacgagatcacccgcaagctcaagaacgacttcatcaacgcgctcgtcggccggcgcaaccgcatgcggcgctcgcacatcaagagcgcgcagaacttcgatgcgcgcgccaccatcgcggccaacctgaagcactacgacgtcgagcgcaagcagctcgtcatcgagcacccgcgcttcaacgcgcgcgtgaagcgcaacctgccctgggatgtggtgctgtgcgtggaccagagcggctcgatgatggattcggtgatctacagcgccgtcatcgccggcatcatgagttcgctgcccgcggtgcgcgtgaagctcgtggtgttcgacaccgcggtggtcgacctcacgcacatggcgcacgacccggtcgaggtgctgctcacggtgcagctcggcggcggcaccgacatcggccgcgcggtggcgtactgcgagtcgctggtcggcaacccgcagcgcacggtgttcgcgctcatcagcgacttcatggaaggcgccgcgcccggtccgttgctggctgccgtgcagcgcatggcgcaggcacgcgtcaggctgctcggcctggccgcgctcgacgagtcggccaacccggtgtacgaccggcagatggcgcagcggctggccgacaagggcatgcacgtggcggccctcacgcccacgcattttgcgcactggctcgccgaggtcatgaactgatggcctggcacgacggctaccgcgcctacgacgacgacacgctggccacgctcgcgaaccccggcctgctgcggcgcgccgcaaaggacgtggaggcgggcaaggtcggatgggcagaagagggcgccgaccgtggtgtggtgatggccgatagccagcgggtgcagctcgatgcgcgcggcccgcagcaggcgcgctgcgactgccaggcgccgggcatctgcaagcacatcctcggcgcggccctgtggctgcgtgcgctggagccggtggcatcgggcgatgcggccggggcgtccgcaacccgggaggaagaaaagccaacgcccgccgctcctgacccgctcgcggaaatcctcgcgctcgacgccgccgcgctcttcaaggccgcgggcgtggccgccgtgcgccgtgccgcggccgccgtcagcagcgtcgtcgaatggcgggtgcagggcggggcgctcgtcatggacctgcccgagctcggcgcctcgtgccgctgggtggcgggcgcgggctacgcgggcatggtgtccgaggtgccggccgccgagcgcaaggctgtgcacctgatcgccatcgccgcgctgcgcagcgcgcacggccagcccttcgcatggcctgaaggcgcgcggcccgcgccggtcgaagacaccgcgcgcctcggcgaccgcgagcgggccttcctgctgcaagtcgaatcgatgctgcaggagctgttgacgggcggcctctcgcatgtgagcgaactgacctcggcgcgcttgctggcgctcaacatgtccgcgcgcggcgagggcctgccgcgtctcgcggccttgctgcgcaacctcggcggcacggtcgatctgctggtgcgccgcgaccaccgcgccgaagagcgcgatgccttcgcgctcatggcgcgcatccatgcgctgtgcgcggcgctcgcgcgggccgaaggcgatcttgccgtggccttgcgcggccggctgcgccgcgatttcgacgagtcctccgcgctcgagctgctgccgctcggcgcccactggtggcagacgcgcggcggcgcgcgtgggctcaccgtggccttctgggacctggccggcgcgcgcgtgctgcaggcttcgctggcgcggcccgatggcagcgacaccgccttcacgcgcagcggcgcatggtctgtgaacgcgctgtggtcgggcgcgggcgccgcgcaaagcgtgtgcgaagccgctctgcggctcgaacaacctcgcctcgccgaagacggccgcctggcgctcggtggcgccacgcgcgcccagcccttgcccgcatggacggccgacgatccgcggctgcaggccatcggctgcggcaactggtccgaactcggcgagcgcctgcgcgccgccaccggccttgcggccgagcccttcgatgcggtgctgctgcgccccgccggtacccgcccgcccgtgctcgatgaagcgcagcagcggctcgactggctggtgcaggacgatgcgggccagtggctgcggctgggcattccggtcgggcccgagcaccggcagcgcgtcgacagcctcgaccgcttcaccgcgcgccgcgcgccggtgcatgcggtgctggtgcgcatcgagcgctccgccgcgaacaccgagctgatgcccatcgccgtgctgagcagcgatgcgaagaagaagctgcaggcggtgtcgctcgacttcgcccaggaggccgcgcgcaccacctcgctggccaaccgcatcctgcgcttgttcgaggcacgccagcagcggcaggcggcgcccgtggccgcgcccacgctgtcggcgcgcctgctcgcgccggtgatcgacgtggccgagacgcaggccgcgaccggccgcatggcgttgacggcgccgcaacggcaacgcctgcatgacgtgctcgaccgcgccggctcggtcggcctcgaggtgttgtcgaatgccctgcgcgcgcacctggccgcgccggccgcggtgccgctgctgaagctgggctttctctgccagctgctcggcgagctcgacgggctctcggaactcaaggaagtgcagctggcttagaacctttggcttcggttgtttccacagggcgggcggtggtcaaagcgtcatcgccaactgccaaaatcgtcggttgctttgaggagaacgcatgggatttctggacaagatcttgggcgccgtcacgggcggcgccagccccagggccgagggaggcctcacgcgcgagcaagcgagtctgctggagcaggccgtcgcatgtttcgagaaagcaggcaaggaactgccggccaaggccaccgcattcctggtcgaaggcacgcaggaaaccgtgctgctcgacctgcaggcggcccgcgccttcgaacccggcacgctgctcggcgatcccggccgcctgcgctggggcttcagcaaccaccagaacaagccgttggagaagatcggcaaccagagcctcgagcagcgcggccgcttctacgccagcgtgagcgccgagacgccgccgctcaatgcgctggtgcggctgggcaagctgctcgcggcggccgatggcggccagtcgctcgagcacccgggcgcggccgtgcccgactggctccagtacctcgtcaacgacgcggtgttcgcgagcttcaacaagggcggctccaacaccagcgaccgcgaccttgccaagcaccgtcccgcatggaacgtgcatctcattgcagccctgctcgcgcatgaagggctcgatgcgaagctcgccctgcaggaagtcttcgagcgcaagggcctcgacagctggtaccacgaccggctcgacggtctcgtcgaagcctccgccgtggccgactacatgcgcagccaccgtgaagtcaccgaggcgctgcccgcccagctctcggctgcgggccgcgtgctgctggccaagcgcatcggcaaggacaagacgctgctgaacgacttcgcgccgctgttcgttcgcctggccatcgatggcagcaagacggtgcgcgccgaggctacgccgcaccttgaaggcattgccgaggcgcagcggctcgaactgctggggcagttgctgaaagacggcgacaccattcagcgcacgcaagcggccgagctgctcgcgcgcctgcccggcgacgccgctcgcgccctgcttgccgcggccgccgaaaccgagaccagcaaggccgtgcagcaggccatccgctcggccatgtcgcggctcgacgcggccggcgatgcgggcgagctcgaactgcccgagccgccggcctggcagccgttcgaagacctgccgctcggcgaagaggccgtgcaactgctcatcgccaaccgcatcgaactgctcgagaagagccgcatcgcggccgaggccgagatcgaggagaacaaggcctccaagcaaacgtacaagtacaagtggcgccaggacagctatgccggccacaagaagctcaccgacgaggacatgcgcgtggccgtgcgagtgctcaacggccagggcagcaagcacgaccagaaccgcgtgaagaacagccagcttcagcaggtcgtgagtttcggcaaccgcctgcaggcgctgccgggctttggcatgccgcacctgatccgctggctggccgtgtcgcgccactggaccagcttctggttcgacgacggcttccacaagtggctcggccgccaacccgtgggctcggtcgacctgcgcgcgctggccgagctgctgaagcgttccggcatgccgatcgacgacgtggcccacaccgcgcttttccagtactggaaccaggcctcggcggtcgaggtgttgccggccgaccgcgtgtggccttttttcgcggaacaccccgagtacatcgacgaaggcctgggcctcgtcgccccgcccaagcgcgaaggccgccagacccagctcgacctgaacgccacgctgcgcacgctggccatcttcccgaccgtgcaggcgcgctggctgccgcgcgtgatggaactggccctcggcgaaggcaagacgcaccgcgccgccgcgcaaaaggcgctgtcgatgctgccggacatcggccggcgcgtggtcgagtcgctcgacgccaccaagagcgaggtgcgcatcgaggctgccaactggctggccgaactcaaatacgccgaggccgtgcccgccatcaccaagggcctggagaaggaaacgcgcgagaccgtgcgcgccgcctatctcacggcgctcgaagcgctgggcgacgacatctcgccgcgcctcgcgcccgcgatcctgctggccgaggcgaagaagggcctgaaggccaagccgccggccggcctcgcgtggttctcgctcgatgcgctgcccgcctgcaaatggcaggacggcagcgcggtcgagcccgagatcatgcgctggtgggtggtgctcgcctgcaagctcaaggagccgggcggcaatgcgctgctcacgcgctacctcggcttgctcgatgcggtcagccgccaggccatcggcagcctggtgctgcgccaattcatcgcgcaggacacacgccacccctcgctcgacgaaggcatcgcgcacgccaacgccaacgcgccgcagcgctaccagggcaaccagcagcgctaccagaacgccaaggccgagcacaagcagtactacgagaccgacttccagaagacgcaggagcaggtcttcgaggaatgcaagcgcgaaaagatgagcgaatacctcggcagcgccatcggcgagaagggcatcctggccctcaccgcgcacgcgccgggccacgaggtggtcacgctgctgcagcagtacatgcgcgaccactaccagcgccgctcgcagatcgaagccatgctcgaaggcgtggcgccgggcaacgacccggtggtgatccagctgctgctgggcatctcgcgccgctaccgcaccgcctcggtccaggagaaggcgcgcgcgctggtgcagcaaattgccgaccgcaacggctggacgcaagaccagctggccgaccgcaccattcccaccgcgggcctggacgacaccggcaagctcgaactcgcgtacggcgaccgtgtcttcaccgtggtgctcgacgccgcgatgaagcccgaactgcgcaaccccgagggcaaggtcgtcaaggcgctgcccgagccgcgccagaacgacgaccccgcgctcatcaaggacgcgaaggcgcaattctcgaccagcaagaaagagctcaagcaggtcatcgacctgcagaccgcgcgcctgttcgaggccatgtgcaccggccgcgtctggccccaggccgagtggcgcgaatacctgcaccggcacccgattgccgggcggctgatacagcggctggtgtggctcgaactggacgcggaaggcgtggttcgcggcagcttccgccccaccgaggacggcagcctgatcgacacccaggacgacgaggtcgagctcgcggccgacagccagctgcgtctgggccatgcctcgctggtcgacgaggccacggcgaccgcctggaacaagcacttcaaggactacaagctcgcgccgctcttcgcgcagatgacacgcaagccgccggccgttgccttcaccgacgacaagggccatccggtgagcgagatcaaggaccgacttggctggatcagcgacaccttcacgctgcgcggcagcttcgccaagctcggttaccagcgtgcgcaggccgaggacggcggcttcttctaccagtacaccaaggagttctcgtcggccggcgtgcgcgtggccatcgacttttccggcaacaccctgccggaagaaaacgtgcccgccgcgctcaagaccctgggcttcgaggacatgaagacccgcggctacggcgaccgggcgctgccgctctcgggcgtgccgccggtgctcctggccgaggcctatgcagactacctggccattgcccaggcctgcgccggattcgacgcggactgggaaaagaagatgccatggtaggccggcttcatgctttcgtcttactgtgccgttgcggtgcggacacgcgaaaatcaggcgggcgctcctgccacggaaaagaaagcatgattcgttgccgctgaggcggcaaccctacacgcatggctctcacactcgaccctgaagatacgcgcggacgcatccacgatctcgtgtggggcggcttctattccgatgccgatgtcgagtggatgatcaccgatgagtacctcgaccccgacgagctcacgagcgaggaccgggcctgggtaaaggccgaagccgggcgcatctgcgccgccaagcgcaccgccgaggccgggtggccagcgcaaacggagtacgaccggctcgaagccgtgttcgcccagctgcgcggcgaaaagatcatcgcgctgcaccacgccggcaacacgctgtccgacggccatgacgatgtgcgcgagcagtggcgcgctgccgggcgtcttgcttccggcatccgcggctgctgcttctatcactcgcaggacctcgacgcggcggtacgcaccggccggctgcatctggcgttcagcggcggcatgattgcgcagatcgagcagcgcgaggccaacaccgtggtggtcggccaccgcatcgtcgagttgctgcgcgcggccggcttcgaggcgcgctggagcggcaacatcaacgagcgcatcgaggccgacctcggccaatggcgcaagcgaagcccgtcggtgtgagcgccggggcctggcagccgccgcgccgcatcgatgccatcgacttctggctgcgttcccgactgctggccaccgcccatgcgctgcgcgaggcgctgcaggcctcactcgccgccacaccagcggctacgatcgccaagggctgacccgcagcgaaaaaccagcagcaacaacaccatgagcaccggcacttcaccgtcttcctcccccgctacccaggccgtgcgcctggcccccgaggcacgctatgcggacgaactcgcgcgcctgcacgcggccgacgccgatgcgcggcccaccggatggaagctctcgccgcgcgcggtgcggcgcttcatcctcggcgacgagaaactgcgggtgagccgcaagttctacggcgacgatccgttggtggaccgtgccatcgtcacgctcatgggccatcaggggctgatgctcgtgggcgagccgggcaccgcgaagtcgttgctctcggaactgctcgcggccgcgatcagcggcgattcgggtctcacggtgcagggcacggccggcaccaccgaagaccacatcaaatacagctggaactacgcgttgctgctggccgaagggccgagccagcgcgcgctggtgccgtcgccgctctaccaggcgatgcgcgcgggcaagctggtgcgcttcgaggaaatcacgcgctgcccgcccgagatccaggacgtgttgatctcgctgatgagcgacaagcagctcatgattcccgagctgggcgacgacgcgcggctgtacgcccagcgcggcttcaacatcatcgcgaccgccaacctgcgcgaccgcggcgtgcacgagatgtcgtcggcactcaagcgccgcttcaacttcgaaacggtgaagccgatccgcgaccatgccttcgaggtcgaactggtgatggcgcagctgcagcgcgaactggacggcggcggcgagtcgccggtcgatgtgccgcgcgacgtggtggcgctgctggtcaccaccttccaggagctgcgcgcgggccagacgcaggacggtacggccatcaagggcctcgatgccgtgatgtccaccgccgaggccgtgaacgtggcctacgcggcggccctgcaggcgcgccatttcaacgacggcaagctcaccgcccgcgagatcgcgggccagctgcagggcgtggtgctgaaggacagcaccgacgacgtgaagcgcgtgcgccactacttcgacaccgtggtgcgcgagcgcggcaagcgcgacgcgcaatggaagacctttcacgacgcggcgcgcgcgctgtggcaatagagccggctcaggcgcttcccgccgcgctggaggcctcgcgcggccggctgttcggcgaggagggcgtgttcttcgtgccggtgcggcatcacagcccggcctgcgccttcgcattgcgcgggctgctgcgcgagatcaagccggcggccgtgctgatcgaggggccggacgacctggctgcgctgatgccgctgctgctgcatgaacagaccaaggcccctgtcgcctggctgtgccagagcacgcgccaggtgccggtcgacgacgccgatgcggaagagaaaacgcgcaccgaatcgcgcacatccttctttccgttctgcgactacagccccgagtggatcgccgtgcgcgaaggcgcggcgctcggcgcgcggctcgggctgatcgatcttccctggagcgacaaggcctggcaccgcgatgacgacgagagcgatgagggcgacgcacgcgatgccgcgcgcagcttgatggaagaacgccacttcgcacacagccgctacctgaacgcgatggtctcgcagctcggctgcgccgaccaccaggagctgtgggaccggctcttcgaactgcgcaccacggccgcgctcggcgactggcgcgccttcttctccgatgtgttcagctggtgcgccgtggcgcggctcgactacgagcccgaggtgctcgaggccgaactgagcctgccgcgcgagcgccacatggcggcgcacattcgccgctggcgcaacgaggtcgaggggccgatcgtggtcgtcaccggcggcttccacacgctcgaactcgtcgaccagtggcagaaggccaaaccctcgaaggcacccgccggcaaggatgcgccggccgatgcctggctgatccgctacagcttcgagcggctcgacgcgctcaacggctatgcctcgggcatgccctcgcccggctactaccagcaggtgtgggaacgcctcgaagccggagacgccgatccgttcaccgcggtgacgctcgacagcctgacccgcttcgcgcgccggacccgcacgcaggaccaggtcgatgcggtgtccaccgcgctggtgcaggccgccgccgcgcaggccatgcggctcgcggcgctgcgcggcaatgcggggccgggccgccaggacctgctcgatgcgatccgctcctgcttcatcaagggtgcgatcgacgaaggcacgcgcggcttcacggccgacctgcgcaatttcctgagcggcacgcgcatgggcgacgtgccgccatcggccggctcgccgccgctgatcgaggatgcgcggcggctcgcgcgccaggccggcgtgcggctggacgacagcaccgcacgcgtggcgcggctggacctttatcgcaagccttcgcaccgcgagcgcagccgcttcttccatgccatggcgtacctcgatgcggggctcggtacctggctcgcggggccggattttcttggcaacagccgcctgcacctgctgttcgaagagtggcgtgccgcctggtcgccgctggtggaggcgcggctgatcgagctcgcagccgacggcgcgagcgtggaggccgtgtgcatggccaagttgcgcaaggaagaaatcgcgctctccgaccagggccgtggacgcagcgcgagcgcggcggtgacgctgttgctgcgcgcctgcctggtcgggctgcagtcgcgcctgcctcaactgctttcgatgctttccacgcacctcgacgaagatgccgcgctcggctcggtggtcgactgcgggcatcggctcgtcacgctgtggcgtgcgcgagagccgctgggcgtgcagcagcatccgcaactgcgcagcctgctggaacgggtatggcccgcggcgctcttcctgctgcccgatgtgggcgagtgccccgaagagggtgaggccggtgcggtgaagcaactgctctcgctgcgcgagctcgggcgtctgttggcctcgctgcagagcgagctggaagaagccgacggcaatgccgtcgaccttgacctgctgcgtgcgcagctcgagcgcttcgcgaccggcgcgctgaccgcccccgccgtggcgggcgccgcttcggccctgctgtacctcgacgggcactgggacgagcatgcgctcgacaccgtggtgcggcagcgattcggcgcgggcgcagagccgcgcgaagcggtgcgttttctcaatggggtgatggccgccgcgcccgagctgctgctgcgcctgcccgcgctgctcgaaggcctcgacggcctggtgcaaggctgggacgccgaagccttcgtggcgcacctgcccgacctgcgccaggccttcacgcgcctcaagccgcaggagacctccgaccttgccagccgcgtggccgcgctgcacggcatgggcgaggccgagggtgaggcgctctaccaggtgcattacgaaaccaccgagcaagacctgcacgaaggcgcgcagttgcagctcgcacttgccgagtgcctgcgccgcgacgggcttgccgcgtggctggccgccgcggataacaagaagaacacggaaaccgcttcatgaccatcgacctccagacgctcaagtgcggcgagtgcggcagcaacgcgctgaaacgcaccggcctgaaccagtacgcctgccagcactgcgggtcggtgacgctggtggaggacaacgtgtccgaccggctcgaccgcgtgctcgaccaggtgaagaacgcggcgggagagcgcctcgcgcaagagcaggcgctgaagcagaagatggtcatgcgcaatgcgggcatcgccgtggcggcggtgctcggcgtggggctggtggccatggtggcgagcctgatctccgcgcgcgacgagcggccccgagcgcagcccgcaagggcttcggtggccgatcgcacgatcccggtcgacgggctccggctcggcgaaccgcgccaggtgctggtgggcagcggcggctcggcgcaggccaggctgctggtggtggcgcgcaacgaaaccggcaagccgctggagcgcgccaacatcaaggcggtgttctacgacggcgatacccggctcgaagaacgcagcgagtcattgcccatcggcgtgctccagccgggcgagagcgcaccggtgctgatcgatctgccaagagcaacaaccgcaacccgccaggagctgcaggtgcagcgtctctcggcgccgtaccgctcggcggagggggcgcggctggtcttcgagcgcgtgcggctggtgcagcagggcacggacgcggcccggctggtcgggcgcatcgccaatggaaaggacaacggcgccacgctggccggcatcgaagccctggtgacgctgtacgacgacgcgggaaacgtgatcggcatcggccacggctacgcgcaggcgagcgaactgaagcccggcgcacgcacgtcgatggacatcggcattcgccgtttcggccgcagcgcggcggtggccgcgtgggactaccgcatcggctacagcacgctcgaggccgatggcgcgcgcgtggcggtgcagagccccgaccgcgtgatccgtgccgtgggcgcgccggaggttttcaatcccgagctgcgcatgggcaccgaagacctgctggccgacgagagcgagcgcttcgacccggcccagctggagctgctgccgctgatcccggggctcaacacgattcgccagcgcacctacatgaccgagctcgtgaatcgcagcaaggaccagatcgccatcgcccccgcggcggtggtctcgcgcttcgacggcagcaagctcgacggcacgaccgtgctcggcggcccggcgtacctgtatccgggcgagcgctttccggtgcagatcgatccgtcgcgcgccgaccgcatcacgcagacccgcgtcgaatggaaaccgatgcggcgcgcggcgctgcccggcccgcgcacgccgctggaggtcaccatagacagcacccgagccaccacgggcagcgtgctgctcaacttcagccagcgcttttcctacaaggcggtggacatcaagggcagcgtgaagaaccccggcactggcatcgtgcgcaaggcccgcgtatgggtcagcctgcgcgaccgcgagggccggctcaccggcttcaagatggtggagaacctgccggccatcgcccccggcgagagcgcgcctttcgaggtgagcatccagcagcaggcgcgcgactttgcaacagtggaagctgtctaccagagcgcggaatagcctgcacgagcagggatggccggatcacgccatcatccggcccatgattccgttctcgatcctcgatctctcgcccatcaccgaaggcagcgacgccgcgcagtcgttccgcaactcgctctcgctcgcgcagcacggagagaagctgggctaccggcgctactggctggccgagcatcacggcatgccgggcattgccagcgcggccaccgcggtgcttctcgcctacgttggcgctggcacgtcgacgatccgcatcggcgcgggcggcgtgatgctgcccaaccattcgccgctggtgatcgcggagcagttcggcacgctggagtcgctgtacccggggcgcatcgatcttggcctgggccgcgcgcccggctccgaccagcgcaccgcgcgcgccctgcgccgcaatctcgaatccgatgccgaccagtttccgcaggacgtggtcgagctgatggatttcatgtccaagacgccgcagcagcccgtgcgcgcggtgcctggcgcggggctcgaggtgccggtgtggattctcggatcgagcaccttcggcgcgcagctggccgcgcacctgggcttgccctacgcctttgcctcgcacttcgcgccgcagcagctcatgcaggccatccagatctaccgcgagaccttcaagccgtcggcgcaactgcagaaaccgcacgtgatgctgggcttcaacgtgttcgtggccgacaccgacgaagaggccgaatttcgcgccacgtcatggcagcaggccttcgtgaacctgcgcagcggacggccggggcgcttgccgccgcccgtcgaaaactatcggcagaaggtgggcccggcggaaaacgcgctgctcgactcggtgctgtcctgctcggccgtgggttcacccgccaaggtgcgcgaaggcgtgcaggccttcatcgagcgcaccggtgccgacgagctgatgatcacctcgcaggtgttcgaccacgtggcgcggctgcgctcctacgagctgctggccgggctgcgcgggcagggctgattcccccacgccgccgggcctggcgcggggctgggacaatggcgggcttattggtgggcgtatggcagcaaagcaacggatcgtggtgggactgagcggcggggtggattccgccgtgacggcgcacctgctcaagcagcaggggcacgaagtggtcggcatcttcatgaagaactgggaagacgacgacgacagcgagtactgctcgtcgaacatcgacttcgtggacgccgccagcgtggccgacgtgctgggcatcgagatcgagcacgtcaatttcgcggccgactacaaggaccgcgtgttcgccgagttcctgcgcgagtacaaggccggccgcacgcccaaccccgacgtgctgtgcaatgccgagatcaagttcaaggcctttctcgaccacgccatgcgcctgggcgccgagaagatcgcgaccggccactacgcccgcgtgcggctgaacgaagccaccggcaagcacgaactgctcaaggggctcgatccgtccaaggaccagagctacttcctgcaccggctgaaccaggcgcagctgtcgaagacgctgttccccgtgggcgagctgcacaagaccgaggtgcgccgcatcgcggaagaaatcggcctgcccaacgccaagaagaaagattcgaccggcatctgcttcatcggcgagcggccgttccgcgagttcctcaaccgctacatctcgaaggagccggggccgatcagggacgaccgcggccgcaagctcggcgaacaccagggcctgagcttctacacgctgggccagcggcaggggctgggcattggcggcgtcaaggagaagggcgcccagcgcggctcgggcgaccattcgccatggttcgtggcgcgcaaggacgtcgagaaaaacacgctgcgggtggtgcaagggcatgaccacccctggctgctgtcgtccgcgctgacggcaggggacgcgagctgggtctcgggcgaggcgcccgcaccgggcggctacggatccaaggcgcgctaccggcaggccgatgcggcctgccagatggacgagatggaagacgaggcctatgccgcgggggtcttcggccttcgcttcggcgagccccagtgggcggtcacgccgggacaatcggccgtgctttatgacggcgagcgctgcctcggcggcggagtcatcgtctgaccgcctgaaaccggtgcgcggcagccgtcagcgcaccgaatcgtggacgtggatcagatcgagcgggtagcgccgtccggccagatggtcttcgacggactccagcagcagcggactgcggtgccgcggcacgctggcgcggatttcgtcggcgctcatccagacggtgcggacgatgccttcgtcgagggcgcgcccggtttcctgtgggccaagaataccggcaaaggcaaagcgcatgtagatcacatcgtcttcgttccggcccgtccgatggctcgaacgcgccatgtagatgccgatcagcgcggtgggcgtgaaggcgtgggcggtttcctcgagcgtttcgcgggcacacccttcgatgggcgattcaccagggtcgaggtgtcccgccggcgtgttgagcttgaggccctgggccgtcagctcctcgaccagcaggaacttgccgtcctgctcgatcaccgctgccacggtgacgttgggtttccagcggaatttcgtcatatgtcgcgcgggcaagtggggagagagcgattggagacagtatcgctccatagattccccgggtgtcagtcgcgtctgtccggctgtgccggacgacgcagccggctgcgccgcactattgctgtcttgcgtctagcgcgaaaggcattccgccagcgtattggcctcgacggcttccagccggtaacccagcccatagatggccagcagcagaaatccgttctcggggcgcaagcccagcttggttcgaaggcgggacacgtgagtgtccagcgaccgcgaaagggcttccacgccggcgccccacacggcttcgtgcaggtgctcgcgcgagagcatgcggccgaggttctggaacaggaacagggccagttcgtactcgcggttcttcagttcgaccttgacgcccctgaccttgagggtgcgcgcctgcgggtagaagtggtagtcgccgaacacgagctccgcatcgtgctgagacggataggagcggcgcagcaacgcattgacgcgggcctcgagctcgctggcccgaacgggattggtcatgaagtcgtcggcgccggcgttgagcccgtcgaccgcgtcggcatcgtcgtgctggtcggtgacgaaaagaatcggcaagcgactcctgagttcgttgcgtaccgacctcaccacgtcgatgcccgggatgtcgggcaggcgccaatccaggatgaggagatcgaaggtttgccggcgcaagtcctgcaacaggattcgcccttcggtgtaggggtggcattcgtgtccaaaacccgccatggcctggcagagagcctgatcggcctcgtgatcaagtaccgcaatacgcaattccgtgccccttcatgttgacagcctctgcgggccgccgaataaaaggaagtctatcgatctacttgcccgggaaggtcggcgtgcatgcaacaaatgcacgatatcggcgatattcggagaaattaagcgcacttggcgacaaatgaaaaataattgacattcttgcgcggctcgatgcgctgcggtccggcgaatgcatggggcgccgcgcgcggcgggattcggtccgggtttcggcgcccgctagcatttatgtagctataaatgcaatgacggcggtcatcaggaggcgaatcggcatgcagatttaggcgacagtggcatctgtaatcttgctgtaagctctgcccgcgttccgtattgcccttgccctgaggagatctctatgctgataggcgtgcctgccgagacgacggccggcgaaacccgtgtggccgttacgcccgagacggtgaagaaacttgtcgccacggggcacgcggttcgcgtgcagtcgggggcggggattgcggccagcgtcaccgatgccgcctaccaggccgccggtgccgagatcgtcgacggggcaggcgccttcggggccgacatggtgctcaaggtgcgcacgcccggcgaggcggaaaccgcgctcatgaagccgggcaccgtggtcatcggcatgctcaacccgttcgatgcggccggcctgcagcgcctggccggtgccggcctcacggccttcgcgctcgaagccgcgccgcgcaccacccgcgcccagagcatggatgtgctctcatcgcaggccaacatcgccggttacaaggccgtgatgatcgcggccgacaagtaccagcgcttcttccccatgctgatgaccgccgccggcaccgtgaaggcggcgcgcgtcgtcatcctgggcgtcggcgtggcgggcctgcaggccattgccaccgccaagcgcctgggcgccgtcatcgaagcttccgacgtgcgcccgagcgtgaaggagcagatcgaatcgctcggcggcaagttcatcgaggtgtcctacgacaccgacgaagaaaaagaagccgcggtcggcgtcggcggctacgccaagcccatgcccgccagctggctcgcgcgccagcaggtcgaggtggccaagcgcgtggcgctggccgacatcgtcatcagcaccgcactcatcccggggcgcgccgcacccaccctcatcaccgaggacatggtcaagtcgatgaagcccggttcggtgatcgtcgacatcgcggccggcaaggggcccgacgtgaacggagagatgaagggcggcaactgccccttgtcggaagccgacaagaccgtggtgaagcacggcgtgaccatcgtgggcgagaccaatcttgcggcgctggtggcggccgacgcgtcggcgctctatgcgcgcaacgtgctcgacttcctcaagctcatcgtcaccaaggagggcgggctcaagatcgacctcgaggacgacatcgtcgccgcctgccgcgtcgcgcacgacggccaggtcacgaagaaataagccgccaccccccggcactcacgcgaggagaagaacccatggatcccgtttcccacaccgtcatcaacctgatcatcttcgtgctggccatctacgtgggctaccacgtggtgtggaccgtcacgcccgcgctgcacacgccgctgatggccgtgaccaacgccatctcggccatcgtgatcgtgggcgccatgctggcggccgcgctcaccgaaaccgctctgggcaagaccatgggcgtgctcgcggttgcgctcgcggcggtgaacatcttcggcggcttcctcgtcacgcggcgcatgctcgagatgttcaagaaaaaagagaaaaaggccgcacccaaggctgaagcgggagccgcccaatgagcatgaacgtcgtcacgctgctctacctggttgccagcgtctgcttcatccaggccttgaagggcctgtcccatcccaccacgtccatccgcggcaacatgttcggcatggccggcatggccatcgcggtggtgaccaccggcgcgctgatctacaacctggccggcggccacctcatgggcctggcctgggtgctgctggggctggtggtgggcggcggctatggcgcctaccgcgccaagacggtcgagatgaccaagatgcccgagctggtggccttcttccacagcatgatcggcctggcggcggtgttcatcgcggtcgcggccgtggtcgaacccgcggccatgctcgaaggcatcgccaagggcgcgcccattcccaccggcaaccggctcgagctgttcctgggcgcggccatcggcgccatcaccttcagcggctcggtgatcgccttcggcaagctctcgggcacctacaagttccggctgttccagggggcgccggtgcagttcgcgggccagcacatgctgaacctcgtgctcggcctggccatggtcggcctcgggctggtgttcatgttcaccgaaagctggccggccttcttcgcgatgctggcgctggccttcgtgatgggcgtgctcatcatcatcccgatcggcggcgccgacatgccggtggtggtgtcgatgctcaacagctactccggctgggcggccgcgggcatcggtttcagcctgaacaacgcgatgctgatcgtggccggttcgctggtgggctcttcgggcgcgatcctgagctacatcatgtgcaaggccatgaaccgctcgttcttcaacgtgatcctgggcggcttcggcggcgaggcggtcagcgcggccggcggcgccaaggagcagcggccggtcaagagcggcagcgccgacgatgcggcctacatgctgtccaacgccgagaccgtgatcatcgtgccgggctacggcctggcggtggcgcgtgcgcaacatgcggtgaacgaactggccgagaagctcacccacaagggggtgacggtgaagtacgcgatccacccggtggcgggccgcatgccgggccacatgaacgtgctgctggccgaggccgaggtgccctacgaccaggtgttcgagatggaagacatcaacggcgagttcgcgcaggcggacgtggcgatcatcctgggcgccaacgacgtggtgaacccggccgcgctgcaaaagggcacgccgatctacggcatgccgatcctggaagcctacaaggccaagacggtgatcgtgaacaaacgctccatggcggcgggctatgccggcctggacaacgagctcttctacatggacaagaccatgatggtctttggcgatgcgaaaaaagtagtggaagatatgggcaaggccatcgaataggcagaaggtccgcgcccgcgcagtgcgggccagatcatcgcggcgccatcaagtgcgccgttttcgttttcagataactcgatttggaggagacacatccatgaccgatcgtccctggctcagcagctacccgcaaggcatgcctgccgatatcgacccttcgcaatacccgtcgctggtggcactcatggaagagagctttaccaagtacgccgaccgcaccgcctacagcttcatgggcaaggacatgagctacagggaaaccgacaagctgagcaaggctttcggggcctacctgcaagggctgggcctggtcaagggcgatcgcgtggccgtgatgatgcccaactgcccgcagtacccgatcgcggtggcggccatcctgcgcgccggcctgatcctggtgaacgtgaacccgctgtacacgccgcgcgaactcgagcaccagctcaaggactcgggggcgaaggccatcgtcatcatggagaacttcggcaccacgctgcagcagtgcatcgcagccacgcccatcaagcacatcgtgctcgcggccatgggcgaccggctcggtttcctgaaaggcgcgctcgtcaactacgtggttcgcaacgtgaagaagctggtgccgcacttcagcctgccgggtgcggtgcgcttcaacgatgcgctcgaccagggcgcgggccgcaccctgcaggtgccggtcatcggccctgacgacgtggccgtgctgcagtacaccggcggcaccaccggcgtttcgaagggcgcggtgctgctgcaccgcaacgtgatcgccaacgtgctgcagtccgaagcctggaacgagcccgtcatggcgcaggtgccggccggcgagcagcccacgggcgtttgcgcgctgccgctttatcacatcttcgccttcacggtgggcatgatgctgagcatgcgcacgggcggcaagctgatcctgatcccgaatccgcgcgacctggcgggtgtgctcaaggagctctccaagcacacgatccacagctttcccgcggtcaacacgctgttcaacggcctggccaaccatcctgacttcaacaccgtcaactggaagaacctcaaggtctcggtcggcggcggcatggccgtgcaggccgcggtcgccaagctctggctcgagaaaaccggctgcccgatctgcgagggctacggcctttccgagacctcgccctcggccacctgcaacccgaccaacagcaaggcctacaccgccaccatcggcctgccgctgccgagcacctggctcaagctgctcgacgacgatggccgcgaagtgccgccgggccagcccggcgaaatcgcgatcaagggcccgcaggtgatggccggctactggcagcgccccgacgaaaccgccaaggtcatgacgccggacgggtacttcaagagcggcgacatcggcgtggtcgacgaacgcggctacttcaaggtggtcgaccgcaagaaggacatgatcctggtctcgggcttcaacgtgtacccgaacgagatcgaagacgtggtggcgcagattccgggcgtgctcgaatgcgcggccgtgggcgtgagcgacgacaagacgggcgaagccgtcaagctcgtgctcgtcaagaaggacgagtcgctgaccgaagcgcaggtgcgcgaatactgcagagcgaaccttacgggttacaagcagccccgaaccgtcgagttccgcaccgagctgccgaagacgccggtcggcaagatcctgcggcgcgaactgcgggaagccagaaagtaagggttcggcccgggtagggccgcggcatcgatcttgcatattgcgggtcgatgcttcgcttcctactcactcgggtgagcttgctggtgccgaccttcatcggcatgacgctgctcgccttctttctcatccggctggtgccgggcgacccgattgaaaccatggccggcgagcgcgggatcgaccccgcgcgccacgcccagctgcgcacggcctatggcttcgacaagccggtgatcgtgcaatacggcatctacatcggccgtgtgctgcatggcgatctgggcaaatcgatcatcacgcaggaatcggtcgcaagcgagtttctcgcgctgtttcccgccaccgtcgagctcggcgtgtgcgcgattgtctttgcgctggtgctggggcttccggccggcattcttgcggcggtgcggcgcaattccatcttcgaccatggcgtgatggccacctcgctcaccggctattcgatgccgatcttctggtgggggctgctgctgatcctgttcttctcggtgcagctgggctggacgccggtgtcgggccgcattgcggtgcaatatttcgtcgagcccgagaccggcttcctgctgatcgacgcactgcgcgcgggcgacaccgatgccttctggtcggccctgcaccacctgattcttccggccatcgtgctcggcaccgtgccgctggcggtcatcgcacgcatgacgcgttcggccatgctcgaggtcctgggcgaagactacattcgcaccgcgcgcgccaagggcctctcgcgctttcgcgtggtggcgctgcatgcattgcgcaacgcgctgatccccgtggtcacggtgatcggcctccaggtgggcgtgctcttcacgggcgccatcctcaccgaaaccatcttctcctggcccggcgtcggcaagtggctcatcgaagcgatcggccggcgcgactaccctgtgctgcagggcggcatgctgctgctgggcggcatcgtgatgctggtcaacctgctggtcgatgtgacctacggcgtcatcaaccccaggatccggcgctgaacatggcctcgaccgacatcatgtccccgtccggtgcgagcaaggcgccgcccgggccctggcgcgagttctggacctccttctccgccaaccgcggcgcggtcatcggactcgccaccatcgtggtgctgctgctcgtggcgctgttcgcgccgtggattgcgccgcatgcgccgaacgaaaccaacagcgccgtcttcctgcagccgccggcctggcagcagggcggctcaatgagctacctgctgggcaccgacgccatcgggcgcgacattctttcgcgcctcatgcacggcgcgcggctctcgctgtcgatcggcgttgccgtggtggcgctctcggtggtgacgggcatcgtgctcggcctgattgcggggttctttcgcggcgtgctggagatcgcgatcatgcggctgatggacatcgtgctcacgctgccgagcctgctgctggccatcgtgatcgtggccatcctcgggccggggctggtcaacgcgatgctcgccgtggcgatcgtggtgctgccgcactacgtgcgcatcacccgcgcggccgttatcgccgaagtgtcgcgcgactacgtcacggcggcacgcgtgagcggcgccggcacgctgcgcctgatgttcagcgaggtgctgcccaactgcgcggcaccgctcatcgtgcaggcctcgctcggcatctccacggccattctcgatgcggccgcgctcggcttcctgggcctcggcgcgcagccgccgtcacccgaatggggaacgatgctggccgatgcgcgcgagttcgtgctgcgcgcctggtgggtcgtcaccttcccgggcctggccatcctcgcggccgtgctggccttcaacctgctgggcgacggcctgcgcgacgcgctcgacccgaagctcaagagatgaacatgctgctggacatcaaggacctgcatgtggagttccccacgcaaggcggcgtgctgcatgccgtcgacggcgtgagcctcacgctcgaggagggcgaggtccttggcatcgtcggcgaatcgggctcgggcaagagcgtgaccatgatggcgctgatgggcctcgtcggctttccgggccgggtgcgcgcggaccacatgcgctttgcgggcaaggagctgctcggcatttccgacaaggcccgccgcgcgctggtcggcaaggaggtcgcgatgatcttccaggagccgaccaccagcctcaacccctgcttcaccatcggcttccagctgatggaaacgctgcggctgcatctgcacctggaccggcgcacggcaaagaagcgcgcgaccgaactgctcgaacaggtcggcatacccgccgcgtcgtcgcgccttggcagctacccgcaccagctttcgggcggcatgaaccagcgcgtgatgatcgcgatggccattgcctgcaatccgcgcctcttgatcgccgacgagccgaccaccgcgctcgacgtgacgatccaggcacagatcctcgacctgctgcgcgacctgcagaaagagcgcggcatggcgctggtgctcatcacgcacaacatgggcgtggtgagcgaaatggcgcagcgcattgccgtcatgtatgcgggccaggtgatggagcagcagcgcgtcgaccggctcttcgcgaatccgcaacacccctataccgaggccctgctggccgcgttgcccgagcgcgcggcgcccgaggggcggcttgccaccatcgcgggcgtggtgcccggcgtgcacgaccggcccaccggttgcctgttcgcgccgcgctgcagctacgtgacgacgaaggcctgcaacgtgcggccggcgctgcgtgcggtcgcgtctcaaccgggcgccgaagtgcgctgccattttccgctcggcgagccggggcggctggccgccatcgaggcagaccggccgcggtcgcaagccatggaggtgctgccgtgagcgccgcactgggcgatgtggtcgtcgatgcgcgcaacctgcagcgcacctacgccgtacggcgcggcatgttccgcgcgcctgcgcagctgcgcgcggtgggcgatatctcgtttcgcatcgagcgcggccgcacgctggcggtggtcggcgaatcgggttgcggcaagtccacgctcgcgcgcatggtcgcgctgatcgagaagccgacggccgggcagctcacgctggtcggccacgatgcggtggacccgcccgccgagcgccggcgcgagctgcgtcaggccgttcagctggtgttccagaacccctatggctcgctcaatccgcgcaagaagatctccaccgtgctcgaagatccgctggccatcaacaccacgctcggcaagaccgagcgcgctgccaaggcgcgcgagatgctcgcgcgcgtgggcctgcggcccgagtacgccaaccgctatccgcacatgttctcgggcgggcagcgccagcgcattgccattgcgcgcgcgctcatgctggagccgcgcctcctggtagccgacgagccggtgtcggcgctcgacgtgtcgatccaggcgcaggtgctgaacctgctggccgacctgcaggccgaactcggcctggcctacctcttcatttcgcacgacctgggcgtggtgcggcacatcgcgcacgacgtgctggtgatgtacctcggccatgcggtggagcagggcccgaaggcgcgcatcttcgcgcggccgctgcatccctacacgcaggcgctgctggcgtccacgcccgggctcagcagccagcgcatcgtgctcaagggcgagctgccatcgccgctgaatccgccgcccggctgcgtcttcagcacgcgctgcccgcacgtgacagagcgctgccgcgaagagcggcccttgctgcgcgcgctcgacgagcggctggtggcctgccactacgccgagaagtttctcgaaggcgctgcgccggtgcgcgccgacttgccgttgtctccgccgttcgtcgcgcctctggcgatgaaaacctagttcacttcaacccgtgtcccaaggagttgccatgaagacccagccatccatttcgcgccgcttgccaaagcttgccgcgctgctcgcgccgacggcacttgccgtgctcaccctcgcctccggcgccgtgtccgccaagacgctggtctactgttcggagggcagccccgagaacttctatccgggcgtgaacaccaccggcacctcgttcgacgtgaccacgcaggtctacaacaccatcgtcgagttcgagcgcggcggcaccaaggtcgtgcccggcctggcagaaaaatgggacatctcggccgatggcacgcagtacaccttccacctgcgcaagggcgtcaagtggcacagcaccagcaagactttcaagcccacgcgcgacttcaacgccgacgacttcatcttcatgctcgaacggcagtggaaggagagcgaccccttcttcaaggtcacgagccagaaccactcctacttcaacgacatgggcatgcccaagctcttgaagtcggtcgaccgcgtcgacgagtacacggtgaagatcgtgctcaaccaggccgaggcgccgttcctggccaacctcgcgatgcagtacgccggcatccagtcgaaggaatacgccatcgccatgctgaaggccggcacgccggagaaggtcgaccaggacccggtcggcaccggaccgttctacctcgtgcaataccagaaggatgcggtcatccgcttcaaggccttcccgcagtactggggcggcaaggcgaagatcgacgacctcgtgttcgcgatcacgcccgatgcctcggtgcgctgggccaagctgcagaagggcgaatgccacgtcatgccgtacccgaacccggccgacctcgatgcgatccgcaaggacccgaacgtgcaggtgctcgagcagcccggcctcaacgtgggctacctctcgtacaacaccaccaagaagccctttgacgacgtgcgcgtgcgcaaggccatcaacatggcgatcaacaagaaggcgatcatcgacggcgtgtacctgtcgaccggcgtggccgcgaagaacccgatcccgcccacgctgtggtcctacaacgacgcggtcaaggacgacccctacgatcccgaggccgcgaagaagctgctggcgcaggccggttttcccgatggcttctcgaccgacctgtgggccatgccggtgcagcggccctacaacccgaacgccaagcgcattgccgaattgatgcaggccgatctcgccaagatcaacgtcaaggccgagatcaagagcttcgagtggggcgaataccgcaagcgcctgcaggccggcgagcaccagatgggcatgctgggctggaccggcgacaacggcgacccggacaatttcctctacacgctgctgggctgcgcctcggccaagtcggcgagcggcagcaacatctccaagttctgctaccagccgtatgaagacctggtgctgaaggccaagagcgcaaccaagcaggccgaccgcgatgcgctctacaagaaggcgcaggtcatcttcaaggaacaggcgccgtggttcaccatcgcgcatgcggtgcagctgaagccggtgcgcaaggaagtcgtcgacttcaagctcagtcccttcggccgccacaccttctatggcgtcgacatcaagtagccgatgagcgatgcaccgtttgccatcgtcgctgcaatgcacgaggagctcagcgcgctcctcgcgcagatgccggacgagcagcgcgtgcgcgtcgcgggccgcgacttctgggtcggccatctgcacggccagccggtggtcgcggtgctgtcgcgcattggcaaggtggccgctgcggtcacggccacggtgctgctcgagcgcttcggcgtgcgggccatcgtgttcacgggcgttgccggcgggcttgcgccgggcgtgaacgtgggcgacgtggtggtcgcgtcggaactgctgcagcacgacctcgacgcctcgccgatctttccgaagtacgaggtgccgctctcgggcatggcgcgcttcgcggccgacgcggccattggcaatgcgctggcggaggtggcggccggtgtgctgcgcgacccggtggcgttgatcggccagcaggccgtcgacgagttcggcattcaagcgcccaaggtgcaccgcggcctgctggtgagcggcgaccgcttcgtgtcgaccagcgccgagagcgaggcgctgcggcgcgacctgcccgacgcgctcgcggtcgagatggaaggagccgccatggcgcaggcgtgccacgactatggcgtgccgttcgcagcaatgcggacgatttcggaccgcgccgacgacgccgcgcatggcgacttcgcgcgcttcgttgtcgaggtggcgagccgctacagccttgcgctggtcgatgcgtggctggccacgctgccttcttcctcggtaacgcccgctgctacttgagccagccgcgccggcggaagtaccacatcggcaccagcgcgctggccgccatcaatgccagcgcatacggatagcccagcgaccagtcgagctcgggcatgaacttgaagttcatgccgtagatgctcgcgatcagcgtgggcggcagcagcgccacgctggccaccgagaagatcttgatggtcttgttctggttgatgttgatgaaaccgacggtcgcatccatcaggaagttgatcttgtcgaacaggaaggccgtgtggttgtcgagcgattcgatgtcgcgcaggatctgccgcgcctcctcgaactgctcggcgttgagcatgcggctgcgcatcatgaagctcaccgcgcggcgcgtgtccatcacgttgcggcggatgcggccgttcaagtcttcctggcgcgcgatcgccgccagaacttcgccggccagctcgtcgctgacgttgccttcgagcaccttcttgccggccacttcgagttcgtcgtagatgttctcgagcgtgtcggccgagtattcggcgtcggcgtcgaacagcttgagcagcacttccttcgcgtcctcgatgagtcccggcgcgcggcgtgcgcgcatgcgcagcaggcggaacacgggcacgtcttcgtcgtggatcgagaacagcacgccgcggctgcgcagttcggtgttgtgctggttcaggatgaacgccacgcgcaccgaccgcgggtcttcgtcgtcgtcgatcaggaagtcggagcggatgtgcagttcgccgttgtcttcttcatagaagcgcgccgactcctcgatgtcctcgtccatcgcgtcctcgggaatcgaaaggccgtagtactgcttgatccagcgcttctcttcgagggtgggcgattcgaggtcgacccagatcggctggaacttggaaagctcctcgagcgcttcgatctcttcctggacgaggcggccgttggcgagcgtaaagatattgagcatgggctcactcccgtgaaatggctgaggcgatggggcgagggaaggggcgctttcaattcccggtcccgcgcaggcaaggcgtcagaggggagttgaaagctgccgagacggggcggtttccaaggtgcggtctccagttgcagcgaggcgcgattatgtcatcggccatgtgacgggaggctgccgatctggatggacatacagtaaagttgcggccatgcagaccgctgcgctccctgttttttccgccgccggtgccacccaggccgagcgcctggccgcggcgctctctacgctcaacgacgagcagcgcgccgcggtcgaacacctggacgaacgtccgctgctggtgattgccggtgcgggctccggcaagaccagcacgctggcgcaccgggtggcgcacctgatcgccggcggcgtcgacccgcagcgcctgctgcttttgaccttctcgcgccgcgcggcgcttgaaatggagcgccgcgcgggccaagtgctggcgcgcgtcctcggactcaagtcagaaaagccacccgcgctgccgtgggccggcaccttccacggcatcggggcgcgcctgctgcgcgagtacgccgcgcacatcggcctcgacgaccacttcacgatccacgaccgcggcgacgccgaggacctgatgggcctggtgcggcacgagctcggcctgtcgtcgagcgtgaaccgttttccgcgcaagggcacctgcctttcgatctactcgcgctgcgtcaacacgcgcgccccgctggccgatgtgcttgcggaagcttttccgtggtgcgcagaatgggaggccgagctcaagcgcctgttcggcgcctacgtggaggccaagcagcagcagaacgtgctcgactacgacgacctgctgctctattgggccggcatggtggccgagccggcgctcgccggactggtcggcgcgcgtttcgaccacgtgctggtcgacgagtaccaggacaccaacctgctccaggcctcgattcttcttgcgctcaagcccgatggccggggcgtgacggtggtgggcgacgacgcgcagtcgatttactcgtttcgcggcgcaacggtgcgtaacatcctcgactttccgttgcagttttcgcaggccgcgcgggtggtcacgctggagcgcaactaccgctccacgcagccgatcctcgacgtctcgaaccgggtcatcgcgcaggccgccgagcggcatgccaagaccctctggaccgacaagccctcggcgggcaggccccaactggtgctggtgcccgacgaggcgcagcaggcggtctgggtggccgacaaggtgctggcgcaccgcgagggcggcctcgcgctcaagtcgcaagcggtgctgtttcgcgcttccacgcacagtgcgccgctcgaactcgagctggcccgccgcaacatcccgttcgtgaaatacggcggcctcaagttcctcgaggcctcgcatgtgaaggacctgctcgcggtgctgcgctttgccgaaaacccgcgcggccgcatggcgggttttcgcgtcacgcagctcatcccgggcatcgggcccgccacgggcgcgcggctgctcgacgccatggaccaggcggccgacccggtggcggcggtgcgcgagttcgtgccgccctcggccgcgcgcgccgaatgggcggtgttcgccgaggcctacgcggcgctgtgcgcgcctgcgctggcatggccggccgacgtggaactggcggtgcgctggtacctgccgcatctcgagcggctctacgacgacccttccggcgtgcggcgcggcgacgtcgagcagctggcgcggctggcgtcgggctatgcctcgcgcgagcgcttcctgaccgagctcacgctcgatccgcccgaggcgacgagcgaccggccgggcccgccctcgctcgacgaggactacctcatcctttccaccatccactcggcgaaagggcaggaatggaactccgtgcatgtgctcaacgtggtcgacggctgcctgccggccgacgtggcgcagggcgcgcatgaactcgaagaggaacggcggctgctctacgtggcgatgacccgcgcacgcgaccatctgcacctgctggtgccgcagcgtttctacgtgacgcagcaggccgtgcggggagaccgccatctgtacgccaaccgcacgcgcttcatcaccgaggcggatcttgcgggcttcgaacagcagacctggcccgcgccgcccgcgcgtgcacccgccgtgccgccaccggccgccgtgatcgatctgcgcaaccgcatgcgcgccgcctggagctgaaaccgcaggccctccgcctggcagggtcaccgctggtgacgcactgaaacacttgctgccaaagcgccgcagcggcgggcccgcgtgcgccggcagctatggaagctgtagcgaagtggcgccgggccgcttgcgcatgccccggtggaaagcccgactattgcaataccgtgacagcttgggcatagtgaatcgaccttgcctctttcctcccctctttcccctcttttcctttcccctcttttctcttctccccccgacccacatctgatttcgccggccacgcttcattccggagcggggtcattttcccaaccgtcaattctcaggaggtcattcatgaatttgacgatcagcggtcatcacctcgacgtcacacctgctttgcggacttacgtcacgagcaagctggatcggatcacacggcacttcgaccaggtggtcgatgtgaaggtgctcctcacggtggaaaagcagaaggaaaaggaacgccgccaacgggcggaatgcaacattcacgtcaagggcaatgacatgttcgcggagtcgagccacgctgatctctacgctgcggtcgatgaactggtcgacaagctcgaccgccaagtggtgcgccacaaggaccgtctgcaggaccaccatcacgcggcacccaagcgcgtgatgtaggtagccacgggcaagggcttcgcggcccctgcgacaagccgccttcgggcggctttttgttgcccggtttttgttcttgcgccccggcgccgcgaggcctctgggcaacatgtagcctaaaagtaagtaacaggattggggtttttaccaagcgggtgcataatcgcccccgacttcccccaccatgaatcgcctcgcgtccatcctgccgcccgctcaagtgcttgtgagcgttgacgctaccagcaagaagcgtgctttcgaagaagcgggcttgctgttcgaaagccttcatggcctcggccgcgccctgatcaccgacagcctgtttgcgcgcgagcgcctcggttccaccggtctcgggcacggggttgccattccgcatggccgcatcaagggcctgaaggcgccgatggccgcggtcttccagctcgccaaccccatcgggttcgatgcgccggacgagcagcccgtcgggctgctgatcttcctgctggtgcccgaagcggccacgcagaaacacctcgaaatcctctccgaaattgccgaattgctgagcgacgccggtctgcgcgagcagatcaagtcgagcaccgatgcggctgcgctgcacggactcattgccaactggcaatcgacgcaggtcgcgtagaggtggtcgtcgccccggcagagccgcttcgcggtattctgggctgctccaaactgggcgctgagcgccgactcccctacgcatgaagccgaccgtcatcagtgccgacgccatgttcgaggaattccgcggatcgctccgctgggaatggctcgccggcctgggtgcttccgaacgccaattcgaccccgaggtcatcagccgcgcccagtcggctgccgatctggtcggttacctcaattacatccatccctatcgcgttcagatcctcggtgcccgcgaggtgacctacctgacgcgcggcagccaggaagactgcgcgcgtcgcatcgcccgcatcgtcacgctcgaaccgccgatgctggtgctcgccgacggccaggccgcgccggacgagttgctatcgatttgcgagcgcgcccagctgccgctgttcgccacccgcgagtcttcggccttcgtgatcgacctgctgcgggcctacctgtccaagcatttcgcggaacgcacctcgatgcacggggtgttcatggacatcctgggcatgggggtcatgatcaccggcgaatcggggctcggcaaaagcgaactcgggctggagctgatctcgcgcggcaacgggctggttgccgacgacgcggtcgacctctaccgcatcaaccagaacaccatcgaggggcgctgccccgacctgctgctcaacctgctggaagtgcgcggcatcggcctgctcgacatccgcgccatcttcggcgagacggccgtgcgccggaagatgcggctcaagctcatcgtgcacctggtgcggcgcgacagcttcgagcgcgactacgagcgcatgccctcggcgccgctcacgcaggacgtgctgggcatcccggtgcgcaaggtcatcatccaggtggtggccggccgcaacatcgccgtgctggtggaagcggcggtgcgcaattcgatcctgcagctgcgcggcatcgacacctatgccgatttcgtggcgcgccaccacaaggccatggaaaacggccgcgacggggactgaggggcgtttgccgctaccttttgctcgcgcagtcgccgcacaggccgtagagggacatggcgtgatcctgcaggatccagcccttgtcctttgaaatcatctgctggcggcgctcgatttcggcgtcgtagaactcctcgaccttgccgcacgacgtgcagatcaggtggtcgtggtgcgtgccttcgttgagctcgtacaccgccttgccgctttcgaaatggctgcgctccaggatgccggcctgctcgaactgggtcagcacgcggtagaccgtggccaggccgatgtcggagtgctcgttcaaaagcacgcgaaacacgtcttcggccgtcatgtggcgctggctgccggtctggaagatctcgaggatcttcaggcgtggcaatgtggccttgaggccggtattcttgagttcgtcgatgttggccatgatggttcctgcgccctgggctgcggatgggccctaaaagggccagccgctacaatggccgatcatatcgctaccccccttttctcccatgcctgccattctccaacgccgtccctggctgctggctgcggccgtcgccgcgacgttctgcctcggcgcctgcagcggcttcagcgaccgcacgcgtggtgcgctgtcggccatcacgccctacaaggtcgaagtggtccagggaaatttcgtgtccaaggaacaggtcgaggcgctcaagcccggcatgtcgcgccagcaggtgcgtgaaattctcggcacctcgctcttgaccgatgtcttccacaaggatcgctgggactacgtcttcacgatcaagcgccagggcgtcgatccgcaggaacgccgcctgaccgtcttcttcaagggcgagctgctcgaccgctacgaaggcgactcgatgcccagcgaagaagaattcgtcgccacgctcgacacccgcaagaagagcggcaaggttccgccgctcgaggcgtcggaagaagagctcaagaaatttacgcccaaggaagacgccaagaaggccgacgccaccacgacggccaccaacctgccgccgttgccggccgcataccccccgctcgaagcggcgcgctgagcacgcgccagacagcgaacgagcgagcgagggcgggctcacccgtcgagtcgggcgggcgcgtcccggtctccatgccccatttcgaaggctgaatccgcgtgactgaaaccatttcttcctcttcttcttccatttccgagtcttccacgcctgccctccggcgcatcgcgatcgcgggagcgtcgggccgcatgggccacatgctgatcgaggcagtgcgcgaggcgcccgattgccgcctggccggcgcgctcgacgtggcgggcagcaacgccatcggcgccgatgcggccgcgttcctcggcttcacgagcggcgtgcccatcgtgtccgacctgcgcaccggcctgcaggacgcgcaggtgctgatcgacttcacccgtcccgaaggcacgctcgcgcacctcgccatctgccgcgaactgggcgtgcaggcggtcatcggcaccaccggcttcagcgacgagcagaaggccgagatcgccgaaatcgcgaaggacatcgcgatcatgatggcgcccaacatgagcgtgggcgtcaacgtcaccttcaagctgctcgaaatggccgccaaggcgctgtcgaccggctacgacatcgagatcatcgaggcgcaccaccgccacaaggtcgatgcgccctcgggcaccgcgctcaagatgggcgaggtcatcgccgaggcgctgggccgcgacctgaaggaatgcgcggtctacgcacgcgaaggcatcaccggcgcgcgcgacccttccaccatcggcttctccgccattcgcggcggcgacatcgtcggcgaccacaccgtgctgttcgcgggcaccggcgagcgcatcgaaatcacccacaagtcggccagccgcgtcacctacgccgagggcgcgctgcgtgcggtgcgcttcctggccggccagaaggcaggcctgttcgacatgttcgacgtgctcggcctgcgctgaaacaaacccgatgagcgtgctcgaactgctgacccagggcgacggcgtcagtcgttcagtggcggcgctgctgctggcgatgtcgatctccagctgggtggtgattctctggaaggcctggctgctgcgcggcggcacgcgcgacgtgctgcgcagcattgccgcgttctggcaatcggccacgctcaccgatgcggagcagcggctcaaggccttcgaccgcgccacgctggtggggcctgcggtaagcgccatcaagaatgcggcaactgcagaggcaggcggtgcaacgctcggcggcaccaccggcgatcgcaaccagcggctcacgcgagccctgcgcggcgcgttgcacggcgcgctgcggcgactgcagtccggccagatcctgctggccaccgtcggcgccaccgcgcccttcgtgggtttgctcggcaccgtgtggggcatctacggcgcgctgtcgggcattgccggccagaccggcggcttcaccatcgacaaggtggccggccccgtgggcgaggccctggtgatgacggcgttcggcctggccgtggccattccggccgtgctggcctacaacgtcttcggccgcgtcatcggccgcatcgaagccgagctcgagggctttgcgcacgacctgctcggcagcttcggcagcgcgccggtacccgctgcgccgccgcccgcgcggcccatgccggtctcggcctaaccccggcggagcgcagagccatggccttcggtcgcacctcgctgggcagcagtgccgctggcggagggcgcgcgacgggcgccggtggacagcggccgctgtccgacatcaacgtcacgccgctggtcgacgtgatgctggtgctgctggtgatcttcatcatcaccgcgccgctgatggccagttcgatcaagctcgacctgccgcagaccgacgccggccagcccaacgacacgcccaagttcgtgagcgtgtcggtcgatgcctcgggcaagatcttcttcaacgaccaggcggttaccgacgaagagctggccgcccgcctgcagaaagccgcggccgacagcaaggacactgaagttcagctgcgcgccgaccagaccgtgccctacggcagggtggtggcgctgatgggcattgccaacaaggcaggcttgagccgcatcgggttcgtgaccgatgcgggtgccgcaaacccggcaccgccgaatccgcgctgaagccaaaagggcgatcgattcaatcgggcgccggggcttcgcgcttcttcagacccggtagcgtccagcccagcgtcatgcccgcggccgccagcaggatcgcggtcgcgccgaaaagctgcgcgggatgcagccgctggccgaacgccaggtaatccacgccgatggccaccacgggatagatgaaggacagcgcgccggccatgtgcgtcggaagcttctggatcgctccatagagcagcgtgaagacgagcccggtgtagacgacgcccatggccaggtgcgtgccccacacgcccgcatccgtgggcagctctgccaggttggcgaacggggcgagcagcacgatgcccacacagacctgtaccagcgcgatcaggtgaggtggcgtgccgtcgagctgcttggcgacgacggccgcaatggcatagaaaaacgcagcgcccagggccatcaggatgcccaggaaatacgaggcaccgttggcgccgccacccggcttggcctcggcaatcagcaggacgccggcaaacgcaatgcccagccagcccagcttggtcgccgtcaatcgctccgagaagaacagcgcgccgagacccaccagcatgaagggctgggtgttgtagaccgccgttgcgatggaaatcgacgcatgcgagaacgacgcgaagatcagcagccagttgagcaccagcgcagcgccgcccaaggcggccagcgccaccacgcgaagcgtcagcagccgcctgcgaagaaggccgagcgcggcgcagaccgcgagcagcgtggcagcgccgaaagcgcagcgccagaacagcaggtcgaccagcggctggcccgagcggatgacgaaccagccgatggttccggaaatgaccatggccgcactcatctcgagcgcgccgcgcagttgtctttgcatgatccggggtcttgttggagcaagtctcaggttgccatcgaagccgcatcgagcctatgatttttcgaagggaagaatccattcgaggctcacaaaacaaggcggggccgcgatatcgccaaaggatcgaaaaaatgctggacgaagtcgaacaaaagattctcgaggtcatgcagcaggatgcgcgcatctcgctgaaagacctggcggcccgggtcggcatgtcttcgccaagtgtctcggagcgccttcggcggctcgaagagcgccgggtcatccgcggctacacggtcgagatcgatcccaaggcgctgggctaccagctgcaggccatcgttcgcatccggcccttgcccggccacctgcatgccgttcaggcattgatcgaaagcacgcccgaattcagcgagtgcgacaaggtcacgggcgaagactgctacatcgcgcgcttgttcgtgcgctccatcgagcagctcgaccaggtgctggaccgcatcgtcgacaaggccgagacgcacacggccatcgtcaagacgcagccgatacggcggcgggcgccgccgctgcgcatcggctgaagcaccggccggcgccgcaacgccgcgtggtcagccgagcaccaccggcttggtgtgccagatctcgtgcgcgtactgcgcaatggtgcggtccgacgagaacgcgcccatgcccgccacgttcaggatggccatgtgcgtccaggcatccgggtcgcggtagagcgcatcgacttcggcctgcttcgcgacatagctcgcgtagtcggccagcagcaggtagtggtcgccccagttcaccagcgcgtcgtagatgccctggtagcgggagggctcgccggcggaaaactccccatcgcgaatcgcatcgagcacgcgcttgagttcggcgttctcttcgtagatgtcgcgcggctggtagccgtgcgcgcggatgtcggccacttcgggcgtggtgttgccgaagatgaagatgttctcggcgcccacgttgtcgcgcatttccacgttggcgccgtcgagcgtgccgatggtgagtgcgccattgagcgcgaacttcatgttgccggtacccgaggcctcagtgccggccgtcgagatctgctccgacaggtcggccgcgggcatgatcacctcggccaggctcacgctgtagttgggcaggaacaccaccttcagcagcttgcccacgcgcgtgtcgctgttgatggttttggccacgtcgttgatcagccgtatcacgagcttcgccatctggtaggccgaggcggccttgcccgcgaacaccaccacgcgcggcacgatgtcgatcggcccgcccgccgcctgcgcatcgaggatgcggtggtagcgcgtgatcacgtgcagcacgttgagcagctgccgcttgtactcgtggatgcgcttcacctgcacgtcgaacattgcgtcggtgtcgaccacgatatccatgtgctgctccacccagttggccagccgcagcttgttctcgcgcttggcatgcctgaaggcgcgcgcgaaggcgggctgggccgccatcggccgcagcgcctcgagctgcgagaggtcgcgccgccagcccttgcccagccgctggtcgagcaggccggcgagcggcgggttggcctgcgcgagccagcgccgcggcgtgacgccgttggtcttgttgttgaagcgctcgggaaagatcttcgcgaagtcggcaaagatcgactgcttcatgagttccgaatgcaggcccgacacgccgttgatcgagtggcttgcgagcaccgccacgtaggccatgcgcacgcggcgctcgcccgcttcgtcgaccagcgacagccggcgcagcagctcgacgtcgtttcccgccttctgcgtcacggccgcgagaaacttcgcattcatgtcgtagatgatctgcaggtgccgcggcaggatgcggccgagcatctcgaccggccaggtttccagcgcctcgtgcatcagcgtgtggttggtgtagctgaacaccttctgcgtgtgggtccacgccacgtcccacgccaggccgtgctcgtcgagcaacaggcgcatgagctcgggcaccgcgagcaccgggtgcgtgtcgttcaggtggatgctgaccttctcggccagctggtcgaaggtcttgtggttgcgcaggtagcggcgcagcaggtcttgcatgctcgcgctgcagaaaaaatactcctggtgcagccgcagctcgcggcccgagggcgtggagtcgtccgggtagagcacgcgcgagacgttctcggagtggttcttgctctccaccgccgccatgtagttgccgcggttgaaggccgagaggtcgatttcttcggtggcccgcgccgaccagagccgcaaggtgttggtggcctgtgtgccgtagcccggaatgatggtgtcgtaagccacggccagcacatcgtgcgtgtcgacccagtcggccgcgccgtagggggcgttctttccctcgcgcctttgcacgtggccgccgaagcgcacgcggtagttcacctcgggccgctggaactcccaggggttgccgcgcgtgagccagtagtcgggcgtctcgacctgctggccgtcgacgatgcgctggcggaacatgccgtattcgtagcggatgccgtagcccatgcctggcacgccgagcgtggccatggagtcgaggaagcaggccgcgagccggccgaggccgccgttgccgagcgccgcgtcaggctcgcgctcggccagcgccgccacgtcgacgccgaagtcggccagcgcatcgcgcacggtgtcgtagaggtcgaccgccagcagcgcattggtgaaggtgcgcccgatcaggaactccatcgagaggtagtagacgcgcttcaggtcctgcgcatagttggcgcgcgtggtcgccatccagcgctcgaccagctggtcgcgcaccgcgagcgccgtggcgtgcagccagtcgtcctggctggcggcgacggggtccttgccgacggcatagatgagcttgttggcgactgcgcgcttgaacgcggccacgtcgcggtcgggatggtcgtaggcgaagtctttgatggtcatgggcttcgatgaaaggttgtggggttcaggggttgtggcgccgtggtgcagatcaggtgccggctggctcgagcgcctgccggtagacctcgatgtactgggccgccgcggtggcccaatcggccgggcgccgcatggcagtgccgcgcacgcggcgccagtctggcgcgtgctggtaaagcgcgaaggcacgacgcagcgcacggccgtagtcagcgtcgtcgaaacggtcgaagacaaaaccggtggcgtcgccgctggcgatgtcttcgagcgtgcagtcgaccaccgtatcggccaggccgccgacgcgacgcaccagcggcaggcagccgtatttcaggccatacatctgcgtgaggccgcagggttcgaagagcgatggcaccagcgtcacgtcgccgccgccgaagagctggtgcgccagcgtttcgttgtagccgatggtgacgctgaccgactgcggcgccgctgccgcgcgctcgcggaaagcatgctccagccgggcgtcgccgctgcccagcagcgccagctggccgccctgggcgatcagcgcgtcgaggccgccgagcaccaggcgcaggcccttctgctcggtgagccggctcacgaggatgaaaagcggcgcgtcggcgcgttcggccaggcccaactggtgttgcagcaccgccttgcagcgcgccttgccggccatgtggcggccttcgggcgtgtggaagccctgaacaagcgctgcatcggtggacggattccagacctggtcgtcgaccgcattgaggatgcccgtgagcgcgtcgccgcgcagccgcagcaggccgtccaggccgaaaccctgctcgggtgtctggatctcgcgcgcgtaggtcgggctcacggtggtcaggcggtctgcatagtagaggccgcccttcatgaacgacagctggccgtggtattcgagtccgtccatgtggaaggccggcgcgggcaggccgagatcgacgaagttccagggcgcggagatgccctggtaggccaggttgtgcacggtgaacacgctgccgacatggggcgcaccggcctcgcgcgcaaagtgcaggtaggccggcgcgaggcccgcatgccagtcgtgcgcatgcacgacctcgggccgccacgatggatcgagcccctgtgcaagcagcgccgccgcccagcccagcagcgcgaagcgccggtgattgtcgccatagggctggcgtgtggtgtcttcgtagggattgccgggccggtcgtacagcgccggtgcgtcgatcacgtaggcggggatcggcgggttgccgtcgatgacgatgcggcccgcgcgcagcacgaagcgctcgccccagggcgcgtcgaactcggccaccggcgccggctcgcgcaggcccgccaggatggccgggaagcccggcagcagcacccgcgcgtcctggtcggccgccatgagggcgatcggcaaggcaccggccacgtcggcaaggccgccggtcttgagcaggggaaaaagttcggcgctgacctggagtattcgcatcgtgggacggtgcggcctcaggcggccagtcgcttgagcatctcgcgcgtgaccagcaccacgccggcctcggtgcgctcgaagtgcgcggcatcggcctcggcgtcttcgccgatgaccatctcgtcgggaatgacgcagccgcggtcgatcaccacccggttgagcttgcagccgcggccgacttccacgtcgggcagcagcacggcctcgttgatttcgcagaacgaatggatgcgtacgcccgagaacagcaccgaactgctgaccttggagcccgagacgatgcagccgcccgagacgatggtgttgacggtcatgccgtgcttgccgtcgcgatcgagcacgaacttggccggcggcaactgccgctggtaggtccagatgggccagtctgtgtcatagatgtcgagttcgggggtgatcgaggccagatcgaggttggctgcccagaatgcatcaatcgtgcccacgtcgcgccagtaggccttggcgcctggcccgcgcgaggcccgcgtgacgcacgacatgccgaagggatgcgccagcgcgcggccctgcgccaccgcgcgcggaatgatgtccttgccgaaatcgtggctcgaattcgggttggcggcgtcttcctcgagcagctggtagaggtattcggaatcgaacacgtagatgcccatgctggccagcgccacgtcggggtggcccggcatggcgggcggatcggccggcttttcgagaaaggcggtgatctggcggccgtcgtcgatggccatcacgccaaaggccgtggcctccatgcgcggcacctcgatgcagccgaccgtgcagcccaggccgcgctcggcgtggtccttgaccatgatcgagtagtccatcttgtagatgtggtcgccggccagcaccaccacgtagtcgtgccgggtcgagcgggtctggatgatgtccaggttctggaacaccgcatcggccgtgccgcggtaccagtgctcgtcgcccgtgcgctgctgcgcgggcagcacgtcgaccatttcgttgagctcggcgcgcaggaagctccagccgcgctgcaggtggcgcatgagcgagtgcgacttgtattgcgtgaccacggccatgcggcggatgcccgagttgaggcagttcgaaagcgcgaagtcgatgatgcggaacttgccgccgaagtacaccgccggcttggcgcgccggtcggtcagctgcttgaggcgggagccgcgtccgccggccagcaccagtgcgatggtgcggcggaccagttgatgcgcctgcaggggcgcctgcggcgtggtgctgctgttgttgtccatcttgtgtctccgttcgttcttcggttcgttcggtttcgtcgtcagggtttcgcgatcagcctagcaccgccccgcgcggctggctcctaccttcttgcaatccagaggcctgaacgaggtacttttaccgtgccggcctggggcgcctgcgaggcggcgccggggtccagcgccggatcggtcgccagccggcactgccaggcgcccgcgggcagcgcgaaagacatggcctccggccccgcgttcaccagcaccagccagtggccctcgttcgtgaccggggcttcgaaatggattgcaagtgccgtgccgccgttccagtcggccccctgcatcggcgcgccgtccggccgcagccagcggatgcccgccgctccctcgggcggttcggccggccaccagtgcgtgctgcgcagggcgggcgcttcccggcgcagcgcaatgagccgggccacgaaggcgctcaggtgcgcggcttcgctggcggcgtcgtgggtgccgatccatgcgagccacgtggtttcgttgtcctggcaataggcgttgttgttgccctgctggctgtggccgagctcgtcacccgccagcagcatgggcgtgccctgcgagagcagcagggtggcgagcagtgcgcgctgcagccggctgcgctcggcctgcacggcggggtcgtcggtcggcccttcgatgccgcagttgttgctcaggttgtgggcatggccgtcgcggttgtgctccccgttggccaggttgtgccgcttttcgtagctcagcaggtcgcgcagcgtgaagccgtcgtgcgcggtgatgaagttgacgctggccgtgggtgcgcggccatggtgggcgaactgcgcgctcgacgcagtgaagcggtgcgcgaagtcgcccaggccggtggcgccgtcgcgcccttgccgcagccagaagccgcgctgcgtgtcgcggtagcggtcgttccattcgagccagcccggcgggaattcgccgagccggtagccgcccggcccgatgtcccagggctccgcgatcagcagcgtgcgagacagcacagggtcttgcgcaacggccgcgaagaagggcgcgcgcggatcgaaatcgccgctcgtgccccgccccagcaccggcgcaaggtcgaagcggaagccgtcgacgccgagctcgcaggtccagtggcgcaggctgtccatcaccagttgcagcacgcgcggctcggccaggttgaggcaattgccgcagccggtccagttggcatagagcgcgcggtcgtcggagcgcaggtggtagtacagcgcgttgtcgatgccgcgcagcgagagcgtggggccgaactcgtcggtctcggcgctgtggttgtagaccacgtcgatcaccagctccatgccgcgcgcatgcaccgcgtcggccatggcgcggaactcgctcgctggcgtggtgccggcgcggccgctccagtagcgtgcctcgggcgcgaaccagccgacggtgttgtagccccagtagttgctgagccccatgcggagcagccgttgttcgtcggcccggtgctgcaccggcatcaggctcagcgtggtgacgccgaggcgctgcagatggtcgagcaccatgggttcggcgaggccagcgtaggtgccgcgcaaggcggcgggcacgccgggatgcaggcgcgtcagcccgcgcacgtgcagttcgtaaagcacgcggtctccggccgcgatacgggcatggcccggtacggccgagctgccggcgggcaacgccacgcgggccttgagcgcgacggcgccgttgtcgcgcgtgttccgctgatgcggatcggcagggtcgtgccccaggaacagatcgctgccgtcgtagcggccgacgatctcgcgcgcatgcggatcgagcagcacccgggcggcgttgaagcgctgccccgcgtgcggcgcccacgggccgtgcacgcgatagccatagaccagcccggcgcgtccgctcggcagcaggccgtgccagacgccatcggtgaaagcaggcagccggatgcgctgctgctcgtgctgtcccgtgccgtcgaacaggcagagctcgacggcctcggcgttcggcgcgacgagcgcgaagttcacgccattcggcgagagcgtcgcgccaaggggaaagggagcacccgtgttcagcatcgtgtcaggccagcacccacatcacggtcgccagcggtggcacgctgatggaaatcgaatggtccttgccgtgccagggagccggcaaactctggaccacgccattgcccacgccgctgccgccgtacaccgcgccatcggtgttgatggcttcgcggtacgcgcccgcggcgggcaccccgagccggtagccatgccgcggcagcggcgtgaagttgcacacggccaccacgaaggagccgtcgcgggcctttcgcacgaaggcgaacaccgactgctcccagtcgtcgtgcacgatccactcgaagccggccctttctgtgtccagctcgtacagcgcggggaagtgccggtacacgttgttcaggtcgcgcaccagccgccgcacgccctggtgcgacgcgtgctccagcaggtgccaatcgaggctgcggtcggcgttccattcggccccctgggcgaattcgccacccatgaacagcagcttttttccggggtaggcccagaggtagccgtagagattgcgcagccccgcgtacttctgccactcgtcgccgggcatgcgcccgaacatcgagcccttgccgtgcaccacttcgtcgtgtgagagcggcagcacgaagttctcgctgtgcgcatacatcagcccgaaagtgatctgctggtgatggtgcttgcgatggaccgggtcggtgccggcataggccagcgtgtcgttcatccagcccatgttccatttgtagtgaaagcccagcccgccgtcttcgggcggccgcgtcacgccggggaaactggtcgactcctcggccagcgtgacggcgcccgggcgctccacgcccaccacgcggttcatgcggcgcaagaagtcgatggcctcgaggttctcgcgcccgccgtatgcgttgggcacccattcgccgggcttgcggctgtagtcgcggtagagcatggaggccaccgcatcgacgcgcaggccatccacgccatagcgctcgagccagtagagcgcattgccgaccaggtagttgcgcacctccgtgcggccgtagttgaagatgagcgtcttccagtcgttgtggaagccttcgcgcggatcggcgtattcatacagcgcggtgccgtcgaagcgacccaggccgtgcgcatcggtgggaaagtgcgcgggcacccagtcgaggatcacgcccagccccgcggcgtgcgcggcttcgacgaaatgccgaaagtcgccgggcgtcccgaagcgcgaggtgggtgcatacagaccgatgggctggtagccccatgagccgtcgaacgggtgctcgctcaccggcagcagctcgatgtgcgtgaagcccatgtcgcgcgcgtagggcaccagcgtgtcggccagctcgcggtagtccagccattcatggccgttcttgcgccgccacgagcccaggtgcacttcgtagatgctcatcggcgcatggcggccgttggcggcggcgcgctcgggcggcatggccaccggcgcgggcagcggcgccaccacgcaggccgtttcgggccgcaggcgcgcggagaaggcgaaggggtcggccttgcgcagcacctcgccctccgccgagagaatctcgaactcgtagctgtcgcccgtggccacctgcggcgcaaagatttcccacacgccgcattcacggcgcagccgcatcatgtggcgccggccgtcccagttgttgaagtcgccgaccaccgacacgcgccgcgcattgggcgcccagaccgcaaaggccacgcccttcacgccgtcgatctcgcgcagatgcgcgcccaaccgctcccagggccgcaggtgcgtgccctcggccagcagccacacgtcggtgtcgccgagcacgaaaggaaagcggtaggggtcgtcgagccgcgaggtgtgcgtgccccagtcgacctggaacgaatagcccagcagcgcctcggccgccggcacgaggcccgtgaacaggtcggagccttcatgccgcgacagcacggacagcggccagcccgtgcgcgtgtgcatcacggccacgctctgcgcgccgggcaagagcgcgcgcactgccagcccgtcgcgtgtctcgtgaggacccagcaccgcgaacggatcgccatgctcggcgcgcatcagcgcgtggacttcgcgttcgggcagttgcatcgggggcatgtccttcaaatccgttgttcttcttcgccagcgggtcgaccgaaaaagacgccgtagggcgccagcctcagcatgcgccttttttcgccatcggcctgcaggcgcgcgtcggccgacggtggatgcggatggcccggcagcggctctagcggctcgcgcagcgcgaccgacacggactcgcccccgaggttgaagatcgcctgcagcgaccgcttcccgtcgcgccgctcgaaccacagcaccggctcgggcgcatcgaagaaggtgatgctgcccgtgcgcagcagcggctggctgcggcgccagcgcagcagtgcacggctgaacacgagcatcgagtcggggtcgctggtctgtcggtcgacggccagcggcaagtggcggccgtggaccggcagccacggcccgccggtggtgaagccggcgtgcagctcgtccgccttccagggcatgggcgtgcggcagccgtcgcggcccttgaactcgggccagaacgcgcggccgtacgggtcttgcagcagttcgaacggcacctcggcctcgggcaggcccagttcctcgccctggtagatgctggcgctgccgcgcagcgtgagcagcagtgtgagccagagccggtcgcgccgggtgtcttcggacgcaccgccgctccagcgcgtggccacgcgcggcacgtcgtggttggacacggcccagcagccccagccgcccgtgggcgcgagggcatggtcgagcgtctcgacctggtggcgcagatggctggcgctgtgctcggccgtcagcaggctgaagctgtaggccagatgcaggcgcctgcccagttcggtgtactgcgccatcaccggcggcgcattctcgtcgcccacctcgccgagcgcgacggcgccgtagccgtcgaggagctggcgcaggttttcgagaaagagcaggttctccgtctggctcttgtcgtacaggtgctgctgcatcgcgtaggggttgtcggcccggacggtgctcacttcatcgaccgatgcggcgctggccggcgggttgtcgcgcaagagcgcgtcgtggaactggtggttgcaggcgtcgaagcggaagccgtccaccccacgctcgcaccagaagcgcacttcgcccagcaaggcttcctgcacctcggcgcaatggaagttcaggtcgggctgttccttgaggaagctgtgcagatagtactgccggcggcgcgaatcccattgccaggccgagccgccgaagaccgagagccagttggtgggcggcgtgccgtcgggccgcgggtcggcccacacgtaccagtcggccttggggttgtcgcggctcgcgcggctttcggcgaaccaggcgtgctcgtcggaggtgtgcgagagcacctggtcgatgatgatcttcaggtccagcgcatgggcgcgcgccagcatttcatcgaaatcggccagggtgccgaagatcggatcgacgtcgcggtagtcggccacgtcgtagccgaagtccttcatcggcgagcggaagaagggcgacacccagatcgcatcgacccccaggcccgcgacgtgctcgagccgtgaagtgatgccgggaaggtcgccgataccatcgccgttgctgtccatgaagctgcgcgggtagatctggtagatcaccgcgccgcgccaccattcgctgttgctgccgtgattgctgcgcatgctgtccctgtggtctgaaaatcattgtggcatgcgagatccgggcccgatccatgcaaggctcggccggcgctcctcaaaaagctttctacactgggcgcgggtttccagaatgtgaaccctggctttcagttccgtttccgcaagatgaccaccgactccgcttcccccgcactttctccatcggcagaaggccttgccgcgctcgagcagcggcttgccaaggacctggagtgcctcggctggcccgcgcgcgcctggctgcccgttcgcgagcacgcgggccagccggtgctggacgtggccatcatcggcggtgggcaggcgggcctggcggccgccgcggccctggcgcagcaaggcatccgggccgtcgtcttcgaccgctcgccggcgggcaacgaaggcccgtgggccaccacggcgcgcatggaaaccctgcgttcccccaaggaactgaccgggccggcgctgggcctgcccgcgctgaccttccgtgcatggttcgaggcccagttcggtgccgaggcctgggaggcgatggacaagatcccgcgtctccagtggatggactacctgtcctggtaccgccgcgtgatgaacgtggacgtgcgcaacgacaccgccgtcaccgggattcggccgctgcccgatgcggcgctggtgcggctggaactgcgcacccccgccggaacgcagcaggtgctggcacgccgcgtcgttcttgccaccggccgcgatggccttggcggccccgccgttcccgcctttgtcaacgcgctgccgcgctcgcaatgggcgcactcgtccgacgccatggactacggcaggctggccgggctgcgcgtgggcgtgatcggcgcgggctcgtcggccatggacagcgcggccaccgcactggaggccggcgcgcacagcgtcgaactgctgatccgccggcccgacctgccgcgcgtcaacaagggcaagggcgccggcgtgccgggcctgacgcagggccactacgacctgcccgatgagttcaagtggcgcatccgccactacatcaacgtggcgaacgtgccgccgccgcatggcagcacgcttcgcgtctcccggtttccgaacgcgttcttcaacttcggctgccccgtgctctcaatcgagccgcagggcacgtcgatgcgcgtggccacgcccaagggcgagttcgtgttcgactttctcattgtctcgaccggcttcaagatcgactggaacggccgtcccgagttcgacgccattgcgtcgcacgtgcgcacgtggaaagaccgcttcgtgccggcgcccggcgacgaagatcaggaactggccgattcgcccgatctcgggccggcgttcgaattccagccgcgcgcggcgggcgaatgcccggggctcgaccgcatccattgcttctgctaccccgcggccctgtcgcacggcacggtgtcgggcgacattcccgcgatcagcgaaggcgccaggcggctcgcgagcggcgtggccagcctgttctaccgcgaagacttcgagcaccacttcgccaacctcgaggcctacagcgagcccgaactgttcggcgacgaatgggtgcccgcgccgccgcccgccgaacggacctgaattgcagaccctcatttttcgaagcgcatgacaacttcctacgacgcatctccttcgatcgacgtgatcgacgccacggtgccgctggcgcccggccaggccacccgcacactgcggctgcagcgcgacaaggtcgtggcggccacgcagggcagctacgacgcgatgttttcacccaccgtcgagggcctgtcggtggcagagcgcctgctggttgcgctgcacgcctgcagcgtctccaaagccgcgacgcttgccgcgcattaccgcgagcgactgctggccgagggcgcggaccgcgagttggtcgcggccgtgggaagcggcgccccggtggcggatgcgcgcctcggcacggtgctggcattcaccgccagcctgatcgagcgtcccatcgagggcgacaaggcctcggtcgacgcgctggccgaggcggggctttcgacgcccgccatcgtcgcgctgggccagctgatcgccttcttgtcctaccaggtccgcgtggtcgcgggccttcaggcgctggccgccgcggaggtatcgccatgaccgcgccgattcgcatcaacggtttcaccaacgaggtgctgagctggaagccctggctcgatccggtcgttgtcgccacggccacgccggctcagctggcagcgctcgacgagatgagcccgcaagcgcgcacctcgccctattttttggtgctggcgcaccagcccgagatgctgctgcagcgctccatcgccttcaacgcgatcatgtttgcgccgggaggcatgccgcgggccgaacgcgagctgggtgccacggtggagtcgcgcgtcaatggctgcgtgtactgcgcctcggtgcatgcgcagcgcttcgagcagcttgccaagcgcaacgacgtgatctcgcaggtgttcgaggagccggcttccgcgggcaccacggcgcgcgagaaggcgatcgtcgaattctcgatccgtctcggcgccgagcccgacaaggtgtcggccgaggacgtgcggacgctgaaagaagcggggctgagcgaactcgagatcctcgacctgatccactccgtggcactcttcgcctgggccaaccgcctgatgctcaacctgggcgagccggtctttcccgcggcggcagcgtcataggcgggcgagcagcccggccacggtctcacgggcgaggccgagcggctccagcaggtcgttctgctgccggtagtcgatgccgttgaccagcgaggcggcatccacgatggtgcgggtcgctggcgtgggcacgccggcaatcctgcccaacgcctccacgaaagccaggccgtagggcatgtcttcggacacatagcgggtgtcggtgcgcacgggcccgggcgggccgccgcgcttcgcatgcaattcggcggcgatgtcttcgagccgcgtcgacgtggtgccgaaggagcgcccgaagtgttcttcgatgggaccgagttcgatgccaaaggcttgggccacggcgcgtcgttccaggtccagcgcctcgatcgcgcgggacaccccgggcgtcatgcagtggtactgcggccagttttcggcacgctcgatgcgggtccagttgaagacggccagtgggccgtgggactgcgggttgacgttggccaacgcgctggcgagcgtgttttgctgcgcgaagaagccgccgccgaacaacgcggcgcacagttcgagcaccccggcgatgccggcacccggcagggcggacacgccgaccgcctggcgccgcgtcatcacccgcacctcggtgcccgattcccggcgcgcggtcagcaccgtggtgccaaagctcgcgacggtgatccgccggcccgcacgccgtgcgctttcgtaaaggtagagcgacgacagcgaggccatcgagctgacgatcgccgtctgcccatcgcgcaggaagggcaatagcgcatccatcacgcgccggtggccattgaccggcagcgcaagcagcagcacgtccgaggcgtggcaaagctgcgctgcatcgtcggcgacgtcgaccgtgacgctgcacggctgcacgccgatggcttccagcggttgcgtgcgcaaggcctcagcgccccggccgcccggcgaccagagcatgacgtcgtggcctgcctgccggagccacgccgcactggccaacgcaatcgctccggtgcccgcgatgccgacccgatacaggccgccagccaccgtcatcctgcgggcccccttcgcgaacaccgcggaaccggctctgccgggccgccggtgttgcccccggtgagggggagggagaagcgacacgaagtgcgcgaagcctgggggagagccacgtcactcaaccttgatcccgccctgcttgattactttggcccagcgctggctgtcttcggcgatcaccttgcccagcgccgcgccgctgccgcaggtgttcaccgcgccgagctgggcgaagcgctgcctggtttcgggcaggttgcacacctcgaccagcgccgcggaaagtttctcgacgctggccgccggcatgcgcgcgggcgccatcacgccgacccataccggcacgtccatgcccgcgagccccgccgcctcggcgacggtgggcggcgtgccgaggctgggcagcgccgcgcgcgagaaggtgccgagcacccgcgccttgccgctcgcgaccatcggctcgatggaggccgcgctggtgacgatcagcgccacctggccgcccagcaggtcggtcagcgccggtgccgcaccgcggtagggcacatgcagcaggttcacgccgctcgcctgtgccagcagcgcgcccgtgaggtgcgacaccgtgccgttgcccgtggaggcataggtcacctgccccggcttggccttggcatcgcgcagcacgtcggccaaggtcttgtaggggctttcggcgcgaacggccagggtcatcggcgtgtcgccgaccagggccacgggcgccaggtcgtgcacggggtcgtagggcagcttcgcctggagatgaggcgcgatggtgatggcgccgccggtggccagcagcacggtggcgccgtcggtcgccttggccaccgcgtcggccgccacgatgccgcccgcgcccgccttgttgtccacgatgacggtggcgcccagcttgtcgccgagcttggcgcccaggtagcgggcgatcacgtcctgcgccccgccggccgcgaagggcaccacgatgcgcagcggcttgtcgttgttctgctgcgcgtggagcggcatcacggccaggctggcggcggccgcgaggcccagtgtcaggtatttcaggagcagtttcatggcattccaggcggtgcgaaaaacctgccggagggcaggcgttacccgcgcaacacgcaggttacgtgcctcaagtctagagtctgccggcccgggaggccgcccgggcgcgataatccgccttccccggccgctccgagccgggctctgccgaaccgtcatgaaccccagctacaaacccagcgacgtcgagtccgctgcccaggcgcaatggagcgccgccgatgcctaccgcgtcaccgaggacgcgagccgcaagaagtactacgcctgctcgatgctgccgtaccccagcggcaagctgcacatgggccatgtgcgcaactacaccatcaacgacatgctcacgcgctacctgcgcatgagcggctacaacgtgctgatgcccatgggctgggacgccttcggcctgccggccgagaacgcggcgctcaagaacggcgtgccgccggccaagtggacctacgagaacatcgactacatgcgcggccagctccaggccatgggcctggccatcgactggagccgcgagatcgccacctgcgatccgagctactacaagtggaaccagtggttgttcctgaagatgctcgaaaagggcattgcctaccgcaagacccaggtcgtcaactgggacccggtcgaccagaccgtgctggccaacgagcaggtcatcgacggcaagggctggcgcaccggtgccacggtcgagcgccgcgagatcccgggctactacctgaagatcagcgactacgccgaggaactgctcgagcacacccagcacaagctgccgggctggcccgagcgcgtcaagctgatgcaggagaactggatcggcaagagcgagggcgtgcgcttcgccttcacgcatgacatcaaggatgcgagcggcaagctgatccaggatggccgcatgtacgtgttcaccacgcgcgccgacaccatcatgggggtcaccttctgcgccgtggcgcccgagcatccgctggccgtgcacgccgccacgctcgatcccaaggtcgcggccttcatcgaggaatgcaaggccggcggcaccaccgaggccgagctcgccacgcaggagaagaagggcgtgcccacgggcctgaccgtgacgcatccgatcaccgacgagcaggtgccggtgtgggtcggcaactacgtgctcatcaactacggcgacggcgccgtgatgggcgtgcccgcgcacgacgagcgcgacttcgcctttgccaacaagtaccgcatcgagatcatccaggtggtgctggtcgacgacgagccgcacttcgactatcacaagtggcaggactggtacggcgacaagcagcgcggcgtgaccatcaattccgacaacttcagcggcatgacctacaaggaagccgtgaccgccgtggcgcatgcactgagccagaggggcctgggcgaaatgcagaccacctggcgcctgcgcgactggggcgtgagccgccagcgctactggggcacgccgatcccgatcatccattgcgacgagcacggcgcggtgccggtccccgagaaggacctgcccgtggtgctgccgaccgactgcgtgcccgacggctccggcaacccgctcgccaagcacgaaggcttccacgccggcgtggtgtgcccggtctgcggcaaggccgcgcggcgcgagaccgacacgatggacaccttcgtcgattcgtcgtggtacttcatgcgctactgcgacccgaagaacgaccaggccatggtcgccgagggtgccgattactggatgccgatggaccagtacatcggcggcatcgagcacgcgattcttcacctgctgtatgcgcgcttctggaccaaggtgatgcgcgacctgggcctcgtgaaggtcgacgagcctttcagcaagctgctcacgcagggcatggtgctgaaccacatctactaccaccgcgacgagaagggtggcaagaactaccacccgccgctggaggtcactcccgtgctggacgcgcagggccgcatcgtcggcggcaccaccgccgacggcaccaaggtcgagtacggcggtgtcggcaagatgggcaagagcgagcgcaacggcgtcgacccgcaggacctgatcgaaaagtacggcgccgacaccgcgcgcctgtacaccatgttcaccgcgccgcccgaagccacgctcgagtggaacgacgcggccgtcgaaggcagctaccggttcctgcgccgggtctggaacttcggcgtggcgcagtccgacgtgcagcccgcggcagtgaagggcaaggccttcggcaaggccgcccaggcgctgcgccgcgaagtgcacaccctgctgcgccaggtcgactacgactaccagcgcatgcaatacaacaccgtggtgtcgggcgcgatgaagctgctcaacgcgctcgaaggcttcaagccggacggcagccctgccgatgcggccgcgctgcgcgaaggtttcggcatcctgctgcgctgcctctacccggccacgccgcacatcgcctgccagctctggcaacagctcggctacgacaaggagctgggcgatctgctcgacgcaccctggccggtggtggacgtcggtgcgctcgaacaggacgagatcgaactcatgctccaggtcaacggcaagctgcgcggcgcgctgcgcgtgccggccggcgcctccaaggccgagatcgaggaactcgcgctttcgtgcgacgacttcgtcaagttcgccgaaggtgcgtcgcccaagcgcgtcatcgtggttcccggacgcctggtcaacgtggtcatttgaacgatagaagcatgaacaatcgcatcgcctcgctgccgcgccgcggctttttcctgggtctcgccgcggcgggcgccagcctcggcctggccggctgcgggttcgaactgcgcaaggcgccggtgttcgcgttcaagacgctgtcgctgtcgggcaattcggagctgatcaaccgggtgcggcgcgaaatgcgggccgcgggcaccgtcacgctggtgccggccaccgaggcgcagaccgccgacgcgatcctcgagatcctgggcgagaaccgcgaccgcatcgtgatctcgaccaattcggcgggcctgctgcgcgagttgcagctgcaattgcgcgttcgcttcagcctgcgcacgccgggcggcaaggttctgctggcgcccaccgaggtttcgcagacgcgcgacctgagcttcaacgaaaccaatgcgctcgccaaggaaggcgaggccgagctgctgtaccgcgacatgcaggccgacatcgcgcagcagctgatgcgccgcctggcggccgtcaaggaaatctaggccgaggcctctgccctgcgatgcaacttgccagcgcccaactgggctcccatctgcagaaggggctgaagtccctctacacgatccacggcgacgagccgctgctcgcgcaagaggcggcggacgccatccgtgccgcggcgcgcgtgcagggctacacggagcgcagctcgtacaccgtggccggcgcgcacttcgactggagcgcggtgctcgcggccggcggctcgctttcgctctttgccgacaagcagatcgtcgagatacgaattccctcgggcaagcccggcaaggacggcagcacggcgctgcagcagttggccgaggcggcacagggcaacgacagcacgcttaccttggtgatgctgccgcggctggacaaggccacgcgcaccggcgcctggttttcggcgctcgagaacaacggcgcgaccctgcaggtcgacccgatcgaacgcgcagccttgccgcaatggatcgcgcagcgcctgggcttgcagggccagcgcgtgatgccgggcgacgaggggcagcgcacgctgcagttctttgccgaccgcgtcgagggcaacctgctggccgcgcaccaggaaatccagaagctcgccttgctgcaccccgcgggcgagctgagctgggagcaggtcgaaggcgcggtcaacaacgtggcccgctacgacgtgttcaagctctcggaggccgtcctggccggcaatccgcagcgggtggcgcgcatgctcgacggcctgcaggccgagggcgaggccgaggtgctggtgcactacacgctggccgaggacatccgcgcgctcaagcgcgtgaaagatgccatggcctcgggccggccgctccccatggcgctgcgcgaaaaccgcatctggggtccgcgcgagcgcgccttcgaacgcgtgctgccgcggctggacgaccgaatgctggcgcggctgctgcgcgccgcgcatgtggtggacggcatctgcaaggggctgaagcagcccgactggcccgcgagcggctggcaggctttgcagcgattggccttgatgttgtgccgcgcctgcagcagcggtccagctccctcttcctccgggagagggttgggatgagggccggcggccgtcatcacatcgcgcgttttcgagtgccgcggccctcaccctagccctctcccggagggagaggggacaacacggcaagggtccaaagcccggggttgatccaaatgcaggaaaatgccggcatgaatgcgttcaacgtcagcgagcacatgcaggccctcggcctgcaggcaaaagccgctgcattcctcatggcccgtgcggatgcagctaccaaaaacagagcattgaaggcgctggcccggcgcctgcgcgaagccggcccggccttggccgaggccaacgagaaagacctggcgcgcgccatggccgccggcctttccgcgccgatggtcgaccgcctgaaactcacgcccaaggtcatcgagaccgtggccctgggctgcgagcagctggccggcatggccgacgtgatcggcgagatcatcggcatgaagcagcagcccagcggcatccgcgtgggccagatgcgcgtgccgatcggcgtcttcggcatgatctacgagagccgccccaacgtgaccatcgaggccgcgagcctcgccatcaagagcggcaacgcagccatcctgcgcggcggctccgaagccatcgagtcgaacaaggcgctggcgttgctggtgtccggggcgctgtccgaagccggcctgccggtggatgcggtgcagctggtgcagaccaccgaccgcgaggccgtgggacggctgatcgccatgcccgagttcgtggacgtgatcattccgcgcggcggcaagggcctgatcgagcgcatcagccgcgatgccaaggtgccggtcatcaagcacctcgacggcaactgccatgtctatgtggacgacacggccgagttcgaaatggcgctgcgcatcgtcgacaacgccaagacgcagaaatacagcccctgcaatgcggccgaaggcctcctggtgtcggccgcggtggcggaagatttcctgccccgcatcgcggccatcttcgcggccaagggcgtggaaatgcgctgcgacccggtcgcggcccgcatcctgcgcgccgacgacaccctcggttcgggcgcaagaatcatcgacgcggtcgagtccgactggtccgaggaataccttgccgccgtgatcagcatcaaggtggtcgaaggggtcgacgaggccattgcgcacatcaaccgctactcgagccaccacaccgacgccatcgtcacgcgcgaccacgtgcatgcgcagcgtttcctgcgcgaggtcgattcggccagcgtcatggtcaatgcgagcacccgcttcgcggacggtttcgagttcggcctgggagccgagatcggcatcagcaccgacaaatttcacgcgcgcggaccggtcggcatcgaagggctgacctcgctcaagtacgtggtgctggggcagggcgaagtgcgcagttgatgcccggtgagcaggcggactgaaccaagtccgctgtacgtagtcttgtcattggggcggccacccccaaatcctacaattccgctctacctttcaagtacaaatccaacaaggccgccgcatggttccgcatctcgtcaccgccctgaccggcccgatcaacgaactggagcagcgggtactcgactcgacgcccgccatcgagcgctggtttcggctcgaatggatggagcacacgccgccgttctacagcgcggtcgacatccgcaacgccggcttcaagctggcgccggtcgacaccaatctgttccccggcggctggaacaatctcaccaaggagatgctgcccctcgcggtgcaggccgcgcaggccgccatcgaaaagatctgtccggaagcgcgcaacctgctcgtcattcccgagaaccactcgaagaacaccttctacctcgccaacgtcgcgcaactggtgcgcatcttccacatggcgggactcaacgtgcgggtgggctccatcgatccggcgatcaagtcgcccaagaagatcgagctgcccaacggcgaaacggtgtgcctggagcccgtggtgcgcagcaagcgccgcctcgggctcaagaatttcgatccctgcaccatcctgctcaacaacgagctgtcggccggcacgccgggcatcctcgaagacctgcacgagcaatacctgctgccgccgctgcatgcgggctggtcggtgcgccgcaagagcaaccacctgcacagctacgaagagctgtccaagcgcttcggcaagctgctgggcatcgatccctggctgatcaaccccatttatgcgcggggcgatagcgtcgatttcgccgaaggccgcggcatcgacgtgctgaccagccacgtggatgcggtgctgaccaaggtccggcgcaagtacaaggaatacggcatcaacgaaaagcccttcgtggtcgtcaagggcgacaccggcgccgagggcccgggcgtgatcacgatccgggacgccaaggaggtcgaagccctggtcggcaagccacgcggcgcttcgttgggcaaggctgctggtgcggcccgggaactgcgcgagcccggcgaggtgatcgtgcaggaaggcgtgctgaccaacgagcgggtgcacaacggcgtggccgagccggtggtctacatgatggaccgctacgtggtgggcggcttctaccgcgtgcatgccgagcgcaaccccgacgagaacctgaagtctccgggcgcgagcttcgtgccgctggctttttccgagagtgcgcacttgccgcagcccggcgccaagcccggcgcgagcgcgccgaaccgcttctacatgtatggcgtggtgggccgcctggccatggttgcggcgagttacgagatggaagccaccgatccggacgccgaaatctacgaatgattttccggggcggcttgcggcggcggcggtcggcggcaaaatagcggccccacagcaaaggaaacaaaagggcggaagggatgtgcgcggcgactggaaattgattccaccgctgctgcgtctcggtgcgtgtgacctccggttacgcgcttgcagcctgccctttttcccatcgacttcgtgtcacctcccaaatcttcttccgccgccgccttgatcatcggcaccatcggtgtcgtctatggcgacatcggcaccagcgtgttgtatgcagtcaaggaagtgttcggccacggccacctgcctttcactgtcgaaaacgtctacggcatcctgtcgatgttcttctggacgctcaccgtcatcgtgtcgatcaagtacgtggtgctggtgctgcgggccgacaacgaaggcgagggcggcctggtcgccatgctggcgctggcttcgcgcgcggtggccgacaagccaaggctgcgcaacgtgctgctgctggtgggcatcttcggcacctcgctcttctatggcgacggcgtcatcacgccggccatctcggtgctttccgccgtcgagggtctcgaagtggtgtccccccacttcaagcactatgtgctgccagtcacgctggtggtgctgttctgcctcttcgtggtgcaaaagcgcggcacggcgggcatcggcaagttcttcggcccaatcacgctggtgtggttcctcgtcatcgcggtgctcggcgtgtcgcagatcatccaccatcccgagatcctcaagtcgctgaatccctggttcgcgctgaagttcatgtgggacaacccgggcacggccttcatcctgctgggcgccacggtgctgtgcgtgacgggtgccgaggcgctctatgccgacctcggccacttcggcaagcggccgatccgcgtggcgtggttcacggtcgtgatgccggcgctcacgctcaactacttcggccagggcgcactgctgctcgagaaccccgaggccgtgaagaaccccttcttcatgatggcgcccgaatgggcgctcatcccgctggtgctgctggccacggcggccacggtcattgcctcccaggcgctgatcaccggtgccttcagcgtcacgcgccaggtcatccagttgggctacctcccgcgcctgaacatcgagcacaccagcgtgcgcacggcgggccagatctacattccgctggtcaactgggggctgttcgtcgccatcgtgctcgcggtcgtcatgttccgttcgtcgagcagcctggccgccgcgtacggcattgcggtgaccaccgacatgctcatcaccacggtgctgaccttcttcgtgatccgctacgcctggaagctgccgctggcgctgtgcattgcatcgaccgcggtcttcttcgtggtcgacttcctgttctttgcatcgaacctgctcaagctgttcgagggcggctggttcccgctggtgatcggcggcgcggtgttcacgctcatgatcacctggaaggaaggccggcgcctgatgggcgaggtgcagcgcgccgatgccatcgagctgcaggccttcctcgactcggtgttcgagaacccgcccgcgcgcgtcgacggcaccgcggtgtttctcaccgccgaacccggcgtggtgcccaacgcgctgctgcacaacctgaagcacaacaaggtgctgcacgagcagaacctgttcgtcacggtgcgcaaccacgaagtgccctggatcccgatgaacaagcgcatcgagatcgacgccctaggccaccattgctggcaggtcatcgtgcactacggtttcaagaacgacatcgacctgccgcgtgcgctcgacaacgcgcgcatgcgcggctgccagctggagccgatgacgacgagctacttcctctcgcgcgacgtcgtcattcccacgctgggcagcggcatggcgccgtggcgcgaaaagctgttcgcgcagatgcatcacaacgcgagcggcgcggcggcattcctcgggttgccgaacaacgccgtggtcgagctcgggtcgaagatcgagatctgagggactgcgcggccgctgtgttcacgcgcgccgccttcctcatgcaaagtccgcgggccgatccgccgccagctgctgcatgtgcgatgcaatggcgcccggcgtggtgacccagatgtcgccgcggtcgcgggcacgcgcgatgtgcgcgagcgccgtgcgcagatggcgcagccggtaaggctggcccacgatgtagggatgcagcgcgagccccatcaccagcggctgcgcgcgtgattgctcgcgcatctcgtcgaagttgtcgacgaccatcgcggcgaagtcctttgcatccatcgagcggcccatgatcatcgggatgtcgttgagctcctgcggatagggcaccgaccatatcgagccgccgccccgtgtgcgcatgcgcaccggctggtcgtcatggcaccagttgagcgtgtagccatagccggtttcggccagcaggtcgggcgtgaccgcgctttccgatatccacggcgacaaccatccggcaggtgccttgccgctctcctgctgcatgcgttcgcggcaacgcagcagcagtgcgcgctcttgcgtttcgtcccatgcgccctggcgctccgcgttgctgtggccgtggccgatcagttcgtcgccgcgcgcgacgaaggcccgcaccacctccggacaatggtcgtacagcgcggtgttgatgagcgcgcccgtcggcagtgccagcgcatcgaacagttcgaggcagcgccacgcgcctacgcggttgccgtattcgcgccagccgtggttcagcacgtcgggctctggcgaggccgggccgatgcatgcgcccaagccgtcgccgaacgcgaaatgctcgatgttgaagcccaggtacacggccaggcgcgcgccgttgggccacgcatagtcgggccgccgtgtgatggggctgtagtcgaagcggccgtgcgcgggcagcaggttgggccagcgtgccgtcatgtgccgtgcctcacagtaccgcgagcccggcgcgcaccagcagccattcggcgctgtcgttccacacgtccatctgcacgatgagcccgtggcgcaccacgtagcggtcgacatagcgattgccctcgaacgccgtgccgtcgggccacgcgccgtagagcgtgccgaggctgtagaccaccgtttcgtcgggcgtgccgcctgcgaccacttcggtgcgttcgatcttcttcttgacccaggcgtagcgcttcgcattgaaggccgaggtgtcgccgggcgcatgcatttcgcggttgccggtgaagcggatgcggatgccgggcgcggtgtggcgggaggccgattgcgggtccgggatcatcaccaggcgaaggaattcgtcgaccacctcggccggcgtggaagggacgggcagtgcatcgagcgaagcaagggcggtcatgggttctccatttggagccacggcagtgcatggcggaaggcatgaggggccaaagcaaatcctgcgccgaatctcttcggcgttgcggtcccggcggccccggcacaatcgcccgatggcgcacaaaggcctccgccggcaagggcatcgccgcttccggcaacatcgcgccagacatcaacatggcggccacacccggcgccggaaagactcccagatgaaaaacattctcttcgtcgccgatccgctcgaccacttcaagatctacaaggacaccacgttctcgatgatgcgcgaggcgcagcgccgcgggcaccgcatcgcggcctgcctgccggaagacctgcagtgggtgtcgggcggcatggtaacggccaacgtgcagcagatcacgctcaccggagacagcaaggcctggtaccgcgaggacatctgcgaatcgaaggcgctgaaggaattcgacgcggtgctgatgcgcaaggacccgccctttgacgccgagtacatctacgccacccacctgctcgaacaggccgagcgcgaaggcgcgcgcgtggtcaacaagccgcgctcgctgcgcgaccaccccgagaagctcgcgatcatggagtttccgcagttcaccacgcccacgctggtcacgcgcagcgcccaggccgtgcgcgacttccatgccgagcacggcgacatcattttgaagccgctcgacggcatgggcggcatgggcatcttccgcgtccggcaggacgggctgaacctcggctccattgtcgagacgctcaacaagaacggcgccgaaaccatcatggtgcagcgcttcgtgcctgacatcgtgcagggcgacaagcgcatcctgatcatcgcgggcgagccggcgccgttcgtgctggcgcgcattccgcagggctccgaggtgcgtggcaacttggcggccggcggcaagggcgtggcgcagccgctcacgccgcgcaaccgcgagatcgcggaaaccgtgggccgggccctggcgccgcgcggcctgctcctgatcgggctcgacgtgatcggcgactccgtgaccgagatcaacgtgaccagcccgacctgcttccaggagatcaccgaacagaccggcttcgacgtgccggccatgttcatcgatgcgctggaggcgcagctggccggcggctgaggccggcccggttcagaacggcgcccgctgtccgtccacgaacacgtgcagttcgccgggcgcgaacgcggtccagtgctcgttggtggtgagcggcgcggtcaccaccaccgccacgcggtcattgggcgtggtgtgcttggcaaagtcgatctccaggtcttcgtccgacagctgcgccgtcacgaacggatggcggcgctccacgtaccagaggtgggtcgaagcgtgggcccagagcgcctggccgttcgacagcatgaagttgaaggtgccgtgtcccgcaagctgcggcgccagttcgcgcagcgtgagcgtgagctcctcgatgctcggcacgcctgcgtgcgacttggccagttcctgcatcagccagcagaaggcgtgctcgctgtcggtgttgcccaccgggtggaagttgccgtgcaggcgcggcctgaagtccttcaggtcgccgttgtgcgcaaacacccagtagcggccccacagctcgcgcacgaaggggtggcagttctgcaggttgatggcgccctgtgtcgccttgcggatgtgcgcaatgacgttgcggctctggatggggtagcgccggatcagctcggccaccggcgactcgctcgccggcatgtgatccacgaagtggcgcagcccccggtcctcgaaaaacgcgatgccccagccgtcggcgtggtggtcggtgcggcccccgcgctgggcgaagcccgtaaagctgaaggtcacgtccgtgggcgtgttgcagttcattccaagcagttggcacatggcgctattaaagcgcgtgtgccagccgccgggcgaacccgcccgcccgttcagcgcacgaatcggccttcgggcgtgacgcgcaccatttcgatgaagcgcgagccggtggtggcgccggtcgaaaagtcgatgtccatgccggccaggcgcagcttgaacgcgcgcagcgtcgcgtgcaggcgcgcgcgcgtcaggtcgcgcccggtgcgcttgagcgcctcgatcatcaccaggccgttcagatagccctcgaagctgccgtagcccaccggcacctgggcgcgttcggccagccggcggtagtcgcgcgtcaccgtttcgacttcgccccaggggtacggcatgacctgcgagatggccagcccgctggcctgcagttgcaccaccttggccgtgatctcgcccgggacgaccgacatgccatagaacatcggcttgctgccggcctcgtaggtggacttgatcacctcgccggccaccgtgccggccaggtacatcagcacggcctgcggacggctgtccgccagtgccttgcctgcggcggcggaggtcgagccgtcgcccttgaccgataccaccgccgtcggagtctgcttgtgcgtggccatggccgcctcgatcagcttcacagcctcgacgccgccgggattgtccaggtgggcaatcgcgatcttgttcacgccgatggtgatcaggtgctcgaccagcgcctgcgcctcgcgtgcattgctggcgcgcacgaagtacgccgagcccgccacgcgttcgcgggcgctgtcgcccacgccatagccgccgacgctgggggcgccgctttgctgcagcagcttggatgcggcggctgtggtgcctgagcccacgcagccgaagaacgcgaacaccttgtggtcgctcagcagcttgccgtagttctccagcgctttctcgggtttcagttcgtcgtccagcgcgatcagcttgatcttgcgtccgcccacgccgccctgttcgttgatggcgtcgaaggccagcgccgcgccgttgtgcaccaccttgatctgcgagccgagcgggccgctcaggacggccgagctaccgagcaggatctcgctgtcgctcacgccaacttcggcggcttgtgcggatgacagacgagccaggcccgcggcgaaaaccgccgtggaggcgacaaaacttctgcgttgcatgagtagcccattccatcattaactaacaacattaacaattagaaacgatggatgcttaggtattacattgggagtaaccctagctgtttggtcggcgcaactgccacgcagcgcaaatggccagcgcgcacagcgcggccagcatcagaaacacctcgtcgaaggccgccagccgcgcggggctggttgcggcattggccagcgaatcgccatgcgctgccaggcgccactcgagcacgatggcgcacaggctcacgccggccgcgccgcccagcatgcgcaggaagttgatcgcgctggcgccctgcggaatcagcggcttggccagcggccgcatcgagccgaggttgagcgaaggcaggatgaagccgagcccgatgcgcccgatgatggcaaacgccaccagcagccagagcgcgctgtcgagccggagcaccatcatcagcgcgaaggaggccgccagcagcgccagcccgatgctcaccagcagccacgtcggctgccggtcggccagccggcccacgccggcaatggtcacggccagcacgatgcccgccggcagcaggatggtgcccacgtgcgaggccgacagctgcagcccgacctgcatgtacacgggcaagaggtaggtcgagccgaacagcgccgtgccgtagatgaaggcgaccacgctgcccatggcgaactgccgatactggaagagccccaggttcatcagcggttcgccgccgccggccgcgatccggcgctgccaccagacgaagccggcaaaagccagcaccgcgccggccagcagcaggccggcctgcagcggcgaatcgccgcgcagctcgaccagcccgttcagcaagcagagcgtgcccacggtgcccagcgccaggccgcgccagtcgagcccgctgccgcgcgtggcagccacaccgccgggcgccgtggtgggcacgaacttgtaggccagccacagcgaggccaggcagaagggcaccaccatgaagaagatcgagcgccagccgaacaggtcgaccagcacgccgccgatgctggggccgatggccggcgccagcaccacgcccatgccgaagatgccgctggcgcgcccctgctcatggggctcgaaggcgcgcaggatgatgatggcgggaatgggctgcaccacgcccgccgccagcccttcggccacgcgcgccagtagcaccagcgagaagtcgttggccacgccgcccgcaatgccgcccgcgagcagaagcgccatggtgcccgagtaagtgcgccggtagccgtagcgcgacagcagccagggcgtggtcagcatcgagactgtcatggccaccatgaagcccgagctcacccattgcgcccgctcctggccgagcgagaagtggtggctcatgcccgggatcgccacgttgacgatggtcgaggacatgatcgacgccatcacccccaccatgaccgaaagcagcaggtaccagcggtagcgcgggccgtagcgttcgcgcatcgttccaagggtgggcggggccggcggtgcggcttctggcgggggattgggggtcatgagacggcggcccggcctggatgcgggtccgtcgtcctacaagcatatcggtctttgcgcggcgaggcatgcgcccggccgctccacaatgcatgcgctgtcccgccttgcccctcagaacaacgacatgaaccctcgacccggcgctccagccaatgcctccgatccggtcgcggcgcccaacctcgcgtccgagcttgcggcgccgaccgtcagccgcgcctaccgctgccagtgcgggcgtccggtgttcctgcgcaacagccagtgcctggcctgccacacgccgctcgggtatgtgatcgaccggctcggcgtggtgccgttgtcgccggtccagggcgaggccgaagcccgaacggagggcgagggcgagggggagagcgagagcgaaggccaagccgtcgagcccgacaccttcaccgtgttcggcaatccggacggcaagagataccgccgctgcgccaacctcctgaccgccgccagctgcaactggatggtgccggccccgcgcgaaggcgacgaccctgccttcaacaccgacgggctcgcgcccggcttttgcctgtcctgcagcgtcacccgcaccattcccgatctgtcggtggaacggaacggcgaactctggcgcaagctcgagcacgcgaagcgcaggctcatctcgcagttgctggcgctcgggctgccagtggtcagccgccacgccgatccggtgcacggcctggcgttcgactttctcggcaacatgccgggcgccccgcatgtgatgacggggcatgaacacggcgtgatcaccctcaacgccgaagaggccgaagacgcggtgcgcgaacgcatccgggccgagatgcgcgagccctaccgcacgctgctcggccatttccgccatgagatcggacactactactgggacttgctggtgcagcccacgccttggctcgaggagtttcgcgcgctcttcggcgacgagcgggccgactacaccgcggcactgcagacgcactatgaacagggccccccaaccgactggttcaaccgcttcgtgagcagctacgcgagcatgcatccgtgggaagactgggccgaaacctgggcccattacctgcacatggccgacaccaccgacacggccatgagctttggcgtggacgccaccaacgtggagctcgcgagcgacctgttctccaccgacgacctatggcagcccgagcaccccggcgcgaccaagttcctggactttctcaacggctgggtgctgctcaccaacgtgctcaacgaactctcacgcagcatggggcagcccgactactaccccttcgtgctgccgcgcgcggccgtgggcaagctccagttcatccattgcgtggtcacgcagcagcgcgacacgacggtatcggccgcggccgctccggacgtgccgcttccgccgcagcccgagcctcccgcgccggccgccgggcctgccccggcgcaggggcagtcacaggcgcaaggccagcagcagaaccccgctcagtcctgagacgcggcggcaggcgttcccgcggcgcagcgggcgcagatgcaggccttgccgcgcgatgctgccggcagcgatgcgagcggcgcattgcggaagtcggtcgccatgcaccagcagggtggttgcgcctggccggtttcgcgcgcgacttccatggcgcagcggttttcttcgccgcacagcggacagcgcgtggcgtcgatggtgtccagggcggctaccgtgcgcatcaggcgagctcgaaaaccggcagcttcttcgccacggcgacgttgcgcaaggtggtgtacaccggcagtccgttgcggtaggcggggtaatcctcgccctcgatcagcggcagcaggtagagcctgcacttgtcggtgatgccccagccgtcgtccgagatgaagtcgcgcggcatcggcttctcgacgttggccaccgcatcgagcggcgcgctgccgatgcggtaggcatagggcgcgtcggaggtgcgctcgatggtcggcatcaccgcgttgcggccttcgagcgcgagctcgaccgcgcgctgccccaactcgtaggcctgcttcacgtcggtggccgaggcaatgtgccgtgccgcgcgctgcaggtagtcggccaccgcccaatggaacttgtggcccagcgcgtccttgaccatctgcgccaccacgggcgcggcgccgccgagctgcgcatggccgaaagcgtcgcgcgtgccttgctcggccaggaaggtgccgtccgggtagtggcagccctcggacaccaccaccgagcagtagccgtgctgcttcaccagctcatcgacccgcgcgagaaagcgggccttgtcgaattcgatctcggggaacagcaccaccaccggaatgccgtggtccgccgccagcccgcccgccgcggcaatccagcccgcatgccgccccatcacctcgagcacgaacaccttggtcgaggtggccgccatcgagcgcacgtcgaacgaggcttcgagcgtggacaccgccacgtacttggccaccgagccgaagccggggcagcagtcggtcagcggcaaatcgttgtcgatggtcttgggcacgtggatggcctgcagcggatagccgagcgactgcgacagctggctcaccttgaagcaggtgtcggccgaatcgccgccgccgttgtagaagaagtagccgatgccgtgcgccttgaacacctcgatgaggcgctcgtattcgcgccggttcttttcgagcgacttgagcttgtagcggcatgagccgaaagcgcccgcgggcgtggtgcgcagcgccgcaatggcttcggccggttcggcgccggtgtcgatcaggtcttcggtcagcgcgccgatgatgccgttgcgcccggcatagagctggccgatgcggtccgggtgttttcgtgccgtctcgatcacgccgcaggcggacgcgttgatgaccgaggtgacgccgcccgactgggcgtagaaggcgttgaggatgggcatgcggccattctcccgcagcccttcgccgggcgccagtgcccctcggtttcagcgcccgccgagccccatcgagcgcgtgatcacttccttcatgatctcgttggtgccaccatagatgcgctgcacccgcgcgtcggcatacgcgcgcgtgatcgggtattcccacatgaagccgtagccgccgtgcagctgcacgcattcgtccatcaccttgcactgcaggtcggtggtccagtacttggccatgctggcagtggcggtatcgagcttttcggccatcagcagctcgatgcacttgtcgacgaacacctgcgccacctgcacctcggtctgcagctcggccagcgtgtagcgcgtgttctggtagttgcccaccggctggccgaacaccttgcggtccttcacataggccacggtctggtcgatggcggcctgcgatgcggccaccgcgctgatcgcgatctgcagccgctcccacggcaactgctccatcaggcagacgaagccgcggttcagctgcgcggcatcgccgagcagcgcatcggccggcagatgcacgtcgttgaagaacagctcggaagtgtcctgcgccttcagccccagcttcttgagccgcttgcccttttcgaagcccggcgtgccgcgctcgaccaggaacaggctggtgcctttcgcgccggcggccgggtcggtcttggccaccacgatcacgaggtcggcatgccagccgttggtgatgaaggtcttgctgccgttgagcaggtagctgccgtcgggctgcttcaacgcgctggtcttgaccgcctgcaggtcgctgcccgcgccgggctcgctcattgcgatggcgccgaccatctcgccgctcgcgagcctgggcagatggcgctgcttctgttcctcggtgccgtagcgcaggatgtacggcgccacgatctcgctgtgcagcccgaagccgatgcccgtgaagccgcgcgcccagagttcctcgaactggatcaccgaatagagcaggtcggcgcccgcgccgccatattcttcgggcagcgccatgcagagaaagccgttctcgccggccttcgaccagacggcgcggtccacgtagccttgctcctcccacgcctcgtggaagggcgcgatttccttgtccatgaagcggcggaagctgtcgcgaaaggcttcgtggtcggcgtcgaaaagcgtgcgttggatcagggtcatggtgctcaggctttccgccgggccgccccaaggaaggcctgcgccccctcggggggcagcgaatacacgaagtgacgagcgtgggggcgcatgtcaccggctctcgaagaccggaggccgcttctgcaggaacgcgctcacgccttcgcggaagctggggcggtcgatcagctcgcgctggcgttcgctttcatagtgcagctgttccttcagcgtgtggcgttcggaggcctcgaaggcttcgcgcgcttccagcaccgcatgcgccggcaggcgtgcgagccgccctgcgatcgcgcgtgcttcgtcgagcagctgctcgtcgtcggcgcaggcccagatcaggccccactgcaccgcgcgtcccgcgctcaggcgctcgtcgagcagcgccatgcccatggcgcgcgccctgccggcccgccgcggaatggcccaggtgcagcccagatccggcacgatgccgagcttgggcaagaagggcaggtagaagtaggcgctgcgcgcggcaatcgtcacgtcggccgcaagcgccaggcccacccccgcgccggctgcggcgccgttgaccgcggccaccacgggcacgggcagcgtgcgcagggtttcgatcagcgggttgctgagcgactgcatccactccgccgtctgcgtgccgagcgacttgccttcgtctgcgggcgccatcgcactcagatcggcgcccacgcaaaaggccttgccggcgccggtcaggatcacgacgcgcaccgcgcggtcatcgcggatgcgctccagcgtgtcgcgcagttcgatctgcagttcgcgcgcgatcgggttcagcttggccggcaggttcagcgtgagcgtggcgatgccgtcggccagctcgtagagcacataaggctgttgtgtgttcatcagagcctttccacgatggtgacgttggccatgccgccgccttcgcacatcgtctgcaggccgtagcgcttgccgcgccggcccagtgcgtggatcagcgtggtcatgagcttggtgcccgaggcgcccagcggatggccgagcgcaatggcgccgccgttcacgttgagccgcgccggatcggcctccagcgcctccagccacgcgatcggcacgggcgcgaaagcctcgttcacttcatagaggtcgatgtcctggatgcgcatgccggcctttttcagcgcatgcagggtggcgggcagcggtgcttccagcatgatcaccgggtcgtgccccatcacgctcatgtggtggatgcgcgcgagcggcttcacgcccagggccttcaggccacgttcgttcaccaccagcacgccgctcgcaccgtcgcagatctggctcgcggtggcggccgtgcagcgcccgccctcggcaatcagcttgacgcccgcgatgccttcgagcgtggcgtcgaagcggatgccttcgtccaccgcgtgccgttcgccggtgcccgtgccatcggccgagagaatctcgatcggcacgatctcgtcgtcgaaggcgccctcgcggctcgcgacgatcgcgcggcggtggctttcgagcgcatagcgatcgagcgtttctttctcgatgccgtagttcctggcgatcatctcggcgcccgcgaactggctgaactccacgcccgggtagcgcctcttcatggccgggctcatgtaggtgcccaggcccgccttggctggcagcgcgttgggggtgaacatgggcacgcgcgtcatgctttcgacgccgcccgcaatcaccgcgtccatgctgcccgacatcacggcctgcgccgcgaagtgcagcgcctgctgcgacgagccgcattgccggtcgaccgaggtgcccggcaccgattcgggcagcttcgatgccagcaccgcgttgcgcgcgacgttggtcgcctgctcgcccacctggctcacgcagccgaggatcacgtcttccaccgccgccgggtcgatgccgctcttcgccatcaatgcgtcgatcacctgcgccgccaggtcggccggatgccagcccgcgagcttgccgccgcgccggccgccggccgtgcgcgcggcggccacgatgtatgcctctgccatggtcatgtccttctcgataagaaaacagccggatccgcgctcccaacgcaaaaaagccgcccatcggggcggcggcgttcggtgcgtggaaagtccatggcatcgaggttcgatgccgggggtcttcaggtcaagccggggacaacccgagaggccgcagtcgccaaggcgaccggcggcctgccggcgccggcagcggcatggccgcgggctgcgcgtccgagacggtgatgcacgaagcctccagcgcggagaccagcacgcgccggtgttcggtgccctcgaagcgttcgcccggcgccagcacgatgtcgcgcgggtcgcggtcgagcgtgacccagaccgagccgctgcggcattcgatgcccacgccggcgccgtcgggcacggcaaagatggaacgggtcggcaggctgacgtggaaacgggaagaagggttcgggtgggtgctcatggcaagctccattgcattcgtgatacgaatgaatatagtgagttgacctccctcttacacgcggtcattcggaactcgttgcatgcatccagagaatgcgaaaacgccgaccggcgaacttccgccgctcgatctgctgcgcagtttcgaggccgcggcgcgccggctgagcttcacgctggcggccggcgagctgcacctcacccagtcggccgtgagccggcagatccagcagctcgaagccagcctgggcgtgctgctgttcgagcggcgccaccgcgcgctggcgctcaccgaggccggcggcgtcatgcagcgggccgtgaccgacagtcttgagcgcctgcgcgatgccacggcgcgggtgcgtgccagttccgcgccgcggcaggtggcgatcaccagcacgccgggcttcgcctcgctctggctcattccgaggctggcacgcttcaccgtcagccatccgcaggtcgacgtgcgggtgtcggccacgctggacgtgctcgacctggagagcagccgcatcgacctggcggtgcgcttcgtgccgatcggccgcggcatcggtccggcgctgttcgaggaatcggtgatcccgctgtgttcaccgcaactcgccgcctcgctgcgcgagccatcggatttttcgaagctcaccttgctgaccgtggaataccccgaccacggcgaggcccccaccgttgactgggagccctggctccgggtgatggggttggacgacttgcgcatgaagagcacgctgcgcttcacccagtacgccgatgcggtggccgccgcggtggcgggccagggcgtggtgatcggccggctgccgctgctgcgcgaactggtgcagggcgggcggctcgtggcgccgcttggcgaaggcgtggcctcgcatcgcggctacttcatcgaaacctcgcggcgcgcagcgggcaaccgcgatgcgcaggagttcgcgcagtggctgcgcgacgaagccgaggcggcgcagcgaacctgaccaggcccgccgcgcaaagcctcctgcgggagaacgttcagcccggcagcagcaccttgtcgaccacgtggatcacgccgttcgactggtagacattggcgatggtcaccgtcgccgtgccgcccttggaatcgctcatcatcacgttgctgccgctcatcgtcgcggtcagcatgccgccgctcgcggtcttcagcgtggccttgccaccgcctgccttgatggcgctcatgagggccgcaccgtccatcctgccgggcaccacgtggtaggtcagcaccttggtgagcgtgggcttgttctcgggcttgagcagggtgtcgaccgtgccggccggcagcgcggaaaaggccgcattcgtcggcgcaaacacggtgaagggaccggggctcttcagcgtgcccaccaggtccgcggccttcaccgcggcgaccagcgtggtgtggtccttcgagttcacggcgttgtcgacgatgtcttttgtcggaagcatcgcggcgccgcccaccatggggtggggcgccgtggcgttgctgccgctcatgcccatgccgcccgcgcaagcgccgagcaagaccgaaacgcccactgcaatcacgagttttttcattgaaaggctcctggtaagaatgttctcgaaagacctctgcggcgaccgccgacagttcggaagcgcgatgcgctcaacacccatacggagcgaatgcgcgattggattcgcgaacgcatccgcgtcggctttgcgccacagccattcacgcgccgcttgcgcaccgcgcgcgtgctcgccagaatccgcccttcgtttttcagcaacagttttccatccgcgcctggcgacgaccaacctcctgggcgacaactgcattcaatgaaccgttttctgaacacctgacccgcacaccgaccgccccggccggatgtgcatccacgcatccgccgaggcccatcgacaaaggccccgcgcagccattcgccggggcctttttgtttttggagtgtgcgcacatgagtgctcaacgaaaggcccgcgacgatcagaagcgcctgggccggttttacttttcggtgccgtccgcggcgccgcgcaatcctgtggtggccgcgatggcgcaccgcgaatcgagccagggcgcagggcgccacctgcgcacgcaccgcgcggagcggcgtgcgcagaaggtcgcattgcagaaggcagcgcgaagcctcgggcgggagggctgaccatgcgtgaagacatggacaaagtcatcgtcgagcggccgcgccgaggcggcggtgtgcagggcgacgggcgcaagtggcgcaacagcagggaacgcggttcgcacctgggcatgacgcagggctatggccatccgaagtggctcaacgagaacctcgcacccctgaagcgctggctgcacaagcaggtgcaccggccgtgggacaaggtgtatgcggagctctgcagcggcatcgaccgccgcagcacggtgcaggcgcacatcttcgagcacatcgacgatttcgtcgcgcgcgacgctgcgatgcgaggctgcgaggtgtgggtgagcgagtcccggtgggggcgcggtggccgcgtgccgctcggcgaagctgcacgcgtcgagttgttcgtgcacccgctcacgggcatcctcttgcccaaccggcggctgcacgaggcgcgtgcggcgcgaaaggcacgctacggcagctgggccgagcggcggggtgacacgccctacgcggtctatcacgtgatcgacgaggccacgcagtggcaccgcctggacggctgctggttcgaggtcacgctcgccgcgtttcccgaaaggtcgggcggcgcgaagccggaagaaaaatgctacgacgtgctgcgccgctgcctcgtcacgcgcagtggcgcaacccagcgtcccgcgccgggcctgcccacccacgtcggcatgtacgggcgcggcgacgtgtacgcggcggccaagcggcagctcggccgccgcgaggtgcgggcccgtctcggcgaccgggcgctcgaataaaaaaaagccgggctgcaggagcccggctttcattcagtcatcggcgcggtggcttcaggcttcgcccttcaccttcaagcgccatgcatgcagcagcggctcggtgtagccgctcggctgctcgatgcccttgaacaccaggtcttgcgccgccttgtacgcggccgaggtgtcgaagcggccggccatcggctggtacaccgggtcgcccgcgttctgctcgtcgaccaccttggccatgcgctggaaggtctcgtcgacctgcgccttggtcaccacgccgtgcagcagccagttggcgatgtgctggctcgagatgcgcagcgtggcgcggtcttccatcaggcccacgttgtggatgtcgggcaccttggagcagcccacgccctggtcgatccagcgcaccacgtagccgaggatgccctgcacgttgttgtcgatctcctgctgcttttcggcgtcggtccagttggcttgcggtgcgatgggcacctgcagcagcgcgttcaggatgttgtcgcgttcggcatcggcgtcgatcttctcgagctcttgctgcacggccgtgacgctgacctggtggtagtgcagcgcatgcagcgtggcggcggtgggcgagggcacccaggcggtgttggcgccggccttggggtggccgatcttctgctcgagcatggccgccatcaggtcgggcatggcccacatgcccttgccgatctgggccttgccgcgcaggccgcacgagaggccgaccagcacgttgttcttttcataggcgccgatccacgcgctcgacttcatgtcgcccttgcggatcatcgggccgccgtgcatggcggtgtgcatctcgtcgccggtgcggtcgaggaagccggtgttgatgaaggccacgcgcgcggcggcctcggcaatgcaggccttgaggttgacgctggtgcggcgctcctcgtccatgatgccgagcttcacggtgttggcggcgaggccgagcaactgctcgacgcggccgaacagctcgctcgcaaaggccacttcggccgggccgtgcatcttgggcttgacgatgtagatgctgccggtgcgcgagttgcccttgcgcttcaggtcgatcatcgcgatggtggtcgtcaccacggcatcgaggatgccttcggggatttccttgccgtccgcatacagcacggcagggttggtcatcaggtggcccacgttgcgcaggaacatgagcgagcggccgtgcagcttcacgggctggccgtcggcgccggtgtattcgcggtcggggttgaggccgcgcgtgaaggtcttgccgcccttggccacgtcttcggtgagcgtgccctgcacgatgccgagccagttcgcatatgcgatgaccttgtcggccgcatcgaccacggccaccgagtcttcgaggtcgaggatggtcgagagcgcggcttcgagcacgaggtcgctcacccccgccgcgtcgcccttgccgatgggcgtggtgcggtcgatgcggatgtcgaggtggatgccgttgtgcttcagcagcaccgacgacggcgatgccgcgtcgccctggtagccgacgaaggcggagggatcgcgcagcgcggtgccgctgctttgcagcgcgatgtgcagctggccgtccttcacgctgtagccggtcgccatcttgtgcgaaccgttttcgagcggcgcggcctggtcgagcacgttgcgcgcaaactcgatcaccttggcgccgcgcacggggttgtagcccttgcccttttcggcgccatcggtttcgggaatggcgtcggtgccatacagcgcgtcgtacagcgagccccagcgcgcgttggcggcattgagcgcgtagcgggcattgaggatgggcaccaccagctgcgggccggcctgcaaggcgagttcggaatcgacgttggccgtggtggccttcgcgcccttgggctgaggcagcaggtagccgatcttctcgaggaaggcgcggtacgccggcatgtcggtgatcgggccggggttcttcttgtgccaggcgtcgagctcggtctgcaggcggtcgcgctcggccagcagcgcgacgttcttcggcgcgaggtcgtgcacgatggcgtcgaagcccttccagaagacgtcgctcgccacgccgctggcaggcaggaccttgtcttcgatgaagcggtggagctcggtcgcaacctggagtccgtgggcggtggtgcgggcggtcatgttttttctcctggaaagcggtgcaattcggatgctggatcagttgagggacggtgtctgtcagaagaagaacacgagcgcattcgtactggctgctgtcgatgcgatcggcccggagtcttcgatgcagtgactttattcgatactttgtcggtgagtaagggccgaaagtgggatttatcggtgacaaaaatgaaggtaatcgcaggaggctgcctgcattccggtgtcagatcaggctgctgagttcgcgtgccgcggcgcgcaccggctcgatgtggcgctcgtcgtagcggtgcgtgggcatcgtcagcgtgagcgccgcggccaggcggccgtcggcatggaacaccggcgccgaaatgcctgccagctcggcggtgcggtcgcccaccaatgcgcagtagccctgcgcgcgaatggtgtcgtacagcttgcgttccctgccgccgctcggccgctcggcctccggcccgaaggcgatcagcacccgcgccccggcaccccggtcgttggacagcacgtcgcccgcgcgcacgtggtcgcgcaccacgtgcgacgaatcgacgcggaactggcacagccgaacccagctttcgccctggtcctgccgcacgtggtaggccgcgctctcgccggtagcggcggccagcgcgcgcagcaccggcagcacgacgcggtcgagcgaaagcgacgccgcatacaggccatgcaggcgcgcgacctctgcgcccagcgcatagcggccatcttcctggcggcggatcagccgcgcatgttccagcgacgccaggaggcgcagcaccgtgctcttgtaaagctgcgtgcgctgcgcaaactgcgccagcgacagcgcctcgtcgccgggctggaaggccgagaggaggctcagcgcgcggtcgaccgcggcggcacccccgggggcggcgttgaggtcggacacggattcggcttgggctttgcggggcatgagaagggaagggatcggcttgacagccttgtggatcgacggtctaattctgtttaacggaatatagttctgtaagatagaacagtcaagcgatcctgcaaggagacaaatccgatgacaccccccgacgtcctcatcagcgaggtcggcccgcgcgacggcttgcagtcggtcaaggccaccatgcccacggccgacaagctgcgctggatcgatgcgctctacgccgctggtgtgcgcgagatcgaggtcgcgtccttcgtgccggcgaagctgctgccgcagatggccgacgccgccgaggtggtgcgccacgccgtcacgctgcccggcctcgtggtgatggcgttggtgcccaaccgcaagggcgcagaggcggcgctcgaagccggcgtgcacaagctcacgatgccggtgtcggccagcgtggcgcattcgctggccaacgtgcgcaagacgccgaccgaaatggtcgatgaagtgcgtgccatctcggatctgcgccgcgccatcgcgccgcgtgtgaagctcgaagccggcatctccaccgccttcggctgcacgctgcaggggctggtgcccgaagacgacgtgatccgcctggccgcgcaatgcatcgaggctggtgccgacgagtcgggcctgtccgacaccgtgggctatgccaaccccgcgcaggtgcgccggctcttcaagcggctgcgcgccgagctcggccgccacgccggcgccgcccacatgcacaacacgcgcggcctcggcattgccaactgccttgccgcctgggacgaaggcgtgcgcaccttcgacgcctcgctcggcggcctcggcggctgcccctatgcgccgggcgcctcgggcaatgccgtgaccgaagacctcgtgttcatgttcgaggccatgggcgtgcgcaccggcatcgacatccagaaactcatcgcggcgcgtgcgccgctcatggccggcctgcccggcgaaccggtctatggcatgacgcccgaagccggcctgcccaagggctttgtccaacaggaaacctctgcacatggttgaatcccaagctttgccaaatcctctgccctatgccggcattcgcgtcgtcgagttcacccacatggtcatgggcccgacctgcggcctgctgctggccgacttgggtgccgaagtcatcaaggtcgagcccatcgagggcgacagcacgcgccgcctgctcggctcgggcgcaggcttcttcccgaccttcaaccgcaacaagaaaagcatcgcgctcgacctcaaatcgcccgaaggcgtggaggccgcgctgcgcctcgtcgccaccgccgacatcgtcagcgagaacttcaagcccggcaccatgaagaagctggggctcgactacgagacgctcgccaagctccacccgcgcctcatctatgtgagccacaagggctttttgccgggcccgtacgaccatcgcacggcccttgacgaggtggtgcagatgatgggtggcctggcctacatgaccggccgcgccggcgacccgctgcgcgcgggcaccagcgtcaacgacatcatgggcggcatgttcggcgccatcggtgcgatggccgcgctgcgccagcgcgagctcaccggcaagggctgcgaggtgcagtccgcgctgttcgagaacaacgtgttcctggtggcgcagcacatgatgcagttcgccgcgaccggcaaggcggccgacccgatgcccagccgcatctcggcctgggcggtgtacgacgtgttcaccgtgaaggacggcgagcagatcttcctcgccgtggtgagcgacaagcagtgggccatcttctgcaaggccttcggcctggaagagatgctggccgatccgcgcctgcagagtaacaacgaccgcgtgctcgcgcgcgactggatgatgccgatcctgcgctcgcacctcgcaggctacagcgcggccgagctcagcgcggtgttcgagaagaacgagctgcccttcgcgcccatcaccaagccgcaggacctgttcgacgacccgcacctcaacgctaccggcggactcgcgcccgtgcgcatgaacgacggcgacatggccaaggtgccgctgatgccgttcacgatcggtggcgagcgcccgggcatccgcatgcagccgccgcacatcggcgagcacaccggcgagctgctgcgcgaggtgggctacagcgacgaggagatttccgccttcgaagcgcgcagggccggcgtcgcccgctgaacccgcgcgaaaccccgggcgatatagttcgggcgccatggaccgcctgaagcaactcgaatccttcgtctcggtggcaacccgcggcggtctcacggccgcggccaaggccgagggcgtggcgcccgccatcatggggcggcggctcgacgcgctcgaagcgcggctgggcgtgaagctgctggtgcgcaccacacggcgcatcaccctcacgcacgaaggcagcgcctttctcgaggactgccagcgcctgttgaccgaattcgccaacgccgaggccagcgtgagcgccggcggcgtcaaggccagcggccacctgcgcgtgacggcgccggccggcttcggccgccgccacgtggcgccgctggtgccgcgctttcatgcgctgcaccccgaggtcacgatttcgctcaacctgagcgaccgcgtggtcgacgtgcgcggcgaaagcttcgactgcgcggtgcgcgtgggcgacatgcccgattcgtctttggtgagcgtgcggcttgccgacaaccgccgccgctgcgtcgccacgccggagttcgtgcgccgccacggcatgccgcggcatccgagcgagctctcgcgctttgcctgcctcacgctctcgagcgatgcctcgcaaacgcgcggctgggcattccgtgtccccaccgaagacggcggcgaggaattgatctatctgcgccccgacggcccgctggactgttccgacggccaggtgctgcacgactggtgcctggccgggcacggcattgcgtggcgcagcacctgggaggtggaggccgagatcgatgccggcctgctggtgccgctgctcgatgaatttgccgcgccgccaaacggcatctacgcagtcttcaccggcaccaagcacctgccgcttcgggtgcgactgtggcttgatttcctcaaggcgcactacggacgtccggaattctggggcggacgggggtaaagcgcgcgaggggcggcacaatgtgcaagcatttgcaaccccactgaagagaacggaagagaagaaagccgacgatgaccctcgaagccatccttgcctacctgcacttgctggccattctcacaatggtcgtgttcatctccagcgaagcggcgctgtgccgcgtgcagtggctcaatgccgccgtggtggagcggctcgccaggatcgacatggtctacggcatggccgcagtgaccgtgctggccaccggcatcgcgcgcaccgtgtggggtgtgaagggcacggcctggtactggaccaatccgctgctgcacgtgaagctggggctgttcatcgtcatcggcgtgctctcgatctttccgacactgacctacctgcgctggcgcaaggcgctgcgcgccaacggcacgctgccggccgaggacgacatcaagaagacgcgcaagctggtcatggtgcaggcgcacctgatcgcgctgatcccgctggtggccgtgttcctcgcgcgcggtttcggcaagtaggccccccatgggacgcgccggcatccagcttctgtttgcaggcaccatcttcagcagcgcgttcctgctgttcctggtccagccgctgatcgccaagcagatcctgccctggttcggcggctcggccgccgtgtggtcgatctgcatggtgttcttccaggtcgtgctgctcgcgggctatgcgtactccgactggatcacgcgccatcttcgcgtgcgggcgcaggccgcgctgcacgtgggactgctgctcgcgagcctggcgttccttccgctcgtggtgggcgcggcctggaagcccaccggcaccgaagacccgacgtggctgatcctgggcctgctgttcgcgaccatcggcctgccgtacttcctgctttcgaccaccgggccgctggtgcagtcgtgggtggcgcgcacgccctggggcgcgcaggtgtaccggtacttctcgctgtcgaacctcgcatcgctgctgtcgctgctgtgctatccggtgctgatcgagccccgcagttcgctgctgcagcaggcgctgggatggtcgtggggctacggcgtgttcgtggtgctttgcgccggcacgaccctgctcgtggcgcgccgctggccggaggccgcgccatccccggcagcggcgggccaggccgcggccgacggcagcgaccggccgccgcgctggaccgacggcgtgctctggctcgtgttgccggcactggcctcgtggctgttgctggccgtgaccaaccacatcacgcagaacgtcgccgcggttccgtttctctggatattgccgctctctctgtatctgttcactttcgtgctgtgcttcgagagcgaccgctggtaccggcgcggcgtcttcctgccgctggcggcgggcgtgctgctgctttgcgcctttggcctgcagcaccacatcggctccgatgtgcgcacggggctgccgatctatgtcggcggcttgttcgtgctgtgcatgttcctgcacggagaaacggcaaggctgcggccggcgccgcgctacctcacccgcttctacctgatgctctcgctgggcggcgccatgggcggcgcgacggtggggctggtggcgccgcacgtgctgccggcgtactacgagctgggcatcggcctgatgctgacggcgctggcggccgccgccgtgctgcgccggcgcacctggctgcgggtgttcagcgtggcgctggccgcctgctgcgccttcttcctgatcgtgcagatcggcagcgacagatcggacgcgcgccacctgctgcgcaatttctatggcgcgctgatcaccttcgacgtgcgccgcaccgacccggcggacaacgtgcgcctgctgtcccatggctccatcaagcatggcgaacagttcctcgcgccgtcgcgccgaagcgagcccaccacctactatggcgccacctcgggcgtcggccgcgccatggccgccgcgccggccggaccgcgccgcgtcgggctgatcggcctgggcgccggcacgctcgcaagctacggccgcagcggcgacgtctatcggatctacgagatcaatccgcaggtgttcgaactggcggacagcgaattcacctttctgcgcgacagccccgcgcgcatcgagcgcgtgctcggcgatgcgcggctggcgctggagcgcgagccgccgcagggcttcgacctgctcgcggtcgacgccttctcgggcgacgcggtgccggttcacctgctcacggctgaggccatggacgtctacctgcggcacatgaagccggacggcatcgtggcctttcacgtgaccaaccgattcctcgggctggcgccggtggtggcgcggatcgcgcaggtcaagggcttgcacgccgtgctggtcagcgacgacgcggaagcctcgaagtggctcaatccgaccgactgggtgctggtggcgcgcgatcccgccgtgctggcgcgcgaacccctgcgcgcggtggcctcgcccatcgcgatgcccgaagacgcccgcccctggaccgacgatttcaacaatctcctgggcgtgctcaagtagcgcccatgaaaaagccccgccggcgcgaagcgcgtgcggggccctttgtgggagcgatcaggccctggcgctcaggcgctcaggcattccttcatgaaggccttgcgggcatcgcccttcagggtcttggccttctggtcggcattgcaggtcttcatcttttcctgctgggtcggcttggcagtcatgaccggcttggcgctcaggcagctcttcatgaaggccttgcgctcgtcgcccttcttgtcgccggcttcctggttgcaggtcgtcatcttgctttgctgggcggtcggggccttggccgccggcgtggcgggggtggctggcgttgctggagtggcgggtgctgccggcgccttggcggccggcatggccggagtggctggcgttgccggggtggcgggcttggcagccggggcgaccgcaggcgcgggggccttgtcttgtgcctgtgcggcgccgaacgaaaggcaggcgcccagggcgaccagggaaaggagcttcttcatggtgatatgtccttgcagggtgtttgtgacaggtgccccgccccggggctgctcacactaacggtccacatcggccgccggatgaccatcgccgccggcgcccgggtttgcccccggtaaaatccgcagatgctattggtcaaacaggagctgctcgcggcgctcgcgaacacgctcgaatccctctcgcccggcgccggctccaaagccgcgttcgagtcgcccaaggtggccgcccatggcgacttcgccagcacggccgccatgcaactcgccaagccgctcgggcgcaagccccgtgaactcgccgaagagctcagcgccgcgctgctcgccacccccgtgttcggccagtgggtcgaagccatcgagatcgccggccccggctttctgaacatccgcctcaagacctctgccaagcagcagatcgtgcgcgaggtgctgaacgcggccgacaccttcggccagcagcccgccaccggcgaaaaggtgctggtcgagttcgtctccgccaacccgaccggcccgctgcacgtcggccacggccgccaggccgcgttgggcgacgccatctgcaacctgcgcgcttcccagggcgacaccgtctggcgcgagttctattacaacgacgccggcgtgcagatccagacgctggccaacagcacccagctgcgcgcccgcggcttcaagcccggcgaccccgaatggccgagcggcgaaaaggccccggcctacaacggcgactacatcgccgacatcgccgaagacttcaaggccaggaagaccgtcaagtcggacgaccgcgaatacaccgccagcggcgacatcgacgacctcgactcgatccgcgaatttgccgtggcctacctgcgccgggagcaagacctcgacctgcaggccttccgcgtgcgcttcgacaactactacctcgagtccagcctgtacaccagcggccgcgtcgaggccgcggtgcaaaagctcgtggccgccggcaagacctacgagcaggacggcgcgctgtggctcaagtcgaccgactacggcgacgacaaggaccgcgtgatgaagaagcaggacggtacgtatacgtacttcgtccctgacgtcgcttatcacatcgccaagtgggagcgcggcttccacaaggtggtcaacatccagggcaccgaccaccacggcaccatcgcgcgcgtgcgcgccgggctccaggccgcgggcgtcggcattcccgcgggctatcccgactacgtgctgcacaccatggtgcgcgtgatgaagggcggcgaagaggtcaagatcagcaagcgcgcgggcagctacgtcaccttgcgcgacctgatcgagtggaccagcaccgatgccgtgcgcttcttcctcctgagccgcaagcccgacaccgaatacaccttcgacgtcgacctggccgtgaccaagaacaacgataacccggtgtactacgtgcagtacgcccatgcgcgcatctgctcggtgctggccggctggggcggcgaccccgccacgctcaagaacgtcgacctgtcgccgctcgagagcccggccgcacaggcgctcatgctgctgctcgccaagtaccccgccatgctcacggccgccgcgaaggatttcgcgccgcacgacgtcactttctacctgcgcgaactggcggcctgctaccacagctactacgacgccgagcgcatcctggtcgatgaagaaccggtcaagctggcgcggctcgcgctcgtcgccgccaccgcgcaggtgctgcacaatggcctcgcgattctcggcgtcagtgcgccgagcaagatgtgaaaacaccatgaagaagacaaccagacaacgcggcaacatcgtcatcgggctcatcatcggcctggtgctggggttgggtgtcgcgctgggcattgcggtctacgtgaccaaggtgccgatcccgttcgtgaccaagacccagcgcggcggcgccgagcaggacgaagccgaggcccgcaagaaccgcgattgggatcccaacgcgcccctggcaggcaaggctggcgcacccaagccggtcgcccccgctccggccgcgccggccggcggcgacaccacggccgtggcaccggccaccgcgccgccgcctgctcccccggtgccggtggtcgtggcgccgcccaagcccccgcgtccggcgccggtgccggccgaagccaattcgctgccgccttcgaacgatccgctgggcgaccttgcccgtgcgcgcgccggtggcaacaatggcagcaccaccactgcttccgccgcgccaagcagcaacaacggcgccgcagcgggggccgacccgttcatgtatttcgtgcaggccggcgccttccgcaccaccgaggacgccgaggcccagcgcgccaagctgtcgctgatgggtgtcgaggcccgggtcaccgagcgcgagcaggccggtcgcacggtctaccgggtgcgcgcgggtccgttcagcaaaaaggacgatgccgaccgcctgaaagagcggctcgacggcggcggcctcgaatccgcgctggtgcgcgtccagcgctgacgcccccgcgaaccgccggccgcggcctccgcgagcggcggtcacgaatattctttaagctttgccgcgcggcacgggccgccgccaacccggattgtcctgggcaagccgcatgcgggaactccgcgcggcgcgccggctcagtctgccgtacccaacaggagaactctttcaatgaaacgtcgtgacttttcgctggccgccacctcgctcgggctgctttccctggccggcaacaccgcgcacgcccaggcgcgcgtgcccaaggccggaaccgagtacctggtgctcgacaagcgcgtggcggtcgatgcgcccgcgggcaagatcgaagtgatcgagttcttctcgtacaactgcccgcactgcaacgatttcgagccgcagctcgaagcctggctcaagacggcgccgaaggaagtggcattccgccgcgtgcccgtgcctttcgtgggcaacgacgtcgaagccaagcagcgcctgtactacgcgctcgaaacgctgggcaaggtcgacgaattccagccgaaggtgttcgacgcgatccacaagcagcgtcagaacgtgaacggcgacgccaacatcattgcctgggccaccgccaacggcctggacggcgccaagttcaaggaggtgtttacttcgttcggcgtggccagcaaggcgaagcgcgcctcgcagatgaccgacgcctacagggtggccggcgttccggccctggcaattgccggccgctggtatgtggacggcgaaacggccggcaacatgaccaaggcgctccaggtcgccaacttcctgatcggcgaagccaagaagggctgacccccttttgcagggggtatcacctgcggccggcagagccggtttcgcggtgtttccggatggatgtcaagcccgctttggcgggctttttcatccgtgcgtgcagggctggcgccatctgccgcatacaatgcagagcaagtttcgtgcctctatgacattgcactcctactccaacaccactcctcttgttcgccgcttcggccgcctggctcgcctgagtgttggcgcgctgttgctggccggtctcgcctcgggcgccctggccgagacggccgaccgcaccaagccgatgaacatcgagtccgacgccatgcgttatgacgacctcaagcagacgagcgtgttcacggggaacgtgctggtcaccaagggcacgatcatcatccgcggcgcgcgcatcgacgttcggcaggacgccgagggctaccagtacggggtggtcacggcggctcccggcaagcgggcctactacaagcagaagcgcaatgcgcccgacgagtggatcgagggcgaatcggaggtcatcgagtacgacagccgcgccgacaacgtcaagttcatccgcaatgccgtgatgcgccgcctgctgggcgccacgccaaacgacgaaagcagcggcgcgctcatcgtctacgaccagagcaacgacacctacacggtcaacggttccaccgtgccgcccaacaccggggtgaatgcccccgcgggcggtgggcgggtgaagaccatcctgacgcccaagagcgccacggcgcccgcgccaggcgcctcggcgccggccggcggacgggccgcgccagcagcgccccagccggcacccggtgccggcctgcggccgagcaccacgctcagcggcagcgaaggggaagggcgcaagtgatagaaaccgctggaagccacaccgccgatggcacgccgggcagccgcctggtggtgcgcggcctgcaaaaaagctacggtagccgcaaggtcgtcaaggatgtctcgctcgacgttcaaaagggcgaagtcgtggggctcctgggccccaacggcgccggcaagaccacttcgttctacatgatcgtgggcctggtgcgggccgacgccggcgagatcaccatcgacggcgaacccattgcgcacatgccgatccaccggcgcgcccgcatgggcctgagctacctgccgcaggaagcctcgatcttccgcaagctcacggtcgaggaaaacgtgcgtgccgtgctcgagctccagcgcgagcccgatggcaacggcaagcccgcgcccctgtcgaagcagcgcaccgaagagcggctctcggggctgctggccgacctgcgcgtggaccatctgcgcgattcccccgcgctcgcgctctccggcggcgagcggcgccgggtcgaaattgcccgcgcgctggccacccagccgcgcttcatcctgctggacgagccctttgccggcatcgaccccatcgcggtgatcgagatccagcggatcatcagcttcctgaaggagcgcggcatcggcgtgctcatcaccgaccacaacgtgcgtgaaacgctgggcatctgcgatcacgcgttcatcatcagcgacgggcatgtgctggcacaaggcacaccctcggagatcgtcgacaacgccgaagtacgcagggtgtaccttggcgagcacttccggatgtaagggaggagccggtctccatgaagcaagggctgtcccttcgcgtttcgcagcatctggcgctcacaccgcagctgcagcagtcgatccggctgctgcagctctccacgctcgaactgagccaggaggtcgagcagatgctcgacgagaacccgttcctcgaacgcaccgcggaagaagcggcgcgcgaggaattcggcctcgatgccatcgataccccgatgccgcgcgatgaatcatcgggcgaggccggcgagagcgacttcgcctcggctccggcgagcagcgcggccaccacctccagcgaaaccacggccgcggccgaaaccgacgttcccgccgccgacgccaccgagcgcgagcccgactgggaaggcgacggcaccgtcgacatggcgccggacgacagcgagtggggcagcgatgctcccgcgcgccagaacaacctgggcgacgacgagcgcgccgacgccaccgaactcgcgcgcagccaggagtcgctgcagtccttcctgcaccggcaggcgctgagcctgcggctcaacgagaacgactgcgccgcgctgcgcttcctgatcgaatcgctcaacgacgacggctacctcgaagattcgctgccggcgctggcctcgggcctcgcgggcgacgacaacgaccagttcgacgagctggtgcatcacttccaggtggcgctcggcctgctgcaaagcctggagccggccggcgtcggcgcgcgcgacctgggcgaatgcctcggcatccagctgcgcgcgctcgccagcgaagacgaaaccgaagaacacgccctggtccgcaagaccgccatcgccatctgcaagcagccgatggagctgctcgcgcggcgcgacttcaagcgcctggccacgctcacccgcaccaacgaagagctggttcgctcggcgctgcagatcatttcgcgcctggagcccaagccgggccgccgttttgtcgatgtcgagcgcaacatcgtgatccccgacgtgatcgtcaccaagatcggccgcggcaccaacgtcaagttccgcgtcatgctcaaccccgaggtgatgccgcgcctgcgcgtgcacgacatctatgccggggcgctcaagtcgcacaagggcgagggcagccaggcgctgtcgcagcggctgcaggaggcacgctggttcatcaagaacatccagcagcgcttcgacaccatcctgcgcgtctccaacgccatcgtcgagcggcaaaagagctacttcgtgcacggtgaactcgcgatgcggccgctggtgctgcgcgagatcgccgacgagctcggcctgcacgaatcgaccatctcgcgcgtgaccaccgccaagtacatggccacgcccttcggcaccgtcgagctcaagtacttcttcggctccgcgcttggcaccgagaccggcggcaatgcgtcgagcaccgcggtgcgcgcgctgatcaagcagttcgtgagttccgagagcatcaagaaaccgctgtccgacagccagatttccgagatgctcaaggagcagggcatcgaatgcgcgcggcgcaccgtggccaagtaccgcgaggcgctgcgcatcgcgcccgccaacctccgcaaggcgctgtagaaagccgtcgatggcccctcgccgcctgctgtcgcgctgtgggcactgggtcttggccgtggcggtggcgctgctcgttgccggctgcgccaccctgcccgacgaagcgccgcgcccacccacccgggccatggcggtgtcggccgacaccgcgctcggcaagatcgcgctggccgcgcagcccgacctcgatctcagcggttttcgcctgatgccgggcggcgatttcgccttcgacacgcgcatccaactcgcgcggcgcgcccagcgcacgctcgacgtgcagtactaccaaatcgagaacgacgagaccggccgctacctgctgcgcaccctgcgcgatgcggcggagcggggcgtgcgcgtgcggctcttgatggacgacctctacacttcgggcgaggacgaactgctgctcggcctggccgccacgccgaacgtcgaactgcgcctcttcaacccgtttccagccgggcgcggcagtctgctcaagcgcttcgcggcctcgctcttcgacttcagccgcgtcaaccggcgcatgcacaacaagctcttcatcgccgacggcgcgatggcggtggcgggcggccgcaacatcggcaaccagtacttcaggcgcacggcgggcgagaattttctcgatctcgacaccttcgtgaccggcgcgctgatgccgcgtctcggcaccctgttcgaccagtactggaacagcgtgtacgtgcggccgatccagtcggtggtggccacgggcctttcgcgcgaagaactgcaaaagcgcttcgaagccgccaccggccccgacaccacgccgccgccgccgcggcccgcccccaacgacctgctcggctacagcccgatggccgaggaccttgccaccggcaagctcggcctgatctgggcccttgccgaggcctacgccgattcgcccgaccgcgtgatcggcaagacggcgtcctatggcggcgtgccgctgctcgacgtcgacagcgtgcgctacaacgtggtggagcagatgcgccgcgcgcgctccgaggtgaccatcgtctcgccctacctgattccgggcgaggccggcctggaggtgatgcgcgagatccgccggcgcaacgtgaagatcagcgtggtcaccaattcgctcgccgccaccgacgagccgctggttcacacggcctaccgccgctaccggcccgacatgctgaagctgggggccgacctgtacgagctcagcaccacgcgcacccggcgcagcgtgcggctcggcctcttcggcacctcggtcggccggctgcacgccaagtcggccgtgatcgaccggagcattctcttcgtcggctcgatgaatttcgatccgcgctccgaaacgcacaacaccgagatcggccttttcatccgcagccccgagatggcgcagcaggcgctcaagctcatcgacgtgctcaagcagcagggcgcttatcgcctgcgctttgccgaggacggcagcaagtcgcgcatcgagtggatcagcgaggacgccggcaagaccaccgtgctgaacgaagagcccgactccggcttctgggaccgcgccatgctcgagctgctggcgccgctcacgcccgagagcctgctgtaggccggccgttcatgttccctattgctgcacgttgaccgcttcgacctgcaccagcagcttcaccttgttctcgaagccgaagttcagcccccaggtgatgccccagtcgctgcgctgcaccgtggtttcgaagtcgccgccgcagacctggcggttgatgagcgggttcaggtagcagttgaagcgcacggccttgagcgtgaccggcctggtctggcccatcagcgtgagcgtgcccggcacgtcgaccaccttgtcgccgctgaattcgatgcggtccgccacgaagcggccggtcggaaactcggccacgttgaagaagtccttgctttgcacgtggcggttgagcaggtcgacgccggtgttgatggagctgatgtccatcgtgatgtcgaccttgccgctgctgccgctgccgtcgatctgcaccgagccgtccttggtgctgaagcggccgcggttggtggtggtgccgtagtgccccatctcgtacatcacgaaggtgtgggtcgggtcgatcacgtagctggcgttctttaccgggccgcccgcgggcttggcggccacgggcggcgccgtgtattcctgcgccagggcgggggtggcaagggtcgctgcagacagcgcggcagcgaggaagagcttcttcatggcaatgggcgtgcttggcgtgaaaacaaaatcagttgagaggacaaaaaaggggctcaaagcggagcgaggcccgcgagcgtgaacttgaagcgaacctgcacgtcgttgccgaccaccgaggtgtcggtccattcgccgtcgcccaccttgtagtcgagccgctggatcgtaaagcttccggtcgccaccgcgtagccgcccgatggcgcaatggtcaccggcaccgtgacctgccgcgaaatgttcttgatggtgagcttgcccgccatctcgaaccggccttcgcccagcgccttgatggcgctcgactggaagctggcctgcggaaaatgcccggtgtcgaaccacggggccttgggcagttcggcgtcgctcatcggcacgccgagcgatgcgctccccgtgtcgatctgcagcgcgacggtgccgccttcgggcttcctcgggtcgaatgccacctgcgcgtcgaatttcttgaacgtgccttccaccggcacgcccatctgcttgctgacgaaggcgatctggctcttgtcggccacgagccgggtcgccgttgcgggctcggcacctgcgggcgccagggcggcgaacgcggcggccgcgagaaagagacggaagactcggttcatctggcggattcctggcgtggcgcgggccacatgcgtttcaagatgccgtcgcggtcgatccagtggtgcttgagcaccgccgccacgtgcagcagcgccaccgcggccagcgtgaacgcgctgcccttgtgcagcggcttcagcacggcctcggccagttccttgtcgaccggcatgagatccggcagcggcagcacgccgaaccacacgaccggaaacccgagcgccgaactgtaggcccagccgaacagcggcaccgcgaggaacagcaggtacatcagcgcgtgactcgcccggtagccagtgcgctgccagcgcggcatggtggcggccgcatgcgacggcagcggcggcggcggatggcgcagccgccacaagagccgcagggccgacagcagcaggatcgtcaccccggcccatttgtgccagttgtagagcttgatgcgggccggcgacagcggcaggccggtcatgtagagcccgacacccagcgagccgacgatcatggccgcgagcagccagtgcagcgccatggccaccgggccatagcgcaggtccgcgggcgtttcggcaatggcggtggcggaagatggaggtatgtaggcaggcatcggaagcaggaccagcggcctgtgcgcggagcatatatcggaagcggcgaaggcaccgcacgagccgtgccaggcccatggccggcggggtcagtgccccgatgacgcctgctgcgcctgcagcagcaccgcatgcagctcggccggctgcaccggcttgcgcagcgcgtgccagccgcgctccgcggccagccgatgggtggcttcgccgatgtcggccgagatcagcgcgatggtgagcgacggcttttgccgctgcagccgttccgccaacgcgatgccgtcgagcccgcccggcagccggatgtcgcacagcgccgcgtcgagcgcgcgcaggtcggccagcgccagcgcctcggccgcgctgccgtagacgcgcggcgcaagctgccattgcctcagcagcgcactgaggctttcggccaccacggcgttgtcttccaccaccagcacggcaaggcccggatgcaatgcgcgcgccgccgcgtcggacggtggttgcggcagcggcgaaggagccggcggcaccggcgcatcggcaggcgccgcgggcagctcgaagccgaacaccgaaccacgccccggcgccgagcgcagcgacacctcgatgccgagctgccccgccagccgccgcacgatcgccaggcccagcccgtggccgcgctgcaggttgcgttcgacattgccgacctgctcgaagtcgccgaacacccgctcctgcgagtccacgggaatgccgatgccgctgtcgcgcacctcgacgcgccaggcgcgcccggtgtcgcgccggcgcgcccgcaccgccagcagcacccggccgcgcggcgtgaacttgacggcgttgtcgaccaggttggccagcacgcggcgcagcgagacggcatcggcccaggccaccgcgtcggccgggcagcgcaacctgacgcggccgtggccgaactggcgcgccagctcgcgcaagagcggcgccagcgacaccgccaccggctgcagcggatcggccgccgcctcgatgcggccgatttcgagcagctggttggtgaggccttcgagcgcctgctgcgctcgcgcgagcgacgccaccgtgtgctgcaccagcggcgcgtcggcgccgttgttcagctgctggcgcagtacctcggtctgcaggccgatggccatcaccggctggcgcaggtcgtggttggcggccgagaagaagcgcagccgctcggcctgggcccgttcggaggcgcgcaggccggccagcgcctgctcgcgcaagctgcgctcgttgaggcgcaggccgatgttttcctcgagctggcgcgagcgttcggccaccagcttccacatcatcgcggtcaggccgatgccgatcaccgacacggccatcatcgtcggcgcgccgagccacagcccggtgaggatcacgggcgccagcagcagcgtgatcgccagctgcgtggccggcgtgtagaacgagaccgagaacgccgacgagagcgtcattcccatcagcatcagcgcgagcagcagctgctgctcggcgtggcccgtgttgaacagcagcacgccggccagtccgtgcgccagctcccagatgccggtgcgcacggtgtgcaggcgctgtgcctcgcgcaaattctcgggcgtgaagggatcgggcaggcgctggggaaagaagccgcgcatgaccgtcaccaacgtgatcagcgagatccacaccagcgcatgagcgagcgagtattgccaggcgaagagggccgccacgccgcagttcagcaggtattgcaccagcagcaccgggccgatgggccggaccgagagccgcagcacctcgcactcgatcgcaaagcggtcgtttccggcaacaaccggagcaaccatgggcgcggtggtggaattcatcggccgagccactatatagagaagcggccgggcgcggcgacaatggcgtttccccagccggccgatgatgatggcaaaccccttgtgaacgatctttctctttttctgccttgcgccgccggcgtcgaggaattcctggcgcaggaagtccacgcgctcacgggccgcgtcgggcaagacctgctcacgctgcgcgggggcgtgcgggtgcgcgccgagtggcgcgacgcgctcaagctcaacctgcacagccggctcgcgcagcgcgtgctggtcgagctggcccatgcgccctaccgcagcgagaacgacctgtacgccatcgcgagcggcgtggcctgggagatctggttcacgcccaagcagaccttcaagatcgagaccacggcgcagcacagcccgctgcagagcctgaacttcgccacgctgcgcatcaaggacgcgattgccgaccgctttcgcgccaaggccaacggcgtgcgccccagcatcgagacgcagtggcccgactgccgcgtgttcgcccacctgaccaccgagcactgcacgctctacatcgacacctcgggcgagccgctcttcaagcgcggctggcggcaggacaagggcgacgcgccgctgaaggaaacgctggccgccgccatgctggctgccagcggctggtggaaccccgaaaccggccaggtggccgccgagccgctgtacgacccctgctgcggcagcggcaccatcgccatcgaggcggcgcagattgcgcgcggcatcccggccggatcgctgcggcgcttcggcttcgagaagctgctgccgttccaggcccacgtgtgggaggcgatcaagcagggcgccgcatcgtcggcctccgtgcgagaggtcgcgatcttcggctccgacgtgtcgcaccgcatggtcgactttgccgagcgcaacgcggagcgtgccggcgtggccgacgccatcgagtttcgcggcggcgatgcgctgcaacgcatgcccccggccgagggcggcgtgatcatgctcaacccgccctacggcgagcggatcgaggtcggcggcgtcgcgcgcttcggcgcccgcgaggccgcgcagacggccggcaatgagaatggcgaaggcggcggcgaaggtgaagacggcggcgagttctttccgcagctcgccacgcactggaagaagaactaccccggctggaccgcctgggtgctcacgcccgacctgaaactgcccaagcgcatgcggctcaaggagtcgcgccgcgtgccgatgtggaacgggcccatcgaatgccgcctgttccgcttcgacatggtggccggctcggccagaaagtaggtaggtaagcgggcgatccggtgggcggttacttcacgcccacgccgcacgccgcgttcaccgtcctggccgccaggtcccccggcaggccgtcgaatttcatcggacggacatcggtttcgtcgaactcccgcaccgccagcggcggcccgacgaaattcggctgcccgaagtaggtggcgctcacgtagcgtgccttgcgggcgtcgcagtccacgctcgcctttgccgcgacagaccggaacttgaggccctcctggctggtgcggggctcggccaggctgatgcgtaccgccacgagccgcttgcttccgtccaccaccacgctggtggggtcgacctgcacatagctgttggtcgcttccccggccgaaccggtcagggtgagccactccgcatgggccagcgggccggccagaagggcaagcaacagcagggaaggtcgtttcatcattcggaagtctcgaaaggcgccgtgacggcccggggcagcagattgtgaatggacgatacggtttgtgccttgcgatggcgcatggtgcaacatcggggttattccaaacgcacaaattttcatttctccagaagaagcaaacgccgcgccgggcgccttcgttgtcatcgacaccaacatcgcgctcgatttgctggtgttcgacaaccccgactgcctgccgctggccgccgctcttgcggccagcgaactgcgctggctggcgactgccgccatgcgcagcgagcttgcgcgggtgctcggctatccgctcatcgcggcgcgcctggcgcgcaggaacctggcggcagaggccgttctcgcgtccttcgacgagcgggtgcaactggttgcggaggcgccgccacgcgcctcttgcgtctgcaaggaccccgacgatcaggtcttcatcgacctcgcggtcgcgcggcgcgcacggctgctcagcaaggaccaggccgtgctgaccatgcgcaagcgcctcgccgcgcaaggcgtggtggtgcaggcggtgctggcgccctagccgacggagggcggcggcgcgccgtgccagcgccccaggagccgcgccaccgcgcgcacgcgctgcgtgtcgcggccccagcggcggctcgctggcagcttctgcgcccacttcatgcgccgcgccgcctcggcgatgcgctggcgcacgtcctcgcccacgtcggcgagcgcggcgtgccagtgcaggccggcggcttcgggcgcggcggcctccagcatcatggccgtggagtgcaggtagctgagccagtcgcgcgcctggcactcggccagcgtcatgacttcagccgggtcgtcctcgaagtcgatgtagccgatgaccccgtcggggcactgcaccaggttgcggtcgaaggcctggctcaggtgctggccgcgtacgtgcacctgcgcaatggcggccagcccttcgcgccagaccgcgagcagcgcggcgggcccggccgccgcagcctggtcgagccgctcctgcagcacgacggtggtgcggccgctttcgcccaggtcggagatcagcaggccgtccggctgctgcgccagcaccgcgggcacccgcaggcccgcggccgccaactgcctgaggcgccgcgcctcggtggcaatggcggcctcgccgcccgggttgggcaccggcttgatgatgtccagccgcgccatgcgcgcaaccgccgccatcacgcggtagccccacttgccatggcgcgggccggccttcttgagccagactcgctcgctgcccaggcggtggctggccacgttcttctgctgcttgggcagcgtgacgcgcaggaactcggcgtagtcgcccggtgccggtgcaaagggctgcgcgtcgaggggggcgggcgccgaggccgcccccttggcgctgtgcggccgcgccgaagcgccgcgtcgcaggggattcatgcggccagcggcaggttcgacaccaggccgtgcggcccctgcgtcacgggctgaaagctctcggcactggccagcggccagtaggtgcggaacacgttgtgctgcttgtcgagcgggcccagcaacgcgcccggctgcacctgcatcaccaggttgctgagcaggcgcacttcggtgtcggagatgcgccgcacgatgtggtgcgcggtgatctgctgcggatggtccaggccggcggcctgcaccagctcctgcagcgcgtgcagcgtgctgcgatggaagttgcgaacgcggtcggccttggtcggcaccaccagcgcctgctggcgcaccgggtcctgcgtggtcacgcccgtggggcaatggcccgtgtggcagctttgcgcctggatgcagcccagggccatcatgaagccgcgcgccgcgttgcaccagtcggcgcccagcgccatcatgcgcgccacgtcgaaggccgtgatcaccttgccggcgcagcccagcttgatgcggtggcgcaggttcacgccgatgagcgtgttgtgcaccagcagcaggccctcctgcagcggcgcgcccacgtggtcgctgaactcgaccggtgccgcgcccgtgccgccctcggcgccgtcgaccacgatgaagtcgggcgtgatgccggtcgcctgcatggccttgacgatcgcgaaccactcccacggatggccgaggcagaacttgaaccccgtgggcttgccgcccgacagctcgcgcagcctggcgatgaaatgcatcatctcgaccggcgtggagaaagcgccgtgcgaggcgggcgagatgcagtccacgcccacccgcacgccccgtgcggccgcaatttcgggcgtgaccttgggtgccggcagcacgccgccgtggccgggcttggcgccctggctcagcttgagctcgatcatcttcacctgcggatcgcgcgcgttggcgctgaaacgctcggcgttgaagctgccgtcctcgttgcggcagccgaagtagcccgagccaatttcccagatcaggtcgccgccatgcacgcggtggtgctgcgaaatggagccttcgccggtgtcgtgcgcaaagccgcccatcctggcgccctggttgagcgcgaggatcgcgttggccgacagcgcgccgaagctcatggccgagatgttgaacacgctcgcgctgtagggctgggtgcaaacctgggccggattggcctccgccggctgcggcgtgccgccgatcacgatgcggaaatcgtgattatcgagccgggtcggctgcatggagtggttgatccactcgtagcccgcgatcgtcacgttgagttgcgtgccgaaagggcggttgtcggggtcgcccttggcgcgctggtacaccagcgagcgttgcgcgcgcgaaaacggcgccgcctcggaatcgctctcgatgaaatactggcgcatttccggccggatgaattccagcaggaagcgcaggtggccgatcaccggatagttgcgcaggatcgcgtggcgcgtctgccgcaggtcgtgcacgccggtgccgctgagtaccgcaaaaaccaccagcgccacccaggcggcccacaggtgcggggacaccagcacggcgaccaggctggcggccaggcccgccacgcacagggcaaaggcgctgtaacgcgttggaaacggaataatcgtgggcatggagatgagtggactgccggagcctgctgcatcatagagggctgccccgaacttgccatgatgacgaccaccaacgacaccccccaggccgcagcacccgcccccgcccccctcggccccgacgatttcgacgccctcgaccaggcgctcgacgccatgcgcgagcatgacgaggaaattccccagtgggagttctgcgaaggcttcatggccgcgctgatctgcacccgccggcccatcgagcccgccgaatactggcccgtgctgctgggcgacggcttcgtgccggcccagcacatggagttcgtctggaactggaagcgccgctggctcgaaatcgaggaggggctggacgccgacgtgcagtcgctcgacgacgaacgcagctggcagcccgaagtgctcgacacccgcggcgccatcgcctcgctgcccgaggaagagcgcgccgcggtcgagggcgacgaaattccctccttcgcgcaggtctgggcgctgggcttcatgtacgcggtcgaaaactggcccgaagactgggccaccccgcgcgacaaggacgccgcgcagatgctcgacgatgcgctcgacaacatcgtcgcgctgaccgaggacgacaaggccaagcccacgctctcgatgttcagcgacgacggcccgcccagcgtgagccagcagcggctggacgatttcggcgccgccatctgggccgtgtacgacctgcgccagctctggaagagcctggggccgaaggtcgagaccatccgcaaggaagcgacccccggccgcaacgatccctgtccctgcggcagcggaaaaaaatacaagaagtgccacggtgcctgacaccaggccggccagcgcagcgctgacgccgcgcgcggcgtgggccatggtgctggcgctttgcgccggggtggcgctgagccaggcctttcgcaccgtgggcgccatcatggcgagcccgctgcaggccgacttcaggctctcggcccaggcactcggcattttctcgggggcattccatttcgcctttggcgcgatgcagctcttcatgggcatcggcatcgatctgcacggcgtgcggcgcacggtgctcgtcgcctttccgatcgccattgcgggcgcgctgctgtcggcggtggcgcccagctacctggtgctggtggcggggcaggcgctgatcggcatcggctgcgcgccggccttcctggtgtgcaccgtgttcatcgcgcggcactttccggcggcacgctttgccaccgtgtcgggcctggtgctggccatcggcggcgtcggcatgctggtgacaggcacgccgctcgcgtggctggtgcaggcgtattcctggcgcgccgggttcctggtgctggccgtggcctcggcgctggcttggctcgcgatctggcactgggtgcacgagcccgcgtcggccgttccacggacgaatgaatccattcccgaggccatccgccagttcggcgcgctgctggccatgccgcacacgctgggcatcgtcctgctcggcgccgtgacctacgcggcgttcatctcgctgcgcggcttgtggctcgggccgctcatgatggagcgccacggctattcgctggtgcagagcggcaacgtcgcgctggcagtgtcggtgatctcgctcttcggtgcgccgctgttcgggcgcctggaccgcgacggccctgcgcgccgccgctggatcgtggcctgcgcgctcggctatgcgggcctgtttgcgctcatcgccttcacgcattcggcttggctggacatcggcggcatggtgctcatcggcatgctctcgggcttcatcgtctggcaatacgccgacgtgcgcgtggcctatccggtcacgctcacgggccgcgcgatggcggtgttcaccatggcgatgttcctcggcgtggcgctcatgcagtggggcaccggcgtggcggcctcggtggccgcggcgcatggcggcgatccgctcacggccgtgctggccaccattgccctgctgctggtgctgggcatcgcggccttcgcctggctgcccgcgccaaaggcccaagtcctcagatcttgaaggcgcgctggatgtcgggccgcacgaggtccgcgtattcgcggtgcttgcggatgtagcccgcgatgaactggcacaccgggatcacgtgcaggcccttggcgcgtgcctcatcgagcacgtagcgcgcaatgcccgagcccacacccttgccctcgtgctcgggcagcacctcggtgtgggtgaacatgatggcgtcggtcagcaggttgtattcggcgtaggccgcgagctggccctcgagcgtggcttcgtagcggtgctgggcttcgttgttggtgatgacgaggttgctgttgctcatggctggcgtgcgagataggtggcgaggttggcggccgcggtggtgcgtaccttggtgcgcagcatcggtgtccagccaagcagaagaccgggggcgcccaaggcctggcgcgaccaggtccagaacgcaaagctgtcgcgctgcgtggcaatcagcccgtcgggcgtgaagccgaagcgcgaatccacgctgttgtcgaccagccggccggtggcgctgaagcggtagtgcgcgtcccagtgggcctggccgctggtttcgtcggcgtgcacgtcgcgccaggtcaggcgccagacgtcggcgcccttggcccgggtggcatcgcacagcatgcgccacatgccgcccacctggcgccggccgcgcagcgaaaaggcctcgtcgtcgaacgccgcgtcgctggcatagcaggcggccatggcgggggcgtcgagccatgcaaaagcctcgtagaagcgttcgatggtctgggcattggctgctgctgtcatgtcatggggcctcttttgttgtgtcggggtgcgggccgagcaggcccaccaatgtctggagcgcgtagtgcaccgtggccgcgcgcaccgcggcgcggtcgccctcgaagcggcggcgctcggtgcgaacctgcccgccgaccgaccagccgaaccacacggtgccgaccggcttttcggggctgccgccggtcgggccggccacgccggtcaccgccactgcggcctgggccgccgatcgcgcgatggcgccttcggccatggcgcgcgccaccgcttcgctgaccgcgccatgggcttcgatcagcgccgcatcgacgccgagcagctcggtcttggccgcattcgaataggtgacgaagccgcgctcgaaccacgtgctggagccggcgagttcggtgcacgcgcccgcaatgagtccgccggtgcagctttcggccgtggccagcatccagcccttcttcagcagcaggtcggccgtggtcgccaccagcgcgggcgtggcctggtcggcaagaaagttcgacggcaaggacggttccatgaagttcaccatgcgcgccagagcgcgatgaccagcagcgtgcagaacgccgccaccaggtcgtccaggatgatgccgaaaccggcgcgccaccagcgcacctcggtggcatcgcgttgcttgaacaacccgtcggcccaggccaccggaccgggcttggccgcgtcgaagaagcggaacaggccgaacgccaccgcctgcgcgagcaggcccgccggcgtgaccagccagagaacgatccagaacgcgatcacctcgtcccacacgatgctgcccgggtccgccacgcccatgtcgcgtgccgtgacgctgcaggcccaccagccgatgggcagcgaggccaggatgacccaaccgatggtggcgggcgagagccagagctgcatcacggcaaaggccgcccaggcccacagcgtgccgacggtgccgggcgcgatgcgcggcagccccgagccgaagccgagggcgatgaaatgcgccgggtgagacagcaggaagcctgttgtcgggcggggcgtggcttgcggcatggcgcctgcggaggaggaagaagaaggggaagaggcagcttgcatcaaggccagagtgtcgcgcattcgggggcctgtccaagaccctctatttatcaaagcaatagcttgtttaattcagggcagaggcctagtatccgggccttgcttcgctcccgatcgtccgccacggaccgcgccaaatgaccgctgcctcatccgactcccctgccgtcgccgacccttcctcgcggctgcgcccgctgcctgccaccgccgcctggagcgacctgttccgcgggcgcaacggctggcgcgccgtggctctcacgggcggcgtcgcgctgcatgcggtcaacgtgcacatcgtgaccaccgtgctgccgtcggtggtgaacgaaatcggcggactcgactggtatgcctggagcaccacgctgttcgtggtgggatcgatcctcggcgccacgctgtccgtgcggctgctcgccaggctggggccgcgcggcgcctgcctggtggcgctggcggcattcaccgcgggctcgatggcctgcgcgctcgcaccgggcatgtcctggctgctggtgggccgcacggtgcaggggctgggcggtggcttgctcgcggcgctgagctatgcgctcatccaattggtgttcgcgccgcggctgtggcctcgcgcggtggcgctggtgtcgggcatgtggggcgtggccacgctctgcgggcccgcggtgggcggcctgttcgcagaggcggggcactggcgctgggccttctggtcgctgctgccgctggcggcgctgcaggcgctgctggtcatggtgcagctgcggcccgcggccggcgtacggcacgagcgcgcggcccgcatgccgcgcattcccgcagtgcagatcggcttgctcgcggcatcggtgctggtgattgcggcgagcgagttcctgccggcgctcgcctggcaggccgcgggcgtggcgctgggtctggcgctcggcgtggccgccacgcggatcgaccggcacgccgcggtgcggctgctgcccaccggcgcctacgcggtgcgcgcgcccatgggcgccatctatgcgagcgtggtgctgctgttgatcggcaccaccaccgagatcttcgtgccgtacttcctgcaattgctgcacggccattcgccattgtcggcaggctatctcacggccgcgatggccggcggctggagcgtgggttcgctgctgtcgtcgggccgcggcggcgcgggcgccgaccgcatgctgcgcgcggggccggtggcctgcacgctggggctggccgcgctcgcgttgttgctgcccgcgcccggccgcttcgggccgggactcgaagcgctgctggccggccttgcactggcggccgtcgggctgggcgtgggtatcggatggccgcacctggtcacgcgcgtgatgtcgctcgctccggccggacaggagggcctggcctccgcctcgatcacgaccgtgcagctctacggcatggccgtgggcgcggcggtggcggggctggtggcaaacgcagccggcctctcggagccgggcggtgccgcgggcgcccgatcggccgcgctatggttgttcgcgagctttgcagtcgcgcccgcgctggcggcatggctggttgcccgcttcgttgcgccacgccgccgatgacggacggcgcccttcaggccaccacgccttcccatcggagctgccgcctctggcccgcaaggcgccgcgcttctccgcgcagcagcgccaccagctcgtaggcgtcgggtggcacatgggcgccgcgccaggccacgtgctggtcggcgcggcacagcaccaggcggtgcatgtaggcgcgcggcacctccgcggcgtcgatgtcgaccacggccagcggcatgccgtaggcgcgtgccgcgcgctcgagcgccgacacgtccgcgctgcggtcgaaacgcagcagcgtgtagcccgggccgaacgcgtcgtagagcgagcggccgtcggccagccagaaatgcggcgcgcggcagcccggcacggtggaaggggtgaagccgcccatcgaataggccggcggcgcgtgctcgccatcggccacgatgattggcgagccgccatagaagtagccgaaattcaggcctgcgcagcagaactgctgcacgttgagttcgtaggcctcgcgtccgagctcggcgcgcagcgcatcgccttcggggccgggcgcctcgatgtcctgcggcacggcgcggcgcgcgcggatcatcttctgcgcatggtccatcgcgaagttcgacacctgctcggtgatcggcaggcgctcggcttcgtacgcatcgagaatgccttcgtcgccccagcccctcacagaggccgcgagcagccacgagaggttgagcgcatcggcaatgcctgcgttcatgccgtagcccgcgtacggcacccacaggtgcgccgcatcgcccgccaggaacacgcggccttcgcggaaccggttggccaccaggcggcggccgatccagtcttccttgctgatgaggtcgtacgagaactcgggcccgacgccgaggatgctgcgcagcgcctggtcgcggtcgaccgaatcgaactcgggctcctcggcgttcaggtggttgtgcaccagccaggtctcatgcccgtcgatggcaaacatcgtgccgcagcggcgagggttcatcgcgtagtaggaccaggccggcttgccgggaatcagcgcgcgcagctgcggtgcgcggatgagggtcgactgcacgcgctggatcacggccgtgccctcgagcctggcgccgatctgcttgcgcaccgcggagccaccgccgtcgcagcccaccaggtagcggcagcggatgtggcgcgtcgcgtggctgtcgagatcggtggccaccgcgctcacgccatcgctgtcctgcgtgaacgccgtgaactgggtgcggttgagcagctgcacgccgggcagggcggccgtgtgcttgagcaggatcggctccaggtagatctggttgatgcggtgcggcggttcgggcgtgggccaccaggcgtcgggcccttcggtctcggtgtagcggtcgcgccggcacggaatgggaatgcgcgagagctccatgccggtcacgctggtgcgaaacgccacgtcgttgggatagtccgcgggcagccccgcatcgcgcaactgctgcgccacgccaaggcgccggaactgctccatggtgcgcgaggaaacatgattgcacttcacgctcggcggctcggcgaaatggcgggtttcgcagatgaccaccgagacgccgtgcgaggccaggtccatcgcgagcgtgagccccaccgggccggcgccgacgatcagcacgtcggcatcgagcgtcttgtctgtcatggcttctccaggctttcagtcgagcttgatgcgggcgtcctggatcaccctggcccacttcttcgtttcggcgcgaatgtaggcatcgaaggcctcgggcgagcccggcgcgggttccacgcccaggttgcgcatcgcggccttgttctgttcgtccgccagtgcggcgttgatctcggcattgagccttgccaccacggcggccggcgtgcccgcgggagccaccacgccgaaccagccggtggagtcatagccgggcagcccggcctcggccaccgtcggcacgtcgggcagcatcggcagccgctcggggctcgtcaccgcgaaagcgatcagcttgcccgccttgatctgctgcagcgccgagggcaggtccaccaccgcaagcggaacctggcccgccagcgcatcgagcgcggccggcccggagccgcggtagggcacttccaccagcttgatcccggccatctgcgagaacaacgcggccgacagatgcatggccgtgccgttgccgccgtggcccacggaaagcgagcccggcttggccttggcaagcgcgatcagttcggcctgcgtcctggcgcccacggaggggtgacctacgatcacgaagggaatggccgcgagcatgcccaccggcttgaagtccttgagcggatcgaagggcatctgcggatacaggctcgtgttggccgacagcgcaccggccgcgcccacgcccagcgtgtagccatcggccggcgccttggccaccagcgagagacccacgttgccgccggccccgggccggttgtccaccaccacctgctggccgagcttctcgttcagccgcggcaccagcatgcgcaccacgccgtcggcgctgccgccgggcggaaaggtcaccaccacgcgaatcggtttgttcggaaagtcgccggccggggcttgggcctgcgcgggcaaggggctggcgaagagcgcgcaggccgcggccagcagcatctgccggcgaagttcgtgccgtgccctgcgggccgtcgttgccgtcatcgcatccccttgatgtcatgtagttttggtttgatgcggattgaacgatgcccgcattcattcgtaaatcaagaaattccgaatgaaatatcatcttttctgatgaatacgaacttcagtcctacgatccgccagctgcgcgcttttctcgccgtccaccagctgcgcaagctcagcgctgcggcgcagcggctgttcgtgacgcagtcggcggtgagcatgctgatccgccagctggaggaaggactgggcacgcggctgttcgaccgcaccacgcgctcgctcaagcccacggccgcggcggaagagatgctcgccacggtcgagcgcgtgctgcgcgacgtcgattcgctctcggccgactttcgcgaactggccacgctcgagcgcgggcgcgtgacgctggccatcacgccgacgctcgccgcgatgctgctgcccgacgcgctgcgcatattcagccagcagcaccccaaggtgcgcgtgctggtgaacgactgcgcgcccgaccagttcatttcgcgcatcctcggcgagcatgtggatttcggcatcggcacgcccgagcggcccggcgccgaggtcgagacggagcgcctgatgcgcgaccacctcgcgctggtgtgccgcagcgaccatccgctggccaaggcgcgcgtggtccgctggaccgatctcggccgccaccccgtgatcaccgtgcgtcccggctatggcgttcggccgctcatcgacggcaccgcggccgaagccggcgtggcgctggacgtggtcaacgaggtgtcgttcctctcgaccgcgctgtggatgacggcctgcggcatgggtgcgtcgatcatgccctcggcctttgcacgggcggcgggcgatccgtcgctggtgatcaagatgctcagcgcgccgcgcgtgtcgcgcgacgtctcggtggtcaccaagcgcgggcattcgctgtcggccgcggcgcgcagcttcatcgacgtgctgaagcaatcgctgtaggccaccgtagaccgctgcatgccgtccgacgtattcgccggcgtcgtcggccatcgtatgctcggcggctcattctcaagcgaaggcatggtcatcatgaaaagaaccctggtccgtttcaacgccttgtggctgtgcctcgcgttcagcgtgctgctcgccgcctgcggcagcaaggaggcggaacagcgcaccgccttcatcggcttcctgcagacccgcgtgctcgacaagccgggcctgcgcgtgcccacgctcacggccgacgagaaagcctctttcggcgactatgcgcagcactacgcggtgattgccgatttcaacgaaggcatgaacaagtcggtcggccagccgatgagccaggtgatggccaagggcgcgctgcgatcggtggccgacctggcatcgcgccgcgacgacctcaaggctgccaaggacggcctgggcggcctgcgcaccgcgctcgacaaggagctggccaaggccgacgccgcgcatgccgggctcaagcagccggacgacctgaagcaggtctacgacaaggcttatgaaaagaccgtcgcggcaccggccgccaccttcaaggaggtgttccccgcgctcgattccgtgttcgacggcgcgctcgcggtgggcgactatctcgaaaagaacaagtcgaagatccaggtgtcgggcgcgtccatgaccgtgagcgatccggccgtgcaggcagaactcaacaagatgctgcaggacctcaatggccattcgaaggccatcaacgctgcccagaccaaaatgcaggcaatggtccgcggatcctgatcacgcgaagtggtcgaaggagccgaatcgctgggcaatcggtgccccgctggcgtccacgatgcgcaggccggcatcggcctcgatgcggccgatgcgcgtgacgcgcgtggcgctctccttgccggcttgctcgaccgcggcacgcgctgaaggcgccgcggtgaagaccagctcgtagtcgtcgccgcccgagagcgcgcaggtgcgcagcacgtcggtgccgaggcccgagcccgcggcggccgccacgacggacgcggccgcatcggcgtcgagcgtggcgcccacccggctcgacgccaggatgtggcccaggtcgccgacgagcccatcgctcacgtccaccgccgcggaagccgtgccgcgcagggcgaggcccagtgccacgcgcggcgtgggctgctccatgcgcatccgcgccgctgcgaacacatcgcccggcagtgcgagcgtgccgcgaaacacctcgagcgcgagccgtgcgtcgccgagcgtgccgctgacccagatgtcgtcgccggtgcgcgcgcccgatcgcagcagcgccgcgccggtgggcacctcgccgaacaccgtaatgcagatgttgagcggcccacgcgtggtgtcgccgcccacgagttcgcagccgtgttcgtcggccagcgcaaagagcccgcgcgagaagccttcgagccagggctcgtcgacaccgggcagtgccagcgcgagcgtgaaggccagcggcctggcgccgcaggctgcaaggtcgctgaggttcacggccaacgccttgtggccaagccgcaccggatcgacggtcgagagaaagtgccggccttcgaccagcatgtccgaggacacggcgagctgcatgccgggcgccggtgcgagcaatgcgcagtcgtcgcccacgccgagcggagagcgcttggcggggcgtttgaagtagcgtgcgatcaggtcgaattcacccatggggcgagcataagcgctacgacactcatgcccgcgcgcgccggttggacatcaccacgttgtccttctcgatcgcctgcccgccctgcatggcagcgatccaggcctcggtgctcgtcacggctgcgaaattgctgtggaacacgacgctgaacacgcggtggatctcctcggcgctcacctgaccggccgcattcgaataaggcagcgcgccggtggcatccgacaggaactccacgttcagcccgcggtgcatcgcctcgaacacggtcgatgcatcgcagttctgggtcatgtagccggccacgctcagcgtgtcgatctcgtggcgcgcgagccagtcggcaaagtcggtgccggtgaagacgctcgggaaggccttggtgatcaggtggtcgtgcggccgcctggcgatttccggatgcagctggccgttgtgcgtgtcggcccggaacaccggggcgcccttgggcgcatggtggcgaaccaccaccacgggcgtgccggcggcatgggccgcgtccatggcccgggcgatgttcggcagcgactgctcgacgggcgggtattcgatcggcaatccgccgccttcgaaatactcgttctgcacgtcgatcacgacgagggcgcggcgcggtgcggtggtgttgctcatggtctttctgctccgttggatgtgttgtggaatgaggtgattgttcccgccggggcgcatgcgagaaagtggcccggaagccattcatcgataagatcgggccatgcaacgcaaacccgccgaaaccatcgccgtcgtggctttcgacggcatcagccccttccacctgtccgtgccgtgcatggtcttcggcgaagaccgtaccgaatcgggcgccccgcgttttcgtctccaggtgtgcgccgctcagccaggccaactgcaaaccaacgcgggtttcacactcgtggtgacgcatgggctcgaagccatccggcgggcgcagatcgtggtggtgccttcatggcgcgacgatgggaggcccgcaccgcccgcgctcattcgtgcattgcaggcggcgcaccgccgcggcgccatcgtggtcgggctgtgcctgggggccttcgtgctggccgaggcgggcctgctcgacggccgcccggccaccacgcactggaacctggccgaagcctttgcaaggcaatatccgaaggtcatgctgcaacccgaggtgctgtatgtcgacgatggcgacgtgctcacttccgcgggcacggccgcgggcatcgactgctgccttcacctgctgcgcgtacgctacggcgccgaggcggcgaaccgtgccgcgcggcgcatggtcgttgcgccgcaccgagagggtgggcaggcccagtacatcgaacggccggtgcctgccgcggccgagagcgaccgcctcgcgccgctgctcgaatggctgggccgccatctccacagcccgcatgagctggacagcctggccaggcgtgcgctgatgagccggcgcactttcacgcggcgctttcgtgaagccaccggcaccacggtcggccaatggctgcagaaccagcgcctggcgctggcccagcggctgctggagaccaccggccaccccgtcgagcgcgtggccaccgatgcgggtttcggctcggcggtatcgctgcgaaagcacttcgtcgcggcgttcaagacctcgcccaccgcgtaccgcaggcagttctcgcaggaggtcgtggccgcctgaatcagatcgatcaggcggcgccgcggaagcgcagcgctgcctgccgcaccacctcggccagcaggcgctccttgccctgcttctcgcgcagccatcgcgcatcgttgcggttggcttcgacgctggtgcgcagttcgcccagggcctgcgtggcgttgagcgcctcactgtgccattcgagctgcgtcatcgtcatgaggatgtggtcgcgcagcggcatgtgctggccgctggccgggtccacgtacaccgcgtcgagtccgaagcggcaggcctggaagcggttgtaggtgtagacgaggtagtcgtcttccgtcggctcgaagggctgctcctgcagaaaccacgcggcaagcgactgtacgtagcccgccagcgcggccgcgcgctcgacggtgagcggcgtgtcgaacacgcggatctcgatggtgccgaactccggcttgggccggatgtcccaatagaagtctttcatgctgcgcacgacgccggtgcgggtcatgcgctcgaaataggcctcgaactctttccagctcaaggtgaagggcgcgcggcccgagagcggaaacgcgaacaccgaattgagccgggccgagtcgaactgcgtgtcctgcccctgcacgaacggcgacgaggccgacagcgcgatgaagtgcgggatgtagcgcgacatgcggtgcagcatcagcagcgccgcatcggcgtcggggcagccgatgtgcacgtgctgcccgaagatggtgaactgcttgctcaggtagccgtagagctccgacagctcgcgaaaacgcggcttgtcgtagatgcgccgctcgtgccattgctggaacgcatgcgtgccgccgcccaccaccgcgatgttgagcttgtcggcattcttgatcagcgcctcgcgaatgggcgagagctgcgtgatcacgtcctgcgccgagtggcagatgtcggtcgagatctcgatcatgctcgaggtcatctcgggcaccacgctgccggggagcggcgtctgcgccatcagccgcagcatgtcttcggcgtagggcgcaaggtcgtagtcgtgcgtgttgacgagctgcagctccagctccacgccgagcgacagcgcttcggagtggttgaagggctcgagcttgaccacgcggcgcgcggggtccacgggcagcggtgcggaacggaagtcgtcgctgtccgccgcgttggacatgttggagttgtcgggaaaagccatggccgcggtcatcgctgcgtgtcctccgtggtgctgaaggcctggggcgtccagggcaccgagctttcgcccaccgcatggatggccacggtggcgatcacggcacccaggacttccatcaggagaatcgagggcagggccacctgcgtgatcatggtgccgagcagtggcgacgcggtggtgaagttcgaagcgatgagcagcgcgatcgacgacagtggcgacatcgcgcagccgacccagaaagcctggttccagctagcgccgctgcccgggttggcaatggccacgccggcgatcttggcgaacaggcggatgccgatcaccgccagcaccacgctggccaccggcagggtccagtcggcctgcgccgccacgatggacaccagcacgaacatcagcatggtgagcagcgacgaggccgtgccgagctgccgctgccaggcccagggcttggggttgagcgtcttgagcagcaccccgccgatcagcgcggccagcggggcggagccgccgacgtgggccgtgagggcgctggcggcggcgatgagcgcgagcagcaggatcgaggtgttctcgctcgtcgggctcatgaagcgcagggccgtgcgcagcgccagcgccaggatgccgccgatcacgaacgaaaggccgagcaccaccgccaccggatagagcttttgcagcagcgtctgcggcgcccgctcgatcaggccggcctgcgcatagccgagcgtcagcgcatagaaggtgttgagcgtggccagcgtcatggcgcgttcggtcaccggccccgaggcgcgggtgtcgatgatcacgcggctcagcaccgccggcgatgccacgatggccatcagcgcgatcgggttggccaccggatcgggcaggcccagcagctgcagcatccagaacacgccgaagtaggtgagcgtggcttcgagcaggctttgcaccagcaccatcgggttgtggcggaaccagcgcagcggcagccggccaccggcctcgaacagcaccacggccgcgcccagttccagcagaaacaggctgatgccgcgcagcggccagatggcgccttcgaagccggccaggccgaccaccgcgccgaccgccgaatagcccaccaccttgggcaagcccaggtagcgctgcaccaggtgaccggaggcggcggccgcggccaagaggagcgaccacagcacggtcggcaggcccgccgaagggcgcagccactcggaccagaagcccagcaggtcgttgaagagactcgtcagattcatgcaggtagaaaaaagctgatggaccggctgcgccagcgtgcacggatcgcgccgcggatgcgcacgcagtcaccgaggttgacgccgtgcgcgcgcagcgccagacgaaaagcgaaatagaaaacccacgcgcacgtcgagcgcgcccactccctggaatgggcgccaccgctcaccgaagcgagggctgcccggccgacagtgtcgcatggtgccatcccggcgatgcaggacaaaggcggtttctgccgatcccctgatgaagaaaggagtcaggccagaaacactgcggaaccggctttgccgggccgctggtgttgcccccgagagtactaatgcaatacgcgcgagaccggtgcgccgccgatgtccgcctccagcacgaacatcggaatcggcacgtcgaagcgctcgccgtcctcggtcaccacgaaatagcttccgtgcatggtgccgctcggcgcctgcaggcggcagccgctggtatagcggaacgattcgcctggcgccaggagcggctgctggccgatcacgcccaggcccttgacctcctgggcatggcccgaggcgtcgttgatgagccagtggcgggcaatgagctgggcaccgatttcgcccacgttggtcagggtgacggtgtaggcaaaggtgtagatcttgtccttcggcgaggactggtccgcgagatagcgcggctctacttggacactgatggggctttgcggcatgcgcgcgatggtaactggagccttctcttgcgctgctttccgggttttgcgccggctgcgacaatcggcgcatgagcacgccgttccgcatcgccccctccattctttccgccgatttcgcccatctgggcgacgaactgggcaaagtcatcgccgccggcgccgactggatccatttcgacgtgatggacaaccattacgtgccgaacctgaccttcggaccgatgatctgcaaggccctgaagccctacgccaagacggcggacggggagccggtgccgatcgacgtgcacctgatgatccagccggtcgacgcgctggccgcatctttcgcggaagcgggcgccgactacatcagctttcaccccgatgcctcgccgcacgtgaaccgcagcatccaggccatcaagggcgcgggctgcaaggcggggctggtgttcaaccccggcctgggcctggaagcgctcgactgggccatcgacgacatcgacctgatcctgatcatgtcggtgaaccccggctttggcgggcagagcttcatcgattcggcgctgcgcaagatcgaactcgcgcgcaagcgcatcgagcagagcggccgcgacatccgcctggaggtggacggcggcatcaaggccgacaacattgcgcgcgtggcttcggccggcgccgacaccttcgtggccggcagcgcgattttcaacgccaaggactacggcgcggtgatctcgtcgatgcgcgagcagctcgccggcgtgggcaagaagtaagtccggctcagcgcttgaccttgtcgttgtagacgcggtccgtcacggggccgcggtcggtgtcgaccgtgccgcgctcgatgtcgtcatggcccctgcggcccacctcgggcggctgcccgtcctgcgcttcctggctgtccgaagactggtcatgttcgtggggcaggcgcggcgccgaatcgccgccctgttcgatcttggtgtcgccgccgccggcgtcccgcaccgggtcttccggggtgctgggttccttcggacggggcttgctgctggtcatggcgctttccttctcgatggggtcaggctgaagcctgcatggcacccggcgcgcttccggtaggacaggcgaggcatgccctgtaggccccccgcgccggacctcgggcggccttgcttgcgggtcatgtggatgattgcgccgctatgaaacgagtagcagctttgcgccaagggcaaggcctccgcaataatcgcccgcatgtcctccgatccttttgccggcgccgccaccgacagcctgcgcatccacaccgtggcctcgctgaaccccggtccccggctgctcgtgatgggcggggtgcatggcgacgaaacctgcggcaccgtgggcatcgagcgcgtgttggccgaactcgacagcggctcgctccagctgctgcaaggccagctcacccttgtgcccgtggccaatccgctcgcgcggcggcgcctgcagcgcgaaggcgagcgcaacctcaaccgcctgttcaagccgagcgaggcgcctgccgactatgaaggccgcgtgaccaacctgctgtgtccggtcatcgagcggcacgacgtgctgctcgacctgcactccttccagagcgagggcgaggccttcgcgatgattggcccgcgagacaacgccggccagctggagccctttgcccgcgccagcgaggaggggctgctcgcactgcacctgggcacgcccatcgtggtggaaggctggctcgacatctacgccgccggactcgcgcagcgcgcggccggcgctgcggtcggcgacgacgcgctcgacttcggccgcggcaccaacgaatacatccgcaactgcggcggctatggcgtcacgctcgaatgcggccagcaccgggacccgcaggcgcccgaggtggcgtggcgcgccattcgccgcgccctcgcgctgctcggcatggcgccgctgccgccagggttggcgatcgagccgcccaggccgccccaattgctgcgcctttcgagcgtgacggaccggctcgatgaggaagacagcttcgtgcgcgactgggccaccttcgatccggtgcagcgcggcgagcccatcggcatgcgccacgacggcacgctggtgagcgcgccggacgacgggttcatcgtctttcccaatgcgctggcgctgcccggcgccgaatggttctacttcgcgcgtccgagcgaacgcgtgctcggccccgtggccagcgccgccaacgtcgcatcggcctgaagcatccctccttccccctctgggggaaggctgggatgggggcaggcagagcgctcggtgggcacgccgcatgcccccatcccagccctccccgggaggggagggaaaaaataccggcctgggccctacggcgcgcgccgccgcgctcctacatcgcgcaacggccccgggcgaaagtctggaggccatggcagtctcgaaaaaggcacctctgccgcgcatcacccatgccgagcgcgtgatcgatgccgcgagcggcatcaccaagggcgagctcgcggcctactacgccaccgtggcgccgttgatcctgccgcacctcgagggccgccccgtggcgctggtgcgcgcgccggagggcgtgggcggcgagctgttcttccagaaacacgcgcagcacagcgacatcgccggaatcaagctgctcgatccggcactggatccggggcacgacccgctgctgcagatcgacaccgcgcaggcattgctgggcgccgcgcagttcaacaccatcgagctgcacacctggaacgccacctcgcgcgccctcggcaagcccgaccgcatgaccttcgacctcgatccgggcgaaggcgtcgactggcagcagatgcaggaggcggcactgctggtgcacgtgctgctggacgaactgggcctgccggcgttcgtgaagaccagcggcggcaaggggctgcacgtggtggtgccgctccggcgccagttcggctgggacgaggtccggggcttctcgcgcgccatcgtcgagcacctggcgcgcaccgtgccggagcgattcgtcgccaagagcggtccgcgcaaccgcgtgggcaagatctttgcggactatcttcgcaacggcttcggggccaccaccgccagtgcctggtcggcgcgcgcccgcccgggcctgggcgtgtcggtgccgctggcctgggaagagctgccggacctgggtagtgccgcgcactggacggttgccaacatcggcgagcgactggccgtcggcaacacgccctggaatgcgatggaacgcagccgcacggcgctgggcgctgcgatgcggacgctgggctacctgccgtagcgcacggggcctactgcgggatttcgtcggtcgtcacttcgaagcgctgcaacgagttgacgccgaacaccatggtgatcggcacgtcggccgcatcgcgtccgcgcgcaatcacgatgcgcccgatgcgcggcacgttgtggcgcgcgtcgaaggtgtgccagcgctcgcccaggtacacctcgaaccaggcgctgaagtccatcggatacggcacgggcggaatgccgatgtccccgagatagcccgtggcatagcgcgccggaatgttcatgcagcggcacagcgtgatggccaggtgggcaaagtccctgcacacgcccgtgtgctcgcgaaagccctcgagcgcggtgcgcgtgggccgcgcggtctggtagtcgaagcgcaggtgctcgtgcacgaagctgcagatggcctgcacgcggtgccagcccggcgccacgctgccgaaggtgtcccatgcgaactgcagcagttcgctgtcgacctcgcaatagcggctcggcagcaggaagggcagcgccgacaccggcaggtcggccgccgcgtgttcgacggcgccgtagtccaccgggtcggcccagccgggatcgaacaccaccgcatggttgcgcagccgcacgctcgtcacgcccgcgggaatgcgcacgcgcgcgcagtggttgtcgaagctgtccatgaagtagtcggtgtgcagcgccggggtgatggtgatgtgctcgccgtcctggagatccgccgcgcgcgagggatgaacctgcagcatgtagatcaaggccgtgggtgccgtgacggcgagctcgatgtcgaaaccgatcctgatctgcatttgctttttccctgtgtgtgaatcgtgtgttgtcggtgtcgtgcaagcaggcttcatgccgtctgcgccgatgctatcgagagcctcgtgccgcggcacgcgggcggatacgccaggcgccgtaggcgggggccagggggtgtcggtgcgctcctacctttttggcgccgcctctcccacacccgagggcgagccgccactacgggtaacagtgtgagaaaaacataacctttggattcgctcgcaaccgcctcgcgatctcgctttggtcgcttcatggaggctgcagcgcaagcatcgagtcattgaaatctgatctgctggagcgaatcatggagttttcttcgctgttcgattcactcaccggtgcctggggagatgaaatccttttttgggtggtggccgccgtggcgggcttcatttgcctgattgcgctggtgaacgtgctggacctttttatcgacaacgaagttgaccctcccatgaaagatcatcgatgacgcctcagaacaaggccgccgccggacgccggtcaaaggccacggatggcagcaatgccaagcagcagcaactcgatggcttcgcgaccgatcatgcgcccaatctgacgaccaaccagggtcttcagattcccgacaaccacaactcgctcaaggccgggttgcgcgggcccacgctgctcgaagatttcatcctgcgcgagaagatcacgcacttcgaccacgagcgcattcccgagcgcgcggtgcacgcgcgcggctccgcggcacacggcttcttccaggtctacaagtcgatgtcgcagttcacctcggccgacttcctgcaggacccggatgcgaaaacgcccgttttcgtgcgtttctcgaccgtggccggctcgcgcggttcggccgacacggtgcgcgacgtgcgcggctttgccgtcaagttctacacccgcgaaggcaattacgacctcgtgggcaacaacatgccggtgttcttcatccaggacgcgatgaagttccccgacctcatccacgccgtcaagcccgagccgcaccacgaaatgccgcaggccgcgagcgcgcacgacaccttctgggacttcgtctcgctgatgcccgagagcacccacatgctgatgtgggcgatgtcggaccgtgccattccgcgcagcctgcggatgatggaaggcttcggcgtgcacaccttccgcttcgtcaacaaccgcggcgagagccacttcgtgaagttccactggaagccgaagctcggcatccatggcctggcgtgggacgaagcgcagaagatcgcgggcaaggaccccgactttcaccgccgcgacctgtgggaggccatcgagcgcggcgactttcccgaatgggaactgggcgtgcagctcatcgcgccggacaaggcgcagtcgctcggcttcgacctgctggacccgaccaagctcattcccgaagagatggtgcccgtgcagcgcatcggccggctggtgctcaaccgcaaccccgacaacttctttgcggaaaccgagcaggtcgcgttccatccggggcacgtggtgcccggcatcgacttcagcaacgatccgctgctgcagggccgcctgttctcgtacaccgacacgcagatctcgcggctgggcggcgcgaactttcacgagctgcccatcaacaagagcgtgtgcccgttccacaatttccagcgcgacggcatgcaccgccagaccatctcgcgcggccaggtggcctacgagcccaattcgctcggcgacggcaaggagttcagggtcgacggcggcagcgtcggcttccaggcgtatcccgatgagaccggggggaccaaggtgcgccggcgcagccccacgttcgacgaccacttcacgcaggcgcggctgttcttcaacagccagagcgcagccgagaaggagcacatcgtggcggccttccgcttcgagctttcgaaggtggatgtgccggcgatccggcagcgcatggtcgacaacctcgcgcacgtcgacgagaagctcgcgcgccgcgtggccgagccgctgggcatcggtgcgcctgacgccaaggccgccgcgggccgcgcaggctttcgtgaacaccgcatgacattgccgatcgaggaatcgcccgcgctcagcatggccgacaccggcgacggctcgatccgcacgcgcaagatcgcgatcctggtggcggacggtatcgactccgcatcgctcaagccgatccgcgatgcgctcgagcaggccggcgcgcgctgcaaggtggtcggcccgcgcctgggcactgttgccagcgcatcgaagcggcagatcgacattgacatgacctttgccaacgcaccttcggtgatgttcgatgccgtgctggtgcccggcggcagcctgggcgccgcggcgctcgcgggcacgggcgatgccgtgcacttcgtgctcgaggcctacaagcattgcaaggccatctgcaccgtgggcgagggcgtgcggctgctgtcgacactgggcattgccgccgacacgccaccgggcagcctgcctcccggcgtggtggtggccgccaccccggtgaccaacctcggagacgccactgcggccacgcagatcgcgcaggacttcattgccgcgatcgccaagcatcgccattgggaccgcaccgacatcgattcggtccccgcatgaaatagtccttttgcgctagaccgtcttgcgaataggcggggcgcagggccgcttctagactttccccacgaggcctgaacggcgcgcacttccgcgacgtcgacccccgcaaccgcgggcacacgggccgcgcgcgggggtccaatgacgtggttttcgagaacgggatgggggcgctcggcacgtcgtgcaggagtcgcgggtgccctcgggctggctggcattcttctgctgggccatgggccgttggcatcggcacaacagcagcaggcgcccaacgccgaggccgcggccagcaaggccgaacaggcccggcttgaggacaccgacactttgctggcactgaccagcgagggcgcggtgctctacgggcaagacgccgtcaagctctccggctaccagtactgcagccaggcggtggccttggccgaggccggtgaattccgccagagcgtgcgcgccgcgagcaaggcgctgcacctggccaatgccacgcgcgatccgaacctcatggccatggccaaccgcgacctggccatcgtctacagctattcgggccagctcgacaaggccgaggagtttgcgcgcgaggcgctcaggcacccggcgcgcgaccccaagctggtggtcggcccggtgcagaaggtgatcggcgacgtgcgcacgcgccgcggcgactacgccggcgccgtgctcagctatgacgaagcgctggccaacagctcgccgcgctatgcgccgctggtgcaggcctcgctcgtcaatgcgctcatcgaatcgggcgatgccgcaagggcgcgcgagacgctcggcagcatggcgccgcccaaggatgcgccgctcaccgcgcagctcgaccgcacccgcgcgcggctgctgctggccgagaacaagccggccgaggcccgcgacctgtaccgcgcgctcaccgcgcgccaagtgggcaccgacaccgagtactaccgcctctgggcctgggacggcgtggcgcgcagcgaactcgcgctgggccagaagcaggccgcggccgaagccatggcgcgcgcgctgggcggcgtcgaccaggtgcgcgcgagattccgcagcgaagaattcaagatgggcctgttctcggacctgcaatcggtgttcgagcgcggcgtgtcgatctacagcgacgcgggcgatgcgcgccaggccttcgaagtgagcgagcgcagccgctcgcgcgcgctgctcgacgcggtgcgcggccgcgcgaagatcagcgaccgggccgcgaacatcgtcgacctggccacgctgcagggcgccctggcgcccgacgagcgcgtggtgcagttccattcgctgcccgaccggctgctggtgtgggtcgtgagcccctccggcatcgaggccaagaccgtggcggtgcgccgcgacgaactcaccgaactggtcgaggtgtttcgcaactcgatcgtgcgcggccgccgcaccgccatcaccaatgccgagaagctcggcgcggcgctgctcggcccgctcggcctcgtgccggggcagcggctcatcgtggtgccccatgggccgctgcactacctgccgttccaggcgctgcgcttgaacggccgctacgtcattgagcagcatccagtggccgtcgcaccgtcgatcagcatcgccgtgcagctggcgcagcgcacgccgcgcgtgagcgcatcgctcactgccttcggcaatccgcgcatcgaagacaagtacgacctgccgggcgccgagatcgaagtgaagcagctcgcgcaactgttcccgcgcaacaccgtgtacatgggcgccgcggccaccaagacgcagttccgcgacatgtccgcgcgttcgccgctgatgcacgtggcggcccatgccgaggccgacgcggtcgatccgctgtactcgcgcatcctgctggccaacgaaggcggcaagcagaactttctcgaggcgcacgaaatcctcggcctgccgatggacggcacggcgctggtcacgctctcggcctgcgagtcggggctggggcgcatcgcgcagggcgatgaggtgctgggcttcacgcgctcctttctttccgccggcagttcgagcctgattgcttcgctgtggcccgtgtcggacgacgcgaccgccgtgctcatgggcacgctctacggcgagctgtccaagggccgcgacatccagaaggcgatgcaggccggacagctggccgtgctgaaggatcccaagatgtcccatcccttcttctgggccccgttcaacctgatcggcaactggcgcctcacggtggggagttgacatgaaaaagcacccagaacacaagcaatccgcagcacaacacgcggtggagcactgagatgcgcgttcgccaacgatccacgcccattgcctttgcggtcactgccctggtgggggcaacgttgctggtcgcagcccagcgcgcgcacgcggccgagcccgaagtcaataccttgctgccgaccaaggacccatgcggcacctgcgaccgcccggtcgcccaggccacgggcactgtcgcgccgcaaagcctgcccgcgccgccgcaaccgcccgccgcctcgttcaagctcaacgacctgcgcctcaacggcgcgaaggcactgaccaacgaggaactgcagtcgatcaccgcgccctacatcggacgcaatgtcacgctcggcgatctcgaaagcctggcgcaagccatcaccgcgcgctacaaggagcgcggctactttctcgcgcaggccgtggtgccggtgcagaccgtgcgcgacggcgtcgtcgagatcagcgtcatcgaaggccggctcggcaaggtcgacgtgacggtagcgcccgatgcgcccctcagcgaggcgcgcgtgcgcggcttcctcgcgccgctgcggcctggcgaagccgtgagcgcaccggcttacgagcgctcgatgctgctgctgtcggaccagccgggcatcaaggtttcgtcggggctgcaggaaggcacgcagcctggcaccaccgatctttcggtcgaagtcgtcgcggcgccgcgctgggccttcacggccgaggccgacaaccacggcaccaaggaatcggggcgctttcgcgtcggcggcaccgcgcgctggctcagccccttcggcatcggcgacaacctcgacatgcgtgcgatggtgtccaacaacagcgggctgcaattcggccgcgtggcctatgaggcacccatcggcaccagcggcctgcgcgccggcctcgggctcgcgcgcgtcaactacgagcttggcggcgagttcgccgagctcggcgcgcagggcaaggcggacgtgctcgatttctcgctcaactacccgctcatccgccagcgccagcagaacctgttcctgcgcctgggtgccgacgtaaagaacctgaccgacgagatgaatgcggtcgatttcacctcgaagaagcgcgtgcacggctttggcctcggctgggcctgggagcggcgcgacgagatgttcggcggcggctactgggccagctcgggcacgctctaccgcggcgacctctcgatccgcgatgagcagagccgcgcgttcgaccagagcatcgcaggcaatcacaccgagggcggctacaccaagctgactttccagctctcgcggctgcaggccatcgtgccgaaccattcgctctatgtgtcggtcggcgggcaatgggccagcaaaaacctggatgcctccgagaagctctcgctgggcggtgcgcgcgcggtgcgcgcctacccgtccggggagttgctggtggacgagggcgcgatcggcatcgtcgaatggcgctggtccctcaactcggagctcacgcccttcgtgttctacgacgccgcgcgcggaaagatcgtgcgcgatccttcaccgttcgacacctccgccaaccgccacagcctgcggggtttcggcatcggcctctcatgggcccggcccggcaacttctcgatcagcgcgacgctcgcctggcgtgacggcacacggcccgcgcagaccgatggcggtggccgcaacccgcgtttgtacgtgcaggcgcaaaaggtgttctgacatggcaatgcacaaccgttccccacgattccaaccgcgcctgcagctgcgccccgtcgcgctcgcgctggtgtgcctgggcctggcgcccgcgctggcccagaccctgcccaccggtttctcggccattgccggaggcgtgaccaccgcgacgccaaacgccgcgacgatgaacatcaaccagacgacggcccgtgccatcgcgcagtggaacaccttctccatttcgacgggcgccacggtcaacgttgcgcagccgagcgccagcagcgtgctgctgaaccgcgtgatcggcggagaggcctcgaccattgccggatcgctcaacgcgaatggccgcgtcttcctggtcaacccggccggcgtgacgttctcgaagggttcgtcggtcagcgtcggcgggctggtcgcttcgacactggacatgtccaccagcaacgccgatttcatggccggtgcgtccaaacttgagttcaggcagccggacggcgcattcggcaccgtggacaaccagggcaacatcacgctggtgggcagcggcggcaccgcggcgctcatcggatcgcgggtattcaacagcggcagcatcattgccgacggcggcacggccgccatggcgtcgggcgagaccgtcacgctcgactttgccggcgacgggctcaccacgctgcgggtgacgccaggcctatacagcggcgtggcgaacagcggcaccatgcaggccaacggcggccgtgtggcgctggtggcgacgagcggctcggaagtgtcgaacggcgtggtcaatttccgcggcgtgctgcgagccgactccatggcttcgcgcaacggcgaaatcatcttggacagcggcctgtcgtccgagggcgtgcgcatgacgggcggcctggtgtccgcggcgggcaatggcgccggcctcacgggtggcaccatcgacatcaagggccgcgcgatcggtctggtgccttacacgcctccgctcatcatcgacgtttccgcgcccgtggagccaccgccaccgccgcccggaaacgacgaccgcggcgtcctcgacgcgagcggcagcgcgggcggcgggcgcatccgcctttatgcgaacgcggtgaccgaaatcggcgataccggcgcgatcgcgttcggcgccggttcgatcctgcgcgcagacgccgttgcatccggcagcggcggcgacgttcgcgtgctggccgagcgcaccctgcgtgccttcggcagcatctcggcgcgcggcggcgcgggcggcggaaacggcggcttcatcgaaacttccggtggtttcgccgcgcccgccgatgggctcggcggcggcttcagcatcgacgggctgcgcgtggacgccgccgcgcctgccggcaccgcgggcacctggctcatcgacccgttcaatgtcgacatcgttcccggtgccgcggccggcacgctgccgaccaaccccttcgaaccgctcgcggccagcacgatccaggacggcgacatcaatgcggccctgaacggcggcaccagcgtgcgcatcacgactggcgatcccggggcgggttcgcccacggatggcgacatccggatgttcaacggcgtgcgcatcaactacagcaccgccaacggtccgttgaccttccagctcgacgcccaccgcagcgtgcgcggcgacgccaacgtggtgatcgagtcctcgggcgccggcgggccgctcgacgtggtgttcaacaccgacgtcaacggcgggggtgccgcgaccggtggcggacaggtgagctacagcggcgacatctacaccaacggcggcaatgtggtgatgaacggcgcctggtcggcctcgggggcgggcccgagcgtgaacctcaacggcaacgtcatcgacacgcgcgtcggccgcaccgatgccggtgcgggcggctccgtgacgatcttcggcaacaccagcgggccatcgggcggcggcttcacggaagcggcggtcaacatcagcggcgtgcagatcgccacctcgaccggcaacgtcgacatcacgggcatcggcgccaacaccagtggcgtgcggctcggctcgcgcttcacggtcaccggctcgccgaaccggcagaccgacatctcgaccaccagcggcaacatcacgctgcgcggcatcggtaacttctcgggcaacagcagcgagaacccgggccatggcgtggtgctcaataacgcggtgcttcgctcggtcgacggcaacatcgcggtgcgcggcctgcgccaggccggcgcagccggtccgggcactggaggggacggagtgctgctgcgcaacggctcgcggatcgcgaccaccggcagcggcagcatcgagatcacgggccaggccgagggcaacggcgccggcgtgcggctcgggcccgtggcgcccgtgccgggcgtgttcccaacggtgctcgcgggcgtctccgtgtcttcggccggcggcaacgtcgtgctgcgcgccagcaacgacggcagcaccgatgcgctggtcatcgatggcaccgcgagcgcgggcaacgtcgtcaaccttcgtcccggcggcgtggctgccgacggcacggccttcgaccaggttgcgacgccgatcacgctcggcggcacggccagcacgggcttcgcggtgtcggccgacgagttctcccgcatctcggccggcaacgccgtggtggcgggcagcaatgcgcatgcggccgacatcaacgtcgtggggccgctcgccctggcctcgggcctcacgctgcagaatgggggcggcggcaacatcgcactgcaggcccccatcacggcgccgcgcgtgggcctggtgtcggccggcaacatcacgcagaccgcggcggcgccgatcacggccggcacgctgctggccctttccaccggcggcagcgtgctgctcgaccgggcggccaacaacgtgagcgcgaacacgctgggcgggggggcggcaggcgcgttccgctaccaggatgtggacgagctgcgcgtcggccccgtgtcgatcatcggctacgacgcggccggcaacgcgccgcaggtggtgtcggccggctcgatggccgcggacacggtgttcgtgcgcacgctgagcggcgacctgcaactcggcacggcggtgagcagcacctccggcaccgacctggttgccgcggcgcgcttccagaacgtgggtggtgccagcctgggcggcgcaccgtggcgggtgtgggccgacacctgggtcggtgaaacgcgcggcggcatcgccggctcgggcctgctgccgaatctctacaactgcgcctacctgggcctgtgcggcgtgaccgtgtcgccgggcgacaaccacttcatctatgcgcagcggccgaccgccaccgtcgtgatcggcaatgcgtcccgaccggccggcctgaacaacccgctcttcacctggagcatcacgggcctgatcctcggcgaccgcggcgccggcttcaacggtgcggtgggcaccgcggccacgcggtcgagcccgcccggcgcctatgcgatcaacggcagctttacctcggccgaaggctatctggtcaatgtggtgccgggaacgctcacggtcggcggctttccgcagattccgcaggtcgacgtgatccgcgaactgccgaccacctggctctacgaccgcaacatcggtccgccaccgatctgcttcgcgacgggcccgctggaaggcgaccgcgcttcgcagggcaacgacgtgctggcgcgcgaatggtcgcgcgtgcgctcgcggccgaatctcacgagttgcgtcgactccgagaagcgcaacggctgcgccgatttctaggggctagcccgcagcgccgaagcggcccgtgtaggtgcgcaggccctggtgcgccaggtcggactgcgcatcgatgtggaccttgccgcccagcgcctgccagcgacggcagaacgcatagtcctcgctcaggtagcggccattgccgggctcggccagcaggtcgaagaaccggtagtgcggccacgcttgcgccgcggcatcgcgcgacggctcgggcgtgtagcgcaggtcgggccgggcgtcggccaggcgctcgaacaccgagcgcgcgatcagcatgaagcccgtgggcgcatcgagcacctcgacgaaaccgtcgtcatcgattgcgcgcgcgccggtccatgcgttggccggaaagcgcgcatgccgagcctcgaagtcggcgcgcgtgctgcccgcgggcaaggcctcgcgcaggccaccggcgggccagccgtcctccttgagcggatagacaccggccaccacgtcgcggccggccagcagcagccgcaacgccgctgcgggctcgaagccgatgtcggcatcgatccagaacagatgcgtccagcgcgtgtcggccatgaactcggcgaccagccggttgcgtgcgcgcggaatcaggctgtcgccgtcgaggaagcgcgtctgcatcgaaaagccgtgggtccaggcgaggttcacgaggccgagcaggctgcgcacgtagatcgaggtcagcgcgccgttgtagtttggcgtggcgacgaagggccggatgtctttcagggcggcaaggtcgagcatcggtgatgagattcggtaggtgggcgttcaggccggtgtggccgcatgccgccgcgtggtgagcagtgcgcgcagcttggccggcgcgaccggcttggtcaacagcatcacgccgccatgccgcaggcgctgcagcacctcgggcccggtggcgccggagacgagcacggccagcgcgtcgggctgcagccgcttggcggcggtgatcacgtccatgccgtcgtcgtcgccggccagttgcaggtcgcacagcacggcatcgaaatgcaggtcgcccgtgcccagccgcgcgatggcctcggcgccggtggaaacgcattcgacctggcagccccattgctccagcagggcgcggctgccgtcgaggatgaccgggtcgtcgtcgatcaccatgcagtgcaggcctgcgaggggcgtgagcgccacgggcagcggcgcgggcgtggtggcctcgtcggcatgggccgcgggcacggtgagcgcaaaggtgctgccggcctgcagcgccgatcgcaccgtgatgcgggtgccgagcagcgcggcaatgcgcgcgcagatggccaggcccagcccgaagccgcggcggcggtcgcgctcggtgttggccacctggtagaactcctcgaagatccggccctggtggatgggcgcaatgcccacgccgttgtcgcgcacctcgatgcggacgttgtcgccgtccttgcggctgcgccgcgcggccaccagcacggtgccgcccgaaggggcatggcgcagcgcgttggccaccaggttgccgacgatgcgctgcagcagcgccgcgtcgctgcgcaccgcaaggccgcggtcgctccagcgcagccgcacgcgggtttccgacgcggtggccgcatgctgcgcatcgagctggtcgaacagcgcggccagcggcaccttggtgatcgtgggggtcagcacctgggcatcgaggcgggagatttcgagcaggtcgtcgagcagcacgcccatgaactcggtgctctcctgcaggcgcagcacggccgggcgctgcgcggggctggcgcccggcagcaggccgtcgataaaaagccccatggcatgcagcggctggcgcaggtcgtggctggctgcggccaggaaccgagcacgcgacagcgccgcctgttcggcctcggccatgcgctgcagcgccaccgccgtggcttcgcgcacgcgctcctcgctgatgcggcggttgctctgcagccgctcggccagccggtcgatgtcgcgcgcgagcaccgcgagttcgtgcgagtcgcccctgccggccaccggcggcgcgtggtgcgaatcgccctcgaccacgtcgcagcgcgcctcgaaatgcccggcctccagcgcggccaccgtgcgcgacacccgtcgcagcggccgtgccacggtgcgcgccatgtggcgcaccgaggcccaggccgcgagcagggcgaccagcgcaatgccgatgcccgccatgagggagcggctgcgctcgcgtgcataggcggtcgtgtcgcgaaaggtctgcaccagaccgatgggcgtttcacccgccgcggtggagcccgcgggcgcgaaggcgctggcgcgcgaggcttcgcgcagcgtgaccggcgaggtgaacatgcgcagctgcgcgagcgacgacgccttgggcccggccgtcacgaagacgccggcgctgttgctgatctcgacccgcatcacctgcccgccgcgcagcgcggcgttggccacgttctgcagcgccggcaggtcgccggcatagaggctcaggtcggacatggccgccacctggcgcgccacggcctggccctcggcgtcgaaggccgcctcgagcgtttgcagccggctgtgggtgaaccagccggtgagcgcgagcgccaccgcggcgcacggcaccacgccgagccggaacaggtcgcgctgcaggttgccgcgcaccatcagcttgggcgcggactgtggcggcggcgaggtgatgtcggcgcgcgtgccttcgggcggcagcttgtcgctcatcgcgtgacggtgagccgctcggccagttcccgctcctccggcaagcgcagtccgagtccgcgcgccacggtggcgttgacgcgcacggcggcgggcgtggccgactccaccagcggactcgcgccgccgccgctgctggcgagcttctgcccgagcagccgcgcctgctgcgccagctgcgcgggcgtcgacaccgccgcggcaagcccgcccgagcgcaccagcccttcgctggcgccgaacaccggcaggcccgcctccgcgccggcgcgcagcaccgagagcgtggcggcctggctgtcgccgatcaggtcgggcagcaccatcagcgcatcgctgcgcggcaccaccgcgcgcagcgatgcggccagcgatttggcgtcgggcgcgtattcgacctgcacgtcccacggcgggctgccgccctgcgcggcgcgctgcagctcgcgcaccagcggctccgattcgggcgtggcgaccacgccgatgcgctgcttctgcggcagcaccgcgcccaccagggcgagctggtcggccatggccgggtcgcgcagcagcacgcccacgcgacggtcgccacggcgcagcgcggggctggtggcgcgcaggttctcgtagtcgagccggctcagcatggcgagcaccagcggctgctggcccggccgttcgagcgcggcgcgcgcggccggcatgccgaccgccatcgtgaggttggcgtccgacgccagcgcgcgcaggctgcgcgtgcgcacgccggcgttgacgctggcattggcgctgcgctcgggttcggtgctggccgtctccgtggcttgcggcgtgtccgcgccgcccggcgaaagccgcaccaggtcgaagcgggacccgggctcctggcccgcgcgaagatactgaacgaactccgagtgcgccgcgagctcgtcccccatcaacaccgtgagagcggcggccggggtgtgggcggcgagcagcgccgcgcccatggcgagcgcgatgcgggcgccgcggtgcagccgtttccggaagagcgagatgaaagggttcacggcgacaaacatggactgcctctgcagcaaggggcagtacccaatgtacggaagccctctgcttcgcgcgataaggcggagggcttatgtcggcacccgccaccgcttgccagcgtgacgaagtgcacagtgcggcagctgcttggcctatgtccgatggactagggccccgcgaaggggcctcaggcgtcggcgctcagcagtgcaaccgcgcgttgcgcctggatcgcctggcgcagcacgcgcggcgaaaccggcttgtagagcaccgcgatgccggcgctcgccacttcgcgcagccggtcgggcttggtctcgcccgtgaccagcaggcgcgccgtgcccgggccgatgccgcgcgggtggcgctcgagcgcggcgatcacgtcgagcccgttgtcgcccccttgcagcagcaggtcgctcaccaccacgtcgggcggctgctcccacgcatcggccagcgccagcgcttctgcgcgtgtctgcgccgccatgacctcggcgccccagttggtcaggaccacggtgaggccttcgagaatggtgcgctcgtcgtcgatcacgaggatgcgcagctgctcgaggctggcctcctcctcgatggcgccgatggcgggcgtggcatcgagcgccggcagcgcggcgggtgccgaacgcaccaccacgcgcacgcaggttcccttgtgcggcctggaggtcagctccacgcgggtgttgagcaggtcggccaggcgttgcacggtggccagccccaggcccatgccgcgctgcccacggggcgcctggcggccggtgctttccacttgatagaactcttcgaacacccgtgcctggtgctgcaccgcgatgcccacgccggtgtcgaccacgtcgatgcgcacgccccggccgcgccgccgggcgccgatcagcacgccgccctcgatggtgtggcgcagcgagttcgacaccaggttgttgagaatgcgcgagagcatcacgtagtcgcagcgcacccagaggtcggtcttgcgcgccaccaggcgcaggccctgctgctcggccaccggccggaagttgcggctgatctcgtcgaacagctgatccagcggaaagtccgcccactgcggctgcagcacgccggcatcgagttgcgagaggttgagcagttccgagaacagccggtcgagcgaatccacgcattcgcggatgtggccgatgcgctgcaggcgcacggggtcggtctcgccgttggccaggccgtcggagaacagcgtgagcgcgtgcagcggctggcgcaggtcatggctggccgcggccagcaggcgggtcttggcctggctcgcgacttcgagctgctggttcttgcgcgccagttcggccgtggcctcgctgatgcggctttgcagcagccggtggctttcggccagcgcgcgcgccgcctggttgaagccatgctgcagatgtcggacttcggaggtgccctcgatggccacgctcgcggcctcgcccgcgcccaggcggtcgacggccttgcccagcgcgcggatcggctcgctgatgcgccgcgccgcccaccagcccgccagccccacgcccaccaggctgacggccagcaccagcaccacgttgagccacaccgagcgccgtgcgtgctgcacggcgtccaggctcatctcgaccatcaccttgccgctctgcttgccctcttcgctcacgatcggcaccaccacctgcaggccttcgccgcgagcgcggtcgaccgtttcggagttggccacgatctcgccgtcgtccgaccagatctgcacctgctgcacgtgcggctggtaggtacccgactgggccgtgcgctgcaggatgcggcggtccatgcgcaccagcggggcctgggccgccgtggcgacctgcagtgccaccgtctgggcattggcgcgcatcagctcggtcaggttgtccaggtgctggcgcgtcagaacggcaatggccgccagcgtggccgcggtggcaggcaccagcgcgagcaggatcagctgctgcgcgaacgtgaggcgggcgagccctcgcaggacgtggaagttccagttcatgagggcattggaagcatggctgtcaagcttaggggactggctgcgctagcgaaatatgggaaaaacatcacgaaaataacccgtacttggtatctaattgcgtcgctttacggatgttagacccgctggtccgcagcggccccctgtctacgtgtcaaaaaatgcaggcctccttatgcagcgtccggaaggcttccggcactcctgacgcgtttcgcgccacccgccgttgcgcgcgattctggcgtgccgccgccgtggtgcgaagaggcgccgccctgttgacgctgctcgccgtgctgcccctggtatctctgccggcagcggcccagcctgcgctcctgcccgatgcgccggtgcgcttcggcatcctgccgctcggcggcgccttcgaatcgcgcagcgactgggatcccctcctggccgaattgagccgcgccattgcacggcccgtgagcgtgctgtcggtcaactcgtacgaagcgctcgagcaggccattcagcgcgacgaggtcgacatggcgttcctgtccgggaagatggcgctggacgccgtcacccagcgccgcatgaaggtggtggcgcaggtggtgcggcacgacgggctgcccggctaccgcgcgttgctgctgacccgcaagacgccgccgttcaacaccaagaaaagtctgctcgcggagccggaacgctggcgcctcgcgcgcggggagcggcagtcggtgtcgggcttcatcgtgccgcagctgcagttctttttgcccaaccacatcgcgatggagacgcgcttcctgagcgagatcgtgggcacccaccagacgacggcgctggccgtggccaacaacgaagccgacgtggccaccaacaacacggccgatttcgagcgcttcaagcagcgctttccggccgaggcccagcggctggaggtgctgtgggaatccgagctcattccgcatgcgcagatcgtggtgcggcgcgaatacccgcccgagttgcgcagccgggtgcaggccttcctgatcggctacgggcgcgccaagggcccgcgcggcgacggcgaacgcctggtgctcaagtcgctgcacgacctggccggtttcgtggccgcggacaacagttcgctgcagcccgccgccaagctcgcctaccagctggccaagcaaaacgccatgaccgcgcagtgggtcaacgacgcggcgcgacaggcgcgtttgcagcgcatcgaaaccagctacgcggagcaggtcaccgtcttgcgggatctgtcgccctgatgttgcccatggcgttttcgcgcgtcctccgcctgtttgcggtggcgacggcgctggccgccgcggccgccggttctctggcgcagggcggcgcagtgggcgctcacaaggcggcgccggtcgcgtcgatccgcttcggcgtgctgccgctgggcggcaccgtcgaatcgcgcgccttgtggatgccgctgatggccgacttgagccaggccatcggcgtacccgtgagcgcctattcggtggcgtcttacgaagagctcgaccgcgccatcaagcgcgacgagatcgacatggcttttctgtcggccaagatggcgctcgacgccgtgatgcagcagcgcatgaaagtggtggcgcaaatcgcgcgccgccccggcatgccgatgcaccgcgcggtgctgctgacgcgcaaggccggcgtgcccaacacgctggaagccgtgctggccgaacccgagcgctggcggctggcgcgcggcgacagccgttcggtgaccggattcctcgttccgcaaagccagctcttcctgccccgcaacatcgaactggagacgcgtttccgtggcgaggtcgtcggcaaccaccaggccaccgcgctcgccgtggccaatggcgacgccgacgtggccaccaacaacacgacggacttcgagcgcttcagggagcagttcccggtcgaggccgcgcggcttcacgtcgtctgggagtccgagccgccgcccggtgcgcagatggtggtgcggcgcgcctatccgcccgagttccaggcccggctgcaagccttcctggtcggctatggccagggcaagggcccgcgcggagacgccgagcgcgaggtgctcaagacgctgcgcgcggcctacggttatgccccggccgacgacagcgcgctgctgcccgaggcattgctcgaatacgagctcggcaaacagcgcgccatggccgccgcgtgggtcaacgaggcggcgcgcgagcagcggctgcggcgcgtcgagcagacctataaggaacaggtcgaggcattgcgcgcggcttctaccgccccgcgctgagcaaggcgcacggcgcttggctggatatctccgttgacagcatcggacttatcgggatctggaacctactcgcgccaatgaacgattgatcgtgatcgtgatcgtgaaatccatccgcgcaacgcggctggttaggcaggcgatgagatcgtgcagcgtcttctcggatgtacgcttgatcgtcacacatccatcaataaaacagccgcgcaaatgagcgcggaaagggaaattcatgatctggacacattcaattccccagcctcctgtgccgcagttcctgcgcgagacgctcaaggactatccggagctgattcaggaaattcaggatgttcttaccaaggtcgtcatggacggccctgcctcgattccgccctttgaatgggccatctggcgcctcgaagacaccctcagcgccctctattccgacgcctacgaagccctcaaggaggccgagcaaaccggcgattcgcaggcaatctatcgggccaagatcaagtacgacgcgctggtagtcgcaggccgcccccggagcctccccgaattgcgggactacttcgagacctataagggggcgttcgaatgagcgaccccaccggcaaactcgatcccgaaacccatcgccgtgtcttcgcggaacgtgttgtacccagaagcgctctgcctgaaacaacacctcaagcacgccctcacgccatcgttctggcgggccagcccggcgccggcaagggcaatcttgtcaaggctgcgcagtttgagttctccgacaacatcgtccccatcgacccggatgcccagcgcgaactccatcccgacttcaagaagcttcgcgaagcccatccctacacctggtcgggccacacgcactacgacgcgagccgctgggccggtgaactgcgcgatgctgccgtcgcgggacggcgcaacctgatcgttgacaccacattgggcaatgcagacggcgccatccagaccatcaaaggattgcaggccaagggctacagcgtcgaggtgcgcgttgttgccacgcaccggctggagagcgaactgggtgttgatcggcgcttcacagaatcactcgaccagaaaggctacggccgccacgttcctggcgagtttcatgatgccgcctacaaggcactgccagccaacctcgacaaggtgcaggagcaaaccggcgcgcgcattcgcatctacaaccgggaaggcgcgcagctgtacgacagccacaccagccctctgaagcccggtgctgctttggagcaggcgcgcgaggcccgcatggccgaccccaagatcacgcgcgacacagcaaaggacgctcgcacccagcaggacttccatagaaggttgcccgacaccctcgaacgcaaccccaagatcaacttggagacagcgaagaacctcccgcccgagcgccaggcgcagggtgtggcgccaagagtagagcgcgtcgccaccgaaaccgccgcggtcgaccgcagcgttcgcatcgagcccggcgctgcacgtgttgcactcggcctgaaggtcttcggcaccgccgctctggcccacgacgccgtcaccaccggccaagacaccaagaacctgctcgaccagaacaatctcaccggtgcccagtcgcaggtgatgcacttcgcgggccgcaacctcggcatggccggtggcgccatggccgtgggttcggcagcagcggcagccggcatcgagaccggccccggggccctggtcgcaggcttggccggcggcttcgtgggcgccgtggccggcgacaagatcatggatgtggtggatcgcgcccgcatctacaaccagcgcggcagcgacggcaacgactggaacctcgaccccagccagcccgcgcagggctggacccgtctgccccggcccggtgagttcggccctcagggacctcctgagggtgcaggctacaggaaccacctgctgcacgccgcgccccgcttggccgacgagctgaactacaaggccagcagcaccgccgtcgaactggcgctggcccacccgcccgcaccccaagacccgttcaggcaagcgcccgagagcatcggcgaaacggtgcgccccggcatcggcgccggccagccgtggacacgcgatccgcaaagccatgcctggacgcggcagaccgccgaagcgcccacgcccatgacccacggcatgccggttcagcgcacggtcacggccagcccggagcagggccggcaactggacgcagcggcacagcgcgtcatcgcggacaacatcgtccacagcccacaagccatcgcgcagcgctatctggacgcctacgctcagtatggatggaaacaacacggcccggtgccggccgccttcacccacgccgcccaaggccatgcgcgcgaggagcccaatgccacacgccagcagatgcccacaccgcctcagcccacgagcggccatctgacacctcagcagatcgaacgcatcaccacgcacgaacagcgcgtgacacgcacgcccggcggcatgagctttgccgaggcgcacaagcgccgcgacgaacccgagcagatttctcagggctcattgcagccggtgggtaagctcgatgcgacccaccacgccaaaggcagcccgctgtaccggatgcaccaggcgcaggagcaggacctgatgcgtggcctgggcatcgcgcaggcgcaggacagggagcggttcaggaacgagccgagccctcaaaggacgctgcagccttcggtggaacgcacgcaggaccgtacgcacaggcatctgctggaggaggcgccggtgcagagacagcccgcgccgcctgtccccgccatacagactccgcccccaacccgaggggagcatgcgatggcgcctgtggcacaggatcatgccaaccctgtgcggcctgcccctgccgaacggcgagccgccacgcccacacatgcccagccgatggccccatccactgccgcagacattgcggcggcgcaagcccaggtggccgcggcgcaggccgaattggctgaaatgcgggagcagatggcacgcatggccggccagcgcgggcaaagcggcctggagcggcgcgatgagagcgaccagaggcaggccgcgcaacctcccgcggccgcttctcgccctgagcttcggatcgaccaccccggccacccgggctacgaactgttccagcaggcccgggaacacatgcgcgcgctcgatgccaggatgggccgctcctccgaccagcgcacggacaacatggccgcgtgcctggcggtgcaggcctgccgcagcggcttggagcgcatcgatggcgtggacatcggcaccagtggcaaggacgtctggatggcgcaggggccgctgggcacggtgtggatgaaggtggcgggcgtgccggtggagagtgccgatgtttcggtgcagcagacgagccagggatgggcgcaggcgcagcagttcgtgcaacagcagcaggctgacaaacaccaggagcagcaggagcaccagcgggcgcagcaacaggggaacgagcatctagtcccttcgcggtagctccaaatgccccgcctaggccgttaggcggatttgccgccggccctctgcgccggaaactccgtgcttctttcgggcagcccttgcctttgacggagtgcggatgagttggcgaacaaaagtggtctggagcgaggggatgctgctgcagccccagcacctgcagcagagcgagcgtcatggcgaccatgcgcggcatgtgctgttgcgttccaccacgccttatgcctggggcttcgcggagatcgagatcgatcaggccgcgctcacgctgggcaagctggcactggtgcgcgcggtgggcatcttcggcgacggcaccgtgttcgacatgccggcggtcgatccgctgcccgagcccatcgacattccgcccaccatgcgtgacgaggccgtgatgctggcgctgccgctgcgccgcgccggtgcccgcgaggccgatgccgaggaatacgaagagctggtgcgccaccgcgtgctcgagtccgaagtgcccgactccaacaccgccggcgagcgcaccgccatgctgcaactgggccagcttcatacgcgcctgatgcgcgccagcgaagcgaccgacgcgtggaccaccctgggcgtggcccgcgtggtcgagcgccgggtcgacaaccaggtgcagctcgaccgcgccatgctgccgccgctgctcgacgtggcgggccatgccgtgatccgggcctggctcgacgagctgctgggcctcatgcgccagcgcggcgaggcgctggccggtcgcatgacgcagggtggcaccggcggcgtggccgagatcgccgacttcatgctgctgcagacggtcaaccgcaatgaagcgatctttgcgcacctggccaagagcgccatgctgcacccgcagcatttcttcgagcatgcgctcgggctggcgggcgatctcgcgagctttcgcgattcgcgccgcgtggcgcgctttggcccctacatccacgacgacctggcgctgagcttccgtccactgatggacgacctgcggcgcagcctctcgatggtgctggagcagtcggccatccgcatcgacctgcatgaccgcaagcacggcgtgcgcgtggcggtggtcaccgacgtcgagctgcagcgcaaggccaccttcgtgctcgcggtgaacgccaacatgccgagcgaagcgctgcgcgcgcgctttcccacgcaagtcaagatcggcccggtcgagcgcatccgcgacctggtcaacctggcgctcccgggcgtcacgctcacgcccatgccagtggcgccgcgccagatccctttccacaccggtgccaactacttcgagctcgaaacgcgcaacagcgacctgtggcgccagctggagcaatcgggcggcatcgcgatgcatatcgcgggcgactttcccggcctcgacctcgcgttctgggccattcgttcctagccgcaccgggctgacggaaacggaacaccatcatgaccacaccagaccccttcgccgcttttgagtcggagcgcacggtcatcaagcccaagccgcgcacgccggcgggtacgccgccgcccgctgccgcgcctgcgcctttcttcggcggcgcggatccgacgcccgcggtggagctcggcgagatcggcctgctcaatccgctggtgtcggcggccggcaagctgctggtgctgatcggcaagctgcgcaacctcgtgcagccgcccaacgtgccagccctgcgcgcctccaccgccgaagcggtgaaccagttcgatgccgccgcgcgtcgcgcgggcgtgagcaacgagtcggtgctggccgcgcgctacgtgctgtgcaccgcactggatgaagccgtggccaacacaccctggggcgtgcaggccggctggaacaagcagagcctgctggtgcagttccacaacgagacctggggcggcgagaaggtgttccagctgctcgccaagctcgcgcaggacgtgcccacgcaccggcagctgctggagctgatctacagcgtgctcgcgctcggcttcgagggccgctaccgcgtggtcgacaacggtcgcgcgcagctcgactcggtgcgccagcgcctggccgacctcattgcgaaggaccgcccgccgctcgaagccgagctttcgccgcattggcgcgggcagggcgccggcacggtgcggctgcgcgaatcgctgccgctgtgggtgttcgcggccggcttcgcgctgctgctggcattggcgtggttcggcctgcggctcacgctcaattaccgctccgacaccacctatgccgccgtgttgggcctgcgcgtgcccaacctccagatcgcgccgcccgccgcgccggccaagacgccgcggcttgcgcgctttctcgagcccgagatcaagcagggcctggtcaccgtgaccgacgaggccgaccgcagcgtggtgcgcctgcgcggcgattccttcttcggctccggcagcgccgagccgatggcggcttcgctgccggtgctgcgccgcatcggccaggcgctggctgaagtaaagggcgaggtgctgatcaccggccactccgacaaccagccgatccgttcgctgcgctatccgtccaactggcatctgtcggccgcgcgcgccgatgcggtgaagggcgcgctcaccacgctggtcgacccggcgcgcatgcgctccgacggcaaggccgacgccgaacccgtggccgccaacgacacgccggccaaccgcgcgcgcaaccggcgcgtcgacatcgttctgttgtccgagccggaccgggtcgctgcggcgggagtgacgaaatgatcaagaaaatcttcggcttcctgttcagcccggtgctgctgaccatcctcgcgctggtcatcgttgcgctgctgatctggtggatcggcccgctggtgaagatcggcgcatgggcgccgctcgaaagcgagcttgcgcgcgcgctgctgatcggcgccatcgtgctcatcgtggtgctgcgcgcgctctaccgccggtggcgcgcgcgccgtgcgagccagcacctgaccgacggcctcatgaaggcgcctgccgccaagaccgatgcgccggtcaacggcgagcagaagatcctcgacacgcgcttcagcgacgccgtggccacactcaagcagatgcgcctgcatgcggccggcaagaagcccggctggcgcgattggctttccatttccggcggcagctacctgtacgacctgccgtggtacgtcttcatcggcgcgcccggcgcgggcaagaccacggcgctggtcaactcgggcctttcgtttccgctggccgagaagttcggccccggcgccatccgcggcgtgggcggcacgcgcaactgcgactggtggttcaccgacgaggccgtgctcatcgacaccgccggccgctacaccacgcaggacagccaccaatcggaagacaagagcgcatgggaaggcttcctcggcctcttgaagaaagcgcgcccgcgccgcccgctgaacggcgtgttcctgaccgtgagcgtggccgacctgctgagccagggccccgagcagcgcacgcagctggcggcgtcgatccgagcgcgactgctcgagctcgatgcgaagctcaccacgcggctgccggtgtatgtgctcgtcaccaagagcgatctgctgtacggcttcaccgactacttcgacgacctcggaaaggagcagcgcgcgcaggtgttcggcttcacgctgccggccgacgagaacgtgcaggccgacgacaagggcctttccaccgccttcaaccgcgagttcgcgctgctgcacaaccgcgtcaacgacgggctcattgcccgcatgcagcgcgagaccgatggcacgcgccgcgcggcgatcttcggctttccggcgcagttcggttccatcggctcgatgctgtccgacctgctcgaccaggtttttaccggctcgcgctttgcgcagccgccgtgggtgcgcggcgtgtacttcaccagcggcacgcaggaaggcagcccgatcgaccgcgtgatgggcagcctcgcgcgcagcttcggcctggagcgcgccatgctggcgccgcagaagtcgagcggccgcagctactttctcaccgcgctgctgcgcgaggtggtgtttcccgagcagcgcctggccggcgccaacgtgaagctggaacgccggcgccacacgctgcgcatggccggcgtggcggccatgacgctggtcacgctcgcgctgctcgcgagctggggctacagcacgctgcagaacgtcaactacctgaagtcggtcgaggcgcgtgtcgagcccgcgcgccagaacctcgcggctctgccttcgcgggtgcagaacctggtcgaggtggcgccggtgctgcagggcctgcgcgacatctggaagacgcccgacaaccgccagggcaacgagccgctgtcgatgacgctcggcctctaccagggcgacaagctcgatgcggccgccatgctcacgcaccagcgcgcgctcaacgatgccttcctgccgcagattgccaagcgcatcgaagaccagctgcgcaccgcgcagaaggacaacctcgaatacacgtacgaggcgctcaagagctacctgatgctctaccagcccgagcacttcgatgccgaggcgctcaaggcctggatcacgctcgactgggcgcgcagcctggaccgcggcattcccgaagaccagcgccaggcgctcgaagaccagctcgacgtgctcatcgcccaaggcccgccgcgctcgccgctcaagatggacgagaacctggtgcgcagcgtgcgcgccgtgctcgcgagctatccgctggagcagcgcgtgttcagccgcctcaaacgccagcgcgccaccaaggacattccggggttcagcatcgccaccgccgcgggcccctcggcgccgctggtgttcgagcgcatcagcggcaagccgctgaccgaaggcgtgccgggcatgtttacctacgacggataccacaagcgcttccagaacgaggtgacggtgctcaccggcctgctcgcgcaggaagacccgtgggtgctcgggcaagaccgcggcgccgccgaccgcatgcgcgacgtggccgcccttggcgcgctgaccgaccgcgtgcgccggctctacctggcggaatacgtcaaggtgtgggagacgctgctggccgacgtgcggctgatccgcgccagcgggctcgagaagaacatcgaggccgcgcgcattctctcgggcgtgggctctccgcttgcgaactttctgcgtgcggtggtgaaggaaaccacgctcattccggccgaccagcccaaggacgtggtgagcaaggccaccgcgacggtcgccaacacccgcaagggcctggaagacctgttcggcggcgatccgaacaaggcggtggccagcggcaagcgcatcgagagcatcgtggacgaccgcttcgaaccgctgcgccgcctggtcacgcccgttgcgccgaaccagcctgcgcccatcgatgacgcgctcaagctcttcaacgaggtgtacgtgtacctcaacgccgtcgacacggccgtgaagggccgcacctcgccgccgcccggcgacgtggccggcaagctcaagtccgacgcgggccgcttgcccgagccggtgcgcacgatggtcgagaacctgagccagtcgggcgccgcgcaggcccaggtggccgagcgcggcaacctgagccaggacctgcgccccgtgaccgagttctgcaaccgcgccatcgcaggccgctaccccttcgtgggcagcagcaagcgcgacgtgctgcccgaagacttcggccagatgttcggcgccggcggcctgatggacgatttcttccagaagcggctggccgcattggtcgacaccagcaccaagccgtggcgctacaagcccgtggccgagcgcggcgccgtcaccacgcaggcgctggcgcagttcgagcgtgccgcgcgcatcaaggacatcttcttccgcggcggcggccgcggcccttcgatgcggctggacttcaagccggtggagatggatgcgggcatcacgcaattcattctggacgtggacggccaactggtgaagtacgcgcacggccccgtggtgcccatggccgtgcagtggcccggcccgaagggcagcaaccaggtacgtatccaggtgagcccgccttcgaccaccggcagttcggggtcggcagtcgatgggccgtgggcgctgttccgcgcgctcgacgacggccagctcgaagccggcgatgcacccgaaaaattcttcatcactttccaggtcggtccgcgcaagacgcgcttcgaggtgacgacgaacagcgtgcagcatccgatccgtttgaaggaactgcgcgagttctcctgtccggaggggttgtgacttcttctccagatgcgctgccggggtggttcggcaagttgccgggcatgggggactttgcgcatcggcgcttgcctgagtcgtttcgttccgtgtgggaccagtggctgcagcgtggtttggcgcggttgaaggatcgtcatgctgactggactgcgcactacctggaggcgccgatctggtgttttgctttggggccgcaggttgccggcgagggggcgtggattggtgtgttgatgccttcggtggatggggtggggcggtactttccgttcactatcgctgtcgagctgaatgcttctgcgggagaggtgctgcggggggatgcgctgcaagttgcgttgcgctggtggtcgcgcgggactctggctgcgctcgaagggcttgagggggatctggatgcgctgcggttcgatgctgtgcttgagcggttgtttgttgctgctgctgctgccggtgacgtgcacgttggtgcggtggagtctttggtgttgccgggggctgggggttcgttgtggatgagtgatccgggcgctgatgggactgctcgaatggtggttgccgggttgcctttggatgggcagttcgaggctttgtttgttgggggtggggaatgaagtccttgctttcttttgttgtccgaggccgggtctcgccccggcgggcgactcactttctttgcttcgccaaagaaagtaagcaaagaaaggcgacccctactgtctgcgtcccttcgcttcgctacgggcaacctgcggtgctcgactccggcgggggtccgcagaactcgcttcgctcaaacagctgcggccctgatcccgcctccatctgcgctcctcggcgcatacagaaggggtgggagcgggcagccttcgctctcgctcggccccaatacaaaactcaattcgataccaaccaccgcaggcgctacgcgcctgcggtggcttggtggccgagcgaagcaaaggcccgttcggtctccaagcccctctgtatgcgccgaggagcgcagggtttcgcggatcagggctcgcagctgtttgagcgaagcgagttctgcgagaccccgcgaaacccgagcaccgcaggttgcccgcagcgcagcgaagggtcgcagacagtggggtcgccttttctttgcttactttcttttggcgaagcaaaagaaagtgagtcgcccgccggggcgacacccggcctcggaaatcaagcacccgtcgacgttcaaacgggagccagccaatgaccgaagaaaacacgccccccgaagacgaccgcacacaggtcatgtcaaggccagcccaacaacccgcgggcaacgaacaagacacctcggccaccgtcatcacggccaagccgacaaccttgtccaacgccccggtcaccggccccgccacggaagccaacgaagccggcctcctccccgtaggcagccgcctagcagaattcgaaatcacccgcgtcgtaggccaaggcggcttcggcgtcgtctacgaagcctgggaccacaccctcgagcgcgtcgtcgccatcaaggaatacctgccgacttcgctgtcgaccaggcagcaggacggaacagtggtccccctgtctgagcgacacagggaaaccttcgacctcggcatgcgcagcttcatcaacgaagcccgcctgctcgcgcagttcgaccatgcctcgctgctgaaggtctaccgtttctggcaggagcgcggcaccacctacatggtgatgccgttctaccgcggcgacacgctgcgccaggcgctggtgtccattcccgcgggtgtggacgaggcgtggctgatccgcatcatggacggcgtgacgcaggcgctggcggtgatgcacagcgccaactgctaccaccgcgacatcgcgccggacaacatcatcctgctcgaaggttccggccggccggtggtgctcgacttcggggccgcgcgccgcgtgatcaccgacaagacgcaggcgatcaccgtcatcctgaagcccggctacgcgcccatcgagcagtacgccgaaatgcccgacatgtcgcagggcgcatggaccgacgtctacgcactggcggcggtgatgcacgtggccgtgtgcggccgcgcgccgccgccttcggtggcgcggctgttgtccgacagctatgtgccgctggcgggcaacgagatcctgcgccagcgctacagcctgcggctcctgcaggccatcgacgcgggcctgggcgtgcggcccgagtcgcggccgcagtcgatggccgagtttcgcgccgcgctcgacctggaggtgggccacagcatcgcgccgacgccgcggaccacgccgccgggctcgggcgctcgcaccaacagcaacgccgacctgccgacgaccatcggccgcggcaaggcgatacccgcgcctgcacccgctccaggcgcgggtgccggtgcgaacgcaaagaacggcaaggccgtggccgcgatcgcctcggtggccgtgctcgccgctgtggcgggtggtggctggtggtggtaccagggccgcaccgcgggcgcggagggcgatggcggcaagcaggtggcagttgcaacaccgccgccgcccgagccccgtgtgacccaggcgcccccaccgccgcctcccccgcctccgcccacgccccgtacgccgctcgaatccctgcagtcgctcgcggccggcgcggcgccgggattcgacgtgacggccacgccgaagaagcccgaagtggcgataggcaaggacaagctggccttcgaggtccgcagcaagcgcgagggtttcgtctacgtgttcctgctgtccagcggcggcgagatgttcctgctgttccccaacctgctcgacaagtacaacaagatcaccgcgaacagcccgctgtcgctgccgcgcgcctcatggccgatggatgccggcggaccggccggcaccaaccagttcgcggtgctcgtcagccagcacgagcgcgacttcagcgcctcgggcatgcagaacgacggcgtgtttccgcagtttccgctgcccgtgctggcggcgctcgaagccagccgcggcacagggccgtcgcccttgctgggcaagcccgcttgcgcgcccagcaccccatgcaacgacgtctacggcgtcgcgaatttcaaaatcgtcgagaagtaatcgtctgtagagcgttggcccgctgggccgtcttttcggacaaggaggctttcatgtacacgcagtcgccgattttcatttccgcccttcgctgggttgccgccgccgcggccgtgcttgccgcgggctgcgccaacacgccgcctgcagccaatgccaacgccaacgtcaatcccaacgcaggcaccgctgcgcccgacactacggcggcatcggccggcacgccacggccggcctccaccgggtcgagcgtggccggccaggcgcgcaccttctcgacccagctggccacctacacctcggtcagcttcgatgccgtgccgggctgggcgcgcgacgatttctccgagagctggcccgccttcctcggcagctgcaaggtgctcaccggccgcggcgcggagtggaaggacgtgtgcgcgcgggctcttcgggtcgacagcaagaacagcaccgccattcgcgccttcttcgagcaggagttctcggcctaccagatccgcgatgacgaccgcaagcccgacggcgtggtcaccggttacttcgagcccgagatcccgggcagccggcagtacgcggcgccgtacatctatccggtctacggccagcccgaagacatgctgtttgccgacgtgcgcaagctgccggccggcagcggcaccgtggcggcgcgtgtggaaggccgcaacgtggtggtgcagaccggcctcagcacgcgcgacatgggcgcgccgggcctctatgcgctcgacctctcggccctcacgcgcgacacgctcgaccgcaaggtccgcctgcgcatcgagggcaagcagctgctgccctactacacgcgcgaagagatcgagaccaagggcgcgcccaatgccaaggtgctggccttcgtgagcagcgccaccgcgctctacgaaatgcagatccagggctcgggccgcatcaagctggccaacggcgacatcattcgcgtggcctatgccgagcagaacggccagcccttccgtcccaccctggcgcaggcggccaacggaaagccgcgcacgccggtcaaggtgcgcggttcgtccatcgagctgcagctcgacgacggcgacgaggacgacgacgtgggcggcacctcgaccagcaccatccgcacgcgcggcttcacgctcgcacggcccgtcgccagcggcgcggtcgtggtgccggggcggcgcgcggccggtccggtcatcggctccggcatccaggacccgagctacgtgttcttcaaggagtcgacgtcgccttcgggcgggccggtgggtgcgttcggcgtgccgctttcggcgggccgctcgatcgcggtggacccgcgcagcacgccgctcggctacccggtgttcgtctccacccgcgcgcccggcaccggcgcgcccatgcagcggctgaccattgcgcaggacaccggcggcgcgattcgcggcgcggtgcgggccgactatttcttcggcaacggccagcaggccgccaccaacgcgcgccgcatgaaggagcgcggccagctctggatcctgctgccgcgcggcctggccgtggcctccgcggcggtgtcctcggccatccgcacgcgcggcggcccggtgggcgccggcctgccgcaatgcctggtgccgaccgaaggcgtgtgcgtggacgactagtccgatcgctcccgatcgcctggttcgcttcgccatgcaagaaaccctttcgtccgcggaaagcactgcgctcgtccgcctctggcggcgccggcagacgctgtccccggacgacatgggcaccatgtaccgcatcgtcggcgatgcgctcgtggcctgcaatccgcccgagctccaggtgctgggcgagggccggcaggagctggtggcgcagttcatctatgtgaaggtgctgcggctcgatgccgatcccgacgaggccgacgaacgcgcgggccacagcgcgccctcgagcgcctttgccttgtgcgcctacttccggcgctacctgatcgactgcacgcgcgcgagttcgttccgccgcaagttgtcgatcggcgaccaggtcaccgaggcgcagctcgaagacgcgctgggcgcggatgaagatccggacggctgcctggcggaacacggcctgagtgcgggcgcggtgcagctcgccgcgcgtgccttcatcgccgagctgcccgagcccgagcgcatcctgctgtgcgagggtttcggcaaggaagccgaaggcggcctctcgggcattgcctcgcgccatgccattgcctcctaccactaccgcgcgggccggctgggcctggtgcacaagcgcgaaggactgaccgccgactacgccaagacccgcctgggcggctggatccagcagacgctgggcattgccatcgagcccgggaacatggcggcgatcctgcaggttttcaaaatcctcggtgctgaagcgtcttatgcctgaagacatagccattcaggaacagaccgccatgcacaccgacctctggccccccctcagcgtgatccgaagtgcgttccagtccgggggcgccgcgcccccggtgcccgacgcctccggccgcgacgccgtcgtggccatgccgggcacggccgcccgcgccgcggccggcacgccgcgcgccgtgctcgatctcgtgcttccgctctccgaattggcccggcgccgcgaggctgtcgcccagcgcgcctttacggcacgctgggcgccgggccgcctcgtcagcgtggtggtcgaagggcgcctgctcggcgtgctgctcgaccgctgcatccacggccagctctggcagggctggatggctgcgggcgaggccgactgggccggtgcgtacgacgtattgctcgagcccgacgacgagcccttcgagcccgccttcggattgatccaggcgtggaacgtgctcacgctcgaacccagcccgcagctttgcgcgcgcgtgctcggcgaggtctcggccacgcggctggccgccatccgcgcggtgcacgacgaatgggccgcgcaagtgccgctggccattgcgcccgaaccgggacgcatcgcattgcgcaccgtgggcggcgtcttctcggtgctctgcggcacgccgctgggcgagaaagacccgcgcgccgaataccaggcgatctatcgcgatgccgcgtcgcagctgagcacggcactgcagccgggttcgagcagcgcatcggttgcaccaaccgcgccgcgcgcaacgccgcagcccaggcccgagggcggctggtggggcagcatccgccgctggttcggcgccgagggctgggtgcggcctgcgttcgcggtgcttgcgctggtcgtggtggtgcagaacgtcggcctgcccggcggacgcccggcggaagacgaggaagtgcgctttcgcgccgtgccggccgcgcctgcggctgcgccggcgaacctggtcgtgcgctggaaagacggcgtgcgcatcgacgaagccggccggctgttgcagtcgatctcggccgaggtggtgggcggccccggcacccagggcgcatggcgcctgcgggtgtccgatccggtgcaagcccaggcggtgctggcggcttcgccgctggtgcagtcggccggcccggccacggagcgtccatgacgtgcacggcgcacttgtctttctccctccccctctgggggagggcaggggtgggggcaagcggcgtatccatcgggcgctctgcctgcccccatcccaaccttcccccggaaggggaaggagccatgcgatcgcttttctcgcggctgctgttgaccttggcgctgctggtctccggcaacgccgtcttcgctgcccaacgcgccttgctcgtcggcgtttccgagctcgtcaatcaaccgcagtcgctctggcttcaggcgccccgcaacgacgtgatgctgatgcgcgaggccctgctgaagcagggcttcgcggcgcccgacatcacggtgctggccgatggcgtcagcggcgcggcgctgcctgaatcccgcgccatccacgaggcgctgggccgcttgctcgcgcaatcgaaaagcggcgacttcgtgctgctgtatttctccggccatggcgcacgctggcgcgacggcaccaagcgctaccaggagcccgacggcctggccgagaacttcctggcgcgcgacgtgcgcggcgcggtgggcgtggacaccgtgctggccggcggcgtgcgcgacgtggacttcgacgcctgggtgcaggcctttctcgcgcgcaacgtgttcgtgtggtcggtgttcgacacctgcgccgccacctcgatgacacgcagcgccaatgccggcgcggcaaccgccacggccgaaggcccggccgacgacgaagtacgctggcgcggcctgcgcgccgcgcagctgcgcggcgccgcacccacggcaacggcaacggcaacggcagcggccgaggcgcctgcgccatccgcaccgcctgcttcggagagggtggcgcgggcacgctatgtggcgttcttcgcgtcggagagccaccagatcacgccggagcttcgcctgccgcgcaagagccgcggcgcgcagccgcagggcttgctcacctgggccgtggtcggcgcgctcgagcgcaggcccgccacctggcgcgagcttttcgacggcgtgctctccttctatccgccggtcatcgacgaactcgcgcagcgctttcccacgcgcgaactgccttcgccggtggccgaaggcaatctcgatgcgcagctgttcgccaacagcgccgtggccgcctcgacgcggccggtgtggcgcgcgcagcgcagcggcgacaccctcacgctgcaggccggtctcatcgacggactgcagccgcagcaggaagtgcggctcgcggccacgatggaagacggcaccgttcgcagcgcgcaggcgcggctgctccaggccaatatcgactccgcgcgcgtggcggtgccgcccgcgctgcgcgccctctcgggcgccgcttcctggagcgccgcgccgctcgcaccgccgcccgcgctcgcactgcgcgtgcgcagcgacaagggcttgttgccgccgcgcatgaacctggactatccggcttcggtcgtttcggccggccatgccccggcgcccggagaggccccggccgatgtgcgctggaccgatctcggcgcggcaggccagcgcatcgaagtgctttcgcccgcactcaggagcggctcggaggctgccatccaggtgttgcccgaccaggccgcactgcgccgccggctcgaggccctggcccgcctgaagtggtggacccagctctccgcactcggcaacggcagcagtgcgcaggtcgacggactcgaggccgttctcgaaatctggagcagcgagcgcctggtgcgcagcgagccggtgcagaaggccggcgcgtcgctgctgccgcttcgcagtggcgagcgtgcggcgctcagtgtgcgcaatgccagcggccattcaatcgacatggtggtggtgggcgtcgacgcgcagggcggcctgcgcgcggtctaccccgacgacccgggcgagaccaaccgcttcgaacgcggcacgcagggcgcgcccgccaacaaacgcttcgagctgccatggttcgacgcacccgggggccgcctgctggtgctggcttccacggccagcccctacagcagcccgcgcctcttcggcgcggggccggtggaagcggctgcgcccgaagtccgcgtgcgcgggcagctgtccgagggcaaggcccggcagacctttgccgccatggtgcattgggcgggcgatgcgccgcccgccaagtaactgtttttgttctcaggagatcgacatgagctggacctacgatggaaaactggaccccgacgaggcactgcgcctgctcgactacctgtcgggcgaatcgggcaacgacttctcgatgatgatcgagagcaagggctcgccgatcgaaggcgagtcggcgcgcacgtatgaagacggcaagcagcgcatggaaatcggcggctactcgtacaagtccgacgtggtcattccgccgggctcgaccaagggcaagctgcgcagctattcgttcatcgtcatccgcgactgcgatgccgccacggcctccatcgccagcctgctgaagaaccaggaaagcgacctcaaggtgacggtgtcggtcttcaaggccggcggcgacagctccaaggacttgcagtcgcacctggagttcgtgctcgaaggcgcgcgggtcgactgccacgccatcgtcacgggcggcacgcccaagcggccgtgcgacatcatcttcttccactacaccaagctggaaatccgctcggcgccgcagcagaaaaccggtgcgcgcggcgcggtgcgcacctgcaccttcagcggcaactgagccggccgaaacggagaacaccatgagcacctctgccgaactcatcaagtctgccgaccccgccgctgccctcaaggcattgagcgacgaggttcgcgccaagccatcagacagcaagcagcgcgtcttcatggcgcaattgctctgcgtgctggggcagtgggagcgcgcgctcaaccagctcaccgtggcggccgagctcgacgcgctggccgtgcccatgaagcaggtctacggcgaggccgtgcgctgcgagggcctgcgcgccgaagtgttcgcgggcacgcgcacgcccatgatcttcggccagccggacgaatggctggcccttctcatcgaatcgctgttgcggcagggccgcggcgaagtcgagctggccgaagacctgcgccagcgcgccttcgatgccgcgcccgccatcggcggcaccatcgacggcgtgcccttcgaatggctggccgatgccgacatgcgcctgggccccgtgctcgaggctttcgtcaacggcaagtactactggattccgtacgcgcgcctcgcgcacatcaagatcgaagcgcccgaagacctgcgcgactgcgtctggatgcccgcacacctgctgctcgaaaacggcggcgagacgctggcgctcattcccacccgctacgaaggcaccgagaagagccaggacggcgaactgctgcttgcgcgcaagaccgagtggcgcgagctgcggcccgaggtgtgggcagggagcggccagcgcgtgctcggcagcgatgcgggcgaatacgcgctgatggacgtgcgcgagattctcttcaatccggcggtgccggtggaggaggagggcgcgtcggaacaaggcggccaacgtggttgacctcacggcccaggagcgcctgcagccctcgctgctcgaccggctggtggaccatgcgcccgacgaaaagcgcgagagcgacgacaagcgcacgctgaccaagcaggcgctgcgccaggccgtgctgcgcgacctgagctggctgttcaacgccaccggctacggccttgcaatggacgacaggcagtacccgaatgccgcgcgctcggtcatcaattacggattgcctatgctgtctggccagttcacctcgtcggtgcagcgtgtcagcatggaacaggctttgaagaacgcaatcctgcagttcgagccacgaatcctgccccgcaccctcgaagtcgaactcgtcatggaaggctcagcattggactcccacaacagcattggcctgcagatccgcggcatgctttgggcgcagcccgtgccgctcgaattcctgatgcgaagccgcgtcgacctcgaggaaggccgcatcgagatcgtggacatgacacaaagatcatgagcccgcggcttttactggagtgatgccgtggacccccggttgctgaacctctacgagcaggagctgcgctactttcgcgagagctcctcggagttcgcccgcgcgtttcccaagatcgcgcaccgcctgggcatcgagggccaggaggtcgccgatccgtatgtggagcggctgatcgaggccacggcctttctctcggcgcgcgtcaacctcaagctcgatgccgaatacccgcgcttcacgggccacctgctcgacatcgtctaccccaactttttggcgcccacgccggccatggccgtggcctcgttcgcgaacgaccccgacgatgccaacctggccaccgggcccacgctgccgcgcggcagcgggctgcgcgcgcggcaggcggtggggcagaacacgcattgcgagttccgcaccgcgagcgcgctgcggctctggccgatcgaggtgcagcgcgcgcagtacttcacctatgcgccggacctgccgctcaacacgcacccgcagtcgcgtgcgattcgcggcgggttgcgcatcggcctgcatgccaccgcgggcctcaagttcaaccagatcgtcatcgacgacctggtgctgcacctgggcggcgccgaagacgtggcgtggcagctgcacgaatgcgcgctggggcagcccatcggcgtgatggtgcggcccttgtcgcccaccggcgcgctgcagggcgcggcgcagaacctgccggcgagcgccatcggcgccgtgggcttcgaggacgacgaggcgctgctgccggtcaccgccaccggcttctcgggcttccggctgctgcaggagtacttcgcgtttccgcagcgcttccagttcattcgcatctcgggcctgcaggcgctgctgtccaccatggcggtgtccgacgtcgagctggtgctgctgttctcgcgcggcgatgcggcgctcgaaaagctggtgggcgtggacaacgtgcagctgcactgcgtacccatcgtcaacctgttcaacaagcggctcgaccgcgtgccgctgaccgaaggcgtgagccagttccacctggtgcccgaccgcacgcggccgcaagacttcgaggtgcacacggtgaccgaggtggtcggccacggcgcgcccggtgccgatgccgccgcggcagagcagctcttccggcctttctattcggcctttcacggcacgcggcacagccacccggcctacttcacgaccacgcgcgagccgcgcatgctctcggtgcggcagcgcaccgaaggccatcgcagcagccacatcggctccgaggtctacatgcagatcgtcgatccgcagcaagcgccttattcggccgcgctgcggcagctggccgtgtccgcgctgtgcaccaaccgcgacctgccgctcctgatgccgctcggccgcgagaacgacttcgactgcatcgattcgtttccggcgcagcgcgtgcgcatggtgcgcgggccttcgcgcccggtgtcgccggtggtgagccaggggctcggatggcgcgtgctcgaccacctggcgctcaactacctttccatctccgacagcacgccggagcagggcgcggccgcgctgcgcgaaacgctgatgctctacgccgtgcatgccgacgagatgcgccagggccaggtgcgtggcctcttgtcggtgaagagcaagcccgtggcgcgccggctgccgctcaagggaccgatcgcgttcggacgcgggctcgaagtgacggtcgaggtcgacaaggacgcctttcacggccacagcgtcttcctgttcggcgcggtgctgtcgcgctacctggcgcgccacgtggaggtcaatcacttcgtcgagaccgtgctgcgcgtggcgggcaagggcgagaacatgcgatggaggccgctgtgcgggacacgccagattctgtagccggccgcgtcgacggcgcgctgcgcgcgtggtcggccgagccctggtccttcgactacttcgcggtgatgcggcggctcgaatcggtggccggcaccacgccgcgctggggccgcgcgctgctgccgagtgccgagccggtgcgcgtggggcaggagccctcgctgtcgttcgcgccggccagcttcagccgcttcgagcccgcgaccgccgactcgccgccgcgcctgcggcagcacttcttcagctacgtggggcccaacggtccgctgccggtgcacctgagcgacttcatccgcgagcgcagcctgaaccatggcgatccgacgtggctggcttttctcgacagcttcctgcatcgcttctcgctgcatttctaccgtgcctgggcccaggcgcggccggcggtggcgctcgaccgtccgggcgaagaccgctttcggctgcaggtgggcgcgctcgtgggcatgggcatgccggggcgcaccggccgcgacgagatccatgacgatgcgcggctgcatttctcgggctggctggcgcgccgcgtgcacaacgcggagagcgtcgagtcggtgctgtgcagctacttcggcgtgccggtgaagctggagcgctgggtcggccactggatgagcctgcccgccggcgaactcacccgactcggccagggcgaggcgtcgcgctcgatgggcatgggcgccatgctcggcacgcgcgcatgggaccggcagcatcgtgtgcggttgcatgtgggtccgctctcgatcgaccagtaccgcatgtttcttcccaccggcgatgcgcagcccgtgctgcagcgctggatgcagcagctgctcggcgacgaactcgagtgggacgcacagcttgcgctgcaaggcgcgcaggtgccgcctacgcgtctcgggcaagccaagggcaacgcgccgcgcctcggatggatcgcttggctcggacagcgcccgcgcgccaaggatgcggcggacgtgcgcataggcagccgcccgatggccgcccgtaccgcccaggccaccgtgggagccgccgcatgacaacgacgcccgcgcttccggacacgatgacgcacgcggccgcgctggcgcaagccgcggccctgatcaaggcgcaaaagctggacgcggcgggcgaattgctcgaccgcatcctggaggccgagccggccgaccccgacgccctgcactaccagggcctgctgcgccatgcgcaaggccgcagcaacgagagcatcgcgttgatcgggcggtcgctcacgctgcaacccgcgcaaagcggtgcctggaacaacctgggcaacctgctggtcgagacgggccgcatcgacgatgcgatgctcgcctacggcaacagcgtctccttcgcgaaaggaggcgacgaaggcgcccatgcgctgagcaatatcgcatcgctcgaacgccggaagggccactggcaagccgccgagcgcgtcagccggcaggcgatcgaactgcggccggaattcagcgaggcctggtacaacttgtcgatcgcactgatggagcagggacgcatccatgagagcgtcatcgccaacagccgggcggtgttgctgcagccgcgcaacctgagcgcccgctcgcaggtgattcgtgctctggaactgctcggcgagaacgagcaggccctcggcatgtaccgggagtggctggccgaagatccaggcaatcccgtggtcacgcacctgctggccgcctgcgaggggcatgcgcccgcgcgcgccagcgacggctatgtagagaccgtgttcgacagctacgccggaagcttcgacgccagcctggagaagctgcactaccgcgcgcccgagctggtggcgcacgcggtgcaggaaatgcatggcgcgccggccgcgagcctggccgtggtcgatgccggctgcggcaccggactctgcgccccgctgctgcggccctgggccgcgcacctggctggctgcgacctgtcggccggcatgctgcagcgcgcggagcaacgcggcggctacgacgtgctgcacaaggccgagctcacccactacctgcacacccagcccggccggttcgacctggtgatatcggctgacaccctgtgctacttcggcgacctgcacgaggtgctggcggcagccgcgcgcgcgctgcgtccgggaggcggagtggtgttcacggtcgaggccatgtccggggggcgggacgacttcaggctcgaaggcagcggccgctaccgccatgcggctgcgcatgtggaggcctgtcttgcggcccccggattcggtgccgttcgcatcgagccgatcgttccgcgccgtgaagcggggcaggacgtgcagggttggctggccagcgcaaggctttctgcacattgacgccgggcacggctcgcagaacttcgaattttccagcatgaatcgtcttcaacagatacggagtcttccatgagtgaaatcagtcgcaccgcccttttcggcaagctcaactcgttggcctacaaggccatcgaaggcgccacggtgttctgcaagatgcgcggtaatccgtacgtggagctggagcactggttcgcccagctgctgcaggtgcaggactccgacctgcaccgcgtgatccagcattacgggctcgacgtgtcggtgattgccaaggacatgacggccgcgctcgaccgcctgccgcgcggcgccaccgccatcagcgatttttctccgcacatcgagaacgccatcgagcgtgcatggacctacgccacgctgcagttcggcgaggcgcaggtgcgcaccggctacatcctcgtcggcatgctgaagacgcagagcctgcgcaacccgctcttcggtttgtcgaagcagttcgagaaggtgaaggtcgaggacctggccgacaacttcgtgaagatctgcgacccttcgcccgaatcgcacatgcgtgcgcaggacggcaccggcatgggcagcggagcgcccggcgaagattccggcgccatggcgcccgccgccatgggcaagggcgatgccctcaagaaatttgctgtcgacctgaccgagaaggcgaagaagggagagatggatccggtgaccgggcgggacgaggagatccgccagatcgtcgacatcctgatgcggcgccgccagaacaacccgctgttgacgggtgaggccggcgtcggcaagaccgcggtggtggaaggcttcgcgcagcgcctggcgcgcggcgacgtgccgccgcagctgaaagacgtgaagctgctcacgctcgacatcggcctcttgcaggcgggcgcgagcatgaagggcgagttcgagcagcgcctgcgccaggtgatcgacgaagtgcagagctcgccgacgcccatcattcttttcatcgacgagatccacacgctggtgggcgcgggcggcgcggccggcaccggcgatgcggccaacctgctgaagcctgcactcgcgcgcggcaacctgcgcaccatcggcgccaccacctgggccgagtacaagaaatacatcgagaaagacccggcgctcacgcggcgcttccaggtcgtgcaggtgcccgagcccgacgaggtgaaggccattctcatgctgcgcggcgtggccagcgtgctcgagaagcaccaccgcgtgcagttgctcgacgaggcgatcgaggcggctgtgaagctgtcgcaccgctacattcctgcgcgccagttgcccgacaaggccgtgagcctgctggacaccgcctgcgcccgggtggccgtgtcgcagcacgccacgccgcctgaagtggaagactgcatgcgccgcatcgagggcctcacggtcgagcaggagatcatcggccgcgaagaagccattggcatcgatgtgaccaagcgcgccgcgcaggtgtcggcactgctggccgaatcgaaggtgcagctcgatgcgctcaatgcgcgctggcaggaggagaaggggctggtcgacaggttgcttgagttgcgcagcaaattgcgtgcgggcagcaagccggtggacactgcatccgccgagggcggtgcaaaggccgacgtacccccaccccagccctcccccagtgggggagggagcgaagaccgggccgcgctgcttgaagaactgcatgtgctgcaagccaagatccatgcggtgcagggcgagtcgccgctcatcctgccttcggtcgatgagcaggccgtggcctcggtagtcgccgactggaccggtattcccgtcggccgcatggtgaagaacgaagtcgaggcggtgctcaagctggcggacacgctcaaccagcgcgtcatcggccagaagcacggcctcgaaatgatcgcgcgccgcatccagacctcgcgcgcgcggctcgacaacccgcaaaagccgatcggcgtgttcatgctctgcggcacctccggcgtcggcaagaccgagaccgcgctggctttggccgaggcgctctacggcggtgagcagaacatcatcaccatcaacatgagcgagttccaggaggcacacaccgtctccacgctcaagggcgcgccgcccggctacgtgggctatggcgagggcggcatcctgaccgaggccgtgcgccgccggccctacagcgtggtgctgctcgacgaggtggagaaggcccaccccgacgtgcacgagatcttcttccaggtgttcgacaagggctggatggaagacggcgagggccgcatgatcgacttcaagaacacgatcatcctgctcaccaccaatgccggcagcgagctggtgatgagcatgtgccgcgaccccgagctgctgcccgattccaacgcgctggccgatgcgctgaaggcgccgctgatgaaggtgttcccgcccgcactgctgggccgcatcgtcaccattccctattacccgctgtcgcccgagatgatgaagaagatcgtgcggctgcaactgggccgcatcaagaagcgcgtcgagaccaaccacggcgtgcccttcgagtacagcgaggcggtggtcgagcaggtggtcgcgcgctgccaggacccggagtcgggtggccgcgtgatcgacgcgatcctgaccaacaccgtgctgccgaccatctcggtcgagtacctgcagcggctggcttccggcggcgagatccgccgcgtggcgctcgacgtgaaagacgccgacttcacttacgccttcgattgaagcttcaacaagagacccccgaaatggccgaccacgagttccgcatcgagagcgattcacccgccaacaaggagctgatgttctggcgcatcgtgggccacgaggcgctcgcgcggccttcggcctatgagctcacggtgctgtcgaagaaccgggcgctcgacgccaaggacatccttggccgagccttcgacgtggtcatcgaattccaggacaaggacggcggcaagcacgagcggcactgccaggggcatgcggtgcgtttcgtgcgcgcggggcacgtgggccggcattttgaataccgcatcacgctgcgctcgtggttctggcttctcaccaagcgcagcaactcccgcatcctgcaggacaagaaggtgctcgaggtgctcgatgcggtgttcgaagacagtccgatcaagcgcttcaagaagaccaagtccgacaacgtcatcggcacgcacaacccgcggcgctactgcgtacagcaccaggaaacggactatcagttcatctcgcgactgctcgaggacgaaggcatctactactggttcgacgcgcacgatgcaccgggaaccatgcacctgtcggacgcgagcgacatggcgcacgagaagttgtccgtggccgacaccctgcgccatgcgggcagcgatgcgagcgaggcgcgctacaacgagatctcgcgctgggtgagtgcgcgccatttccatacgggcaagcaggattcgcgcgacagcgacttcaaggccatcaagaagaagctgggcgccgccatcgacgtgtccgacgatcatgagctggcgggcctcgaagtgttcgagtttcccggcggctacttcagcggcgatgacgccgagaaccgggccaagctgcgcggcgacgaactcaacgcgcgccgcgaccgccactgggccctgaccaactggcccgacgtggccgcgggccgcagcttcaagttcgagggcgacccggatggcgcgcgcgacggcgactacatcatcgccgcctgcaccttcatggccagccatcccggctacgagagcgtggcggccagcgccgccgagcagccgatccacagcgtgctgtccgaggcgttgcgcgacgacgcggtgaacgccgacacgctgcaggtgctggaagaactgattgccggcacgcccatgctgcacaccgcgcaaccgggcacgagcgccttcctgctgaccgtgattccggtggatcgcccctaccgcgcgccgcgcctcacgccgcgcgtgaccatgcccggcccgcagatcgcgatcgtggtgggccccaagggcgacgagtaccacgtggacgaccacggccgcgtgaaggtgcactttcattgggatcgctacgacgagagcaacgagaagtcgacctgctgggtgcgcgtgtcgcagccctgggccggcaagggctggggcggctatttcattccgcgcatcggccaggaagtgatcgtcgactttctgaacggcgaccccgaccgccccatcatcgtgggccgcgtctacaacgacgaccagccgatcccgtacaagtcgccctcgcaaagcggcttcaagacccgctccacgcccggcggcggcgcctcgaactacaacgagatcatgttcgaggacaagaagggcgaagagaacatcaacatccacgccgagcggaacatgagccgcagcgtggagctggatgattcgaccacggtcgaccgcgaccagtcggtcaccgtcaagcgcgaccagacgaaccacgtggaccgcgaccgcaagagcacggtgacgcgcaacgacaccaacatggtggcggtcgaccagacgaacacggtcaagggcaagcagaacaaccaggtggtgggcaaccgcgacacctttgtcgatgccaatgacatgctcaaagtgaagggcactggcacgcatgaggtgatcggcgcgcgcagcgacatctcgcgcgccggagaaacccgcagcgtgaccggcaaccagaccatcaccgtcagcggcaacctgacctacaaggctgcgaagatgagcttcgaggccgcgcacatcgattggctggtgaccggatcgagctcgaagtacatcacggtgcccaccgggcccctggccttgatggccaacaagatcaagctgatgagcaacaccggcatcgacatgatggccgcgggcgacatcgacgccgtttccatcggctccaacaccacggtgcttggcgccaacagcagcgggtacatcggcaacaacagcgaagcgaacatcggcatggcccgatccaccttcattggcttgaacatggaaaccgcgcttgcggcgagcctctccaacttcctggggctgcagatggacaacaccgcgggtctgaagttggagacggtcgctgccgccggcatcgaacagaagacgtccagcttcagacagtccgcgctggcctgcttcacacccggagccggaggtgcggctgcgggcatgggcgctgcggtggccgctgggctcggcgccgtggcaggcgccggatccgccatcgtcgatgtgcttgccactttcgagcagtatgcgaaggcggccgacaagctgcagaaagccgcggaagaggcggcggctcaggacccggcggtgccgggacttgccgacaggctgtcggccctttcccgcattacgcggcgccgtgcaaccgacgccaaggtgggtcttgttgcaacactcggcatcggtgtggtggcgcaggtcggctccgacatgctgggcggccaaggtgccgcttcgcaagcggatgcgctcggcagagcgatgcccgaccccgatgccaactgagcccacgcctcatgcaagtgctcaagcctcaagccctcggactctcgacgcggccaatcgaattccgcaagcgctacggcttgtccatcactgcttgcctgcacctgccttttgcgcaggacaagaacggcaccctctggtcggagcaatcgatgtggtcgttcctcgggaaggaaatggcacaacccctgatcgacgagggcgttgccaagctgaccccggagttcctggtgcacggcaaggcctttccgccccgcgacaggcctgaggcctgcgcggtacgcgcccgcctcggtgcacgggaaaagaccgtactggtttttggcgagcgctactgggacggcgggcgtgccagtgcgccgcaggccttcgagtctctttcgctggattggtccgcggcctatggcggcccagacttcgcatccaacagccagggtagagggaggcaagccaaggacagcgtgacctggctgccgaacaccgaactgccgcaagaccggttgcagcgtcctgaccaggccatcgttccggcgggtttcggtgcattggatgtgatgcatccgcaacgcgtgcagtatcgcggcacctatgacgcggactacctgcgcgagcacgcgcccggcttcgctcccgataccgattggcgttatttcaatctggcgccggccgatcagtggatggacacggcgctgatcggcgacgaggcgttcgcgttcgatcacatgcatcccgaaaagccgcgcatcgagggtcggttgccgggcatgcgggcacgcgtgttcgccggctacaaggtcgaaggcgctgaacccaagatccgggaagtgccgctacggctgaccacggtgtggttctttccgcacgcggagcgctgcatcgcgatcttccaggggcttgccgaggtggacactgacgatggttccgacgtggtcagcctgatgggcgcggtcgagcgcctggcggaagccagggacgatcaccactacatcgatgctgcggcgaaacgggccgacccgaaaatgggggctatctacgccatcatcgacagcgacctgctgcccgctggtgtcagcaccctggaccccgacgtggaagccgccaaggcgcctttcgaaatggcgggcctgcagggagaagcccagtaccgccgtgcgcagatcgatgtggagctcgcgcgtgaaaaggccaccgcattggggaaagacccggatgccctgggcatccggatgcctccgcgcgaaaaggttccgacgggcgacgagctaccgccgtacctcgaaaagaagatgcaggaagcgcaggcgcagcagtgggctgccgtcgaggatgccgtcacggtgctggagaaagcgctggcgatatcggaagaaaacaagatcgacctggcgaagctgcagcatcgcgggccgccccggtacgacgccgagaagcacctggcccagatgcacgcgcaggccgcggccggtacccggcccatcgaccttcagccggtgcttcccaagctgcgccagatcgaagacgctcaccgcatgggctacctgcagtccgcgcacatgcagctaccggcgtttgcaatgccgcccgatgaggcggcaacgctgcgggacgaggtgtcgcgtgccgttcaagccggcatcaagttctttgccggcatcgacttcaccggtgctgatttgtccggcctcgatctgcgcgaggcgaacttcgaaggcgcctggctggagagtgtcgatttcaggaattccaacctgtcgaacgccgatctgtcgggcgcggtgctggcccacgccaatctcgaaggcgtgattgcgatcggtgcgaaattcgacaaggccaacctgggaaaggccattctggcccgcggcgttttcgacgactcggatttcaccgaggcggtgctgatgcattgcgcattcgccggcacgcagatgcgccgggcccggttcgccaaggccaatctgctggagacgacctggggtgacgcggattgggagggtgcccaacttgcgggtcagactttctacaagctggatatcagggggatgcgttggcccggtgcggatctgtctgtctgcaatttcctggaatcggacctttcgggcgtcgatatgcatgccgcgagcatcgcaagcgccaccttcgcgacctgcaagctggatggggcgaacatggtggctgcgcaatgtgccggcgccgtagcggtcaaggactccagtcttgtcggcacggacatgagcggggccaacctgcgccagttcaatttcggcgcatcggacctgcgcggcgcgaagctggttcgcgcggtgctggatggcgccaatttcggcggcgcacgactcgagggggcggacctgcggcttgcaagcgccaaaggcaccctgatgcacaaggccgactgcaggaaggcattgctctctggcgtgaatttcaccgacgcgatattgcagaaagccgatctgcgcggtgccgatctgcggcgtagcaacctcttcggcgccgacctcagccgcgtgcggctcgatggttcgaccagtttcgacggtgcgctgctgaagagggcgcgtacctggccccgtctgacgcacgaacaacaggcggtcgcatgagtccggaactgttgagcattgccgtcggcatcggggaggccctgcaaggtctcgatctcggcaaggggcggtacgccgggcttgtgctgggcggagcaactttctccaaggtcaggttcgccgaggccgattttcgtggggccgacctgcgcgaaaccgtgttcgaccagtgcgacctgcgcggtgcgatcgcttcgggcgccaacctgcgcaaggcgctgttcaatcgctgcgtgcttgaccatgcggacttgcgccaggccaaccttcatggtgcggtgttcaccgaatgcgacatgacgcatgcgcaactcgcacaggccgtgctgtcgatggctacggtgtcgaaatgcaagatgggccatgccaacctgcgcggcgcctgcctcgattcggcggtgttcagtcagtcggtcttgcttgacgtgtgcgccgacgacacgagctggcaatacaccgccgtgaccgaatgcgacctttcgcacctcacgtgggcaggggcgcgaatgctgcgcaacgtgttctccaatacctcgctcaagcgcatgtcattcgcgagcctgacgctcgacggatgccagttcgcgtcggccgacctccgcggggcggatctcggcggcatcacgctgcagcagtgcaatttccagaatgcgaacctcgaaggcgcgagcttcgcgaaggcggtggcaccgtcgaccatcttctgcgaagccacgggcaagggtgctgatttctcgggcgcgcgcatgcggcaagcactcttcaccggcgccgcgctggcagaggccaacttcgccggctgcgacctctaccagacgcatttcgcgggcgcgaaactgcgcggtgcgaacttcaccggcgcggagttgacctatgccgacttccgccatgccgacctcggcggggccgacctgcgaggcgccaccctgttgcgcacggtgctgcatggcgccaacaccgggaacgcacaaatgaccgaccgcgcacgcgcgctcgaatccgacccggagctggcggaatccgagcgatggcagccgctggccgcctgatccgacgaatcgacagatagggaaacatgcaatgaccgaaaccaccacactcgaacatgccgcgcctcgagcccgccggcggcgcgaaccctccaaggccatcaccggcgaatggtgcgtgggcatcgtcggcacagatgccggcggcgcgcaggtcgtcatcagcggcgacctgcagctgcgcgcgcggcgcgctgccagttgcctgctcgagcccgctgccggcgacagcgtggcctgcctgcgcatcgcccctcaagaggtctggatcatggcggtgctgcagcgcgaggagggcaccgccaacgtgctgcgttgcgcgggcaacctgcgcatcgcggtggacggcggcgcgctggaacttgaggccgcgcgcgtcggcctcaagtccgaggaactcgacatcgcggcgcaaaagacccgcgtggccaccgacaccgccgacttggttggccgcgagtttcacctgatcggcaccagcatcaaggtggtgggttcggtgctgtcgtcagtcatggagcgggtgcagcatttcagccggcattacctgcgcaccaccgacggcatcgaccgcgtggcagccacgcacctcgagtgcgaggcgaagcagctgcttcgcctcgaaggcgagcacacgctggtgaacggccgcgagctcatcaaggcgcgcggcgcgcagatccacttcggctgaagaagaaagaagcggagcacagcatgttcgccaactgccaactgatggggaccgacatgggctttcccgatgtctgcatcacgcccgccgcgccgtcgccgattccggtgccctatccgaacatcgccatggggccgatggcgattccgaattgccccacgatcctgatcatgggcggcccggcccacaacctgggcaccacgattccgatgaccaacggcgacaactccggcgtgctgctgggcgtcgcgtcgggcaccgtgatgggaccgagccgccatctcaccggcgccttcacggtgctgtggaacggcatgcccgccacacggctcaccagcgtctcgctgcagaacagcaccaactgcccgggcgtgcgcaccgtgccgagccaaccgctcgttgtattgctggcgccctgaggggcctggtgccgccacggcgcgccgcatgcggggtgcgccggacaactagaaagtgtgggagatagggacggaaaggagaggctcagagccgaacgccatggccgaccacgagttcagcataaaaagcgattcgcccgtcagcgacaagctgaagttctggcgcattgtggggcacgaagtgctcgcgcgcccgtcggcctacgagttgacggtgttggccgagaacgagacgatcgacgccaaggacattcttggccgatcgttcgacgtggtgatcgaattcaccgacaaggacaacggcaagcacgagcgccactgccagggccacgcggtgcgcttctcgcgcgtggcgcagatcgggcgctacttcgaataccgcatcagcctgcgttcgtggttctggctgctgaccaagcgcatcaattcgcgcatcctgcaggaaaagccggtgctcggcgtggtcgacgcggtgctcgaggacagcaggatcagcggtctcaagaagatcaagtcgggcaaggtgatcggctcgcacacgccgcatacctactgcgtgcagtatcaggagagcgactaccagttcctttcgcggcttctggaagaggagggaatctactattggttcgacgcgcacgatgcgcccggcaccatgcatctgtcggacacgagcacgctcgcgcacgacaaactccccgccgcggacacgctgcaatacgcagccacccacgccaccgaggcgcgcttcaacgagatcacgcgctgggtcagcgcgcgccagttcgagtcgggccgctttgcttcgcgagatcgcgacttcaaggtcatcagcaaggaactgcgagccgacaggggcgacccggacacgcacgagctgtccgatctcgaggtgttcgaatttccgggcggctacaccgcgaccgacgacaccgacaacctggcgcaggtacggctggacgaactcatcggccgccgtcagcgccactgggcgctgaccacctggcccgatgtgacggcgggccgcagcttcaccttcgagggcgaccccgacaccacgcgcaatggcgactacatcatcggcgcctgcactttcgcggccagccaccctggctatgagtccatcgccttcgacgagatccggcgcccggttgacgaggtgctgcacgaggcgctcgaagacgatccggtcaacgatggaatgcttgcaatgctgcgcgacatggtggccgggacgcccgccctgcatgctgccgagcgcggcaccagcgcctttctcatgaccgtgatgccgctcgacgcgccttggcgccccccgcgtctcacgccgcgtgtcgccatgcgcggaccgcagaccgccatcgtcgtggggcgaagcggcgaacagatctggaccgaggagcatggccgcgtgaaggtgcagttccattgggaccgctacggaaagaacgacgagaacagctcttgctgggtgcgcgtgtcgcacccatgggctggcaagagctggggggccatcagcatcccgcgcatcggccaggaagtgatcgtcgactttctcgatggcgatcctgaccagcccatcatcgtcgggcgtttctacaacggcgagtcgatgtcgccctatggcctgccggcgggcgccgtggtgagcggcatcaagtcgaatacgcacaagggcaagggctacaacgaactgtcgatggacgataccgccggcaaggagaaggtgacgatccacggccagtacgacatgaacaccacggtggagcacgaccagacgacgaccgtgcacaacaaccgcaccgacgccgtcgatgtcgacgactcggagaccgtgggcagcaaccagacccagagcatcggggccaaccagacgatttccgtgggtgcaaaccgcgaggagtcggtgggcggcactgaaaccatcaccattggcggccaccggaccgaaaccgtgaacggcggcgaaaccgtgaccatcaacggcgggcgcagccacaccgtgaacggcatgcagaccaccaccatctcggtggctgaggcgcacaccgtgggcgcggggcgcatgcacagcgtgggcgccggcgaggccatcaacgtcggcggcgtgcaggccgtgacggtgggcggcgcgcagatcgtcagcgtgggcggcgtgcagaaagtcagcgtgggtgccctgcagtcgatctccgtcggcggtccgcacaagctgtcggctgcggtgatctccgagacatcgaaggggccgatcaagatcaaggcgggcgccatctgcatggtcgaggcacccaccatcatgctcaaggccggcggcagcaagatcgtcatgaacgccagcggcatcaccatcaagggcgccaagatcaccatcaaggccgacggcagcgcgtctttcaaggccggcggctcgatcaagatcaagggctccaacctgggagaggactgagccgtggaagaccacaccgatctccagagcgcgcgcagcgtgctgcagagcgtggcggcctggtcgaagctgtcgggccaaggcgtggcggtggccatctttgcaggcttcgatgccgaggggcgcttcctggtcaccctgggcgaaggcatggcgccggtgcaggcgctctcgaccgtcggcctggcacccggcgatgccggcgcggccatcgtcgtggcctttgagcagggcgaagcgcggcaccccgtcatcgtcgggcgcgtgcagccgccgcacaccgacgcatcgcaagcgcgcgaggcgggcgcttacgccaacgtcgacggcgagcgcgtcgtgctccaggcgcgcgagcgcatcgagctgcgctgcggcgacgccagcatcgtgctcacacgcgcgggcaaggtactgatcaacggcaactacgtgctctcgcgctcgcgcggcgccaatcgcgtcaagggcgcctacgtgggcatcaactgaaaaggcatgcgccatgtggcagctcgacaaccgaacgccctatgccgccgaacgcacctgggtgcgcgaccgcgacggtgcggagatctggttggtggcggtgaagtgcagcttcgacatttcacccgatggcgagacaagcgtcgcacccgagcagccacccgtcgcgcaggcgcccgtcttcgtcgacgaggccgcgccccagccgagcctgctctacgagatggacctggtgcgcaccaagcagacgaccgacgtggtgctgatcggccacgcgcatgcgcccggcggcgcgcccgtgacgcagctcgacgtgggcctgcgcgtcggccccatcgccaagcgactgcgcgtgaccggcgaccgcgtgtggctgggcggcgcgccatcggagcccgagcctttcagcgccatgccgctggtgtgggagcgcgcatacggcggcgtcgatccgtggacgcgcaacgcgccgttgccgcagttcgacgtgcgcaaccccgtgggcacgggctttgtgacggaggctatgcatgcggaaggcctgcggctgcccaacatcgagtacccggaccaatgcgtgcggacgtggagcgaccggcccgagcctgcgggtttcggcccgctgtgcaaccactggcagccgcgcgcggggtttgcggggacgtacgacgaggcgtggcagcgggatcggttgccgttgctgccggtggattttgatgaccggcactatcagtgcgcgccgggggatcagcaggcgccgcagttcctggtgggcggtgagccggtcgtgctgatcaatgtgtggccgcatggggaggtgctgcgcttcgaactgccgcgggtgattctgggcctggagacctttttctccgacggtcagcggatgccgcacgaacgccctgtgctgcacacggtgatcgtcgagccggatcgatcgcgcgtagcactggtttggcacagcgcgttgccttgccatcccaaggtgcacaagctgctggagacgcgcatcgtggagaagcgcctgctgcgcctgggcgagatcgcgtccgggcaggcaatggtggcttgagcatggccggcagcacattgcacatcctcgggctcggcgccagtacgccgatcgggcgcaacgtgtgggccagcgccgcggcaacgagggccggcgtgtgtggcttttccgagcatccgttcatggtcgacacggctggcgagccgatgcgtgtcgcgcgggcaccctggctcgatgtgggcctcgacggtgccgcgcgcttggccgcattgctgttgccagccatgggcgaagcattggtgccgctggcgcaggcaggacgagacttgccgttgtgccttggccttgcattggcactgccgccatcacgaccgggccggcccgacaccctcgtcagagagttgctgaaagccatcggagagcaactgcccggcgacttcgggcgcaccgcgctcttcgagttggggcacgccgctggctgtctggcgctgtctgccgccgaggtgggttgcgcccgcggggccttcgatgcttgcctggtggccggcgtcgattcctacctgtcgcccgagacgctggaatgggtggaagcctgtgatcagttgcacggcggtgggccgctcaataacgcctggggctttatccccggggaggctgcgggcgcggtactcctcggcacatccgacctggtgcagcgctgtggcctcgcgccactgggcgaggtggtttcggtcggcatcggcatggagtccaagctcatcaagaccgaggcggtgtgcatcggcgagggcctgacccaggcctttcgtgcggcgcttcaggccctggcacctggcgagcaggtgcacaacgtgttctgcgatctcaacggggagccctaccgcgccgacgagttcggcttcgccgcgctgcgcactggggagcactttcgtgcagcgtcgggctttgtcgcgccagccgactgctggggcgacgtgggtgcggcgggctcgctgctgcacgtcgcgttggcgatcatcgccaatcgcaagcgctacgccaaggggccgctgtcgatggtgtggggcagttccgagtcgggcgaacgcggggcagtgctggtgcgctgcgccgatccagtagggggctgagccgtgccagtcaccatcagggtcaatggcaccagtctcacgctggtccacaagttcagcatcggcatcagcacagcgacgattcctgatgtgtgcaaaacgccaagccccggtgggcccgtgcccgttccctatccgaacattgcgaactcgatcacgctgtcgagcggcaccacgaccgtcaagggcgacaaggcgatggctgcgaacaaaggttcgaagttcgccatctccaacggcgacaacgcgggcgtggcgggcggagtgaagtccagcaccttcatgaaggaggcgacctggatcctctactccttcgatgtgaagatggacgggaagaacaccgcccgcctctcggacaagatgttccacaactcggagaacgcggcgaatctggggggagaggcgcagcagcccttcgccgatgcggtcggcaaggcgttggccgacaagctctgtgatgcggcctgcaaggcgatggacgacaagaagaagaaagacgcggcagacgtgaagaaagggaaaacgcccacgtcaaaattccagaatctcatgcgcaatcgcctcgaccccaagccgcgcgggcgccaggcgggactgatcaccgaggcttcgcaggagatcggcggggatttcatcggaaagtggggcgcggcaaccggcagcggatcgggattcgtcaaatgggacatcgtgctgaccggtgccaagaaggccgtggaaaaagggacggtggcactcagcaaggtgaccaagatcatcgaggtcaagtttccgggagactcccttacggacaatcaggcagccatgatgaagaagtcgggcacagcgaagaaggtgacggtcatggatgttgaaaatgactgcgtttgcacatgaaaggtagaaccatggattggtcccgattcacgttcgagaagggcgatcatgtcctggcgatgccgtgcctcgaggtcgtcgcgttcgcctacggcgcgccggccagcggtgcgggtttcgagagattcctgcgcgcgttcaccgaggcgttcagcgatcaccttcgcttctatcgcaccggcgacatgaagcgctcccggaccttcgacgcgggcgtgctcgatggcccccatcactggttctccgacccacgcctttttgccaccaagatgcttggtttcttggctcactctggcgaatcggcgcgcaacatccgtcctccggccgtgaagatatcgctgctaggcgtcttcaagccgccgtgcttcgtggtgcgaatgatgctgccggtcgagtggggcagcgagccggaggaagtgatggggctggtccagaacgccctggcggagtttccgttcaagggtggccactgcggatactctcttgtctgggaggagacggatatttcgttggagcgggaggtctgcgcatgggctgcaccgcttcttcgccgccatccgggtctcgggtatggcgatgccatcacgttgtcgaatgcggccgaccggggcttggtcgcggtgaactggttgacgttccttgaggccgaaatggccgagattcttggcggccaagcagcactggcacaccgcgctcccgccgatgtgtccgtgcttcctctcggcaagggcggtgtgatgttgcgtgccggcgatgcgccgcagctcggcgacgtgaaccgccagaatctgctgcccgcctaccacgccgcaggccagctcgtcgcacccgtgacggcacccgacgaagcgctcgatgatctggcgatcaacggcatgtccgaagaggatgcgcatgactggcttcgacgtttcttcgtctgaacgctactccggccccatcgcaatcgatgttgcagtggccgaaggacccgagggcgccatcgaactcgtggagcgccgcatccgagtcttcctcaaggccgtcggcgcgggatacttcttcccggggcgcctgcgccatcccgtgcgcgttgaagttcggaccagcaccgcatcggtccacgcaaggctggaggtcgacgacatcgcgatcgcggccttcgccgtgctgggcggcatgctggcggattgccaccatcacgagatattcttccgatcggcacatgccgtgctgggccgcgacggactcgatctgatgaccgagagcggcttgcgcccggcagccgtcccgcagctgccattcgtcgtcgagtttccggaggacatgggcggcaactacgcattgctggtcgagatcgaattcgcgcagccggtgccgcccgaagcccggcagggcctgctcgaaacccttgcgctgtgggatgcgctcacgcttgcgtatccctccgatcccgacgaggcggtggaagtcagcggcgcgcaggccatgttcaatgatccgcgcacgatccactatcacgaatggatctgggacaacgcggacgccgaggcgtgggatctcatcgtcaatctctgctgcgcctggcacgagacgctgcccatcgtgcggctgcacttcgagtaggagcccgtcccgtggaatccgacacgctgcttccagtcgtcgccgagcacgccgacgaagccgccttcctctggctgcaacgcgccagcgcggttcacgcgcccaactactcgccccagcaattcgccgacctcgacgaacgcctcgccgctcacatcgacggcctgcgcgttgccggcgaagaaggctgggagcatgcactggcgctcaccgacaacgaaggccccgaagacttcttcgttgccgccgtgctcgccatcgaagcggtcgatggccgcttcgacgatctggtcgaacgtgcaaaagatttgcccgaggtcgtgcccggcctggtctccgcgctcggctgggtcgagccgaagtatctcggcggccgtgccaaggcgttgctcgacgacgcctcgccgctgcggcagaagctcggcttggcggcttgcgcgctgcatcgacgcgatccggggcccgtgctcgggcaactgatcgcgggtgcgccggacagcgtgcgcatccgtgcgctgcgcgcagccggcgagctgggccgtgccgatctgttgccgcaggtgcagtcgctgctcggcgagaccaagcccgagctgcgcttctgggccgcatgggcggcggtgctgttcggcgaccgggggcaggcactcgacgtgctcgcggccttcgcgctgaagagcgggccgcgccagccgcgtgcgttccagcttgcgctgcaggcgatggaggtcgcgccgggccacgcgctgctgctcgaaagtgccacactgcccgaggcgcagcgcctgcgcatcatcggttcgggattcatcggcgacgcgcgctacgtgccatggctcatcgagcagatggcgcatcctgccatcgcgcggattgcggccgaagcgttcgtcaccatcaccggcgtcgacttcaacctggagcagatggaaatcccgccgcccgatgatttcgaagacggccccaccgaagaccccgacgatgaaaacgtcgaactcccggaggacattgccttgccctggcccgatgtagggaagatccgccaatggtggcttgcaaaccagtcgcggttcgtgcccggggggcgccacttcatggggcagccggtgtcggcctcctcatgcgccggcgtgctgcgcgagggcttccagcggcagcgcgtggcggcagcgctgcacctgtgcctgctcgacgccggagcgccgctttttgcgaccagcgcgcctgcctggcgacagcagcgctggctcgacaaggtggcgtaaggcgccatcgcaataaagacatacctcttaaggcgagattgccaacccgccccacggaatgaatactccttctgagttttttcgcccgtgcacgcgcgggctgtgttcgggcgtagaagggcatagagcctcgggggccgattcatgatccatattgctgtcatcacccggcaaggcgccccggcggggcaggccattgccgccgatttcggccccaacgggggcaccatcggacgtgcggacaccaacacgctggtgctggtcgatcccgaccgcacggtgtcgcgcgtgcatgcgcaggtgctgtgccgcgacggccagtatttcgtcatcgaccgcggcagcaatccgatgcagtgcaacggtgtgccgctgggctcgggcaaggaggcggcgctcaccgacggcacgcagctcgtggtgggaagcttcgagcttcgcgtgcgcgcggtagctggcgtcgcacctccgtcgctggcggtgccgaacacggtgatgaaagcagcagcccccgcatccacggcagcggtgtcgagtgacgatccctttgcggacctgctggccgggcttgcgcctccgccgccaccgtcgggacctgccgcctcgcccagggcgcctgccgctgcttcggccgcgtccgccgactcgctgctgttccccgatccgatgcaaagcggctcgcgcaatgcgcaagccgcgcagatcgatccctttgccaatctgctggggcctgcgtcttcttctccatcgccgtcgtcggcaccgggcacgaacttcggtgcgctcgatgatttttcggacctgggcgcaccgcccgcgcaaggcaaggccgccggcatcgacgagctgttcggcggcatgggcggtggaggcggcatcggcggcgatccgctcgcgctctctccgctggccgacccgctgctgcaacccaacacggcctcggacgccgatccgctggcggcgctgcagcgcgccgcgccggccaccccggtgccgcgcgcggatcacctccccatcgaccagttcggcttcacgccgccgaaggcgatcaccgcgcctccgccgccgccaccacccgccacgccgagggcggagctgccgcagttcgacgacatcacgggccagccgatccgcatcagcgggccggaggtttcgctgctcgacccgatcgagccgttgccgcaaccggcgcctcccgcgccgcggccgcagccgcaatcgctgccgcaatccgcggcagcgccagccgccaaggctgcggcgccggcagcgcagcgcatggcctctgacgacgaactgctcgccgccttcctgcgcggccttgccagcacgcaccagccgcccgagatgctcacgcccggcctcatggagcgcatcggctcgattcttcgcagcgccaccgagggcacactgcagctgctgctcacgcgccaggagttcaagcgcgaggtgcgcgccgaggtcaccatgatcgcgtcgcaggccaacaacccgctcaagttctcgcccacggtggaggtcgcgctcgcgcacctgctgggcccgggcgtgcgcggcttcatgccacccgaagccgcgatgcgcgatgccttcaacgacctgcgcgcccaccagttcggcgtgatggtgggcatgcgcgcggcgctggcgcacgtcatcgcacgcttcgagcccgaagaactcgagaagaagatcgcttccaggtcggcgctcgacgcgttgttcagcgccaaccggaaggccaagctctgggaccagttcgtggcgctctatggtggcatcgcgagcgaggccgaagacgacttccacaacctcttcggcaaggcctttctggaggcctacgaagaacagatggcgcgcttgaaagccgacgtgccgcccgctggcaactgacccccccgacacagaagcaaaaggcactccgcttggaaatcgaaatcgtcacgctgtcccggcagggcggccgcaactacaacgaagacgtgcatggccactggcacgacgagcgctatgtcgcgtgcctggtggccgacggcgcgggcggccatggcggcggcgacgtggcggcggccacggcgcgcaccagcatgctggccggcttctcggccgcgccgagcctggacgaagcgagcctgcgcgcgctggtcgagcaggccaacctcgacgtggtcgcgcggcaggccgaaggcggcaagctggccggcatgcgctcgaccatcgtgttcgcggccatcgacctggagcagcaggtgctcgcctgggtgcacagcggcgacagccgggcctacctgttccgcggcggcgcggtggtggcgcgcaccaccgaccacagcctggtgcagcagatggtggcagggggcatgctcgacgaggagggcgcgcgcctgcacccgcagcgcaacatgctgctgtcggcgctcggctcggtggaagaggcgcccgacatcacggtgtcggaccgcatgcgcctgttgcccggcgacgtgctgctgctgtgcagcgacggcgtctgggagcccctgggcgacgaagcgctggtcgacacgctgcacgcttcgcgcacgcccagccagtggaccgaactgctcgacacgcagatcaagtcgcacgccaagcccgggcacgacaactacacggtgctcacgctgtgggtgattgcggacgacggcgatgcgacgcgcctgctgccggcgggcggcgaagtgacgatgccggcgggcctggaaccgactgaaaagccggcggactagacgcgcagtgccgcgtctgtccgtcggcaggcgttctcagagactcagggcttcttgggccggtaggccttgagcgtgcccgtcacggtcacgtccaccgtcaccaccaccagggccgattccagcttgccgttgtcctggcgcttcatctgcttgcgggtggtggtcgaggtcgagttgcccttccagcggatcgtgctcgaacgcaccgcctccttgttccccatgtagttctgctccagcaccgtgatggcgccggtgcccgggttcttggagaggatcgaggtgtggtgcgggtggccgaccgtcacggtgggactgtccacccagcccgagtcgtcggaaaaggtgacgtcggtggtggtcgtcgtcgtcatctcgtagtcgcggtactggaggatgtcgccgggcagggcatccttgagcgcgacctcgtcgccccagacgtagtcggcgtcgtcgcccatcggaccgaagtccgacgaggtgccggcgccggcctggagcagggccttgttggccaggtcccagcattcgcccgcgccgatctgcttgccgacctgtgcactggcccactgcagggccttggcgttgagtgttgccatcgcgtgtctccggctcgaaggttgttgaagcggcctccggccgcgagcggcagccggagacgcgcgttcagaccttcttgttggccgcgatgtcccagccggtttccttggtgccgtcgccggaaccgtcggacttctggggcgtgtactcgtacttgaacttcgagaagttcagcgtgacggtttcggtgaggcggtcttcgccgccgctgccgccggtgtggacgttgctgacgatgatgtcttccatcgtgagcttgatgtattcgagcggcgtggcaccggccttgcggaccaccagcgtgcccttcttgatgtgctggccgttgcagcagtccagaagcagcaggtgcgaggaggaatcgacgtacttggtgaccgagagatcctgcacactcaccttgccggcgcccgaaccgccgcccacgtggccggtgccggattggctcgcgccccagctccaggcgagaacgtcgatttccttcttgtgcgaatcgtccttggattcaccgtcgacgccttcgagcttcaaaaacatgtctgcagccatgatgcttacctttcagttgtgtgagtcagaaaaagacagggcttccgggcggtgcgagagcgttgttgcccgggagctatggagagaacgagcgatgagcctggttttcaaaggcccaccaaaggcatatgccgccggttatttgccgcccttggcggacggcagcttggacaccaggcgcagggagacggtgaggccttcgagctggtagtgcgggcgcaggaagaacttggaggtgtagtagccggggttgccctcgacctcttccaccaccacctcggccgcggccagcggcttgcgggccttggtttcctcggacgagttgaccgggtccccgtcgacgtagttcatgatccatttgttgagccagcgctgcatgtcgtcgcgctccttgaagctgccgaccttgtcgcgcacgatgcacttcaggtagtgcgcaaagcggttgcaggcaaacaggtagggcaggcgcgccgccaggttggcgttggccgtggcgtccgggtcgtcgtattccgcgggcttgtgcagcgactgggctccgatgaaggccgcgaagtcggagttcttgcggtggatgagcgagagcaagccggccttggagagttcggcctcgcgccggtcgctgatggcgatctcggtcgggcacttctggtccacgccgccatcgtcgctcgggaaggtgtgcagcggcaggttctccaccgcgccgcccgactcgatgccgcggatgcgtgagccccagccgtagagcttgtaagaacggttgatgttggtggccatggcgtaggccgcattggcccaggcatacttgctgtggtcggcgccggccgtgtcttcctcgaagtcgaactcttccaccggattggtgttggcgccgtagggcgtgcgcgccaggaagcgcggcatgcacaggcccaggtacttggcgtcgtccgattcgcgcagcgaccgccagccggcatactcgggcgtcgagaagatcttggtcaggtcgcgcggattggcgagctcctgccacgactccatctgcatcaggttggagctggcgccggtgatgaagggcgcatgcgcggaggccgcgatcttggccatctcgcccagcagctcgacgtcgggcgggctctggtcgaagtggtagtcgcccaccagcgcaccgaaaggctcgccgccgaactggccgtactcctgctcgtagaccttcttgaacagcgggctctggtcccaggcggcgcccttgaatttcttgagcgtcttgctcaggtccttcttggagatgtccatcacgcggatcttcaggtgctcgtccgactcggtgttgttcaccatgtagtgcaggccgcgccaggcgctttcgagcttctggaaatcctcgttgtgaagaatcgcattgacctggtcggtgagcttcttgtcgatggccgcgatcatggcctggatcgacttggtcacgtccttgccgatgaccgtgctgttgctcagcgcctgctgcgcgagcgtgagaacggccgcctcgacggcgctcttggcctcgtcgctgcggggtttgaattccttttgcaggagcgatgaaaagtcgcttcccgcgtacgcaacgtccttgagtgcgctctgctgctcgagtgcttctgccatgatgctttctcctggtggtccggtggtgttggtcaggcggcgggcgcggtgccgtcttcgggtttcttgctggcagccagggtggccagcagcgccgggtcttccagcaccttggccagcaggtcttcggcgccgcccttgccgtccatgtaggtcaccaggttcgacagctgcgtgcgcgcttcgagcagcttgctgagcgcatcgaccttcttcgccaccgcggcgggcgagaagtcctccatgttctcgaaggtgatgtcgaccttcaggtcgccatcgccggtgagggtgttgggcaccgagaacgccgcgcgcggcttcatggccttcatgcgcgagtcgaagttgtcggtgtcgatctcgagaaacttgcgatcggctaccggtgccagcggatcgaccggcttgccggagaggtcggccagcacgcccatcacgaagggcagctggatctttttctcggcgccgtagagttcgacgtcgtactcgatctgtacccggggcgcccggtttctggcgatgaatttctgactgctcttggccatggaagtgctccttgcgggtgtgaatgggacgggtcgataaaactggcaaacggaaagaatgaggcgggcttattcggacgggcgcttgccggtcacgttctcgatggtgtccatcgcgttgggcgcgaggttggccatgatctcgaggaagctcacgccaatgagcttcttcgcgcgctcgatcagcagcggcgccggattgccgggctcggcctgttcgagatagcggatcacgcggtcgagcatctgcacggcgtcctgccggttctggatctcgccgcgcgcggcggccgagcgcggagaagccgcgccctgcgtttcatcggggccggcatcgccggcggcgtccacctcttcgggggcgccgctcgcaaggctgcaggcccgctgcagcacgcggccaatgctgcgcagcggggcgaggtcgacggcgtcggcgcggccggtgcgctcgaccagcagcgcctgcaggcgctccaccagggcgggcacgctcacggccgcctgcaggagttcggggcgctccgcctggatcgcttcgaggccgccctggatctgcgacatcgaataggtcggatcgccgccgacggcggtcagcgcgttgctcgcaatggcaatgtcgcgtacgcggatcgggccgacaccgggcgccacgcccacctgcgcgtcgtacaggtcgcgcagcaccatgttctcgtcccacagcggtgccagcgcgttgaggcgcatcgtggggtcgttgtcgtcgtcggcatcgagcgttggatgtatgccgtcccagaagcggtcgaacaaaccgatcagcaattgaaggcccgcgatgaagccggccacgccctgcagccgcgtggaggcgcgcaagagcagcaccgcggcgcgcacgtccttgctccggcgcaggatcgcgtcggactgttcggccacgtcgcgccactccggctccaccgccggtatgacggtgtcgccgaactgctgctcgggcttgccctgcgaggacgccgccagcgcggtaaaggctgcgtcgtactccaggtcgtcgccgcacggcgatgcctcgccgatgggcgtgagcagggcttcgacaagttcgttggtcagcatgttgcctgttcgagttggctggtgataatcaaagatgcgtcggaaccggtcaatgcaacgaagggaatagcatgcgcacgctgggtacacaccattcgtcctatggacgcactcctgccgcggtttcgcggcgccttgcactggcctctggcctggtgttgacgggtgtgctgctcgcaggctgcgcacccaagcccgtggtcacgacggtgtcgatcacgctggctgcaggtgccgatgccaaccccgatgcgcgcggccgcgcttcgccgctcacggtgcgcgtgtatgcattgaagtcgcccggcccgttcgaaggcgcggatttcttctcgctgttcgaaaaagaccaggccacgctgggcgcagagctcgtgcagcgcgaagaaatgctgctgcgccccggcgagacccgcaagctcgatctcaccctgccgcccgatgccaaggccattggcgtcatggcggcgttccgtgatctggatcgtgcgcgctggcgcgaagtgcgccccgtgcaaaccggcaaagcccaggccatgacggtgaccttcggcgcccgccagatccgcgtcgaaagcaaatagccccgcgcgcggagcgttcatgggggtgccgcgcttccgctcgaagccgcaggccggccgggccgcacgagcggctggtcggccggcaggaagtgcgcgaacagatcgttcacgaacgcgccgccggcggcccctgatgcagcggccgtgaagtagaggccgcgccaccgaagcccgcgcgaaccccggccctggctttcgaacaaggcgtccgccacctggcgcagcgcgggttgcagcgcccgcatcgcctcgacgaattcatggatcgcaagccggcccgaagcgctcggctgttcgcgcagcaacgccatgcgcagcgcgtgcaattgccgcgccatggggtcgaacaaggcatcgagccgcgcggccgccgcgtcgttgccgccatgcggctcggccagccgatggccgatggcttgcgccagcacctcgggaggcagcgcgccgcgcagcgtggcatagccggccagctgttcgaggccggtcacgacgaggtagacgggcaactgcaggcgcagggtgtcgccggcctcttcgagctggcggcgtatccgggccgcgagtggcttcatcgttccggggtccgcgcgctgcagctcgctcgcggcgacgcacaccaccagcccgttgagcggcaggcggtcgcgccgctcggccagcgccagcaacgcctgcaaccagaggccgcgcgtgtgcggcgccgcggccgcttcgctgacagccgtcggatggagttcgatggcggccatcgaaccggtgagccaccagcgccagtacggttcgccgaaaggctcgctgcccgaaggcacgagccgctcggcgtgcgccgccgccagcaggcccggcagattggccgccgcgtcgcccaggaagagaaaccacggcgccgggccgctgcgctgccgcggaggctggcgcagggcctgacgggcctgcgacatggcatcgcgcacggcttcgacggcggcctcgtcggtttcggcggccggcgggcccagggcatcgattcgccgccgcagtgcgcgccgccgcgcaccgcggcccgcgtcgcgcacggtgccgtacagcagcatgaagccgatcaggcacagcaacagcagcagccagaagagaagggcgggcgacggcgcggcggtcatggcgatggcttggcggttcttgcttcttctcagcgcgcggcggtgtcgagcgacacgaaatccgcgatcagccggtctccgcccttgttggcagcgagtgcctcgcgcaggcgcagcagataggccgaggccagttcgaaaggcggccggtcggcggtttcgttgaacggcgtgggggacgagagcaccgtgatcagcacgctgccgaagggcggacccacgagccagctggagggcacctcgcggcccagctcgagcttttcgccggcgcgcagccgcgtggccacctggccggcgttcaggtgcatgaccgaaccatcgaccgtgtagtagtcgacccacaggtagctgtcgtggttcggtgccgccacctgcacgcgcacgctgtcgccttcgcgcagctggccgttccgggccgtgagggcttccacatccagtccgtaggccttgtcgcggtttcgcagctggtagggcttcaggatggcgaacacctcgcagtgcggccacaggcgcagctcgacgtcgaacgcgggcgacttgacccccggcatcgcggccacctcgtgctcgactcttttcaggtccgcgggcagcgagacgaagccgctcacgcgcaggttgccgtccttgtccgcggcggccgcgaggtcggcgcatgcgtaggtctgcaggtgctgctcgatgcgctggcccaggctcggctccaccgcggccgggccggccggccacagccaccacagcagatagacaagcggcagcagcaacgcgagcgcggcgttggcgcgcagcaatgcgcggtcgcggcgccgcgtgtcgtgcggcccgggcgggtccgccacgcggtagggttgcggcgtgatgcggtcctgcaccaggctgccgagcgccagcggccgcagccgcagctggcgcgcgtgcaggtccttcagcttgccgagctcgccccggtcgccgttctcgaagtaatactggcccttgaaaccatgcaccagcgcatgccagtagacctcgcgcacctcgtcgtcctgcgcggtcagtgccgacaggtgatggaagaactcgctgtgcgcgttgttcgaattgaagagttgcacctgcagcggtgcggcactgcttgccgccgcgggatggcgcgccaggatctcgtcgatccaggccaccatggcaaaggcggccgattcgacctgcggcgcgggcgtgtccgatgcggcggcacaggcgcgcgccgcatccagcaggtggcgggcctgttgctgcgcggcgtcatgggagagcgtgctgcggccggcggcaatcgatgcgtcgagagccaggccgaatgaaaagaatgccgaaaaacagtcgagcagccgggccatgaaccgcgcccgttcactgcgcttgcatggcgagggatgccttgcaccggcgtctgcagcgatggcacatgcgcatgtccccggttccttcgaataggcgttcattcttccaaacgcggcgcggcgggcgccatatcgcttggggtctatgccgttcgtcgggcaaaccggccttgctgtgcggggcaatcgccggtatcttctgcttccgctgagttcaatgcacgctgggactgggacatgccatgaaaattctgatcgccgacgaccaccggctcgtcatcgaggcggtcaaagccaagttgtcggagctcgagcccggcatcgagttcgtcctggcgatgagcgtcgacgaactgcttgccggtgcaaccgacgagctcgacctggccctgatcgacctcaacatgcccggcgccgacgggcaggcccacatcgacgaaatccgccgccgccatccggccgtgcccgtcatcgtgctttccggctacgaagacccggccatcatgcgcagcgcgctcgaacgcggtgtgctcggattcattcccaaggcgtattcgcccgaggtcatgctgtcggccgtgcggctggtgctggccggcggcgtctacgtgccgcccatgatgctgacggcgctgccgccgggcatcgtggccggcgtggcgcccacgcagaacggcgaggcgcgctccccgggcgcatcatcggcaacgctggagcacctgcgcagcgtgctcaccgagcgccaggtcgaggtgctgcagctactctcgcagggcaagcccaacaagctcatcggccgcagcctcggcatcagcgaaggcacggtcaagatccatctggccgcgatcttccgcgcgctgaatgtgcgcaaccgcaccgaagcggtggtggctgcgcaggcgctgaccgaggcgcagcaggcctaagccgcgcgcagctgcgcggcggcctcggctgcgtcttcatcgccgggttgacctcccgctgccgccaacgtcctcttctgcgcaatcgcttcagcaagaaactccgcatcgcgcgccacgcccgagaagcggcctgaaccccaggtgtgcagccagggcaagcccaaaaagtagaggccgggcacggccgtgacgccgcgctggtgcaccggcgagccacgtccgttgaacaccggcgcatccacccactcgaagtcgggcgagaagccgatgcaccacagcacgctcgtgatgcccgcctcctccaggttgagccgcgtgcgttcctcgggcggttcccacaccggcgtgtagaccgaaggcggcggtgcctcgatgtcccgggccgcaatgtgcccgtcgatcgacgcgttgatgcggttgtagacgctgtccgcgcggtcgaggttgtcgcgcaggttgggcttgaacgcgagcacgccgccatccaggccctcgagcaggccgaagagttccatgccctccagtgcgaagcgccgcaggtcgatgtcgcgcccgccgtcgcggccggtcacgtagtggttggtgttgtctcgcacgccttcgcgcagcggatgctcggtcaccggcatgtcgtaatacttcatgtcggcgagccagtcgaccacttcgcgtccgcggtagaagcgggcgcagcgcggtgcgtcgccggtggccacgtagaccttgcgtccggccaggtgcaggtcttcggcgatctgcgcgcccgattgtccgcagcccaccaccagcaccgcgccttcgggcagctgcgcggggttgcggtactgcgccgagtggtactgcaccacgctcgcgggcaacttctcggccaggcgcggcacgatcgggcggtggtagccgcccgaggccacgacgacctggtcggcggtgtagctgcccgcatcggtctgcacggcgaagcggtcatggcttcgctcgcccgtgcccggcacgcgcgacacgcgttcgaccgtgacgccttcgatggccggcgccttcacctgcgcgacgaagccggccagccattcgttgatctggtccttcaccatgaagccgtgcggatcgtcgccgccgtaggaccagcccggcagctggcactgccagttgggcgtgaccaggcagaacgagtcccagcgctgggtgcgccagctgtgcaccaggctgcgcttctcgatcacgaggtggtcgatgccgcgctgctgcaggcagtggctcagcgagagtccggcctggccgccgccgacgatgatgacgctgtagtggctgcgcccgccatagggataggacatgggattcttctttctctggaggaggggagacatcagtcgaaagcgacgacggtgacttcggcgttggccgcatcggcgaagcgcgcggcgatgtgctcgatctcggcgagctggtccatggcctgcgaacacgcgaagccgtacttggcgcgcacgcgttcggaggccatggcgagcgcttcgcggctgtgctggagaaaatcgtcgagcgcatagcgccggccgggcgcaaggaagtcctgcaccacggaagagggcgagtagcagcgtgtttcgctggcatcgggccagcggacccggaagtgcatcacgggcatgcgagcgcctcctgcggcggctggatgaaggcatcgctgccgaagtcccacagcagggcctcctcgccgccggcccgcaatcgcacctgccgggtcgcatcgacttcgccgaccaccgcgcaggcgatgtcgcgcgcggcgaagcggctcagcacctgcgccacctgcgccggcgccacgctgagcacgaagccgtagctcggaaaggacgagagccagcgcatcggcggaactcccgcgggcctgggcagcgcatcgatgtcgatggttgcgccgacgcccgagcattcgagcagcatcatggccgtgcccaccgcgccggccatgctgatgtccttggcggcgcggctgaggccgtcctccgcaatggagggcagcacttcgaggtcggcgcgcagccgcgcggccggtgccgaggtcgatgcattccagtagggaaagggctcctcgtaggcgccgcgcaggtcggccgccatcaccagcaggtcgccgggcttcgcatcgaagctcgtcagaagccgccgcgcatggccgaggatggccaccgccagctgcggccgttcgctgcggttgttgctgtggccgcccaccaccggcacgccgtaacgcaccgacgcctccgccatgccgcgcagcacgtcgtcggctgggctcatgccggtgctccacagtgcatcgaccaccgccgtcggtcggccgcccatcgcatagatgtcgctcacgttgaccatcacgccgcagtagcctgcgaaccacggcatgcgcacaatgaagtcttccaccatgccttcgatcgcgaacagcaggtagccgccgtggccgtcgggaatggccgcgcagtcgtcgccgatgggcacggcctgtgccagcgccgcgtggccgcccggcagcgagcggccgagggccgacaccacgtcgctgatgtcgcgcttgtgcgcaaagccgcgcgaggcgcgcagggcttcggcaatggcgtggacattcgtcatgacagcaccttcgcgcgcgtgacgaagccgctcacgggatcgtggcagggcggatagaagtccaggtcggcctgcatgcgcgcatgcgggcgcccgtggatcgaggtctcctcgagcatctgccagcccagcttgcgaaagagcggcacgttctgcatctgcacctgcgcaagaaaggtgctgcagcccagcgcgttggcgcgcgacaccgcgagccgtatcagcgtggcgcccaggtggccctggctgcggaaggcgggatgcaccgcgaggcgcgagccccaccattcgccgggtgctgcgccgcgatggatgcgcaccgtgccgaccacctgttcgggcatgccgccgttgcacgacatggccgccagcaggtgggcatggccgtcgatggcatcgcggtcgtcgcgcgcgaagatgccctgctcgatgcagaacaccgcacggcgcagggccatggcttcgtcgcgctcccactgctgcgcggcttcccgcaccaggtattcgactggggcgtagtgcaggtcgagttcgctgaggtcgtcgatgcacagcatgttcagctttcgctttctttttcgtagatcgagagcgacgagcacgcgccgcacttgccgcagccggccttgatgtcggccgaccgcaggccggcattcaccacgcgctcgccgagcggcgcgagcaccgatctcatgaactccggcgaaggcgcgggatggtcctcgagcggcgtgccgctgatcggcacgaagggcaccacgaagggatacacgccgcgcgcgagcaactggtcgcagatgtcgaggatggcttcgcgcgtgtcgcccaggccggccaggatgtaggtgctgacctggccgcgcccgaacacgcccaccgccgcctcgaacgcgctcatgtagcgcgagatcggcaccgtggccttgcccggcatgatgcgttcgcgcacctcgggcgtgaccacttcgaggtgcatgcccagcgtgtcgatgcccgcggccttcatgcggtggaaccactggtcgtcgtcgggcggctcgcactggccctggatcggaatgtcgaccgcggccttgattgcgaaggcgctctcgcagaggatggccgcgccgcggtcggtggcgttgggcgtgccggtggtcatcaccatgtgcttcacgccgtcgagcagcacggcggcgcgcgccacctcggcgagttgttcgggcgtcttgcgcgcgatggtgcggccggccgcgagcgactggccgattgcgcagaacttgcagctcttcttgcggctctcgtagcggatgcaggtctgcagcacggtggtggcgagcacgtcgcttccgtgcagcgtggcgatgtgcgaatagggcacgccgtcgaaggtctgcatcgcgtagaagcgcggctgcttcggaaagctgatgcgcgcaatgggaatgctgccgcgcatcacgcggctcatgccctctgcatcgggcgcctcggccgtgaagggcgaatgccaggcgctggaggtgtggaccggcaccatgatcgtgtggccgtccacggtcacggccttgtggtcggaggggcccgcgccgccgcggcggctggccgcgccggccgaaggatcaaccagccgcaacccgaaggactggagctcggtcatcagctgccggctgtccggcggggtcgtcgtggcgatggtcatggtcggggctccgtggaacggtgggggtggggaaagcggcatgcatgggcacggtggtctctgccggccggtcgttgatggcgagggacagcagctcgggccgcgcgtagtggccgaccgaatccatcattcgcttgcgcttggcgatcagcgccatgtcgaggtcggcgaccaccatgccttcgccctcggtgagcggcggcgccaggtgcttgccttcgggcgagacgatggcggtgtggcagccgccgcgcagcgccttctgcaggttggcatcgggcgtgacgctgcggatctgctcgtcgctgagccagccggtggcgttcaccacgaagcagcccgactcgagcgcgtggtggcggatggtcacttccatctgctccgcgaagatcggccccaccagcgagcccgggaattgcgcgcagtggatttcttcatgctgcgccatcagcgcgtaccgcgcgagcgggttgtagtgctcccagcaggccagcgcgccgacgcggccgacggcggtgtcgaccaccttgaggccggcgccgtcgccctggccccacaccatgcgctcgtgataagtgggcgtgatcttgcggcgcttgagcagcagcgtgccgtcggcgtcgaacaccagctgcgtgttgtagaggctgccgtggtcgcgctcgttcacgcccagcaccacgaccatgtggcgcgcacgcgcacgttcggccacggcctgtgtgaccggccccggcacgacgaccgcgcgctccgccagccgcaggtgcggcgcgccctgcagcaccggcggcagcacgaagctgaagtaggggtagtagggcacgaaggtttcgggaaataccgccagctgcgcgcccttggcggcggcctcgtcgatggcgccgcacacccggtcgagcgtgccgtcggggcggtcgaagtcgggcgcgatctggatcgccgcggcacgcacgatgcggggtggggaagccatcgctcgggtcccgccttacagcgtccaggtgtcgaggatgaccgcgccggccttcttgtgcagcagcacgatgtccagcacgtcgagcggattgatcggcttgatgccttcgatgagcgcgccttcgccatggccgtacagcgcctgcagcgcgaagcggcaggcgtagaccttgccgccttcttccatgaacttgctgatctgcttgttgaagttctggtggcccggaaaggcctcgtcgcccagcgtcggaaagccgcgctgcacgcccagcgtcacgccggggccgtagagcaggaccgacgtctcgtagcccttgcgcctgagccgcgtggcctgcagcaggttgacgaagccgatcgagccctcgaaggccaccgtgtggaaggtgacgagcgctttctcgccaggctcggccttgacgtcttcgaacaccttctcttcgtagtcgacgaggaactcgcctttctcgttgcgggggcgggtgactttgggcatggggtactccggttgaggggttgaacgcaggtcttgcgtgtcctactcttcgcaggcgatgtgccagcgcccggagcggggcgtgcgatcaacgcgcgatcaacacgcggcggcgcgggccgccagtggatagaaattttttcggcacccgaaaagaccggtgcgcaacccttcggcaaggcgctctccgcaccggaaagacgcatccgccatgcgatcaatgcacccgatcaatggggttgatcgcacctgatcgaagcattcggttcctatggagcgggcgcgattcctgcgtgccgaccggtggctggatgcaatcaatggatgcaatcaactcctccgatgaatacgatcaccacccactggcgcaagcagctgcgcaacaccaccaggcccgcctacctgttgctggccgagctgattgccgacgacatcaagaccggacgccttgccgtgcgcgaccgcctgcccacgctgcgcgaactcgcggccgacctggggctcaactacacgaccgtggcgcgcggctatgccgaggcgcgcaagcgcggcttgatcgattcgcgcgccggcaccggcaccttcatccgctcgggcagcccgagcctgcggctgcgcggcggcagcggggccgagatgaccatgaacatgccgcccgagcccgacgacgagcacctgatggcgcgcctgcacgacagcgcaagcagggcttttgcaggggcggacctgcacgacctgctgcgctaccaggacttcggcggcactgcgcacgaccgcgaggccgcgatgcgctggctgcggcctttcgtgcccggcgcgggcatcgatcgcatcctcgtgtgcccgggcatccacagcgtgctcacggcgctgttctcgcagctggcgcggccgggcgagctggtctgcgtggagtcgctcacctatccgggcgtgaaggccatcgcggcgcagctgggcgtgcaactgcaggcgctgcagctggacgacgacggccccattgccgacgccttcgagcacgcctgcaagacgctcaagcccaaggcgctgtattgcaaccccacattgctgaacccgaccgccggcaccgtctcgcgcgcgcggcgcgaggcgctggccgacgtggcgctgcgctatgcggtgccgatcatcgaggacgacgcctacggcatgctgccgcgccagacccccgccgcgctggccacgctggcaccggggctcacctactacgtgagcggcttctccaagtgctttggcgcgggcctgcgcagcgcctacgtctgttcgcccacggtggtccagtcgcagcggctggccggcgcgatgcgagccaccaccgtgatggcctcgcccatcaccaatgcgctgaccacgctgtgggtggaagacggcaccgccgaggccatgctgcaggcggtgcgaagcgaatcggcggcgcggcaggcactggcggcacgccacctgggcgccagcgggctgcaagcgcatcccgaaggctttcacgcctggctgccgctcacgcccggctggagcccggtggagtttgcctcctacctgcgcacgcagaacgtcggcgtggtggcgagcgcggcgttttcgaccgatggcgatccgcccgatgccgtgcgcatctgcctgggcggcccgatgtcgcgcgagcagtgcgaccaggcgctgcggctcatcgccgacacgctggcgcatccgctgcatccgcacgccacgttgcgcggggtgtgaaatctccgcgaatgactgctgcccggatgcgcccctttcctacgcaagtcagtgcttcgaacgtccagtctggcggtcgagcccatccattctttttcaccaccgaaggaggccatggacaagcccgatggaggcgagtccggtgtgtcgcaccatgcacggccctcttgattgcgcgcttcagagtctccagcagcttgcctatgcacgcatcgcgcgggaattccttcgcgccaggcagcaggggccggatctgctttcgccctacgacatcctgatggacgaggcgcaccgccgggtgctgcactgggagcgggtgctcgcggagttgcggctcctgatcgacgatccgcgccagattgcaagagtcaaggtcaggcgagcgctctatctgcgcatgttgctggaaagcgcacccatgcgcctgcaatcgtggagcgacagcgacagcctcggcaccatgccgaagtcccacttgttcgaatggatttcctacgacttcgagcggcttgaactggccgaactggaaggctccatgtcgccggaggaagccgcgtcctacacgcaggcactcgacgcgcgggccagcagcatgcgcgaggagtgagcgggctgcgctgtcagccccggcccagcacgacggcgccctcctggatgtagcgatcgaattcgatcttgggaatggccgcggtcagcgactggccgccttcctgccaggtgaccacgacgctgtcgtcggccatgaggatctggcagttcccctcggggatcttcaggttcggaccgtcgcccgcacggaactcgacagtgcccacgatacggccgtcaatctgcgtggtggaagtcataggaatcctcgaaaagaaagaacgctgcaaacccttttcttccgcatgccggtgcgccgctgtaggcagggacagcattcccgcgccggttgcatgcctgcgagcgattcgctcgcagtgcaggaacgagccgaccctggctgtgcccgaagaacgcttacagcggacgtcgggcgaaaccgacaccggcccctgttcgctcgaccaccatttcatttggaaccagcgcattgcggctgcctcccggcacccccttttgctggcgatttttcaacccgcctcgatttcaacgaggcccatgaatgaaggagtcatgacatggccaatttcacgaacactgccgacaccgccaccaccgaagacgtggtcaaggtgctgaacgacctgctcgaaacctcgcgcgacggtgaatacggcttccgcgtttgcgccgaggaggtcgactcgccgcagctcaagcaggtcttccagggccgctcggccgattgcgccaaggctgcgggagaactggtccagctcatccggcgtttcggcggttcgcccgacgaaggcggcacggtgaccggcgccatgcaccgcggctgggtgcacgtgaagggcgcggtgggcgccaacagcgcgcactcgatgctcgaagagtgcgagcgcggcgaagacgctgcggtggcgcgctaccgcaaggcgctgaaggccgatctgccggccgacgtgcgcgccctgatccagcagcaggccgatggtgccaagcgcaaccacgaccagatcaagcagttgcgcgatcagacgaagaagtcgtgatttgacgaagagggacggctccgcaccaactcgcgaccgtccgggatgcgcgccctgttgcgcctcagttggcgcagcgggcctcgagcgcatcgaggaaggagcggtcccaccggccttccttcatggcctggatcgtgcgggcctccgtggccaggtgcgcatgggccttctcgatgagcaactcggcttcgtcgcgcgcgaaggccatcaggccgtcctggtcgcccaccacgatgtcgccggggttcaccaccatgccgcccaccgagacgggcacgttgatctcgcccgggccgtccttgtacgggccgcggtggttgacgccgcgcgcgtacaccggaaagtcgcgaccgcggatctcggccacgtcgcggatggcgccgtcgagcaccacgcccacggtgccgatggttgcggcatagaacgacaggatgccgccgatcaccgcattggtcacgtcgccgcccgcatcgatcacgagcacgtcgccggggcggcagaactcgaaagcccgcatcatcgtgaagttgtcgccgccgcgcgtcttcacggtgactgccgtgcccgccatggtcttgtgtcccgggcggtggtagggctcaaggccgacgctgccgatgttgcggtgcatgttgtcgctcagcgcggcgaccgggatgtcgtgcagcgcggcgatgatctccggtgccacttgcggggccgacgggttcttgcggatggctttgtagggcatgggtgttgtcctcggtaattcaggcacgcttcagcgcagggcggccacggcccgcgcgatgcgcgcgcagccttcttccagcgtctcgatggcggtggcgatggaaagacgaaagtagggcgacagcccgtaggcggtgcccgcgaccacggccacgccctcgctctccagcaggtacatcaccacgtcgccgtcttgttccaggcgcttgccctggggcgtggtcttgccgatcaggccgccgcagtggacgtagaggtagaaggcgccgggtggcggggtgcagcgcaggccggggatgtcgttgatgagcgcgagcgtgcggtcgcggcgctgcttgtagaccgccacgctctcggccacaaaaccctggtcgccattcatggcggccgcggcggccgcctggctcaccgagcagcagttgccggtggactgcgacagcagcgtgtccagcgcctggaccagatccgccggcccggccgcatagccgatgcgccagcccgtcatcgcataggtcttggagacgccgttgaccaccagcgtgcgctcgcgcagcgcgggcgccaccgcgagcagatgcggcgtggcctggccgtcgaagcggatgtgctcgtagatgtcgtcggtcatcaccatcacgtgcggatggcgctgcagcacctcggccagcgcgcggtattcgtcggccgtgtagctggcaccggtcgggttgctgggcgagttgatcagcagccagcgcgtgcgcggcgtgatcgcggcctccagctgcgcgggcgccagcttgaagccgttggcttcggggcaggccacggtgaccggcgtgccttcgcaggccagcaccatgtcggggtacgacacccagtagggcgcgggaatgatcacctcgttgcccggctccagcgtgatcgcgaaggcgttgtagatcgcgctcttggcgccgctggtggcgatgatctcgttcagtgcatagcgcaggccgttctcgcgttccagcttggcggcgatggcctgccgcagctccaccgtgccggccatcagcgtgtagcgcgtcgcgcctttctcgatggcggcggccgcggcctgccggatgtggggcggcgtgtcgaagtcgggctcgcccaccacgaggttcacgatcgacttgccctggcggcgcagctcgttggcgcggtcggcggccgatgtgctgggcgagggcttgatgcgccgcacgcgggcggcaatgcgggacgtggtcacgtgacttcctgtgtctgggattgcatggaccgaacggtacgcagatcgaacaggcgaggccaagacgacttttcactggtcgtataggcgcagcttatggtgagcgcctataccggccatgcgggggcggtgctaggctcggcttttgcttgggggacaaggcgtgaacctgcgacgcctcaaatatttcgtgaagatcgtggacatcggcagcctgacgcaggcggccgaggttcttttcatcgcccagcccgcgctgagccagcaactggccacgctcgagggcgaggtgcgccagcagctgctcgtgcgcaccaagcgcggcgtcacgcccaccgaggccggcaaggtgctgtaccggcatgcacagatcatcctgcgccagtgcgagcaggcgcgcgtcgacatggaagcggccggcgaagggctgtcgggccaggtgtcggtcggtcttgcgcccggcacggcggcctcggcgctctcgctgccgctgctgcgcaccgtgcgcgcccgccaccccggcatcctgctctacctgaacgagaactacggcaccacgctgagcgagctcatcatgaacggccgcatggacctggccgtgctctacggcgacaaggccatccatggcctcagcttccagccgctgctcaaggagccgctgttcctggtcgggccggccgcgatgccggcgccggcgcagccggtgaagctggccgacctgcgcgacatcgagctcttcctgccgcgcccctacaacgtggtgcgcaagctggtcgatgcggctttcgtgcgtgcgggcatggtgccgcgcgtggtggccgagatcgaatcggccttcaccctgacggcggccattgccgacgggctgggcgccaccatcctgccggcatcgatggcgcgcgaagtggtggcgtcctgcggtgcctggcaattccagatcgtcgacccggtcatcgaggcgccgctggcgctgtgccagtcggaccacctgccgctctcggagccggcgcaggcggtgaagagcatcctgctcgagctggtggtcgacctcgcaggcacctttgcggccacgcccgaacccggtctcgccgcgctgtcgtaacgtgccgtcataagccggccttatcccggcacagccattccgtcttgggctttgcgcccgcggcccgttacctttcatgcctgccgtcacgcgttcgcggaatgcgtcggccaccaaggatgttctgtcgccacaggcaggcccggcatgaagcaggaacagatcaagacgctcatcgacgcactcgccgcatcggatcttgcggagctggagtacagcgaagacggcagcacgctgcggctggtgaagcagtcggccctgagggccgcgcccaccgcgcggcgcccggccgctgcgcgccaggcgcgcgccgcggtgtccgcggaaccggcgctgccggaggccgccccggccgaatgcctcgcgccgctctacggcgtggcgcacctgcagcccgcccccggggagccgcccttcgtgcagccgggtcaggccgtcgaggccgggcagctgctctgcgtgatcgaggccatgaagatgttcaacgaagtccgcgccgacgctgccgccaccgtgcaggccgtgctggtgcggtcgggccaggaagtggatgcggggcagcccctgttccgcttcggttgaggaagggcgcgcgatgttcgataccgtcctcattgccaaccgcggcgagatcgccttgcgcatcctgcgcgcctgccgcggcctgggcctcaggaccgtggtcgcgcattccgaagccgacggcgaagccagctacgtcgcgcaggccgaccaggcgctgtgcatcgggccctccgcgccggggcagagctacctgaaccagtccgccatcctcttcgctgctgaagtcagcggggcgcaggccatccacccgggctacggcttcctgtcggagaacgcgggttttgctgcgcgcgtggaagaggccggcctggtcttcatcggccccagcgccgcctgcatccgcaccatgggcgacaaggtctcggccaagcgcgcgatgcgcaaggctggcgtgccctgcgtgccggggcccgacgaaggtctgcctgaagacccggccgccgtgcaggccatcgcccgcgagatcggctacccggtgatcgtcaaggcggcgggcggcggcggcgggcgcggcatgcgcgtggtgcacgacgaggcggcgctgctgaacgcgatggcattgacgcgcgaggaagcgcgccaggccttcggcaaccccgaggtctacatcgagaagttcctgctgcacccgcgccacgtcgagatccaggtgctggccgacagccacggcaatgccgtgtggctgggcagccgcgactgctcgctgcagcgccgccaccagaaggtgatcgaggaggcgccggcgcccggcatcgacgacgcgctgatggccgaggtgggcgagcgctgcgccgccgcctgccggcagatcggctattgcggcgtgggcaccttcgagttcctctacgagaagggcgccttctatttcatcgagatgaacacccgcctgcaggtcgagcacccggtgaccgagatgaccgccggggtagacatcgtgcagcagcagttgcgcatggcgcgcggcgagcgccttgcgctggcgcagcacgaggtgcgatgccagggccacgcgatcgagtgccgcatcaacgccgagaaccccgagacctttgcacccgcgcccggccgcatcaccggctggcaggtgccgggcggcttcggcgtgcgtgtcgattcgcatgccaacgccggctaccgcgtgccgccttactacgactcgatgatcgccaagctgatcgtgcacggcgccacgcgcactgatgcgctcgaccgcatgcgcttggcgctcgccgagatgcgcatcgacggcatcgccaccaacgtgccgctgcaccgcgaactgctgcgcgacgagggctttgccgtcggcggcgtggacatccatcacctcgaacgctggctgcagcaaaggaatgcggcgtgatcgcgcagcgcccatccctcagcctgctgggcacgaccgcgctgctcttcgaggcgcccggcgagatgaacctcgactcgcagcagcgcatctgggcgctggcgcacgaggcacaggcctggcctgagattcgcgaagccgtgccgggcatgaacaacctgatgctgaccttcctgcgcccgccgcgcggcctcggcgcgctcgaagccctggaggcacgcctgcgcgatgcgtgggatgcggccatcgcgctgccgcgggagggccgggtggtcgagttgcccgtggtctacggcggcgcgggcggtccgcacatggccgacgtggtggcgcacacgggcctcagcatcgagcggatcgtcgagctgcacagcgcgccgctctatccggtgtacgcgctcggcagccatccgggctactgctacctgggcggcatggacgcgcgcatcgccacgccgcgccgcaaggtgccggtgctgagcattccgggcggcgcggtgtcgatcggcggcgcgcagaccggcgtgtcggcctcggccgggcccagcggctggaacaccatcggcagcacctcgatgtccttcttcgatcccgcgcaggacccgccggcggcgctgcagccgggcgacatgatccgttttcgcgtggagggcatcgtccgatgatcgaagtgctttcatcggcggcgctcgccaccgtgcaggacctggggcgcaccggcagcctgcgctggggcgtcggcacctcgggcgccatggacaacctggcgctcgcggccggcaacctgctgctgggcaatgcgctcgacgcggccgccatcgaagtgccggtgtttcccttcaaggtgcgcttcggcgaggactgcgcctttgcgttgaccggcgccgattgcgcggcccggctggacgaccagccgctcttgccctggtgggtccaccaggcgcgggccgggcaggtgctgacgctgggcctgccgcaaggcggcgcgcagcgcggcagccgcgccatgctgtgcctggccggcggggtcgacgtgcccgaagtactgggctcgcgcagcacgcagctgcgcggcgccttcggtggccacgaagggcgcgcgctgcgccggggcgacgtgctgcgcgcggcaggcgcgggcgccgcgtgcaagaccggcttcggcctggtgccgcccgcgctcgcactgccgctgcagcagggcggcgtggcggcggtgcgcgtcttgccagcggccgaatacatgggcttcgaacccgcgtcgcgtgccgccttctgggccggcgaatggaagatcacctcgcagagcgaccgctacggctaccgcctggagggcgaggcgctgcgccccatcgcgccgatggaactgcgctcgcacggcatcgtgccgggcgtgatccaggtgccgcacagcgggcagccgatcatccagatgcgagacgcccagccctcgggcggctaccccaagttcggcacggtgatcgaggccgacatgtggcgcctcggccaggcgccgatcggcagccgcgtgcgcttcatcgaaaccggctgggacgaggccgtggccgccctcgacgaagtgcgcgcctggctcgacaaggtggcgcgcatggtggaactgcaccgcggcgcacccgcggcaaggcgctgacatgcaagacgtcgtgctgcaagccagccagttcgccgcgtggctggccgacacggacatcggcctgttcgaattgcgcacgccgcacggaagcttgcggctggggcggcagggcgacgacatcgtggttctgccggcatccgatgcgcgagaggccgctgccgtcgagccagccgtggtccgggcgccctcggtgggggtgttcctgcacggccacccgctggccggcgcaccgctggctcgcatcggcgagcacgtgccggccgggcagaccgtcggcctgctgcagatcgggccgctctttctgccggtggtcacggccgaggccggcgagattgccgccatgtgcgttggccatggcctccctgtcggctacggcacgccgctggtcgaactgcatttgcatcccctctgacgagcaaggacaccccatggacatcgacctgaatgcagatctcggcgagggcttcggcccctggcgcatgggcgaggacgaagcgctgctggacatcgtttcttccgccaacgtggcctgcggctttcatgcgggcgatccggtcatcatggaccgcaccgtgcgcatggcgcgcgcgcggggcgtcgacgtgggggcgcacgtgggctttccggacctgctcgggttcggccgccggccgatgcagatcgagccgaaggaactcgtcgcctacgttctctaccagctgagcgcgctggacggcatggcgcgcaccgccggccaccgcatgacgcacatgagctttcacggcgcgctcggcaacatggccgcggccgatgcggcgtttgccgaaccgctggtgcgcgcggtggcggatttcgatccgacgctcatcgtcagctcttccgccagccgcgccatcgaggatgccgccgcgcgctgcggcctgcgcgtgcgcaccaccttcctggccgaccgcgcctgcgacgacgacggcctcctggtgccgcgcaagctgcccgattcggtgatccacgaccggagcgcggtgctggcgcgcgtgcgccagctgctggaggagggcaccgtcaccagctacagcggccggaagatcccgatgcgcgcgcattcgatcctgctgcacggcgacacgcccggggcggtggacctggcccgggccgtgcgcggcgtggtcgagcaggcggggcgcgtggtgcccatctcgaagcagtcggaccaatagccacagaaagctccggagcccggacatggtgcttaccctaggtcgtacgcacgaacacggggcaacataagggcggcttatcgctccacagccaatccgtcttggcgccgcgaagaagcggtcgatacagtgaattcaacgcaaagcagcgatctccagttccaacgaaagaaacaaagatgccgttctctgactacaagaccgcgctggtgacgggggcctcctcgggcatcggcgccgccgtcgtcgaacgcctctgcaaggaaggcctccaggtccatgcgctggcgcgcagcgccgacaagctggccgacctggccgcgcgcaccggctgcattgcacacgccatcgacgtgagcgacctcgccggcatcacccgcctcacgcaggaggtggagttcgacgtgctggtcaacaacgccggcgtggaccgccccggctcgatcctcaaggccgacgccgagggcatcgacctgctggtcgacgtgaacctgcgcgccgtgctgcacctgtgccgcctcgtggtgcccggcatggccgcacgcgaccgcggccacgtggtcaacatcagctccattgcagcggcctacaacttcggcggcaacagcacctaccacgcgaccaaggcggccgtgagcatgctgtcgcgccagctgcgcatcgacgtcttcggcaagcgggtgcgggtgaccgagatctgtccggggcgcgtggccaccgacatcttcgcgcacgtgcacggcgactccgaagaaacctacaagcgcttcgtcgaaggctacgagctgccgcaggccgaggacatcgcgaacgccatcgcctttgcgattgcggcgcccattgcggtcaacgtgggccacatggaaatcacgcccacgctgcaggtgcccggcgggctctcgaccacgcggccggaagcgccgcaggcctgagtggcaccacgtccacaagccaggcaaaggaaccgcgcatgaaggacttcgacctgctggcgatcctgctgaaaccggagttcggtgcgatgctctggcacgggctgcaggagacgctgaagatcgcggccggttcctggctgctggccatggccatggcggtcgtgttgctggtcgtgcgcctcacgccgagccggctggccgaacgcgtggtggccggctatgtctcctatcaccgcaacgtgccgacgctggtgcagctcatgctctggtacttcggcatcttcagcctgctgcccgatgcgctgcagggctggctctcggcgcacaacgcggaaacgattctctcgatcgtcgcgctcggactctgccaggccgcctatttcagcgaagacatgcgctcgggcctgcgctccatcccggccggccaggccgaggccgcgcgcgcgctgggccatggctacatcggctcgatgcgccacgtgatgctgccgcaggccatccgcaacgcggtgccagcactggtgaaccacagcgtgtcgctgttcaagaacagcagcctggccatggccatcggcgtggccgagctgacccatgcggtgaaggaaatcgaaagccagagctttcgcaccttcgaggcctacagcatggcaacggtgctgtacctagtgtgctcgctgctcatcatggcggtgggcggctggctgtcgcggcgctaccgcatcgtgggagcgaggtaggccatgttcagcgtctttgaaatccttcgcgacaactggctactgctgctcatcggccagtatccgagcggcccgctcggcggcatcgtcgccacgctgatcctgtcggtgctgggcatcgtgctggcgtttccgctctcggtgctgctggcgctcgcgcggctgtcgccctggcgcctgctgcgctggccggccacggtgctggtctacgtggtgcgcggcgtgccgctcctgatggtgatcctgtgggtctacttcctggtgccgatcctgatcggtcgggatgtgtcgggcttcaccaccatgctgtgcacgctggtgatctacgagggcgcctacctgtcggaggtggtgcgcgccggcatccaggccctgcccaagggacagaccgaagcggcacgcgcgctcggccacagccacctgggcaccatgtggttcgtgatcctgccgcaggcgctctataacatgctgccgagcatgctgagccagttcatctccaccatcaaggagaccacgctgggctacgtgatcaacgtgcaggagctgaccttcgcggccaaccagatcaacaaccagctgctgaccaagccgttccaggtgttcttcatcctggcgatgacgtactacgtcgtctgcttcagcctgacccagctggcgctgtggctggagcggcgcgtggcccacaagcggctcggcgcagccactgcgaagacatccgaagacggtgtgtcgctgccgccaccggtggtggtgaatccgtaaggccgcgcccgacggccatcgacaggaaaacaaggagacagatccatgaaacccgttccacatcccgcaggggatgacaccatgatcctgttctccaacatcaacaagtggtatggcgactaccaggcgctcgccgacgtcaacgccgaggtgaagaagggcgaggtggtggtggtctgcgggccttcgggctccggcaagtccaccctgatccgcaccgtcaaccggctggaagaagtgaagtcggggcagctgctgttcgacggccacgacatccacgcgcccatgagcagcgcggcgctcaacaagctgcgcagccgcatcggcttcgtgttccagagcttcaacctgtttccgcatctctcggtgctggagaacatcatgctgtcgcccgtgcgcgtgctcggcgttaagcgggccgaggcgaaggcaagggcggcgcagctgctcgagcgcgtgggcctgtcgaacaaggccggcgcctacccggcgcagctttcgggtgggcagcagcaacgcgtggcgattgcccgcgcgctggccatggagccgcccgccatgttgttcgacgaacccaccagcgcgctcgaccccgagatggtgggcgaggtgctgtcggtgatgcgcagccttgccaacgacggcatgaccatgatgtgcgtcacgcacgagatgaacttcgcccgcgaagtggccgaccgcgtctggttcatggacgcgggccgcattctcgagaaggccgaccccgagacctttttcaccagcccgcagcatccgcgcgcgcagcgcttcctgtcggacttgcgcgcgcactgattgatcgtcgttttcttcatcccctcgaatttatccaggagtccagcatgtcgaacagaaccgctttccgtcttgccgccattggcgcctgcctttgcgccgcgcctttgctggccctcgccgaccagtggagcgacatcagccagcgcaaggaactgcgctgcggcaccttcgccgacgtgccgcccttcgccgcccccgatccgaagacgcgcgagatggtgggccacgacgtcgacctgtgcaatgcgctggccaaggaactcggcctcgcggccaaggtcacgccgttgtcggtggaggcgcgcgtgcccgaggtcaagctcgggcgcgtcgacgtgaccgtcgccaacctggcctacaccaagagccgcggcgaacagatccagttcagcgacccgtactacgtggccaaggaaatgctggcggtgaaggcttccgacccgggcacggccaaggccgacttcaagggcaagcgcctgagctcgaccaagggctcgacctccgagctgtcgatcaagatgaacggctccgagccggtcaccttccaggacacgggctcggccttcatggcggtgcagcaaaacaagtcggtcggcatggttgcgaacacgatgaccatcaccaagctggtcaaccagtcgaagaccgaaggcgtggcgctgaagatgatcaaggaaccgatggtgctgcagcccatcggcgtcggcatgaagaaggacgagccggcgctgctggccaaggtgaacggcgcgctctacgcgctggagaagtcgggcgagctcgacaagatctgggcgaagtggctcggcccgaacaccgaatacaagatgacgcgcgaagaaaaggtcatgccgctggcggaactcaagttcgaactcctgccctgaccgcgctcacgcccggcggaaagcatctccctggcgcccggcctccgggcgccagggatgaagggggttacttgcgcgcggtgacctcgggcatcgccgaagagtggtggtgagcgatcagccattggccgttgacccactcgtagacgtaggtgtagcgggcatgcactttcttgccgtccttgaacttgaaggtgtaggtgccgacgtcctgcgccacgttgcaaccgatcttgatgatgcggtggtcgatcgtgccctgcggcgcgtccttcaggaacttgacgaagtagtcgcggacctcggccggattggtgcgcggctggttcgagacggtcggcagcagtacgccgtcgactgcgtagttggcaacgaccttgtcggcatccagcgtgcgcagcgagtcgttccagcggtcgaacagcgccgcgatctgcggctcggtcgctggcacgcagatccccgctgccggcgtctgcgcaaaggcagaggttgaaatggcgaggactgccgcggtggttgccgagagggagagcgtacgaagcacattcatggagttttccttttgcaatgggtagtcaatcgccggcatcaccggcgctgcatcgtcttgcgatacaggacttcattcttcggtctctccatgaacgccaccggggcttcgcgatgaaccccgggtgacgcgcacatgaatatcggatgaaccgcctcagcccggctccgcgtccagccgatagcccaggccgcgcaccgtcttcaacaacgcaacgggatggccgtcgtcgatcttggcgcgcaggcgacgtacatacacgtcgacgatgttggtgagcggatcttcgttcgtgccccacacattggaaaggatgcgctcccggctgtagacacggccgggcgccgccatcaacagttcgaggaaggcaagctccttggccgtgagcgggacgagcttgccggcacgggtcacctccatgcgctcccggtcgagaacgaggtctgccacctgcagcgtggtggcccttggcctttgctcccggccgcggcgaagcagggcctcgatgcgcgccaggagctcctcgaacgcaaagggcttggtgaggtagtcgtcggcgcccaggcgcaggccgctcaccttgtcctcggtgttgctcaacgccgtgagcatcaggaccggcacatggttgccttcggcgcgcagcgtctggcacagctccaggccgctcaggccgggaagcatcaggtccagcaggagcacggacagctcgttgctgcgcgcgagttcgaggccttcggggccggtgcgcgccagctgcacgcggtaaccctcggcgctcaggccccgcagcagaaagtcggcgacgcgcgcgtcgtcttcgacaaccaggatgttcatgttcgttgggtccggacggaaaattggcacggcagttcgatccgcaccgtggtgccgtgcgagggaatgctagcgatgtcgatgcggccgtgatgggcatgcacgatggcctgcgcgatcgacagcccgatgccggtgccgtcggcccgatgaatgcgtgcgcggcgaccgcggacgaagcgatcgaacaccttcggcaactcgtcctcgtcgatgccgatcccctcatcggccaccaccacctgcacgcggccgtcgatcagctgccagctcacctgcaccgtcccgtcactgcgcgaatagcgcaccgcgttgtcgagcacgatgacgagggcctgccggagacggtcggcatcggcctgcagcgtgaccgcgggcgcctcggcgccggggggctcgagctgaacgcgaacgttgtgccgcgcacccagcgcctcggccatttcggtggcgtcgcccagcagctccgagaggtcgaccgcgtcgacgtgcatcgccagctggtcggcctcggccttggcgaccaggagcaggtcgtcgatcacgccggtgagctgcttcacgccacccacgatgcgcgtcagcgtctgccggtactcggcaagcggcttgtctgcgccgcgcagcgcgatctccgcctcgccgcggatggccgtggccggcgtgcgaagctcgtggctgagatcggcgagaagctggcggcgccgctggtcgatctgttgcagggtttcgtgcgcggcgctcagctcgctggtgcgctccagaacggcctcctcgagccggcggcgcgcggcatcggcgtcgagccggtgccgctgcagttcggcggccatcgcattgaaatgttcggcaacccggtcgaactcgtcgcgcgaacccagcgcgatgcggtggtcgagtgcgccggcccgcaaggcccgcgtgccttcgagcagacggtccagcggccgctgcagccgctggttcaggtacagcgccagcaggacggcggccgccagcgtgagggccgcgaggccgatggcctgctggcgcaattggtccaggccccgctcggtcgccgcgcgggcaaccggcatcacgttgcgctgccgctcgatggcgccgttgatcaactcgcgcagatcacggccgcgtgccttgtcgaagacttcgttcagctcctgccagacgctggcgaactcggcgccacgctccagcggtgcgagtttcagcagtcgggcgcggaccgcggcgatgttgtcgttgagcaggtcgctgacggcgaccagctcgacgacttccggcgggatgggcacgccttcgcgttccgcgatcccgccccacagggaaaggtcgcggcgcgcgaactgcctgagcgtttccgtgctggcctgcatgcgcgccagctggctgtcgcgcacctcgggcgatgcgttcgcacccatcagctgctgggacgcccagacccgcagccgctgcttgctggccgagagttccagcagttccgacaggatgtcgctggccagccggctgtgctgggcgtagtcgttgacccggttcgatccccagtagacgaagccggcctggatgcagaccagcgcgacgagaacggcaaatgcgagggaaaggcggagtcggaacatgaggcactgtagcggcgcggtgcgggcttctgcatgaacatcagatgaacgttctcgtccagcgcggattggccggcatcgttccgcgccctggtcacggtgcagtcttgctggtgcgggctcgcgtgagattcgtgggtgccacgccgaaacgatgcagcacattgccgagcagttttccgaagagcgggtcgctgccgatcacccaggccgcgccgactgcgcccgcatgaaacacgcgcccgccttgcggccgctcccaatagatcatttcggccgagagtccgtcgagcgattcggtgagcctcgagtagtagtcgagataggcgtccgacttgcccgggacgcgccggatgcccttggcgatgacttcgatgccctcttgcgcgacgggcagggaagcgcccgtggggagccgcttcgtcatcttcgcgaggctcgagagggtcaggtcccactcgtgcccgatggcgcgcggcaacccgccgccgggcgcgtggccgaaggtttcgcccttgccgaggcccagcggctgcggctcgttgaagagcgcatgcgccggcagctcgacgtggtagacgccgaagtcgtcgccatcggcgaaggcccaacccgcggtttcgaggccgatgatgccggcggccggccggcccgatgccttgagccgtccgccgcgcgcccagtcctggctgtggtactgctcgccgaacgcgcctgccggcgggccgacgggcggcctggcgtcgtcgtgatcgggcccgttcaccttccgctgttccatgacggtgaagtcctcgtcgtagctcacgcgcaggtacatggtgttgcccgacagcacgaccgcgctgccgccgcgcctcaggaaatcgtccagcccctccacgccgggcagcgaccagtattcgctgtggccgttgatgaagacggtcttgtagcgcgcaagcagagacgggtcgcggtgcaggtcgatgtcgccgatcacgtcgtagtcgtagccctgcttgtcgagccacacgtgcaggtggcgttcgagccgcgtccactggctgaagccgctcgcggccgggtcgtagagcgcattggggctggcattgggccagggcatgcgcaggccgacctggtagcagggctggccgtggcggtggtagacgtagctgctgtaggccggcgcttcgggatggctgttctccaggccctccgaacggcgcggccacaccggatcgtcgaccacgttcttcgcgaatggcgtggtggcgtaggcgagccagctgttgaccgcgcacagcacgaggatgggggccggcgccgcgtgcgccggcttgcgcacgatgaaggtgatgtcgtaatccgccttgcggccttcgatgtcgaagcgcgcgcgtccgacgtacacgcccgacctggcgtcgccgggaacgcggaattcgtgcaccgcgtcccagcggcaatcgtagagatcgtcgccggcaaaacgcaggccgtgcccgcgcgtcggatcgtggagcgggtcgtagggagattcgtcttcttcgcagtggcctaccttgccgggctcgaaggccgggccgacgatcatccaggttgcgtggttgacgatgcggccggtgcgttgatgcccgctggcatcggccacttgcgacccgcgctcttcccgcagcggccagcaggcgagcaccgaacggcccgttgcgatctgcaagccgcgttgctcgcggcgcgcggcaatttcgccggccgacagcgcccggtcgtacagcgccggcatgacgaggtcggcctcgaggaacaggtcggcctggccgtcgatggcgcttgcgccgagccgcagcggcgcggtggcgggctcgacggcctgcagtgcgggccactccgccacgcacaccccatcgatgcagagcgtcgcgaactcgccgttccacgtggcggcaatgtgctgccaacgacgcgtcgcgagccggccgtgcgatggcgcggcgttgtctcccaggtggaacgacagcgcgccccctggttcgatgaagagcgcaaagccgcggtgcgcgaggtcgtcgtgctggctgacgatggtctgcctgacgtcgaccgtccagggcttgatccagcattcgaagctcaatccgcgcagcggcaggccggccggcaaaccacgttcgacatgcacgtaggagccggggtggatcggctgaacgcgcgcccgatgcggcgcgaacgcttcgagcgccacgtcgtcgctgcgtccttcgacgtcgctgcccagccggcagaccgcgaattcgtaaggcacgtcgctgctgacgtgaaagcggacgagatcgcccgccgccaccgtcttggcatcggcgtagccgtggaggccgggcagctgcagcggtttgtgcggcgggatcgggtgcggggcggtcgctgtcattccgacgtgaagcccgaggccttcaccaccggtccccagcgcttgatgtcgtcggcgatgagggccgagagttcttcgggcgtgctcggattcggatcgctgctgagcttcagcagccgttcctgcacgtccttgttggcaagcgccttgccgagtgccgcatgcagctggtcgacgatgggccgcggcgtgccggccggcacgaagaggccggtccattccaggttgtcgaagtgcggctggccgagttccttgagcgtcggcacgtcgggcagcaatgcggcgcgtttggcgccattcaccgccagcaccttgagcttgcccgactgctggtgcgcgacgagatcggcaatgggaatgatgccggccgagatctggttgccgagcaggtcttgcaccagcggcgccgcccctcggtagggcgcggccacgaggcccgccttggcatcgctgcccaagcggtagcctatgaattgcgcgacgctgcccggagcgggcacgccgtagttggccttcttcgggtccttggcggcaatgtcgagccattgcttcacatccttggccggcagctccgcggggacagcgatgcctacgtagaagctcgcgatgcggccgacgggcttgaagtccctgaccgggtcgtagcgcaccgacttcgtggtgagcggcagcatgaccatcatgtgcatgttggcgagcaacacggtgagtccgtccgccggcgccgtgcgaacgtagtcggccgcgatcgcgccgcccgcgccggtgcggttgtcgacgacgacggtcgtgccgagttcggcggccagcttgtcggcgagcgtgcgtgcctgcacgtcggccgagccgccagccgggtagccgacgatgagcttcagcgggccgtgcgcggtgttgatctgtgccgcggccgcggcggcgaaggccaatgcggcgcaggcgagcgtggccctgagagtgaacgagagcttcatcggaggctttcctgggtggggttgcgaaatcggtgcggtcgccgggttcagtgcgcgaggcccttgcgtgcgatctcgtcggcgagatcggccagcgacttttcgagcaggtcggccagctcgtcgatctccgtttcggtgatcgtgagcggcggcgtgatcatctggaaatcgccgaaagcgccgaggttcgcccggcggttgtagagcgcgatgccatgcttcaagccgtgctcggtgagccgcgcaggtgcgttgaaagcgaccggcagctggctgcgcgtggccttgtccgagacgatctcgatggccgtgagcaggcccttgccgcgcacgtcgccgacgatcggcgagtgcgatgcgatgtcgcgcaggcgtgccatcagcagttcgcccatgtcgcgcgcgcgggtcacgaggtcttgccgcacgacctcgtcgaccaccgcgcgcgcgaccgcgcacgacagcggattcgtgaagtaggtgtggccgtgcacgaagccgccggcacccgcaatcgcatcgaccaccctgttcggtgcgagcaggcaaccgagcggcgtgtagccggcggccaggcccttggcgagcgtgacgaggtcggggcgcgcgccctcccagtggtgcgcggcaaggaaggcgccggtgcggccggcgccgctcatgatttcgtcgaagatcaccagcacgccatggcggtcgcagatctcgcgcacgcgctggaagtacgccgccgaggaaaccaccgcgccggtcgagaggccgccgatgggttcgaggatgaaggccagcaccgtctccgggccttcgcgcaggatggtttgttcgagcgcgtcggcgcatgccttctcgtgcgactcgaccgtatggccatcgggcaagcggtatgacaagggcgccggcaccttgggcatcgggcggaccatcgggccgtacaggttgagcgtgttggcatcgcccgtgaccgccagcgcgccgagcgtcgagccgtggtagctcggatcgcgcgagatcaccttcgagcggctgccctggccggtcacgaccgcgtactggcgcgcgagcttgatcgcagcctcgttggcctccgatccacccgatacgaaaaatgcgcggtcgaagccttcgcccgcgagtccgcagacgcggtcggccagcgcgatgttgtgctcgctctcgaaaaagcgcggatacgcgaaggtcaccttcgatgcctgttcggtcatcgcggccagcacgcgcggattgccgtggcctatgttcgcgacgacggcgccggcggttgcgtcgagatagcgcttgccgttcgcatcccacagaaagatgccttcgccgcgggcgacgcgcggcggacgggccgaccccttgggtgcgtagaagccgaggacggagccgcccttgggctcgtcaccgatccgggcgatgccggtcgcgggggagttcgaggtgttcatgacccgacgatacgaatcgcggccgctttgcggtagacgcatggagtgatgaagtgctatacgttcgccgtatgaagcacgtacatgaccggctcgacctgctcgacactttccagaagatcggcgagagcggatcgctcagcaaggcggcgcggctgctgggcacgacgcagcccacggtcagccggcggctgctcgaactggagcggctgctcggctgcaagcttgcgctgcgcacgaccgcaagcttttcgctcaccgacgaagggcgctcgctgctcgtcgaggcccgcgacctcggcgaccgctggtcaggcctgtcgcaacgcctgaagggcgggcagagccggcccgaaggcacgctgcgcgtgatcggcccttcggggtacggaacgggcttcctgaccgacgcggtgaccgacctgcgcgcggcacatcccgcgttgcgcgtcgaactcacgctgaccgatcgggtgctcgacctgaccgcatggggagcggattgctgggtctgcgtgggcgaggtgcgcgatcctggattggtgagccgcaagctcggcacgatggaacgcgtgctgatcgccacgcctgaattgctcaggaagctggggcccgtcagcatcgcgcgcctttcgcagttgccctgcgtcgggctcgtgccctacgtgaccggcaacgtgcgcatgctggatcgatcgggccgctcccgcatggtgatgctcgacacgccgatccagaccgacagcctgctgtcgagctaccgcgcgattctcaatggagccggtatcggcgcggcggccccctggatgtgccaggaagacctcaagaccggccgggtgcagcgtgtgctggcgaactggtggctcgaacccatcgccattcatgtcgcgctgcctcccggcatctacaggcccgcgcgcgtgatcgcattcatcgaggccctcaaggcaaggatgtttgccctttccgggttccggccatcggcctgaacaggccaagccggggtcgcgccgcttctgtccatggtccggggtcctcgacatgctccgaactctgcttttcgatgttctgtaaagtgacggatggttttcgcaactccattcgcttgtcttgaactctattagcttcgaccccacccgcttcgatgccgccatcgtcgatctcgacggcaccatggtcgacacgctcggcgattttgcggtgtcgctgaaccacatgctcgccgacctctcgttgccgccagtggctccggcagccatcgagaaaatggtgggcaagggttcggagcacctgattctttcggcgctggcgcatgtgatgtcttccagcgaaggcgccgcggcgggtgccggcgcggaggcgctgcaggcacaggcgcaagcgctgttcgaccgggcctgggagcgctaccagcaccactacctggccatcaacggacagcactcggcggtgtacccgggcgtggtcgaggggctcaaggcacttcggtcgcgcggcctgcgcctggcctgcctcaccaacaagccgacttcgttcgccaagccgctgctggccaccaaggggctcgatggcttcttcgagttcgccttcggtggcgatgccttcgcgcgcaagaagccggacccgctgccgctcttgaagacctgcgaagcgctgggcaccgttcctgcgcgcacgttgatgatcggcgactcgagcaacgacgccaaggccgcgcgtgcggccggctgtccggtgctgctcgtgacctatggctacaaccatggcgagccggtgcgcggcgtggatgccgacggcttcgtggattcgctcgccgaactcgatcgcgcggcggcctgagccggaaggccgcggctacggctgctttccgagcagcgcgtccttcagtttccagtcggccggcacggggccgagccagatgcgcagcagcgcgttgaagaaggcctgttccttgatcgggtcgggctgcgccacgccgcgcacggtgatcaccgtgcccgtgccgggcagccagtcgatggtgaaggtgtcgccggccttgagctgcttctggtcggcgaacatctggcccatgcgaagcagccccggaatgaggttgaccatttcgctcttgggcgagttttcttccacgcccttggtgaagagcttgccgagctcgttggcctcgatgtcgcgcaacatggtgattgccacgcgcttggggcccggcgcggccagcgcttcttcgggcgtggagactttcttgcccaagtagaaccccgccgcgtagaccttgaacacggccttgtagcgcacgcccgcgccattgagctgcagggtgctgccgcgcaggtcgagggtgtcgttcagcttgacgccggccacgtcgacctgggcggccgaggcgccgagcacggccgaagcgaaggccagggcggccaggcgggagaacgacggggtcgggagcgaaggtgcggccaaaggatctcctcgatttgcgaacgatcgtgctaatgtatcttttcgttctaccccgtccccctcgggggaaccctgaagcgagctgttgcacgcggcggcgttttcgtgggctaaactccacgttccatgttcgttcatcacatcattcaaacaggtgaaggcagccggggagcctggccctggcgtcgccatacatcgctgactgtttgattgcacggcgcacgccgtgcgcccgcggtaccggatcgctcatcgactccggaccaccagtgaatgaccttgccaccggccgaactcgagcgccggaggcaattggagaacgaatccgtgatcaccgaacttgaattcaagagcctcagcgcccagggctacaaccgtattccgctgatggccgaggcctttgccgacctcgaaacgcctctttccctctacctcaagctggctcattcgcagggcggcggcaagcacagcttcctgctcgaatcggtggtgggcggcgagcgcttcgggcgctacagcttcatcggactgccggctcgcacactgctgcgcgcgtcgggcttcggcgccgaggccgtgaccgaggtggtgaccgacggccacgtggtcgagaccgccgcgggcaatccgctggattttgttgccgagtaccagaagcgcttcaaggtggcgctgcggccgggcctgccgcgtttttgcggcggccttgctggctacttcggctacgacacggtgcgccacatcgagcgcaagctcgaaaaaagctgtccgcccgatgcgctgggctgccccgacatcctgctgctgcagtgcgaagagcttgccgtcatcgacaacctctcgggcaagctctacctgatcgtctatgccgatccgaagcagcccgaggcctatgcgacgggcaagcgccgcctgcgcgagctgaaggaaaagctcaagtattcggtgagcgcgcccgtggtgaagcccacgcagccgcatccgcccgagcgcagctttgccaaggccgactacctcgcggccgtggagcgcgccaaggagatgatcgccgccggcgacttcatgcaggtgcaggtggggcagcgcatcagcaagcgctacaccgagtcgccgctgtcgctgtaccgcgcgctgcgttcgctgaatccgtcgccctacatgtactactaccacctgggcgatttccacgtggtgggggcctcgcccgaaatcctggtgcgccaggagaacaccggcgagggcgagcagaagatcaccatccgcccgctggccggcacgcgcccgcgcggcgcctcgctggagctcgacaaggcggccgaggaagaactcatcaacgacccgaaggagcgcgccgagcacgtgatgctgatcgacctcgcgcgcaacgacatcggccgcatcgccaagaccggtaccgtgaaggtgaccgaggcctttgcggtggagcgctacagccacgtgatgcacatcgtgagcaatgtcgagggcacgctgaaagacggcatgaccgccatcgacgtgctcaaggccacgttcccggccggcacgctcaccggcgcgcccaaggtgcacgcgatggaactcatcgaccagctggagcccaccaagcgcggcctctacggcggcgcctgcggctacatcagctatgcgggcgacatggacgtggccatcgccatccgcaccggcatcgtgaaggatcagatgctgcacgtgcaggccgcggccggcgtggtcgccgattcggtgcccgagctggagtggaaagaaacggaagccaaggcgcgcgcactgctgcgcgccgccgagttggtcgaggagggactggaatgagcaacgtaccggacatccagaacgatttctcgcacgaaatcatcggcgccgccgtcgaggttcagcgcgtgctcggcacgggcctgagtgaagacgcctacgccgcggccctggccatcgaactcgccgagcgcgagatcggctttgcgcagggcgtggcgctgtcggcgagctacaagggccgttcgcttggcgaggtgtatcgcgcggctttcgtggtcgagcagtcggtcatcgtcgagctcaaggcggtcgacgtgctgaccgacctgcaccgcgcgcaggtgctcgccgcgctgcggctctcgggcctcaagctgggcctattgatcaacttcaacgtgttccccgtcgtcaagggcgtgcaccggattgtgagcaagccatgaaactgctgatgatcgacaactacgattccttcacctacaacatcgtccagtacctgggcgagctgggtgcggatgttcaggtgcaccgcaacgacgagatcagcgtggcgcagatcggcgagctgatcgcctcgggtgtcacgcggctcgtggtgtcgccgggcccttgttcgccggcggaagcgggcgtttcggtggcggccatcaaggaattcgcgggcaagctgccgattcttggcgtgtgtctcggccaccaggccatcggcgcggccttcggcggcaagatcgtgcgcgcgcagcagctgatgcacggcaagaccagcgagatcacgaccacgcaggaaggcgtgttcgcggggctgcccgagaagttcaccgtcaaccgctatcactcgctgtccatcgagcgcgaaagctgcccgaaggaattggcgatcaccgcctggaccgacgacggcgagatcatgggcgtgcggcacaccggctttgcacacgacgtgcgcatcgagggcgtgcagttccaccccgaatcgatcctcactgagcacggccacgccatgctcaagaacttcctggattgaccagcatggctctcccccagccttcgcgcacttcttgtcgcttcgccaaccccctcgccgggggcaataccagcggcccggcagagccggttccgcggtattcccgctaaggatccaaagacatgtcgacctctcattccatcgtcgatctgcgcagcgacaccgtcacgcagcccaccccggcgatgcgcgaggccatgatggcggcgccgctcggcgacgacgtcttcggcaccgacccgagcgtcaacgcgctgcaggaaaagatcgccgcgctgctgggcttcgaggcggcgctcttcgtgcccaccggcacgcagagcaacctgtgcgcgatcctctcccattgcggtcggggcgacgaatacatcgtcggccagcaggcgcattgctaccgttgggaaggcggcggcgctgcggtgttcggcagcgtgcagccgcagcctctcgaccatgcgcccgacggcacgctgccgctcgcgcagatcgaagcggccgtcaagcccgacgacgcgcactttgcacgcacgcggctgctggcgctggagaacacgctgggcggcaagctgctgccttttgaatacgtgcaggccgcgaccgatctggccaggagcaaggggctgcagcggcacctggacggggcccgcctcttcaacgccgcaacggcgcaggcggcgctgaacaagcgcagcgacatccgcgccgaagcacgccgcatcgcgcaatgcttcgacagcgcctcggtctgcttcagcaagggccttggggcacccatcggctcggcgctggccggttcgcgcgagttcatcgcgcgggcgcaccgtatccgcaagatggcgggcggcggcatgcggcaagccggcctgcttgccgcggcggcttcgcatgcgctcgaccaccacgtcgaccggctggctgaagaccatgcatcggcccggcgcctggcggaggggctcgaaggcatcgagggcctgaaggtcgaggcgccgcacacgaacatcgtgttcgtcgatctcacgggcgcggcgcaggcgcgttcggcggagctgctggcgcacctgaaccagcagggcattcttgcgaccgggctctatcggctgcgcttcgtcacgcacctcgatgtcgatgccgccggcgtggaccgcgccgttgccgccatccgcggcttcttcaacgcctgaacctcgaggagccgtgcgatgcccgatctcccgcatctgctcgctttcatcgccgccggctggctgctgaacctcactccgggccccgacgtgctctacgtcgtgacgaattcgctgcgctccggcgtgcgcgccggcaccgtcgccgggctcggcatcaccgccggctgcttcgttcacatctttgccgccgcagtcggcgtcggcaccctgatggccacgtctgcggcggccttcacggtgctcaagtacgtcggtgcggcctatctgctctaccttggcgtgcgcatggtgctgtctcgcgcggcgccgcccgcagacctggacaaggccgcggccgcggtgagcggggaacgcagcctcaaggcgatcttcctcggcgggttctggacgaacgtgctcaaccccaaggtggcgttgttcttcctggctttcgtgccgcagttcatcgcgcctggtgcggacaacaaggccctgtacttcgtgctgctgggcgtgctgttcaacctcaatgcgatccccgtcaacgtgggctgggccgtggcggctggctggatggcgcgccgcggcgccgtgcaaaaaggcatgcactggctcgatcgcgcggcgggcgtcctcttcatcggcttcggcctcaagcttgcgttcacggacgcgccggcggttcgcgccggacactgacaaacacccaggagacttcccatgatcactccccaggaagcgctgcagcgcaccatcgagcaccgcgaggtcttccacgacgagatgctgcacatcgtgcggctcatcatgagcggcgagtgctcgcccgtgatgatggcggcgctgatcaccggcctgcgcgtcaagaaggaaaccatcggcgagatcacggcggccgcgcaggtgatgcgcgaggtgtcgaccaaggtgccggtgaaggacaccacgcacctggtcgacatcgtcggcaccggcggcgacggctcgcacaccttcaacatctcgacctgctcgatgttcgtcgcggccgcggcgggggccaaggtgagcaagcatggcgggcgcagcgtgtcgagcaagtcgggcagcgccgacgtgctggagtcgctcggggtcaacatcaacctgcagccggagcagatcgcacgctccatcgaagaggtgggcatcggcttcatgttcgcgcccaaccaccatccggccatgaagaacgtcgcgccggtgcgtaaggaattgggcatcaagaccatcttcaacatcctcggtccgctgaccaatccggcgggtgcgccgaacatcctgatgggcgtgttccaccccgaccttgtgggcatccaggtgcgtgcgctgcagcgcctgggcaccgagcacgccatggtggtgtacggtcgcgacggcatggacgaaatctcgctcggcgccgccaccatggtgggcgaactcaaggatggcgagatccgcgaatacgaactgcaccccgaagacttcggctttgccatgtcgagcaaccgcgcgctgcgcgtggaaacgcccgagcagtcgaaggccatgctgctgggggtgctcgacaaccaggccggcccggcgctggacatcgtgctgctcaacgccggcgcggcgctgtatgcggccaacgtggtcgattcgatcgccaagggcatcgaacgcgcacgcgaggcgattgcatcgggcgccgcccgggccaagctggccgaactcgtcaaggcctccacggccgtttgagccgcaacagattgctgggaacacagaacatgtccgacatcctcgacaagatcgttgccgtcaagcggcaggaaattgctgcggcgcaaaaaagaagcccgctcgaagcggtgcgcttcgacgccgagagccgcgtgctgacgcgcgatttcgaaggcgcgctgcgcgccaagatcgctgccggccacgccgcggtgatcgccgaggtcaagaaagccagcccgagcaagggcgtgctgcgcgaagacttcattccggccgacattgcccagagctatgccgagggcgacggcgagatcagcgccgcctgtctttcggtgctcaccgacaagcagtttttccagggcagcgtcgactatctgaagcaggcccgtgcctcgtgcgacctgcccgtgcttcgcaaggacttcatcgtcgacgcctaccagatctacgaatcgcgtgcgatgggcgccgatgcgatcctgttgattgccgctgtgctcgacgacgcgcagatgaaggactacgaagccattgcgcgcggcctcggcatggcggtgctggtcgaagtgcacgacgcggccgaactcgagcgcgcactcaagctcaagacgccgctcgtcggcgtgaacaaccgcaacttgcgcaatttcgaggtgtcgatccaggccaccatcgatttgcttccccaactgccggccgaccggctggcagtaacggaatcgggcattgccacgcgtgaagacgtggccacgctgcgcgcggcgggcgtccacgccttcctggtcggcgaggccttcatgcgtgccaaggaacccggcgaggcgctcgccgcattgttcaaatgagccggccggaccagctgtccagcagcgatccggccgactggcccgtggcaccgggctggcagccgctggtcgacgagtttttcggcagcgtcgtgggggtgaagctgcgcagcttcctgcgcgagcgcctcgatgccggcgccgtgatctttccgccgcaaccgctgcgggcgctggagctgacgccgcccgaggacgtgcgcgtcgtcatcctgggccaggatccgtaccacgggcgcggccaggcggaagggctcgcgttctcggtggcgcccggcgtggcgctgccgccctcgctgcgcaacatcttcaaggagctccagcgcgacctcggcacgccgcctccgccattcccgaatccgggcggcagcctggtgaaatgggcgacccacggcgtgctgctgctcaacacctgcctcacggtcgaggaagggcagcccgccagccattcgggccgtggctgggaagtgctgaccgatgcggtcatccgccatgtatcagccggcgagaaacctgttgtttttatgctctggggttcgcacgcacaaagtaagcgtgcgttgatcgatgttgggcgccataaggtgctgatatcgaatcatccgtcgccgctttccgcgttgcgcccgcctgcgcccttcatcggctgcggacatttcggcgaggcgcgtgcgtggcgggaggcgcgccaggcggccggctgaattcgcggataatccccgcagttccgcctcgtgcagttcctcacgcttcttcttggtgctgggggttctgtgtagtcacaaaaccgtgctatatttcgaggttcgccggagaggtggccgagtggttaatggcagcagactgtaaatctgccctcttacgagtacgctggttcgaatccagccctctccaccagcgatgaatttggtttctaagaaagagcgattggatctagcgctttgggtgccttggagtgcccccgatgcgggagtagttcaatggtagaaccccagccttccaagctgatgacgcgggttcgattcccgtctcccgctccagagacccggttcgacgccggaagcgattggttagacaaaagcccttttggctcagtggtagagcactcccttggtaagggagaggtcgcgggtccgattcccgcaaagggcaccagtttctgggggttgcaacagcaggtttgcaacccatctgcatacgttgaaatcgtttttttcggagtcgaaaaatggcaaaaggtaaattcacccgcaccaagccgcacgtgaacgtgggcacgatcggtcacgtcgaccacggcaagaccacgctgacggcggccatcgccacggtgctgtcggccaagttcggcggcgaagccaaggcctacgaccagatcgacgcggcgcccgaagaaaaggcccgcggcatcaccatcaacaccgcccacgtcgagtacgaaacggccaaccgccactacgctcacgtcgactgccccggccacgccgactacgtcaagaacatgatcaccggcgcggcccagatggacggcgccattctcgtgtgctcggccgccgacggccccatgccccagacccgcgagcacatcctgctggcccgtcaggtcggtgtgggctacatcatcgtgttcctgaacaagtgcgacatggtcgacgacgccgaactgctcgaactcgttgaaatggaagtgcgcgagctgctggacaagtacgaattcccgggcgacgacacccccatcatccacggctcggccaagctcgccctggaaggcgacaagggcaagctgggtgaagaagccatcatgaagctggccgaagccctcgatacctacatcccgacgcccgagcgcgccgtggacggcaccttcctgatgcccgtggaagacgtgttctcgatctccggccgcggcaccgtcgtgaccggcgccgtcgagcgcggcgtgatcaaggtcggcgaggaaatcgagatcgtcggcatccgcccgaccgtcaagaccacctgcaccggcgtggaaatgttccgcaagctgctggaccaaggccaggcgggcgacaacgtcggcgtgctgctgcgcggcaccaagcgcgaagaagtcgagcgcggccaagtgctgtgcaagcccggctcgatcaagccgcacacccacttcaccgccgaggtgtacgtgctgtccaaggacgaaggtggccgtcacacgccgttcttcaacaactaccgtccgcagttctacttccgcacgacggacgtgaccggcgcgatcgagctgcccaaggacaaggaaatggtcatgcctggcgacaacgtcagcatcaccgtgaagctgatcaacccgatcgcgatggaagaaggcctgcgcttcgccatccgcgaaggcggccgtaccgtgggttcgggcgtcgtggccaagatcctcgacatctaagccgagcgtaaagagtaccggaggggtatagctcaattggcagagcgtcggtctccaaaaccgaaggttgtaggttcgattcctactgcccctgccacctaggtggcgcctccgaaaaagccccgtcgtgcaccggcggaaggcaaaaaaagcccatcgcaacccgatgggcttcggcgtctcaaaaagacgcattgaattgaaggccgaaaggccacaggaaatcagccgaacatggccacttctcaaatcgaaaccgtgagcacgggtgccgacaaagccaaactggctgcggcggtggtgctggcagtgggcgccatcgtggcgttctatctgctgtcgcgccaaggctcgctggtgcaatgggctgcgctgctggtcggtctggccgcggccgtgggcgcattcggcagttcggagaatggccgccagttgtgggcctttggccgcgactcatggcgcgaggtcaagaaggtcgtctggccgacccgcaaggaagcgatgcagatgacggcttatgtgtttgccttcgtggcaatcatgtccgtcttcctctggctcaccgacaagacgctcgaatgggtgtttttcgacctcattctgggctggagaaaataaatgaccgctgatccagtgaacgcagttgacaccaccccgggcacgccggaagaagaaagcacttccgtgctggctcccgccgccaaccccgatctgcgttggtacgtggtgcatgcctattcgggcatggagaaggctgtcgagcgcaacatcaccgagcgcatcaaccgcgccggcatgcaggacaagttcggccgcatcctggttccgaccgaagaagtggtcgaaatcaagaacggccagaagcgcaccaccgagcgccgcttcttcccgggctacgtgctggtcgaaatgatcatggacgacgagagctggcacctggtgaagcacaccaacaaggtgacgggcttcgtgggcggcgccaagaatcgcccggccccgatctcgcagaaagaggtcgaggacatcgtcaaccagatgcagcagggcaccgagaagccgcgccacaaggtcgagttcaccgtcggcgaattcgtgcgcgtcaaggaaggcccgttcaccgacttcaacggcacggtcgaagaagtcaactacgagaagagcaaggtcagcgtgtcggtcatgatcttcggccgcgcaacgcctgtggaactcgaattcagccaggtcgaaaagacctgagccccttccggtcttcgggccggaaccatttccggctgcgcgttgtccgactcggcgcgcggccttgatcgaagagtcgttaaaccccggggagctgcggcgagagccaaggcgatatcacccgcaaggagcaaagcatggcgaaaaaaatcgtcggcttcatcaagctgcaagtgccagctggtaaggccaacccgtcaccacccatcggtcccgcactgggccagcgtggtttgaacatcatggagttctgcaaggcgttcaacgcgcagacccagagcgtcgagcctggtctgccgctgccggtggtcatcaccgcgttcgctgacaagagcttcaccttcatcatcaagacgccgccggcgatcaccttgatcaagaaggccatcaagctggacaagggttcggcccgtccgcacactgacaaggtcggcaagatcacgcgcgcacagctcgaggaaattgccaaggccaagatgaaggacctgactgcagccgatctggacgcagcagttcgcaccatcgccggctctgcccgttcgatgggcgtgaatgtggagggcgtgtaaatggccaagatcaccaagaagcaaaaagcgctcgcaggcaaggtcgacagcaacaagctgtacgccctcgttgaagccatcggcctcgtgaaggacgccgccaccgccaagttcgacgaatcgatcgacgtggccgtgcagctcggcatcgacgcgaagaagtcggaccaggtcgtgcgtggcgccgtcgtgctgcccaacggcaccggcaagaccaagcgcgtggctgtgttcgcccagggcgccaaggctgaagaagccaaggccgccggcgccgacatcgtcggcatggacgacctggctgccatggtcaaggctggcgacatgcctttcgacgtcgtgatcgctgcccccgatgccatgcgcgtggtcggtacgctcggtcagatcctcggcccgcgcggcctgatgcccaaccccaaggttggcacggtgaccccggacgtcgccacggccgtgaagaacgccaaggctggccaggtccagttccgcgtcgacaaggccggcatcatccacggcacgatcggccgtcgctcgttcgacaccgacaagctgcaaggcaacctggttgcgctgatcgacgcgctggtcaaggccaagccggcgaccagcaagggcgtgttcctgcgcaaggtggctgtgtcgtcgaccatgggtctgggtgtccgcgtggacacgcaaaccatctcggcgagctaaagagattggcccggctccgaaaggagcagggcgaatgtggtgggtcgcggcagcttcggttgccgtgagccatccaagaccgctggtgtgcagggttgcctgcacttaatagccggaccttttgtccggcaatcagcgcagatggcgaccccactgcaaggaatttgattttttgttcctaacagttggtcgctgcatgaagcgcgatccgaggccccggccgaaggtcgcattaaaaggagtagaccttgagtctgaatcgcagtgagaaagaagcggtcatcagtgatgtgaccagcctcgccgcaaaagctcaaacgctcgtgctggcggaataccgtggcatcacggttgccgatatgaccaaactgcgcagcgaagcgcgcagcaagggtgtgaacctcagcgtgttgaagaacacgctggcacgccgtgctgtcgctggtagcgcattcgaagtcattggcgaccagatgaccggcccgctgatctacggcttttccgaagacgcagtggccgccgccaaggtggtggccgacttcgcgaagaccaacgacaagttggtgattcgcggtggtgcgttcggcggcaaggccctggatgtgaacggcgtgaagcagctcgcaagcatcccttcgaaggaagtgctgttggcgcagttgctgggcttgatgcaatccccgatttcccgtacggcacgcgttctcgcggcgctggccgcgaagcgtggggaaggcgcagcagcacccgcagccgatgcaccggcagaagccgaggcgcagcccgcataagccggcttgcgtttgaaatattcaacccaattgttaggaaacaaaaatggcattcgataaagacgcatttctgaccgcgcttgacagcatgacggtcctggaactcaacgaactggtgaaagccatcgaagagaagtttggcgtgagcgctgccgccatggcaggtcccgcagctgcaggccccgccgccgcagtggccgaagaacaaaccgaattcaatgtcgtgctggccgatgtcggcgcgaacaaggtgtcggtcatcaaggccgtgcgcgaaatcaccggcctgggcctcaaggaagccaaggacctggtggaagccgctcccaaggctgtcaaggaagccctgtccaaggctgacgctgaagccgccaagaagaagctggaagaagccggcgccaaggtggaactgaagtaattcagaccccctagagggctggaggtgcctgaaaaggccctccagcctttgccgctttcagagcgcacccaaaagccggcttggcgccggctttcccggagaccttcaggtcgacggaaaagcaaaagccaagacgtttttgagtgtcttctgaccccgactgcagaagaccccttggttcgggcgatgtgcaacgcatcgctgtccgccaacggctggtagtggccagccgccaagcagtggtgcctcggcactgctgacaagtcgctgaagatctcaagctccggagctctcatggcccaatcgtccgcgtacagttacaccgaacgcaagcgcatccgaaaaagtttcggtaaccgcgacagcgtcgtagaaattccctacctgctgcagatgcagaaagacgcgtacaccgcgttcctgcaagctggcattcctcccaaacaacgcaccgtcgaaggcctgcaggccgcgttcgacgccgcgttcccgatcgtctcgcacaacggttttgtcgagatgaagttcctcgagtacaacctcgcgaagcccgccttcgacgtgcgcgagtgccagacccgtggcctgaccttcgcctcggccgtgcgcgccaaggtgcagctcatcatctatgaccgcgagtcgtcgacctcgcagtcgaaggtggtcaaggaagtgaaggaacaagaggtctacatgggcgaagtgccgctcatgaccgaaaagggttccttcatcatcaacggcaccgagcgcgtgatcgtctcgcagctgcaccgttcgcccggcgtgttcttcgaacacgacaagggcaagacgcacagctcgggcaagctcctgttctcggcccgcgtgattccctaccgcggttcgtggctcgacttcgagttcgacccgaaggacatgctgtacttccgcgtcgaccgccgccgcaagatgccggtcacgatcctgctgaaggccatcggcctgaacccggagtcgatcctcgcgaacttcttcgtgaacgacaacttccgcctgatggacagcggcgcgcagatggaattcgttcccgagcgcctgcgcggcgaagtcgcgcgcttcgacatcaccgacaagtcgggcaaggtcgtggtcgccaaggacaagcgcgtcaccgcgcgccacacccgtgaactcgagcagtcggccaccacgcacatcagcgtgccggaagacttcctggtcggccgcgtcatcgcccgcaacatcgtcgacgctgactccggcgaaatcctggccaaggccaacgacgaactgaccgaagcgctgctgaagaagctgcgcacggccggcgtgcaggacatccaggtgatctacaccaacgaactcgaccagggcgcgtacatctcgcagaccctgcgcatcgacgagacggtggacgagttcgcagcccgcgtggccatctaccgcatgatgcgccccggcgagccgccgacggaagacgccgtgcaggccctgttccagcgcctgttctacaacccggacacgtacgacctgtcgcgcgtcggccgcatgaagttcaacgccaaggtcggccgcgacgaatcgaccggcccgatggtgttgaccaacgaagacatcctggccgtggtcaagatcctcgtggacctgcgcaacggcaacggcgaagtcgacgacatcgaccacctgggaaaccgccgcgtgcgttgcgtcggcgaactggccgagaaccagtaccgtaccggcctcgcccgcatcgagaaggccgtgaaggaacgtctgggccaggcggagcaagagccgctgatgccgcacgacctgatcaacagcaagccgatctcggccgcgctgaaggaattcttcggcgcctcgcagctgtcgcagttcatggaccagacgaacccgctgtccgaaatcacccacaagcgccgtgtgtcggcccttggcccgggcggtttgacgcgcgaacgtgcaggcttcgaagtgcgcgacgtgcacgtgacccattacggccgcgtgtgcccgatcgaaacgcctgaaggcccgaacatcggcctgatcaactcgctggccctgtacgcccgcctgaacgaatacggcttcatcgagacgccgtaccgccgcgtggccgacagcaaggtcaccaacgagatcgactacctctcggccatcgaagaaggcaagtacgtcatcgcccaggccaatgcggtcctggacaaggacggcaagctgaccggcgacctggtctcggcgcgtgaagccggcgaatcgatcctggtcggtgccgagcgcatccagtacatggacgtgtcgcccgcgcagatcgtgtcggtggccgcctccctcgtgccgttcctggagcacgacgacgcgaaccgcgcgctgatgggcgccaacatgcagcgtcaggccgtgcccgtgcttcgcccagagaagccgatggtcggtaccggtatcgagcgcgtttccgcggtcgactccggcaccgtggtcacggccacccgtggcggtatcgtcgattacgtcgacgcgacccgcatcgtggtgcgcgtgaacgacgccgaagcggcagccggtgaagtcggtgtggacatctacaacctgatcaagtatcagcgttcgaaccagaacaccaacatccaccagcgtccgatcgtcaagcgcggcgacaagatcgccaagggcgacgtggtggccgacggtgcatcgaccgacctcggcgaactggccctcggccagaacatgctgatcgcgttcatgccctggaacggctacaacttcgaagactcgatcctgatctcggaacgcgtcgtcgccgaagaccgctacacctcgatccacatcgaggaactggtggtgatggctcgcgacaccaagctgggtgccgaagaaatcacgcgcgacattccgaacctggccgagcagcagctcaaccgcctcgacgaatccggcatcatctatgtcggcgccgaagtgcagccgggcgacacgctggtgggcaaggtcacgccgaagggcgagaccacgctgacgcctgaagagaagctgcttcgcgccatcttcggcgagaaggcttccgacgtgaaggacacctcgctgcgtgtggaccagggctcgcaaggcaccgtgatcgacgtgcaggtgttcacccgcgaaggcatcacgcgcgacaagcgcgcccagcagatcatcgacgacgagctgaagcgcttccgcctcgacctgaacgaccagcttcgcatcgtcgaagccgacgcgttcgaccgtatcgagaagctcctgaccggcaaggtcgccaacggcggcccgaacaagctggccaagggcaccaagctcgacaaggcctacctgtcgtcggtcgagaagttccactggttcgacatccgcccggcggacgacgaagtggcaacgcaactcgagtcgatcaagaactcgctcgagcagacgcgccacagcttcgacctcgcgttcgaagaaaagcgcaagaagctcacgcagggcgacgagctgcccgcgggcgtgctcaagatggtcaaggtctacctggccgtcaagcgccgcctgcaacccggcgacaagatggccggccgtcacggcaacaagggtgtggtgtcgaagatcgttccggtcgaagacatgccccacatggccgacggtacgccgtgcgacatctgcctgaatccgctgggcgtgccttcgcggatgaacgtgggccaggtgctcgaagtgcacctgggctgggccggcaagggcatcggccagcgcatcggcgacctgctgcagcaagaagccaaggtggccgagctgcgcaagttcatggagcagctgtacaacggttcgggccgcaaggaagacctcagcaagctgagcgacaccgacctgctcgagatggcggagaacctcaccagcggcgcaacctttgcgacgccggtgttcgacggtgcctcggaagaagaaatccgcggcatgctgaagctcgcctatccggacgacatcgccaagctcaagggcctgaccgatacgcgcacgcaggcctacctgtacgacggccgcaccggcgaccagttcgagcgtcccgtcaccgtgggctacatgcacttcttgaagctgcaccacttggtggacgacaagatgcacgcccgctcgaccggcccgtactcgctggtcacgcagcagccgctgggcggcaaggcgcagttcggcggccagcgtttcggtgaaatggaagtgtgggcgctggaagcttacggcgccgcctacgtcctgcaggaaatgctgaccgtgaagtccgacgacgtgcaaggccgtaccaaggtgtacgaaagcatcgtcaagggcgagcacacgatcgaagccggcatgccggaatcgttcaacgtgctggtcaaggaaatccgttcgctgggtctcgacatcgagctcgagcgttcgtaatcagaagaggaaagagtcacatgaaatcgctactcgacctgttcaagcagttcacacccgatgagcatttcgatgccatcaagatcggcatggcttcgcccgagaagatccgttcgtggtctttcggcgaggtgaagaagcctgagacgatcaactaccgcacgttcaagcccgagcgcgacggtctcttctgcgccaagatcttcggccccatcaaggactacgagtgcctgtgcggcaagtacaagcgcctgaagcaccgcggcgtgatctgcgagaagtgcggcgttgaagtcacgcagaccaaggtgcgccgcgagcgcatgggccacatcgacctggccgcgccctgcgcgcacatctggttcctgaagtcgctgccgtcgcgcctgggcctcgtgctcgacatgaccctgcgcgacatcgaacgcgtgctgtacttcgaagcctacgtgatcaccgaccccggcatgaccccgctgaagaagttcggcatcatgtccgaggacgactatgacgcgaagcgcaaggaatacggcgacgaattcgtcgccaagatgggcgccgaaggcatcaaggacctgctcgaagggatcgaactcgacagcgagatcgaacgcctgcgcggcgacctgaccggctccgaagtcaaggtcaagaagaactccaagcgcctcaaggtgctggaagccttccgcaagtcgggcatcaagcccgagtggatggtgctggacgtgctgcccgtgctgccgccggacctgcgtccgctggtgccgctggacggcggccgctttgcgacctccgacctgaacgacctgtaccgccgcgtcatcaaccgcaattcgcgcctgcgccgcctcttggagctcaaggctccggaaatcatcgcgcgcaacgaaaagcggatgctgcaagaagctgtcgactcgctgctggacaacggccgccgcggcaaggccatgacgggcgccaacaagcgcgcactcaagtcgctggccgacatgatcaagggcaagagcggccgcttccgccagaatctgctgggcaagcgcgtcgactactcgggccgttcggtcatcgtggtgggcccgacgctcaagctgcaccagtgcggcctgccgaagctgatggcgctcgagctgttcaagcctttcatcttctcgcgcctcgaagccatgggcatcgcgaccacgatcaaggctgccaagaaggaagtcgaatccggcacgccggtggtctgggacatcctggaagaagtgatcaaggaacacccggtcatgctgaaccgtgcgcctacgctgcaccgtttgggcatccaggcgttcgagccgatcctgatcgaaggcaaggcgatccagctgcacccgctggtttgcgcggcgttcaacgccgacttcgacggcgaccagatggccgttcacgtgccgctgtcggtggaagcgcagatggaagcccgcacgctgatgctggcctccaacaacgtgctgttcccggcttcgggcgaaccgtcgatcgttccttcgcaggacgtggtgctgggtctgtactacacgacccgcgaccgcatcaacgccaagggcgagggcctgatcttctccgacatcggtgaagtccagcgcgcgctcgacgccaacgtggtcgagctgaccgccaaggtcgccgtgcgcatcacggagtacaccaaggacaaggaaacgggcgagttcacgccttccacgtcgctggtggacaccaccgtgggccgcgcgctgctgtccgagatcctgccgaagggcctgccgttctcgaacatcaacaaggcgctgaagaagaaggaaatttccaagctcatcaacgtctcgttccgcaagtgcggcctgaaagagaccgtggtgtttgccgacaagctgctgcagaacggcttccgcctggcaaccaaggccggtatctcgatcgccatcgacgacatgctggtgcctgctgaaaagcacggcatcatcgagcgctccgccaaggaagtgaaggagatcgagcagcagtacgtctcgggtctcgtgacttccggcgagcgctacaacaaggtggtggacatctggggcaaggccggcgacgaagtgtcgaaggtcatgatgtccaagctgtccaagcagaaggtcatcgaccgccacggcaaggaagtggagcaggagtcgttcaactccatctacatgatggccgactccggcgcccgcggttccgcggcgcagattcgccaggtggccggtatgcggggcctgatggccaagccggacggctcgatcatcgagacgcccattaccgcgaacttccgcgaaggcctgaacgtgctggagtacttcatctccacccacggtgcccgtaagggtctggctgacacggcactgaagaccgcgaactcgggttacctgacccgtcgtctggtcgacgtgacgcaagacctggtggtgaccgagcaggactgcggcacgcacggcggctacctgatgcgcgccatcgtcgaaggcggtgaagtgatcgaatcgctgcgcgaccgtatcctcggccgctcggcggcggacgacgtgctgcacccggaaaaccgttcggtgctgctgaaggccggtgagatgttcgacgaggacaacatcgaagagctcgaggcgcaaggcgtcgacgaggtcaaggtgcgtaccgcgctgacctgcgaaacccgcttcggcatctgcgcgacctgctacggccgcgacctgggccgcggcggcctgatcaacatcggcgaagccgtcggtgtgatcgcggcgcagtcgatcggcgaacccggcacgcagctcacgatgcgtacgttccacatcggtggcgcggcatcgcgtgcggccgtggcctcgagcgtcgaagccaagtccaacggcacgatcggcttcaacgccacgatgcgctacgtgaccaacagcaagaacgagctggtggtgattgcacgttcgggcgagatcgtcatccatgacgaacacggccgcgagcgcgagcgccacaaggtgccgtacggtgcgaccctggccgtcaaggccgaccagcagatcaaggccggccacgtgctcgccaactgggatccactgacgcggcccatcatcaccgagttcgccggcaagacgcagttcgagaacgtcgaggaaggcctcacggttgccaagcaggtggacgaagtgaccggcctgtcgaccctggtcgtgatcgacccgaagcgccgcggcgctgccaaggtcgtgcgcccgcaggtgaagctcatcgacgcctccggcgccgaagtgaagatcccgggcaccgatcactcggtgaccatcggcttcccgatcggctcgctggtgcagatccgcgacggccaggacgtgggccccggcgaagtgctggcgcgtattccggtcgaaggccagaagacccgcgacatcaccggcggtctgccgcgcgttgccgagctgttcgaagcccgttcgccgaaggacaagggcatgctggccgaaatgaccggtaccgtgtcgttcggtaaagagaccaagggcaagatccgcatgcagatcaccgatccggaaggcacggtctgggaagacctcgtgccgaaggaaaagaacatcctggtgcacgaaggccaggtggtgaacaagggcgaaagcgtggtcgacggtccggcggacccgcaggacatcctgcgcctcttgggttcggaagaactcgcgcgctacatcgtggacgaagtgcaggacgtgtaccgtttgcagggtgtgaagatcaacgacaagcacatcgaggtgatcgttcgccagatgctgcgccgcgtcgtggtcgacaacatcggcgatacgagctacatctccggcgaacaggtcgaacgcagcgaaatgctcaacaccaacgacgccctgcgcgccgacggcaagctgcccgccacgttcaccaacctgctgctgggtatcacgaaggcatcgctctcgaccgactcgttcatctcggccgcttcgttccaggaaacgacgcgcgtgctgaccgaagccgcgatcatgggcaagcgcgacgagctgcgcggcctgaaggaaaacgtcatcgtcggccgcctgattcccgcgggcaccggcatggcgtaccaccaggcacgcaaggtcaaggatcagatggacgaggccgagcgccgcgccatcgccgaatccgaagccgctgaactggccggttcgaccagcgatgtttccagcacggccgacgccagcgaaggcgccgcgtccgaataactggttagcatcaccggccatgaccggtatccgacgccccccgaccgaatccggttggggggcgtttttctttgagccgttttttccatgaagtgtttttgccgatgagcgcattgcccgattcgcttgccagctggatcgtcgttgccgtgctgttgttctggttcgtgggggcctacaacaggctggtgcgcctgcgcgccgccgtgctccaggcctacgccacgctcgatgcagcgcttcgaaagcagctggacttcgtcctggccagcatcgcggccaccgtgcccgaaaaagatgcgccgtcgcccggccattcttcggcggtggcaccgctgcaggccgccgccacccagctggccacgctgctgggcgcgacccggctgcatccgctcgatccgggcggcatggccgcgctggccacggcgctgcaggtgctgatctccgcatggcagcgccagcatccggatgcggtcacggtcttcgacgcggacggaacgctctcgcggcccgcgccgctgctgccgagcagtaccggaaacggggctggtgccacgtcgtccggcacggcggagcccgtggcctggcctgagccttcggccgcggcggaaatcgctcgcagccaattcaacctggcggtggaacagtacaacgcagccatcgtccagtttccggccttgctggttgcatggatggtgcgtttgcgaccggccgcgcccctgctctgattttcgaatcgccgggaaacgccttcttctttcttgatccgcgcggctttgtgcgtcttgccggcccgttaccatcgccccaacttgccagaactatcttccgatcatccaggcagcagcccctcgccgctgctgcaacccccgctctggcgccagctgcagttgactgccgtggcgctggcgtcgattcgcgccggcagctcgggcaccgtcgccttcgaagcggtggagccggccatgcggccgggcgtgcaggcgctcggcttccaggtgctgcgctggctgggccgcgcagaggcgttgcgccgccacctcgccaagcgtacgccgccgccgttgcccgacgccttgctgtgcaccgcattggcactggcctgggatgcgcagcacgccccttacgagcccttcacgctggttgaccaggcggtcgaggcggcaaagcgcaacccggccacgcgcgcacaggccagtttcatcaacgcctgcctgcgccgcttcctgcgcgaacgcgatgagctcgtggccgccaccgaccatgaaccggtcgcacagtggaaccacccgcgctggtggatcgagcggctcaagcgcgaccactcgcgcgattggcagcgcgtgctcacggccgacaacgcccacgcaccgatgaccctgcgcgtcaatctgcagaagaccacggttgcctcataccagctcgcgctggaggccgtcggcctggcggcggtgcgcgtgggagcggccggcctgcagctggtgcgcgcccggccggtgcagcagctgccgggcttcgcggacggcgaatgctcggtgcaggacgcagccgcccagatggcggcgccgctgctgctcgaagggatgctccccgcggccggcgccgcgccgctgcgcgtgctcgatgcctgcgcggcaccgggcggcaagaccgcgcacctgctggagtttgccggtccggaggccgtcgaggtgacggccctcgaagtcgacgcggtacgcagccggcgcatcgacgaaaccctgggccggctcgggctgtccgccaaggtggtggtggccgatgccgcgcggccgtccgcatggtgggacggcacgctcttcgacgccattctgctcgatgcgccctgcacggcgtcgggcatcgtccggcgccaccccgacgtgcgctggctgcgccgcgagagcgacacggcccagctcgccgtccagcaggcggccttgctggcggcgctctggccgctggtcaggcccggcgggcggctgctctattgcacctgttccgtgttccgggaagagggctcgcaacaaatcgatgcgtttcttgcgcacaacaccgacgcccgattgaaggcatcgccaggccatttgcttccccaaagcggggcgaatgcccgcgccgtcccggacaatgcctcaggtgaccacgacggcttcttctacgccctgcttgaaaaacgcccgcgctgagccccgcgggtggcgcggcgccacggcattggcggcgctgctgatggcctgcgtgctgttgctgagctggctgcccctcaccgcggccgcgcaagggcgcgccgctgcgtcggtcacccagatgcgcctcgagcaggccgacgacggtgtctacctcaccgcggccgtgcagttcgagctgccctcgttggtcgaggaggtgctcgacaagggcattgccatctatttcgtggccgaggccgaggtttttcatgagcgctggtactggaccgaccgcaaggtggcccaggtcacgcgccacatgcggcttgcctaccagcctctcacgcgccgctggcggctcaatgtgtcgcccgtgcccatcaccggcaccgcaggattcggcgtctcgctgaaccagaacttcgacagccttgccgacgccatggacgccgtcaagcgcgtaggccggctgcggctgggcgatgcggccgagatcggcgacgatcccacgcaccaggtcgtgttccgcttccggctcgacacttcgcagctgccgcgcccgttccagatcggcgtggtcgggcaggccgactggaacatcgtggccgagcgcagcgccaagctgaccctggagaagcagcggtgagcaccaaaccgcgcagcggcgcagcggccagccccgccgcccgccgcgcgcgcgcgatccgctgggccgttggcgtgggcgccgcgctggtcacggccatcggcctggtgctgatgttcctgctggcgcaagccaccaataaccgcgcgctgtacgagcgctattacgtacggcttttcggtatcaacgtggtggtggcggtgctgctggtgctggtgatcggctgggtcgcgttccgcctgttgcggcgcttgcgccagggcaagttcggcagccgcctgctcatcaagctggcggccatcttcgcgctggtgggcgtcgtgcccggcgcgctggtctacgtggtgtcctaccagttcgtcgcacggtcgatcgaaagctggttcgacgtcaaggtcgaaggcgcgctcgatgccggcctgaacctgggccgcgccacgctcgattcgctctccgacgatctggccgccaagacgcgcgtggccagcgcgcagctggtccaggtgcccgacgcgagcgccggcctggtcctggagcgcattcgcgaccagctccaggcgtccgacgtggtgctctggaccggcaccgggcagctcgtggccagtgcgggtacctcgcgcttccagctcaaccccgagcggccgaccagccagcagctgcggcaggcgcggggcgaccgcgccatcgcccacatcgaaggcctggacgaaacggcaccgccgggcgccaccctgcctcccgccagcgtgcgcgcgctggccatggtgcagcgcccgggcttcgacttcgacaccgcgccgcgctttctgcaggtcacgcagccgctgccacccgccgtggtggccaatgcgctcgccgtgcaggaggccaaccgcgaataccaggagcgggcgttggctcgcgaaggcctcaggcggatgtacatcggcaccctcacgctgagcctgttcctggccgtgttcggcgccgtgctgctggcggtgctgttcggcaaccagctggcgcggccgctgctcgtgctggccgacggtgttcgccaggtggccgccggcgacctgcggcccaccaccgtgctgcaaggaaaggacgagctgggcggcctcacgcgctcctttgccgtcatgacccagcaactggccgatgcccgcggcgcggtcgaaaaaaccatgggccagctcgacgccgcccgcgccaacttgcagaccattctggacaacctgacctcgggcgtgatcgtgctcgacgccaagggcaccatactgtccaccaaccccggtgccacgcgtgtgctgcgcgccccgctggcggcttacgagggcatgccgctcgcccaggtgcccgggctggccgacttcggcaacagcgtgcagcagcagttcgacgaattccaggtcgagcgcctgcagcacggcctcgaccactggcagcacgccttcgagctgcacgccaccggcatcgatctgccgcagcaggacagcgccatcaacatcgttgcgcgcggcgccgagctgcccggcgccgcccggctgctggtgttcgacgacatctccgagatcgtgtcggcccagcgcgcccaggcctggggcgaagtcgcgcgccgcctggcgcacgaaatcaagaacccgctgacgcccatccagctttcggccgagcggctcgagatgaagctctccggcaaggtcgctccgcccgagcaggccgtgctggtcaagtcggtcaagaccatcgtcgaccaggtcgacgcgatgaagcgcctggtcaacgagttccgcgactacgcccgcctgcccgcggccgatctcaagccggtcgacctcaatgccctgctggtcgacgtgctccagctctacggcgccgacaacgcccccattgcgctgcgctccgagctggacgagcgctgcccgccgatccgcggcgacgcgcagcagatccgccaggtcatccacaacctgctgcagaacgcgcaggacgccgccgaggccgccgccagcagcaccgggcgtgccggcgaagtcgtcattcgcacccgcctcggcgattcgggccagcgcgtgcgcctcaccgtgcaagatagcggccccggctttgccgaaaacatcctcaagcgcgccttcgagccctacgtcaccacgaaaacaaaaggtaccggtctggggctggccgtggtcaagaaaatcgcggacgaacacggcgcgcgcatcgagctttccaaccgtgttgtcgatggggctgtagcaggggcgcaagtctcgctatcattcgcgctggcaggcgagtcgcaggcagcggccgctcacaccgaagattcgaagtcttccgccgcctgagcgcgaaagaatccatcgcctccaggcgacggataggctggcggacacccatacacatcattcagataccagcgcacaagacaagcagcactcatggcaaacattctcgtggtcgatgacgagctgggtattagggacctgctcttcgaaattctcaatgacgaaggccacaacgtggagctcgccgaaaacgcggccgaagcacgcgccgcacggcaacgcgcacgacccgacctcgtgctgctcgacatctggatgcccgacacggacggcgtcacgctcctcaaggagtggtccacggccgggctcttgagcatgcccgtcatcatgatgagtggccacgccaccatcgacacggcggtcgatgcaacgcgcatcggcgccttcgcattcctcgaaaaacccatcaccctgcagaagctgctcaaggccgtggagcaggggctcgcgcgcgagagtgcaaggcgcgcagccgcgggcgttgttcccccggccgcgggcgtcaacccgtcggccgccatcaccaccacgggcgacagcctgctgctggcctcgctggcggccgtgccggtgcccgatgccgggccgcaatcgacccagagcttcgacctggaccgcccgctgcgcgatgcgcgcgacggcttcgagaaggcctacttcgaattccaccttgccatggaaaacggttccatgacccgcgtggccgagaagaccggccttgagcggacccatctttatcgcaagctcaaacaacttggggtcgatctttcgagaggccgcagaagcgctgtataatttaaggctgcacaccaaggcccggtagctcagttggtagagcagcggattgaaaatccgcgtgtcggtggttcgattccgccccaggccaccaaattcgaagcccttgatcctcccaggatcaagggctttttgctttggcgctcgctgctgccgttcggccttcgccctttttcaagatgcaacggtccgcttcacctacgccgatgtgagcatcaccctacagaaagcgtgcgcctgaaaaatagagtggctcatgtgcgaggcaaggttgtttcgcgcacgagaaaatcgaaatgtcttcccaagccagcctcatcgaacggcagacgcttcgagtccgcgtcaaaactgtctcgctcgaagccgatctgagcttgcccgtcgcggcccgaggcatcgtgttgttcgcgcacggcagcggcagcagccgcttcagtccgcgcaaccgggaggtcgccgagcggctcaatgacgccaagctcgcgacgatgctggtcgatcttctgacctccgacgaagaagccgtggatgaacgcacgcgcgaattgcgttttgacatcggcctcttggccgatcggctcgtcgggttgaccgattggctgcgcgtgcatgaaagaaccgcggcgctgcggatcggctatttcggcgccagcaccggtgccggcgctgcgctggtggccgccgccgagcggcccgacacggtcgatgcggtggtgtcgcgcggcggccggccggacctcgccggagcggctctggtgcgcgtgcgggcgcccacgctgttgatcgtcggcggcaacgatgggccggtgatcgacatgaactggcaagcgctcgcggcgctgcacagcgagaagcggctgtcgatcgtgcccggcgcaacccacctgttcgaggagcccgacgcgctcggcgccgtttccgtgttggcacgcgactggttcaagaggtatctcgaacaacccaggagtgcgaaatgagcaaatcgccaggacaccgcaaatggcccgatcaccaagtgcgggaggagcagcttcaacagcccatggaagtcgaggttgaaggcgtcgtcgtcgccaattcgcgagacgtcatcaaggtggtcgaagacaggtctccggatcgctactactttccgcgcactgacgttcgcatggacaagctgaagcgctcgcagaccatttcagaatgtccgttcaagggccatgcgagctactacagcttgagcctgggcgaacggcagatcgacgacgcgggctggacctatgaacgcccgtacgacgaacacaaggccctgaaggaccgcatcgccttttacgacgacaggtttccggagatccacattcgcccgaaggcctgagccgttgggacttgtacgttgcgcccagcgagggccgtcgcgccgtggcgaaggggaactggccactcaggattgaccaaggcttcgctccacggccgccagcaggtcgtcgggacgcagcatcgcggcccgggcttttaccgcggtttcgtactgatgcagcgcggcccgcaagcgcggcgcattctggagttcattccatacgggagcgagagcggcatgcggcggcgattcaccgcgcgcaatttgctccgcgaaggcgaggctcgcgggctcggcgagcagcacggccttgctcgctgcactcaatacctgcggcggcggctcggccgcagccgagcagcaatagatcacgtgccccggcagtgaatggccggcgggttcgagctcgcgaagcgaggctccgagaacgcgtgcctcgccatcgaccgatgcaaaggcgtagaccgcgtcggcacttgcgtgcgcgagccgtcgcagtccgcgcagcaggcgaggaaagtcggatgccgccgcactgggcgacgccttgatctcggcgagaagaaccagttcggcagcagcgcccggttcactccgcaagagggcggcgtcccactcttccttggccttgttcgccgctcccggaaacccgcgcggcgttcgaagactgcgcaccacgcggtaggcagctgtcccttcgtggtggcgattcagcaactcggccatcttgccgaatgcctcggcggcggcctgctcggccctttcgccctcgcgcgccgacgtgcggccttcggcggcagcggcatggctgcccgccagcggcccacgccgttcgcacagtgcctggtagcgctgcacggcgtcgaggcgaagcaattcgtcgccgcgttggagtcgtgccagcgccgggctggagagcatggtgttgagtggtgcccgcagttccggctgttcggaaagatcctgcgcgagcgcgcgttcgacagcttgcgccagcgctgcccaggagcccgccgctgcccgcgcgtgcagccgcgccagtgcctcgcgcgcctcgccggtgggcatgcggcgcagcttgccgggatgcgcgatcgcatcggtcgcggttctcacggcgcgctgatcggccgcgcgccttctgcgcagctgcacgtgttcgtgaaccgttgcatcccgcgcctgcagcacgatcgcctgaaaggccgggtcgccgccgtccgttgcgagtgcctgccgaatcaactgcgccagtgcccaggtgaacgtctcttgcgagtgcggcgacggcggtagatgccgccgtaccgcgaggcaggcgtcttcgatcgcgaaggcaagcgcgacgtcggcgccgcttgccacggctgcttcagcgttgtgtggcaaagacagcatgcggtaccggcgcggtgcagtacgcaaggcggcgagaagaagcgcgtcgaggtgtggcaatcgattcgaactcgagacaaaagctgcaggctcactctacccctggctccgccaagtgacattcctgagcccatcggcggctcgatgtgacgccgattgtcatttctgacgcgcccgcggcacgtcgtcatgctcgccaagcgcgatcaacgaatggaaaagatttcatcggccgattggcatgcatgttgcagtaacaatttctaaccatcgccattcgacatgcatccacaagacagcgaaaacaacattcctctagatcgacgtgctttctgcatgggggcggtgagcctggtcgcgctcggcacgaccgcgtgtggcggcggcggaggaggcggtggcctgggggcgggcagcttcggcaccgtggccgcggcgccgcaggacgcctcggcggcgccagttgctgcgcccgctgcggcaacggattccgctgccgaatcagtacccgctccggcaccgtcgccatctccatcccaactccgaaagttcgtccaccccggccttcttcacacggaggccgacttcgagcgcatgcgccagaaggtcaaggacaaggcgcaaccatggctggccggctggaatgcgttgacaggcagcggccgcgcgcaactcggtgcgaaaccgcgtccgctggtcacggtggtgagaggtggcgagggccagaacttcgcgcagttcttcatcgacgtcgcacgctcctaccaactcgcgctgcgctggaaggtctcgcaggacacgcgctatgccgacctggccgtggtcttcctgaacgagtggtcctccacgctcaaagaggtcacgggcaatgcggaccgctttctcgcggcgggcatctacggctaccaattcgcgaacgcggccgagatcatgcgcacctacccaggctgggcgccggccgatttcgcgcgcttccagaccatgatgctggacatcttctatccgatcaaccaccacttcctcaccgtccacaacggcgcccagatcaccaactactgggccaactgggaccagtgcgccatggcctcgatgctggccatcggcgtgctctgcgaccggccggacatctacgacgaggcgctgagttactacaagacgggccagggcaacggcgcgggcctgcaggcggtctatcacgtgcatcccggctacctcggccagtggcaggagagcgggcgcgaccaggggcactgcacgctcggcatcggccttgccggggcgttctgcgagatggcgtggaaccagggcgacgacatctacggctacgagaacaatcgcttcctcgcgggcgccgagtacgtggccaagtccaatcttctggatggcgccggcgccttctacacggtgcccttcttcaccaacgtcaacaggcagggcacgcagtccgtgttgtcgaccggaggccaggggcaccgccgaggaatctgggagagcgtacacaaccactatgcgaaccgcctgggcatcgcgaccccttacaccgccctgcaagtcgcgcagatgcgtcccgagggagacggcaacaacggcgatcaactgggcttcggaacgctgacctacacgcgcgacccgctcgccacgctcgtgccgccgaccgggctcacggcccgggtgcgcggagcgcaggtcgtgttgtcctggtggggcagcaccggtgcgctgagctacacggtcaagcgcgcggccgttgcgggcgggccctacgccactgtgacctcgggcatcaccgatacgctcaccttcaccgacggtgccgtcgctgcgggagaggtgtggcactacgtggtggtggccgtgaacgcgggcggagagagcgccccttccaccgaggcaagggccgccatcaaggccgagctgctgatgcagctcaagttcgacgaggcgcagggcacttcggccgccgatacggcgggccgcttcgccgcaagcgaactcgcgggcggtgcgggatgggtggctgggcacgagggcggcgcggtcgccctggccagcgcggcggccagcgtcaacctgccggcggcgccggtgaagaacctggccgacttcacgatcgcgtgctgggtgtacctggacgccatctcgacgtggtcgcgtgtgttcgatctgggctccggcgagcgccgctacatgatgctgacgccgcgcagcggcgcgggcacggtgcgctatgcgatctccaccgtccacggctacaacacgcagatgatcgaaggctcgtcgccgctgcccaccggccgctgggtgcatgtggccgtcactctgtccggcgcgctcggcacgctgtatgtcgacggcgccgtggccgggagcaatgcgcagatgacgctggcgcccttcgatctcggagagaccacgcagaactttctcggtcgttcgcagtattcagccgatccattcctgcgcggccggctcgacgacttccggatctaccacggtgcgctgagtgcggcggagattgcgtcgctggtggcgtagcaccgcatcgggccgcccatggctaaaccgctccgtgcgactccacgtaaagcgcatagagcgaatggctgctcgccatgtagaggcggttgcgcttcggcccgccgaactcgaggttggcacagcgctccggcagccggatgaagccgatcggcttgccctgtgggttgaagaccttcacgccatcgagctcctccgactttccgagcggcagatgggccttcattccgccgccgatgtcggttggctccggcgcgaatgcgccgctgaagccccagccgcaccagaggttgccgtcgcggtcgacgcgaaatccgtcgagcgcacccgggccgtccgcgtcgatcagcttggtcttgttcgacacgctggcaccgtcggatgaaacgtcgtagctccagatgctgcggtgaggcgtgcctttccactcgaccacgtagagcttcttctcgtcgggagaaaacgcgaggccgttcgggttcacgagatcggtgatcaccgcggtgagcttgccgtccgtggcgatgcgatagacgttggtcgtcggctgttccggcgccgccctggagccttcccactcgccgttgatgccgaagatcggatcggtgaaccacacggtgtcgtccgacctcacgaccacgtcgttgggcgcgttgagcttcttgccatcgaaactgtcggccagcaccgtcatgcggccgtccttctcggtgcgcaccacgcggcgcgtgaccgagtgttcgcaggtgacgagccggccctggcgatcgcgggtgttgccgttggcgaagttggcgttctgcttgtgcaccgtgaacctgccggtcttctcgtcgtacttcatgatccggttgttcggaatgtcgctgcacagcaggtagccgccctcgggaaagtacaccgggccctccgcccagcgcatgccggtgcccacctgctcgatggtgctgctgtagatgcggtacttcgcaaagctcggatccaggatcagcaccgacggatccggatagcgctggttgggcttgaattcaaaagattgcgcatcggccaggcccgtgagggccgccaatcctgatcccgcagcggacttcaggaattggcggcgatgacggtttccgttctgcatcggtagatctcctttgtcgttgtgaaagggggcggctcgcctgtgctcgcaggcgagggcccagtccgatcttacgtatcgaaggaaatcaagtgccgctccagcacgcgcggcaggcctcaccgcttcatgaggcctgccggcggatcatgcgttctcggcgtgggcgggtgcggctcgtcgtcgaatttcagtctgcagcgcacgttgcccggcggccagtgcggcttcataagtgtccgccgcgtcgaaggcgtcgcgcagcactttgggattcgctccctccgtgtcggtttcgagcaggcgccagacatatgaaccgagggttggctcctcgatgatgagttcgatgggttgtgtcatgcgctcaacttgcacaagttgcggcggaatgtctgtaggcggaattcgaatgctgcttgaattggccgttcggcacctcggcaggcgctactcgaccggcagcttgacgggcccgctcgctctcagccgcagcgcattggtgatgaccgacgccgagctcaggctcatcgccagggccgcgatcatcggcgacagcagccatcccgtgaacggatacagcacgccggcggccaagggcacgcccagcgcgttgtagatgaaggcaaagcccaggttctgcttcatgttggcgatggtctgctcggagacgatgcgcgcctgcgcgatgccgcgcaggtcgcccttgaccagcgtgacctgggcgctgttcatggccacgtcggtgccggtccccatcgccacgcccacgtcggccttggcgagcgcgggcgcatcgttgatgccgtcgccggccatggcgacgatgcgtccttcgcgctgcagccggtccaccaacgccagcttgtcggcgggcttgacttcgccgtgcacctcgtcgatgcccagcctggcggccaccgcgtgggcggtggtcaggccgtcgccggtggccatgatcacgcgcatgcccgaagccttgagcgcctgcaatgcctccgcggtggtggccttgaccggatcggacacggcgagcaggccggccagcttgccgtcggcggcgaggaacatcacgctggccccttcggcgcgcagggcctcggcctgcggcttgagatcgctgaccgcaacgcccagttgatccatcagcgcagtgttgccgagcgccagcctcttgccgccgacgctgccgctcacgccgatgccgctggcggattcgaactcgtccgccgtgcccagcgcaaggttgcgctcgcgcgccgcctgcacgatggcatgcgccaatggatgctcgctcccctggtcgaggctggccgcgaggcgcagcacttcgtcctcggtgaagccggacgtggccaccgcgcggtcgaaccgcggcttgccctcggtcagtgtgccggtcttgtcgacgatgagcgcgtcgaccttgcggaagctctcgatggcggccgcatcgcggaacagcacgccctgcgtggccgccttgccggtggccaccatgatcgacatcggcgtggccaggccgagtgcacaggggcaggcgatgatgagcaccgccacggcattgatgagcccgtgggtccagctcggagccggcccgaagaagccccatgcaaagaaggtcagcaccgcgatgccgatcacggtcatgacgaagtagccggccacccggtcggccatgcgctgcatcggcgccctggagcgctgggcctgcaccaccatctgcacgatgcttgcgagcaaggtctgcgagccgaccttctccgactgcatcaccagcgacccgctggtgttcagcgtcgcgccgatgagcttgtccccgacgcgcttggtgaccggcagcggttcgcccgtgagcatggattcgtcgacagcgctgatgccctcgaccaccacgccgtccaccggcaccttttcgccgggccggacgcgcagcttgtcgccgacatgcacatgcgcgataggaacatcttcttcaacgccatcggccttgatgcggcgtgccgtcttgggtgcaaggcccagcagcgacttgatggccgccgaggtttgcgaacgcgccttgagttcgagaatctggccgagcagggtgagcgagatgatcaccgcggccgcctcgaagtacaccgccacgcggcccatcgacatgaacgaatcgggaaacacgcgcggcgccgccgtggccaccacgctgtagacgaacgcggcggcggtgcccaggccgatgagcgtccacatgttcgggcttcggttcaccgcggattgcaccgcacgctcgaagaagggccacccgccccacagcaccacgggaacggcaagcaccagttcgatccagctctgcgtcgccatttcgaaccattgcaggcggtgtccagccatgccgagcacggtgaccgcgatggtgagcggcaaggtccagacgaatcgccgcttgaagtcgcgcaactccgggtcttccttttcatcgaggctcggcatctcgggctccagcgtcatgccgcacttggggcagttgccggggtggtcctgccggatttccggatgcatcgggcaggtgtagatggtgcccggcgatccgaccgccgcgtccggcgcgtttggctttcctcggttcaccggcgcacgatggccttcgtgatgatgatgatctttggaattggaacgcgtgtcgttcattcgaattctccagcgggaaaccatgaaattgcgcgtgccgcagtcgcgcttgcggtcagcctcgggtcaggttggcatccggacaatcgtcagtttcacggttgacatcatgtcaaggtcaagaggctgcgccctggcgctgcccgaacttgcacctctagatctcgcaaactctcttgaaacccctgcccatgcctcctgtttttcgccatctcctgacggttgcgctgctcgcgacttcaacggtccacgcccaggcgctcgactacgaccaccaggaaaactggaaggcggttcacgacagcgcccagtcgccgatcgatattcctaccggtgaagccaaggctggcgatgcgctcgagccacaagacattcgcctgagcaacgctcgcgcggagctcgacgtcgtcgacaacggccatgcggtggaggtcgaggcgaaggggccggacgccatgattcgcggccggcacttcaaactgctgcagttccacttccatgccgagagcgagcacacggtggacggcaagcacttcccgctcgaggggcatttcgtgttccgtgccgtggacggtcgcctggccgtggtgggtgtcatgtaccgcgaaggcgcggccaatccgctggcggccaaggtgctgacggcgctcgagaaggaaggccacggcgagctgtccaaggccgacatctccgttctcctgcccaaggacaaggcctactaccactacctgggctcgctgaccacgccgccgctgactgagaacgtcgagtggtatgtgctgcagacgccggtgtcgctgtctccggcacagattgcgcagttccgcgcgcgctatgcccacaacaaccggaagctgcaggagctcaacgggcgtccgctgatccgctttccgtcggtgtcgctgacgtccaatcgcgcagcccccgccagccgctgaacgccaagccaaaaaaagcccccggttcttcgcagagccgggggctttttcagtttggcgcggttttctcagacggcggaaactgctggccgggccacagccgcagggctgccgccatgcgggcccggcggtgtcgtgacgatggaggtgagcgcaggttccgccatgcgcaaagccgaaaggtcggggcgcgggcggcgcagttgtccatcggctgcgaatgccatttccatggcatgcgcggcgcccagcacctggtggtcggcgcggaaaccgccgatgatctgcagcccgaacggcatgtccgcgtgatcgatgccgcagggcagcgaaagcgcgggatgcgtcgtcagcgtgaccacatacgtcaacgccagccagcggtagtagttggcctgcttctcgccattgatggtgtccgcgtacagctgcgtccacgggaacggcgacacgggcgtggtgggcgaaagaatcaggtcgtagtcggcaaaggtcgcttgaaagcgcttgatgagccgggtctgctcggcctgcgcccaggcgctgtcgagcaggctcatctgcgcgcccatctcgtagttcgcgcgcgagttgggtcccaggctggccgggtcgcgctggtaggcggcctgcatgcccgccacgaaggcttcggcacgcagcacgtcgaagcagcggtgcgcttcgcccaggtccagctcgatcttgtcgcagcgcttgaacaggtgccgcatggcgtcgatcttgcggcgcatcgtggcgcggatgccgtcgtccaccgcgcagacgccgaagtcttcggtccacgccacccgaagcctgctcaggtcgacgtccgccggcttcaaaaaagacagcgggtccagcgggtagctcagcgggtcgccggcgtgcatgcccgcggaggccgccatctgcaggcaggcgtctgctacggtgcgccccatggggccgacgacggagatgggtgtccagcccagcagctttcgcacgctgggcacgatgcctggtgaaggccgaaagcccacaacgccgcacttggcggccggtatccgcagcgagccgccggtgtcggagccggtgcacacgggcagcatgtcgcaggccagcgccgccgccgaaccgccggaagagcccccggcattcaggttcgggttgaacgggttgccggtggcgccccacacgtcgttgcgcgagttggcgccggcgcccatctcgggaacgttggtcttgcccgccacgatggcgccggccttgcgaaggcgggccaccagttcgatgtcttcctgcggcacgtggtcgcggaagatcgcggagccccaggtggtgagcaggccttcggtgggctccaggtccttcacgccgagcggaaggccgtgcagcaggcccagcgagtcgccgcgcatcacggccgcttcagcggccttggcttcggctctcgcgcgatcgaagcaggtggcagtcacggcattgacgaacgggttcactcgctcgatctgcgcgatgcaggcctccagtagctcgaccggcgagaccgccttgctgccaatgaggcggcgcagttcgacggcggattgttcgatcaattcggtgcgagtgctcatgtcggtggttgttccaaggggcccggtccagtgcacccgcggatcgggctttgcccggccgccgggtgcgccccccagtggggggaggcgccgaaggcgcttcggggggcgttcatctagtcggaggtgatgttggcgcgcgcggcaatggcgcgcatcaagggcagttccttgctgatcagttcgctcacggcggccgaattgctgtaggccggctccaggccctgggcggtcagcttggcccgggtgtcggcgtcggccatggttgcggccagcgccttctcgagcttggccttcacctcggcaggcaggcccttcggcgccgacaccaccagccagctgtccatgttgatgtcggggtagccgctttccgccagggtgggcacgtcgggcaacagggcggagcgcttggccgtggtcaccgcaatggccttgatcttgccgttcttgagctgggggatggcggcgctcaccgtgtcgatgctgaacggaacctggccgcccatcaggtccgtcatggccggggcgctgcccttgtacggaacgtgcgtcatcttgaggcccgcgacgtggaggatggtttctcccgtgaactgcgatgtggtgccggtgccgtacgacgcgtacgaatacttgccgggcgatgccttcacgtagtcgacgaattccttgaccgtcttcaccggcacttcgctgttcgcgagcaggatgaggccgacgcgtccgaccaggccgatctggtcgaagcccttgaccgggtcgtacggaagattcgagcggatggccgggttgacggtgaacgtggtgcccgagctgatcagcagcgtgtagccgtccggcgcggccttggaaacgtagctcgccccgatcaccgtgccggcacccgcgcggttctcgatgaccacgggctgcccgagctccttgcccaggcgctgggcgatcacgcgcccgttcacgtcggtggcgccgccgggcggaaagggaatcacgagcgtgaccggccgcgtcggaaatccggtctccgcggcagccgctgccagagtcgacagtgcgaggcaggacatcagcaccatgctggcgaaagcgggaaagcgtttcatgaagagttctcctgaggggacgggacgctgcaataaaaggcgaggctgcgaaagcgtgaagcgggaaggcagtttcatcctaggagccgaagtcccctgccacaagcgcaatgtttagaattgtggattgccgttttggcaatccacgcaccgcggtttccgataacagctgcccaggagaatccatgtcgcttcacgcacttcaggagacggcggtccggtactttctggaggtcgtgcgaaccggctcggtgaaggaggccgcaaccaggctcaacgtggcgccttcggccgtgagccggcaggtggcgcgcctggagcgcgagctcgacaccttgctgttcgaccggcacgcacggggcatggtgcccaacgcggccggcgagctgctggccgcgcatgccaagcgggtgcaacaagacatcgagcgggtcgcgagcgacatccagggcttgcgcggcttgcgcagcgggcgtgtgcgggtggccagcaccgaaggcttcgcgttcgacttcctgcccacgctgatctcgcgctttcgcagcaagcacgagggcatccgcttccatctggaagtctgctcgccgcgcgagattcccggccgcatccgcgatggcgaggccgatgtcggcatcaccttgagcgcgctgcccgagccgggcatcaagatcgagctgcgccacccgagcccgatcctcgcggtgatggccaacgaccatccgctggcggcgcagcgccagctctccttgcgccaggtggtggcctatccgctcgggctgccgccgcaggacagctccatctgccaactgctcgacatcagctgcagcaggcaagggctgcgctacgtgcaggccatgtccagcaaccatgcgaatgcgctggtcagttttgcggccgcgggcggcggcagcatcgccttctatggcgagttgtcgatccgcacgcagctgaaatccaaggcgctggtcgccattgcgctgaaagaccgcgaaatgaacgagcgccacctggaggtcgagacgttggcgggccgttcgctgcccgatgcgggaaaagccttcgtgcgatacctgacggatgccatcaaggaagcaatctgaaagcacccgggaaagcggtctttgcggggctgcaaaagcgcctccgatctttggaggccgccgcgtgcgctacactccgcgccgcttgcagacggcctcagccgctgcgccgtcattggcaacatgacgagaacaatccaaaggaaattttcaagtgaaccgtatcgaactggtcgaaaagatcgccaccgcccacaccgtcagcaaggctgaagccgcccgcatcctggaaaccgttaccggctccatcatcgccgcagtgaagaagggcgaccccgtgcagctcatcggcttcggcaccttcaagcaagtggcccgcgccgcgcgcaccggcttcaacccgcaagccggcgcgaagatcaagatcgccgcgcagaaggtgcccaagttcgtgccgggcgcagcgttcaaggccgccatcgaccccaaggctgcaaagcgcaaggccgacaaggcagcagccaagcctgccgccaagaaggcagcgccggcaaagaaggccgccgctcccgccaagaaggccaagaagtaaatcgcgcaacgcgcaagttcgcggcggctgcaaggctgctgctgcgacgacggcccttcggggccgttttctttttcaggacttcttcagttgagggtgcccagccgcgcaaggatcaaatcgtgcagcgtctgggccgccaccgacaggctcccttcccgccgctgcaccaggtagatggaccgcgtcaggccgggcagcggcagcggccgtgtcaccagggtgtcgcgccggaagtgaaaaagcgtgagctccggcaccacgctgatgccgatgcccgcctccaccaggcccatcaccgtggccaggtgctcgacctcgaacaccgcgttgagccggagcgggtgcagggccgcatcgagcgactggcgcacgctgctgttgcgagccatctggatgaagggccagggcgcgagctgctttgccgtgagcctgcgtgcgccggccagcggatggtccttgcggcacacgaggtgaaaacggtcgtcgcagagcttgcgcccacgcaggtcgctggccgcggccgcaccggcccccgtggccgccagcgcgaagtccgcctggtggctgcgaagctgcgcaatgcaggcgtccgacagcgcgtcgtgcagctcgaccgtgatgccgggccactggtgcatgaattccgcgaggatggcgggcagccatccggccgcgagcgagggcagcgccgccacgctcacgcggcccttgcgccgctgggcgtggtcggcaaggtcgccgatggcgccttgcatgtcgtccagcaggcgccgcgccgaaggctcgaacagccggccctcgggcgtgagttgcacgctgcgggtgtcgcggtcgaacaggcgggcgccgagcgtctcttccagcgtgcggatcagcgcgctgaacgcgggttgcgacagatggcaggtctgtgccgcccgcgtgaaattacgctgctcggccagggcggtgaacgcgcgcaactggcggctggaaaggtcgggcgctggcatcggtctggaatctggatgaaatggtccgcggttccggaatttcggctcccgggcctgcggatggtagccctgtgccctgtacgcaacgcgctctcgcgaacatcgatgggcgggatgccagaatcgtggtcttttgtaaaaaaattgtgacttaaggcgcaattcggcatcatgatccgggccatgaagtccggcgaagcatcttctgctgcttggcaacgcgtcgtgtggatggcgcaggttgccgctctttttctggctttcgcagcgacaaacagcgaggcccagcaggccgcgcccgcgcaaaggctgcggatcgtgggtggcctggccagcgtgagccagtacacgcttcaggaggaacccttctggagcaaggatctggcgcgattgagcggcggcaaatacagcgcgagcattgttccgttcaaccaggccggcgttcccggcccggaaatgctcaacctcatgcggctgggcgtcattccgttcgggaccgcgctgctgacccagatcagcaatgagtaccctgaactgggtaccccggacatcgcgggcctgaaccccgacatgccgaccttgcgccgggtgatcgccgctttcaggccttatctggaaaaaacgctgcgcgagcgccatggcgtcgaggttcttgcggtgtatgtctatccggcccaggtgatcttctgcaagcagcccgtgaagcagctctcggacttggcagggcggcgcattcgcgtttcgggcagcacgcaggccgacttcgtccgagccctgaagggggtcccggtgttcaccgaatttgccgaactcatggccaacatgagttcggaaaacaccgaatgcgcgatcaccggtgccatgtccggcaacacgctgggcctgcacaagatcaccaactctctctacacaatgcccatcagctggggcatcgccgtgttcggcgccaacatcgatgcatggaacgcccttcctccggacttgaagctcctgttgaaaagcgaacttcccaagctcgagaccgcggtgtgggccgaatcggagcgcgacaccggcaacggcattgcgtgcaacacaggcgcttcgacatgcgtgaaaggcaccaagggcgccatggtggaggcacgcccttcggcggatgacgagcgccgcaggcgcgacatcttcgccacgagcgtattgacgcgatgggtgcagcggtgcggggcggtgtgcgcggaggtctggaaccagaccgccggccccgtggtgggcatcaaggcacccgtcggacagtgaacaagccgctgccccgccgcatcaccgccttcgtctatggggttgcggcgctgtttctcggcgccgttctgtcgattgccgccctgacgatgtggcagacctaccagaaggcgattgccgaaagcgagatcgaggccaagcggttcgtcggcgcgtcggaagccgcgctcaaccgaagccttctggccgtggacatgctgctcgcgggcatggggcagtttctgcgcaaatccaccgaagccaacgttgcggcggatattgcgcaacccgagacggcgcaattggtcgagaccatcgtgcgccagagcctgctggtgcggtaccttgctttcctgaagccggacggtgcggtcgtcgggtcttccgatcgccggggcgccgggctggcggtacagctgcccgacggattcctgaaagagctcctgaaccggccgggatccctgctggcgatcagcgcgccttcggtcagcctggcgacatcgcagcaggtgctgtacttcgggcgtgtgctccggctcgccgacggcagccggctggtggcggtggccgaagtgcaggtgtcgatgctcaccaccattcttgcgcagggcgcgagtatcaaggggctcgaggtcacgctggagcgcgaagcggggccgctcttggccagcatgccgccgcgcgacgaccttgccggccggtccatcagccccgcggtgaccgaccagatcagcgacgggagtccgcggcggatgcttgcacggctcagcggcactcccgccatcgtcgtggcccgccccacgctgcaacggaacctgctgatcgtcgcgggcatcccgctcacttttgcgctggaggattggcgcagggagcgcgatctgatcctgggtacggcgctggccttcacgctgatgattcttgccgtcagctacttcgcccatctgcagctgcgccggcaatggcgtgcccggggcgacctgcttcgctccaaggccacgctggaccaggccctcgaatccatggtggacggcttcgtgctgctcgaccccgacggccgcatcgtcacgtggaaccgccgcttcgtggactattttccctggaccgagacattgcttttgccgcgggcgacgttccaggagatcgacgaccagaacgtgcgccacctgcaggcacaaaacgagcaggaactcgtcttgccgaatggccaggtgattcttgcggtgaaaagtcccacgccggacggcggcctggtgtgcgtctaccgcgacgtcaccgagaagaggcgccatctcgcggacatcctcgaaggcaaggcgcagttgcaggccacattggacgcattgcccgacgtgctgctcgaagccggcatcgatggccggtgctaccacttccattcgccgcgccgcccgaggtcctccatcaaagtgcgagagccggtcggcaagctgatgtccgaactgttgccggccaatgccgccgccgaagtgatggtggcgctgcgcgacgctttcgagttcggattctcgtccggcaggcaattcgaaagcaggggccccaaaggcgcgctctggttcgagatttccgtttcgcgcaagctgatcggtgaaggcatcgacgcgcggttcatcgtcatcctgcgcaacatcaccgacagcaagctggcggcgcgcgagatcgagcacctcgccttctacgacatcctgacgggcctgcccaatcgccggctgctgctccatcggctgcaagccagcatcgactccaacacccggcggtcgcggcacggggcattgctgtttctcgacctggacgacttcaagacgctcaacgatgcactcgggcacaccatcggcgatgagctgctgaagcaggttgccgtccggcttcagggctgcctgggcgaaggcagcaccgttgcgcggctcggtggcgacgaattcgtggtgctgctcgaaaacctcagcgaagacccggccgttgccgcgatgcagaccaacgccagcggcgaggccattctcacggcgctgaaccagtcgttccagctcgacaaccaccagtaccacagcacgtgcagcatcggtgccgtggtcttcaacgccacgcatcaatcgctggaagacctgctgaagcaggcggacatcgccatgtactacgccaagtcggcgggcggcgacgcgctgcggttcttcgaggtcgccatgcagacggccatcacggcccgcgcgacgctggagagcgaactgcatgcggcgctggaaggccagcagttcttgctgcactaccaaagccaggtcacgtcggaaggccacatcgtggccgccgaggtgctcatccgctggcagcatccggtgaagggattggtgaatcccggaggcttcatcgaactggccgaggaaaccgggttgatcgtgccgatcggcatgtgggtgctcgagaccgcatgcgtgcaactggagcgctggagccacgatccgaggcgccggcacctgcagctggcggtcaatgtcagcgcgcgccagttccgcaccgacgacttcgccgaccgggtctgcgaggtgatccggagaaccggcgccgacccgacgaggctgaaactggagctcacggaaagcctgctgcaggacaaggtgaccgaaacgatcggcaagatgcagctgctcgcggccatgggaatccacttctccatggacgacttcggcaccgggtattcgtcgctttcctacatgacgcagctgccgttgaaccagatcaaggtcgacaagttcttcgtgcagaacatcggggtcgatccgaaggtcgaactgatcatccaggccatcatcgggatggcccgcaacctggacctccagatcgtggcggagggcgtcgaaacgcatcagcagttcgagtttcttcaggcacacggagccatgctgtgccagggctatctgttcagcaggccggtgccgatcgaacaattcgaagcacagctggacctcgcgatggccgactgaacgcatgccgcgctgagcgagttcacacgatgcgccttcctctcagcctcccacgctccagccagccgcgtttcagcctgcgcgctcgtctgtccgcgggcgtggttgcgatcgttttcctgacgaccttcggggtgaccaccgctgcgctctacttcatcaagcggaacatgcaggccgccattgccgacgagcagctcgaacgcatatcggccattgccgacgcggtggaccagaagttcctgagccgccgcaccctgctcaagacctttggcgacagcgtcgagagccacaatttcaccagtgccgacgggctgcaggacctcgtcatgcggcacgagtcgctgaaagaggccttcgacaacgtcgccttcgtggacgtcgacggcaagctggtcgccaacctgaacggcgcgcaccagatcgggcgggtcaacatcaaggaccgcgagtacttccagcgcacgatggcagccaaggccggcgtgatctccgagccctaccgcaatcggctgaacggcttggcgcagatcgccatgaccgaaccggtgctggaccggcagggcaacgtggcctacgtcatcgccgcctcgatcaacctgaaggagcagaacttcctcggtgaacttgccaacgtgaaattcggcaagacgggctacatgttcatcaccaacacggacggcatcgtcgtcgaccatcccgacaagtccaggctgctccagcacgtcaacgccgatggcaggagcaatgccgccgcggagcgcgccattgccggccacgagggcacgatagatgccgtgaaccgcaagggcgtgcgcgggctctacgccttcaagccgatccgccagaccaactgggtgctgggcgcgatgtatccgcgcgacgaagcctttgcccggatcgagcagatcgagcgcttcgcatgggccggcgtattgctgctgacgttcgtggccggcaccattgccttcgtgaccgcgcgttcgcagctcgcgcccttgtcccggctgcgcgagcacatgcaggtctcgcgcgcggctgcggcctatgcgcccatgaaggaggcgcctcccggggacgaggtcggcgacctgtcgcacaccttcgattcgctgatgcaggagcgccaggcatctcaggaacgggtgcaggcgagcgaaagattcctgcgcgacgtgaccgacaacctgccggcggtggttgcctacttcgacagcgagcagcgctgcctgttcgccaacaaggcggggctcggcatgcgcggcaggacgcgggccgacatcgggcgcatgaccatgcaggagtcgctgcccgatccggtctaccagcagctcgttccgcacattgccaaggtgctcgcgggaacgccgacgcgtgcggagggcacctacgaccgcaacggcaaggaaggcttcttcgagtgccatcttgcgcccgatattcgcgacgacggcgtgctggccggcttttacgtgatgaccttcgacatcacgcgccagaaggtggccgagcgcgagcgggcggccggcgaggcccgggtacgcaccatcaccgacaaccttccggcgctggtgtcccacgtggatgcgtcgctgcgcttcaccttcgtgaacgcgcatctgcgggccttgttcgacggcatcgagctggtgggaaagctgctgcccgacgtgcgcggcgccgaggatttcgaggtggtcgagccctacgtccgccgcgtgctcgccggagaagcggtcaccttcgagaagaagggtgatcccgcacgcggcgtcggccaaaaatggtaccagtcgcactacgtccccgaccgcaacaccgacggcaccgtgcgcggcttctatggcatgaccttcgacatcaccgagcgcaagcaggccgaaatgcgaagcgccgagagcgagcgccgcctgcggggcctgaccgacaacgtcccggcgctcctgaccgaactggaccgcgaggagcgggtggtcttctgcaacggccgctaccagacctggctcggcatatcgccggatgcgatgatgaaccggcccatccgggagttcatcggcgatgcgcactacgaaatgcgcaagcccctgctggcacgcgccttcgcgggcgaggtggtgtctttcgagcagacggcccggctgctgatcggcgagcggaccctgcagacaacctatctgccgcagaagaatgccgagggcgaggtcgtcggcctgtacgtgctggcgaacgacgtcagcgacctgaagcaaaagcagctgcagctggacgttcttgcgcgcgaagatgcgctcacgggcctgcccaaccgccggtcgttcgaagagcatgtgcgcgacgccatggccaggtcgcggcgcgcggggctgtcggtgtgcctgctgttcctggacatcgactatttcaagaccatcaacgattcgctgggccatgcggcgggcgatgcggtgctgagggagttcggccgccggctccggcagagcgtgcgcgacaccgacatggcggcacgctacgccggcgacgaattcgtgatccttctcgaaggcgtggccggtgccgccgaagcgcaggtggtcgcgggcaaggtgctggccgccatgcggccggccttcaacctgcccggccgcaccctgcatgcgacgaccagcatcggcgtcgcgctgtcggaagaagacgaggacttcgcttccttgttcgtgcgcgccgacaccgcgttgtatgcggccaagaaagagggcaagaaccgcttcatgatggccgcgcccagggctgaagccaggcccggcgcctcgtggccgcgccaagagccttacagcgcctgaggccgcgcgcccgtcgggccgacaccgcccgcaatctcggccttgtcctacgcggaaggtatctgctgctgcacagaattggcggcggtactttcacgggcagtactttcacggacaaaaagcaatggcagaacacggcggtgggggtgcaccactcaaccaacgcactctgaccgacgccgactaccggctgatggtcgagacggtcaccgactacgccatcaccgtgctggatcccggcggcatcttcgtcagctggaacgacggagcgagaaagctcaacgggtacgagccgccggaagtgctcgggcgccacttctcgctgctctacccgagcgagctgctcgaccagaaccggccggaccacgcgctggcgacggcgcgtgacgccggccatctcgaagaagagggctggcgcctgcgcaaggacggcacgcggttctgggccagcgtcgtcatcacgccgatgaccggtccgggcggcgaaatccgcggctactccgtgatcacccgggatctcagcgagcggcgccgccaggacgagatgctgcgcctgagcgaggagcggttccggctcctggtcgaaggcgtgaaggactacgcgatcttcatgctcgaccctggtggccacatcgtgagctggaatcttggtgcgcagaagaacaagggctacgaggcgtcggagatcatcgggcagcacttttccaagttctacccggccgagctggccgcgagcggctggccggaacaggagttgcgctatgcgcttcgggacgggcggttcgaggacgaaggctggcgcatccgcaaggacggcagccggttctgggccagcgtggtgatcaccgcgctgcacgacgccaccggcaagcaccgcgggttcgccaaggtcacgcgcgacctgacggagcggcgccgcgtcacggcgctcgaggacgaggggcgccgcgtgacgaactttcttgccatgctcgggcatgaactgcgcaatccgctggcgccgatctcgaatgcgctcgagctcctcaagcgcgaaaagacggattcagcggtggttgcgcacacccgcgacatcatcggccggcagctcaggcagatgacgaggctggtcgatgatctcctcgacgtgggccgcatcacgagcggcaagatcctgctcgaaaacaagccggtgcggctgcgcgacgccattgcccaggccatcgaggcagcgcgcccgctgatcgaaggcaaggcgcaggccctgcacctggagatgcgggacgcggatccatggattgccggagacagcgctcgggtcatccagatcgtgagcaacctgatccacaacgcggccaaattcacgcaggacggcggcaacatccatgtgtcgctctcgcagagcggcaccgatgccgacatcagcgtgcgcgacgacgggcccggcatccagcccaaggacctgcaccgcatcttcgaccttttcgtgcagggcgagcagaacatggcaagaacccagggcggactgggcctggggctcagcctcgtgcagcagctgacgacgctgcatggaggccgggtgagcgccttcagcaccggaagaacgggcgagggcagcgagttcgtggtgcagtttcccatcgcacaggcgccgattgccacgctcgaggcgcagccccggcccttgggagagcagcgcgtgctggtggtggacgacaacgtggacgcggccgagaccatggcgctgctgctggaggcgctcggctacacgtccagcattgcgcatggagggctcgccgccatcgaggccgtcaaggcgcacgacccggacatcgtgctgctggacatcgggctgccggacctgagcggccacgaggttgccaggcgcttgcgcgcggagttgatcaacccgccgccgctgatcgccgtgaccggctacggccaggccagcgaccgggaaaccagcctcgaagccggctttcgcgcccacctgacgaagccggtcgacgtcgacaagctcgcggcattgctcgaacgcctgctggagccgccgcttcagtcgaaggcggcgtagcacgccgccggcgacacctcctcttgaggcggactagaaatccaccaggctcaggccgatgctgagcaccgtgcgcttgcggttgtagtcgaccagcgtgtcgccgtagccatggaacagctgcgtgtggaagcgcaggttgctcgcggtcgagtcgccgatggccttgagccattcgagccggaccgatccgcggccggtgtcgcgcaggttgttgcgcaccgtgatgcccagggtgttgtcgcggttgaagttccagcggcccgtgacttcggcgcggccgatgtagttggagatgtcggggttgtcgtcctttgccgcatcttccgacatccgctgccagatgcgcccggtgatgctgaagcggtcgtcgagctcggcaccgcccatcaggtacacgcggttccaactgcgcgacagcggcaggctctggccattcgactggtgcaccacgcccacgcccgcgtagcgccagcgccagccaccgggcaggttgaagtcgagcggatagacgtacatcagctcgggctcgtggtcggtggtgcggaacggccgcgagaccgagccgttgaacagctgccaggtcgactgctgcgagtacgcgaaccacagcgagtccttcttggccggctcgttctgcgtgagcaggccctgagcgaccttggtacgcacggaaaggccgatgcgcatttcgttggcctggtaggccacgtcggacgcggtgtggccgttggagggcgacgtgggcgtctcgggcttgctgctggcggccgaggccgacacgttcagcggccgatagccgcggaacacgaaggcgccgcaatcagtgccgttctcgagttcccagaagcgagacaggatcgaatactgccggtcgcggcagccttcgctggtggcgaccgaaaccacgcgggtggccggaatcgaggcgtccaccggcggaggcggctgcgtgctggccagcacgggcggcgccaccggcaccgagaccgaaggcagcgtctgctgctgggtccagcggtcgaagcaggccaggcgcgcttctttgttgttgctgagcgcggcgcattgctgccaggtcagttgggcatcggccagcgggctgcgcggcctgtcgaccgcttgtgcgtgcaccggcgccgcaaagaggccgggagccagcagcaggcctgcggccagcgtggtgcgtagatggattgcgttcatttctctcgggtccgttccgtctttttcagagtgaagggatgtgtgctgtcgtcggcggcattgcgccatgtgcccttgaactcgcggccgcacgagtccggctgcagcgagcccgaccacacgccgctgatgctgcggccgtcgagcgattcgtcgatggcaagttcgccctcgtcgtcgacgtcgcccgcgagctgggccacggaagtgcgcgccgaaggtagggctgccgtgcgcgtgatggtgccgcgcacgcccgcgtactcggggtgcttgccgagccgcaccagggccgcatcgggcaggccgtcgaagcgcgcctgccagtcgccatagagcgcctcgatgggcaggtcccgcgcggtggccgggcagccggcctctgccgtgtgcgggcccgcggggccggcgcatgccgtgcagagcgccgccacgaggagaagagcgaacggtgtcttcatggtgcggaggcggctgctgcggcggcggccgcgctgtcctgggccttgcgcgcgaactcggcgcgcagtgccttgagtttttcgcgcgggtcttcgcgggtggtggtcttgtccaggcccatctcggcgatgaagcggctcggcacgcagggcaccatctcgcggccctgcttgcgcttcttggtccagctcaccgccaggctgcgctgcgcccgggtgatgcccacgtacatcaggcggcgctcttcctgcagccgctgcagcgtctcgtcgctcaccttgagttgtcggccgttgtcgtcttcgagcttgaagggcagcaggccctcggtcacgccgatcagcatcacgtgcggccattcgaggcccttggatgcatgcaacgtggagagcgtcaccacgttctggtcctgctcgcgctcgctgatggtggagagcagcgagatggtctgcgccacctcgagcaggctcttgcgctcgccttcaatgttgtcgttggcgcccgaggcatcgtcgaggccgccgcccgcgcgctgcgacatccagtcgacgaactccagcacgttggtccagcgcgctgccgctgcctgctcgctgtcctcgccgtcgtacaggtgcttctcgtagtcgatctccttcaaccagtcgagcatgaaggtgcgcgaatcttcggcgcccatggtgcggcgcgcgcggtattccaggtcgttgatgtagcggccgaactcgtggatgccctcgagtgtgcgcttgggcatgacgctcggcagcgacgggctgaacagcgcctcgaacaggctcagcttgtactggctggcaaaggtgccgaggctcgcgagcgtggtgtggccgatgccgcgcttgggcgtggtgatggcgcgcaggaacgcggggtcgtcgtcgttgttgacccacaggcggaaccagccgcacaggtccttgatttcggcgcggtcgaagaagctctggccgcccgacaccttgtaggggatctgcgccttgcgcagcgcctgctcgaacacgcgtgcctggtggttggcgcggtagaggatcgcgaaatcgcggaactccttgtactgcttgccttgcgtgacggcatcgcccgcgcgcaggctgacgatgcgcgccacggcgcgctcggcctcgtgcgcctcggagtcggcatcgacgatgcgcaccggctcgccttcgccgagctcggagaacagcgtcttcggaaacagcttggggttggggccgatcacgttgttggccgcacggaggatcgcgctggtcgaacggtagttctgctcgagcttgatgaccttcagggtcgggaagtcgaccggcagcttgcgcaggttgtccagcgtggcgccgcgccagccgtagatcgactggtcgtcgtcgcccaccgcggtgaagcggccgcgctcgccggccagcgccttcagcacttcatattgggtggcattggtgtcctggtattcgtccaccaggatgtggcccagcgcggcctgccacttggcgcgcacctcgtcgaaatcgcgcaacagcttgagcggcatgccgatgaggtcgtcgaagtcgacgctctggtaggccgtgagccgctcttcgtagcgcgacatgatgcgcgcggtgatgcgctcgttgtcgtccgccgcggccgcttcggcgtctgcggcattgaggcccatgttcttccacttgctgatggtccactgccagatgcgcgcggtggccgtatcggtcgtgccgccggcgtccttcaggatcttggtgacgtcgtcgccgtcgagaatgctgaaggcgggcttcaggcccagcacggcgccgtcttctcgcatcatgcgcacgcccagcgcgtgaaaggtgcagatcaccacgtgcttggcgtcgcgcccgatcagccccttggcgcgttcgcgcatttcgctggcggccttgttggtgaaggtgatggccgcgatgcgcttgggctccagcccggcctggatgagccggccgatcttgtgcgtgatgacgcgcgtcttgcccgaacccgcgcccgccagcacgaggcagggcccgtgcaggtaattgaccgcttcttgttgcgcgagattgagaccggaagacatggagagtgggaacggaaggcccgcgggagaacggcggacgcaaagcgcgcaatgatacggggcgcatgtttccggaggggccgccagagttcacgatgcgagacgcaacgacaatggggccgtgctcgctgtatttctcgtaacttttcctttcttcgccttgatcgcggccggctatggcgccgcgcgcgcccgcgtcctgccgctcgatgcgattccgggtctcaacaccttcgttctgtacttcgcgctgccttgcatgttgttgcgatttggcgccggcacgccgatcgggcagctgctcgacggcagcgtcgcgctggtctggggcctgagcgcgctggccgtggtggcgggcgtggtggtcttcacccgcaatgcacgcatcggctggaacgacggtgccttcggcgcgctggtggccgcctttccgaacaccggcttcatgggcgtgccgctcctggtggcgctgctcggtgcagaggccgcgggaccgatcatcatcaccatcgccttcgatctggtcgtgacctcgtcgctgtgcattgcgctgtcgcgcctcgacggagtcagtggcggcggcggtgcggcgcagcgcggcccccggcaggcggcacgccaggcgctgcgcggcgtgctggtcaatccgatgccgtggtcgatcctgctgggcgtgctgctgtcggccgcgcgctggcgcctgccggggccggtggagcgcaccatcgccatgctggccgatgcggcttcgccggtggcgctcttcaccattggcgcggtgttggcgcggtcggccttgcttgcgcgggagcacggggccagcgcggcggtggcggcggccatgggcacccggtcggccgttccgcccaaggcgccgctggccgacgtgctgccggtggtgctggtcaagctgctcgcgcatccggtgctggtctgggcgctggggcagggcgccatcgcactcggcctgccgctctcgtcgtcggcgctggtggtcatcgtgctggtggcggcgctgccgagcgccagcaacgtgtcgatgctggccgagcgcttcggagccgacaacggccgcatcgcgcgcatcatcctgtggacgacggtggcgaccttcttcagttttccgctggcggtggggctgctgcgctgaaccggcgcgccccggcctcaggccgtcagggggtcagtacgccgagcttgaaggggtcggcgtccggcaggcgctcgcacttggagaaatcgcggccctggctgccgtcgcaatagaacgcgttgtagacgagcccgaagagcgtggggctggccgtgaagagcacgccatggtcgggctgccagttgtccttggccgacccggtgctggcctccggctgcctggccgggattgccgccgagatgggcgtgaattccgccagcgtcttgtgggcttcgtcgccgcgccagcgcgacgccagttcggtcgccgagggcctggttgccacgggcagcagcacgccgttcacctgcaggccgtagtcgaagcggtgcgtcttgccggccagaaaggcgtaggcgcatgcggccatgcactggccgcggacctcggtgtccacgccgctcgagcggatggcgtcggcataggcgccggccgcctcggcggtgccgccgaacgaatcctcgaacaccacggtgcgcacggtgcccttggcaaggtactgggtgaaggtcttgacggtgctgccgtcgagcatgcccgacaccaccagccggctgccctgcagttcgagttcggccgccgggcatgcgaggcatgcgaacaaaagagccgaaccgagagataaaggcagtttcacgacaacccctgcaaaccagcgtgcttgcttgatgcgcggagccgaaatgggcttcgcacagcgacagcttgcgcagcgcgcgaggggtcagtcaacttctttttcagaatatttcccgctttgcgactggccgtaagacatacctactggtattaccgttattacttcagatgaatacttgtgttttcattgcacctgctagagtgtttgcaaatcaaagtatgaatgggtagcacgatgacaatacttgttcgtgtcctgttgtggctggcatgggttgctggcgtgagctggttctggcacgccggcgagctcggcaccggcacttcgctggccctgggcgccctcagcctggtggtgttcgcatggcccggcagcatcgcgcggcgccgcagctccgaactgcgctatatcgacgtcggcaaggagcccgcaggcctgcaccactgaccgcgcggcgcgcacggctcagatgctgtgcggatcgacgtcgacgagccagcggatcacgcccttgccttcgggcgtgcgccgcaacgcgtgcaagagcggctgccacccggccagcaggcgctgcagcgccgcgcgcgaggggctttcgatgagcatctgggctctttccacgttggccacgcgctggatggcaagcggcaccgccggatagcgcaccacgcggtcggcgccttcgagggcatcggcggccgcgctcgcggcattcaagaaagcctgggcggcctcctgcgtgcgcgcatcggcccgcagcagggcctggaatgcgaacggcggcatgccggccgcggcccgctcctccagctgctgccgggcgaaagcggtgtagtcgtgcctgcgcagcgcggcaaaaagcgggtgctgcgcatggtgcgtctggatccacatctcggccgtggcgccttgggccgccaggtacgcagcgtcgcggccggcgcggcccgccgattgcatcagcaggctgaacagccgctcgggtgcgcgaaagtcgctggagaacagcgcgccgtcggggttcaccgccgccaccagggtgatgcggcgaaagtcatgccccttggcgatcatctgcgtgccgaccagcacgtcgacctcgcccgaatgcacggccgccagctgcgattcgagcgcgccctgcttcttggtgctgtcggcatcgatgcgcgcgatgcgcaccgcagtgccgtcgggccgcttcaccgccgcgaacagttcggccaggtgttcttcgagccgctcggtgccgcggccgacgggtgcgatgtcgggattgccgcaggacgggcaggcgcgcggcacgcgctcggtaaagccgcagtggtggcagcgcagcgtgcggtcgatcttgtggaacacacggtaggcgctgcaatgcgggcattcgctcttccagccgcaatcggcgcaggccagaaccggcgcgtagccgcggcggttcaggaacaccatgctctgctcgccgcgcgcaatgcgctggccgatggcgtcgagcagcgcgcccgagagcacggtcttgggcggctgcaggttcgtgtccacgagccgcaccgcgggcagctcgcccgcgccaatgcgcgacggcatggccagccgcacatagcgcccgcccgggtcttcgccctcggcggggcggctctggtgccagctttcgagcgagggcgtggccgagcccaggatgacttttgcgccttcgcgctggccgcgccacacggcaaggtcgcgcgccgaatagcgtgcgccttcctgctgcttgtagctggggtcgtgctcctcgtcgaccacgatgagcttcagccccggtatcgacgcaaacaccgccatgcgcgtgcccagcacgatgcgcgcggcgccgctgtgcgccccgagccagctcgcgagccgctgcgggttggtcatgccgctgtgcagcgacaccaccgcctcgtcgccgaaacgcgccttgaagcgtgcttcgagctgcggcgtcaggttgatctcgggcaccatcaccagcgcctgcgcgccggcatcgcgcgcgagcaggtccgccacgcagcgcaggtagacctcggtcttgccgctgccggtgctgccgaccagcaggaaggtgcccgtctcggcttcgatgcgggccagggcggccgtctgctcggggctcagcgcgatcaggttggcggcttcgtcggtggcggccacggggccggtcgtcgccttgcgtttgaggcggcgcgccagttgggtcgtcgtcaggtcgcgcagttgcggcggcagggcggccagggcgatttcgccgatcgagcgctggtagtagcgcgcggcaaaggcgaccaggtcgcgccaggcttcaccgagaggcgacagcgcatccagagccgcgccgacgggcttgagcgccatgtcgggctcggcgccgtccagcgagcttgcctcgttccagaccacgcccagcacctcgcgccggcccagcggcacccgcaccagcgtgccgggcgcgagcggcgccgcgccggtgtagctcagcagatcgccaagggcggcatgcgcgggcgtttgcaccgcgacgtcgagccgccaggccatcgctgcgggtgcgctggccggtgttgctgtttccgtttcgggggcttcgacggggggagaaatgggcgtccttgttggcaaggtttgttaatgcgactttgagcaaaaccacttaagttgttgatttttcagcggtttgacagtcgtccagagtttctgtggataactttgttgacaacagggctcgacacgcccgcaagccttacagatcaagcgtctgactgggttgccctcaaaaaaagcaaaatccaaatcctatatgaatcaacaacttacggctgctattggtttggaagcaaagagcgaggctcttcagatgttctggcgcagtgcagcacatgttttgtgcataagtcgggcctcctacaccgtttttacgcttgacaaacggcttggattggattttcaacgccgcgagcgtcctggcgcagcccgcccgcgcggttacacaagtatcagccctcagccctcagccctcagccctcagccgcgcagggcgcgcgattgggcgtgcaccgcctgcaccagcgctgccacgtggtccggcggcgtgaactggctgatgccatggcccaggttgaagatgtgggtcggcccgggcacgccggcatcggtgtgcggcttgccgaaagcgttcagcaccttggccacctcggcttcgatctgcgcgggcggcgcgaacagcacgttgggatcgatgttgccttgcagggccttggccttgtcgccttcgcccaccagccgacgcgcggccgcgaggttcacggtccagtcgacgccgagcacttcgcagtcgagcgcgcgcatggcctcgagccacaggccgccgcccttggtgaacacgatgcgcggcacgggttgcccgtcggcgccgttgcgcttcaggccggccagcacgcgcgccgtgtaggcgaggctgaattcctggaacgcgccgtcggccagcacgccgccccagctgtcgaacaccatcacggcctgcgcgccggcgtcgatctgcgcattgagataagtggccaccgaatcggcattcactgcgagcaggcggtgcatcaggtcggggcggccgtagagcatgctcttcacgagccggtagtcgctcgagcccgcaccttccaccatgtagcaggcgagcgtccaggggctgcccgagaagccgatcagcggcacccggccatcgagcgccttgcggatcgacgccacggcgtcgaacacgtagcgcagcttggccatgtcgggcacttcgagcgccgcaacggccgcttcgctctgcaccgggcgcgcgaagcgcgggccttcgccggcctcgaacgacaggcccaggcccatggcgtcgggcacggtgaggatgtccgaaaacaggatggccgcatcgagcggatagcgcgcgagcggctgcagcgtgacttcggtcgcgtagtcgacgttggtcgccagtcccatgaagctgccggccttggcgcgggtggccacgtattcgggcaggtagcgcccggcctggcgcatgagccagacgggcgtgtggtctgtggcctggcgccagcaggcccgcaggaaagtgtcgttttgcaatggggcgaaaggcatgtcccgattgtcgcaggggcccgtgcccgcgcgcccgcggttatcccggaagccgaccggtggcggccgtgcgctcagaccgccggcactcccacgggcggcgacttggccgcactgcgccggtacagcaccagcgttgccaccagcccgcaaacggcggccgccgtcatccacagccccggcgcgcccttgtcgcccgtcatctcgatgaggccggtggcaatggccggcgtgaacccgccgaacagcgccgtcgcaaggctgtaggccagcgagaagcccgcggtgcgcacattgaccggcatcacctcggtcagtgccaccaccatcgcaccgttgtagctggcataaaggaacgacagccacagctcgacctcgagcatgcgcccgaagctcggggcgcccaccagccatttgagcgacgggtacgcggtgaagatggtcagcaccgtgaacaggatcaagagcggcttgcggccgacgcggtcggacagcgagcccatcaccggcagccagatgaagttcgagacggccacgcacagcgtgacaatcagcgcatcggtcgtgctcaggtgcagcaccgacttgccgaaggtgggcgtgtagaccgtgatcaggtagaacgacaccgtggtcatcgacaccagcatcattcccgccaccacgaggccccagttggccaccatcgactggaagatctcgcgtgcgtcgggccggtgcttgcgcgccatgaactcctcggtctcctgcagagagcgccggatgacgaagagcaccggcacgatcaggcagccgacgaagaacggaatgcgccagtagaagtcgccgatctgctgcgaggtgaaggtcacgttgagccaatagcccagtgccgccgccacgatgatcgccacctgctggctggccgactgccaactcacgtagaagcccttgcgccccggcgtggccatctccgacaaatagaccgagacgccgcccagttccacgccggccgaaaaaccctgcagcagccggccgacgagcaccagcagcggcgccgcgaagccgatggtggcgtaggccggtacgcaggcgatgagcagcgtgccgagcgccatgagcgcgagcgtgacgatcaggcccttgcgccgccccacgcggtcgacatacgcaccgagaaaaatcgcgcccagcggccgcatcaggaagcccgcgccgaaggtcatgaacgtcagcatcagcgaggcgaactcgtcgccggccgggaagaatgccttcgagatctgcgtggcgtagaagccgaacaggaagaagtcgaacatctccatgaaattgccgcccgtcacgcgcaggacggtggccagtttcgaggaggagccggtgcttgaagaaagggcgcgggcggccgtgcccggttgcgcgtcggagtgcgcaggattcatctcgttgtccccttgggcgatgtaatgcgccaagggtaggccggggttcccgaccgctgcctgaccgtgcgagtcaggtagctgtcactgcgcgactgttctgcttcagctcttgtacttgaccgagcagccgtagggccgcgtcgaggccgccgagatcggtttgccgccaaagacttcgcccagcgcctggttcacgtagttggtcgcggccttgatgtcgtcgggccgggccgacgcgatgctgtcgatgccgcccgcgtacaccagcatgcccttgggatcgatgatgaagatgtgcggcgtggtgcgcgcgccgtaggcctggccgatcacgccgtcttcgtccatcagcaccgcggtgggcgacgccttttgcgacttcatccatgcgtcgagcgcggcgggctgcaggtagtcgctggccgcacgctcggtggagttgaccgacagccagaccacgccctgggccgtggcggccttctgcgtggcgggcatgttgccgctgttgtagtgcttgcgcacgaacgggcagcccgggttggtccactcgagcaccacgaacttgcccgcgaagtcggagagcttgtgcttggcgccgctggtgtccacggcaacgaagtcgggcgcctgctggcccacggcgggcgcggcgaaggcgtggttgcccatcaggaaggtggcacccagggccacggcggcggccaccacggcgcggcgcgaggcgcggctgagggcggcgcgggcgtggcgcgcggcgcgaatggaacgcgagtcggacgatggcgaaagtgacatggccagcttgaactccaaaagaaaaaaacgaacgacggcgacagcttagagcgctttgctcacgtgcatgtgacaacccatgtcacgccggggtcaaagcgcggcgagcgccgcgcgcacctcgtccttgcccagaatctcggtcagcacgatcggcggcttgccgggcgcctgcagcacgtacagcggcacgccgctgcgcccgaacgaggtcagggcggcggtgatggcgggatcgcggcgcgtccagtcggcccgcagcatcgcgaccttcttgctgtcgaagtcggccagcagatcggcatccgcgagcgtggccttcttgttgtactggcaggtcacgcaccatgcggcggtgaagtcgatgaacacgggccgcccggcgccggtgagttcggccacgcgctcggtcgaccacggctgccagcgctggccggcattggacgcgagcctggcgggctccaccgtctgcatcacgttgcggccgatggccgcggtgagcaccgccgtgaaggcgaccagcaccgtggcaatcacgagccgcgtgcggccgcgcagcgtcagcgcccagacgatggcggccatgcacaccagcagcgcgagcagcgtgcccgcaccgtcgatgccgctttgctggcccagcacccagaccagccaggccacggtggcgaacatcgggaacgccagcagccggcgcagggtgcccatccacgggccgggcttgggcagcagccgcgccacggccggaatgaagccggcgaccaggtacggcagcgccagccccaggcccagcgccgcgaacagcagcagggcctggacggccgggagcccgatggcaaagccgagcgaagcgcccatgaacggcgcggtgcagggcgatgcgatcaccacagccaggacgcccgacaggaagtcgttggcgatcgggtgcttggcctgcgcggaacacagcgacgaaggcgccgcacggccgaactcgaacacgcccaccaggttgagcccgatcagcgtgaacagcgccgccagcgcggccaccacggctggcgattgcagctggaagccccagccgagctgggcgcccgccgcgcgcagcgccagcatggcgccgccgagcgcgaggaacgagagcatcacgcccgcggtgtaggccagccccgccgtgcggtgggcgctgcgattgccggcctgccgtgcgaagcccagcaccttgatggccaggatcgggaacacgcagggcatgaggttcagcagcaggccaccgagcagggcgcccagcaacgcgaggacgaaggtgcccgcgggctggggcggcaacgccgtgggcgaggccggcgcgccggcattggccgcgttcgctgcattggcggccagcgcggcctgcagcgcgggcgacacttcggcgcgcggcgcggcggccgcgggccaggtgccgccgaccggggcctcggtgcgccaggccaccggttggcccggctgccggtcgggctcggccagcgccaccaccagcggcagcgtcgccgggctggcgctgcgctgttcggccagcggcagcgtggcggtccaggtggcgccttgccagctttgcctccagtccttgcccgactccgcggcggtgcggatcagttcgggcgtttcggggaagaagccaagggtcttgccctgtgcggcggcgggcaggccttcgaggcgcacttgcaggttgttgccattgacctcgacggcgcccggcttggcgagcggttgcggctgggccgcctgggccgcgtcgaaatcggccttgtgcagcgcagtcgagccctgcagcggcagcgcgagggtgaattcgccttcctcgggaatgcattccttgcggcacaccagccacgtggccttgagccggacgtcgagcgctgaagccccggtgccaagggccagcggcggcttgaaattgctcgacacctcgagcggcaccggcagcagcaccgtgccctcgtagccgtagttggccaggctgccgaccggaatcttctttggcaccggccaggcgatgtcgccggccgccacgcccggcggcagcgtccagttcagttcggtgggcaggccggaatcgccggcgttcttccagtaggtgtgccactcgggctggtgggtgatctgcagcccgacccagaccggcgcgcccggcgccacgccttggggcgcgtgcgcgaccagttcggcgcgcacgtggggggtggtgaccacggcacccggcttggatgccaattgggccgcagccggcatgcaggctgcggcggttgctaccagaaacgtagccagatgaaagaagcgggaaaagatcatgccggtgagtcggagcaggcgggcggtgcgaagttccgggtattcatggggcctcaagcggcccagcccagcaccacgcggcggctgttggcgctctttttctcgattttggtgaccaccaccgcgccaatctcggaagtgtttgcaacatgcgtgccgccgcagggctggaaatcgatctgcgcaccgccctcgccgccgatgcggatggtgcgcacggtgcccgtgccgcgcggtggctgcacgctcatgctcttcaccagcgccggattcgcgtcgagctcctcgtcggtgatggcgcccacggtcagcggatgcgccgcgcccaccagccgcgcgaggccggcggtcagcgcttccttgtcgagcggatcggtcatgtgaaagtcgatgcgcgcgtagtcgggcgtgatcgagcagccgttgaccggcaccggcacgaggtggcacagcaggtggctggcggtgtgaaagcgcatcagccggtggcggcgctcccagtcgaggcgcgccgtcaccgtgtcgccgggtttcagcgcggcgagcagttcggcctgcccaggggccggcacgtgaacgaactcggcggtgggctggccttcctcgttcttcgcctttcgggtgtcggcaatggcgatttcgcggccatcggccagcgccagcacgccggagtcgccggcctgcccgccgcccagcggatagaacacggtgcggtccagcacgacgccggtctcgtcgatgcgcagaatgcgggcttcgcaggtgcgcaggtaggcgtcggcacggaacaggtcgtcggtcatgcggccgatggtagcggcgatgcgccaatggggtgcgcccacgccaaaaagcgcccatgaccgacagcccttgccggcgccgtccgcatgatctgcttcaaagcggccggcatgccgcgacaaccgaggagagcgaatgaaggtaccgaacatcgccgtttcttccctggtctccatggccgccgtggccgcggcgctggcgctggcgggctgcggcgaagccgccaagctgccccccgaagccaccatcggaccgcggccgcaactggcccagcccaacaggaccctgattcccaccgtcaacgtggccaccgcggtagggtggtcggacgccgccgggcccaaggccgccgacggcctgcgcgtgaatgcgctggcgcgcgggctggaccatccgcgctgggtctataccctgcccaacggcgacgtgctggtggccgaaagcaacaagccgcccaagcccgaaggcagcggcgacggcggcggtcctatggccaagatccgcaactgggtcatgggcaaggtcatgagccgcgcaggcgcgggcgtgccgagccccaaccgcatcacgctgctgcgcgatgccgacggagacggcgcggccgaagtgcggcacgtattcctgtcgaacctgagttcgcccttcggcatggcgctggtcggcaacgagcttttcatcgccaacgccgacgcgctcgtcaaggtgccctacaccgaaggccagacctcggccagcgccacgcccacggtggtcacgccgctgccggcgggcatcaaccaccactggaccaagaacgtgatcgccaatcccgacggcaccaagctctacgtcacggtcggctccaacagcaacatcggcgagaacgggcttgcggccgaagaaggccgcgccgccatctgggaggtcgacgtgaagaccggcacaaaacgcctgttcgcgagcggcctgcgcaacccgaacggcctggcctggcaccccgagaccaaggcgctgtggaccgtggtcaacgagcgcgacgaaatcggcagcgacctcgtgcccgactacctgacctccgtgaaagacggcgccttctacggctggccctggagctacttcggcaaccacgtggatgcgcgcgtcacgccgcagaagcccgacctggtggccaaggccctcgtgcccgactacgcgctcggctcgcacgttgcgccgctggggctggtgttttccgacggccgcggcatgcccgccgaattcgcgagcggcgccttcatcggcgaacacggctcgtggaaccgcaagcccaagtcgggctacaaggtggtgttcgtgcccttcatcggcggcaacccgagcgggccgccggtcgacgtgctgaccggctttctcacggcagacgaaaaggcgcagggccggccggtgggcgtggcgctcgacaagaacggcgcgctgctggtggcggacgacgtgggcaacgtggtctggcgcgtcacgcgggcaaagccgcagtaggccgcaatggcgtctggcttctagcgccgcgggcggccgattcgaaacagccggtgccggcgcagcgcgtgcccctcgggcacgctcgggtgatcgaaagcgccgggcaggtcttcatgcatgccgatacgttccatcacggccgccgagcggagattgccgagcgccgtgaacgccacgatctcgtcgagcccgagccgctcgaagccgacttgcagggcgccgcgcgccgcctcggtcgcgagcccctgaccccaccactggcgcgcgaagcgccagccgatctcgacgcacggtgaaaagggcagcgtggccagcggcgcgttcaggcccgtgaaccccgcgaacccgcccgaatccttgtgctcgacggcccataagccccagccgttggcggcgatgcgtgcctggaggctcgccgccagcgcatcgctgtcggcgcgagtgggaagcggcagcaggaatgccatgacttccgggtcggccgcgagcgcggcaaaaggcgcgaaatcgctctcgcgccactggcgcaaccgcaggcgcggggtttcgaattcgatcgggggctggatgctgtcggccatatgccgattgtgctcagaaccccgcgagcaccaccttgccctgcgcagtgccgctctcgatgagcgcatgcgccttcctgaggttggccgcattgatggtgccgaagctcgcgttggcggtcgtgcggatgcggcccgcatcgaccagcgccgccacttcagccagcagcgcgccctgctcggcgatgtccggcgtttcgaagcgcgagcgcgcgaacatcatttcccagtgcagcgagatgcacttggtcttgagcggcatcacgtcgagcgacggcaggtcgtcgatcaccgcgagctggccctggggcttgaggctttcgatgatctgcgcgtagtgctggccggtctgcgtgaggctcgcaaccatgtcgacctcgccgatgccggcggccttgagttcggccgcgagcggcttcgaatggtcgatgaccacgtgcgcgccgagcgccaggcaccaggcccgcgtctcggcccgcgaggccgtggccaccacgcgcaactgcgtgagctggcgcgcaagctggatcaggatcgaacccacgccgccggccccgccggtcacgagcagcgtctgtcccgctccgccgttcttcggcaccctgaggcggtcgaacagcagctcgtacgcggtgatggtggtgagcggcagcgcggcggcctgcgcgtcgtcgaggctcctgggcgcgagggcggcgatgcgctcgtcgaccgcgtgcagttccgaattggcgccgggccggacgatcgagccggcgtagtagacgcggtcgccgaccttgaagttctcgaccccggcgccgatggcctcgacggtgccggcggcatcccagcccagcaccttggcctggccggcctcgggcgccatgttcttgcgcaccttggtgtcgaccgggttgaccgagatggccttcacccgcaccagcaggtcgcgcgggccggccacgggcgcgggcagttcgatgtcctgcagcgactccgggttgtcgatggggagggcttggtagtagccgatggctttcatgtcgggtgacctttcttgaatggatggcgtcactgtaggatggcaatcaaaaattgataagaccgtccagatcagcaacactttcaaatgaagattgaaaatctctcggacctgcaggtgctggtgcagacggcgcgcggcggtacgctcacggccgccgcccatgcgctgggcatgacgccggccgccgccagtgccacgctcaagcggctggaaacgcagctcggcgcgcggctcttcgagcgctcgacccgcgccatgcgcctgacttcgcagggccagaccttgctcgactacgcggtgcgcgccttcgaactgctcgacgaaggcgaatcgctggtcaccgccgatcgcggcgaactggtcggcaccctgcgcgtggccgctccgtcggacctcacgcgcagcacgctgctgccctggttcgacgaattcctcgcgctgcacccgggcgtccagctctctctttccgtgggcgaccggctgctcgacgtgacccgcgacgaggtcgacgtggcgctgcgctacggtgcgctggccgattcacgcctggtggcgcggccctttgccctgaccaatccgctgctcaccgcgtcgcccggttacctgcgccgccatgccgcgccgaagacgccgcaagacctggtgcaccacaactgcctcaccttcgaccgcggcgggcgccgccaccgcacgtggcgctttgcgcagaacgggcagtggaccgaagtgcgggtcaagggcgaccgcagcgtggacgacgcctcgctggcgcgcgagtgggccgtggcggggcgcggcatcacgctgaagtcggcgctcgacgtgcgcaacgacatccgcagcggccggctggtgcacctgctgcccgagtgggataccgagccctatccgctgcatgcgttgctgccgagcgggcgcttcgtgccggcgcgcgtgcgggcgctggtggactttctggcgctgaagttcgaggcgctgaccgccgccgtttagatcatgggcgtgaccgcgccatccatcgcgacgatcgcgccggtgatgtagctcgcctttggcgatgccaggaacacgacggcattggcaatctcttccggcgcggcgatgcgtccgagcgggagccgggccttggcgcgctccagcgcctcgtcgctgccgatgccctgcagcttcgcatccgccttcaggccttcctgcagccgctcggtcagcgtgaggccggggtttacggcgttcacgcgcacgcccttggccgcgtaggccgcggccatgccggcgctcaccagcatcagcgcggcgttggccgcgccgccggccatgtggaccgggctcgccaccttgccgccctgtccgatcacgttgacgatggcgcctcggccgcgctggcccatgcgtttcaccaccggatcgatcatgtggatgtaggtgaagtacttggcgtccatggcgtcgtgccaggcggtggcgttcagctcgtcgggcggtgtgcggcgcgcggcgccggcggaattgaccagcacgtcgaccgggccgaaggcctgctcggccgcatcgagcgcggccacagcaccggccgggtccttgaggtcggcggcatgcaccgagacccggccttcggcctcggcaaacgcctcgaccagcgtcttgcggccctgttccaggttctgcagatcgcgcgacaccaggctcacgcgcgcgccctcgcgcaggaagcccaacgcgcaagccaggccgatgcccttgctgccgccggtgatcagaacgtgccggtcctggagctggaggtccatgtgagagtccttgtagcgttgaaagagaggagggaagagcgccgcgtggcgcggggtcgcgtggattgaatcaccgctctaagatcggcggatgaacgcatccccggtatccctgccccgctactggtctcaactgacgacgcgcgacttcgccgcgctcgatgtggcagccacggtcgcggtgctgccgctcggcgccaccgagcagcacgggccccatctgccgatgggcgtggacacggtgctggcagacggcatcgtggcggcggcgctgccgctgctgccggcggaattgccggtgctgttcctgccgacgcagcagatcggcctgagccccgagcacgcgcgtttcgcgggcacgctcacgctgtcggccgagaccgtgatccgcatgtggaacgagatcggcgccggtgtggcgcgcgccggcgtgaagaagctggtgctgttcaacgcgcacggcggccatgtgggtgcgatggacatggtggcgcgcgagttgcgcgcggcacacgggctcatcgtctacagcgtgagctggttcaacctgccgctgggcgatgcgggcgcgcagttcggcgcggacgaacaccgcttcggcgtgcatgccggcgacatcgagacctcgatgatgctggcgctcgcgccgcagcaggtgcgcatgggcgaggcgaagaacttccgctccacctcgcagcagcgcgcggccgactacgcgatcctcggcaacggcaagagcgccaagctcggctgggccatggaggactacaacgcagagggcgccgcgggcaacgcggccgccgcgacggcaccgcgcgggcaggcggtggtcgatgcggcggcgcagcaactcgcgctgctgctggccgaggtgtcgcgcctgccgctggacacggccaatacgcagccgctgccctgactttctgggtcaggaattgttgcgggccagcacgccggcaaacatgccggaatcgacattgccaccgctcacgcagatgcccaccgtcttgccgcgccagcgctcccgctgctgaagcgcgcctgccagcgccgcggcgccggcgccttcggccacgttgtgggtgtcgctgaagagaatgcgcatggcctcggcaatctcgtcgtcggtgacggtgatcacgtcgtcggcttcgcgcaggatcacctcgaccgattcgggcaccggcgtgcggcaggccatgccgtcggccagccgcgtgttggccggcgactcgacgggccggccggcgcggaaggaatcgcggtaagccgtggcatgcgccgacaccacgccgacgagcctggtcgacacgccgcaatgcgcccgcgcggcggctgcggcggcaaaaccggagcccagaccgatgggcacgaacagcacgtcgggcggcgcgtctttcagtgcgctgaagaattcgacgtacgcggtcgacacgccgcgcaccagctcgcggtggaacgacggcacgcgatgcatgccgtcgcgctcggcgagcatggccgcatgctcggcagccgcctggaagtcgtcgccatgctcgaccagctgcacgcccagggcgcgcatggcggcattcttctcgatcgagttgccatgcggcaccacgatggtggccgcgagcccgtgccgccgggccgcgaagccgaccgactggccgtggtttccgcgcgtagcgctgatggcatggcgcacgcccggctgctcgcgcgccagcgtttcgaagtaagtgagcccgccgcggatcttgaaggcgcctgcgggcgtgtggttctcgtgcttggcccacaccgcgctgccgaggcgctgcgcgagcagcggccatgcgtactggggcgtgggcggcatggcggcgccgacggtgcgctgcgcggattcgatttcgtcgcgggtgaacctcacgggcggcctttttatttgcgttctgtcagtgcgactcgcaccgccagcgcggccagcacgctgcccatcacgtaccgctgcgcgcgcagccagccggcgctttgcgacagcacggccgtgatgcttgcggcgccgaagatcacgacggtattgaccgcggcgctgctcgccatctgcgccatgcccagctgcatgctctgcagcagcaccgagccccgctcgggatggatgaactgcggaaagaacgagaggtagaacatcgcgaccttcgggttcagcaggttggtgagaaaacccatgcgaaacagcttgcccggcgggtcggccggcagcgcgcgcgcctcgaagggcgcattgccgccgggcttgaccgcttgccatgccagccacagcagataggcggcgccggcaaggcggatggcgtcgaacgcgaccggcacggccagcagcagcgcggtgagcccgagcgcggccgcgaacaggtgggccaggaaagccatcatcacgccgccgagggagaccagcccggcgcggcggccctggatcagcgtgcgcgacacgcaatagatcatgttcggccccggcgtgagcgcgagcagcatggaggcaagcgcgaaccaggcgatttcggtcaaggtcagcatgtcggtcagagcccttcggattgaagcgtgacggggccgtggggcgtgtcgagcacggccacgagattgggtgcgccggactgcacggccatgccggacatgccgatggccgacagtgcggcatccagggcggccgcgcgcggatgcgtggcgtgcagcgatcgcatcgccaggcccgaggcgggcatggcgtcggtggggtgcaccggcccccactggatcagcgtgggcagcgcgccatagaacagccgctggccgtcgtcgcgcaccgtgatctgccactcgagccggccggcgggcgtgtcgcgtgaggcttcgagcaagtggccgcggtcgatgtgcgcgtgttcgtcgtgcgccagcgcccgcagcgcggcgtgcgcgtcggccacgcgcgcaacgaagtgcaccagccgcggcccgtgctgcaagaggcccgcctgcagcgcggcgtcgtccaggtcgaaccagcggcgcgtgccgcggcgcgacggccgcttgccaggctcgatggcgatgatctcgaggtaggcctggggaaaggccgcgctcgcaatgttcagcagccggttgtgcgtgcccatcagcggatgcgaaccgccggggcccggcgtcacgcccagggtggcctcgcaccacgccacgccctcggccagcgaagcggcggcgatcaccaggtggtcgagttgcgcgtgcatggtgccttgccttacagcgttacctggccgtcgacgcaggtcacggcatcgccgccgacccacaccttgccgtcgccgtcgcgctcgatgtacacgcgcccggctcgtccgaggcactggccttgcgcggccacgtagcgccccggcatgtggccgtcggcgatcagccattcggcgaggctggcgttgagactgccggtgaccgggtcttcctcgacgccgatgggcgcggcaaaggctcgcacctccaggtcgatcttcgggccgtcgtcggcttcggccgaggccttgccgccaaaagcgcgtgcctcgcggttcgaccggccgatcagcatcgacgagccctctgccacgggcacgcccgccacgccggccttgacgcccagttccttgagcatgcggtggtccggcgccaggcgcagcacggtgtccgcatcgctgagcagcaggccgaaccagacggggccgttgtcgagcacctgggccgcgacgatctgctgcgccttcaggcccagcgcacccgccaccttggccagcagcgtggggctgggggcgctgcgcttgagcggcggggccgagaacgccaggcgcccgccctcgcggcgcagcggcaccaggccggccgcgcactgctgcacgacccggcccgccgccttgggcttgccgccggcctgcagccaggcatggcagctgccgatggtcgggtggcccgcgaaaggcagctcgccgccgggcgtgaagatgcgcacgcggtagtcggccgtcgggtcggtcggcggcagcaggaaggtggtttcggacaggttcgtccactgagcgaagcgctgcatcgcggcgtcgtcgatcccggtgccgtcgagcaccacggcgagcgggttgccgaggtaaggcgttgcggtgaagacgtcgacttgtttgaacgggcggggtttcatgggtgtcattcgagcgggagatcgagcacgccgcgcgtgcccggacgggagatcagttcgccgtaccagcgttcgaggttcggccagctggggcgctggtattcggccggtggcaggccgaaccagcggtgggcttcgcagccgatgggaatgtcggccatggtgaagcggtcgcccgccatgaagggccgccgtgcaaggtgggcgtcgagcatcgcgaacagggcttcgctcgcatggacggaggcggcgatgagcgccggttcgcgttcggccggggccgtgcgcacccattgcacgaaggcgtcgcggctcgcgcggttcagcgtggtctgctgccagtccatccagcgctcggcgtcgaagcgcgcgggcaggtcgctggggtagagcttgccgtgggagtgcttggcgcacaggtagcgcacgatcacgttcgattcccagagcgtgacgcgctcgctgccttcgccgtcgtcgatggtgggcaccatcgcgttcgggttgagcgcaaggtattcgggcgtctgcaccacgccgaaccggccaccggcttcggtgcgttgaaagtcgagcccgagctcctgcgcgcaccagacgactttgcgcacgttgatcgaactgatgcggccccagatgttgagcatgtgttcagcttccttggacaggtgtggcggacagggcagatggcatggaaggacggtcgagcagcagcaggcgaatcgccaggccgaccatcaccagggccagcaggccgcgctggaatttttcagcccccggtcggcgctgcagccaacggccgacctgcccgctgcatgcgccgagcagcgtgttgaacgcgagcgcggctgccgagagcatgacgccgagctgcaccagttgcaagggcacgctgccatgcgccgggtcgacgaactgcggcagaaacaccatgaagaacagcagcgccttcggattgacgaggttgttgaggaacgccatgcgcacgatgcgcgcgaaggcggacggctgcacccgcgcacccgccgggaggccaccgttgctgcgaagggcctgcaccgccagccacagcaggtacaccgcgccggcataccgcagcaggtcgaaggagggcggccaggccgccaccagcgcggtgacgccggtggcggcgaagagcgtgtgaaccaggtcggccgatgagatgccgagcgccgccgcgaaaccgccgcgcggtccatgcgccacgccgtgcgagagcacgaaggccatgttcggccccggcgacaggaacaacgccaggacggccaggaggaagagcgcgagcgtggcgaggctgatcatggggtgccctgcaatgcttacttcaggcagctgcggccgtggctgccggaaccgaggggagatagggctcgatgttgcgcagggcgcgtgccacgtagtcttctttctcgccgaccggcgcgacgtagtgcagcgcactcgtcgcggcctcgatgccttcgctgcgcgcgatgagccaggccgcgaggtagggcgccgacaggcagccgccggcggtggccacgttgcccttggcgaagaacggctggttcagcacctcgacgccggcctcttgcacccagggcttggtcgtgaggtcggtgcacgccggcaccgcgcccagcaggcccagcttggcgagcagcagggtgccggagcattgcgcgccgatcagctgccgcccggcgtcgagccgtcgcagcacgcccatgatggcgggatcggccgcaatttctcgtgtgcggatgccgctgccgacgagcaccgcctcggcgtcaatggccgcctcgagcgtggaactcgcatgcacggtgacgccgttcatcgaagtgaccgtggcgctgggcgcggccagcgtcacgcgccagcccggcttcttgatgcggttgagcaccccgagcgcaatcagcgagtcgagttcgttgaagccgtcgaatgtgaggatggcgatgtgcatcgtggtctgccccgtatcgtggctcagacgggttcgggcgcgagcttgcgctcgccgagtagcgcgagttcttcgcgcagcgtcagggccagcgcggcgatggcgacatcgatttcttcgacgctggccgtgacgaacgacaggcgcagtgtccgcggatcgccctggccggcatagaagggcgcgcccggcacgaaggccacgttgcgctccaccgccttgggcagcagcgccacggtgtcgatgccctcgggcaggcgcgcccacaggaacataccgcccttgggtgcgttgaacttcacgtccaggccggccatctcgcgcgtgagcgccgccatcatcgcgtcgcgctggcgcttgtagagcgcgcggatcgtgggcacgtggcgctcgagaaagttgtctttcatcacggccgagaccatgcgctgcgtgaagatgggcgtgtgcaggtcgaccgcctgcttggcctgcagcagcttcgggtagatggccttcggtgcgacgagaaagcccaggcggaggcccggtgccagcaccttcgagaacgagcccaggtagatgcagccttcggggttgcgagcggtcagcggcagcggtggggcttcgtcgaaccacagttcgccgtaggggttgtcctcgacgatcggcaggccggctgcggccgcagcggccgacacggccgcgcggcgctcttcggtcatggtgcggccggtgggattctggaaattgggcagcaggtagacgaagcgcgcggcgtcatccgaagcgcgcccgccggtcgcgcgtgccttggcgatcaggtcatcgacgatcacgccgtcgtcgtcgctggccacgctcacgggctgtggctccatcgggccgaaggcctgcagcgcgccgaggtaggtgggcgtttcgaccagcaccttgctgcccgggtcgagcagcactttggccaccaggtcgaggccctgctgcgagccggtggtgatgagcacctgcgcgggatcgacgttccacggcagcatgtcggccaccgcctggcgcagcggcgcatagccttcgctcgcggcatattgcagggccgcctggccgtcgttgtgcagcacctcggcgcaggcgtcggcaaaggcctggatcggaaaggtcttgggcgagggcaggccgccggccaggctgatgatgccggggcgctcggtgaccttgaggatttcacgcagcaccgacggattcatcttggcggcgcgggcggcgagtttccagttcatgggttcttctttcaggcgggtgaggtgagaggcgaaagtgttcaggattgttcggcacgcgcagcgcgcggcgaaacggcctgtgcgggctgcggctgcgaaaggcgcttgccgagcatcaccgtgcagaccacggcaatggcaaagcccagggtaaccacatcgagcggctcgcccagcagcggaatggaggcaattatcgagagaaagggctgcagcagctgggtctggctcacgcgcaatgcaccgcccagcgccaggccgcggtaccaggcaaagaagccgatccacatcgagaacacgccgacatagacgaagcctagccaggccgacgtggcgatgggttcctccggccacagggccagcgtggccggcaaggtgacgggcagcgccatgacgcagacccagcagatcacgcgctcggcgccgagcgacggcgtgacctgcgcgccgtagatgtagccgaacgacgccgcgatcaccgcgcccaccagcagcaggtcggcccactcgaaaccgaagccatggccgttctggctggcacgcagcagcgagaaaagaacgaccagcacgctgccagcgatagcgcacagccagaagccgagccgtgcccgctggtgcagcaccagggcggcgaccgccgcggtgacgagcggcagcagcgccgtcaccaccgccgcatggctggccgtgaccacgcgcaatgcataggccagcagcagcggatagccgatcacgttgccgagcaccgccatgcccaggggcttccactgctgcggcgcgggccggggcgagcgcgtggcgagcaggaagaccgtcgagagaatgcccgccaaggcggcgcgcccgagcgtgacgaaccagggcgagagctgcggtgcgccctgcgtgccggtggccagccgcgtcatcggcaaggtgacagcgaacaacgccacgccgatcacgccgagccacatgcccagggtctcgtccttgatgcggctcatacgctcagcatccaccaggccgtgagcaccagcaccaggcccatcgcacggttgaaccacagcaggcgcttgcccttggacagccagtcgcgcagcagcgcacccgccagtgcgtagacgaaattgctggcgaaggcgtagaccagcatcaccggcgcgacgatggcgaagcggccgagcgcgtcgggctgccccgcgatccagcccgccaccagtgtgagcgcgagcagccaggccttgatgttgacgaactgaagcatcacgccctggccgaagccgatattcaggctggcgctgtccgcgcggccgagcgtgccgctgccgctgagcttgtaggccagccacagcaggtagcccacgcccagcgccttgatgcccaggcgcagcggaggcaccgccaccaccaacgcaccgatgccggccgcgcaaagaaccagcagcagtgtccagccgaccggcaccgccaccacgaagcgcatggcgcgcggcaggcccccgttggccgccagagcggtggaaagcgtggtgttggggccgggcgagaaactcatcgccgtggccagcaccagcagcgcggtgaattcttgccagttcattgcatacactctaaactttgcgaccattacagttccaatacagttgatcgaacatattccaaaactgtattggtctgcctttcgacacagaagcccaagccgatgctgacacgaacctccacccagtcgctcaccgggcaattggccggccggctggctgaacgcatccgcacccggctgctgccgcctggcgcgcgcctgccctcggtgcgcgaatgcgcgcgccagcagggcgtgagcccctacacggtggtggcggcctacgaccagttgctggcccagggcctggtcgaggcgcgccggcagcgcgggttctacgtgcgcgattcggcgcccgcgcaggaagggcgaccgcccaacgcggcccccatggtcgcgcagatgatggcctcgcgcgtgccggccgatgcaagctcgctcatccgcagcatgtttcaccggccgagcgacaagccgcagccgggcatgggcgtgtttccgccggagtggatgtcgtcgaccttcatgccgacggcggtgcgccgcatgaccagtacagccgtgctgcaggagctgtcgctccagtacggggagccctccggcgacgccgcgctgcgccgcagcctgtcgaacaagctcatgggcatcaacgtgcccgccgcgcccgaccagatcgtgacgaccgtgggcgccacgcatgcgctggacatcgtgagccgcacgctgctgcgcgcgggcgatccggtcatggtcgaggagcccggctgggcgctggagttcgcgcggctcgaggcactgggcatgcggatcctgccggtgccgcgccgtgccgacggccccgacctggatgtgatggcgcagtactgcgcgctacacagccccaagctcttcgtgagcgtgagcgtgctgcacaacccaaccggctacagcctcacgccgggcagtgcgcaccgcgtgctcaagctggccaacgcgcatgactttcacatcgtcgaggacgacacctacagccatctggcgcccgagcacgccacgcggctcagcgcgctcgacgggctgcagcgcaccatctacgtcagcggttttgcgaagatcctggcgcccaactggcgcatcggtttcctggccgcctcgcctgaactgaaagagcggctgctcgaaaccaagctgctggccaccctcaccacgcccaccctgttcgagcgggcgctttcatggtgcatcgaccaggggcaactgcggcggcatgccgagcgcatacgcatccggctcgacggcgcgcgcggacgtgcggtgaagctcgccatgtcgcacggctgcaccttcgcatcggaaccggcgggcctcttcggctgggtcgataccggcgtggacaccgacgcgctcacgcagcgcatgctcgaccagggctacctgctggcgccgggttcgctgttccatgcgcggcggccgccgagcacgatgatgcggatcaatttcgcgacctcgcaggacgcggcattctggaaagtcttcagcaaggtccgcgccgagctttgacgggggttttgcctcgcatgacgtgagcgttcgcgagtccaaaagagggatgccttggagtaagctggcatcacaagaaaacccaacccggagaccgccgcatgagcaacgccagccaacccttcgacttcagccaatttgttcctggattcgattttctgaagaatcttgccggcggtgcagccggtggttcgggtggcggcgcagcgccagggttgcccgggcttgcaagctgggtggcgcccacgctaagcgtcgaagaagtcgacaagcgcatccaggagctcaagacggtgcagtactggctcgaacagaacggtcatgcgctcaaggccaccatccaggcgctcgaggtgcaaaagatgacactttcgaccttgcgcggcatgaacgtgcggatggaagatatcgccaacgcgttcaccaagcaggcggccgccgtggcgcctgccgctgctgctgcgccggtcgagcccgagcccgaagccgagccggatgaagacgcaccgacggaagcaccggcgcccgccaggaaggcgcgcagcaagccggcgtcgtccaccggcgcttcggccggcaacggcggggtggtggatccgatgcaatggtggggctcgctgaccgagcagtttcagcagattgccagctcggcgctgcaggatgcagcccagctcaaggtgccggccatggcccagcccgtggccgatgcggtagacaaggtgatgggcaagccggcggcttccgctcctcccaagcctgcggccaagaaagcggcagcaacgcccgccgcgaagaagaaggcgccgggcgccgcgcgaaagcgaacggccagccggcgctgacgccatacacgaacgcatttttgtttgaagagaacgggttggcacgcatcatgaagttgtttccttccggccatgccacccatccgcaatggcgcatggcggccggcctcgtgctggcgcagctgcgggcgcagatggcactgcccgactacgcgtcgtcgccgacgctggggttgctgtacatcaccgaccactacgcgtccgacgcgcaagacatcctcgatcacctgagcgccgagcttcccgaggtcaccgattggtcgggcacggtcggcatcggtgtgtcggccaacaatgccgagtatttcgacgagcccggcctctgcctgatgctctgcgcgctgccaagcgaccagtaccgcgtgttctcgggcgtggcgccgctgggcaattcggagatgagcggtttcgaggcgcacacggcgctggtgcatgcggaccccgcgacgcccgacctgacggaactcatcggcgaaatggccggccgcaccgacaccggctacctgttcggcgggctctcgtcgggccgcgcgggcgcgctgcagttcgcggtgggcggcaacggcaacatccgcgggcacggcgcggcgggcggcgtgttctcgggtggcttgtcgggcgtggtgttcggcgagggcgtgcggctggtgtcgcgtgtcacccaaggctgccagccgctgcgcgcgggcgcggggcgcgagcgcgagatcaccgaggcggacggcaatctgttgctcaagctcgacggcgaaccggcgctcgacgtgctgctggccgacctgcaggtgtcgctcgagcggccgcaggaagccatcgacgccgtgcgcgccaccctggtgggcctttccgatgcgggcagcgacggcatccgccgcaccggtgatctgggcgccgacgtgctggtgcgccacatcatcggcctggaccccacgcgccgcggcatcgccattgccgacgtggccgaagccggcatgcgcctgaccttctgccggcgcaatgcgcaggccgcacgcgccgacctgatgcgcatctgcgcggaaatccgcgaagagctggagcccgaggagcagacgctggccaccgcccgcgccgtggcggccggcgaggccgaggcagcgccgcatccggcgcgccgcattgctggggccgtgtacgtgagttgctcgggacgcggcggaccgcacttcggcgcgccaggcgccgaactgcagatcgtgcggcatgcactgggcgacgtgccgctggtcggtttctttgcggcgggcgagatcgcccggcaccacctgtatgggtatacgggggtgctgacggtatttaccggcaaggactgaaccccggaaccgccgcttggcgctcgttcaagccggctgcagcacgcgcgccgcgggcgcaggcattcctgtgaacgcgaaatccacctccggcacaagcccgctcacgatgcgcgcgatcgacttgcccgagccgcaggcatgcgtccagccgagcgtgccgtggccggtgttgaggaacaggttgggcagctttgtcttgccgatcatcggtacgttgctgggcgtcgcggggcgcaggccagtccagaattgggcctgcgtggtgtcgccggcacccggaaagagttcttcgacgcgccgcacgatggcttcgcagcgcacgcggttcagatcgcggtcgtagccgttgagctcggccgtgccggcgatgcgcaggcgatcgccgctggccgaggtgtagcgcgagaacacgagcttgtattcgtcgtcggtcagcgaaacctggtgcgccttggaggcgtctttgaccggcaaagtcaccgaatagcccttggccggatagatcggcagccggatgcccagcggcgcggcaacgatcgggctgagcgagcccatcgccagcacgaaggcatcgccgcggatgcgctggaaacggccttcgctgtcggtggcttcgacgtggtcgatgctgccgccggtctcgcgcagcgcagtgacggtgtggctcatgaggaacttcacgccggccgccatcgccagcgcgaccagttcgcgcgcgaagcggttggcgtcgcccgattcatcctcggcggtatacgtcgcgccggccagcttcgggcggatgtgggccagcgctggctcgatcttcaccgcctcgtcggccgagatcaccagccgctcgcagcccaatgcgcgcatctgctcggcaggcgcgagggcaccgtcgaactccttctgcgtcgtatagaagtgcaggatgccctgcgtgcgctggtcgtagctgagaccggtatcgcgacgcaactgctgcaacatttcgcggctgtaggtgcccaggcgcacgatctgctcgatgttgtgccgcgtgcgtgccggggtgcattcgcgcagaaactgcaaaccccagagccactggcgcatgtcggcgcgaatgcgaaagagcagcggggcgtcttccctgcccagccattgcagcaccttgagcggtgcgctcgggttggcccagggttccgcgtggctcacggagatctgcccgccgttggcaaagctggtttcggcggccggcgtggcctgccggtcgatgacggtcacttcgtggccgagttgctggaggtagtaagccgaggtcacgccgagcaagccggcgccgagaacgatcacgcgcatttcaagtaccttttggaagttggcgcttgaacggcgggcttggtgtgctactgattcaatagcaagcaaccggacgaccgccgtccaagttgccgctccccctgtccttggtacctgagagattcacccgctgcgcccgcagcgggtttgctccttcggtgcatcacgcaaggtgatggctctccagacggcgtatcagttggtgcagtacaggccccatgccgaaactctttgaaagaagaacttcaagaatccgtggggccgacctgagcgtttatgggagtttgcgccttcggtgaggtagcaaaaagcgctacctgctctcctgcagtggggctattgtaggcgcacgcgccgagctgcctacccctcgattttggtaattcggtccaatgggataatcacgggacagattcgcctgagggcgattgttcgacaacttcgggggactcatgattctggtaaccggcggcgccggctttattggcgccaatttcgtactcgactggatctcgcagagcgacgagccggtcgtgaatctcgacaaactcacctacgccggcaacctcgaaacgctcgcgtcgctcaaaagcgatccacggcatatctttgtgcagggcgacatcggcgacagcgccctggtcgaccgcttgctggctgagcacaaaccgcgcgctatcgtgaactttgccgcggaatcgcacgtagatcgttccatccacggccccgaagatttcgtgcagaccaacgtgcttggcaccttccgcctgctcgagtccgtgcggggttactggagcgcgctgccggccgaccagaaggccgcgttccgcttcctgcatgtgtcgaccgacgaggtctacggctcgctttccaagaccgacccggccttcaccgaagagaacaagtacgagcccaacagcccctactcggccagcaaggccgccagcgaccacctcgtgcgcgcctggcaccacacctacggcctgccagtggtcaccaccaactgctccaacaactacgggccgttccactttcccgagaaactcatcccgctgatgatcgtcaacgccctggccggcaagccgctgccggtgtacggcgacggcatgcaggtgcgcgactggctctacgtgaaggaccactgcagcgccatccgccgcgtgctcgagggcggcaagctcggcgagacctacaacgtcggcggctggaacgagaagcccaacatcgagatcgtcaacaccgtgtgcgccttgctcgacgaactgcgcccgcgcgccgacggcaagccttacaaggagcagatcagctacgtcaccgatcggccgggccacgaccgccgctacgccatcgacgcgcgcaagctcgaacgcgaactcggctggaagcccgccgaaaccttcgacagcggcattcgcaagaccgttgagtggtaccttgccaacgccgaatgggtgcgcaacgtgcaaagcggcgcctaccgcgaatgggtcgagaagcaatacgacgccgcgcccgcggccaaggccgcggcatgaagttgctgctgctgggcaagggtgggcaggttggatgggagctgcagcgcagcctcgcaccgctgggcgaactggtggcgctcgatttcgacagcaccgacctgcatgccgacttcagccgccccgagcaactggccgagaccgtgctcaaggttcgtcccgacgtcatcgtcaacgccgcggcccacaccgcggtcgacaaggccgagagcgagcccgactttgcgcgcaagctcaacgccacctcgcccggcgtggtggcccaggcggcccagcagatcggcgcgctcatggtgcactactccaccgactacgtcttcgacggcagcggaagcaagccctggaaagaagacgacgccaccggccccctcagcgtgtacgggcgcaccaagctcgaaggcgagcagctggtggccgctcactgcgccagacacctgatccttcgcaccagctgggtgtatgcggcgcgcggcggcaattttgccaagaccatgctgcggatcgccaaggagcgggatcgcctgaccgtcatcgacgatcagtttggcgcccccaccggcgccgaactgctggccgatgtcacggcacacgcaatccgcgccaccctgcaagacccggccaaggccgggctctatcacgcggtagccggcggtgagaccacctggtgcggctatgcgcgcttcgtgctcgagcaggcccagcaggccggcgccgaactcaaggccggccccgcggaagtcgatgctgtgcccaccagcgcctttcccacccccgccacgcgccccgccaactcgcggctcgacacgcgcaagctgcaggccaccttcggcctgatgctgcccccttggcagcagggcgtggcccgcatgctgcgcgaaaccctttaaacaacacgccgagcgcggcaaagcaaagaaagcaaggagagaaatacaacaatgaccacgaagacgacaacgcaacgcaagggcatcatcctggccggcggctccggaacccggctgcacccggccacgctcgcactcagcaagcaactactgccggtgtacgacaagccgatgatctactacccgctcagcacgctgatgctcggtggaatgcgcgacatcctgatcatcagcacgccgcaggacacgccgcgttttcagcaactgctgggcgacggcagccagtggggcatcaacctgcagtacgcggtgcaaccgagccccgatggcctggcacaggccttcatcatcggcgacaaattcgtaggaaattcgccgagcgcgctggtgctgggcgacaacatcttttatggccacgactttgcgcatctgctcgccgatgccgattcgaagcaatccggcgccaccgtgtttgcgtaccacgtgcacgaccctgagcgctatggcgtggtggccttcgatgccgagggcaaggccagcagcatcgaggaaaaaccggcccagcccaagagcagctacgcggtgaccggtctctatttctacgacaaccaggtggtcgacattgccaaggccgtgaagcccagcgcgcgtggcgagctcgagatcacggccgtcaaccaagcctatctggatcgcaaccagctgaacgtgcagatcatgcaacgcggttatgcgtggctcgataccggcacgcacgagagcctgctggaagcggggcagttcatcgcaacgctggagcaccggcagggcctgaagatcgcctgtccggaagaaatcgcatggcgccatggcttcatcgaccgggaacagttggcaaggcttgctgcgccgctgcagaagaacggctacggcaagtacctgaaccacctgctggctgaggaggtgcgctcgtgaaggccacacccaccgcaattcctgaagtgctgatcatcgagccgaaggtcttcggcgatgcgcgcgggtttttctacgagagcttcaacggcaaggcgttcgatgaggccgtcgggcggcatgtcgagttcgtgcaggacaaccattcgcgctctgtgaagggcgtgcttcggggactgcattaccaggtgcagcagccgcaaggaaagctggtgcgggctgtgcgcggctcggtgtttgatgtggcggtcgacattcgcagatcgtcgcccaccttcgccaaatgggttggcgtcgagttgaccgaagaaaatcataagcagctctgggtgccggccggattcgcgcacgcgttcctggtgctcagcgagagcgcggattttctctacaagaccactgagtactacgcgccggcgtacgaacgttgcattgcatggaacgacgcgaacattggtatcgagtggccggaaattggaatggcgcctgtgctgtccgcgaaggatcaggccggtgtttcgttgaagcaagccgagatcttcgattagtcgaagacccttgtaatcctccatgcgatggggcaccagccccaagcgcagattgaggggcggactgtccatcgagcgacgagaagctttattcggttaaatctccgttcttaatcattatttttcgcaatgctgcagatcgttgatgctcctgtcggcgcatccaaacacgactggcgacttgcagaccctccgtgcatatctcagtggcacgcgagcgagagtaattttttctcaaaaactcgagccccgccgcctgcataaagtgccatttggcctcgtctgaatacagattaataacgtccctcgcaaaatcaagtgggtcatcttgcaccaacaggtgagagtcctttgctcctgcaatgccctcagcggcaatagtagacgccacgcaaggcactccatgcgcgaaggaatttatgatcttccctttaatgccggccccaaaacgcaggggcgccacgaagactcttgacattgcaaagtgaggtgtcaagtcctccacaaatccggtaacgatgatgcgatcggatgcaagtgccatgacctctggaggaggtttgttgccaaccaccagcaacctcgcgtccgcaggaagattcggttctatatgcggccacatctcctgaacgaaatagagaattgaatccacattcggtgtatgaggaaaattccctaaaaacatgatgtcttttcgctgttgaaaatcagttagaacttcaaccgactcggccagccacggaaataaaatgatgttttccgggcttttcggtaattctgtgttgacgatttctcgttccactgccgtatgaacgaatgacgcgtcagcttcggcaaacattcgaagctcgctggatttcgtgatttgagcgcgaaaggttccgcgctcatccccagtcatttgagcgcctctcgactcgcgcaaatagtgtagatccacgttcgcgaaaattacaggcgctgtcggcataaattctcgtacgtcgtcataggtcatattagcgacctcatgtcgataaatgagcgctaaatcgaagccgccacattgtgcgccgatctccgccacgcggcttgtaaatggttggtagtggcagcaaacccccgctctctgaagattaaaggtgtacttcggcatccaaaacggagaatgcatgggtaaaaaatgctgttcaaagcctagttcccgataaatctgcatggtttcgaacgtcataattgagccggaatcctggtctggagtcggcgttaatgcatccaaaactatcatccgcttgcgggagcggtgcattgaagcctcataaagacttgctcctacagcagggtgggtcgatatgacatcgctatatctctctcgcactttccttagattttccacctgatatgctttgacacccgtggcggtgcttcggccatgcgtaattccttcgtagtgaattacacgagagagcggttgaaaccagacctggtgcccctgttcgcgcaccctgaatgcaagatcaacgtcctcgcagtaggcgggactgaaatgcgagtcaaacccgttcaattgccgccagagtactcctcgaatagcaattgatgcacccgagatgtagtctgctgggcgggcgaagcaatagcgcggctgatttgaattgtcgccgcgaccgtagttataagcagaaccatctcgccaaatgatcccacctgcttcttgtagactcccgtcggcattcaataattttgaaccaaccagccctgcatctttcaagttttcaagactccagatgagttcgtcgagccaaccatcaactacgcgcgtgtcactattcaggaaaacaaagatttcaccctctgcgagcgcggcggcaaaattacagcactctatgaatccgccattctcaggccggcgaacataccgtatccatggaatccttttgagctcgagcatctggccttcgtcaggagacgcgtcgtcgcaaacaataatttcgaaggtatgttccgatttatgacccgccaaggagtctaggcaattcaagacataatcaagctgcccataaacgggaattattattgatgcttttactggcttctttgtcgtgcttgatcccgggaatttttgcataagagtttcaatgcactctctgaaatgacccttcgtctcgcgattaacaaagttaaagccgtgcgcgcagaaaaaggcctcgccggccatgatttcgaagttcacctcatcatcgggcagcgggtacgtccacctactgtccacccacttatgaatttccgaatgggtgggtagtttcctgccttctatgcaaccatggctcagccagtgaatcaacggattaacttcggcgttgcgcaagtcgggatagagtgcgacatatcgattcagggaatattctttaagcggttcgacgctgaatttagacccgacggctaaatagtgcatcactggatcccacggtgttgctttggcggctggcagtcgtctgagatattcctcctcgtcaaataggccactgtctcgaatttgggttgccgcacgttcataatccaaagccgcaggcacccttcccaggcttcgagattctttatggccgcttcggatgtagtgcaaaaatgtcttcgcaatagacccgacgtccgagtttgccgctaagtattcagcgggactgaacctgaggcttggatgtcggccttgctccagcccgatcgtgatgaaatggcttagcgcggcttccgcgtcgtgtggcacatctgtgtaggacaaagcataaaacttccaatcaaactcaccggagtctaggatttcgcgacgcaattctttcaagggtgcctgcccaagcgctgtcgattgactggatccgtttaatttcttgtacaagcgcttcagcccaagacgtagactgtttctacgcggtggttgctgcttttcggcgtaaccttcggcgtgaagttcaatgttattttgaatttgattttgcataacccgtcccttggttaatgtggcccaatgtttttccatctcgtctacgacaaaatcaccgattgcggcgatgcttacaaatcgataattttccgtttttaacgcttgttgcaatgcctcctcagattgaatgtggtctggcgcatcgatcagttcgagaggggtgtaggcgggaagagaagctatttcggactgatttttaacataatgagccggtaaagcttgcgtggttcgcctgttgcagtgcaccacgcctgaacatgaagtgaaccagcctattttgtgctgaacggtcccatgatggcagaaataaaaggtggcgtactgtgccagcaatattgtttcggaaatcgtcaaacccaccgcaaattccactcgaacatgcgcgcccttctcagagcgtagcttgtttgctacgatgtgcgcaacttggagatcttctgtgacaacttctctctgagccgcgggggcatagcccgggttggttgcgagatcatccgcaaaagagtggccatctaagataatcgatcctgttggacaaatggaaagaaagcgtgtccctatctcaatcaacgcttctgtttgattgagtgctgtacgatttcgggtccgaacgctcatccataatattggtccttcatacttctcgacgcgagaaaaaagggattcgatttcgcttgccttgggtagcgtgacagcaaaatgcagcaaccgttcgaccaacctttgttgtacgaaggtgccgccaaggggcaagaccatctttccgaattgatttatatgttccaattcccaatcgggaactcgatgcatagtccagtgcgacaactctggaaaaagcttgggcatgggccctagcggttcatgtgtgctgataagttgagccgtgcacttcactccaccatcaacgatggattgaagtactgataactgattccacgcgtgatgcgcgaagtttgcgtctcccgataccaaagtaatgcctttacttggacccgggcgcatggcggatattacgtcggctagcattgggagatgccgttcctgcactccccagtagtcgtcaatgagtttcagaaataaaccttcctcagggaagattattgccatgatgggaaatccaagtcccaaatgtcctattccaagaacaagcccgtcgaaaataacgaatgtacttttgtcacgaagtacgacggaaaattcggcagcaatccttcggccgcttcgagggcagattatctcgaagcttccttgctgaagacagtcggccaaatatcttctgatgcatgtgccatccacgaaagcagagctaaagttaatgttttctagcgattccgcaagtttaggcagtccatggcaatcggaaagctcagcaactcttttttcatcaagatcgacaatagtcgtatatctcttcaagaggttaccggggtcgggatatgtcatttgtgatgaggagaatttgcacggtaaaactacgggcaacggtcaacattcaagaggccggccgaatttcatggaccgcgtggtgcctgttggaggaactcgcgaggtcacgcagagcaatgaggacgcaaacggcgcggcgcagcaacttctgaattcgtcatcgcttcataacgtcggtgcctctgcatctggcgtcttgacccgccagtctgcaggtgattcttggcccgaattgaatgcgggcaagaggcacatcaccgcctcgcggggagactatatggttgtgagatttccatcgaaagctgagagcatgcgctgcagcgtttccgtcaaggcgggcatttctagctcgactccgtgttttgatagcaatgcattcaaccttgcggggttgccacaaagccgatgtacttcattgcctcggacgaaggccggattcaccaaaacttgcagtttgtgacccgtgatgtgagtgaaagcgtcaataacatgctgaagttcgtagggttgacctgagcagacgttgtaggcggtgcccggctcaccatgcgcgagcaaagccaggtacgcactgcagaccatgcgaacatcgttgaactcgcgctccacatggatgttgccgagcgcgatagaaggtgctcggctagcgaagtgcttggccaatttgggaattagaaagttcacatcttggcctggccctgtgtagttgaaagggcgagtgattaccagattcaggcgatcttcatatgtccgggccatgtattccatggcgagcttgctcatggcgtaatgattgacgggcgcgggtggttgcatttcgctgatcggcgatgcttccgtgttgccatagatgttcgcgctgctggccagaagcacgcgatggggccgaacgggcagcttggcaagcgcatcgagcaggttcgtggtaccgaccacattgacggcgtaaaaagccttttcatccgcatgcccgacgaagctgatcgccgccaggtggaccaccgcgtcaggggaaacctcgagcgcctcctggcgaagtgcttcgtcgtccatgagatcagaccgcagcgcaatgaccgagtgtcccctggccgatgcgcgttcgatgaaatgccggccggtgaaaccctcggcaccggtgagcaggattctcaaaacgagaagccctggcggttgcggcgcaggtctgcttcaaccatcatctggcaaagttcctcgagcgtggttttcggttcccagccgagttgggtcttggccttggccgggttcccgatcagcagttcgacttccgcagggcgatggaattttgggttgattcgcatgacggtcttacccgtggcagtgtctacggccgattcgccctctccactgcccttgaagtccacggcaatgtctgcgcccttgaatgccatgcgaacgaagtcgcgaacggtttcggtacggttggtcgctagcacgtatgtgtcgggtgtgtcgacctgaagcatgcgccacatgccctcgacgtattcctttgcaaagccccaatcccgcttggcatcgaggtttccgagctccagcacgtctagcttgccaagcttgatcttggcgacgctgtcggtgatcttccgcgtcacgaattcgcggccgcgcagtgggctttcgtggttgaagagaatgccgctgcagccaaagatgtcatagctctcgcggtagttgatggtcatccagtgggcatacagcttggcaacgccgtaggggctgcgcggatagaaaggtgtgtcttccacctgcggaatggcctgcaccttgccaaacatctcggaggtggacgcttgatagaagcgaatcttcgggttgacgaggcgaatggcttccagcagatgcagggccccaacgccggtgatctgggcagttgccacaggttgattgaagctcacccctacgaagctctgagccgcgaggttgtagacctcgacgggttcagcttggcggagcagttcgatcgagcttcccagatcggtcaggtcgtactccaccaggtgcaggtcggggttgttctgaatcccaagttcctcgatgcgccagaaattgaccgaactggtgcgccgataggtgccgtagacgacgtaccctttggcaagcagcaactcggccaagtaagcgccgtcttggcccgtgatgcccgtgacaacggcatgttttttcatgagaaccttctctgtattgtctaaatggccgcgcgcgcggcgaatcgagccatccatctggggagcgttgaacggtcgacgggttgaagactggattctgccaaatcaaaacggcgcctctccaacgcatatttggttacgtaacttgctcccaacaaggatgtgcgcctatcgcggagagcactcgcatagatgcgcggatacctcaggtaacacagaaggccaggaggccaaaagtgcaacatagttgaaggcgtgtgtggcttaaagccaacggtccatggggataataaatgtgtagcgcgcctgacatgactcgaaggtggcgtgtccgacgcagggagcaaggactggctcatcggacgggacagcccgacaaatgatcgagatatacaagcaagtatgagccacacaccacgagacgcagaaaaactcgccgaagcagagcggcagatagccgcccttaaattgcggctggagttgcaggaacgactcgtgcaaagcagcgatgaatcgattgaggctcagatcgaagcggcaaatgagcgcgcggcgttggcactgcagcatcaaaacgcgctgctcaactcggcatcctggcggctgacggcaccgttgcgcaaagtgtctgccgcgattcctcctgcgtggcgaggtcatctgcgccgcgcggctaaggccacctggtgggttgcgacgccctggcgcatgccgcaacggcttaattttctcaaggagcgccgcagtacgggtgaggcgaatgcgtcctttttcgtgcccgtggtcggcgctgaagccagccacagctcccagaactcctatcggcaatggattgacgagcacgaaaggcgctctgccttgctcggtgacctatcggcaatacccaggttgagctttctgctttgtgcaagcagtgcacagcttgagatgctgaccgcgacggtgaagtcgatccaggcgcaaagctttcccgagtggcagctcgtcatcgctgtatccggtgatgacgccggagcgctcgataacgcgctgcgagtgctgcaggatgaagagcctcgcatcgtctcggtatctgcttctggcaagaacggcgccgaagcgcttgccgcatgcctttcgctcgtcaatggtgatttcgtcgcagtgcttgatgccggagacgtcatcgcacccggcgccgcagtcgaaatcgccaatgcgttcattgaatcgccggccagcgacatcctctactgcgatgaagacgagtggtcggtcgaaggcggccgcgcccagccttacttcaagccgaactggtcgccggagctgctttatgccttcaactacttcggacgcttgacgctgttgcgccggcagctggtcgaggctgcgggaggaatcgaccccgcgctgggcgccggttccgaatgggatctgaaccttcgcgtgagcgatttctcccaggccatcacccgcattcccaaggtgctgtgccatcgcgcgaccggtggcggtcgccgggaacggccatccgctgactcggccgaggctgcgatgcagcgcgtggccctgcgcaaatactgggcgcagaaaggcattgacgcatcagtccagacgcagcccgacggtacccatcacgcgacctgggccatcgataagccgccgctcgtctcgatcgtgattccgtcgaaaaacaaggaccacctgctgcgcatgtctgtgggtgggctgctccgggaaacggcttatccgaacaaggaaatcatcatagtggacaccggttctaacgagccggaaacgctggcgtactacgccgaacttgccgctgagccgagcgtccgcatcgttcatttcaacaagaccttcaactactctgccgcgtgcaaccatggggcggcgttttcgcgcggcgaaatcctgctgttcctgaacaacgacatcgaaatcgtttcgcccgattggctgcacgaaatggtgcgcgtggcaatgcggcccggcgtgggcgtggtcggtgccaagctggtgttcccgtcaggcgaactgcagcacggcggtgtgggcgtcggcattcacctttgcggcctgatgtatcgcagtgctgaacggcttggttggggcgtgttcggttcgccggatcacgcccggaactggctttcgatcatgggcgcctgccagatggtgcagcgcgatgcctttgagcgagtgggcggattcgacgagtcgtacctgattgcaatgagcgacgtcgcactctgcctgcaggtctggcgagctggttatcgcattgcatatgtaccgcaggcacgccttgtgcaccacgaaggcgcgacacggggcaacagtaacccccagatcgatatgcgtcgaatggccgatgacattcgcaccctgggtatcgacgaagacccctatcttcaccccgagcttgacgctaaccacgcgattccgacccttcgagttggcgcagcgccctcggttcgcgagaagctcaaggccagccttcgcgaattcggctcgcccaggccgcaggtgcagacgctcgacctttcgagcgatggcgcatgcctggcggttgccatgctgccgcgcgaatgcgtgatctggacgccccagccggcgcatggcgtgcgcgatgtctggtctgcagcgcgatggtgcctggatctcttgcgtacatgccccgacatccgcctgcgcttcccagctgcactgtccgaaggcccggaaggtgcgtttgtcggctggctcgaagcagagggtacggatcgtttcggactgggcaaggatgcgctcgccgcgattcgtgcgatgtggtcggaggacttggcgatccgggcgcggcaggcgtttctctttcactcggacgtccgcgcgttgctgccgcacggcttgctgccgattggaaggcgcgagctgttccattggttcatgcagcatggccggcgcagcgcgggtttgaggctcgaagaagtctggtggttgttctggacagccgctgaaaggccggaggccgaactggtcaaggcctatgagttcaccccggaatggcaaaaactctatccggatggcctgacggttttcggccgccgcgcctttgccgcatggttccgcgccaactatcgcgtggctgatctgtgggccgacccggtgcgttggccgatcgatatggcgcctgcccgccagcttcggtctgcgtatcgggcgcgcgagcaatggcagcgtgtccaccccgaagcccttgacgatatcgagtccgcgaaggcgttgatcgactggctgcagtcgtcagaagccatgcagactgaagaagtgcgggcatggtgcgccggcctcgacaaagaggccgtggcagccgagatgacgacgctcggcgtgaatgtcatcggacatttttcgtatccgtctggtcttcgggtctccgtggaggcgctggtcaagggcctgcgagaagtcggcgtgcagaccgcgctgcgtgaccttcgaaccgacaagaaagacgatccggttcacgcgcagttccgcgattttgaagattttgaaacgaccatcatccacacacagcccgagccgttcttcaacgaggcctatagccgcagcgatctgaacgagcacttgccgcgcacttatcgcattgcctactggtactgggagttcgactccattccggattcgtggctcgatgcggctgccaaggtcgatgaagtgtggacggccactgaattcgttgccaagggcctgcgtgatcggctctccatcccggtgcgcaccatattccccggcgttgcgctgggtgcttaccagcagcgagagcgcaagtacttcggcctgaaggatggaagcttcacgttcctgttcacgttccacatgatgagcgtcatggagcggaagaatccgcttggcttgatcaacgcattcaaggccgcgttttccccgcaggaagacgccacgctggtgctgaagacgtcattcggtgaccgtcatccggcgcaactgaaggaactgcgcgccgctgcagcgggccataacatcgtggtgatcgatcaggtctacagccccgacgaagtgctgtcgctgatggatgcgtgcgacgcttacgtatcactgcatcgcagcgaaggtctaggcctgacgatggccgaggcgatgctgatgggcaagccggtcattgccaccaactactctggcaacgtcgatttcatgagcgaggatgacagcctgctggtgccctacaagctggtgaaactcggtcgtccgattccgccttacgacgagaagctggagtgggccgagccatccacagagcacgcggcccaactcatgcggcgcttgtatgaagaccgggtgtgggccaaggaggtcggtgcacgcggcaaagcgcgcgcggccattgatctgtctttgaaaatggcgggccagaaggccgcggcacggctggccgaaattcgagcgacgctccggacagattcgaagagctgagtaaaggagctacggggcgtgttcgcggccccgttaccacttacgcggtcaagccgcgagtcgtgcgcgctcggccatatacgcttccatgtccaccgcctccaagcggccatggtttagtttcacaaccttgttgcactctttggcaatcaggtcaggcgagtgcgaggcgagcaccagaatgcccgatttggacaccacgtctcgcatgcgctgctcggctttctcggtgaactcggcgtcgcctacggacagccattcgtccatgagcaggatgtctgcctcgacgctggtcgagatagaaaaagccaggcgcatcatcatgccggtggagtaggtgcgcacaggcatgtccacatactggccgagtccgctgaattcgcaaatctcgggcgtacgctcgtcgatctccttcttgctcatgcccatcaccaggccgcgcagcatgatgttctctacacccgtcgcgtccatctcgatgcccagtgatggatcgataaggctcgacacgctcccttcccgccggaactcacctgccgagggttcgtaaacgcccgccagggtgcgcagcaaggtcgacttgccggcgccgttgtgcccaatgagacccaaccgatcaccgctgcgcagttcgagattgatgtcgctgagggcctggaccacggtaacaccggtctctttgccaaaacgcccgcccgtcacggaggccgcaagcgtcttcttcagtgaggctgcgcccgcaccgtaaatggggaaattgacggcgacgttcttgagtgaaatggatgccatagatcagagccagtaaacaacgcggcggcggtacttgatgaagagcagtgtggacccaacaacgctcaccgcggtccacgccaggatgccgaaccagctgtgcatctccgccacgccgcccatcagcggcgtacgcagcagatcaagcatttgtgcaaaagggttccacaaaacgtattgggcgcgttgcggcaggctttcgggcagccaaaaaaccggtgtcaggaacatcagcatctgcatgatgctgttcacgatctgcgtcacgtcgcgaaaacgggtgcagatcagcccaagcagcaggccgatcgcatgtgcattgatgaccgcgatcaccatcgcgggaacgatcagcagtgccgaccaagacagcgaaatgcccgcccagagagcgaccggcacatacaggatgatctggtgggcaaactggatcaggttgcgcgcaatgcttcgccagacaaaaaggctgatcggaaagtagccctgcttcaggtagttggacgagcccacgaacgcgttgcacgcttcggagaccacgctggaaaaaaaggcccagaagatgattccgagtgcaaggtgaggaaagaactttgaaagttccgtgccgaaaagcgagctatagagcggacccatgccgccaatcattgctcccatgctcagcgtgagccagagcgggccgagcatcgaacgccgatagcgaagaacgatgtcaaaccaggccagcgtccaccagatgtcggtgcggcgcgtcccttcccaccagtcggatagggcgctacggtggagatttgagtgaatttcttgggtcatgcgcgtccgtaggtgtctgcgagcctgacgatatcgtcctcgccaaggtaaacaccgcactggacttcgataagcaccaatagttcttcgccgatgttggtcaaacgatgtttctccttcaatgggatatggcggtattcgcccggcccggtgacatgttcgatgtcgccgatctgcacgatgccccgcccttgcaccaccacccaatgctcggagcgctggtggtgatactgcaaagacagcgattctccgggtttgaccgtgattcgcttgaccttgtagctatcttcttccttgagtgttgcataggtgccccatgggcggtgcaccacggagggcagatgaaccgcctcgtgcttgcgagacttcagcgtgtcgacgatctttttgacttcctgggcgctgttcttgtgggcaaccagcagcgcgtcgggagtgtcgacaatgacgaggtcgtgaacgcccagcgtcgccaccagtttcggaatatggctgtcgacctgcacatgggtgccggtggtgtcgatcgccacgacgtctgatggcatggtgttgccgctcgcatcttggggctgggcttttgccaccgcaggccaggagcccacgtcgctccattggaacttggccggaaccacgtgcacgttgtcggccggctccatcactgcgtagtcgatgctgatgtcgggctggagtccgaaggcatgcaaatcgaactggatggtgttgccttggtgcgccgagctcttcagcgcttttttggcggcgtccagcagttcgggcgcgtacttctcaaaggcggccactatggcgtttgccgtgaagcagaacatcccgctgttccagtaatagcgtccggtagccagatactcctgtgcggtctgcaaatcaggcttctcgacaaagcgcttggccggttgactcgaccgcgagacctgggccacttcgatatagccgaagccggtgtccggactcgtcgggctgatgccgaatacaaccagcgctccttgcgtggcaagtttgaaagcctgactggcactcgcgacgaaggcttcgacatcgggcacgaggtgatcggcggacagcacgagcatcacggtttcgccaccgaatttctcgatgcattgcagcgccgcgagcgcgatggcgggacccgtattgcggcccttcggctcgagaagcagcgtggcgtccggcgggtcggccatttggcccagcacgtccttggtcaggaagagatgatccttgttcgtaacaatcatcagatcaccggtgccgcaggcttggccgcgttcgatggcctgctgcagcagcgtagagccgcccagcttcataaaaggttttggaaacgcctgccgtgatgctggccaaagtcgggagcctgccccccccgagagcacaactgaaagtacgtgcattttttataggagtgtgaagaaggggataattttaccggccttgctccaaagggcccgtaaccagtggaagcctctatttttgtgacctcgagcaatgttcagtaagcccacgctgccagccgcgcagccccatattcggcgaagagggcttgaaaacggcttgagcagtgcgcagcttcaacgccggatcgccttgctcgagcacgagacgcagtccctcgaaacgcggttattggagatgcagcagtccaccagttggcgcatcacggcgccgctgcgctgggccagccggtatcttcagcgggtcgtgcgcggtgcacccttgccgcaggtcgaagaacgaggagattacgcggattgggtcgagcgttacgacaggatcgatctggccgacaccgatcgcaggcgccgcgaaatcgatgcatcgccgaaacgccagcgtttgctgctgctgcccgcaggcgaactgagcgaaggcacactcgacgcgcagttgtacagcgaatggacgcaaatgccggccggatccttgccccagggcttcaatgcggcggcctccgccgactgggtcatctggatcgaaccaggctgcacattgccgtcgcatgcactctgggtcatcgcccaacagagcactgcgcaccccgaggcccgcctgatctatgccgatgaagacgagctggatgcgaacggtcggcgcatcaatccttttttcaagcccgactggaatccggaccttttcctcagccgcaatctctttgcttcgtgggttgccatcgaggcccacctgttcgatgaatccggcggagttcgtgcggagctgccgccccccgagcagggctatgacctcgcgctgcgctgtgtggagcgggttggcagcgagcagatacgccacatcccatacgtgctcgcccaccgccgtgcttctgaggtcgagttcggtggtcggcctggaggcgttgccgtattgaatgcccatttcatgcgaacggccaccgcagccagggccgaggccacgcagtttggctatcgcacccgttatgcgttgccatcttcgccgccgctggtttcgctgatcatcccgacgcgcaacgcgctgccgctggtacggcagtgcatcgagagcatcgtgctcgagacagactatccgaactacgaaattcttctggtcgacaacggatcggacgaccctgaagcgcttgcctacttcgccgcgctgaatgcgcagcagggcatcaccgtcatccgtgacgatcgtgcgttcaactattcggcgctgaacaacgcggcagttgcgagggcgcagggcgaacttgtcgcgctgctcaacaacgacattgaggtcatctcgcccggctggctcgcggagatggtgtcgattgccttgcagccgggagtgggcgctgtcggcgcgaagctgctttatcccgacacgactgtccagcacgggggcgtgattctgggtgtcggcggcatcgcaggccacgcccacaagcacttggctcgttcggatcccggccatggcgggcgtgcgcagcttgcgcagtctttcagcgccgtgactgccgcctgcctggttgtgcgcaaggcgctttacgagcaagtgggaggactcgacgaggaacacctcacggtggccttcaacgacatcgacttctgcctgcgccttcgcgaagccggttaccgcaacgtctggacgcctgaggccgaactgttccatcacgaatcggcgacgcgtgtttcggatttctccgggccggcgctgcagcgctttcttcgtgaagagcagttcatgcgccggcgctggggcgcgctgctgaaggccgaccccgcttacaaccccaacctgagcctcgccgccgaggatttcagctacgcttggccgccccgaaccccttggctccccccttcgacatgacagcaggcccgaacgccgccgcgccaacacccccctttgtttccgtcgccctttgcacccacaacggcgcgcgtttcctgcgcgaacaggtgcgaagcatctgcctgcagaccttgccaccggtggaaatcgtgctgtccgacgacgcatcgactgacggctcggtggaggtggtgcgcgctgcggtggccgagtgcgcagccgagcggccggagcatcctgtggccctgcgcattttcgagaacaggccggcgttgcgcgtggtcaagaacttcgagcaggcgatcggcgcctgcaccagcggcctcatcgcgctcagcgaccaggacgacgtctggctccctgaccgcctcgcgcagatggtgccgcttttcgaacgcgatccgaagctgctgctcttgcacaccgatgcacgcctggtcgatgccgaacgtcgcgacctgggccatacgctttttcatgcgctcgaggtcacgccatccgaaatcgagcgcatccatggcggaaacgcattcgacgtgttccttcggcgcaacctcgtgaccggcgcgaccacggtgtttcgccgctcgctgctcgagcacgcactgcccctgccagtcgaatgggtgcacgacgaatggctgggaatcatcgcctcggccatcgggcgagtcgacctgctggagcagccgctgatcgactatcgccagcacgagtcgaaccagatcggggcgcggcgcgacacctttgcagccaaggtgcgaaaggccctggcttccaggggcagcacgcacgtcgagcgggccttcaaggccgaattgctcctcgcgcggctgcaggaattcggagacgcggtctcgccagagattctcgcgaaggtgcgcagcaagatcgaacatcagcgctttcgcgccgcgttgcccgcatcgcggatcgcccgttgcctgccgatccttcgcgaagccatgaccgggcgctacgacaagttcggccgcggctttcggggtgtggttcgcgatctgttcgaatctgtgtaggctcgcctgccaccgaaccgcgttcttccagaaaaacaatgaccccaatgaattcctctccaacatccgtcgccagcggcaccggggttgcgcccaccgtggtggtgatcatcccgttctacaacggcgccgatttcatcgagcgttcggttcgcagcgtgttcgaacagtccgtgccggcgaacgaagtgatcgtggtcaacgacggctcccggcctgaagagcgcgcggcgcttgacacactcgcggcccgttatcccttccgcatcctggacaaggagaacggcggccagggctcggcgcgcaacgccggagtggctgcttccacgtccgagtacatctgctttctcgaccaggatgatttttatctgcctaatcacattgagatactggtcgaagcgattcccgctaaggaggcgcggttcggctttgtctatgcggatctctacgaggccgatgcggacgccaatgtggtccggactggtgtggtcaagctgggcgccaaatcgcaccccaaaacggatctcttcgacctgctgcgccacgacatgttcgtcctgccatcggccagcctgatcagccgaaccgccttcgatgctgttggagggttcgatccgcagttcacggggtatgaagacgatgatctttttctgaggatcttcaggaaaggctacaccaaccatttcgtcgatcgggccgtgacggtctggtgcatccacaccgccagcacttcgttcggcgttcgcatggtccgcagccgtttcaggtatttcatgaagctggccgcggcctttccggacgagccgcggcgctcgctgtactacctgcgcgattacctggtgccgcgtttccaggcgtacttcgtcgaccacgcgatcgattcggccaagcacgacaacgaataccgcgccgagatgctcgacatcctggagcagtacgccacggtggtcctcgccaatccatcggtgggccgcaagtccaagctcaagctgcgcatggtcatcttcctgctgcgccgcgtttcgccttcgacggtggcggcgatcggttccctgaccaaggtgccggggctgcgcacggtcaggcgcctgctcgactgatggcgcctggtgtccgggcgaactgagcggccgaccttgccttcatcggccgtggcgctcgagcaggatgtcgtcgaggtagggcaatgtccgagcgtagtccgatcgaaaatggtcgcgatctttgtacaccggcgtcccgtcggccagtgcccggatgcagtgattctcggggcacaggaaaggcagcggatcaacaatcgatgcaccgctgctgttggcgatctcggccatgcgctggttgaggttgttctgcgttgtgcgaagcgcaatgtgaggggtcatccgcccgacgtgcatggtgccgagccgatggccgctgatcagatgctcgggactgaattccagcccgatcgggttgtccagcagcaggtagaccttcttcctcgaagcgatgcgtttcagcagaatctccagcgaggccagcgatgcgtccaccccgctgccttcgcggaagaggagtttttgtgggcctgcgcggaagtagaacccttcttcgctgagcgcgcccgtggccggctgggcctggtccatgaaatagcagttccagcatcccccgatcacgacggtgtcgacatcgtcggtcaaagcgtaatcgatgaaggccgttcgcaactcgtcgcagcccggcgtggcatcgcgaaaaatacccggaacgaaaggacatcccggtgcggttgcgaacgtgatcgagttcagctgctgcgctggatccttcgccagttgtgcggcacggatcgcatattgctggacgtggctgtcgcccatgatcaagacacgctccttgccggagccaacccgaaagacggtctgtccgcttttcagttttgccggggttaggccctccccgaacacccagttctttcgtgccgcctcgaccgtgtcgaagtaagagtcgtccaggcggcctgtgagccggctcgtcagagcgaagacaccgagcacagccaagcaggccacggctgcgccgagcgtgcgcaccatgcgcggcgctgacgaggcccgtgccgggcgttcgacaaatcggtaggtgatccaggccagcagaaccgctgtcgccaacagaaaggcgcgcagggcttcggatggcaggccaccttccacgatgcgcgcgaacacgagcaacggccaatgccaaaggtagagcggataactgatcaggccgatccacaccatcggcctggaggcgagcacgtagcggttgagcacgccggtcgggccggccgcaatgcagtagaacgcacccagcgtgggcaggatggcccagaaccccggaaaagccttgttgccgcggatgtaggcgagacccaggccgatcagcaccagcccggcaatcgactgcgcatggcggccccagcccggcttaggcaggggccggtgcagccgcatgtacgccagcatgccgccgatcatcagttcccagaagcgcgacagcggcgaatagaacgccgccgtgcggtggctgtggatcgtcgagacgttcaacaggaacgacagggccgccacggcccccacgaccgcgagcacgcgccacttgcgcttccacgccaggcccagcagcacgggccagaagatgtagaactgctcttcgatggccagcgaccagagatgcagcagcggcttggtctcggccgcattgtcgaagtagccggcctcgctccagaaggcgaagttcgagacgaagccggcacccgccgccacatgcttgccgagctgctcccattcgtgcggcagcagcgcataccagccgaaggcaaaggttgccgccagcaccaggaccagcgccggaaagatgcgcttcacccgccgcgcgtagaactcgcggtagctgaatccgtcgccctcgaagctgcccaggatgatcgtcgtgatcaggaaacccgagatgacgaagaagatgtcgacaccgatgaagccgcccttgatccactgcggaaacgcgtggtagccgagcaccgaaagcaccgcgacggcgcgcaggccgtcgatgtcgggtcggtatttggggtgaaccaggtgggcgtgttcctgcggggatgtcgggctgctggttgtcgtcatcgttgtcgtgtgggatgggaaagcggctctgctgcgggcttcccggccccggattgtcttcgcaaacgcagaagcgcctttttcagggctggcgagggcgcgcccgcaggtagcgccagaacaccgccgagctccacacctttatcaggctggtcacgtgccagtaaaggtgcttcttgctgctgcggctggcgcgctgggcctcgtggcgtgcgagcaggtcttcccccacctgcagcttccagcctgccagctgggtccttgcgcagatgtcgaagtcttcgccgtacatgaagaaacgttcgtcgaagccgccgatctggcggtaggcgtcgcttcgaaacagcatgaacaggcccggaatccaggccggcaccgccgggcgcacataaccgggcttgcgccgggtgaggatctcgagcggcgtgatgatcgcgcggtgctgctcgggggtgcgcttgcccggctccagaatgcgcggcgtcaagaggccggcatccggcgcggcctgtgcgagcagcggggccagcacgtcgccatcgaagcggatgtccgggttgagcaccaggaaccatggcgtgtcgcagcgctcgaacgcctggttgtggttggccccaaaacccttggggctcgcgttttcgatgcgctcgatggcaaacccccattccaggccggccagcaggtcgggttcggggatgttcagcgtgagcactaccttggcggtcgaggcccggctgaagcggtcgagttgctcgagcagcggcagcaccagcgcgagctggccgtggctgacgatcgagacggtgatcgggggttgggagggggagggcgctggcatggtctaatttcgctcgggaattctagggttccccaacacccacacatgattgctctgatcgtcatcagttttttcgtctccgcctttgcggtccagctgttcatgcgccgcgcgcgcaggcatgcccggctctacggcaccgacatgccccagcgcttccacagggggcacgtgccgcggctcggcggggcgggcatcctgctcggcatgggcgcggcctggctggcttccggcatcaccgggacggatccgttcaacgtgtcctggccggtcaagacgtcgatgctcacgctgctgtgcattgcgccggcggtgctcgcgggcatcgtcgaagacgtcacccagaacgtcagggtgcgctaccggctggggctcaccatcggatccgccttgctcgcctgctgggtgctcgggctcagcctgtcgcgcaccggcatcgagacggtcgacgggtggctggccatggttccgtatggcgccgtgctgttcgcggccctggccatcggaggcctgccgcatgccttcaacatcatcgacggctacaacggcctcgcgggcaccgtggcggtgctggtctgcctggccatttcgcacgtggccctgcaggtgggcgatcgccaactggcggccatgatggtgtgcctggtgggcgccaccgtcggtttcctgatctggaactatccgcgcggcaagatctttgccggcgacggcggcgcctacgtgtggggcatggtcattgccgtggcctgcgtgacgctggtgcagcggcaccgcgtcgtttcgccgtggttcccgatgctgctgctgatctaccccgtgtgggagacgctgttttccatctaccgcaagttggcgcgcgggcagtcgcccggcacggccgatgccctgcactttcaccagttgatcttccgccgcatcgtgcgggtggcatttgccgacgacgaagcccggcaattgcttgcacgcaacaacaggacttcgccgtatctgtggatgtttgcggcgctgtcggtggtgccggccgtgctgttctggaacaacaccatcgtgctcatgctgttctgcctgctgtttgtcacgacctatgtgggcgcctacctcatgatcgtgcgcttcaaggtgccgcgctggttgcgcccctgaccgcgctttctttgcgagaatttcttctcatcgtccttcgctttggagcctgatcgcccatgaccgaccccgtcctcaacatccccccgcgcgacaaggccgagatcctggcccaggccttgccgtacatccgcaagttccacggcaagaccatcgtcatcaagtacggcggcaacgccatgaccgacccggcactgcaggccgacttcgcggaagacgtggtgctgctcaagctggtcggcatgaacccggtggtggtgcacggcggcggcccgcagatcgaggcggcgctcaaccgcctgggcaagaagggcagcttcatccagggcatgcgcgtcaccgacgccgaaaccatggaagtggtcgagtgggtgctggccggcgaagtgcagcaggatatcgtgggcctgatcaaccaggccggcggcaaggccgtgggcctgaccgggcgcgacggcggcatgatccgggcgcaaaagctcaagatggcggaccgctctgaccccaacctgcaccatgacgtgggccaggtgggcgacatcgtctccatcgaccccagcgtggtcaaggcactgcaggacgacgccttcatccccgtcgtcagccccatcggctttggcgaggagaacgagagctacaacatcaatgccgacgtcgtcgccggcaagctcgccaccgtgctcaaggcagagaagctcatgctcctgaccaacacccccggcgtgctcgacaaggacggcaagctgctcaccaacctgagcgcacgcgaaatcgacgacctgttcgcggacggcaccatttctggcggcatgctgcccaagatcgagggcgcgctcgatgcggccaagagcggcgtgaacgcggtgcacatcatcgacggccgcgtgccgcacgccatgctgctcgaaattctgaccgaccaggcctacggcacgatgattcgcgcgcgctgagggcgcttccgggctggtgggccgtcggatctagccgttcaccctggcaaccgcgggtttccggcccaggaattcgaagcccgcggcgccaacttcctgcaccgactggggcagcttttcgaaatcggtccagaggggcgtgctgcgcagcgagggatcgcgccacaagtccacgagttcgcccgtggaggcatcccggaagcgctcggcggcttcgtcggacacgttggcgcgaagcgcctgctcgcactccgacgcgagccagctgacggcgtggttgggcgaaaaattctccgacacccggactcgctcggcttcgaactcccgaaaccactgctccagcccgtaccgggtgcagttgaagaagtgccacggccgttcgtgcagcggctgcatgaacgcggtccgaaccaggatgcggccaccgggcttcagtacccgcaggagctccgccgccaccttctgcggttcgcgatagtgctcgaaggcgttcatgacgatcgccgcgtcgaagactccgtcgtcgaacgggagcacgtgggcgtccgcaaccacgtccgtatgcctgaacaggctgtactcgacctcgaccacgttctcgattttctcctgcgagcctccgccgctgagattcaggacccatcccttggtgctctttgcaagcttcagagcttcgggcggcagcgggttgctgacatgatcgacgggcttcacctcgggctcgccgagttcctcgcaaagaaccggtcggccttggaagatgggccaggtcctccagccgtccacggtcaccagggtgccccgctccgcgtcgtgcgccaacttgagtcccgtcttgggacagcgaagtatcggaagcagcgtttgaagccgcgacttcacagtgtcgtcgcccaggcgcacctgcagggccggcggtttgcgggcaagccgctcgtcgatcagcgacacccagggatgctgggccttgaagttctcgatcaggcggcgatagttctctggaaccgtcgtctcggccttgatcatcgaacccgcatgcacgcggtagtccgcgagcgtttgcggttcccggaatccgcgctggccttgctcggcgagccggcaccagaagtcgtagtcctcccatccgtggcgaacgtggttgtagccaccgacgatcgcccacgcttccttcgagacgagcgccattgcgtcgatgtagttgcccgccacgaagcgctgcggctcgtaggaggcttcgccgagcatggcgctggaggcgccgaagtgctggatggtcggatagacgaatgcgacgcgctcggcgcggagggcgcggcgcagttcttcgcagcactttgcccgcagccggttgtccgcgtccaggggaagcacgtagcaactgtccgccagatggaagccagcgttgcgcgtcaagcccaggccgcagttcgactcatgctgcgcgaccaccacgcggttgaagcgcgtggcgtgctgccggacccatgccagcactgtgttcagcgaatcgtcggtcgagcagtcgtccaccaccacgaggtccagtaccgccagtgtctgtgcccggacggattccagtgcttcggtgatgaactgttcgtagttgtagagcggaatgacgaccgagacctctgcgagctcgctctcgccggccctgtgttcgaacagcactttcagaggcatcaggctgggccggcgaaccggcgccgagcgaacgcgtgcgtcgagcgcaaaggcccgtgcggccagggcgtcgccttgcagctggtcaagcacgcggccgaactgcgcggcgcgctgcagaggtccatacgaagccatggcgcgcaggaaggccgccgaaccgatgctcgccctgagcgcctggtccccggcaagggttgaaaggtagtgataccagtcgtcggcggtggtcgccagaaaacccgagacgccatgttccatcgcccgcgtgaaggggccggtcggagaagcgatggtcggaacatcgaccagcgcggcttcgaagaatttcaattcgctcttggcttcgcagaatggattgccgaattcgagcggcgcaatgttgatgtcgaagcgcgctatttcccgcggcagcgtttccagtgtctggaagggccgccactcgatgcggtgctccaggccggccatcgcggggtattcctccacgtcgaccaggcgcatgcccgattcggtctggaacagcaccaggcggcacagctcgttttcgcggagcaggcgcgcaatcgcctcgatggcaagccccaggtcgcgctgatgcgttcgcgatccgccggcgtagccgatccgcaccaggttgtcgggccgcgcgctacgccattgcgttgcactgcgcctggacagttcgaaagtctggtcgtcgaaaccattcaacaacacatgggtggtcttgcccgcgcagcgcatgtggtaggccagctcctgggtgctcgcaacgcacacgtcggccgcgagcatggccctgcgcacgcttgcgaagagctcgcgcaccgcttcttccgggtgggcgttggacctgatgccatcgatcaccttggtatcggccagatccggttcgatcatcaggtcgtcgatgtcgaacaccaccttcttgccttgcgtatgcatcagccctatggctttttcgagaacgggactccactgagtgcgccagaggatcatcacgtcgtgccttgaagtcagctggagctgcgtttcgagctggtcctgccgcacccactcggccgcgacgccattcatgcgtgctgcctccaggtagcgcgccacgcgatattgatggcctggcgtatccgcctcgccggaaacgtagaagatcgagaaggcccggctcggcaacgggggcagaaccgagtcttccttgtcgtccccgcgcaggccggcgcgccggccttcccgcgcaccgaccagcatgtagtgaagcagaggattgaagcccgctgcgtccgcgtagtgcgctgtgtattcggagccggagaaccacggaccagggtcgcgaccttcgcttgcaccgtaggcgacgtagtgttccgcagggtctacgccagaggtcgccacgtcggggtaggtgttcagataccagtcccgatcgaagtagggtgagaatctaacggtctctactgtcgcaagatcgacacgccggccggcaaggcgcttggcaagcagccggagacgcttacgcatcttggccttcaccctcaaagagggatcgatccgaaggcgcgtaaaacgttcgatcagggagttggcgaagtctttccgtgcgagcaccgcccgcttttgaatagtgatctcttcgccggcttccttcaaatcttctcgcgccttgttgaggtcggttgccaactgggtcacgacattccgtagctccgccacgcgcctgcttgcctgctcgtgtgcgaagctcgtcgcccgagcagcagcttccgcctgggccgccttggctcccgcatcgcccgcctgctttgtcaacgcctccagttgagcggccttatcggcaacctcatgggacaacgcgattacttcaccctcggcgcgtgcgcgggcttcggcttcggcgagccgggctgccgccacttgggcaagttcggcttcaacaggggcccgaagggcattggtctcatggatgcgctgattcagttcggccgaaccgagctgctcgcgtgtggtgacgaaccagcgcgcgcccagatgcgcaaagcgggtcctggcggcatctgcctgttccggttccaggttgcacaacgccatggctgccgcaggtgcgtgctttccgaccgccaggatgccgaggccatgcccatgcaggaactcgaaagaggggtagttttgtgactgctctgcgaaaaagcggaagactccgaaattgccactgcgaacattcgtgtcatggaacaggaccacggccttgtctgacagcttgggaagccaggtctcgaagtcgtgcttgaccgcctcgtaggtatggaagccgtcaatgtgaagcaggtcgatggagccctcggggaaatagggcagtgcgtcgtcgaaggtcgacttgagaagttcggagaacgagctgaagtgcttgtcgtgaaaatcacggagctcgtagtagacctgcgagtcgaaatgtccggcgtgctcgtcgccggcccaggtatcgaccgcgtagcagcgcgtcgccgacttgagccgggccacggcttcgcaaaaggcggcatacgacacgccgttgtgcgtgccgagctccaccagcaagcctggcctgcatgcggccacgatccagaacgcaaacggcgtatgggtccaccaggcgctcgccttgccgagcaggtgcggtgtccagaagagtggatccagcacagggtgcgtcagaacgtcgagcgatttgtcgatcgtcggaagaatgatggtgggttctttcattgttctcgcccagacgcgtccgagcctccgctagattcggtttgatgaaactgccggtgtcagcgtgcgagctgccagcgtggatcgacgttgtttgccaactgggcgccggtgagccagtccagcagcacattcgggttgtgataggggtcgttttcgaagcgatcgatccacttggcgctggtgtagtcctgctcgcgccgggctcgcttctgcttttcttccgaagcgtggtcgtgtccgcgcgacgcgctttcaaggtgcagcagggatgcaaatggcgtgcagatgttgcggtaccccgcatcgctcaccttgaggcaaaggtcaacgtcgttgaaggccaccgccagatgctcgccgtcaaatcccccgacctgctcgaacaccgcgcggcgaacggcgaggcaggccccggtcaccgccaggtaccctcgcgtgcccgcaagacgcccgtccactccggagtccgtggcgtcgtctgtgcggcacacatgcattgcgagcggtccgcgctgcaggatgacgccggcgtgctggacggtgccgttgccgtagaggagctttgcgcccacgcagccaatgtccggccgcatgacttcgccaaccatttcgcgcagccacccggcatccagcacttcgatgtcgttgttcaggaaaagcagcacctcgccagtcgaagcttgtgcgcctgcattgttgatggccgaaaaattgaaagggccgggaacgcgcagcacgcgaacgcgaggatcaccgcgtagttccgcgaacaaggccatggtcgccggctcgatgctgtcgttgtcgagaatgatgacttcgaagtcgggatagtcggtttgctcgagcaaaccattcaggcaggtcctgaccaggctcgcacggtcgcgggtcggcacaagcacactcacccggggcgcagggttgggtagcggcctgcgaacgtggttgacaaactccgcgatgggcgacggccgaacatcgactgcggtccctgtctgttggaaggccgctgccgaggcgacccgcctggcggccgccgcgtaggtctcgatggcgtccgcggtgtcgcgcgcattcaggaccggtggtatccgccggtgatacagcaccgagggcacatgacggatctggctgcaatgcaatggcatggccactctgcaatgcagatcgtagagtgcggccggttcgaactcggagccaaaacccccggcgtccagagcgtttgcgcgcttcatcacgcacaggccatccagcagatcaaaccccagttgcgcctccggatcccaagctgatttgaaccgcggcttgcagcggatgccgtcctcggtgatccagtcttcgtccgaatacacgaccaccgcctccggccggtttgccaatgcgagctgcagggaggaaacggctgacggagcgagccggtcgcctgccaggatcactccgaaaaaggtttcagccgaatgctccagcgcgattttcagcaactcggtgcggcttgccgatgcgcccgaaacgacgaggcgaacattgaccgaatccttgacgcacaggagcgccgcgttgacagttgcggcacgcgagggctggcacgccaccaccgcatcgaatcgatggcaccattggactgaaagcgacgccaacgagtcgcgtagttcttcgtcatcgccgttgtcagcgatggcgaagctgatgccgtgctggtaggggagactcgccagttcgatacccagcgccgccttttgcgcttgcagacacgatgcgccttcttcagtccaggcccggtatgcgtcatccgcaaaagatggaaaccggcgcgctgcggcccaatgggtatatcgtgcttgatcgatagacaaagtcattctcccaagtgttcaaaggtgaagcggtagctggggttctctggcgtgcagaaatcccgtcgattcagaataccgagagaagcagctatgaaagagctgcagggggtaacaggctgtttgagccttggcttactcgatacggaggtatgcgttcgttaccagcgtaatcaattcgaagtaccgcagcctgaaggacaacgcgccgttttgatcccagcgcgtgcctcgtcggctctcgctgcaatgccgccaatgtggtcagcgatcgatggctgcagtgtcgtacccgttcgggttcccctgctgccaccgccaactgtccgcgcacatctgatcgagcccgcgttgcgcacgccagcccaatgttgcttctgcgagcgacggatcgccccagtacgcgggcacgtcgcccggccggcgcgggccgatctcgtaaggcagcatccgcccactcgcgcgttcgaacgcatgcaccacctcgagcaccgaggcaccgcggccggtgccgagattcaacgtgaccaggcccgcttgtttctccgcgtaccgcaaggcctcgacgtgcccctcggccaggtccatcacgtgtacgtagtcgcgcacgccggtgccgtcgggcgtcggatagtcgttgccgtgaatgagcagcttgtcgcgctgccccaccgccacctggcacacgaagggcatcaggttgtttggcttgccttgcggatgttcgccgatgaggccgctctcatgcgcgcccactgggttgaaataccgcagcagcgcaatgcgccagcttggctcggcgcggtgcagatcgatcagcgcttcttccaccatgcgcttcgagcgcccgtaggggttggccggcctgcagggcgcgtcttccggaatgggcgaatggtcgggttcgccgtacaccgtggccgacgacgaaaaaatcagcgtatggacgcctgcctgctgcatcgccgaggcgagcaccaggcttccatgtacgttgttgtcgtagtaggtgagcgggtcggccaccgagtcgccgacggccttgaggcccgcaaaatggatcacggccgagaagcgttcgttgcccagcacgccgtctagaagagccctgtcgcgcacgtcgccctcgatcagccgcggcgcgctgccggtgatctggcgcaaccgctccagcacgcggacgtcgctgttgccaaggttgtcgagaatgaccggcgtgtatcccgcagtggccagcgccacgcaggtgtggctgccgatgaagcctgcacctccggtcaccagaacgctgccttgggccatgtgaactctttcctgtttgcagagcctgattctgtacgagctttttggggattggtttgcacgcgctcactgcaggcgcccctgtgcgagaatcaattgattacatctttgcacgcgctcccatgcagaacgaagagacaagctatcccggcgtagaaacccagacagagacgctgaccactgccgctccggtgcgaaagcgacccaagcctggggagcggcgcgtgcagatactgcaggcgctggcgtccatgctcgaacaacccggcgccgagcgggtgacgaccgcggcactggctgcgcggctggacgtgagcgaagctgcgctctatcgccatttcgcgagcaaggcccagatgttcgagggcctgatcgatttcatcgagcaaagcgtcttcacgctggtgaaccagatcctcgagcgcgagggtgcaacggggggccagcaggccgcaagaatcctgacgctgctggtgcagtttgccgagcgcaaccccggcatgacgcgcgtcatggtgggcgatgcgctggtgttcgagaacgagcggctccagcagcgcatgaaccagttcttcgacaagatcgaagccaccttgcgccaggtgttgcgcggcgccgccacggcggacggctcgaccacgcccacggtggacgcccaggtgcgcgctgcggcgctcacggccttcgtggtcggccagttgcagcgcttcacccgctcgggcttccgacgcgcgccttcggagcatctcgaagccacgatcgcgctgatcgtcggctaaggcgaggcgcagccaggtggcgatcctggcgatcggccgcctatcgagacgacagctcgttgcgatgcagctgactagcccgcgccccagctgacccgcggcggcccgggagggtacccaggggatggcgcgggaccgcgcgccgcactcgacttgccttgttgcgaagcgtacgatcagtgcccccttgccgctgaatcgcggcgacaagtccgtgtttgtgtggcttctgaacggaggttcgtatgagctatcacctggaaggtcgcctgctggaagtgtgcaactgcaacgtcctgtgtccctgctggatcggcgaggaccccgacaacggcacctgcgacaccatcgtcgcctggcgcatcgacaagggaaccatcgacggcgtcgatgtgggcggcaacaccatcgccgccgtggcacatgtgcccggaaacatcctcgaaggcaactggacggcggcgatcttcgtcgacgacaaggcctccaaggagcaagaggaagcgctcctcaaggtctacaccgggaaggccggcgggccgatcgccgacttggccgcgctcatcggccaggtggtgtcggtcgagcgggcgcccattcgcttcaccgtgaacgaaggcaagggcgagctggaaatcggcaaggactactacgccgaactcgaaccctaccgcggcgcgaccggcggacagaccacgctttcggacaccgtgttctcgacggttccgggcgcgccggtgttcgtcggcaaggccccgacctaccgctcgaagaacgccgccctcggcatcgatctcgacatcaagaaccacaacgccctgcagagcaccttcgtcttcgactcatgatcccgatggccggctcgccgctgcgccacgccgtccgccaccgccgcgtgttcctgccggttcttgccgcgctcgccacgctcgcgtggctcgtgctgtgggcctgggcgcgcagcccctacgggcgctatctcgaacacggcgactggaccgtctcgggcccggctgcgttcctgtgccaggccattcccgccggcggcgtgatcgtgcccgcggtgctctacgccgcggcatggatcctcatgacggcggccatgatgctgccgaccacgctgccgctgttcaacgccttcgatcggttgaccacggggcgcccggaccatgcgcgcctgctcgtgatgctggggctcggctacatggcggtgtggggtgccttcgggctgctggcgcacgggctccatagcgcggtgctggcgctgctcgcgagcgcgcccacgctggcctggcacggctgggtgatcggcgccgcgaccatcgcgctggcgggcgctttccagttcagccgcctcaagcaccagtgcctcgaaaaatgccgcacgcctttgagcttcgtcatcgagcattggcgcggacaggcgcagacacgccacgcctttgcgctgggcatgcaccacggcctgttttgcgtcggctgctgctgggcgctgatgctgctgatgttcgcgctcggaaccggcagcctcggctggatgcttctgctggccgtcgtcatggcattggaaaagaacgttccctggggccatcgcctgagcgcgccgctcgggttcgcgctgctgggctgggccgtcttcatggtggcatcgcatgtctgaagccgtgtccgaggcgcgcggcgccccgtccctcctgcagaccatcgtcctcaccgcggcggccatggtcgcgttcgcggccaattcgctgttgtgcaggctggcgctgcagcatgagggcatcgatccggccagcttcggcagcatccggctggtttcaggcgcgctcacgctggccctcgtcgtgcggctcagggcgcggccgccttcgcccgcccgtgtcgattggctcgccgccgccatgctgttcgcctacgtcgcgtttttttcgttcgcctacctcagcctgccggcgggaacgggcgcgctgatcctgttcggtgcggtgcagctcaccatgctcggcgcgggcctgggctccggcgagcgcttcggaccggttgcatggctcggcttcgtgctggccgcgggcgggctcgtctacctggtgttgccgggggtcgccgcgccgccgctcctgggcgccgtgctgatggccgtcgccggcgtggcgtggggcgtgtattcgctgcgcggccgcggcgtggccgacccgctggccgccacggcgcgcaacttcttgcgggccgtgccgctggccctggcgctgagcctggttttcatcgcccgcgcccatgccgacgcgaccggcatcgcgctggccgtggcgtccggcgccctgacctcgggcctgggctatgtcgtctggtatgcggcgctggcccggctttcggccatgcaggcagccaccgtgcagctgtcggtgccgctcctggccgcgatcggcggcgtgctgctgctgtcggaggcgatcacgccgcggctggcggctgcgtcggtggccatcctgggcggcattgcgatcgtgctgagccagaagtcgcgcagcgcacgccgttagccgcgcaggcaggctggtttctacgcgacggccacgcccaccttcgaaccggccgcgacgatttctccccacgttgcatcgtcgagccagatgccttcgcgctcgcgtgcgacgcgcgccgcgcgctccggctcgccggcgatctgcacctggtcgaagccggcgcccggcgggctctgcctgagccagtcgacaaaggcggtcgcctcctgctcgaagctggcctgggttcccagcttgccggggtcgatcaggatcgtcagcatgccgttgagcaccgtgcgggcggtgtcggccgggcggtgccaggttccgccaccgctgagcgcaccgccaagcagttcgcacgccatcgccatgccgtagcccttgtgctcgccgaaggtcatcagcgcgccgaagaggccgttggcctgcggcaccaccaccacgccggggtcgttggtgggcgcgccgcgctcgtcgatcaggtagccgtcgggcacccgttcgcccttgttgtgggcgacgcgcatcttgccctgggcgacccggctggtcgcaaagtcgagcaggaagggctcggcccccgccagcggaatgccgatgcagcaaggattggtgccgaatcgcccgtcgccgccgccccatggtgccaccacgggccgcgacagcacgttgacgaagtgcatcgagaccaggccctcggccgccgccatttcggcaaagtgcccgatgcggcccaggtgatgcgcattcgcaagcgtgaagatacagctgccgtgctgcttggcgcgtgcgatgccgagctccgtcgcctgcacgccgacgatctggccatagccatgctggccgtcgatcgcgagcatcgtgccgatgtcggcattgaccttgaccgatgcattgggcacgagcccgccctcggccaccgcatcgacatagcgcggcagcatgcccacgccgtgcgaatcatggccgctcaggttggccagcaccaggttgccggccacctgcgcggcttcggtgggtgtgctgccggcggcagtcagaatttgggcgcattgcgatcgcaacgctgcggcgggaagggtcttgggcatcaattgactccatgggtttgttcaagggctgcgcagcaacgcccgttcgtggaacaccgcggaaccggctttgccgggccgctggtgttgcccccggagagggggagggcgaagcgacacgaagtgcgcgcagcctgggggtgagctacatcacggcgccgacttgccacggcacgaattcgttctggccgtagccatgtttctcgctcttcgagggttcgccggacgctgtcgcgagcaccagttcgaagatgcgctggcccatctcctggatcgagctgctgccatccacgatctcgccgcagttgatgtccatgtcctcttcctgccgctgccacagcgccgagttggtcgcgagcttgagcgaaggcgagggcgcgcagccgtaggccgagccgcgcccggtcgtgaagcagatgacgttcgcgccgccggccacctgtccggtggcgctcacagggtcgtagcccggcgtgtccatgtagacgaagccgtgcgccgtgacaggttcggcgtattcgtacaccgcctcgaggttgctcgtgccgcccttggccaccgcgccaagcgacttttcgaggatggtcgtgaggccgcccgccttgttgcccggcgaggggttgttgttcatctcgccttcgttgatctcggtgtagtgctcccaccacttgatgcggtccaccagcttctggccgacctcgcgcctgacggcccggcgcgtcagcagatgctcggcgccatagacctcgggcgtctcgctgaggatggccgtgccgccgtgcgccaccagcaggtcgactgccgcccccagcgccggattggcgctgatgccggagtagccgtcagagccgccgcattgcagcccgatcgtgatgtgcgccgcgctgcagggctcgcgcttcaccgcattggcgcgcggcagcatctcgttgatcagcgcgatgcctttctccaccgtcttgcgtgtgccgccggtgtcctggatgttgaaggtgcgaaagttctcgccctcggccaggtggccggtcgcgagccaggcgttgatctggttcgcctcgcagcccaggcccaccaccagcacgcccgcgaagttcgggtgcgtggcatagcccgtgagcgtgcgttccaggatctgcatgcccatgccctgcgtgtccatgccgcagcccgtgccatgcgtgagcgccacgatgccgtcgacgttcgggtagtcggccagcgccgagggattggtcttgcgcgagaagtgatcggcaatggcgcgtgccgcggtggccgaacagttcacgctcgtgagcacgccgatgtagttgcgcgtggccacgcgtccgtcggcgcgcctgatgcccatgaaggtcgcctcgcgcttcgggggcgcgggcttcacgtcggcgccaaacgcatagtcgcgctcgaagtcccccttgtcgggacccatgtcgaggttgtgcgtgtgcacgtgctcgccggccgcaatcggcttgctcgcaaagccgatgatctggttgtagcggcgcaccggttcgccggcggcaatggcacgcgttgccaccttgtgcccggcgggaatcaggccgcgcacggcgaagtcttcgaccttggcgccgccgaccagctggctgcgcgcgatcacgacatcgtcggccggatgcaggcgaatgaagggattcatcgtgaactcgtgttgtggggttggaagaacatcttgatgaaggaaatgctggcgattcaggaggcttttgcgcggcgccagctcgcgctgaatcgttggtgcgagttgtccatgtgggcgtgcatcgcggcgcgcgcagcctcggcgtcgcgcgcggccaccgcgtcgcggatggcctcgtgctcggcaatggccgagcgccaggaggccaccgtttcgaagtagccgcccagccgcgtgaagatcggtccgttgcgcgaatcccagaagctttgcaccgtttccaccagcaccgtgttgccgctggcgttgacgatggccacgtggaatgcgcggtcgccttcgagcggcagtatttcgcggtcggcgagcccgcgcatcgtttcgatggcgcggctcatggcgtcgatgtccttgcgcttgccaacggtggctgcaatggcggcggtctcgccctcgatcacgcggcgcgcgcgaatcagctccagcgggccccattcggtgggcgccaccggcttgctcacgcgatgcgaccggtcgagcacgtacacccccgaacccgtgcgaacctcgacccagccttcgacctcgagcgcaatcagcgcctcgcggaccgaaggccggctcacgccgagctgcttggccaggtcgcgttcggccggcagccgcgcgccgaccgcgaattcgcccttgccgatcagccctcggagctggtcggcaatttggcggtacaggcgctggggttcgacggtctggagcggcacggggtgggcaggcgttaagggttgtcctgaattggacaagtggtaaggccaattcagaatacggtccgtaccgcgccgtcgccatcgggccaaaccctgaacggccgcttccacctttcaaggagacatgcatgagactcaagggcaagaccgcgctcgtcacggcggccggacaaggcatcggccacgcgagcgtgctcgccatggccgccgagggcgcccaggtgtgggccaccgacgtcaacgagaagctgctcgagcgctacgccggcgtggccaacgtgcacaccgccaggctcgatgtgctcgacaaggatgcgatcggcgccttcttcaagagtcttcccgcgctcgacgtgctgttcaactgcgccggcgtggtgcacaacggcactgcgctcgacgccaccgacaaagacctggagttcgcgttcaacctcaacgtgcgcgcgcagttctggaccatccaggccgcgctgcccggcatgctggcggccgggcgcggcagcatcatcaacatggcgagcgtctgctccagcatgaagggtctgcccaaccgcttcgtgtacggcaccaccaaggcggcggtgctcggcctcaccaagagcgtggcggccgacttcgtgacgcgtggcatccgctgcaacgccgtctgccccggcacagtcgatacgccgtccctcggcgagcgcatcaacgccaacgacgatcccgaggcggcgcgcaaggcgttcatcgcacgccaacccatggggcggctcgcgcaggccgaagaaatcgcgcccgtggtggtgttcctcgcgagcgatgaatcggtgttcgctaccggccaggccttcacggtcgacggcggcctcaccatatgaaccagctcgacttcgccggccgccatgcggtggtgaccggcggcgcggcggggctgggtttcggtattgcacagcggctgatcgcatcgggcggcagcgtcaccctctgggaccgcgacgaggccgcggcccgccagacttgcactgcgctgggcagcaaggccttcgcggtgaaggtcgacgtggcgcagcagccttcggtcgccgctgccgtggcggccacgctggcgcacgcgccgcgcatcgatgcgctggtcaacagcgccggcatcaccggccccaacgtcaagctgtgggactacccggtcgacgactggcggcaggtgatggacgtcaacgtcaacggcgtctttctctgttgccgcgaagtggtggcgcagatgcgaaggcagggctacggccgtatcgtcaacattgcttccgtcgcaggaaaagagggcaacccgaacgccagcgcctacagtgcgagcaaggccgccgtgattgcgctcaccaagtcgctggggaaggaactcgccgacaccggcatccgcgtcaactgcgtgacgcccgcggcagtgaagaccgccatcttcgaccagatgacacccgagcacatcgcgttcatgctctcgaaaattcccatgggccgcttcggcacggtggaggaggtggccgcgatggtcggctggctttgcaccgaagattgctcgttctccaccggcgccgtgttcgacctctccggcggccgctccacctactaaccagttaaatcagtctcacaagaaaggacaacatgaaactcgttcgctatggcaaccccggcaaggaaaagcccggcctcatcgacagcgaaggccgtctgcgcgacctgagcgcggtggtcaaggacatcgggcccgagcaactcggcgatgctgcgcttgccaagctgcagaagcagaaggtcgacaagctgccgctggtcaggggcaagccgcgtttcggcagccccgtggccaatgtcggcaagttcattgccatcggcctgaactacgccgaccacgcggccgaatcgggcctgccgatccccgcggagccggtggtcttcatgaaggcgaccagctgcatccagggcccgaacgatcccgtcatgctgcccaagaactcggtcaagagcgactgggaagtcgagctcggcgtggtcatcggcacgcgcgcgcgctatgtctcgcaaaaggatgcgctcaacttcgtggccggctactgcaccatcaacgacgtgagcgagcgcgagttccagatcgagcgcggcggcacctgggacaagggcaagggttgcgacaccttcggccccctcggcccgtggcttgtcacgcgcgacgaagtgcccaacccgcaaaagctgtcgatgtggctcgacctcaacggcaaccgcatgcagaccggcagcaccaaaaccatgatcttcagcattgccaagatcgtgagctacctgagccagttcatgacgctcctgcccggcgacgtcatcaccaccggcacgccacccggcgtcggccttggcatgaagccgccgctctatctgaagaagggcgacgtgatgacgctgggcatcgaaggcctgggcgagcagcgccaggaagtggtgcctttcaagctttaaataaataggcccataaaacggcgcggcgggcgggagctcgttgcgcttttttgtttgcgcgccgtaacgccctcagcgcagcacccggatcagctcgtcatacaccagccgcacgcgcgcgggcaccggcgcacgctgcggacggtagacgttgatcggccatggctccggcgcttcggcctccagcacggacaccagcgcgcccgattgcagccagggttcggccagcggcgcaatgagctggccgaagcccacaccggccagcacggcggcacattcggcatcgatgtcgtcagtcacgaaagccggtgacgtcacagtgacgactcgccgcttgctgaacgcccacggccagggacgacccgagctcaggtcgatcagtgcggtgagcggcagcgccgaaagcgcatcgaggctctggggcgtgccgaccctttcgatgagcgccggtgccgccaccacatgcagcggcattttcccgacggttcgcgcaacaaagcgcgcgtcgcgcatcgggccgacgcggatgccgatgtcgatctgctcgtccaccacatcggcatgctgctcggacaggcgcaggtcgagcaccagcccggggtgcgttgccagcagcggagcgagcgcttgcggtatgagccgcgcatacatgtgcggggccgtgacccgcacggtgcccgcgtggcgggacagcgtgcgccggtcgatctggtggaacagctcatcgacgccgcccacggccgcgcgcgcacgctccgccagctgccgcccgaagtcggtgagctgcacgccgcgcgtgctgcggtggaacaagggctcgcccagctcttcttcgagttcgcgcaccgcgcgcgtcaccacctgcggcgagacggacaggcgcgcggcggcttcgcggaagttggcggcagcggcggcggtgcagaacacgcgcagggcttcgagacggttggccacgggggtactttcaagaggaggtgtattccgaaatggggaattctgaagtcgccagagtttcatttacgggaacgtgtggattttccacactgcatgcacttcttgttcttcttcaacacacccgaaaggaattcccatgacatccgttcaagacaacatccgcggcaaggtcgccatcgtcaccggcgcgagcagcgggcttggcgaatcgaccgcgcgccacctggccgcgcgcggcgcaaaggtggtgctcgcggcacgccgcaccgaccggctcgacaaggtggtcgccgaaatccgcgaagccggcggcgaagccatcgccgtcgccaccgacgtggcgaagcgcgccgacctggaaaagctcgcggccgccaccgtcgaagccttcggccgcatcgacgtgctggtcaacaacgcgggcgtgatgccgctgtcgccgctcgagaagctcaaggtcgacgagtgggaccgcaccatcgacgtcaacatcaagggcgtgctctacggcattgccgcggtgctgccgcacatgcaggcgcagggcagcggccacatcgtcaacgtggcgtccatcgcggggctgaaggtgttcacgccgatcggcaccgtctacagcgcaaccaagcacgcggtgcgcgccatctccgaagggctgcgcgttgaaatgggcaacagcggcgtgcgcgtgaccatcgtgtcgcccggcgcggtggattcggagctgaagttcggcagcagcgacgccgagagcgcggccggcgtgaaggcgttctacgaggcgaaccagattccggccgactccgtggcacgcgccgtggtctacgccgtggagcagcctgcgaacgtggacatcaacgaggtggtgctgcggcccgtgtcgcaggaattctgatccgggcgatcggggcagtggcggccccgccccgcatcgattaaccttcaaccgcggaaggacattgacagcaaaaagtgcaaagcccctgcaaaatagaacgaccgttcgttttattcggagcttccacgatgtccgtcaatgccgtttccgccaagccggtccgcgccgcccagaagggccagcagaccaaggccgtcatcgtcgacgcggcgctggcgctggcagcgcagatcggactggagggcctgtcgatcggtgccgtggccgagatcaccaaaatgagcaagtcgggcgtgttcgcccacttcggctcgcgcgaggaactgcagatctccgtggtgcgcgagtatcacgcgcgcttcgagcaagaggtgttctttccggcccttgaggcgccgcgcggcctgccgcggctgcgcgccatgttcgccaattggatgaagcgcacctcagccgaaatcgactcgggatgcatctacatcagcggcgcttccgaattcgacgaccgtcccggcccggtgcgcgatgcgctcgtggagtcggtcagcatctggcaggcggccgttctgcgcgccatcgtgcagtccaagagcgaaggccatctgcgcgccgacgccgacgagcgccagctcgctttcgagatccacgggctgatcctcgcgctgcactacgaagcgcgttttctccaagtgcccggctccatcggccgcgccaacgttggcttcgacaacatcctggcgcgcagcgccacgcccgaagcaccgccggccgaaacggcctccgccaaggccaagccttccgcttcccgccggctcaagccggtgcgctgagcgcccgtttttttcgttcttcccttttctttttttccagttttcgaccaggagagttccggatgcctacctacaacccacccgtacgcgacatgcagttcgtgctgcacgaagtgctcaacgtcgctgatgaactcaaggcgcttccggcccatgccgagaccgatgccgacaccatcaacgcggtgatcgaagaagccggcaaattcgccgccgaagtcacgttcccgctcaacatcagcggcgacgaagagggctgcaagctcgacaagaccacgcatgaagtgaagacccccaagggcttcaaggacgcctacgccaagtacgttgaaggcggctggcccgcgctgtcgtgcgacccggccttcggcggccagggcctgcccttcgtggtgaaccagtgcctgttcgaaatgctcaacagcgcgaaccaggcctggaccatgtaccccggcctctcgcacggcgcgtatgaggcgctggcagcccacggcaccgacgagcagaagaagacctacctgcccaagctcacgagcggcgaatggaccggcaccatgtgcctgaccgaaccccattgcggcaccgacctgggcctcttgcgcaccaaggccgagccgcagcccgacggcagctaccgcatcaccggcagcaagatattcatctcggccggcgagcacgacatgacggacaacatcattcacctggtgctggcccgactgcccgatgcgcccaagggcagcaaaggcatcagcctgttcgtggtgccgaagttcaaggtcaaggccgacggttcgctcggcgagcgcaacccgatcttctgcgccggcctggagcacaagatgggcatccacggcaacgccaccgcgcagatcgtgatcgaaggtgccaccggcacgctggtgggcgagcccaacaagggcctggccgcgatgttcgtgatgatgaacgctgcacgcctgggcgtgggcaaccagtcgctcggcctgaccgaagtggcttatcagaatgcactggcctacgccaaggaccgcacgcagatgcgttcgctctcgggcacgaaagccaaggacaaggaagccgacccgatcatcgtgcaccccgacgtgcgcaagatgctgctcacggccaaggcgtatgccgaaggcggccgcgcgctgcagatcttctgcacgttgctgctcgacaaggaacacaaccaccccgacgagaaggtgcgcaaggactccggcgaactggtcgcgctgctcacgcccatcgtcaaggccttcatcaccgacaacggccacatcgcgaccaattcgtgcatgcaggtgttcggcggccacggcttcatcaaggaatggggcatggagcagttcgtgcgggacaaccgcatcaacatgatctatgaaggcaccaacaccatccagtctctggacctgctgggccgcaaggtgctgggcaacaacggcgcgtcgctcaagaagttcggcaagctggttgccaagctggtggaagaagaaggcgtgaacgagaagatggccgagttcatcaacccgatcgcgggcctgggcgaccagctcaccaagttcacgaccgaaatcggcttcaagggcttccagaaccccgacgaagtgggcgccgccgcggtggactacctgcgcgtggccggccacttcgtgttcggctacctgttcgcccgcatggcccaggtggcgctgcgcgaaattgccgccggcaacaccgacccgttctacgttgccaagctgcagaccgcgcgcttctacttcgccaagctgttccccgagaccgcgacgctgatgcgcaccgcgcgcgccggcagcaaagtgttgatggacaccgaagcggcactggcttgaggcccacgggtctttcctcgacattcaaccgaaagccgctcatgaaagcaacgcttgcagccgtcttgttcaccgtcgccgctgcctcggccatggcgcagagcacgccggtgggcctgtggcgcaacgtcgacgacaagaccggcgaggccaaggccgagatccgcatcggcgaatccaacggcgcgctcatcggccgcatcgagaagtcgctccggagggacgccaagcccgacgcgatctgcgacgaatgcagtgacgaccgcaagggcaagcccatcaccgggctcgacatcatccgcggcggcaaaaaggccgagggcaaggacgtctgggaaggcggaaagatcctcgaccccgagaacggcaaggaataccgcgcgagcttcacgcccatcgacggcggcaagaagctcgaagtgcgcggctacctcggccccttttggcgcacccagacctggctccgcgtccagtagaccgccgcgttttcaatccaagaaataccaatcaacatgtcccgatttcaagtgaagaaggtcgccgtgctcggcgccggcgtgatgggcgcgcagattgccgcccacctcgtcaacgtgcgcgtgcctgtggtgctgttcgacctggcggccaaggacgcgaccggtgcggtcgctcaaggtgccgcgaagaacggcatcgtcacgcgcgccatcgacaacctcaagaagctcaagcccgcgccgctcggcgacgtggccgatgcggtgttgatcgagcaagccaactacgaggacgacctcgccaagctcggcgagtgcgacctcatcatcgaagccattgccgagcgcatggactggaagctcgatctctacaagaagatcgcgccgcacgtttcgaagcactcgatcctggcatccaacacctcgggcctttcgatcaccaagctcagcgaggctctgcccgaagcgctgaagccgcgcttctgcggcattcacttcttcaacccgccgcgctacatgttcctggtggaactgatcaacacgcccaccaccgagccgcaggtgctcgacgacctcgaggccttcgtcaccagcacgctcggcaagggcgtggtgcgcgcgcacgacacgcccaacttcatcgccaaccgcgtcggcatcgccggcatgctggccacgctgaaggaagtcgagaagttcggtttgacgcccgacgtggtggacgacctcaccggcaagaagctcggccgcgccagctcgggcaccttccgcaccgccgacgtggtgggcctcgacaccatggcgcacgtcgtgaagacgctgcaggacaacctcgacgcagaggccgatcccttctacgccaacttctcgacgccgccggtgctcgcgaagctgctcgaactgggcaacctcggccagaagaccaaggcgggcttcttcaagaaggccggccgcgacatcctgcgcttcgacctccagagcggcgagtacgtgcccgccggcgccaaggctgacgaggtgtacggccgcatgctcaagaagccagcgggcgagcgcctgaagctgctgcgcgagagcgaaggaccgcagggccagtttctctgggccattctgcgcgacagcttccactactcggctgtgcatctggagaccattgctgagagcgcgcgcgacatcgactatgcgatgcgctggggcttcggcatgaagcagggtccgttcgagctctggcaggaggccggctgggcgcaggtcgccaggtgggtgcaggaagacatcgacgccggcaaggcgctgagcagcgcgccgctgccgaagtgggtgttcgaaggccctgtggccgaagcgggtggtgtacacacgcccgaaggctcgtggagcgcatcgcagaacaagttcgtaccgcagcgcaagctgccggtgcatgaccgccagctgttccccgaaagcgtgctgggcgcgaacgcggccgatgccaacatggcgggcatcacgatcagcgatgaaggcgatgtgcgcgtgtggacgctcgacggtgaagtgctcatcgcgagcatccattcgaagatgcacgccatcagccccgacgtggccgaagcgctgggcgccgcggtggacctggccgaagccgaatacaagggactggtgatctggtcgcccgacgagatgttctcggtcggcgccgacctgcaggcgatgctgccggccttcgtggtcgccggcatcggcgcggtcgaaggcgcggaagaagagctgcagaacgtgatgctcaagattcgctatgccagcgtgccggtgatctcggccgtgcgcggcatggcgctgggcggcggctgcgagctggccgttcattcggcccggcgcgtggcggcgatggaaagctatatcggcctggtcgaagtgggcgtgggcctgatccccggcgcgggcggcctgacctacatcgcacgccgtgcggccgagaacgccgcggcttccaccggcaccgacctgctgccgttcctcaccgaaggtttcaccgccgcggccatggccaaggtcggcaccggtgcgctcgattcgaagaagctgggctacctgctcgatagcgacgtgatcgtgccgaacaaggacgagctgctctatgtggcgctgcaacaggccaaggccatggccgacgccggctaccgcgcaccgctgcgccgcagcttccgcgtggcgggccgcagcggcgccgcgaccatcaaggggcaactcgtcaacatgcgcgacggcggcttcatcagcgcgcacgacttccacatcgcgagtctgatcgccaatgtggtgacgggcggcgacgtggacgcgggctcgctcgtgaccgaggaatacctgatgacgctggaacgcaaggcgttctgctcgctgatcgtgcatccgaagacacaggagcggatcatggggatgctgagtacggggaagccggtgcggaactgacgcagcaaagaccatgagcgaagacctcggcgcctctggtcccctctcccgcgagcgggagagggctagggtgagggcaagagccttgcgcgaagcccccaccgacgccgagtcccttctctggtaccacctgcgcgaccgccgcctggccaatcacaagttccgccgtcagcgcccgatcggcccgtacttcgcagacttcgcgtgcctcgaagcgaagctgatcgttgaactggacggcgggcaacatgtggaagctgccgagtacgacgagagccggactcgtttcatggaagcgcagggttttcgcgtgctccggttctggaacaacgaagtgctggcgcagacggatgcagttcgagaacggattctgcaagcgctgcaggcagacaaccctcaccccagccctctcccgcaagcgggagagggagcaagacagccaaccatcgtcgcatcggacgaatgagcaagacaagatacaaggactgaaggtcatgaaacaaatccaagacgcctacatcgtctccgccacccgcacgcccatcggcaagtcgcaccgcggctacttccgcaactaccgccccgacgacctgctcgcgaccacgctcaaggctgcgcttgccgcggtgccgggcctcgaccccaaggctatcgaagacatcatctgcggctgcgcgattcccgaatcccagcagggcctgaacgttgcgcgcatcggcgcggtgctggcgggcttgcccacgagcatcggcggcatcaccgtgaaccgattctgcgcatcgggcctgtcggccgtgcagatggcggcggaccgcatccgcgtcggtgaggccgacgtgatgatcgcggccggtgtcgaaagcatgagcatggtgccgatgatgggcaacgcgccctcgctgtcgccctcgatcttcgagcgcgaaggcgacgtgggcattgcctacggcatgggcctcacggccgagaaggtcgcgcagcagtggaaggtgagccgcgaggcgcaggacgagttcgcgctcgcctcgcaccagaaggcactggccgcgcagaaggccggcaagttcacggacgagatcacgcccatcgaagtgaccgaccgcacgccgaacctggagaccggcgagtcgatcgcgaagacgcgcacggtgagtctcgacgaaggcgcacgccccgacaccagcctcgaaggcctggccaagctgcgcaccgtgtttgccgcgcgcggcaccgtcacggcgggcaacagctcgcagacctccgacggcgcgggcgcactcatcctcgcgagcgagaaggcggtcaagcagtacggcctcacgccgctcgcacgcttcgtgagctttgcgagcaagggcgtgccgccgcacatcatgggcatcggcccgatcgaggcgattccggctgcgctgcgctatgcggggctcaagcacgaggacatcgactggttcgagctcaacgaagcctttgctgcgcaatcgctcgcagtcatcaacacgctggggctcgatccaagcaaggtcaatcccatgggcggggcgatcgcgctgggccatccgctcggtgcgaccggcgccattcgcgcggcgaccgtggtgcatgcgctgcggcgcgaaaacctgaagtacggcatggtcacgatgtgcgtgggcatggggcagggcgcagcaggcattttcgaacgcgtctagcggctactgcgcgggcgatctgcggcgttgcggggcccgtcggaaaatcctcacgaccctgaaggtcgctccggttttccgccacccgcgccttgcatctcatcccgctcgctacgccgcggggcggtgatcgatcacgaagaaagaggcaaacccatgcaagcgcaaaaactttcgggcgacggcggcgtgcaactggcggtgcgccgctacgagccggctggcgaaccccgtgccagcatcgtcatcggcggtgccatgggtgtgcggcagtccttttacgagccctttgcgcagtggctcgcgcagcaggggctgcaggtgtggaccttcgactaccgcggcagcggcgattcgcgcagcggcgcctcgctgcgcggcttcgaggccgacctgttcgactgggcgcgcgactacgaggcggtcatcgacaccgccaaggccgcgctgcccgggcagccgctctatcttctcggccacagcctcggcgcgcagctgccgggcttcctgcagcggccggagcaggtcgacggcctcgtcagcatcgccgcgggcagcggctattggcgcgagaacgcgccgaagctcaagcgcagcatcctctacttctggttcgtgctggtgccgctcgtcacgcggctgtgcggctacttcccgggccgcaagctcaagaaggtcggcgacctgccgcgcggcgtgatcctgcagtggcggcgctggtgcctccatccgcgctacagcgtcggcgccgaaggcgagcgcgcgttgcagagctatgggcgcgtgcgctttccggtgctcgcgctgtcgatcaccgatgacgagctcatgacgctcgcgggcaccgagagcctcgtgagcttctacgcgggcgcgccgagcgtgatcgagcgcatcgcgccggccgacgtgcaggcgcggcgcatcggccacttcggtttctttcgcgagcagttcagccagagcctctggccgagcatgctcgacaagctgcaccggctggctgcgcttaccgcggtgcagcaagccagcgtcccgcacacgactgcgtgacgccattcaccggaggcacactgcagccatgagcacgcaccccttcgacaaagccatcgcgctgcagcacagcgacatccgcgtcggccatttcaccggcgccaccagtccggactactggaacatggtcgggcccttcggcggcgccactgcggccattgcgctgcagtcggtgctgcggcatccggacctgctgggtacgcccattgcgctgaccgtcaacttcgcggccgcgctcgaagccggcgcgttcgacgtgcaggccacggccgtgcgcaccaaccgttcgacccagcactggaccgtgcagatcacgcaggctggcgccggcggcgtgccgaacatgacgaccaccgccacggtggtcaccgccgcgcggcgcgacacctggggcgcaagcgacatgccgatgcccgaggcgcccagccctgagtcagtcgaacgcctcagcatcggaccttcgggcgtggcctggctcgaccggtacgagatgcgtccgttcagcggcggcattcctgccaaatgggacgagagcctgcatcacagcgaaacccggatgtggctgcgcgaagcgcaagagcggccgctcgacttctgctcgctggcggcgatgagcgacgtgttctatccgcgcgtctggctgcgccgcgcaacgcgcgtaccggcgggcacggtctcgatcaccacctacttccatgccggaccggcgcaattggccgaggccggcacgggctacctgctgggccgggcggcggggcagcagttcttcaacggcttcttcgaccaggcggcgcatctgtggagcgagaagggcacgttgctcgcgacttccaatcagatcgtctactacaaggaatagcgagaacgaccatgcaaaagaccgcactcatcgtcggcgccggcgacgccaccggcggcgcaatcgcacgccgcttcgcgcgcgaagggttcgccgcgtgcgtcacgcgccgcagcctggacaagctgcagccgctggtcgcgcagatcgaggccgacggcggccgcgcccatgcctttgcctgcgacgcgcgcaaggaagaagaagtggtcgcgctggtcgagcagatcgaatcgaccatcgggccgatcgaggtgatggtgttcaacattggcgcaaacgtgcccgagagcatcctcaccgagtccgcgcgcaagtacttcaaggtgtgggagatggcctgcttctcgggctttctcaatgggcgcgaagtggccaagcgcatggtggcgcgcgaactcccgaagggcgggcatcgcggcacgatcatcttcaccggcgccacggcatcgctgcgcggcgcggccaatttcggcgccttctccggcgcgaaaatggcacttcgcgcattggcgcagtcgatggcgcgcgagctggggccgcagggcatccacgtcgcgcacgtggtggtcgacggcgccatcgacaccgagttcatccgcagcaattttcccgagcgctatgcactgaaggagagcgacggcatcctgaaccccgagcacattgccgacagctactggatgctgcattcgcagccgcgcgatgcctggacgcacgagcttgacctgcgtccctggtccgagaagttctgagatgccgctcgttgccttgtgcgcaataaggagacacccatgacccaatccgtcgacttctatttcgacttcggcagccccgccgcctacctggccgccacgcagctgccgcacgtgtgcgccgacaccggcgcccgactggtctggaagcccatgctgctcggcggcgtgtttcaggccacgggaaaccgttcgccggcggagatcgtgcccaaggcgccgtacatgaccatcgacctgcagcgctttgccaaacgctacggcgtgcccttcgtgcacaacccgcatttccccatcaacacgctgctgctgatgcgcggcgccaccggcatccagatgaaggagccggcgcgcttcggcgcttacgtcgacgccatcttcgatgcgatgtgggtcgagccgaagaacatgaacgaccccgccaccgtcggcgccgtgctccagaatgcgggcttcgacgccactgccctgctggcgttggccgcctcgcaggaagtgaaagaccgcctgaaagccgtcacgcaggaggccgtggagcgcggcgtgttcggcgcgcccaccatgttcgtcggcgaccagatgttctggggccaggaccgcctggatttcgtgcgcgaagccctcgacgcctgattgcatcgccatcacccgttttacccaaggaccattcccatgaccgacatcctcgtccacaccgaagccggtgtgatgaccctgaccttcaaccgcctcgacaagaagaactcgatcaccggcaacatgtacgccgagctggccgacgcgctggctgcggccgagagcgatgcggccgtgcgctgcgtgctgatccagggcgatccgacgatcttcagcgcgggcaacgacatcggcgacttcctcaatgcaccgcccgccggccaggattcgccggtgttccgcttcctgcgcggcatcgcgaccttccccaaacccatcgtcgcggccgtctgcggcccggccgtgggcatcggcaccacgatgctgttccattgcgacctggtctacgcgggcgacaacgcggccttctcgatgcctttcgtgaacctgggcctgtgccccgaagcggcgtcgagcctgctggtgccgcagatgctgggctaccaccgcgcggccgaggcactgctgctgggcgagcccttcatggccgaggccgcgctcgaagtgggcctggtcaaccgcatcgtgccgccgaccgaagccaatgccatcgcgcaggtgcaggcccgcaagctcgcggccaagccgctgagcgcgctggtcgaaaccaagcgcctgctgaagaaggcccagatgcccgccgtgctcgagcgcatgggcgaagagggcgcgagcttcggccgcatgctgcgcgaacccgccgcgcgcgaggctttcggcgccttcatggagaaacgcaagccggatttctccaaggtctgatggagtgagggtcactccgcgttggcccgaagacagtggccgcgtacactgtccggcgtgcaagtcttcgagacaagatcgcttgaaacgcccgtccaatcggcgagtgatgctactgaaaaagtagcaatcgaccttgcgcgccggcgtactttgggtgtgcttgcgggcaccttggcggcgccttcgctggccttggcgcgcgtgcgtcccctgcgcatcgggctcatcggctcctggtccggtccttattcgggcggtgggcgccagttcgatgccggcatgtcggtctggctcgcggcccacaaccagaccatcgccgggaggccggtcgaattgctgcgccgcgacgtgccgggcagcgcgcccgagcaggcgcgccgccatgcgcaagacctggtcgagagcgaacgggtcgacctgctggcgggcctggacttcagttccaacgcctatgccgtcggcgccgtggccacgcaggccaaggtgcccctgctggtgatgaatgcggcctcttcgggcctcacggcgcgctgcccgtttgcggtgcgggtgtcgttcaccatcgcccaggttacgctgccgctggcgagctgggcgctccagcagggcctgcgcaacgtctgcaccgtggtggccgactacgcctcgggcttcgatgccgaaagcacctttgtcgcgggcatcaccgccggcggcggccaggtcggcgcgatgctccgcgtgccgctcaatacgctcgactattcggcctacatgctgcgcctgcgcgaactcaagccgcaggcggtgttcttcttcctgccttcggggcagatgcccaccacctttctcaagttctggcgcgaccgcggcatggccgacaccggcatccgcctgctcgcgaccggggacgccaccgacgaccactacctcgaaggcatcggcgagctggccgacgggctggtcaccagccatcactattcgtcagcccacgaatccgcggccaaccgccgcttcaccggcaccttcgaggccgagtacggcagccacctgcggcccggctatttcgccgtggcggcccacgatgcgctcgccgccgccgacgccgcgatgagttcgccggccgcgcgcggcggcatcggcggcgaacggctggtggatgctttccgggggctgcggctcgagagcccgcgcggcccgatcgaaatcgacgcccacacccgggacatcgtgcaggccgtctacatccgccgcaccgaacggcgcgacgggcgctggatcaaccgcgagttcgagcgcttcgagcgcgtgcacgacccgggcctctgagcgagcgcgctcagggctgctgttcgatgggcctggggcggccgttgtcgtcgatggccacgtaggtgaaggtggcctgcgtcaccttgatgtactcaccctgggccaggaaacgctcggcaaaaacctcgaccgtgaccgtgaccgaggtgcgcccgacacgcaccagcttcgaatagaacgaaagaatgtcgccgaggcgcactggctgcttgaagatgaattcgttcaccgccaccgtggcctggcgccccttggcatagcgggcgggaatgaccgagccggccaggtcgcactgagccatgacccagccgccgaagatgtcgccattggcgttgcagtcggccggcatcggaatgaccttgagcaccagctccatgtcggtgggcaggctcttgagggcggcggcggcgctggaaatatcggacatgggcacaatctggaacaaacaaagcaaccacgattgtcccccatgcgccgcagcggcgaagccctacctcctccttcccatcccgtcgccggccacgcgccggcgcgcagcgaccgctccgactgggcgacgctgcgccgcctctttccctatctgtggcaatacaagtggcgggtgatcgccgcgctcggcttcatggtgggcgccaaggtggccaacgtgggcgtgccggtgctgctcaagaacctcatcgacacgatgacgcccaagccggacatggcccaggcgctcttgatcgtacccatcgggctcttgctggcctacggcctgctgcggttttcgactgcgctcttcggcgaattgcgcgagctgatcttcgccaaggccaccgagggcacggcacggcagattgcgctggaggtgttcggccatctgcactcgctgagcctgcgcttccacctggagcgccagaccggcggcatgacgcgcgacatcgagcgcggcacgcgcggcgtgcactcgctcatttcgatgtcgctctacagcatcgtgccgaccatcatcgagctggcgctggtgctcaccatcctgggcgtgaagttcgactcgctgttcgtctggatcacgggtgcggcgctggtgctgtacatcaccttcacggtgacggtgaccgagtggcgcacccagttccgcaagaccatgaacgagctcgactcgatggcccagagccgcgcggtcgattcgctcttgaactacgaaaccgtcaagtacttcaacaacgaggagttcgaggcgaagcgctacgacgccagcctggaccgctaccgcaaggcggccatcaagagccagcgtacgctgagcatgctcaacgccgggcagcagctgatcatcgcggtcagcctggtgctgatgctgtggcgcgccacctcgggcgtggtcgaagggcgcatgacgctcggcgacctggtgatggtcaacgccttcatgatccagctctacattccgctcaattttctgggcgtgatctaccgcgagatcaagcagagcctgaccgacctggataagatgttcgtgctgatggagaaggagcgcgaggtgcgcgatgcgccgggcgcgcagcccttgtccttgcaccctctccctccgggagagcgcaacggcgtcgactccaccgtgcgcttcgaagacgtcagctttgcctacgagcccgcgcgccccatcctcaagcacgtgagtttcgaaattcccgcgggcaagacggtggccgtggtcggcccttcgggctcgggcaagtccacgctggcgcggctgctgtatcgcttctacgacgtgcagcagggccgcatcaccatcggcggcgaagacatccgcgaagtgcagcaatcgagcgtgcggcgcgccatcggcatcgtgccgcaggacacggtgctgttcaacgacacggtcgaatacaacattgcctacggccgccccgggtccacccgcgaagaggtggaaaacgccgcgcgtgcggcgcgcatccacgacttcatctcggccacgcccaagggctatgaaaccaccgtgggcgagcgcggcctcaagctgtcgggcggagagaagcagcgcgtggccattgcgcgcacgctgctcaagaacccgccgatcgtgatcttcgacgaggccacctcggcgctcgattcggccaacgagcgcgccattcaatcggagctcaggagcgcggcgcaggacaagaccacgctggtgatcgcgcaccgcctgtcgacggtggtcgatgcgcacgagatcctggtgctcgaggcgggcgtgatcgtcgagcgcggcacgcatgccgagctgctcgccaggcagggccggtatgcgcagatgtgggctttgcagaagagcgaagcggtaccgatgctgtagcccgatcattcgttcctttgttttttaccgatccaggagttcagacgtgtcgaccaagattcccctgctggtgctcaacagcctttcgagcgcccaccaggcacagattgccgaggtctacgacatgacctatgccttcgacgccgccgcgcgcgccgccgccatcgcggagcacggcaagaaatttcgtgcggtgctgaccatcggcgtgatcggcatcacgcccgaagagatcgcggccatgccggcgctcgagctgatctgctgcatgggcgcgggctacgagggcattccgctcgaagtgacgcgtgcacgcggcatcgtcacggccaatggcgccggcaccaatgacgactgcgtggccgaccacgccttcggcatgctgatcagcatcgttcgcggctttcgccagctcgaccggctgtgccgcgaaggcgtgtggcgcgaagaaattccgcagccgccgaacgtgtcgggcaagaagctcggcatcctcgggctcggcaccatcggccagaagatcgccaggcgcgcggctgcgttcgacatggagatcggctatcacaaccgcaagccgcgcgaaggcgcaacgcaccgctacttcggcgacctgaagtcgcttgccgcctgggccgacttcctggtgctggccgcgcccggcggtccggccacgcgccacctcgtcaatgccgaagtgctcgacgcgctcgggccgcagggctttctggtcagcatcgggcgcggcagcgtggtcgataccgaggcgctggccgctgcgctgcgccagaaccgcatcgcaggcgcgggcctcgacgtgtacgaaagcgagcccaagcggcccgagccgctggtcggcctggacaacgtgctgctgacgccgcacatggcgggctggtcgccggaggccacgcaggcatcggtgaaccgcttcctcgcgaatgccgatgggcactttgcggggcgcggggtcatttcccccatctgaggtcttgctccttccccctctgggggaaggctgggatgggggcgggcagggcgcccgatggatgcgccgcttgcccccaccccagccctcccccggaaggggagggagtgatcaagccagggccggagggcgatgagacgcccagccgcacgcctggtcatacgcatgcccgagccgcagcacgtcgagatccgcatggatcggccccgcgagctgcagccccatcggcaagccaccctcgccgaaacccgcgcgcacgttcagcgtcggcaaccctgccagcgtgaaaggcgtgacgatctccatccaccggtgataggtgtcgcttggcacgccggccacttcggcgggccagtgcagttcggcatcgaacgggaacacctgcgccgttggcgccagcacgaaatcgaagcgctcgaagagcttgaggaacgcgcggtacacgttcgatcgatagagcgaggcctggtacagcgaggccgcatcgagatgccggctctgctcgatttcccattgcgcctcgggcttgagctgtgcaaacagcttcgggtcgctcaggtaggcgccgagcttgccgccgaccagcaattgccgcagccgcagccaggcgctccagttgtgctcgcgcggcacgtcgagcgtgcagggctcgacctcgcagccgagggtgcggaaggcgcccagcgcgcgttcacccagttcgcggatgccgggcgcgagcggcagctcgggccagatgctgccgagccagccgatgcgcaggccctgcgcgtcggcatcgagctgcagcgcatcgggcgagggcagcggctgcggcgacgacagcggcacgcgcgcgtcgaagcccgcttgcaccgccagcagccgcgcggtgtcttccaccgtccggcccatcggcccttcggtgcccagctgctgaaagaagagctcctgttcgggatcgcccggcacgcgtccgcgcgagggccgcatgccgatgacgttgttgaatgcggccgggttgcgcagcgagcccatcatgtcgctgccgtcggccaccggcagcatgcccagggccagcgccacggcagcgccgccgctgctgccgccggcgctgcgctcgggcgcataggcgttgcgggtgatgccgaacaccgtgttgtaggtgtgcgaaccgaggccgaattcgggcgtgttggtcttgccgatcacgatggcgccggcctcgcgcatgcgcgcgacgtgcaggctgtcggcccgtgccggggagcgcggcgaaagcggcgagcccatggaggtcggcaggccggccgcgtggctcaggtccttcaccgccaggggaaaaccatgcatccagccgcgccgttcgccgcgcgccagctcggcgtcgcgttcgcctgcttcggccagcagcgcctcgggttcgcacagcgaaacaatggcgttgaagcgcgggttgagcgcctcgatgcgggccagcgaggcctgcatcagctcaaggcaggacacgctgcgggccgcgatgcggcgggaaagttcggtagcgctgaggtcgagcagatcggctggagccatggcgaatgcgggaaaaggagggggagcccagtatggcgcgacgctcgcataatcgccgcgtatggaaacaaagtggctagaagacttcatcagcctggcggaaacgcgcagcttcagccgctcggcccaattgaggcacgtgacgcagcccgcgttctcccgccgcatccaggcgctcgagggctgggccggcaccgacctggtcgaccgcagttcctaccccacgcgcctcacccccgcgggccagacgctctacagccaggcaatcgagatgctgcaatcgctgcagagcacccgcgccatgctgcgcggccattcggcggccgggcaggacgtgatcgagatcgcggtgccccacaccctggccttcactttcttcccttcctgggtgaccagcctgcgcgagcatttcggtcccatcaagagccggctcatcgcgctcaacgtgcacgacgccgtgctgcgcctggtggaaggcagctgcgacctgctgattgcctaccaccacccctcgcagccgctgcagctcgacgccaacaagtacgagatggtcagcctgggcgaggaaaccgtggcgccctgggtcaaggccgatgccgacggcgcgccgcgcttccgcctgcccggccggccgggccagccgctgccttacctgggctacgcgcccggcgcctacctgggccgcgtggtcgaccagctgctgaaggagtcgggcaccgccatccacctcgaccgggtctatgaaaccgacatggccgagggcctgaaggtcatggcgctcgaaggccatggcatcgcctttctgccgcaaagcgcggtacgcaaggagatcaagtcgcgcaagctcgtgagcgcgctgccgcccgaaatcgacagcctcgaggcgacgatggagatccgcgcctaccgcgagcgacccggcgcgccggcgcccgtgaagaccggtggcggccgctccgcgaaggcttcgccctccgacagcctgcagcccaagcgcacggccgacgcgctgtggtcgtatctggtcggcgcccagccgccgcgctgacgtcgatcgattgacgggctggatttgtgcgctgcacaatctataaatgccgcgcatggcaccccccgcaaacggcattggcgttgcgggcgtgtcgcccctacagtcgcggcagtttttgccgctgtcacacagcaatcttccggcacgcgccacacgcgtgcttttttttagccgaggaatctgtatgagccccaatttcaggaccgaacacgactttctcggcgagaagcagattcctgcccttgcctactggggcgtgcacacggcgcgcgccgtcgagaacttcgccatttccgggacccgcgtctcggccatgcccgagctggtgcgcgcgctggccttcgtcaaaaaggcggccacgcgcgccaatgccgacctcggcgccatcgaccgcgaccgcgccgccgcgatcatcctggcctgcgaggacctcatcgacggcaagctgctggacgaattcgtggtcgacgtgatccagggcggcgcgggcacatcgaccaacatgaacgccaacgaggtgatctgcaacctcgcgttggagaagctcggccacgaaaaaggccgctacgacgtgctgcaccccaacgaccacgtgaatgcctcgcagagcaccaacgacgtctacccgacggcggtgcggctggcgctgtggtttgccattggccggctgctcgaatccatggccgcgctgcgcaagagcttcgaggccaaggcgctcgagttcaaggacatcctcaagatcggccgcacccagctgcaggacgccgtgcccatgacgctgggccaggagtttctgacctacgccatcatgatcggcgaggacgaggccaggctcggcgaggcgcgcgcgctcatcgaggaaatcaatctcggcgccaccgccatcggcaccggcatcaacgcgccgcatggctacgccaacctcgcctgccagtacctggccgagcagaccggcgtgccgctcaagcagtcggccaacctcatcgaggccacgcaggacactggcgcgttcgtgcagctgtcgggcgtgctcaagcgcgtggcgtgcaaactgagcaagacctgcaacgacctgcgcctgctgtcgagcgggccgcaggcgggcttcggcgaaatccgcctgccggcgcgccaggccggctcgtcgatcatgcccggcaaggtaaacccggtgatccccgaagtgatgaaccaggtggctttcgaggtcatcggcaacgacatcacggtcaccatggcgtcggaggccggccagctgcagctcaatgccttcgagccgatcatggggtggagcctgttcaagagcatccagcacctgggcaacgcctgcaccacgctgcggcagaactgcgtcgacggcatcgaggcgaaccgcgagttcctggccaagcgggtgcgggagtcggtcacgctggtcaccgcgctcaatccgctgatcggctatgaaaaggcggcgctgattgccaaaaccgcgctggccaccggcgggcccatcgacctggtggccgaatcgctcggcatcatgacgcgcgccgagatggaggcgctgctcgtgcccgaaaacctgacccagcccgtgcgcctgtccgcgccggtgccgccggctgccgagccctcgggcacaaaggctgcttagtgaaagtcggacaatgccaaagggttcacctgcaccaccacagcgcttcgatgcgcgcggccggtgcggtcgtcatcgagaatgcaccgggttggcccgggtattccccatgacgtgaatgtctagaatttcgttgtatctgtatctcatagtcaccctcaggagttttccatatgaacaagcaagtattggcattggcaatcgcggcactggccgcaggcagcgcctttgcacaggccactgacaccctggccaagatcaaggcctcgggcagcatcaccgagggtgtgcgcgagtcctccggtctttcgtacacgctgggcaacggccagtacaccggtttccactacgacgtctgcgccaacatcatccgcgacatccagaagcacctgggcctcgccaagatggaaaccaagttccagcccgtgacctcgcaaaaccgcgtgccgctggtgcagaacggcacggtcgacctcgagtgcggctccaccaccaacaacgccacgcgccagaaggacgtctccttcgcagtgaccacctacgtcgaggaagtgcgtatcgcggtcaaggccaattcgggcatcacctcgatcaaggacctcaacggcaagaccgtggccacgaccaccggcaccacgtcggtccagaccctgcgcaagaacgagcgcgccggcggcatcgacttcaaggagctctatggcaaggaccactccgacagcttcctgctgctcgaatcgggccgcgccgacgccttcgtgatggacggttccatcctggcttcgaacatcgccaagtcgaagtcgcctgccgactacaagatcgtcggcgaagtgctcagcgtcgagcccatcgccatcatgatccgcaaggacgaccccgccttcaagaaggtggtggacgacagcatcaagtcgcagatcaagaacggcgacctcgccaagctctgggacaagtggttcctgaagccgattcccccggccaacgtcacggtgaacctgccgctgtccgacgccaccaagtcggcctgggccaacccgaacgacaagccgatggaagaatacgccgccaagaagtaaacacggcaaggtcatccgcgcaacgcccgccgcccccggcgggcgtttgttttcgcaaatgcggcgcgcgggcacggcctctgcaagctagcagtctggaaatctgaaagaaggagagtccccgatgggatcaaactgggattggcaggtcttcttgcaagacccgggcgggaagtacccgacctactgggagtggatgctgtccgcatggggctggaccgtgtcggtcgccctgctggcgctcgtcgtcgcgctggtgctgggttcgctcgtcggcatcatccgcaccttgcccaacagcccgtggctggtgcgtttcggcaatgcctgggtcgagctgttccgcaacatccccctgctggtgcagatcttcctctggtaccacgtcatcccggcgatggtgccggtcatgaagggcgtgccgagcttcgtgctggtggtgctggcattgggcttcttcacctcggcgcgtattgccgagcaggtgcgctcgggcatccaggcgctgcccaagggccagcgctatgcgggcatggcggtgggcttcaccacgccgcagtactaccgctacgtgatcttgccaatggcctaccgcatcatcattccgccgctcaccagcgaaacgatgaacatcttcaagaactcgtcggtggcgtttgccgtgtcggtgaccgaactcacgatgttcgccatgcaggcgcaggaagaaacctcgcgcggcatcgaggtgtacctggcggtgacgggcctctacgtgatctcggcctttacgatcaatcgcctgatggctttcgtcgagaagaagacgcgcgtgccgggcttcatcgtctcggccagcggcggcgggggacactgacatgatgaatctcgacctgtcgttctataactgggacgtcatcagcaacttcgtcgtcaagggcttctacttcagcatcatgctgacgatcgtcgccaccattggcggcgtgctcttcggcaccgtgctggcgctcatgcgcctgtcgggcaagaaatggctcgacgcgccggccgccatctacgtcaacggcatgcgcagcattccgctggtgatggtgatcctgtggttcttcctcctggtcccggcttcgttctacgcggccttcggctccatcggctcgaactaccgctccgagatctcggccgtgatcaccttcatcgcgttcgaggcggcctacttcagcgagatcatgcgcgcgggcatccagtcgatcccgcgcggccaggtgcatgcgggccaggcggtcggcatgacctacgggcagaacatgcgcctggtggtgctgccgcaggccttccgcaacatgctgccggtgctgctcacgcagaccatcatcctgttccaggacacctcgctggtctacgccatcggcgcctacgacatgctcaagggcttcgagaccgcgggcaagaacttcggccgcccgatcgaggcctacctgctcgcggccgtcgtttacttcatcatgtgctatgccttgtcgtggctcgtcaagcgcctccacaagaagattgccatcattcgctaatcgagtggctgaaccggagaaagaaatgtccgaaaaaatgattgaaatcaagaacgtgtccaagtggtacggcccggtgcaggtgctcaacgattgttcggtgagcatctccaagggcgacgtggtggtggtgtgcgggccctcgggctcgggcaagtccaccctcatcaagaccgtgaacgcgctcgaacccttccagaagggcgagatcaccgtcaacggcattccgctgcacgaccccaagaccaacctgcccaagctgcgctccaaggtcggcatggtgtttcagcacttcgagctgttcccgcacctgtcggtcaccgagaacctcacgatcgcgcagatcaaggtgctcggccgcagccccgacgaagccaagacccgcggcctcaagatgctcgaccgcgtgggcctgatggcgcacaaggacaagttcccgggccagctctctggcggccagcagcagcgcgtggccattgcccgcgcgctcagcatggacccgatcgtgatgctgttcgatgaacccacctcggcgctcgaccccgaaatggtcggtgaagtgctcgacgtgatggtgagcctggccaaggacggcatgaccatgatggtggtcacgcacgaaatggcctttgcccgcaaggtggcaagccgcgtgatcttcatcgacgtgggcggcaagatcctggaagactgcccgaaggacgagttcttcagccacccggaaaatcgtcagccgcgcaccaaggatttcttgaacaagattctgcagcactgatcgattcgctgcggcgccaaagcaaaagccacgctgttcgcagcgtggcttttttattaatttgtccggagcttatggcagccgcgcgatgtgctcggtcagcagatcgaagaagccctgcgcatcgccgtccacgatccagttcacattggcagggcgcttcaggctgccgtaccagtcggccaccgtctgcccaaagcccatgccttcgcggctgtcgacttcgacgttgatcagcctgcccctgaagagcgagggctgcagcaggtaggcaatgacggtggcgtcgtgcaccgggccgccgggcatgtcgtagtgccgcatctcctgcggcgcatacgcgtccaggatgtcggcaacgatcctgccagcctggttgccgatggcgcgcagccgcgcgatgcgctcgctgctcgtgaggatcttgtgcgtcacgtcgagcggcagcatggtgatcggcacgccgcacttcagcacggcctcggctgcatgcggatcggcaaacacgttgaactccgcggtgggcgtgatgttgccgccattgaaatgcgcgccggccatgagcaccagttcgcgcaggccgcgcacgatgtcgggggcttgttcaagcgcgagcgccaggttggtctgcgggccgagcatggcaagcgtcacgctcttctccggtgcggcgcgcagcgtgcggaccaggtagtcgaccgcatgaccttcggccagcggcgcggcgggttcatgcaccttcacgcccgtgacgccttcgtggccatggatgttggccgcatagatcggcgtgcgttccaggggccgttccgcgcctgcgtacaccgggatctccggccggccggcccattcgcacgccaagcgcgcgttgcgcgaagtcttcgacagcggcacattgcccgccaccgtcgtcagcgcctcgatgtgcagacgctcgggcgccgccattgcgaacagcagtgcgatcacgtcatcggcgcccggatcggtgtcgatgacgagcgtgtgcacggtggcgtcggcgggtgggttcggcggcatggcaaggctccgtggcgggcgcggacagcgcgcctctgccgggcaagtctgccagagcccgtgcgacggtcagccgggcctgcccagcagccgccgcgcaaagaaagccaggatctcgtcccgcgcagccactgtcggctggcccgcctcgtcgatcagatgcgccgtcaccacgctgtgcgggctggccaccagctgcgcgaagaagggtggcgtgtcggggttcgcggcgctgtcgggcagcacgcgcgcgacgaagcgctcgcccagcgccagcgagaacgccgcgaagcgctcggccttgcagaaccggtcgccctcgaagcggtaggccatcacgctcaggttttcgcgctccaggcgctggcgcaccgccgccagctcgtcggccgccacgttcgtgcccgccggatcgtccagcggcagcgaaggctggcagaccaccggcgcgagcatggccggctccatcatcatcgagagcgcgaagttgccggtgaagcacatgccgatcgcgcccacgcccgggccgccgcacgcttcgtgcgcgaaccgtgcgagcgcgcgcagccattgcgttatcgggctcgacgcgttcgatgcgaaggcccggaactcggcgctcacgcaggcccgcttgaacacggcggcgccttccccggcctggggcaccgcgccgtcgcggccgaacagcgagggcatgtagaccgtgaagcccgcgtcgcgcacccagcgggcgaagcgcgccacatgcgggctgatgccgggcatctcggtcatcacgaccacggcaggaccccggccggccgtgtagaccttcttctcgatgccgtcgagcgtgatctggcgcggggtgaagtcgtcgagcggatcgtcttctttcatggagcgggtcggtgtcatggggcgccgccgcgtgcggcggccgtgaagcggttgaagcttgcattgggccgccggcctccagagaatgacagtgtcgaatttgactgttttcaggctgtatcggacatgaacgacttcacggtgctggtgctgccgggcgccttcaactccagcgtggcggtcacgctcgacatcctgcgcgcagcgcgggcggtggccgcccgagccggcgtggcgccgccgcgctggcggatatgctcggtgcaaggcggcccggtgcggctgcaggccggcatgagcctggacaccgcccgcttgcctgcgcggccccgtgacgaccgctcgacatgggtggtgccggggctcgggctcaacacgcccggcgagattcaccagtgcctcgaaagcgacgatgcggccaaggccatcacgggcctcgcgcggcatgtgaagtccggcgggcaggtcgcggcctcgtgctcggcggtgttcctgctgaacgccgcaggcctgcttcaaggacgccgcgcgacgatctcgtggtggtatgcgccgctgctcgcgcgcatggcgcccggctgcactgtcgatgccgaccgcatggtgtgtgccgacgggccggtggtcacggccggcgccgcgttcgcgcagaccgacctcatgctgcacctgctgcgcgagcgttgcggcagtgccctcaccgacctggtctcgcgcgtgctcctgatcgacgggcggcaggcacaggcgccgttcatcgtgccggaggttctggccaacggcaacgaccttgtggcgcggctcgccgcgcgggtcgcgtcggcgctgccggatgcgcccgcggtgagcgtgctggcgagcgagttctgcatgtcgcagcgcacgctggcgcgccacatccgcaaggccaccggcaagagcacgcaggcgctggtgcagagcgtgcggctgcggcgcgcgcgcgtgctgctcgagaccagccggatgacggtcgaccaggtggccggcgccgtgggttatcaggacgccacggccctcaggcgcctgatgaagaagatggcgggcgccaatccgagccgctaccgcgaaggcggttacggcgcctgacgcgcccgcaatatcggcgtgctgcgctgacttgctacttcttgcgcgccgcgatcgccttctcggccgttgccaccaggtccgcgcccaccgtgttcttccacttgtcgtacaccgggcgcgtggctttcacgaaggcttcgcgctcggcgggcgtgagctgcgtcacggtcacgcccatgccggcgatgtccttcagcaccggcttgtcggcttcgacgaggcccttgcgcgcgagttcgatctcctgcttgccggcatcgacggcggcctggcgcacgatggcctggtcggctggggtccacgaggcccagatttccttgttgaccacgaagaccagcgggtcggcgacgtagccccaggtggtcacgaacttctgtcccacgttctgcatcttgagcacggtgaacaggaagagcggattctcctggccgtcgaccgcgccgctggcgagcgcgggctgtgcgtcggcccagctcatctgcgtggggttggcgccgagggcggtgaacatgtcggaatagatcggcgagccgacgacgcggatcttcatgcccttcaggtcttcgggcgacttgatcggctttttcgagttggtgatttcgcggtagccgttctcgccccaggcgagcggcaccacgccggccttgtcgagggtcttgaacatttccttgccgacttcgccttgggtgagcgcgtcgatggccgcatagtcgggcatcaaaaagggcatggagaacaggttgagctgcttcacttgcggcgaccagttgatggtcgagcccacggccatgtcgatcacgccctggcgcagcgcgctgaactcgcgggtctggtcgccttgaatgagcgacacgccagggtagagcttgatgttgatgcggccctgggtgcgctccttcacgaggtcggcccagatcttcccggcctggccccaaggggtcggcgggccgagcaccagggacatcttgtattcgggcttgtaggcggcctgcgccatggcgccggtcgaaaagaagccgagtgtggtggcaacggcggcaaggccgagcagagtacggcggaatttcatgagaggtctccttgttttctgaacacaactaagcatggatgtttgggggaacggtactgagcggcgctatggggtcgggaacgttcagggcgcgtgcacaggccaccgggtactcccctccgcgaatgtcccccgggcttcgccctcctcctttatttcgctgcggggagtacccggcgccctgcgcacacaaagcgctgctcttgttccgctcgatcaaccaccgctccgaacaacgatcccgtcgatggggtgccttgcgcagcgaaataaaggaggaggccgcaggccgggggacattcgcggagcaaggtaccccgtcggcgggagcgcgccctgaagcgtgaccacacgccgaacgaagcacttcacgaacagcgcagggcgtcatctcaataccccagcttgcgcggcaaccaaagcgcgagctcagggaacgcgatcaccagcaccatcaccacgaacatcgagaacagcatccagcccacccaccgcacggtttcctccatgcgcaccttcgcgatgcggcacgacaccatgaggttgaccgcgagcggcggcgtgaactggccgagcgccaccttgagcgtgaggatcacgccgaaccacaccgggtcccacttgtagtactgcacgatcggcagcaacagcggaacgaagatcaggaagatcgacacaccgtccaggaacatgcccaccgtgatcagcagcaggatcaggagcgccaggatgccgtattcgcccaggcccgaattcacgatggcgcgcgtcaccgggtcgatgatgccgagcgtcgagagcgagtacgcgaagatgcccgcgagcgacaccaccagcaggatcaccgccgagagctcgcccgattcgcgcaatatgacgaacaggtcgcgcaccttgatggtccggtgcacgcacatgcccacgaagagtccgtagaacaccgccaccaccgccgcttcggtcggcgtgaaccagcccgcgcgcatgccacccagaatgagcaccggcgccgccaggccccagatcgcttcgcgaaaactcttccagaacggcgggcgcggcagcgtcgattcgagcgcgcccatcttgtgctggcgggccagcagcacggccggaatcatcagcgccaagccggccatcacgccggggatcatgccggccgcgaacagcgccggtaccgaggcgccgggcaccagcaccgaatacacgatgaacgcgaccgagggtggaatcaggatgtcggtggccgccgcggcgcccaccacgctggccgagaaagccgccgggtagcccgcgcgcgacatggccgcgatcatcaccgcgcccacggccgcggcattggccgggcccgagccggagatgccgccgaggaacatcgccaccgcaatggccaccagcggcagcatgccagggccgcgcccgacgatggccaccgcaaagttcacgagccgcagcgccacgcccgaacggtcgaagatggagcccaccagcacgaacatcggaatggccagcagcggatatttgccgaggccggcatagaagttctgcggcacggccagtaggccgaaccattgggcgtcgctgttggcaagtgcaatgcaggcggcgccggccaggcccagcgcggcgccgatgggcacgcctaccagcatcatcgcgacgaaggcgacgaagagcagggtggcgatcacgatgcgtcgcccttgccggtgcggttttcgttgtcgccgtattccttgcggccgcggcggatcatcaggcccaccgcgcgcagcgcgatggcaaaggacacgatcggcagccacatcgaataccaccaggccggcagcccgatacccggcgtcgtttcgtcgaaacggtagtcgtcccacaccatgcgaatgctgagcgcgccgatcagcgcgaagaggatggcgatcatcagcgcgccgaattgcgcgagccgcttgcggcgtgccatcgatccgttctcggaaaaatactcgatgcggatgtgccggtcgcgcgccactgcggccgagccggccaccagcgccagcatgatcatcaggaaaaccgagaactcctccgtccacgcaaacgaagagtcggtgaagtagcgcaccagcacgttggcaaaggtgatgagcgccagcgcgcccatgatgatgacggtgagccagtcttcgatggcgagcggcaccttggtgggctcgtcggcggcttcgatgtctgggggaagggggctggcggcgtccagcagcgggccggactcgttgggagtggtcatcgagggagaaggggaagcagctatgaatggtaacgatccatgaccatccgttcatcggggttttcctaagctgcggccccgttcctcagttcccttcgacccctcgaggcccttggcgggctactcgagcttggcgcccgagtccttgatcaggcgctcccagaccgggctttccttcttgtacaccgcgttgaaagcctcgggcgagctctccttcaggtcgaagcccatggccgccacgcgcgcctgcacgtcgggctggcgggtggccttgcccacctcgtcggcaatgcgctgcacgatcggcttgggcgtgccggccggcatggcgatggcgagccagccggtcacgcggtaggcctcgtccttcagcccctgctcggccagcgtgggcacgttgggcagcgttgccatgcggcgttcgccgctcacgccgatggctttgagcttgccggcttcgatgtgcggcttggccaccagcgcgctcgcaaaggccatctggatctggccgccgatcaggtcctgcagcatcggcgattcgcccttgtaggcgatgtggttcatctcggccttctgcgtgaggctcatgtgcgcgcccgccaggtgcgggtaggcgcccacgccgtaagagccgtaagccaccttgcccttgttggcgaccacgtacttcagcagttcgggcccggtgttggcgggcacgctcgggtgaaccaccagcaccagcggtgcagtggcaatctgatagaccagcgtgaggtcgcgctgcgtgtcgtagggcagcttctcgtacaggaattggttggtcagaagcgagttgctcagcgacagcacgatggtgtagccgtcggccggcgccttggccacggcatcggtgccgatgattccggcggcgccgggcttgttgtcgatgatgacgggctggcccagcccggccgccatcttctcgcccagcacgcgggccagcacgtcggtcgccccgccaggggcaaagggcaccaccatgcggatcggcttgttcggataggtctgcgcccagctggcgccggcggccgcaagcgcgagcgaggcgatgccgcagtgcagggcgcggcgggtgagcccgcgaggggtgaaagttgcgttcatgtttgcgatgtctccggatgtcgttgtttggttggcgaaggaaacggggcgtggctattccacgagcacccgcgtcttgaatggaagcggctcgagcgccgtgcggatccgctcctccagcaatgcagcgagcgcgcctgcagcccccgcatcgatgcgcacctgcaccaggctctcgccctcgccgcgcacgctcggccgtgcggcttccgccacgccgagctcgtcgcagatttgcgccacgtcagccgccaccacgcggctcgcggccatcgcgcgaagttcgggcttgtagatcttgccgacgttggtcatcggcatgttctcgatgacgatcaccgacttgggtttggccggcgcctcgtcgacgcgcgcggccgtgaaggccagcaattcgtcctcggtggccgatgcgcccggcaccagcgtggcaaagaccaccggcagttcgcccgcatacgcatcgggcgcgcccaccgccgcgcacagctgcaccgcgggatgcgcgcccagcgcgtcctcgatcaccttggggtcgatgttgtggccgctgcggatgatcaggtccttcgagcggccgctgaggttgagccgcccttcgccgtcgatccatcccaggtcgccggtcgcaagccagccatcggcggtgaaggccttggcgttgtcggccggatcgacgaaacccgagaacaggttgggcgactcgaatagcaccatgccctgctcgcccggcggcaggtcgcggtcgctggcgttgccgttctcgtcgagcgccacgatgcgcatccgcatgtagggcagcggaaagccgacgcagcccgcgggcccgtccacgccgggcggcgtgatggtcgagatgcccgccatctcggtcatgcccaggctctcgtgcacgtgcaggccgaacaggcgctcgaagcgcgcggccagttccggcgagagcacggcggcgcccgtgcggcaatagccgatcgatgaaatgtcggcgccattgagcggcacgttcgccagcgcggcaagcaccgtgggcacggccgagagcgaggtcggccggtacttttcgaccagcttccagtagttggcgagcacctccttgttgcgcagcagcgaggtcgtcggaatgatcacctccacaccggccgagagcgacgccagcgaggccggcaacacgcccgccacgtggaacagcggataaccgttgatggagatgccttgctcgttcatgcccgcgacctgcacgctggcccatgcggtgaacacctgcgcaccgtggctgtggcgcgcgagcttcggggcgccggtggtgccgccggtgtggaagtaggcggcgatgtcggtcggtgcgatgtcgcggccgctcacgaggcgatcagacggttgtgccgaacgcagcacgtcgaactcggccacgccgacgggcagcgcgcccgccttgcccggcgcctcgtcgtgcggcgccacgcgcagcacggtcgtgagcgtaggcacctgcccgcgcaaacgcatcgccttcgaccacatgcccgcctcgctgtcggagccgtaggcgatcagcaccttggcgcggccggcggtcatcagcgccaccagcttctcgtcggtcaagagcgggttgagcggctgcacgatgccggccgcctcgccgccccagagcgcgaggtggtactccaggcagcccggcagcagcaccgccaccgcgtcatcggggcccacgcccagggcgtgcagcatgttcgcggtctggtggatgcgcgcgagcagctcggcatacgaccagcggatcggctcgtcggccgggttgccggtgcgcagaaaggtcagcgcagtcttgtttccgaaggccgcacccgcactgcggaagatctcgtaggtgctgcgaaccgtcagcgcctgcgcaagcggcgtctcttcgagcttgcggatgtctgccaggctgcgaaccggcaacagggggcggaacggtgccccgcccggacttgtcttcttgtcgttgcctgtcatgtcgtctcctgatgttgtctctggccggccgcgcgcgaatcgctgttttactggttcgtgatgttgttgtcgcgaatgaccttgccccagcgttcgaagtcctggcgcatgcgcacgccggtctgctcgggcgtgcgataggccgcgaaggagccgacgctttcgagcttgtcctgcacctccttgtcggccagcgcggacttcagctcgacgctcatgcggtcgaccacgtccttgggtgtgccggtcggtgccagcagcccgccccatgaggtcgcatcgaagccgggaaagccctgctcggcgacagtcttcacctcgggcagcaggttcacgcgcttgcccgagccgaccgcaatggcccgcagcgtgccggcgcggatgtgcggcatcaccgccacgaggtccgaaaacatcgcaggcacctgcccgccgatcaggtcggtcaccgccggcgcgctgccgcggtagggcacgtgctgcatctcgaacttgccgatgttcttgagctgctcggtcgtcaggtggccgaagctgccggcgcccgcggtcgtgtagttgagcttgccgccctcggccttggccttggcgatcaggccctgcaggccggtcacttcgggcagcgacttgggattgaccaccatgacgatcggcaggtcgtacacggtgcccacgggcgtgaagctcttgaagatgtcgtagggcgcctggccgtacaggtgcgcggccagcagcgtgggcgtggccagcatcacgaaggtgtagccgtcgggcgccgccttggcggccaccgcggcgccgatggtgcctgaggcgccgctgcggttgtcgatcagcacgttctgcttcaggccctgcgacatcttctgcgccacgatgcgcgtggcgacgtcggtcggaccgccgggcggaaagggcacgatgacggtgatcggcttggtcggccaggcctgcgcgaacgctgcgccggccaccagaggaagggccagagcgatgagcgcacggcgtgcgggattgcgaagggaacgaaaagaagaaggaaatgccatggacttgttcaagggatcggaagaagaggggcgtcttcagacgacgccgttcgctttcagttgcgcaagcctgtcgtcggagaggccgagcagagactgcagcacctcgtgcgtgccttcgcccagttgcggcggcgcgctgcgcacgggcaggcgttcgccgtcgaagcgataggggggagccagcacgtcgaccttgcccgccaccggatgcggctgctcggtgacaaggccggcatcggtggcacgcttggagttgagcgcttcgagcaggccgagcacctcgccgcagggaatgcccgatttcgtgagcttcgcgagcaggtcgacacgttggcgcctggccagttcggcgtgcagctcgggcagcagcaccgcacggttcgccgaacgcaggatgttggtcttgaagcgctcgtcggcggcgaggtcgggccgttcgatcacttcggtgcagaagcgcgcgaactgcgcgttattgcccacggtgatcaccagcgggccgtcggccgcatcgaacacgccatacggcacgatcgacggatgcgagttgccgtagcgcggcgggtcttcgcccatcagcagcgcctccagcccgtagtaggcggtgatcatcaggccgcagtcgaacagcgccatctccacgtgacggcccttgccggtcttctcgcgctggtagagcgcggcgaggatggcctgcgccgaatacatgccggtgaacaggtcgaccatggccacgccgaacttcagcggcggctggttggcttcgccgttgagcgccatcaggccggcttcgccctgcaccacgaggtcgtagccgggccgtgcggcctcggggccggtgcggtcgtagcccgagatcgagcagtagatgagccccggctgcgccttgctgagttgctcgtagccgagcccgagcttgtcgatgccgccgaatttgaagttctggatcaccacgtcgcattgcttcgcaaggtcgcgcgcgatctgctggccttcgggcgtctgcaggtcgagcgtgaccgagcgcttgttgcggttcacgctgttgaagtaggcagtctcggtcttgccgacgcgcaggccccagtcgcgcgtgtcgtcgccgcggcccgggtgctcgaccttgatcacttcggcgcccatgtcggccagcaccatgccgcaccaggggcccgccaggatgcgggacagatcgagaacgcgcacgccggcgagcggcagcgatgaattgagcatgggcatgagggcaactccctgaaaacgagaaagccccgcagcgtgtgcgaggcgtgaagtcgggtggatcggggcggcggcgtcaggacgacgggttgggcttctggcggcgcagcgcggagaaatccgccgtgcgcttgccgagaaaagcgccgatgccttcggccgcttcggcatccgcttgcgactcgaccatgtacacggcctcggcttcgagctgctcttcgagcgtggcgcggtgggcctggcggcacagcgtcttgatgcgtgcgcttgcgcgctgcgggccattggctaccttggccgcgagcgcaatggcctcggccagtgcggcgcccttgtcggtcaaccggttgaccgcgcccaatgcatgcaggcgctcggccggcatgcggtcgccggtcaggcacatctcggtcagcacctggcgcgagacgaactccgagaggaaggccgtcgcgccgccgtcgggcgtgaggccgaccttgacgtaggcgaccgtgtagaacgcatcgcgcgccgacaccagcatgtcgcaggccagcgccatcgaaaggcccgcgccggccgcgccgccttcgaccgccgcgatgacgggcttgccgcaatcgcggatcgcacggatcaggtcgtgcaggccttcgagcttttcgcggcgctccgaggcgggcagctcgcggcgcttggccagcaggttcaggtcgccgccggagcagaagaaatcgcccgcgccggtgaagacgatggcgccgacttccgggtcgttctccgcatcggtgagcgcggcgctcagttccgcgtacagcgtcggcgtgatcgcattgcgcgcgtcggggttgctgttggtcaggatgcggacggcgccttgctggctgatgagaacggtcttttccgtcatgctgccagctccttgcccagcgcaatgtagcgctgcaggtggtggtcttcatcgccgagctggtggtcgatcatcacgagccgcttggcgtagtgcggcagcggcagctcccacgtcataccgatgccgccgtgcatctggatgctttcttctgccaccagcgcgccgatgcgcccgatgctgaacttggcggccgacagcgcgcgctcgcgcgccacgcggtcggtgccgtcgatggcggccgcggcattgatcacggccgaacgggcctgttcgatctcgagcagcagatccgccatgcggtgctgcagcgcctggaaactgccgatcaggatgccgaactgcttgcgtgtgcgcaggtagtcgagcgtcgcggtcttggcggcttccatcgcgcccacggcttcggcgcacagcgcgagcacgccgcggccgatggcgcgttccagcgtcgcactgccctggccttcggtgccgagcagcgcgtcggcgcccagcgtcacgccgtcgagcgtgagttcggcaacgcggcctccgtcgatggcggggcagccgcgcaccgtgaggcctgccgtcttcgcgggcacgaggaacagcgagatgccggcttcgtcgtcgacgttgccggaagtgcgggcggagaccaggaacaggtcggcctgctcgccctgcggaacgacagccttggcaccgttcagcgcccagccatcgccgctgtgctcggcgcgggtcgccacgcgcgtgcgttcgtagtgcgtgtcggcttcgtcgtgcgcaaaggccgcgacggtgaggccgttgatgatgtcgccgagcttctccttctgcgcatcgctgccggcggcgctgagcgcctcgccgaccatcaccgcgcccagcagcggctcgaccacgaggcctcggcccagcgcctcgaagacgacggcgatgtcgaagccgccgccaccgaagccgccgtcggcttcgctgaacagcgcgccgatcacgcccagttcggcgaactgctggaagatctccttgctgaagccgtgctcggacttcgcgatgcggtcgcgcgcatcgaaggcgtactgctcggcgatgaagcggttcaggctgtcggcgagcatgcgccggtcttcggtgtgttcgaagttcatgtgcgtgtctcctttacagcccgaggatcatcttggagatgatgttcttctggatttcattggagccgccgaagatcgacagcttgcggttgttgaagtagcgcgccgcggcggccgatgcgtaggccgggccgaaggtctcgccgtcgaagccgtcgtgcagcgcttgctcgatgaagggccgaccgtacacacccatcgcgcggcgcgcgagcgacgaaatctcctgccggatctcggtgccgcggatcttcagcatcgagctctccgcacccggcacgccgccgccggccacggccgcaatcacgcgcaggttcgtcgtcttcatgttttccaggtcgatctcgacacgcgccatgcgcgccgcgaaggccgggtcttccgccagcggcttgccgttcttcgtctgcgtggcggcaatgcccttgagctgttcgagcgcggccaccgagaagcccacgcccgcgatgttggtgcgctcgtaggtgagcaggtacttggcgcaggtccagcccttgttctcttcgcccacgaggttctcggccggcacgcgcacgtcggagaagaacacctcgttcacctcatgctcgccgtcgagcgtgatgatcgggcgcacttcgacgcccggcgagcgcatgtcgatcaagaggaagctgatgccctcctgcttcttcgcctcgcggttggtgcgcaccaggcagaagatcatgttggcgtgctggcccagcgtggtccaggtcttctggccgttcacgatgtagtggtcgccttgggcatcgatgccgcgcacggccgaggtcttcacggccgcaaggtcggagcccgcgccgggttccgagtaaccctggcaccaccagtcgtcgccgttcaggatgcgcggcagccagcgctgcttctgtgcctcgttgccatacctgatgagcaccgggccgagcatgttcacgccgaagggcacgatgcgcggcgcaaaggccagcgcgcattcgtgttcgaagatgaacttctccaccgccgtccagcccgggccgccgtactgctcgggccagtggttcgcgagccagccgcgctcgttgaggatggcgtgccacgcctccatgtcggccttggcgaggatcttgccgccgctgaccttcgccgagaggcgagcgggcagcttgtcggcgaggaaggcgcgcacctcgctgcggaaggcttcttcttcgggggtgaagttcaggtccattgccggctcctcagtagatttcgaacaggcccgcggcgcccatgccgccggcgatgcacatcgtcaccacggcgtatttcgcgccgcggcgcttgccctcgatcagcacgtggcccgcgaggcgcgcgccggtcatgccgaagggatggccgatggagatcgcgccgccgttcacgttgaggcgttccggcggaatgcccagcttctcctggcagtagatcgactgcgaggcgaatgcttcgttgagttcccacagaccgatgtcctcgaccttgaggccgtgccgcgcgagcagcttgggcaccgcgaacaccgggccgatccccatctcgtcaggctcgcagccggccacggccaggccgcggaacgcacccatcggcttgaggttggcgcgttctgcatccttggcttccatcagcacgcaggccgaggcgccatcggagagctgcgaggcgttgcccgcggtgatgaacttgtcttcgcccagcaccggcttcagcttggcaagcgcctcgtaggtggtgccgcggcggttgcagttgtcttccgtggcggtgacttcgcggtagctgacttccttggtctccttgtcggtcacggccatcgtggtggtgcaggcgacgatctcgtccttgtagcggccggcgagctgcgcttcttcggtcttgcgctggctctcggccgagaagcggtcctgcgcctcgcggctgatgccgtagcgctgcgccacgatgtcggcggtttcgatcatcgccatgtagagcgcaggcttgtgctcgacgatccacggatccaggctgaggtcgccgccgtcgccagggctgcggccgcggatctgcgagatgctctcgacaccgcccgcgatcatggccggcgcgccatccaccacgatgcggcccgccgccatggcaatcgcctgcaggcccgaagcgcagaagcggttcaccgtggtgccggcgatgctgatcggcaagcccgcgcggatgatgctctggcgcgcgatgttgcggccggtcgtgccttcggggtagccgcagccgaggatcgcatcctcgatcaacgccgggtcgagacccgagcgctcgaccgccgcgcgcacggcaaaggcggccagcgtggcgccgggcgtgatgttgaactcgccgcggtgcgccttggtgagcggggtgcgggcggtggaaacgatgacggcttcgcgcatggggagggctccttagtcagttgaggacagagcaaaaactgctgcgcagtttcttggtctgtcccgcaaggttttcagttttgattgaggctggagaaatcggcgccgcgttcgaccagctccaccagcagcggcgagggctgccagaacaacgggtcttccttcgcgaactcgcggatgtcggccagcaccttgggcaggcccacggtgtcggcgtacttcatcgggccgccgcggtggcgcggaaagccgtagccatagagaaaggtcacgtccacgtcgagcgggcgcagcgcgatgcgctggtgcacgacgttggcgccttcgttgaccatcgcggccatgtagcggcgcatgatttcttcctcggtgaaggcgcgcggcgtgatgcccgcgcgttcgcgctcggcgtcgatgatcgccagcacctcggggtcgggcacgccggtgcgcgcgccttcggggtacaggtagtagccgcgctgcgtcttctggccgaaccagccgcgctcgcaaatgcggtcggcaatctgcacgtagcgcgccttcgggtcgcgcgtggcggccttgcgcttgcgcgtggcccagccgatgtccccgcccgccaggtccgacacctggaacggccccatcggatagccgaagttgcgcaccgcctcgtcgatctggtagggcgaggcgccgtcttccatcatgtggtcggccgcctggcggtacacggccaggatgcggttgccgatgaagccgtcgcacacgccggcgcgcaccggcaccttcttcagcttcttcgcgagctcgaagccggtggcgaccacgtcggcgctcaccttcgcgggcaccacgatctcgagcagcttcatgatgttggccggcgagaagaagtgcaggcccaccacgtcctgcggacgcgagacgctggccgcgatctcgtcgatgtcgaggtacgaggtgttggtggccagcacggcaccgggcttgcacacgcggtcgagttcggcgaacacagccttcttcacgcccatgtcctcgaacacggcctcgaccacgatgtcgacctgcgccagcgcgtcgtaactcgtggagcccgagaagcgcgccatcaccgcggccttggcctcgggcgtcatgcggcccttcttgatcaggccgtcgtacaccttttcgacatgcgcgcggccgcgcgcgaggctgggctcgtcgcgctcgatcatggtcacgggcatgcccgcgtcgagcatcgccaccgcaatgcccgcgcccatggtgccgccgccgacgatgccggccgcgtcgagcgcgcgcggcttggccgccttggtttcgggcgccttcagcacttcgcgttcggcaaagaaggcgtggatcaatcccgcgcgctgcgggctatcgatgcattgcaggaagagcttgcgctcgagcgccatgccttcggcgaagggcagcgtgagcgcggcttcgaccgcttcgatgatcttcatcggcgagaacaggccgcggctcttcttggcggtgtcggtgcgcgcggcctccagtgcggcgcggctggcttcggcatcggccagcgcggtggcttcgcgcgtgcggcgcaccggggccttggcggcgacgagttcgttcgcgtaggcgaggccttcggcgagcgcgtcggcttcgttgccgagccggtcgacgaggccgagcgacagcgcttccttcgcgcccgcatggtggccgctcagcatcagttcgagcgcgggcttcacgccaatcaggcgcggcgcgcgctgcgtgcctcccgaacccggcaggaggccgagcgcgacttcgggcaggcccagcttggcggaaggcgcggcaaggcggtagtgcgccgagagcgccacttcgagaccgccgccgagggctgcgccatggatggcggcgaccaccggcttgctgcagttctctatcttcaggcacacctcgggcaacgatggcggctgcggggtcttgccgaactcgcggatgtcggcgccggcgatgaagttgcggcccgcgccgacgatcagcaccgcggcggcgccgttgtcggcctcggccgcgtcgatcgcagccacgaggccgcggcgcacgtccacgcccagggcgttgacgggcgggttgtcgatggtcaccacgaacacgtcgcctcgacgttcgaaggtgacgggaccggaagacgtggaggggctggagcttgaggtggccatgtgctttgtctcttgcgtggcgagccctgcaacgcgaggggctcgaggctctggggtgaacctcgcattcttggtccgcgccgccgctttgacaattgcatagtccattgacagactgtcaaagaatttttgacacaatcggggcatggacgtccaatcgctgaccctgctggtggaaatcctcgacgccggcaacctgagcgcggcggcgcgccggctcaagatgagccgcgccaacgtcagctatcacctgaaccagctggagcgctcggtcggcgcgcagctggtgcggcgcaccacccgccgcgccgagccgaccgagatcggcctgcgcctgtaccagcacggcgtggccatccagactgagctgctggccgcgaaagaatcggtcaccacgctgggccagggcctgcagggccgggtgcgcctgagcgtgccgagcggctatggccagttggtcatggccgactggctgatcgacttcaagcgccaataccccggtatcgtgctcgacgtggtgttcgagaaccgcatcgaggacctgctgcgcgacgaggtcgacattgcgatccgcgtggtgcccgagccgccgcagaacctggtggcgcgcgacctggggccggtgcgctatgtggcttgcgcctcacgcggctatgcggaaaaacatccgttgccggtgcagctcgacgaactgcagggcgcgccggtggtcacggcggccgtcatcggccggcagctgcgcgtgtcggcctaccagggggaaacgcggcgcgaggtgattttggagccgacgttgatctcggagaactttctgttcctgcgccaggccgtccttgcgggcctgggcatcggcctcgtgcccgactacgtggtgcaggaggacgtgcgcaagggcgacgtggtgaccacgctcgacgactggcgcctcagcatcttcggcacgcagatgttcatgctctacatgcccaaccggcagcacacgcgcgcgatccgcaccttcatcgatttcatcctggagcgggtgcgggcgcctggcgccgaaccggccgatcagtcgcagcggtaggtgacttcgccctgcggcgcgcgggctgccgccttcgggtcgaggtagcgcagcggggcgccgaagttgcggcagtaggcctccgcgtcctttgccgtgggcgacttgtacacgccgtcccccagccgtgtgacgaggggtgccggccccgttgcgcatgccgcgaggagcgcggccggaatgagcaggcagagggtgagggagcgtcgcatcgggaaggcgcagggctgcgcggaggaacaagaagtccgcgactttagcgcctgccggtccggcgccggcagggatgggatgacccgcggcatgttttctgctgtactcgccgcatgaacgatggtgctccccacgccctgctgccgcttgcggcgcaaccgctgacagcgcaagctttcgcgccctacggcacggtgctggcggcgcccgccggcacaggccgcccgatcaacggcggcaacgcgcagcgcttcgacctggtggccgacctgcagcttggcgccgcgggcggccggccgatgctcgcgctgttccgcgcagaggcgcggcgttttccgcacgaggtcacggagatggagcgccacgcgctcggcagccagaccttcgtgccgttgggcgagcggcgcttcgtcatcgtcgtggcaccgcctggtgaagctccctcggccgccgcgctcgccgcgttcatcaccgatgggctgcagggcgtgacgctcgcgcccggcacctggcaccacgcgctgctggcagtggacgccggcgacttcgtggtggtggagcgcgccggcgatgcggtcgattgcgacacctgcgcgctggcggcgccggcggtcgtcgactggaacggctaggcgggtttcttcctggcaaggctttgcgccaccagaacggcttcccttgccagtgccgtcagcgcttcgtggtcttcgatgatctcgatggggacctcgaagtacttcttgacctggacccgccgggccttcgtgtcgtaggcaaagcatttgctgcccagcttctcgtatttcggccgggtgtccttgtccacgacgaagtacacggtgctgcccatgatcatcgcgaattgggtcgcattggccgacagccccgttccgccaaagaaacggctcttggcgatgcgcgggattccggagagccggtccacgatgaaatcgacgaactgcgacgaggcttccgacatgatgttgctggcgccaggcgctggatggaaagagcgcagtgtcgccgagtccagcgaagccgcggcgcgtcagcctgcggcaatgcgctccgccaatgcaatcaacgagcggtccgacccggccggcccgagcagcgagataccgagcggtgcgccctcgcgctgcgcgagcggcatcgacaactgcggaaagccgctgaggccggcgatgcaaagcatccggatcgcgcggttgcggtagtcctccagcccggcctcgccctcgctgcgcagcggcgcaatgtcgggcatggtcggcatcagcagcacgccgtcgctcccgagcagttccgccaggtggctgcgaaaggcggcgcggaaggtgcggccggcggcgatctgcgcatcggtcacgtcgcgcgaccacgcaaagcgctcggccacgcccgggcccagcggcggcgcgtagcgttcgatcagcgggccgtccgtgagccaggcctcgtgcgactgcacgtagcggaagttccagtacatcgcatcgaaggagtcgagcgcaacggtcgtgcctttcgcttcgccgagcacagcctgcacgcgcgcagcggcatccgcgagcgcggcggccgccgccggcacggcgagcgaccaggcgtcttcggggcgcagcagccgcacgcgctgcggcagcgcggccgtgtcgtcgcccagcagcacgtcggcgacgcgcgcgaaggtgccgatgtcgcgcgcgaaccagccgcaggtgtccaggctgggcgccaggtccagaacgccttcgaggctcacgcggccgtgcgtcgggcgcagcccgtacagcccgcagtggttggccggcgcacgcaccgagccgccggtgtcggtgccgagcgcgaagtcgcacaggcccgaagacacggccgacgcggagcccgacgagctgcctcccgtgatgcggttcttggccgcgccgttgacgggcgcgccaaagtgcgcgttgttgccgttcatcgagaaagcgagctcgtcggtcacggtcttgccgacaaagcgggcgccagcatcgagcagcttctgcacggtgggcgcggtgcgcgccttgatgcccgacatggccagcacgatggggctgccgccacccgtcgggtagcccgccacgtcgaacaagtccttggcggcaaaactcaggtcggccagcggaccggtgccggcgcgcggcacgggcacgtcggggtagggaacgaaggcatgtgcggggtcgagcagcggcatggcgatgaagggggtggacgaagaaatttcaggcgaccaggacgggcgcggtggccgctgcggcatccgtgcggatgcagcgcgcgcgatggttcggtgcaagctccacggccgcgggctgcgcggcccggcacatgtcgttcgcgagcgcgcagcgctcggcaaaggcgcagcctggcggcagggcggagagatcgggcggcgcgccgccaatggtttcgagccgcgcaccacgcgccagcgcaccgtgtgcacggctcttgagcagcgcaatggtgtaggggtggcgcggcgagcggatcaactcgcgggcggtgccttcctcgacgatgcgcccggcatacatcaccgcgatgcggtcggccacctcgaccgccgcgccgatgtcgtgcgtgacgaagatcaccgacaggccgaggtcgcgctgcagctcgcgcagcagcagcaggatctggatctgcaccgtggcatcgagcgcggtggtcggctcgtcggccagcaacagctggggcctgcaggccagcgccagcgcaatcatggcgcgttgccgcatgccgcccgacatctcgtgcggataggccgcaagccggcgttcggggctcggaatgcgcacccgctcgaacagcgcgagtgcgcgctgccgcgcctcggcctcgctcacggcttcgtggcggcggatcgattccacgatctgcgcgcccaccgaatacaccgggtcgagtgccagcaagggttcctggaagatcatcgacgccaccttgccgcggaagtcgaacagctcgcgctgcggcatcgcgagcacgtcgcggcccgccacctgcacctggccgcccatgcgcgtgcggcgttccggatgcaggcgcagcagcgtgcgcatggtcacgctcttgcccgagcccgattcgccgatcagcgccaccacttcgccgcgctgcacctccaggctcacgccgctgacggcatgcacgggcttgcgcccgccggagaaggtgacgctgaggtcgcgcaggcggaccatcggttcgccgtcgggaatgatgctgccgttggtgctcatgctgcttgactcatcggttgctgcgccagcggatgcccgctgcccggctcgtggaccaggcagctcaccgcgtgccgcgagcccgtggcgatgcgttcgggaacgacctggctgcacaccggcgcagccagcgcgcagcgcggatgaaagcggcagccggtgggcgggttgatggggttcggcgggtcgccggtcagtgcggcttcctcggtgcggttgtcggggtccatcgagggcatcgaggacagcagcgcgcgcgtgtacggatgggccggcgcatcgtagagcgcttcggccgggccgatctcggccacctggccgaggtacatcaccatcacgcggtcgctcacgtagcgcaccacgttgaggtcgtggctgatgaagacgtaggtcaggccgaactcggccttcaggtcgagcagcaggttgatcacctgcgcttccaccgacttgtccagtgccgacacggcctcgtccagaatgaccatgcgcggctgcagcgccagcgcacgcgcgatgttgacgcgctggcgctggccgcccgaaagctcgtgcggatagcgctcggcaaagcgctgcggctcgagcccgacgcgggacaaaaggtcgcgagcgcgggccacggcgtcgcgccgggacacgccgtgcacctgcgggccgaaggcgatcgagtcctcgatggtgaggcgcgggttgagcgaggcgtagctgtcctggaacaccatctgcacctgccggcggaactccttcagcggcaggtcgcggcttccgacctctcggccgtcgaacaccacttcgccgcgcgtcggctcgatgagctgcatcaggagccgcgcggtggtcgacttgccgcagcccgattcgccgaccacgcccagcgtctcgcccttcatcacctcgaagtccacgccgtccacggcgcgcaccacgccgccgccacggcccagcgggtctttcttgagcggaaaatgcttgaccagtccggtgatggtgagaagcggctgcgcggggccgccgacgtccttcggtgcatccatgcggtccatggtcagcccttgttgtccatcgccgagcgcaggccgtcggagaggatgttgaaagagatcgacgtgatgaagatcatcacccccggcagcgcggccacccagggctgaacatagatcgccgtgcgcagcgtgttgagcatcaggccccattcgggttcgggcggcttcacgcccaggcccaggaacgagaggcccgaggccaggatcatcgacaccgcgatcaggctggtggcgtagacgaagatcggcccgagcacattgcccagcacgtgcacccgcacgatggtgaacgggctcgcacccgaggcacgggccgcctccacgtagtcgcggttgcgcacctgcgtggtcacgctctcggccacgcgcgcaatctgcggaatgaaaacgatggtgagcgagatcagcgaattgaccacacccgcgcccagcgtgcccgacagcgcaatggccagcagcaccgaagggaaggcatagaacacgtcgatggtgcgcatgatcagcgtgttggtgaggccacccgcatagccggccaccaaaccgatgaccgtgccgagcacgaaggcgcagagcaccggcgtgatgccgatgaagagcgacagccgcgcaccgacgatcagccgcgagagcatgtcgcgcccgagttcgtcgctgcccagcggcaggcccgcggtgccgatgggcttgagccgcttgagcatcgacgactgataagcgtcggcgggtgcgatccaggggccgatcagcgcgagcgcgatcaagagcagcacgacgacggccgcgcccacggccacggggtcgcgccggaagcgcagccagacggaggcccagtagccgcgggagcgctgggccggcagcggctcgacggcggccgcgacaggagaagaagcgagcacggtggacatggcttttccggttccttcttcttcaggcacgcgcaatgcgcggatcgagcagcgtctgcagcacgtcgaccagcaggttgagcacgacgaagaacagcgccagcacgaggatggtcccttgcagcagcggcaggtcgcgctggaagatggccgagttcagcagaaagccggtgccgggccatgagaacacggtctcgatcaggatcgagccgccgagcagatagcccagttgcaggcccatcacagccagcgccgtgggcgccgcgttcttcaccatgtggcggaacacgccgaagtgcgtgagccccttggcgcgcaagcccacgatgaactcctggtcgaggatgtcggccaccagcgcgcgcaccgtgcgcgcgatgatgcccatcggaatcaccgacatcgtgagcgccggcagcaccaggaactgcaggtgcgcccagtcccaggcccagtcgtcggaaccgctcgggcccgcgcccgtggccggcagccacatgagctgcgacgagaacacgatcaccatcaccatgccgagccagtagtgcggcacgctcacgcccagcaccgacagcatcgaggcgaagcggtccacccacgagccgcggaagtagcctgccacgaacccgaacaggcagcccagcacgaagccgatgaaggtggccaccaccgccagccgcagcgtgttgccgacggccgtgagcacctccgacgccacggcgcggttgctggcaatggacacgcccaggtcgccgtgcagcgcgcgccagatccacatcgcgaactgctcgggcagcgaacggttgaagccgtacagctcgcgcagttgcgcctgcaggtcggctgaagcatcgggcggcaggatcgacaccagcggatcgcccggcgcgatgtgcacgagcaggaagcacacgagcgccacgccgatcatgatcggcacggcgtagacgatgcggcgaatcaaataggaaaacatgaagctttgttatcaggacgtggcaagcgcagcgaagccccttcggggaacaccgcggaaccggctttgccgggccgctggtgttgcccccggtgagggggatggcgcagcgacacgaagtgcgcgaagcttgggggagagctcattgcatcaatccatcgccatggtggcaatgtcgatgaaccagctcttcggctgcaccacgttcttgaccttggccgacatggcgcgcggacccacgtcgtgcgcgatccagacgaagggcgcgtcgtccacgatgtgggtgtgcagcttggccagcgccgtgtcgcgcgccttgtcgtcgaagctggtgcgcgcgtcggccacgagcttgtcgacctcggcgttgccgtagtagccccagttgttcgacaccggcgggaaggccttggtgctcacgaagcgcaccatcgcaaagaacgggtccatcgccgcgaagctcacgttggtggcgttggcgccgttggccgatgggtccttcgcgcccttgcgccagttggtgaagagcgtgttccattcgatcacgtcgaattgcacgtcgaagaagcactgcttgagcgactcctgcgcgaactcgttcatcggcagcggctgcatctggcccgagcccgaggcggagatctgcaccttcaccttgatcggcttggcggcggaatagccggcctgcgtcatgagcgcctgcgcggccttcacgtcgtacttgatgtcgaaacccggcttgccgaaccaggggtggcccggcggcaccgtgcccttgggctcggccatcatgccgcccagcagctgcttcatgccgccgcggtcgatgcagaggttggcggcctggcgcacgcgcttgtcgagccacggcgaaccttcggcgaacgagagctgccacggccacacgtgcggctgcgcattcgaatagatcttgaagccgcgctgcgtgatctgggccatggcgtcaggcgcaggcgcctcgatccagtcgacctggccgccaagcagtgcggcggtgcgcgcattggcctcgggcatcgggatcatcacgaccttgtcgatcttcggcacgcgcctggcgtcccagtaggtcttgttggccgccagctccagccgctcgcgggcgacgaagcgcgtcaccttgaacgggcccgagccggcggggtcggccgcgaaggcggtccatgcggccttggccttgtcggcgggcgttgcgccggccgcggcgtcgaacttcttctgccactgcgcaggcgaggccatgaacaggttcgtcaagttgatcggcaggaaggcatcgggttcgctggtggtgaactcgaccgtgaggtcgtcgatcttgcgcgccgtgcgcagcgtgggcatgcgcgaggcggtcacgcccacctggctggggtcgaactgcggtgcgtccttgtcgagcaccttctgcacgttccacaccacggcatcggcgctgaagggcgagccgtcatggaacttgacgccggggcgcagcttgaagacccacttggtcttgtccttggcatccacggcccacgacgtggcgaggccggcgatcagcacgctgggcgcatcggccttggacaggtcccattgcgtgagggaatcgtagatcggaatgccggtgaagcggttgccctcgaagccctggtcgggctggccgagcgtgcgcggaatgtcggcggccgtcatggcgatgcgcagggttttttcctgtgccagcgccgtgggcgcgacaccagcgagggcggccagcgccaggcaggcggcgaggggtttcagggacagggcgggggcagcacgcttcacatggaactccggtgtgggatgacaaaaaggacgaaaaaactctcaagcacgacatgtgccagccgggccagaagccctggccgattcagggccatgacagcgcgatctcgcgccttgcgcagcgcaggtccatctcgacttccatgtccacgatcggcggccgcgcaaggtgccaggtcaggccggtggtgagcccgccgcgctgcacgatctcgtcgaacaccagcgcgccgatgtcatgcaccgtgtaggcctgcaccgcggcagcatcgtgccagccgaagcccagcgcggcgaggcggcgctccatttcggtcatcacgtagccgagcttggcgcgcaggccgtcggggctggtgtcgcccaggcggaccatcacgtcgcggtagctcgcgtggccgtcgggcgcctcgccgccgcccgagaccacgaagctcggcgggccggcatcttcgtcggccggcacggtgtacgagaaggcctggaaggccggcgtggccggtgcgccgacgcgtgggcacacgttggtgcgcgccaccggattgcggccgccgcgcaccagctgccagcgttcgagcgtgccggcatagaggcgattgaagtcgtgaaagccgcgctccgagaacggtgcgggcgagcgaagttcgcaggcgcacagcgcggtgggcggccggccgatggcgctcaggtgcgccgcgatggcgtcgaagccgtcggccagcggcacggcctgctggaagcgcacccgctcgatggcaaagccgggcagcgcggccacgccggcggagtactggaacacgccgttcgcgtagcggtagccgccttcggggaatgcaatggtttcggtggtcggggtggtcatgccgtctttcctgttcagcgcccaatgtagggagtgcagggtcagacaggaagtctcatttctgcacgcgtgtgttgccggaatcagaacgcggcgtggcgttgccgccgtatcgccccatgctggtggccagcatttcgagcagcgcgcgcaccgccagcgattggcgctgccccggcagcgtgagcaggctggtcgcggtggcggcaaagtcgcgctcctgcagcggcacggcgcacaggtcgccgttggacacctcgtgcagcgcggcatagcgcggcaggaaggtgatgagatcgctgttgcgcaccacgcccttggccatgtcgagcgtgctggtctcgatcaccagatcgagcgacacctgcgtcttcgacgcgatgcggtcgaccaggtggcggatctggaacgagcggtcgggcagcgccacgcggtggccctcgagctcgcggaacgacacgctgcgccgccgcgccagcgcatgcgtgggcgcgacgatggcgcacagcggctgctccagccttgcgtgctcgcggaaggcgtggcgctcgggcaggttgaaggccagtgcgatgtcgatgcggccttcctgcagcgcttcgagcaccgcgcgcgaacccaccaccgaggcctgcaccttcacctgcggatgccgcttctggaagcgcgcgaggttgtttgccaggaagtggccgaccatgccctcgatgctgccgacgcgcacgatgcctgcgggttggcccgtcagctcctgcagcgcgccgcgcagcgcctcgctgttctgcagcgcctggtcggcatgtgccagcaccagctcgccggccggcgtgagcgtggtccggttggcgcggcggtcgagcagggcggtttgaagctcgccttcgagcttggcgatctggcggctgatggcgcttggcgccacgtccagctgttccgcagcgcggcgcagcgaaccggctttggcggtctcgcgaaagtagagcatcgctgtggacagcatcgcgggggtttcctctttgtcttgcgggtggcctgtgccggccgaaccttgggccgatcggccccggacgtcaagcaacgggcgtgccttggggacggcggccgcgagggcgcccgagcggggccgatgcgacaatcgccttcccatgacagataccctcaccatcacccgcccggacgactggcacctgcacgtgcgcgacggcgccgccctcgaagccgtggtgccgcacagcgcgcgccagttcggccgcgcgctgatcatgcccaacctgcggcccccggtgaccaccgcggcgcaggccatggcctaccgcgaccgcattcgcgccgcggtgcccgaaggcacggccttcgagcccgtgatgtcgctctacctgaccgacaagctgccgcccgaagaaatcgccttggccgccgctgccggtgtgcgcgcgctcaagctctacccggccggtgccaccaccaacagcgatgccggcgtgaccgacatccgccacacctacaagacgctcgaagcgatgcagaagcacggcctgctgctgctggtgcacggcgaggtgaccgacccggccatcgacctgttcgaccgcgaagccgtcttcatcgaccgcgtgatgattccgctgcgccgcgacttccctgagctcaaggtggtgttcgaacacctcaccacgaaagagggcgctcactacgtgcgcgacgccagccgcttcacggccgccaccatcaccgcgcaccatctgctctacaaccgcaacgccatcttcaccggcggcatccgcccgcactactactgcctgcccgtgctcaagcgcgagacgcaccgcgtggcgctggtcgaggctgctgccagcggcagcgaccgcttcttcctgggcaccgacagcgcgccgcacccggcccacctgaaggagcatgcgctcggctgcgccggctgctacaccgcgctgaccgccatcgagctctatgccgaggctttcgacagcgtgggcgcgctcgacaagctcgagggctttgccagcttccacggcgcagacttctacggcctgccgcgcaataccggcaccatcacgctgaagcgcgaaagctggaccgtgcccgagacggtgccctacggcgacgccacgctcaagccgctgcgcggcggcgaaaccatcgcctggagacttgcatgacacccacgctgcgtgtcatgcttctgatcgatgccgacaacgtctcgcccgacgtgatcgagcaggccgtgcagcggaccatggccgagcatggcgccatacacgtgcggcgtgcctactgcaatgccgaaaccgcgctcaagcagcagacgctcttcaagcgcctgtcggtgcggccgatggtcaatctctcggccggcaagaacagcaccgacatcgcgctcgcggtcgatgccatcgacctcgtgattgccgagcgtcccgacgtggtggtgctggtgtcctccgattccgactttgcgccgctcgtgatccgactgcgcgaaaagggctgccgcgtctgcggcctcggccagcagggcaagaccggcgaagagaccgtggcggtgtacgacgagttcaccgacctgcggcaccatggcgcgccggttgcgccggccgctgcgccggccaagaaggccgcggccaaggtggccgcgaagcgcgcacctcccgccaagaccggcaagagcgcgaccacgccagcccgcaagaccgcggccaagacaacaccggcccgaaagacggccaaggccgccaagccggtgcagccgccttccgaagcggccgagttcatcctgcaggcggcgcccgccctgcgcagcggtgccgacgtgccgctcaacgacgtcgcgcaggcattgcgcgcggccgggctgctcggcaagcacggcagctcgctcaagctgttcgacaagctcccggcggagtttgccgtgctgcagcaccccgaccgcatccgctggaccggagcccccgcgccttgagcctggaggcgatcgactgggcacagccctggctcgcgccttatcgggccattggcgaagcggcggcgcacaccgcgctctgcacctccgttgccgcggcgctggcgcagggcgccaagccggcttccgcgcccaccttcgtgccgcaactggacctgcccgcgggccgtgcctacgaagcccacatcttccagaccggcaccgtgccgacccgcgacaacctgcacgacttcttcaacgggctggtctggctggcgtttcccgaaaccaagcgccgcctcaatgaactgcaagccgcggagatcgcccgcaacggtgtcacgtccacgcggggtccggtgcgcgatgcgctcacgctcttcgacgagaacggcgcggtgctcgatgcacccgctgcgttgtggaaagcgctggccgcgcgcgactggcagagccttttcgtgacgcagcgcgcgctgtggtccgaggtgcgcctgatcgtgttcggccatgcgctgctcgaaaaactcgccaccccgcgaaaggcgatcaccgcgcatgtgctgctgctgccgccttcaccgaacggcggcggaccgcaggcgcttgatgaccgggcgctggcgcgcagcctcgatgcggaatacctggcgcagaaacctttcgtcccgctgccggtgctcggcgtgccgggctggtgcgcggacaacgccgcggcggatttctacgacgatccgaaggtcttcaggcccggtccgtagaacttttgctcctatcatcgctctacccgccagccgcggtgcggctcatcgagaacccaaacaacacaggaagagcgtcattttctgcacggcttgaagagggccatccggtcctcatctatgcggcagcattccccacggagaattcaacttgaaacgtatccttctgttcgttttgaccaatgtgatggtcgttgcagtgctcggcatcgtcgccagcctgctcggcgtcaaccgctttctgacggccaacgggctgaacctcacggcgctgctcggctttgcgctgatcatgggctttggcggtgcgatcatttcgctcttgatcagcaagcccatggccaagtggacgaccaagctgcacatgatcgacaacccccagacgcccgacgaggcctggatcgtcggcacggtgcgcaagttcgccgacaaggccggcatcggcatgcccgaggtcggcatcttcgagggcgagcccaatgccttcgccaccggcgcgttcaagaactcgtcgctggtggcggtgtccaccggcctgctgcagggcatgacgcgcgaagaagtcgaggccgtcatcgggcacgaggtggcgcacatcgccaacggcgacatggtcaccatgacgctgatccagggcgtgatgaacactttcgtcgtgttcctgtcgcgcgtgatcggctacgcggtcgacagcttcctgcgccgcggcgacgaccgttcgtcgggccccggcatcggctactacgtgagcaccatcgtgctggacatcgtgctgggttttgccgccgccatcgtggtggcgtggttctcgcgccagcgtgagttccgcgccgacgccggcgcggccgcgctcatgggccagaaacagccgatgatgaacgcgctggcccgcctcggcggcctgccggccggcgagctgcccaaggcggtggaagccatgggcatcacgggcagcatcggcaagctgtttgccacgcacccgcccatcgaagagcgcattgcggcgctgcagaacgcgcgcggctgatcgttccgctcggatagcaaaaagccgccacggtttggccctggcggctttttttttatgggtgccgcggcggcatcatcagtacgaactcagtacgaactcagtacgaacgcagcgagatgccccagcgcccggccacgcgggtggcgatccagaggttgcggtgcgtgctgagcaccatgcccgccccgtcttcgcgcgtgtaggtgacgacgaaatgcaccttgtcggcgcttgccagcaccgcttccttcgactggtagcgcgtgcaccgccagcccgaggccctgagtttctcgaagaagtcggcgggatggttgccgggcgcctgccattcgaggcggtcggcacccgagagcatcacatgcgggaagtgaagctcgccgtccatgcccgcggtgtcgcaggcattgaagcgttccgtgaaacggtcgaggcaggcggaggcttcgcggattgcttccatctcggccgcgcctccgggcgccggtggtgcgacgaagtctgcgaagtcggtcacgggcgccgaagaaacaagcgggccggtcaggccgccggaggaacctgtggccgctcggcccgtgcgcgtgcgagcgtgcgcgccacctcgtcggcgtccatgccgtacatctcggcaaattcatgctcgctgccgcgtccgctggcctcgaaggcgcgcaacagcgcctcgcgcttggcggcctgacgggccagttcggccagcgcttcgtcgagcacggcattggtttcttcgtcgcgcgagcgcaccagcaccgcataggcttcgcggtcgaggccggaggcttccacggcccgggcgatgcgcgccaccaactgcgggcgcaggtcttcaccggaacgctgggtgcggcggcggtggagttcaaggatggcgtggtgcacatgctcgggcgcaacgggttccaccacattgccatcgagatcgtggcgcgcaaggcccgcggccaccgcttcgaggtagcgcgtggagcgtgcgtgcaggcccagcgcgaccttcaggtcgtccttcttgaagtcgtccgggtgcttttcgagcaggtcctgaaacaccccgagcttgagcggcagaaagcgcgcgccgaacatgttcgggtagagctcgaacagtttctccagcgcgggatgcaccttgcgcgaacgcgccggctgttgcggctgctgggccgcctgcttcggcttctgtttttgctgttgctgctgctgccgtggctggcgcggcgggcggggcgaccggggcgggcgtccgtcggcggccggctgctgcggggcggcgccctcggcttccgtcggctggacttcctggatttcttcttgaggcgtggcggtgtcggtcatcggtcggttcttgtcaggttggcagcggcggaaaaaatggattccgcgcgctcagcgcgggcggaacatcttgaagagattgtcggggctgatctcgaagtagtcggcggggccgcctccgcgcaggatgggctgcgccgcggcggtgtcgtagatgccgttcttcagcaggtgccgtgcaatgtgcacgcccaccacttcgccaagaatcagccaggtgggcaccggcacgccgtcgacaccttcgagctgcagcacctgcgtgagccggcattcgaaggacaccgggctctcggccacgcgcggcaccgcaatgtggcgcgaggccgcgggcgtgaggcccgcgagctcgaactcgttcacctcgggcggcacggccgcgcacgactggttcatctgctcggccagcggccgggtggccaggttccagccaaactcgcgcgtctggcggatgttgtgcaggctgtccttggcgccgatgctcgcaaagccgacgatcggcggcgtgtagttgaaggcgttgaaaaagctgtagggcgcgaggttgagcgcgccgttctcgtcctgcgaagagatccatccgatcggccgcggaccgaccatcgcgttgaacggatcgtgcggcaggccatggcccttggcgggttcgtagaagtggaaatcgtcgttcgacatggctgcggttcctcaggcccccgcgacgctgcgcgccacggcttcggccaccttgatgccgtccacgccggccgacaggatgccgcccgcgtagctcgcgccttcgccggccggatacagcccgcgcacgttgaggctctggaaatcgtcgccgcgcgtgatgcggatcggcgacgaggtgcgcgtttccacgccggtgagcaccgcgtcgtgcagatcgaagcccttgatcttgcggccgaaggcgggaaaggcttcgcgcatcgcctcgatggcataggcgggcagcgcctggtgcaggtcggtgggcgtgacgccgggcttgtacgaaggctgcacgctgccgagcgcggtcgagggcctgcccgcgatgaagtcgcccacgagctgacccggcgcgcggtagtcgccgccgccgagcacgaaggcgttcgattcgagatcgcgctgcagtgcgatgccggccagcgcgtcgccggcggtctcggccgtccagccgggaaagtcgcgcggatcgatgcccaccacgatgcccgcgttggcgttgcgctcgttgcgcgagtactggctcatgccgttggtgaccacgcggcccggctcgctggtggccgcgaccacggtgccgccgggacacatgcagaagctgtagaccgagcggccgttgctggcgtggtgcaccagcttgtagtcggccgcgccgagcagcgggtggcccgcgtggcggccccagcgtgcgcggtcgatcaggccctgcggatgctcgacgcgaaagccgatggagaagggcttggcctcgatgtgcacgccgcgctcgtgcagcatggcaaaggtgtcgcgggaactatggccgagcgccatcaccacgtggtcggcgcgcagttcgctcgtctggccggtggtctggtcgagcacggtgaggccgcgaagctggccgttttcgatctgcacgtcggtcacgcgctgttcgaagcggatctcgccgcccagcgacacgatctgctcgcggatgttctccaccaccttcaccagcttgaaggtgccgatgtgcggatgcgcgacgtaaagaatctcgggcggcgcgccggccttcacgaactcctccatcaccttgcggccgaggaagcgcgggtccttgatctggctgtagagcttgccgtcggaaaaggtgccggcgccgccttcgccgaactgcacgttggattcggggttgagcacgctcttgcgccacaggccccaggtgtcgcgggtgcgctggcgcacggtcttgcctcgctccagcacgatgggcttgaagcccatcttcgcgagcatcagcgccgcgaagatgccgcaggggccgaagccgatcaccacgggccggggcgcgccttcgggcgcctgcgccggcggcgtgtagcgcatgtcgggcgcgggctggatgtgcggatggccggcatgccgggcgagcagcgcggcctcgagcttcgcatcggcgagctgcacgtcgacgatgtacacctgcagcagctgcggcttgcgcgcatcgaagctgcgcttgaacaccttgaactcgcgcacgccggaaaccggcgtgtcgagggcggtggcaatggcttgggggagggccgcgtcgtcgtggtcgagcggcagtttgatttcggaaattcgcagcatgtcggtggggcttgtatttatcaagcaacctgcgattttacgtgtcattcgtggaacaccgaggaaccggctttgccgggcctctggtgttgcccccggtagggggttggcgtagcgacacgaagtgcgcgaagactgggggcgagccagattacggtaggaagccttcgaccgagaggtagcgctcgcccgtgtcgtagttgaagcccagcaccactgcgtcgggcggcagcgtgggcagcttctgcgcaatggccgtgagcgtggcgccggaggagatgccgaccagcatgccttcctcgaccgcgcagcggcgggccatttcgcgcgccggttcggcgtcgacctgcagcacgccgtccagcagcgaggtgtcgaggttcttcgggatgaagcccgcgccaatgccctggatcggatgcggcgagggcgcgccgcccgagatcaccggcgaggccaccggctccaccgcaaacacctgcagcttcggccacttcttcttgagcaccttggccacgccggtgatgtggccgccggtgcccacgcccgtgatcagcacgtcgatgccgtccggaaaatcggcggcgatttcctcggccgtggtgcgcatgtgcacgtcgacgttggccgggttgttgaactgctgcggcatccacgcgcccggcgtgccggccacgatttcttcggcgcgggcaatggaggccttcatcccgccggcgcgcggcgtcaggtcgaaggtggcgccatacgcgagcatgaggcggcggcgctccatcgacatgctgtcgggcatcaccaggatcagcttgtagcccttgaccgccgcaaccatcgccaggccgatgcccgtgttgcccgaggtgggctcgacgatggtgccgccgggcttcagcgcgcccgatctttcggcgtcttcgaccatcgacagcgcgatgcggtccttgatggagccgcccggattggcgcgctcggacttgatccacacctgctgcttcgcattgccgaacaggcggttgatgcggatgtgcggcgtgttgccgatggtctggaggatgttctgggctttcactggatctccttgggctttgttggggcagggcaggtcggtcgaggtgccattgtggaacgggccgccagcggatgcgaggggatcaggcgataattgcgcccgtgaagcacgccagaccgccgctggtgcaagcccgaaaggggcgacgccgcaaggcgccgcgtcgaaagaccgcactggaggaacgtccggactgcacaggacagcgcaggagttaacgactctccaccgtgaggtgaggatcagagcaacagagacgagccgattcagttcgggtgaaacgggcaatctctgcgcgcagcaacaccaagtaggccagtatcgaggtggttccgctgagctggcgggtaggtggcatcgagccgtttggcgacaaacggcccagagtaatggcggtcacgttgggggcaacctcaacgcacagaatccggcttatcggcgggcttcacacttttcttccccggtccgacgatcggcgctcgcgggcgtagccgcgggcgcctctgtgtcgttcccgattcgaagggtgcttgactcagcgcgcctcgacctgcagcacagtctcagccccgcagcgcttcttcagatccgtgccaatctgccttgtcagatcggtcaatgcccgatcgaatgcagtctggatttctccctcggagttggaccaattcatcgagtcgtcgaagccacggtaggtccgggttgctgcggctgcgtcatccatcgcgaactgcacgcgcacgacgagattggccgacttcaacgtggccagaccttgaagataggccttcagcactgaaacccggatcgcaggtgcggtcggatcgcgcgtgtagccgggaatcgacgtgatgccgccgatgaaccattcgttgaaatcttcaccgtcgatgtgcgtgcggcccaactggcccaggctacgaacatcgcgctgatcgtcgattgcgctaaaggtgaacgggcaagccgaagctgcgtcgcccggctgcgcagtgcctgcacggcgttgtacgcctgcgaccttgtccgacgcacagcccaccagaaacagcagcgccaacagggcgcagccagcggccttgccccagggcgcgcatctcacttggcaaccgtttccatggcgggctgtgcagcagaaaccgccgcaggcgccgcggtgttggaagcgggcgttgtcggcagcacaggcgtcgcagcggccatgatcggcacggcatcgagattgagcgaaccgtcgggatagcgaagcagtctgccgccgttgctttgtgataccaagttggccttcaggccgttgccggcatcagccttggccgtcgtggcttcataagcggggtacttgcgctggaggtcggcggccagcagtgcgcccgcctgtgtgatgccatcctgcagggccgttttcagcatgcgcgcgttgtcggctttccaggcttcgatattcttcgttgcgtccgcgctggccgccgggtgcttggcccggtacacgatgctgctgcgatacaccgcatttttcggcgcaagcaccggctccgagggtgtcgttgacagcgtcgccggctgtttggccgccgtgcgcgcgctggttccacgcggatagagcaggctgcgggcggacacttcgagtgtcgagaaatcgacggacatgtgatagtcgacattgacgaacatgacggcattcgatgtcgctgccgtgaacgtcttttcgtacgcttgggtgttgaccaccttcgtcaccgccacgttcgcgacctgcatgcctgacaccgactgcagtgcttgtgccagcgactcgttcatgagctggtcgaatttcatgtcgaccatttcgtccttcagtggacgaacactttcttccgccgcctttgctcgcgttgcgttgacgctcgcatctacggcacccattgcaccaccgcatgccgcggccagaagaatgcccagacccggaacggccgcgcaggcggcggcgcccgatgccgctgcgttcgatcgaacgaaagcggcgtacagctcggactgcgaaatgccgaccttcacctcgacgggttgcatggcggccaatacctcgggctggactggctgtgttgccggcaaatgcgtacagccggtgaatacgagcgacaccaataccgggatcgcggcgcagcgaatagcaaacatggattcctccccaaacgattgaatcgaatgcatcgccgcgcacctttttttgcggatattggcggcgatgaacctcggccagggctctcgtcctgtggccggtgggaatcgtacgtgtcgttactttgtgtgcgctggtccgatcgtccaaactgtgcggaaaggcacttttcttcgatttttccgagtcaacgcgtgaacagccagccgcccttgggctggcgcgtcagttcatggcgcctgacggagcgctcttcaccgtcgtcgcccacgtacaccacgtcgaagcgcagcagcttcggcgacaccatcttccagttctggatgcgcttgacggtcacgcaggccgtcttgtcgtggtactgcatttcggccatggggccgccctggaagctgccgctgtcgaacagccggcccggcgccgcgaaggggttgagcacggcgccgttgcgcgcggtgatgcagccttcggtccgcacgaacgactcgatggtgggcgccgcgctgcgcacgatcctggccacggccggcgtgggcgggttggtggcgatctcctcgcgaatgcgttccacctgcccctcggtgatgggcgcgagcccgctgggcgacaccacgggcggcggcggcgccgcgggcggtggctgcatggatgcaggcagcagcggtgccaggtaactgcaacccgccagcgccagcgccagggtagcggtgcacgcgagtgcggctgcggtcctgggtcctcggaacttcatggctcttgcctccttttcgtcaatagcctctttgttgttctctcgtcagaagcgttcgtgcggcgaaagatatcgccactgcccgggctccagcccggccagcggcacgcggccgatgcggatgcgccgcatcgcaaggatgcgcaggcccgcttcgtcgcacaggtgcgcgatctgcccgggccgcgcgcccttgagcgcaaatcgcaggccggtctggtcgtcggtctggcggccgatgctcacgcgcgcgggcgagcgctcgaagcgcaccagctgctcggggctgaccgttcccgccacgtcgaccatgacctcgtgttcgataacgcccgcgtcctcatgcagcttgcgctcgatgcgccaatcctgcgtgtagacgacgagcccgctggcgcctgtttcgagcggcgtcatgcagttctgtcccttggcgtgcgccggcagaaagcgcatgcccgcgcgttcgggctcgtggtggttggcggccaccagcagccggtgcgcggtgtcggtcgccatgccggccggcttgtgcagcagcagcgtgacgggcaccacgggctcgggcttggcgccgggttcgatttcgaccttctgatggtcttgcacgcgcgattgcggcagcagtgccggcacgccatcgacgcgcaccgcgccgttctcgatgagcagttcggcctcgcggcgcgagcagcctgcgagcgcggccacgcgtttggcaaggcgaatgccttcttcgccggggccggtcatggggcggatgccagttgccggatgcgcgccacgtgcgctgccagcgagcgggcagccaccggccacatgcgctggggcacgtcgtcgtaggcaaggggcagccagtcttccggcgtgccttgggggagtttcttcatggcggatgcaatcttggcttcgcgcttcaggcgatgcgctttcagctgggcgatggcggcgcgcgcgctgccgatcacgtagccgtgcgcgggaaggatgaaatcgatgccgcccgcttcgcaggccgcgtcgagcttgtcgagcgaatcgagatacgcgttcatgtcgccgtcgggcggatcgatcaccgtggtgctgccgttcaggatgtggtcgccggagaacagcagcccatcttcctccagcaccaggcacaggtggttggccgcgtggcccggcgtatggatggcgcgcagcgtatgggtgatgcccctgccttcggccgtggtgcccgagagcaccaggcgctcgccgccctgcagttcgcgttcggcggcaaagcgtgccgacgagcgcgccgtgggcgccgaggacagtccgaggatcggcggcttcgtctccttgcacagcgcctgcagcggcgccgcgccgggcgaatgatcggcatgcgagtgggtgcacgcgatcatgcggatgtcgccttgcgtagcgcgccagagccggccgatatgctcggcgtcgttcggtcccgggtcgatcacgaggtagcccgtggccgcgtcgcccacgatgtagctgttggtgcccggaccggtcatggcaccggggttgggcgccgtgaggcgctgcacgttgccgagcagcggcaccgggcgctcgctttgccagtcgagcgcgtgcagcatctggccgtcggggcagaccagcgcgagctcgccataaggcgactcggtttccatgtagcgcgcttcctgcccgcgcagcagcccggcgcgcgggcagctggtccacagcgggttctcggcgccatccttgggcgcgcaggcctgcagcaccgcatcgacactggcataggccgccagccgctgcagcgtgcgaacggtcggaaagatcatgaagaaactgccggcgtcgtggcgcgccagcgcatcggccggccgcacccagcagggctcgaactgctcgctctcgtcggccgtgggcgcctggccctcgggcatgcgcgccaccagaaaaggcacgtcgaatcgcctgggcagatcgcggtcggtgatccagtgcgcgaggctgaacacctggtcggccgcgagcaccaactggcgctcttcgcattgcagggcgaacgagatgggcgacgtggtgctgcggtccatcgatgcgatgtcttccatccgcacgggcctgccatcggcatggcgcgcgagcagcacgccaagctcctcgaagccttcgcgaatggccgtgatggcctgcgtcagctggatgccgctttgggtggggcggtgggcggcgatgcgcttggcggcctcgtcggcttcatcgatgtggccgccgggaaatacataggcgcctggcgcgaagcttgcagtgtcggaacggcgcgtcatcagcacttcgatgccggcctcggaatcgcgcagcagcagcacggtggctgccgcgcgcacgggcgcgggctcgcgtgcggggtgtagttgttgggtggggcggaccatgcggcgattatggagaggtcatgcggcgcgtctgcgctgcgcataagctcattcccgatcgggcatgagccgcgcgccacaatcccgggctgcaacgcccgcatcgaggaaagacagtcatgacccattctcccttttcgcattccttcaagcacaacctgctcgcggccggcgccgccctgtgcgcagccttgtcgtccagcgcctttgcgcaggccgactggccgcagcagccggtcacgctgatcatgggttttccggccggctcgggcgtcgacgtggtggcccgcgccatccaggagcccttgtccaggcagctcggaaagccggtcatcatcgactacaagtcgggcgcggccggcaacattgccagcgagtacgtggcgcatgccaagcccgacggctacacgctctcgtttggtaccgccgccacgcacggcagcaacgccgcgctctacaagaagctgccgttcgacgtggaggccgacttcgtgccggtggcgccggtgctcgacgtttcgaacgtgctcaccatcaacccggacgtgatcaacgcgcggacattgaaggagttcgtcgatctcgtcaaggccaaccccggcaagtacaactatgcgtctacaggcaacggcgcgggtacgcacatggcctttgccgaattcaattcgcgcctcggcctgagcatggtgcacgtgccctacaagggcggccccgaggccatcacgtcggtggtgcgcggcgagacctgctgcatcatgaaccaggtgcagacggtgctgccgcactacaaggccggcaaggtgcgcctcctgggcgtgaccaccgccaacccggtggccgccgtgaaagaggtgcccaccattgcctcgagcggcctcgcaggcaccaagggtttcgacagctcgatctggttcggcatcttcgcccccaagggcaccgatgcgcacatcgtcgacaagctcaacgccgccgtgaagacggtgctcgagcagcccgagatccgcgagcgcttcgaaagccagggcaacaccgtgcgcatcgagtcgcccgcgcagttcaagaagaccgtgcacgacaaccgcgtgaagtgggccgaagtggcgaagaccgcgaacatcagcatcgactgagggcgggaagtcccatccccgccgcctctgccgcatcgcatgcacgggagagctgcttacaaacaacaaagccgttgacagaaaggtcttggggcggattccggccgcgaggccgtatgctggcgtcgccgtcccgctgggcggcgaaagggcttgaattggacacagacctgggtctggaatgcaacccgaggctaccggcgggctgggcgttcgagcttcgtctgcaccgcgacgtggcgggcgacttgatcggcaccgggctgctccggttgcgtggcgtggacatgtgctacctcacgctggccagcctcgacagcgatcgcgccgaggccctgcggcgcatcaagagccgcgtcgaagcgtggctggccgaatggcattcccggtaagccggcgcaagcactgaagaaacggccctttcgggccgtttttttcttctcctcctgcaccctcgcggctcagagcccgtcgcggtccgagtcgccaggtacggcgcgttccactttgtcgctcacgcgctgccatgcgtcgcgcgttgcgtgcttggcgcgctcccactccagcgaagagcgcccacgggccgtgccccaatcgcggctcaattcgggctcgacgtcttcgaacctgcgattcgggtagcgcgaataggcatcgacaccgtagcggtacgcgggtgcatagtcgtcgtagctcgatccgcccgtcacgtaggaacgtccggcgtagttgtcgcgccagtacgcatcctcgacgtcgggatcgatctttgccatgcgccggccggccagggccccggctgctgcgccaactgccgcgcctatggcagcgcccacggggccggtcacgccgcccaccgccgcgcctgcggccgcgccgcccgccacaccaccgatagtgccgccgatcacggccccggcgccggtcgcagcgggatgcgaatcttccttgacgccgggcttgcgggtgtctttgagatcaaccattgaatgtctccttatcacgttgaagggaaaccaaagttgtactcactaccccgtggccgacagcgccaatgcgcttgtcggcatgaagggggcgggcggcacggcgtgacagtgcgcacctacagttgcgaccgccgatgccgcgtcggcgtggcttactacactcgccgcaatgagcccttccacgccaccgcagcaagccgtgcgggattgcctcgtctcctgtttccggagcggcgatgccatgcgcagccggagcgtgagcgacgtggtgctgtcgggagtggtggacgtgcccgtgccgcccgcgaggctggcggccgactgggaacgcgagatctcgtcgcacctgcgcctggagcccggagacgtcgaggcattgcccttggcgcgtgcgcgtgcgcgctggccggactacaagcgctgcgtacaggcggtggccgattggacgcgcacgctcggtctcggcgaggtgcttgcctccagcgacgtcgccctcatggcctgccgcggcgcgcggtaccaccacgacggcgcgcaatatggcgctgcggccttctgcaatctcttcgtgagcgaggacaaggggctggacgtgcactttccccacaccggccatcggattgctcttgcgcggggcacggtgctcgtcttcgacacgggccagcctcatgccgtggttcggcgcggcagtagcgagtttcgtgcggacgacttcgggcccgagcaggactgcagccagctgttcctgacctgggagtttcccatcgaagacgcccacgtggcgcgcgcgcttcaggtcgccttcgatgtcggcgcgccaacgtcggtgccgccgaatgaagagcaggtgtgggtgaacggcgaacgggccagcgtgtgcccggcgtccggccggtggcgccgggccggctgagcctggctggaacacgaagcataaagactgctgcctaaaaccccagcttgacaacggcttggcctgcgcccactgtcgcgcccagttgccatcttccgaagttgccgaacgcgacgagtcgccacgccacgaacctgatgaacacctggaccatacgacagcgcattcttgccagcttcgccgccgtgctggcactgatgatcgtcatgggcgctgtcgcctatgcctgcctcgcgcgcgtggcggaggacgcgaccatcatccagaaggatgccgtgccggggatggcggtcagcggtcagttgacggccgcctggctcgacaatttcgcgctcacgcagaagcacgttctcgaaaccgaggatgccgacatgcgccgtatcgttgcgcagttgcaggtcaaccgggccagtctcgagaagctgtcccgcaactatgaaaccaccatccataccgccaaggaccgggagaacttcgacgcattcctgaaccttcgcgcgccctatctgcgcgtgcaggacgacgttctgaggttgagcacggaaaacaagaactccgaggctcgcacgctgctgcacgaccagctcgatccgcagttcgcaaaaatccgtaccgccctccaggccgttgccgatttcaacacctcgaatggcgaggaggccgcccggcagatcatgggggatgtgacgactgccatcgtagccatcgtgatcagtcttgccgctggccttctgctcgcgctggtgctcggctacgcgctgctgcagtcgatcacccggccgctgggccgcttgctcacggccgccgatgcgatcagcaccggcgactttacccagcggctggacctggagcggcgcgacgagttcggctcgctggcgcaggggttcaatcgcatgacggagcaactgacggtgctgttcggccaggtgcagaagtccggcatccaggtcaacacctccgccaccgagattgccgccacgtccaaggagcagcaagccaccgccagcgagatcgccgccaccaccaccgagataggcgccacgtcgcgggagatttccgccacctcgcgcgagctggtgcggaccatgagcgaggtgtcggaggtggccgaggaaaccgccacgctggcgggcggtgggcaggaaggcctgctgcgcatgggcgagaccatgcacaaggtgatggaagccgtcgggtcgatcaatgccaagctcgcggtgctgagcgaaaaggccggcaacatcaaccaggtcgtcaccaccatcaccaaggtggcggaccagaccaacctgctgtcgctcaatgcggccatcgaggccgagaaggccggcgagttcgggcgcggctttggcgtggtcgcaaccgagatccgccggctcgccgaccagacggccgtggccacctacgacatcgagcagatggtcaaggagatccagtcggccgtgtcggccggcgtcatgggcatggacaagttttcggaggaggtgcgccgcggcatgcaggaggtgcagcaggtcggcacgcagctgtcgcagatcatcgcgcaggtgcaggcgctggcgccgcgtttcgtggcggtcagcgagggcgtgcaggcgcaggccaccggcgccgagcagatcagccaggcgctcacgcagttgagcgaagccgcccagcagaccgtcgattcgctgcgccagtccggccaggcgatcgacggcctgcacctggccgccggcggcctgcgcaacggagtctcgcgcttcaaactggcggaggcgtgaggcaagcgagggccggccagatgctgttcctcctctttcaactcggcactgaacgctacgcgctcgacgcgggccaggtcgtcgccgtgctgccgcggctcggcctgaaagagatcccccacgcgcccccggcggtggcgggcctgtgccactaccgcgggagcccggcgccggtgatcgacctcggccaactggcgctcggccgcccttgtgcgaaccgcctgagcacgcgcatcgtgctcgtccattttccggacccgagccacggcccccacctgctgggcctcctggccgaacgagcgaccgaaacgctgcggcgcgatgaaagcgacttcgttccggcgggcgtcagcatcgatgcggcgtcctacctgggcccggtcacggccgacgcgcgcgggttgatccagcgcatcgaggtgcagcacctgctgccgccgacgctgcaggcgctgctgttcaagaacgaggcgatgccagcgtgatcgacgtcgctccgttcgagcagctgctgaagcaggcgatgggcctggacgccgcctcgatcggctcggcggtcgtccggcgcgcggtgcaggagcggctggccgcctgccagctgccggacgcacaggcctactgggaacggctcggcagttccgcgcccgagctgcaggaactcatcgaggccgtggtcgttccggaaacctggttcttccgcgatccggcgtccttcgcggcgctggcgcgcctggttggcgaagacgcgcgtgccacgcaggggccgatggatctgcgcctgctgagcgtgccgtgcgcgacgggagaagagccttactcgatggccatggcgctgctggatgccggttttccggaaagcgcgctgcgcatcgacgccgtcgacatcagcacccgcgcgctggagcgggcgcagcgtgcggtgtacggccgcaactcgtttcgcggcagcgacctggcgttccgcgatcgctacttcgccgaaaccgcgggcggccacagccctgtggacgcggtgcgccggccggtgcgattccggcacggcaacctgctggagggcctcatggccgaggcggagctctacgacgtcatcttttgccgcaacgtgctgatctacttcgatcgcgccacgcaggatcgcgccatcgcggtgttgaagcggctgctcaagccgcgcggctggctgttcgtcggtccgtcggaaacggccttgctgtcggaccatggcttcatctccgcgaagcttccgctcgcgttcgccttccacaaggggccgccggccgtcggtgacgcgaagctgctgcgcgcggtgcatgcgccaaacacgcccgcgcgcaggccgacgccggtggtcgcggccccatttccacccgccgcccggcctcgactcgtccccgcgcctgccgcgacgccgcggcctgcggcgccggccgaagcgccgaccggcatcgaccgcgcgcgtcgtctggccgaccagggacacctggccgatgccgcggcacattgcgaggcgcacctgcgccagcacggtccttcggccgaggcgttccacctgctcggcctggtgcgcgacgcaagcggcaacgcggaagatgccgccgagcagtaccgcaaggcgctctacctggagcccgaccatcatgaagcgctgatccacctcgcgctgctgctgcgcaagcgcggcgacgaagccggtgcgcagcgcctgcagcggcgtgcgagccggctgcaccagggcggcggggcctgatcgatgaatgccgcaccgatgcttgccgaaggctccgcgcaggccgccatcgacgattgctggaatcgcatcggcgtgcagggcgacggcacctgcccgcaactcaggcagcacgtgcactgcaaccggtgtcccgtccatggcgccgccgcgctggccctgctggaccgggaggcgccgcccgactacctcgccgagtgcacgcgccacatggcacaggcgcccaaggccggccaggccgatgtgggctcggcgatcgtctttcgcatcgggaccgaatggttggccctgccgacgcaggtcttgctggaagttgcggccctgcctccgatccattcgctgcccgggcggcgcggaggcatcgtgcaaggcgtggccaacgttcgcggcgaactgctggtctgcgtgctgctcggcagcatgctgggcctggcgcgcgtcgccgaggccgggcacggacggcagcgcgaggtattgcggcgcctggtggtgattggtcttgacggccagcggctcggcttcgcggtcgacgagatgcacggtatcgcgcgcttcgatcccggcaccttgaaggaggtgccggccaccgtcgcccgcgccaccgccccttactcgaaggcgatcctcgcgtggcacgggcattcggtcggcctgctcgacgagcaattgctgttctacacacttcaccggagcctggcgtgaccgccaaggatctcagcgaactgtcgatgctggagttgttccgcgtcgaggtggagaaccaggcgcccatgctgacggaggggctgctcgccctggagcgggacccggaggccgccgatcagctcgaggcctgcatgcgcgccgcccattcgctcaagggcgccgcacgcatcgtcgacatcgccgccgcagtcggcgtggcccacgccatggaagactgcttcgtcgccgcgcaagagggcaggctgcgattgcgccagggccacatcgacctgctgctcggcggcgtggacctgctcgcgcgctttgcccattccccggagatggagcccctcgactcgccccaggtgaaggccttcgtcctggcgctggaaagtgcgatgcaggacgatggcaagagcgatccggcgccggacgcggcggtgccggcatccgaggaggctctcccgagggcgcctgccgccatggccgaaagcatcggctcggaccgcgtggtacgcgtcagcgccgacaacctgaaccggctgctcggcctggccggcgaatcgctggtggccgcgcgctggcttcggcctttcgccgactcgctgctgcggctcaagcggctgcagcacgaggccgttcaaaggctggaggcgctccacgatcacgccgccgtgccgatggcatctccggacgagcgcgcccggattgcactggacgagatcaagcggcgcgtcgtcgagtgcgagcagttgctggcggaggggctcgccgacgtggagacattcgagcggcgctcggccgacctgtcgcgccggctgtacgacgaggcggtggcctgccgcatgcggccctttgccgacggcgtccatgccacgccgcgcatgctgcgcgacctcggccgctcgctcggcaagcaggtccggctcgagatcgtcggtgccgcgacgccggtggaccgcgacgtgctcgagaggctggacgccccgctgggccacctgttgcgcaatgcgatcgaccacggcatcgagtcgcccgagcagcgccgtgccgcgggcaagcccgcggaaggcgtcgtccggctcgaagcgcgccacagcgccggtgcgctcgagatttccgtctccgacgatggacggggcatttccctcgatgccatgcgccgcgccgtggtcgagcgcaatcacaccaaggccgagcttgcggccgagctgtcggaggccgagctgctggagttcctgttcctgcccggcttcacgctcagcgaccgcgtcaccgacatgtcgggccgcggcgtcgggctggacgccgtgcaggacatggtgaagcaggtgcgcggcagcgtgcgcgtgtcgacagaggccgggcagggcacgcgtttccagctgcaattgccgctcacgctttcggtcatgcgcaccttgctcgcagacgtcggcggcgagccctatgcctttccgctggcccgcatcgtccgcgcctcgaaggtcgcgcccgggcaggtcgaactgctcgaaggccggcagcacatcgaggtcgacgggcggcgcatcgggctcgtgaccgcgcaccagatcctgcaggcggaggagtcccaggccgccggcggcgacctgtcggtggtcgtcatcggcgaccacggcgagacctatggcgtggtggtggaccgcttcctcggcgagcgcgaactcgtggtgcacgcgctcgatccgcgcctgggcaagatcaaggacatcagcgccggcgcgttgatggaagacggctcgccggtgctcatcatcgacgtcgaggacatgatccgctccgtgcagaagctcatcgcatccggccatctgagccaggcccagcctggcggccatgccgccgtcgatggaagaaggcgcaagcgcgtgctggtggtcgacgactcgctgacggtgcgcgaactcgaacgcaagctgcttgcgcagcatggctacgaggtcgaggttgccgtcgacggcatggacggctggaacgccgtgcgcaccggccacttcgacctgctggtgaccgacgtcgacatgccgcgcatggacggcatcgaactggtggccctggtcaagaagaaccccaacctgaagtccctgccggtcatgatcatgtcgtacaaggatcgcgccgaggatcaccgccgcgggctggaggccggcgccgaccactacctgaccaagggcagctttcacgacgagacgctgctccaggcggtggtcgacctgatcggcgaggccgtcgcatgaagatcgccatcgtcaacgacctgccgatggcggtggaggccctgcggcgcgtgctggcgctgcggcccgagcaccacgtggtctgggtggccgggaacggcgcagaggccgtgcagcgctgcgccgagctgaagccggacctcatcctcatggacctgctgatgcccgaaatggacggcgtcgaggccacgcgccgcatcatggccgcgacgccgtgcgccatcctgctcgtgaccgccgacatgggcgccaacaccgcccgcatctttgaggcgatgggccacggggcgctcgatgtggtcgatgcgccggccatcggcaacggcgatccgcgggccggcgctgcggccgtgctggcaaagatcgagatcatcgcccggctgatcggcgaccgcagcccgtccgctgtcggcggcgcgagggtggcagcagaacctggagcgcaccggccggaacgcctggtcgccatcggcgcgtcggcgggtgggccggcggcgctggccacgctgctgcgcgggctgccggccgactttccggtggccatcgtcatcgtccagcatgtcgacgagcagtttgccgccggcatggcgcactggctggcgcagcattcggcgctgccggtcgagctggcccgggagggcgatcggccatcgcccggcagggtgctgctggcggcgaccaacgaccatctgcggctggtcgcgcgcgagcggctcgcttacacgcgcgccccgcagagctatgtgtaccgcccgtcggtcgacgtgttctttcacagtgcctgcacgctgtggcgcggcgagatcgtcggggtgctgctgaccggcatggggcgcgacggtgcgcacggcctgaaagccttgcgcgacaagggccactacaccatcgcgcaggaccaggccagcagcgccgtctatggcatgcccaaggcggccgtcgcaatggatgcggcggtcgacgtgctgccgatcgaagcgattgcggcgcaactgtgcaatgttctttccacccagattgaacccggggggtcaccatgatcgaaaccgaatcgcaggacgacggcgtgccaagagcgcctactggcaaggtctaccgggtcatggtgctgctggtggacgaccaggcgatggtgggcgaggcggtgcggcgcgcgctgctgaatcagccgaacatggatttccactactgctccgatccggccgaagcgctcgcggtggccgagcaggtccgggcgacggtgattttgcaagacctggtcatgcccaccatcgacgggttgacgctggttcgcaggtaccgcgccaatccggccaccgcggagatacccattgtggtgctgtcgaccaaggaagacccggcggccaagggcgacgcctttgcggccggcgccaacgactatctcgtcaagctgccgagccaggtcgaactgatcgcgcgcatccgctaccactcgagggcgtacctgaatcagctggagcgcgacgaagcctatcgcgcactgcgcgagagccagcggcagctgatggaaaagaacatcgagctgcagcgcatgacccattcggacgggctcaccggggtctgcaaccggcgccgtttcgatgaatacatccaggaggaatggagccgggcgatgcgcgaccagagcgcgctctccgtgctcatgatcgacatcgacgacttcaagcaatacaacgacacctacggccacctggccggcgacgaggtcttgaagaaggtggcaaacaccttgcagctgaatgtcagccgatcgaccgatctcgtcgcccgcttcggcggcgaggagttcgcgctcatcatgaggaccacgccccacgagggcgctctcgccgtggccaggaggcttcgcatgtcggtggagggcatggggctggtgcacgggcgttcctcggtggccgggtacctgaccgtgagcatcggcggcgcatcgatggttccttcgcgcggcggctcctttctcgatctcatcgaagccgccgacaaggcgctctacgaggccaagcgagcgggcaagaaccaggaggcgatgtacgagggcgaggccgcagggtgacggctgcgccctggagcgtctatctgccggcgcttcgcggagctacggcaacagcttggcgacggcgtcggtgaacgacggaatgtcggtttgggtgtgggtcgccggatacgtcatctccgtgaccgacaagccctcatacccgcgcgccagcagccgcctgtacatcgcatcgacaggcgcgaagttgcactcgctcgggttgccgcaatgcgtgagaacgagcggtgcgggcaaaggcctgccgccgagcccgtcgtgcatttgctgctcgaggccttcgtactcggcctgctggaaggcgaaggcgctttcgaacgagaggaagtgcgagaacgtcaggttgcccgccgctccttcgagaaagagcgcaatgcccgccatgcttccgctcagcgagagcccggtcagcagacgcttttttacatcggcgcggtactttgtttcgatgaacggcaccagttcgagcgtcagaaagtcgtggtacggccgagcgccgggcagggtgtagtcctgctcgcgccgcgccgagccgccaatgccgaccagaatcgcttgcgtgccgcgcttgtcgaggatgtccttgaagttggcaaagcgcgagccgggcggattgaagatcgcgtcgccgtccatggcatagatgaccggatagctcgccgaaccgccgtcgtaggaggcgggcaggtagatgtcgagcggataggtggcgcccgtcttggccgaggtgatggtgtcggtcacgacgcggctggttgcgggaggcggctgttcagccggaggcgccggctcagcgggtgcgggcggtgcggccggaggaggagcggccggcgtatcggccggcggcgcggtgggcggcactgctgcaacaggcagcatggcgccgccgccaccacctccaccacccccgcaactcgacatgaccagcacaagtgcccagcttccagcaaatacgacaaacgcacgcccaagctgcatcggagttcctcgaaccttgcggtgtgaagaagaggctcatcgacgccatgccaaaaaagctgcgccggccgggtgcggcctcccttcattcaggatgccatggcacaccgaaattccggcgctgatcgaggtagatgaaaagcgcaaaagtcgtatcaggcccaagcgggcgagaggccggccggatcggtcagcggctcgccccgccggcgggcgcgcgtcgaccggctaccctgcgcgtctcgttttcctttccccactacaaagccgatgccagccccgcccgttgccgacaacaagcccgacgaagccgttcccgccgcctgggctcgcctgcgcgatatggtcgcggcgcgaacccctgcggacggccgcaccgatgcgctgtatccgggcctgcgctgctatcgcttctcgcgtccaatccgctacgagaaaacccagcgcctcgcgccgggcgtggtggtggttttgcagggccgcaagacggcgcacctcggcggcgaccgtcgctcactcgactacggcgccacgcagtgcctggtgctcggggccgaggtcgcgtgcctcggcacggttgttggggcgagcgcccaggagccgtacctcgccatccatctcgacctgccgcccgacgtgctggtcaaatccttcgtcgccttggcggaaagcggcacgctgatagctgagcccgaccgcgtgaccgagagcttcacggccccggtggggccggaggtggtcgaggccttcgcccgcctgctgctggcggccgacgacccggtggaccgccgcacgctcgcgccgctggcggtcgaagagatcgtgctgcggctgctgcgctccgaggccgcagccgccatccgcagcgcgggcgccgtcaccaaggcgggcgcacgcatacaggcggccatcgccttcatgcgccgccatctgggtcggccgctgtcggtggccgagatcgccggccatgtccacatgagcccatcgcacttcgcgcacagttttcgcgaggtggccggggtcacgccgatgcgctgcattcgagacttgcgcctggaagaggcgcgcatgctgatgctgggcaccgggctgcggccgggcgatgcggcggcgaaggtggggttcgagagcgcggcgcacttcaaccgcgcgttccgcaggcggttcgaggcaacgcccgcggagtacgtgcggcgcgtgcagtcgggctgatgccgacgcgcggctgctttcttctttcgcagccatggtcaatttcttcgcagcttcgcgccttggcgcgggaaagggggctggctaacctgccggcttccctttttcttttcaagccaacgcgaaatttccatggaccccatcaacgtcatcatcactttcgaagccaagcccgagggcgcctccgccttcgccgagctcatgcaccaggtcaagcagtcgctgccgtcggcggatggctgccggggcgtgcagctgttcgggcgcagcgacaacgcctgcgtgttcacgctggtcgagtcgtgggaatcgcagagccatcatcaggcccatatcgcgggggcggtggcgtcgggggcttgggatgcgctggcggcgcagctggcttgtgcgcctgtcagctgctattgcaaggagctttgagcctgtggcaggcgcgtcaccggatccagttttttaggaagttgcggcgaaacccattgctgtcgtaggtgggttccttgtagatcgggtgggctgctatgaccgcagtcaagataacgacatcggctcctcccacggcgtagccgcccgcaagcaggcccttggcgatgccttgcgcaatggttcgaatgggttgcggcccgaggggcggctttcccaatgcttcgaggtacatggcctcggcaatgtaggccgcagcttcgtcctcatggctcgaatggacgccggtgttctgcatgtccaggtgggcatgcgtgcattcgtgcaccaggtaggcctggtcgctggaattcgaaatcgagaagccgggcttgagatcgagcgtgtcgaagcccatgtagtagctggcgccagcgcccgatttcacggcaccggcaagcttgatggcctcgctgtcgatcgcatcggccacgtcgttctggtaggcgctcgggtacaccttgaaagacttgaaggcgaagttcagccggggaatggtggtgtcgcgcttcaggaagttgacgatgtccgatttgagtgtcatgcaagagccccccagtgaattgaagacaggccggaagtctggcgagtccagtccgctgcggctatatgtcgttggggggtgccgaggcataggccgccaggcggcacaggcaggcggacgagaaaccctcgcgacctgccaacgatgcacgaaagccgcgtttgcgcgcagcgggcactccgattgcagcgctacgattcactgcattcacgccaacaggaagggaagacaccatgcgcatccacccgcagcaccccggtttcatcttcacgcatgcgcgtggcgtcatggcggcggccctttgcgccgcttcgctcttcatggccggctgcgagaccaaaccgcgattccgcccgctcacctccgacgccccacccccgccggtcttcgtgaccgtgaccggcgatgccgattgccaggtggcccaggcgcgctatgcgctcggcagggccatcgacgcgccgctgctggaggaaatgcgcgcccgcaccggttccaggtcggcgcgcaccgcgccagccggcacgccattgccggcgccggccgatccggggcggctcaatgtcgacgtcgatccccagggccgaataatcggggctcgctgcggctgacggaattaacaataattccgcgatgacgaagacgaccatctccacccccatcgcgcttgactgctactacagtctttcctcgccctgggcctacctgggcggcccgcagctgcaagacatcgtgcggcgccaccatgtgcggctcacgctcaagccttacgactttcaggcggtggtgccccaaaccggcggcattccactgaagacgcggcccgagccgcgccgcacgtaccacgcgctcgaactggcgcgctggcgcgattacctgggcatgccgctgaacctggagccggcctactaccccaagggcgcgccggtcgatccgcactggaacaagtacccgggctggatggtgattgccgcccagctgcaggggctcgatgcgcagccgctctcgcacgcgctgctgcgtgccctgtgggccgaggagcgcgacacctccgaggccgaggtccgcatcgcggtggccgaagaaaacggctacgacggcgcgtcgctgcaggcgctggagcaggcggccgagacgctggcgacgtatcgcgccaacagcgcggaggccatcgaggcgggggtgttcggcgcacccacgttcatcctgaacggcgagcgtttctggggtcaggaccggctggtttttctggacagggccctggacaaactgcgcgcggcacgctgaagcggtcttgtagtgcggccgcgaggatcgaccgcactgcctcgatcgttgcggtagccgccgcgcgcatgttctgccgcggacctatcgaacacctcagaaatacgcacggttctacgcagccctggcctttctcatcggtttcatttaattgcaaacgggaagtttgcaattgatcgcattgcatcgccaagaatttcacggtgcggcctccttcgcatcagtgctcgcgttcggtccaccggtgcattgacgatttgccaactgatacttgaagtcagatcttcaacagcgtcatgcctcgtggcgagcggttgatgacgcccaacgaagaatggcgtgtgttcatgcatctcctggctcttgatctctttcgatccagcctgtccacaaggactggcagttcgcgcagattgtgaaatcacttatgaccgaattaccagaatcgccttcagcgcgtttgctcgacacccgttacggaaacgtcagcgtcccggccgggaagagtgatctgatcaccgattttctcgagcactatggagagtgggcgtcgcttgaagtggagtaccttgcgtcgttgctgccattgaaggcacgggtgctggacgtcggcgcctatgtgggcacgttcgggttgggtattgcgcaaacagcaaatgccgcattcatcgcaatggtcgagggcaatccggccatcgcgccacacctggcggcgaatgcgtcccggaatctgcgttgcacacacgaagtcctgaacgcgcttgtcgtcaattcggatgcgcctccggtcgagacagggtgggccgacgcggacaatgcaggatccgcatcgttcggagaaaaagcgagcggcgcggtccccgttccgctgcccgatacgacgatcaacttccgggcactcgtggagcgcttcggtccgcttgacctcatcaagctcgatgtcgaaggaatggaggcgcaactgctcgccgatcatccattgttgctgcatgacaagtccgtcttgctttggctcgaatgcaacgagacccgtggctctctcgccctcgcgcagacgctgatcgatgcgggacggccggtcacttactttgcatggccgtcgcacaacccggacaactatcggggcgtccagcgaaagatgtttccgtttgcctacgaagcgggtcttctgctcggcgcgcaagccacgcccctgacgccgcagcagcagcgcgccgggtgcctgatcaggagcattcatacagtcgaggacctgagagaggcgctgtggctcacgccgcggtgggctccaagggagtgggatgtgctcgaccgcaatgagatcgccgcaattgcgacgcatctctggctgggaaaaaagcgggagcgcttcttggccgaggccggaccgatgaccgggggctgcgcggaagaggccacggccaggcaggcgagcgcgaatccggacacgaacgctcgactcatcgcgttcagagatgccagggtcgccaagcttgaaagcaggttggccgaactcgtcagccagagcctcgaaatggagcgggcggaaagtttggcggttgctgccgccaacgccaacgaactgctcgcccgcgaactgaccagcaagttgcatgcattgcatcaggagcagctcgccgctctgacggcgcaactcgaagaatcccaggtattgcacgaacggcatggctccgtgcttgcaaggcaggttgccgtgctgctcgagcagaacaataccctttcgaatgccttgcatggcatccggagcagcctgacgtggcgaatcgcttcccggtcttcccgcctggctgaccatatccctctcctcaagcgggtcgccaaggggctgctgcgtcgcaaggtggctggggcgcagtcatgaccgagcccaacgaacaagagttcggcaccattgcgccgtttttcgatcgcggctactacctgtctcgatatcctgacgttgcgtcggcgaatgtcgatccggtctggcactactgcgtgttcggttggaaggagggccgggatccgtccgcggcattcgacacgagctactacctgcgcgagaaccgggatgtcgcggcagctggcatcaacccattcgcccacttcatcggaagcgggcgacacgaagatcgcaagcccgtaccagagatggccggcatgcgcaggcaactgctgaatgcctggagcgctgctgctgatcgctttggcgccgaagacggtgaacctgtgctgggtgcgccgcgtgacctcgatgtccacaccctcgtcgcggcgctcacatcgagcgcgagaaatggagaattcgtcatctccgtcagtcacgacgactatgcactcagcgttggcggcatccagaacatcatcggcgatgaactcgcggaattccgcgataggggcatcggctacctgcacctgtgttcggcccgcccgattcgatggcttgccgatgcgtcgagcgacgacttcgtctttgcgctgcgcctggatggcgaagcgctgggccgcgccaatggcgtgacgctgcagcaggcgtttaagcgcctcgcaacaaccggttcgcgggccatgtgggtgatccaccacctcatgagccattcgcccgaattgctcgagaagttgatcgcaaccaacagcgcgcggccgccgcttttctgggcgcatgactacttcgccctgtgtccgagctacacgctgctgcgaaacgacaccgcctactgcggcgcaccgctggtgaactcgacggcatgcgagatctgcgcctacggaaaggagcggccggttcaccaagagcgcatccaggcgttcctgcgcgcggtccggccttcgctggtcgcgccatcgcagtccgccttggaactatggcgccgtgcgagcggggtcgaggcgcctgatacgcatgtgctgcaacctgccaggctaacgcagtcgaatcgaatacgggccaaaggttccagaccgcgtttgcgcattgcttacctgggctcacaggtttttcacaagggctgggacacctaccagcgcctggcgggtgctttccaaactgatgaccggtatgaattcttccaactcggaacacccggtgccactccgtcgttcatccatcacataccggtcaaggtcgaagcatcggcacgtgatgccatggtgcacgcaatagccagacaagatatcgatgtggtgatctcctggagcatctggcccgaaactttctgcttcaccgcgcacgaggcgatggctggcggcgcgtttgtagtggccagacgcgagcagggccatgtgaatgcggccatccataggcatgcaccggaggcctcgcgcaatgtcgacgacgaagaagcgctgcaccgctatttccgcggcggagatgtcttgatcgatgtcgcacggtcgtcgcgccggcatggctgcctggtgccgtccctgggaagcgcggagttgctgcatcccgtctttgaagcagaggtacgtgcatgagagtcgcctgtttcacgagtgcttccttcagctatctcgaccgggcgagggtgctcttcgagactgttcggagatttcatcccgaatgggagaactggttttgcttggtcgatgaagagccggcgaatttcgtgttcgacatcgacgccgaagacatcgatcgagtggtgaagttggatgaattgggtgtcaaagagccgctcgcatgggctttcgagcacgatgtggtcgagctgtgcacggccgtaaagggcgcaatgctgtgccacatgctcgagcagggcatcgacaaggtcatctacctcgatcccgacattgccttgttcggatcgctcgacgaagtgctcaagctgctcgacgagcacagcgcggcgctcacgccgcaccagatcgatcccgacacggagcgctcagctatcgtagacaacgagatcggctcgctgaagtacggcatcttcaatctgggctttgttgcggtgcgcaatagcgcgccgggcagggccttcgcgcgttggtggcgcgatcggttgctggagttctgtttcgacgacattgaaaacggcttgttcaccgaccagaagtggtgcaaccacgcgcccgttttctttcccgagatcgccatattgcggcaccgcggctacaacgttgcgagctggaatctcagtcagcgccgcatccaaatttcaccggacggcaggatcaccgctggcggcgatccgttgaagttttttcacttcacaaaggtgacgcatgtcggtgaaaccatgttggcccggtatgcgggggggcgtccggaagtgttcgaactgatgcactggtacaaaagccgcctgaaggcccacttcgtcaaggacgttccgccgggatggtggcactacggaacctactcggacggccggccgatctcgaaagaggaccgtgccgctcaccggcgactgcggctgcggcagaagcatctggccaatccgttcgcggcctgaacctgctgcgacatcccctgaacccgaaaaacggccgcacgccgatcgcggtcccagcgctgtagcgggtttaacggcgccgggtcgtcaggtgcggtgccggtggcgataatcccccaatgcgaattcgcttcaccaagatgcagggggccggcaacgattttgtcgtgctcgacgaaacgcgcggctcgctgggcctcacggccgcgcaataccgctttctggccgaccgccacttcggtgtcggcgccgaccagatcctcacggtgcggccgccttccaagagcgcggccgagggcgtcgattttcagtacgtgatccacaacgccgacggcggtgaggtggagcagtgcggcaatggcgcgcgctgcttcatgcgcttcgtgcgcgagcaccacctgaccgagaaggagacggtgcgcgtcgaaacgctggccggcatcatcgaaccgcgcatgggcgaagacggccgggtcacggtcgacatgggcccgccgatcttcgagccggcccgcgtgcccttcgacaccgccgggctcgacccgcagcccacgggttcgtggcacacgtggcacctggcgcttggcacgcacgccgattcggccattgtttccgtggcggtgctgtcgatgggcaacccgcacgcggtgcagctggtcgacaacgtcgacaccgcgccggtggcccggcagggaccgcagatcgagcaccatccgcgttttccgcagcgggtgaatgccggcttcatgcaggtgatcgaccgcacgcacgtcaagctgcgggtgttcgagcgcggtgccggcgaaacgctggcctgcggcacgggcgcctgcgcggcggtggtggcgggcatccggctcggcctgctcgacaaccgggtcgacgtgcagacgcacggcggcgtgctcaccatcggctgggagggcgaggggaacccggtgctcatgaccgggccggccaccacggttttcgagggagacatcgaggtgcccgagctgccatgaccaccaacatcagaaacaacaaagacgacgccatgaacccgatcaccgaagacgacatcgccaactacctggcgaacacgcccgactttttcgagcggcatgcgcagttgctggcgcaggtgcagctcaccagcccgcacggcaaccgcgccgtcagcctgcaggagcgccaggccgaaatgctgcgcgaaaagatcaaggcgctggagcatcggctgatggacatggtgcgccacggcaccgagaacgtggtgattgccgaccgcctgcagcgctggactcgcggcctcttgaccacgcgcgacccgcgcagcctgccgtaccgcatcgcggtcgatctgcagtcgctgttcctggtgccgcagaccgccatcaaggtgtgggactgcggggccgactacctcaacgaggcctatgcccagtgggtgagcgacgacgtgaaggcgctggccacctcgctcacttcgccctattgcgggctcaattcgggcttcgaggcggccaactggctgcccgagccgaccggggccgcgtcgattgcgctgattccgctgcggcccgatgccgagtcgccggccttcggcctcctggtgctggcctcgcccgatgcacagcgcttcaacgccgaaatgggcaccgactttctcgagcgcattgccgaactggcctcgggcgcgctgtcgcggctgcggccttgagcgtccggcgccggccctggcgggccgcgcggcccgtgctgtggacggtgctggtggcaggcctgctggcctacctggccattgccgcggtcatctggcggcacgcggacgaggcacttgccaatccgccgcaacagccggccgatgccgcgctgatcctgggcaaccgcgcctacctcaagggcaagcccaacccgtgcctcacgggccgcgtcgacaccggcattgcgctggccaacgcaggccgcgtgaagcagctggtgctgtcgggcggcgtcgacaaggaagacggccgcatcgaagccgaggtgatggagcgccatgcgcgcgccgagggctatgccggtccgctgctgctggagccggcttccacgtcgacgcgcctgaacctggcgatgtcgcggccgatgctgaaggccgcgggcgtgcgcgccgtcatcgtggtgtcggagccctaccacctgtggcgcgtggagcgcctggtgcgggccagcggtttcgacaaggaattcgatgttcagtatgcggccgccgacacgagctgctggcgccgctggggcatggttttcaagggcgcgttgcgcgagccgctggctgtcgtgaacaatgcattcaatggctacctctactgagacggcggaaacggccgccacgccgccctgggtcgagaaatacctggagcacgtgcgcgtggagcgccggctggcggcgcgaacggtcgagctctatgccatccacctgcaagcgcttgcggccaacgcctcggacgccgggctctcgctcgaccgcgtgcagacggcgcacatccggcgctggatggcgcagctgcacagcgccgggcgcgagccgcgcggcattgcgctggtgctgtcgtgctggcgcagcttctaccgctggctcggcaacgaagggctggtgggcttcaacccggtgaaggacgtgcatgcgcccaaggccgcgcggccgctgcccaaggcgctggcagtcgacgacgcggtgcggctcgccgaaatgtacgaccccgaggccgacccctggaccgaggcgcgcgacggcgccatcgtcgaagtgctctacggctgcggcctgcgcgtgagcgagctcaccggcctcgacgcgcaagccagcaacacggcccgcggctgggtcgacctcgacgcgctggaagccaatgtgctcggcaagggcagcaagcggcgcctggtgccgatcggcggcaaggcggccgaagcgctgcgcgactggctcgcggtgcgcggcgaatgcccggcgctggcaacggcgggcctccgcgaccccgcgggcgcggcggcgctcttcatcaacagcaagggcgtgcggatgtcgtcgcaggcggtgtggaagctgttgcgcgagcgcagcctcaaggccggcctggcggcgccggtgcatccgcacatgctgcggcactcgtttgcgagccacgtgctccagtcgagcagcgacctgcgcgccgtgcaggagctgctgggccacgccaacatctccaccacgcagatctatacccggctggattttcagcacctggccaaggcctatgacgcggcacatccgcgcgcgcaggcgcgcccggaagaatcgcgcgccaagcccaaaaaagacgacatcgacaacaaatgaaaaccctccgcctcaagcccggcaaggagcgctcgctgcagcgccgccatccctggatcttcgaatccgccattgcacgcggcggtgccgattcgggcgagacggtgcgcgtcgaatcgcatgacggcgctttcctggcctgggctgcgttcagccccatttccaagatccgcgcgcgggcctggagctttgtcgaaacgcagcgcatcgacgcggcctttcttgcctcggtgtgcgcccgcgcggtggcggcccggtcgcttttcgacctgcagagcgacggtgtccggttggtccacggcgaggccgacgggctcccgggcctcatcgtcgaccgctacggcgacacgctggtggcgcagttcctgtcggccggcgtcgagcgctggaaggccgccattgccgatgcgctgctcgaagccaccggcctgcacaagctctacgagcgttccgacgccagcggccgcgagcgcgaaggcctgaaacccgtcacgggctggttgcgcggggagggcgccaccgaaatcacgatccgcgagcacggctggaagctctcgctcgacatcgcgaccgggcacaagaccggcttctacctcgaccagcgtgacagccgccagcgctttgccgagctggcggagcaccggcgctttcggcgcgtgctcaactgcttttgctacaccggcggcttcacggtggctgcgctcgcggggctgcaggcggcgggcgcgatggatggcgccgaactggtgtcggtcgattcgtcgcaaccggcgctcgaaaaggcacgggccaacctggcgctgaacggcttcggcggcgagggctcgggcgtgaagaccgagtttctggatgccaacgtcaacaccgtgctgcgcgagttcatcgaagagggccgcaccttcgacgccatcgtgctcgacccgcccaagtttgcgcccacggtggcccatgccgagcgcgccgcccgtgcctacaaggacatcaaccgtctcgcgctcaagctgctggagcccggcggcgtgctgctgactttttcctgctcgggcggcatcagcgcggacttgttccacaagatcgtggcttcggccggcatcgacgcccaagtggacggttacatcagcgaacgattgggcgcggcccccgaccacccgatgaccatcgagtttccggagggcgaatatttgaagggcctggtggtggtgcgaaagcccgcttgaccccgcgccaacgcaactgagtggcattggctaaactgccggccaattctttttcttcctgttttccgccttcggagcacaccatggcccttattcccgccaccatcctcaccggctttctgggctcgggcaagaccacgctgctcaagcgcatcctgacggaagcccacggccagaagatcgccgtgatcgagaacgagtttggcgaagagaacatcgacagcgacatcctcgtgaccgaatcgaaagagcagatcatccagatgagcaacggctgcgtctgctgcaccatccgtgaagacctgcgcgaagccctgcagctcctggccgccaagaagcgccagggcctgctcgacttcgaccgcgtggtgatcgagaccacgggcctcgccgatcccggccccgtggcgcagaccttcttcatggacgacgagattgccgagagctacctgctcgactccatcctgacgctggtcgatgccaagcacgcgccgcagcagctcaacgaccgccaggaagcgcgccgccaggtgggttttgccgaccagatcttcatcagcaagagcgagctggtgtcggccgaagaaaccgaggcgctgattcaccgcctgaagcacatgaacccgcgcgcgccgcagcagaaggcgcattttggcgatgtgccgctgaaagacatcttcgacctgcgcggcttcaacctgaacgccaagctggacatcgatcccgacttcctgaaggaagaagaggcgcacgaccatgaccatgcgcatggcgaaaattgcgaccatccctcgcacaagcacgaggggcatggccaccatcaccacaccgatgacgacgtgaagagcttcgtctacaaggccgaccgtccgttcgacccggccaagctcgaagacttcctgggcgccatcgtcaacatctacggcccgcgcatgctgcgctacaagggcgtgctgaacatgaagggcaccgagcgcaaggtgatcttccagggcgtgcaccagctgatgggcagcgacctgggcccggagtggggcaaggacgaggcacgccagagccgcatggtgttcatcggcatcgagctgccgcgcgaaatcctcgagcaaggcctggagcagtgcttggtctgaggctctgacttgctccttcccccgctgggggaaggttgggatgggggcgggccctcgatcgggcgccgcgcttttttgggaggccgtcgtgccccccaccccggccctcccccagagggggaggggggaggaacaccccggggcttacttgcccatgccgcccagcggcttgccgttgaccttcaggctgccttcgctgtactcgacctggctcgtgatgtcggtgccgtcgcgcttgacgaagcccatgccttcgccttgctcgaccagccccgccaccatctcgggcgggggcgtctggccgctctcggcgccggtggcggcaatctgctcgagccattgcatcggcagtcgcgcattggccttgagcacgccgcgcttcatcagcagcgccatgcccggcgcctgcaggtcttcgtcggtcacgccgaccatgccggccgtgtagctgatctcgccgcgcttgccgccgatttcgaccagcatcttgtccaggccgatctcggggttgtacttggccatggccttcaggtcgggcgccagctggtccatcagcgtctgcatggcggcttgcgacgccttggcgccgcccttgccgcagccattgatggcgctcgacttcagccaggcatcggccagcttcttgtagccggcggcgtgaatgcggcgcccgccgctgctcatctcgaacttgtcgatcttggtttcgccgatcttgccggcacccttgatcgtgccggtcgatgcgtagagcccgtccttgatgctggcatcggcaagcatgtcgatgttttgcaacagcacggtcggcagggccttgccctcggcgccttcggcggtgcccaggcccttgggggcggcaaattcgaagctttcgaggcggccttcggtcttgccggtggccaggatccagcccgcgctgctgtccatgtcggccttgccggtcagcttgcccatcttcatggtggcgccggtgcgcatgtcgctgacgtccagccccggcatggtcaggtcgtagtgcacctgggtgcgggcaccgttcacctcgatgcgggcttgcgcgccttgccaggtgaactgggccttgccttcgtcggtcaccttggccggcgccacggtcaggtcgctggtgtagccgccgtcgaacgccaccttggtgtgcgccgtcaggggcttggccttgccgaagagctgttcggccttggcctggcctttcacgtcgagcaccagttcgctgtcgatggtggctgcggccagcgtgccgcctgcaagcgggccgtggcggatggtgtcgcggaaggtgagccgcacgggcttgaacggcgtggcggcatcgtcgtcttcgtcgtcaccctcggcgggattgacggcgggcacctgcgccgcggcatcggctgcgcatccgagctcgagcgtcacggtgctcactgcgccgaaaaagccctgctcgtagctgcggttgaccacgcgtaccagcgcggtctgcttcggcagctcgtccagcgcggtgtcgtaactggactttatttttgtgccggcccaccaggtgctgccgccataggcaagcgcaatggcggctgccagcgcgcccaaaactgcttttttgctcacgatttcttctcttgtatgaattgttggtcgacccgcaccgtccctcggcggcttggcgggccttcgttgccccctccggcaacgctggcgatgctaccggaggcggcccggttgcaggcacatcccccttcatttcgagttctctatacaatcgcgcgcctgttccggcagccacgccctcgtccgaacgacgggatgtggcttacggcacggggcgccgcacgtttctggcgggctttcgggggtataaccccggggttcgtcactgcgagcactccgacgagtggagcccaggcggcctgaaacccgcaaaggctcccttgggaggagacacccagtgaaagcgcgttccagttcgttcaaggagccagtcaccgtgaagaaacccgccgccaaggccacgccagcaaccaagcccgccgctaaaaaagcggtggctgcaaagccggctgtaaccgcggcgaaaaaaatctcttccgctgcaaaagctccggccacgaaagaaaaaagcgctccaaagaagccagcaacgccatcggccaaggccgcgaccgttgcaaagcccgtcaagcctgcaaagtccgttgcggcgccggtggcatccgccccggccaagagtgcaaccaaaactgcagttgcgggtctaccgccatccaaaaccgtcggccgcactgctgccgttccttctgcccctccgatcccaatgaaaaaaacggctgccgcctcttcttccgccacggcgacaccttcgatgcccgttcagaccgctgcacccgcgcccgcgcgaggtggccgcgtgtcccggctgtcgcagctgaccgtgccttccatgccgcaatcggtggcttcgaccgctgccaagtcttcgttctcgcaggcgccctccaatgcgctggtgccgccgccgcccgtggcggtgaaaaaagacccgaagctcgccaacaactggaaaaccaagtcggtcgacgagttgagcgacgccgaagtcatcgcgatgcccgacaccgagtacatgaacgaaaagcagatggcgttcttccgcctgaagctggtcgaactcaagcgcggcatcctcgaaaacgccggcgaaaccaccgagcacctgcgtgaagacaccgtggtggtgcccgatccggccgaccgcgccaccatcgaggaagagcacgccctcgagctgcgcacgcgcgaccgcgagcgcaagctgctgaagaaaatcgagcagtcgatccagcgcatcgacgccggcgactacggctattgcgacgaaaccggcgagcccatcggtgtcggccgcctgctggcccgacccaccgccacgctgtcgctcgaagcgcagcagcgccgcgaactcaagcagaagatgttcggggactgagccggcaacacaaaaaaagagagaacctgatcgcctcgaagtttttgtcgatgccaaaggaagagtcgggccgcctgttttcgaaggtggcgaagttcgtccgcaatccgctcaaggattggtcggagctgaatgcgaccgccgattccacgctgcccgtggaccaggcctacagccgggaaatgctcaaggagatgatcgagcggcgccagcgcaacgatttcgttcgccggcgcgagttcgacatgctccgcaagctgcgccagcgtgaagcggccgcccacgccttcgaaggaacggtcacaccgtcttccttcaacctgaacagcaccaccgaaaaatcggagggtcgcgccctcacgctcaagaagatcgacgagatcgaagagcagatgtcgcagcagtggtggaagggccgcggccccaacggcgaggtgctggccaatgagccccccgacgccggcgccgaaaccctgccgccgccggtggatgcggccgagctggccagcttgctcgggacgccttctggccgtgcggcgccggcacctgcaccagcgcctgcgcctgcgccggtatccacgcctgcgcccgccgccgccgtggcgccagcttcggctcccgcccctgtcgggcctgggcctgccagcgccgaggtgagcgtcccctcgctgctgtcggcgcggctggcgcgagacggcgcgctcgaagaggccgtgatccgcttcgcgcacggcgacgatgccggtgccgaggccattcttctgcaggcgctggcctcggagagtgtggcggtcgggggtgaaggcgaccacgccaccgccgagcgcgacgacgcgcgctggcatgccttgttcgacctgtatcgcgccaccggcgacgccacccgctttgccaccgcccgcatgcgctatgcgcaacgcatgaagcgcatgggcccggactgggtgccgctcgatgaactggcgcgcaacgtgaaggccgtggtggccagtgaatacgccgaactggcgccggccggcgccgactggaccagcccgccacgcctggcgcgcgacggattgatgaatctcacgcgggcgctgtccaaggccggttcggtctggacgctcgactggcgtgcgctggccgccatcgagcgcgatgccgctgcgccgctgcgcgtgctgttcgcgcactgggccgattcgccggtgcaactgcgtttcatcggtgccgccaagttgcaggccgtgctggccgaggccacgcccaacaacgagcgcagtaccgaagacgtctggtggcagctgcatctggcggcgctgcgcatgatgaacatgcccgacgatttcgagctggtggcgctcaactactgcatcaccttcgaagtctcgccgcccgcctggcaagacccgaagggggaatgcgccttgctggctccccccgagggaagccgctcgggcgccggctccgtgtggtcgctgttgtcggtcggcggcgaatcggagagctttccgtccaccgacagcggctttgcggcactggcgggcgatttgcgcggagaaacgcattcgagcctgcagcggctcgacaccgacctgcgcaacacgacggcgcctgtcatttcgtgtgccgcactgctgcgcatggaccttgccgccgccggcacgctgctgagctgggtgcgggcgcgggacgcccagggcgaccgggtccagttcgtcgatgcgcaccggctgattgcggcgctgttcgacatcgtcggcattgccgaccacgcgaccgtggcgctccgaaagaactaggcccaatccagagcaaagcgcggggttgtattggccccggccatccccagatggcttcgatggaacagtttcacggcaccaccatcgtgagcgtgcgccgcaagaccccccaaggcgatcaggtcgccattggcggggacgggcaggtcactctcggcaatatcgtcatcaagggcacggcgcgcaaagtgcggcggctctatcacggcaaggtgctggctggctttgccggcgccacggccgacgccttcacgctcttcgagcgcttcgaggccaagctcgaaaagcaccagggccacctgacccgcgccgccgtcgagctcacgaaagactggcgcaccgaccgggtgctgcgcaagctcgaggccatgctggccgtggccgacgccaccacctcgctcatcatcaccggcaacggcgacgtgctggagcccgaagacggcgtgatcgccatcggttcgggcggcgcctatgcgcagtccgcggccaaggcgctgatcgacaataccgatctcacggcggagcagattgtgcgcaaatcgctcgcgatagccggcgaaatctgcatttacacgaacatgaaccacaccgtggaagcgctctgaccatgtccatgaccccccaggaaatcgtctccgagcttgacaaccacatcgtcggccagcccgccgccaagcgcgccgtggccattgcgctgcgcaaccgatggcgccgccagcaggtcgaagaaaagcttcgcgccgagatcacgcccaagaacatcctcatgatcggccccacgggcgtgggcaagaccgagatcgcgcgccgcctggcacgcctggcggatgcgccgttcatcaaggtcgaggcgaccaagttcaccgaggtgggctatgtcggcaaggacgtcgactcgatcattcgcgacctggccgagattgccgtcaagcagacgcgcgaagccgaaagcgccaaggtgcgcgcccgtgccgaggacgccgccgaagaccgcatcctcgacgtgctgctgccccccgcgcgcggcgccgatggcaccacgccggcgctcgatggccccaaccccactcggcaggccttccgcaagaagctgcgggagcaccagctcgacgacaaggagatcgagctcgacctggccgaaacccgtgccccgctcgagatcatgggcccggcgggcatggaggaaatgaccgagcagctgcgcggcatgttcggccaactgggcggcggcaagcgcaagacgcgcaagctcaaaatcgccgaggccatgcgcctcctgatcgacgaggaagccgccaagctggtcaacgaggacgagatccgcatgcaggccatcaccaatgccgagcagaacggcatcgtcttcatcgacgagatcgacaaggtggccacgcgcagcgaagcccagggctccgacgtgtcgcgccagggcgtgcagcgcgacctgctgccgctggtcgagggcacggccgtgagcaccaagtacggcgtggtgcgcaccgaccacatactgttcatcgcgagcggcgcgttccacctcagcaagccgagcgacctgattcccgagatgcaggggcgctttccgatccgcgtggagctgcaatcgctctcggtgtcggacttcgaaagcatcctcacgcagacccgcgcgtcgctcgtgaagcagtaccaggcgctgctcgcgaccgaaggcgtgacgctcgaattcacgcccgaaggcgtcaaccgcctcgcggccattgccttcgaggtgaacgagcgcaccgaaaacatcggcgcccgccgcttgtccaccgtgatggagcgtctgctcgatgaggtaagcttcgacgcagcgcgcatcgaaggacagaccatccgcatcgatgccgcctacgtcgacgagcgccttgcggcactaagtcacgacgaagacctttcgcgcttcatcctctgaagctgctttgcggcccctgtaacggggccgcgcttcacgcatcacattcactgcgtgagctaagtgcttcattctcaacgaaattcaccggtttccaggtttggaaatcggcgctaagtcgttgattccattacaaaaaataccaccaacgaccagttgcgcctgaagtgtttcctgctacagtgcaaaaaagtgcagttaagtgggaaaaagtgcgggtggtgcctctttcgggtgctgcggcgctcccaacacaggggttctggtcgtgtttcaaggcgcttcatcgctcagtctggatgccaaggggcggctctccgtgccgacccggcatcgtgacgtcctgagcgcgacggcgaacggccaactcacgatcaccaagcatccgcacggctgcctgatggtgttcccgcgtcccgagtgggagaaattccgcgagcgcatcgccgcgctcccaatgtcggcacagtggtggaagcgcgtattcctcggcaatgcgatggacgtcgagatggacggcaccggccgcatcctcgtttcgcccgaattgcgtgcggccacgggcatcacgcgcgagacgttgttgctgggcatgggcaatcatttcgagctctgggacaaggccagctacgaagccaaggaggccgaggccacccagggcgagatgcccgatgtgtttcaggacttcgcgttctgaggactcgtgtgaacactccatggatccataccaccgtgttgctgaacgaagcggtggaagcccttctttcaggcagcgccgcggccacgggcacctacgtggatgcgaccttcgggcgcggagggcatgcgcgcgcgatcctcgcgaggctggcaccggaaggcaggctgatcgcattcgacaaggatgcggaagcagtggccgaagcagcgcgcatctcggatgcgcgtttttccatccggcaccagggattccgttcgctgggcgaattgcccgatgccagcgtggcgggtgtgctgatggacctgggcgtgagttcgccgcaaatcgacaacccggtgcgcggcttcagttttcgattcgacggcccgctcgacatgcgcatggacaccacgcgcggcgagagcgtggccgattggctggcaacagccgaacttcagcagattgcagaggtgatccgtgactatggcgaagaacggtttgctgttcagattgcaaaggcgattgttgctcgcagacaagaacggggcgcaatttcaaccaccaccgaactggccgagctcgtggctggcacggtcaaaacccgcgagcagggccagaaccctgcaacgcgcacatttcaggcttttcggattttcatcaacgccgagcttgaagagctgcaacaggcgctagaggcgagcctctccgtgctgcagcccgggggccggctcgcggtgatcagcttccactcgctggaagaccgcatcgtgaagcagttcatcgccaagcattcgaaggaggtgtacgaccgccgcgcgccgttcgccgccccgaaggtgatgaagctgcgcgcgctcgagcgcatcaagccttcggccgaagaggtgaaaggcaacccgcgctcgcgcagcgccatcttgcgcgtggcagagcgcacggaagctgcttgacatggcacgcctcaacctgctcctgatgctcgcggtggtcgcctccgcgctctacctcgtgcacacgcaatacctgtcgcggcagctctataccgagctcgaccgctcgcagcaggaggcgcgccggctcgaactcgaccgcgaccggctgcaggtggagaaacgcgcccaggccacgcccctgcgggtggaaaagctcgccaaggagcagctccagatgcgcaccaccacgccggccatcacgcagtacgtgcggcccgacggctcggtgattccggccgtggtggcgccgccgcccgccccgccggcgggtccggcgaccaagcccgccgcgagggcccagcgatgagccgccgcagcgtccgctacaccaccagccccttgctcgcgagcaagacgccggtctggcgcagcaagttcatcgtcgcgggcattgccttcggcttcgtcgtgctggcgggccgggctgcgtacgtgcaggtcttcaacaacagtttcttccagcggcagggcgaggtgcgctttgcgcgcacgctcgagctgccggccaaccgcgggcgcatcctcgaccgcaacgggctcatcctggcctcgagcgtggtggcgccgagcatctgggccattccggaagacgtcgaacgcgacgaccccgaagtccgcgccaagctcaagcaggtggccaagctgctcgaaatgccgcagaaggacttcgacaagaagctcgaggacgaggacaagaccttcgtctggatcaagcgccaggtcgacgagcccattgccaagcagattgccgcgctcaacctcaagggcatctaccagcgcaaggaatacaagcgccagtacccggagggcgaggccgcggcgcacgtggtgggcttcaccaacgtcgaggacaacgggcaggaaggcatcgagctgtccttcaacaaggacctggccggcaaggccgggtcgcgccgcgtcatcaaggaccggctgggccgcgtggtcgagggcgtgggcgaacaggtgccgccggtcgacggcaaggacatccagctcagtgtcgacagcaaggtgcagttcttcgcctaccagaagctgcgcgacgccgtgaccgcgcgcaaggccaaggccggcagcgtggtggtgctcgacgcggtcaccggcgaagtgctggcgctggccaactacccgagctacgtgccggacaagcgccagaacctcaccggcgagcagctgcgcaaccgcgcgctcaccgacaccttcgagcccggctccaccatgaagccgatcaccgtcgccatggcgctggaagcgggccgcgtgaagccctcgaccctgatcgagaccggaccgggccgctatcagatgggcggcttcaccatcagcgacacccacaactacggcacgctgacggtcgagggcgttatccagaaatcgagcaacgtgggcgcgctcaagatcgcgcagaagatgtctccgcacgagatgtgggacacctacaccgcgctcggctacggccagaagccgcagctccagtttcccggcgccgtgagcggccggctgcggccctggaagacctggaagccggtggagcaggccaccatggcctacggctacggcctgtcggcgtcgctgtttcaaatggcacattcgtacaccgcctttgcgcacgacggcgccatcattcccgtcaccatcctcaagaattcagagccgcccgccggcgtgcgggtgttctcgccgtcgaatgcgctggcggtccgcaagatgctgcagatggccgccgggccgggcggcaccggcacgcgcgcgcagaccatcggctactcggtgggcggcaagtcgggcacggcgcacaagcaggtcggcaagggctatgcaagcaacaagtaccgggcctggttcaccggcatggcaccgatcgagaagccgcggatcatcgtggccgtgatgatcgacgagccgagcgacggccagtatttcggcggcgtggccgccgcgccggtattcagcgaagtcgtgcagcagaccctgcgcatgatgaacgttccgcccgatctcgccgtcaaaccgctggtgatgacgcaaggcgtcgacgagagcttctgagcatgctgacactcacttctccccaactcgccgcgctctggctcaaggagcgcgtgcagggtgcgctgcatgcggacagccggccggtgggcgctggcgacggcttcattgcgtggcccggtgccgccactgacggacgcaagcacgtggcttccgcgctggcgcagggcgcggcggcctgcctggtcgagcacgacggcgtcgaggctttcgacttccacggcgacgaccgcattgcaagctaccccggcctcaaggccgccaccggcccgatcgcctcggctttttacgacaacccgtcggccgcgctcgaggtgctggccgtgaccggcaccaatggcaagacctccaccgcctggtggctcgccgaatcgctttccacgctggccgtgcccggcggcgttcgcccgttgcagccggacggttcgaccgagcgctgcgtaccgtcgccgtgcgcggtcatgggcacgctgggcatcggcgtgccgccggagctcacctacaccggcctcaccacgcccgacccggtgatgatgcagcgcgaactgcgctccctggtcgagcgcggtttcggcgcctgcgccatcgaggcctcgtcgatcggcattgccgaacgccggctcgacggcgcgcgcatcgcggtggccgtgttcaccaatttcacgcaggaccacctcgactaccacggcagcatggaagcctactggcaagccaaggccgagctgttccgctggcccggcctccgcgccgcggtcatcaacatcgacgatgtgcatggcgccagcctgtgcgcgaacctcatcgaagccggcatcggtgccctcgacgtctggaccgtctcggcggcaggcagccccgcgcggctgatggcgcgggacgtcggctatggcgcgcagggcctgcagttctccgtggtcgaacacggcgtcccgggcgtggagcgcatctcgaccggcctgatcggacagtacaacgtggccaacctgctgggcgtgctcggcacactgcgggcgctggggctttcgctggcgcgggccgtggcggcctgtgccaacctcaccagcgtgcccggccgcatggagcgcgtgggcaccggcatcggtatgccgctggcggtggtggactacgcccacacacccgacgcgatcgacaaggcgctggcgggcctgcgccccctggcgcggcagcgtggcggcgcactctggtgcctgttcggctgcggcggcgaccgcgatccgatcaagcgcccgatgatggcggccgtggccgagcgccaggccgatcgcgtcatcgtgaccagcgacaacccgcgcagcgaaaaccccgacgcgatcatcagccagatgctgctcggcctcgcgcgccccgaggcggcccaggtgcagcccgaccgcgccgccgccattgccgacgccattgcgcaggctgcgcccgaagacgtggtgctcatcgccggcaagggccatgaagcctggcaggaaattgccggacagcgcatcccgttttcggaccggacccatgcgctcgaagcgctcgcgaatcgaggtggggcatgaaccaatcgacgccactcatgctgaccctggcccaggtgcagcaatggattcccggtgcgcgcctggtgggcgagcccaccacgctcatcacccgcgttcacaccgacacgcgaacgctcgccaatggcgacctgttcgtggcgctcaagggcgaacgcttcgacgccaacgaatttctggccgatgccaaggcgcgcggcgccgttgcggccattgcgcaccacggcctgcaggaagcgggcctcgcggggctcgaggtgcccgactcgctggccgcactcggtgcgctggccgcgggctggcgcgcgcagttcgacctgccgctgatcgcggtcacgggcagcaacggcaagaccacggtcacgcagatgatcgcggccattctggtcgcgttccgggccgaccgcgcgctggcgacggccggcaacttcaacaacgagatcggtgttccgctcaccctgctgcggctgcgcgcgaagcaccagcatgcggtggtcgagctgggcatgaaccacccaggcgagattgcccggctggccgccattgcatgcccgaccatcgcgctggtcaacaacgcgcagcgcgagcacctggagttcatggacaccgtggaagcagtggcccgcgagaacggcgcggtgtttgcctctttgccggaggacggcacggccgtgtttccgcacggcgacgttttcacttcgctgtggaacgacatggcgcattccggcgcgatgcgacgctgcatgacattcggcgagcaggcagacgccgacatttcgctggtacgggccgaatggcagcacggcgcgtgggaagtccgcattcacacgccgctgggcaactgcgatgcgcgtttgcacattgcgggccggcacaacgtggtcaacgcattggcggccaccgcgtgcgcgctcgctgcgggcgtttcgctcgaaaccatcggcgcgggcctcacggctttcgagccggtgaaaggccgctccaaggcgagcgaggtggtgctggtgggcgggcatgcgctcacgctggtggacgacagctacaacgccaaccccgattccgtgcgcgccgccatcgacgtgctcgcggccctgccgggcccgcgcctgctggtgctcggcgacatgggcgaggtcggcaaccgcggacccgaattccatgccgaggtcggcgactgggcacgccagcgcggcatcgaggcgctgtacggcctgggcgccgaaaccgcgcatggcgtggccgctttcaacggcgctggcaacggccgccatttcgacaacgtggatgcgctcaacgccgcggtgctggcgcggctgccgcaggttgccagcgtgctcgtcaagggatcgcgcttcatgaagatggagcgggtggtgcaagccatcgagcaatcacaacaacaaaaggaggccggtcatgacgcatgagccgtgcaagacaacatgctgatgagcctggcccaatggctgcaaacactttcgcccgaattcgggttcttgcgcgtttttcagtacctcacgttccgtgcgctgatggccgcgctcacggcgctggtggtcggcctcgtggccggcccctatgtgatccgccgccttgccgcgctcaagatcggccagccggtgcgcggctacggcatggaaacgcacctgaccaagagcggtacgcccaccatgggcggcgtgctggtgctgtttgccatcgcctttgccaccgtgctgtggttcgacgcttcgaaccgcttcgtctggatcgtgctgtgggtgacgctgggcttcggcgccatcggctgggtcgacgactggcgcaaggtggtgcgcaaggacccggaaggcatgcgctcgcgcgagaagtatttctggcagtcggtggtcggcctgatcgcgggcttctacctgctcttcagcatctcggaaagttcgaactggcgcgtgctgcagctgttcttcgcctgggtgcagtcgggcttcgatctcgactttccgcccaagatcaacctgctggtgcccttcttcaaggaggtgagctatccgctcggcggcatcggcttcgtgatcctgacctacctggtgatcgtgggcgcgagcaatgcggtcaacctgaccgacggcctcgacgggctggcgatcatgccggtggtgatggtgggctcggcgctgggcgtgttcgcctacgtcacgggcagcgccgtgtattccaagtacctgctgttccccaacatcccgggttcgggcgaactgctggtgttctgctcggccatggccggcgcgggcctggcctttctctggttcaacacccatccggcgcaggtcttcatgggcgacgtgggcgcgctcgcgctgggcggcgcgctgggcaccatcgcggtcatcgtgcgccaggagatcgtgttcttcatcatgggcggcatcttcgtggtcgaggcgatctcggtgatggcgcaggtcatgtacttcaagtacaccaagaagcgctacggcgaaggccgccgcgtgctcaagatggcaccgctgcaccaccacttcgagaaaagcggctggcgcgagacgcaggtcgtggtgcgcttctggatcatcacgatgctgctgtgcctcgtgggcctttcaacgctgaagctgcggtaacaggcacatgcgtcatctgaaagacctccccgtcctcgtcctcggcctcggtgcgtccgggctggcgatggcgcgctggtgcgcacgccacggcgcgcaggtgaccgtggccgacacgcgcgaggcgccccccgcactcgccacgctgcaggccgagctgcccgaggtcgctttcatcggcggtccgttctcggccgcgctgatcgaaggcacgccgatccgcgcggtgtaccgctcgccgggcctgtcgcccgcgaccatcgcgccggtggtcgatgcggcacgggccgtgggcctcgcggtcggcggcgaactggatctcttcgcacatgcgctgcgggatctgcaggccgtcgagctgccggcggtggaagcggagcccgaggctgaagccgctgcggaagctgtcgagccagaggcgcaggccgagttggacctggacgtcgaagctgcggaagctgcacaggccgagcctgagcaggccgacgcggtcgagccgaccccggtgcctgagtcgattgaagctggcgagcatgcctcggcagctgaaacacctgaagcagtcgagcccccgccaacggccgagccgaccgaggccgaacccgcgccccccgccatggcggaagccatgccgcgtgatccttcgctgagcgttccggtggcgcagcctgcggaagaagcgccggccgcaccgtcggcagagacgccagaaaacccggaagccgcagcgcccgcgcccgccaccgtttcgcgcctgccgagcaccggcaagccttacgttcctaccgcggccagggaagcggccgagttcgtcgccaagattgccgagctctctgcctccaacccggcctccgcggccgtcgaggaagagcccacgccccagctcccgctggtgccgatcgaggaaccgccggcgccaaagggctacacgcccgcggtgctcgccgtcacggggaccaatggcaagaccaccgtcaccgcgctgaccggccagctggtcgagcgcgccggcaagagcgtggccgtggcgggcaacatcggccccacgctgctcgacacgctggccgcgcacatcgacgcccagacgctgcccgatgtctgggtgctcgaactctcgagcttccagctcgacggcgtgcagggcttcgagccgaccgccgcgacggtcctcaacctcacgcaggaccatctcgactggcatggcgacatgccgtcgtatgcatcggccaaggcacgcatcttcggctccaaggggctcatggtgctcaaccgcgacgacccgggcgtgatggcgatgttgcctccgcccatcaaggtgaagctgcagcgcccgcagatccgtgcgcacatcaccttcggcagcgcgatgccgctgcgtcccggcgactacggcatcgagcgcgtcaacggcatgacctggctggtgcgcgcgctggaagccgacgagacgcagaagcgcaagcgcggcgccgtggtcgaagaggagatcttcctgcagcgcctgttgcccgccgatgcgctgcgcatccgcgggcgccacaacgccatgaacgcattggcagcgctcgcgctggccagcgccgccgattgcccgctcggtcccatgctctacggcctgcgcgaataccgcggcgagccgcatcgcgtcgagccgatcgcgctggtggacgatgtcgaatacttcgacgacagcaagggcaccaacgtgggcgccacggtggccgcattgagcggccttggcgaagaccgccgcgtggtcgtcatcctgggcggcgaaggcaaggggcaagatttcgagccgctcgccgatcccgtgcaccgctgcgcgcgcgccgtggtgctcatcggccgcgatgcgccgctgatcgaacaggccctggccgccaccggcgtctcgctgatgcatgccggctcgatggaagaagccgtcaagctcgcggccgcgcgcgccaaccctggcgatgccgtgctgctgtcaccggcctgtgcgagcttcgacatgttcaaggactacgaacatcgcgcggccgtgttccgcgaggccgtgcaggcgcttgcggacgatccgcatgaagccgcctcgtccaacgatgccgacttttcttcgggagacccggtttgaacaccgcagccgccggcgccacgcccaatgcaaagaccagccgcttcggtggctggttcaagcgcgcgcgcagcggcatcgattcgctgcctgtgcacctgccggtgcggctgggcggcgccggcatcacgcagaccaaggccgcgccgatgcgcgtgctgggcttcgaccaggcgctggtgtgggtcaccgtcgcgctgctcacctggggcctggtgatggtgtattcggcctcgatcgcgctgcccgacaacccacgcttcgcgcgcgccggctacagcgcctcgttctttctcacccggcatgcggcctcggtggcgttcgcgttcatcgcggcgctgctcgccttccagatcccgatgaagacatgggagcgcgccgcgccctggctcttcgtcgcctcgctgctgctcctggtggcggtgctcattccgcacgtcggcatcaacgtgaacggtgcgcggcgctggctgccgctcggcttcatgcgcttccagccgtcggagctggccaagctcgcgatggtgctctacgccgccagctacatggtgcgcaagatggagatcaaggagcgcttcttccgcgccgtgctgccgatgggcatcgcggtggtggtggtgggcatgctggtgatggccgagcccgacatgggcgccttcatggtgattgccgtgatcgccatgggcatcctgttcctgggcggcgtgaacgcgcgcatgttcttcgtgattgccgcgctggtggtggtggccttcggcaccatcgtcgcgaccagcccatggcggcgcgagcgcatctttgcgtatctcgatccgtggagcgaagagcatgcgctgggcaagggctaccagctctcgcactcgctgatcgccatcggccgcggcgagatcttcggcgtgggcctgggcggcagcgtcgagaagctgcactggctgcccgaggcgcacaccgactttctgctggccgtgatcggcgaagagttcggcctcgtcggcgtgctgctgatcatcggcatgttcctctggctgacccgccgcatcatgcacatcggccgccaggcgattgcgctcgaccgcgtgttctcgggtctcgtcgcccagggcgtgggcgtgtggatcggtttccaggccttcatcaacatgggcgtgaaccttggcgcactgccgaccaaggggctgaccttgccgctgatgagcttcggcggttcggccatcctgatgaacctggtggcgctggctgtcgtgctccgtatcgactacgagaaccgcgtgctgatgcggggaggtcgcgtatgacgcggaccgcactcgtgatggctggcggaaccggtggtcacatcttccccggccttgccgtggccgaggcgctgcgcgaccgcggctggcgcgtgcactggctgggcgcgcccggcagcatggaagaaaagctggtgccgccgcgcggcttcgcgttcgagccggtgcagttcggcggcgtgcgtggcaaaggtccgctcacgctgttcctgctgccgctgaagctgctgcgtgccttctggcagagcctgcgcgtggtgcgccgtgtgaagccagacgtgctggtgggcctgggcggctacatcacctttccgggcggcatgatgggcgtgctgctcaacaagccgctggtgctgcacgaacagaactcggtggccgggcttgccaacaaggtgctggcaggcgtggccgatcgcgtgttcacggcctttcccaacgtgctcaagaaggcgcagtgggtgggcaatccactgcgcgcggcgttcacctcgcaacccgatccggccgtgcgcttcgctggccgcaccgggccgctcaagttgctggtggtgggcggcagcctcggcgcgcgcggcctcaacaccgtggtgccgcaggcgctcgcgcgcatcgagccgggcacgcgtccgcacgtgctgcaccagagcggcgccaagcagatcgatgaactgcgcgccaactacgcggcggccggtgtcgaaggcgagctcacgccgttcatcgaagacaccgcgcaggcctacgccgacgccgacatcatcgtcgcgcgcgccggggccagcaccgtcacagaaatcgcggccgtcggcgcagcagcgctgttcgtgccttttccctcggcggtcgacgaccaccagaccaccaacgcgcgcttcctcgtcgacgcgggcggtggctggctggtgcagcagaccgacctcacacctgaattgctggctgacttgctacagaaaaccgagcgcaccgcgctgatcgaacgggccaccaaggccaaaaccatgcagaagaccgaagcggtcgacgcggtcgtccgcgcctgcgaggagcttgccaaatgaagcacgctatccgtcatattcacttcgtcggcatcggcggctcgggcatgagcggcattgccgaggtgctgttcaaccttggctaccgcatcaccggctccgacctggccgacagcgcgacgctgcgccggcttgcgggcctgggcatcggcaccttcgtgggccatgcggcggcgcacatcgacggcgcggatgcggtggtcacttccaccgcggtgcagtcggacaaccccgaggtgctggccgcgcgcgagaagcgcattccggtggtgccgcgcgcgctgatgctggccgagctgatgcgcctgaagcaaggcatcgcgattgcgggcacgcacggcaagaccaccaccacgagtctcgtggccagcgtgctcgacgccgccgggctcgacccgaccttcgtgatcggtgggcgcctcaacagcgccggcgccaatgcgcaactgggcagcggcgactacatcgtggtggaggccgacgaatcggacgcctcgttcctgaacctgctgcccgtcatggcggtggtcacgaacatcgatgccgaccacatggaaacctacgggcacgacttcgaaaagctcaagaaagccttcgtcgatttcctgcaccgcatgccgttctatggcgtggccattctgtgcaccgacgatccggcggtgcgcgacatcgtgagccacgtcacctgcccagtcaccagctacggcttcgacgagggcgcccaagtgcgcgcggtcgacgtgcgcgccgtgggcgggcagatgcatttcacggcgcagcggcgcaacggcgtgacgctgcccgacctgcccatcgtgctgaacctgccgggcgagcacaacgtgcgcaacgcgctgtcggtgatcgcggtggcggtcgaactcggcattcccgacgaggcggtgcagcgcggtctggccggcttcaagggcgtgggccgccgcttccagagctatggcgaggtggcggtgcaggggtctcagcccggcagcttcaccgtgatcgacgactacggacatcacccggtcgagatggcggcaaccattgccgccgcgcgcggtgcgttcccggggcgtcggctggtgctggccttccagccgcaccgctacacccgcacgcgcgactgcttcgaagacttcgtcaaggtcatcggcaatgccgacgcggtgctgctgggcgaggtgtacgccgcgggcgagccgcccatcgtggcggccaacggccgcacgctggcgcgcgcactgcgcgtggcgggcaaggtggagccggtatttgtcgacgacatcaatgccatgccgcaagccattctggacaacgcgcgcgacggcgacgtagtgctttgcatgggcgcgggctccatcggcgcggtgccgggcagggtcgttgaaattgccgccacggcgcgcggcgcggaggttaccccatgacccttcaggatctaaaacaattcggcaaagtggccgtgctgttcggcggaagctccgccgaacgcgaaatctcgatcatgtccggcacgggcgtgctcgaggcgctgcgctcgcgcggcgtcgacgcgcatgccttcgatccgtccgagcgcgatctggtcgagcttcggcgcgatggcttcgcgcgctgcttcatcgccctgcatgggcggcatggcgaagacggcacggtgcaaggcgcgcttgaactgctcggcattccctacaccggctcgggcgtgatggcgtcgagcgtggccatggacaaggtcatgaccaagcgcatctggcaggccgacgacttgccgacgcccaggtacgtgcgcctggctttcgaccagcagagccgcgagcaggtgagggcggtgcccgatgtgctgggcctgccgctgatcgtgaagcccccgcgcgagggttcgtcgatcggcgtgaccaaggtcgagggctactcgcagatgcaggacgcggtggcgctatcggcgaagtacgacgccgacgtgctgtgcgaggagttcatcgagggcgaggaagtgacctgcgccgttctcggccaggggctcgaagcgcgcgcgctgcccgtggtgcgcatcgccgcgccgcagggcgcctacgactaccagaacaaatacttcaccgacgacgtgaagtaccagtgcccgagcggcctgcccgaagccgaggaacacgagatccagcgcatcacgctggccgcgtaccacacgctcggttgccgcggctggggccgcgccgacgtgatgatccgcgcgagcgatcgcaagcccttcctgctcgagatgaacacctcgcccggcatgaccggccattcgctggtgccgatgtcggcgcgcgcggcgggcattgcctacgaagacctgtgcctgagcgtgctggcctcggcttcgctggacgccaagggaggagcgcactagccatggccgatagcattcccgtgccttttgacgtcaagctcatgaacatcgtcgcgaacctggcgttcgtggtggtggcgctcatgctgctggcggcgggcgcatggtgggtgctgcgccagcccttcttccccatcggcggcatcaaggtcgacggcgacgtgacgcacaacaacgccgtgacgctgcgtgccaacgtggcgccgcaactggccggcaacttcttcacggtcgacctggggcgcgcacgcacggccttcgagtcggtgccgtgggttcgcaaggcggtggtgcggcgcgagtttccgaacaagctgcgcgtcacgctgaccgagcaggtcccggtggccacctggggcgacgaggccgggtccaagctgatcaacggctttggcgaggtgttcgacgccaacgtggccgaggtggacgaccggctgccgcggctcgatggacccgtcgagcaggccgggcaggtgctgggcatgtaccgcgtgctggcgccgatcttccagccctacgacttcggcatggaagaactcacgctgtcgagccggggcagctggaaggtggtgctcgataccggcgccgagatcgagcttggccgcggccagcccgaagaggtggcggcccgcacgcagcgtttcctgaaaaccgtgacccaggtcgcgggccaataccaccgcaccgcggcggacgtcgaaggggccgacctgcgccacaacgacgcctatgcgttgcgtcttcgcggtgtcaccacggtcgtgaccgaccccaagaccaagaagaaataaatagcgaataccgaggacattcaatgcccaaagaatacaaagacctggttgtcggactcgacatcggcaccgccaaggtgatggtggtggtggccgaggtgctgcccggcggcgaactcaagctcgccggcctcggcattgcgccgagcaacggcctgaagcgcggcgtggtggtgaacatcgacgccaccgtgcagagcatccagcaggccttgaaggaggccgagctgatggccgactgcaagatcagccgcgtctacaccggcatcaccggcagccacatccgcggcatcaattcgagcggcatggtggcggtgaaggacaaggaagtgaccccggccgacgtggcccgcgtggtggaaaccgcgcgcgccatcaacatctcgagcgaccagcgcctgttgctggtggagccgcaggagttcgtgatcgacggccaggacgtgaaagagccgatcggcatgagcggcatgcggctcgaagccaaggtgcacatcgtgaccggtgcgcagagcgcggccgagaacatcatcaagtgcgtgcgccgctgcgggctcgaggtcgaccagctgatgctcaacccgctggcctccagccaggcggtgctcaccgaagacgagcgcgagcttggcgtggtgctggtcgacatcggcgcgggcaccaccgacgtggccatcttcaccaacggtgcgatccgccacacggccgtgatcccgatcgcgggcgacctgatcaccagcgacatcgcgatggcgctgcgcacgcccaccaaggacgcggaagacatcaaggtcgagaacggctacgccaagcagctcttggccgaccccgacacgcaggtggaagtgcccggcctcggcgaccgcggcccgcgcatgctgagcaagcaggcgctggcgggcgtgatcgagccgcgcatcgaagaaatcttttcgctggtgcagcaggtggtgcgcgagtcgggctacgaagaggtgctgtcgtcgggcgtggtgctcacgggcggcagcgcggtgatgcccggcatggtcgagcttggcgaggacatcttcctgaagccggtgcggcgcggcattccgaagtattcgagtgcgctctccgacatggtggcacagccgcgcgccgccacggtgatgggcttgctcgaggaagcgcgcttcgcacgcatgcgcggcttcaaggtcgcgcagaagaacgggtccgtaaagactgcgttcggacgtttcaaagacttcatcgtggggaacttctgaccatgaatcactccccactctggctcgcacgcggcggtccgcccttgcatttcaacgagcgatggcggcgcacaggtccaccgccgcgacgacagcttcgttgaactcgtcaagacacttaaaagattcatacatacacaacggcaactgcaaattcaaggagttaaaaatgaccatcgaaatgatcgaagtcgaagaattcaatcaaggcactcagatcaaggtgattggtgtcggtggcggcggcggcaatgccgtcgcgcacatgatggaacgtggcgtgcagggtgtgcagttcgtttgcgccaacaccgatgcgcaggcgctccagcgcagcaatgcccacaagatcatccagctgggcaccagcggcctcggcgcgggcagcaagcccgacaagggccgtgacgcagccgaagccgcggtggacgacatccgcgccgccatcgacggcgcgcacatgctgttcatcaccgccggcatgggcggcggcaccggcaccggcgccgcacccgtgattgcgcgcgttgccaaggagatgggcatcctcaccgtgggcgtggtgaccaagcccttcgactgggaaggcggccgccgcatgaccaacgccgacaacggcctggccgagctcgaggcgaatgtcgattcgctgatcgtggtgctcaacgagaagctgctcgacgttctgggcgaagacatcacccaggacgaagccttcgcgcatgcgaacgacgtgctcaagaacgccgtgggcggcatctcggaaatcatcaacgagtacggcggcgtgaacgtcgacttcgaagacgtgcgcactgtgatgggcgagcccggcaaggccatgatgggcaccgccgccgccgccggcccggaccgcgcgcgcatcgccgccgaacaggccgtggcctgcccgctgctcgaaggcatcgacctctcgggcgccaagggcgtgctggtgctggtgaccgcatcgaagggttcgctgaagctgaacgagtcgaagctggcgatgaacaccatccgcgcctatgcctcgcccgacgcgcacgtgatctacggcgccgcctacgacgaaagcctgggcgaccagatgcgcgtgacggtggtcgccaccggcctctcgcgcgccgatgcacgccgccaggcaccgacgctcgaagtgatccgtaccggcaccgacaacatcccgttcaacgtgccgacgctcggcgcgggccatgcaggccatgcaggccatggcggccacagcgtgagccagccaaactacgacggcatggcggtgcccagcgtgtggcgcaccaaccgcacgatggcggccgccaaggtggacgcgctgtcttcgggcggcatggacgacttcgagattcccgcattcctgcgccgtcaagctgattgacgccaggccaccgaacgcagagggcacgaaggttcgcaaggggtacggggaagacctgaaagggacttctgccggctctaggcgctgcgtccgcttcgtgccctttgcgtccactatcgggcgcttgaaatagaacctatgtctatcggtgccatagcgaggggaataggccggcatgcgcgcagcgcgcctaaaatcccccgcgtgctgcaacaacgaacactcaagtcgatcagccgcgccgtgggcgtggggcttcacagcggacaacgcgtggagctgacgctgcgtccggctccggcggacaccggcatcgtgttccgccgcgtcgacctgcccgagccggtcgacatccgcatgactgccgaagcggtgaccgacacgcgcctggcttccacggtctcgaccggcggggcgaaggtgcagacggtcgaacacctgatgtcggcctgcgccggcctcggcatcgacaacctctacatcgacatcacggccgatgaagtgccgatcctcgacggatcggcctcgtccttcgtgttcctgctgcaaagcgcgggcatcgagctgcagaaggcaccccgccgcttcatccgcgtgacccgcaaggtcgaggtgcgcgaaggcgagggcgccaacgagaagtgggcgagcctggagccgtaccacggctacaagctgagcttcgagatcgacttcgatcatcgcgtggtcaattccaccggccagcgcgtggagttcgatctcggcaaggactcctacagccgcgacattgcgcgcgcgcgcaccttcggcttcacgaaggaagtcgaatacatgcgcagcaagggcctggcgctcggcggcggcctggacaacgccatcgtgatggacgacaccaaggtgctcaatgccgggggcttgcgctacgacgacgagttcgtgaagcacaagatcctggacgccatgggcgacctgtacatcatcggcaagccgctgctcgcggcctataccgcgttccgatcgggccatgcgctcaacaacaagctgctgcgcgaactgctggcgaacagcgacgcctacgaggtcgtgaccttcgaggacgagaagcgcgcaccgcgcggtttcggcgaagtggcgcgggcctggtagggcgccttcggccgatgcttctcttccgctgggccatcctgctgcttctgctggtggcgggcgtgtcgttcgcgttctatgccggaaccgggaaggtcaagtaccggcgccttggctggatcgtgctcaagtggacgctgctcgcggcgttcggcttcttcgcggtgctgatcgccgaacgggtggtgtagccccaggccaggaagccaaggcctgcaaggcctgtagctgctgcgccagcaagggtcccctgcgatgcagcggagccagcagcacgaccgtgtctcccaatgccttgggccgtccccacggcgcatgcagcttgccttgcgccaggagcggggccaccagccgttcgcggcccatgagcacaccttcgccatcgagcgccgcctgcagcgcaaggctgtagagcgagaagtccggacctgcggccagtgcgtcggcctctgccgcggtagtgccgggacgcacggcctgcagccagcgcgcccagtcgtcgtgccacacggtgtcgtgcaatccgccgcagcgggccagcacatcgatcaggtcatcgagcggacgtgggcgaccgctctgcaacgcctgctggatgcgcgggctgcacaccggcacgagccggtcgcgtgcgagagcgatgccttgcgcaccgacggctgcttcgacgtgatcgccggcacgtgcatagaacagccccagatcgaaaggctcgcgccggaagttcggcggctgctccaacgccgtaaccgagacctgcacgcccggcagcgccgccttcagccgcgagagccggggcgacagccacagctgcgccacggccggcaaggccgccacctgcagggtgctgcgccgcgcggcggtctgggtttcgtggcgcagcgactgaaccgcaaggccgagctggtcgaccgcagcgctgagcgcgggcagtgcgcgccgtccgtgcgcactgaggcgaatgccctggctgtggcgctcgaacagcgcgccgccggcccaggtttccagggccttgatctgctgcgcgacggcagccggcgtgacgaacagctcttcggccgcacgcgcgaagctgccgtggcgcgccgcggcctcgaaggcgcggacggccgtgtgcggtggcaggcgagggcggggtggtgcgagcggcatgaaaaaggagggcaagtatttctatggctcaggcccagattatccgtgttgccgttcgagaaagggcaggcgacgatgcggccactcaccacttccagcgagacacgccgcatgcccgccgccctccaacgccgaccctgggttcccgccgccagcgaagagcatgtgctcgccattgccggagatgccgccgcgcgcgatgccgcgggcgtggtggccgagatcgagaggctggtcgacgacaaccaccgcatccacgaccgggaagggctgaacctgaaccccgccaccaacgtgatgaaccccgccgcggaggcgctgctgtcgcgcgggctgggttcgcgcgcgtcgctcggctatcccggcgacaagtacgaggtgggcctggaggccatcgagcgcatcgaggtcatcgcggccgagctggctgccgaggtgttcggctcgaccttcgccgaagtgcgcgtgagttccggtgcgctgtcgaacctctacgtgttcatggcgacctgccagccgggcgacaccatcattgcgccgccgccggccattggcggccatgtcacccaccatgcggctggcgcggccggcctctatggactgaagaccgtgcccgcgccggtcgatgccgacggctacacggtcgacgtggccgcgctggcacggctcgcacgcgaggtgaagcccaggctcatcaccatcggcggcagcctgaacctctttccgcacccggtgccggccatccgcgagattgccgacagcgtcggtgccaagctgctcttcgatgccgcgcatctctcgggcatggtggccggcaaggcctggccgcagccgctcgaggagggcgcgcatgcgatcaccatgagcacctacaagagcctcggcggcccggcgggcgggctgatcgtgtcgaacgacgcagcgctgatggaacgcatcgacgccatcgcctacccaggcctcaccgccaattccgatgcggggcgcgctgcggcgctggcccgcggcctgcttgactggaaggtgcatggcaaagcctacgcggcagccatgcgcgacaccgcgcaggcgcttgcgcgtgccctcgatgccgagggattgccggtgtttgccaaggcgcgcggcttcacgcaatcgcatcagttcgctgtagcggccgcgcgctggggcgggggtcagcaggccgcgaagaagctcgcccgcggcggcctgctggcctgcggcatcggcctgcccatggcgccggtcgaaggcgacgtcaacggcctgcgactcggtgtaccggaaatcgtgcggctcggtttcacacctgaagacatgccgcagctcgcctcgtggatcgcccgggcgctcgaaggggacgcggtctccgttgccgccgaggtgcgcgagcgccgcacacgccagggcggcctgcgctacatcgttcgctgagtcagcgcgaacgtccttgccggtaggtgccggcgtgggtcttcgacagctcggcagcctcggccagccgcgccatcgaccggcccacctgcgcatgcgtgatggcaatgcccagtgcatcggccgcatcggcgccaggcagccccggcaggtcgagcagccgcttcaccatctcctgcacctgggccttggcggcctggccgtggccggcgaccgccttcttcatctgcagggccgtgtattcggccaccgtgagattgctgttcaccagcgaagtgacgcaggcgccgcgcgcctggcccagcagcagcgtcgattgcgggttgacgttgacgaagatgatttcgaccgccgaggcatcgggctggtagcgcgcggtgatttcggcgatgccgtcgaacagcactttgaggcgcgccggaagattgccgctgcccaggtgccgcgtgctgatggtgccgctcgcgacatagcgcagcgcatggccgtccgcatccaccacgccgaaaccggtggtcagaaggccggggtcgatgccgaggatgcgcatgtcagaggttgaagtaccagcggatcgagtgaaagaagatgggcgccgcgaagcacagcgcatcgacgcggtcgagcaggccgttcgcccccgtgacgcccacgcccttcttgccccagttgggaatgccgcggtcacgcttgagcgccttcatcaccaggtggcccatcgagcccgcgatgcaggcgatgacggacaccgcgagcgcctggccgaacttgaaaggcgtgatgaacgagaacagcgcgcccaccaggctggccaccccgatgccgatgccccagctggtccagttgaagctgcggctcacgttgggcgcaaagggcgtgcgctgcgtgcggcgcgaaatcacgtgctgtaccagcaccgaggtctgcaccacgaacaccaggaagaacacgagaaaggcactcttgccctcgtagcccggaaagctcaggagcagcagcgccggcacatggctcatgccgtagacgcagaccatgatgccccactgcagcttggcattgcgctcgagaaaatggcttgggtcgtcggccagcgcgctcgcgaccgggatcgcgaggaacacgtagaccggaatgaacacggtgaacaggtcgaagcgcgcggtggccacgagccagaactggattggcaacaccacgaagaacgccaggatcaggctgcggtggtcgccgcgccgcgtgggcgagagcgtgatgaactcccgcagcgcaaagaaggcgatgagcgcgaacagcacggtggccacggtttcgcccaaggcccagccgacccagaacacgatcaccatgaaccaggtggtgcccagcagttttcggtagtgcgccagctcggcttgccaggcggcgtcgtgcacggggttgcggcgctccctgaaggtcaggaagaaggccgtggtgctgacgatcacgagcaggccgaagacgatgagaaaaagggccgcgacctgctgggtcggggtgaggctgcgcaggaactggttcatgtcaggcgtcgcgcaatgcaatcaccgcggcacgtgcgcgatcgaggaagggacggcgctcttcgctttcctcgacgcggatcggcgcaccgaaagtgacggagcacaggatgggcaccggcacgatctcgcccttgggcatgacgcgctgcacgttgtcgatccaagcgggcaccagcaccacttcgggaaacatcgtcgcgagcgtgtagaggcccgacttgaacttctgcggctccccggtgtggccgcgcgtgccttcgggaaagatgatgatcgagtcgccgctgcgcagcgcctcgaccagcggtgccagcggatcgggcgcgggcggctccgttgctgcttccatggccggcggctgtaccggtgggagagggggcgggggaggaggtggtggtggcggagcggggaggtcgagccgcccctgaacttcgtccaccgcctcgggggtgacgtcgaccaggaacggcgtcatcggcagcagcggctccatggaaggctcgatccgctcggcttgcgctgcagccacgttccgcgcgggcgcaggcactggcgctggcggagcctcgggcgctggcggcgcggctggcgacgtggcacccgccggcgccgtggccgcgcgctccacgtacaccgcgttgaacacctcggtcgtgatccagcgcttgaacggcgtgttggcccagtagtcgcgcgccgcaatcggccgcgtgatgctgcgcaactcttcgggcagggcggcccagatcatcacgaggtcggcgtggctctggtggttggcgaaatagatgcgctgctcggccttcggcggacagccataccagcgtgcctgggcccccgtgagcaagcggacgatccccaacaacaaccaacccgtgagctttgccagcatgggcgcgatgatacggggcatgcgatggcgtttcgatcctctttctctggtgtgggcggtggccctgttgcttgttctcgtgctgctggccaccgtcggtgcgcgctggggctggttgcggagtttcttcggcgacgtgctggccgtggcgtgggtctacctcgtcttcaagagcttcgttgccgcgcgcgtgctgccgctcgcgctggcggcgctcggcgtgggcctggcggtcgaactggggcagttcctggcatcggcctggcacctgcacattccgaaccgcgccctgcgcatcgtgctcggcagcacggccgactggtgggatgtgctggcctacgtgatcggcttcgcggcggtgctggccgtcgaggcggtgtgcggcgccgtcagggcagctcggccgccggcatccgcgccacgatggtcgaaacccgcccgttgagataggacgagccgaccctgcgctcgaagaacttggggctgggcagcatcacggccaggcgcgcggcctcgccggcgctcaagcgcgaggcgggcttcctgaagtagtactgggacgccgcctcggcgccgaacacgccttcgccccattcgacgttgttgagatagatctcgaggatgcggcgcttgtcgagcagcacctcgagcagcgtggcgagcaccagctcctggcctttgcgcagcagcgtgcgctcgccggagagcagcaggttcttcgcgagctgctgcgtgatggtggagccgccgcgcagctgcaccgggcgcaccggcttgccgcgcgccacggcacgcgcggcgcgccgggctgccagctcctcggccttggcattgcgctgccgcgcgcgctcgatggcttcccattccacgccgttgtggtcgatgaagtcggcgtcctcgctggcgatgacggcacgcttgaggttgtcgctgatctgcgtgtagggcacccactcctggcgccatgcgcccttgctgccctgatggatggcgatctgccaggcttcggagcgctggaatgcggtgctctgcggatcgaccaccgccatggccgcgatgcgcgccacgaagaagagctccatcgccaggcccgccaacagcaggcaggcgaccaggcgcagcaggcccttcattggccggcggcgagcgaggcgcgcagctcggccagcacctctgcggcgggcgggcgcacgccgcgccagatctcgaaagcttcggccgcctgctcgaccagcatgccgagcccatcgcgcggcacggcaccgtgcgcctcggcccaggccatgaagccggcggcggcggggccgtacatcaggtcgactgcgagcgcgcccgcgcgcagcacctgcgcgcgcaccggcaccgcatcgcccgccaggctggaggcggtggcattgaccaccacgtcgaaattgccgggtacttcgtcgagcgcccaggcttcgagcgtggcgccgtggcgcagtgccagggcggcatggcgctgcaccagggccatcgccttgccgacggtccggttggccaccacgatgcgcgaggcgcccgcatcgagcaacggccccagcacgccggcggccgcgccgcccgcgccgatgagcagcagttcgcagcctgcgagcggcacggcggcgttgcgcacgatgtcgttgacgaggccgatgccgtcggtgttgtcggcgtgaatgctgccgtcggcttcgaagcgcagcgtgttgaccgcctgggcgagcagcgcccgctcgctggtgtgctgcgcaatggcggcggcgtcgaacttgaaaggcacggtgacgttgcagccgcgtgcggtgtcgccgcgctctgcggcttcgcgcctgaagccggcaatgccgtcggcaaaagcgccgatcggcacgagccggcggctgtagtccatctgctggccgcagagttcggcaaatcgggcatggatgcggggcgagcggctgtgctcgacggggttgcccactacgcagtacaggtccatggtgccgtgattcgccgttgttgcgatgctattgggaggagatctcgatggtttcgtcgcgcgtgaacttgaagcgcgactgcagcacgatctggtcggtctcttttcgcatcgcgtcggtgaacttgccgaagttgccgatgctgtgcacgatggccttggcacggcggtcgagcgtggtgtcgcccgagctttcatccaccacggtatcgagcagcttgccgtcgtggttgatggtgatcgtcatcttgagctcgccatagagcttcttgccggccgccgtggggaagttctcggtgcctcgcagctcgacgcggcggcgcagcgtgtccacgtagatggcataggccgcctcgcgggtggaggggctcaggtagcgcttcttggggcgtgcgttttcttcgttcacgcgccgttcgatttcggccagcagctccaccatctggcgccgcttttcctcgcgcgcaacggattccttcggatcgcccgaggcgcgcgggtccggcgcgggcatggcggccaagtcgcgcttgagttgcgcgagcaactgcatctgctgggcctgcatggcctcgacctggcgccgcgcttcctcgaccgagtcgcccacggcggtgaagctcgacggcggcagcgggctggtggcgcggccccgttcgaggtcgccaccgcccgcgagcgaggtctgcgccatcacccgggtcttggcgtcgggcttgtcgtgcgtcttgctgttgaccaggatcacttcgagcggcgtttcgctgaagacccggttgaacgactcggggtcgacgaagcgcaccgcgagaagtgcggcgtgcagaatgaccgacacgccgagtgcgatctgcagcgtgctcagatccctgaagttcatggacgacggtcctccgggctcattgaatggcctctgctgccctgcgggctgcggtgctgggcaccttcgggtggccgggcggtgctcatgccggcgtgttctcgggtgccgcctcgctgtcggtcaaatcgacggcaatggcgatggggcccgcgacttcttccagatcttcgtcgccgccttcttcttcctcggccgcggcatcggccttgggggcgtcgaggcgctcgagcaccgtgccgtgcacgtcgagcgcgatttcatcgatctcgccgagcttgacgcgcaggcgtgcgccgcgttcctgctggcccgccaccggaaacaccagcggcagcgtgtccgcgcgcaccagggcgccgttctggatgtccttgatgacggtcgcttcgatctcggtgatgccctgctgctccaggtacttgagcgtccagaagcgttccatgccgccctggtaggcgttgtaggtcgcgtaggcagcgtcgaagcccgaaagaatcgagaacaggtcggcatccttcggcttgaagggcgcggccagcgcggcggtcttgccgtggcgcgcggccgcgatgatctgccactggttcacgaggtcggtgtagcggcgcagcggcgaggtgctccaggcatagctcttcacgccgaggcccgcgtgcggcagcgcccgcgtgcccatgcgcaccttgatgccgggcgccaggctggcctggctgcggtagagcccgggcacgccgagttcgccgagccagccgccccagctgctgttggccaggatcatcgcttcggacacgatcaggtcgagcggcgcgccgcgctggcgcgtggtgatctgcacctgctcgctgccgttcggctcgccgtcgttgccgaccaggcggaagttgtagtcgggccggttgaagttctcgggcttgccgcgcaccacttcgcgctgggccttgagctgctttgcgagacggaacaggaaggagagcggggcgcgcagcttcgcagccgcctcgggcgtgttcccgttcgagaacgaggcgtcctcgagccagggctgcgtgacgacgctgtccagctggtcgtgccgcaggttggccacgatgggcacgcgttcgagcttcgtctcgctcgattgcagttcgagcgtggcttcgtcgaagcgcacgtagagcgacaccgcgggccggtcaccgccttcgagcagcgtgtaggcgttgaccacctcgtcgggcagcatggtgatcttgtagcccggcatgtagaccgtggacatgcgattgcgcgccacctggtcgatggggctgcccggcgtcagcgccaggccgggcgccgcgatgtggatgcccaccgtgacggtgccgctgcccaggccctgcaccgacagcgcgtcgtcgatctcggtggtttgcgaatcgtcgatcgagaatgcctccacgcctgtggcaaccggcaggtcgtccacgatggccggtgcggcgagcgccggaaaaccggtgcccttgggaaagttctcgaacaggaagcgccgccagtggaactggtaggccgagtcgatggcgcccgcgcgctccagcaaatcgagcggcgggcgctgcgtggcgcgcgcggcatcgaccacggccttgtattcgggcgcgttcttgtccggcttgaacaggatcttgtagagctgttcgcggatcggcggcgggcacacgccctcggccagctgaccagcccattcgacgatctgcgcctggatgacctttttcttctcgatggcggccagcgcctgctgcaggatctcggcgggcgctttcttgaagcgccccttgcccgcgcggcgaaagtagtgcggcgcctcgaaaagcgcaaacagcgcggcggcctgctgcgcgagcgtgggcttgtcgctgaaatagtcggatgcaagctcgccgtagccgaactctccctccggcgcaaattcccaggcgaggtcgaggtccatcgcggcggcgagggcgcgcgcttcggcgatcagctcggccggcgccggcttctcgaaacgcaggacgatgttggcgcccttgaccttgacgcgcttgcccgtgtcgagctcgacctgcgccgatgcttcggcctccgacagcacgcggccaccgaggtacttgccggcttcttcaaacaatacaaacatgcccggattgtcccagacttggtacacccccaggcttgcccgcttccgcggcgtgttgtccggacttcagatggggttgatgaacgccatcacgtcgtcgaggtggttttcctcgaagtcggacagcgcgtggtcgcctccctcgagcagcttgatgttgctgtcggggtagcgcgccgaggtttcatgccagtcgagcgcctcgtcgcccttggcgatgatggccagcacgcgctcggggcgcgtgagcgcgccgacttccatggtgcgcagctcctggatgtactcgggccgaaaatagaaatgctcggccgggtcttgccacgtggtctggtcgccgatgtagagcgcgaggtcgcgcgccggatgcaccgccggattgagcagcacggtgcggcatcgcgtcatgcccgccacataggtggcatagaagccgccgagcgaagaacccaccaccgccatcgacttgcgcggccagtccgcgatgcccttcatgatcatgtcgatggcttcgcgcggagagggaggcaactgcgggcaccaccactgcaggtccggatgctcccgtgccacgcgctgtgccatgagccgcgccttggtcgaccggggcgaggagcgaaatccgtgcaggtacaacagatgagtggtttgcgggtccatgcgtggtggagactgaaagtggtgcggtcgactcaactccttcggtaaaggagccgggtaattttgcatgaggtccatgggcgcaaagcgccctccggagcccaggtctccgggatgcgggcttcttgcaggaaggtgtcggtgtaccactgtggccccctgagcgcggggattttctttgctcgatctgctcggcgtctgccttcgggaaatcgaaagtattcaactttcgcctgcggcgatttcggccgggccgcaggtgtggcaagccagcctcagtttcgcggcccgcggaggcggggggcatcccatgaaaacgggaggcttcgcggccgtgcggcctagcgccgaggcttatgctcacgccatgaacatcgaggctctggatgcgggactgacacgccgttggggcgtgctcgtcgtcgaggacgacagccgcgcgcgcgccttcttcgaggccagcgtgcagcgcagcccgcgcctgttctggctgggaagcgcaggcacggtgcaagaggcgttggcctggctggcccagaccagcaccattcccgacgtgctgctggtcgacctcggcatgcccgatggcagcgggctggacgtgatccgcgaggccgtggcgcgctttcccggctgcgagccgctggtgatttccgtcttcggcgatgaagaaaacgtgctctccagcatcgaggccggtgccgtcggctatatccacaaggacgccgcccccgaggacattgcacaaaccatcgtcgagatgaaggccggcgcatcaccgatctcgcccatgatcgcgcggcgcgtgctcgccaaataccgcagcttgcaactggcgggcacccccgccaccgtggctgcgcccgaggccgccgccgacatcgcggcgccgagcctgctttcggcccgcgaacatgaagtgctgacgctgatcgcgcgcgggttctcctatgcggaaattgcgcggctcaaggggctgagcgttcacacggtgcagacgcacatcaagaatctctacggcaagctggcggtgcattccaagagtgaggccgtgttcgaagccacgcgcctcggcctgctgtcccacccgggctgaaccacgtggccgggcgcatgttcggaggcccggcacgggctcttctcgccatggggctcgcggtgatgctgctggtcgcggcgcgtgccgcagcggctgcgccggcggagatcccgatcgaattgcggcgcggcaccgtcactaccaccatcgacggcgtcacgcaccaggcacccgtcgagctgtcctaccactgggatcgccggcacgccggacgcccgggtcttgcggatttcgagctgcctttcacgctggcggccgagcccgcgacgccctggggcatcttccttccccgcgccggcaacgtgctcgaggtgcggctcaacgacgccttgctgcaggcttttggcgacctggcccggggcaacggcgccgactacgccaaggcgcccatctatgtgccggtgccggggcacctgctgaaggcgggcgacaaccgcctgcagattcgcatccgcgccgacagcgcccgccgcgccgggctttcgcgcgtgaccatcgggcccgcgacgccggtgcgcaccgagcttttcgagcgcgcctatgcctggcgctttaccggctccgtgctgctgaccgccttcagcctcatcgtcggcggcatcgcgctggccttgtggctcacgcaggtcgatgccggtgccgatggacggcggcggcgcgacggcatctatttctgggccgcgctggccgagttctgctgggccttgcgggtggccgacggcgtgattgccgaaccgcctctttcctggggcttctggggtgtgctcatggccacctgctatgcggggtgggccgcgtccgccatgatgttctgctaccacctggccggctgggacggcaacccgcgcatgcgctggctgcgctggccgatggccgccgtggtggccggaaccttcgcggcgagtgccatggcgctgtaccgcgagcagccctattggctcaccggctggctcgcgctggaaatcgtgctcgttacgctgttcgtcggcgcctttgcggtggcgacggtcaggcggccgaacgtggggcgcctgttggtggcggccgcggcgctggtgacgctgggcttcggcacccgcgactggctcgtgatccgcctgagcgatgcctacggcgagaccacctgggtgcggtattcgtcggtgttcttcggcattgcgctgctcctgatcgtgcttcggcgcttccatgccgcgagcgtcgaggcgcgtggctgggtcgcgaccctggccgagcgcgtggcgcagcgcgagcgcgaactcgcgtccaccttcgcggcgctggagcaggtggcgcgcgaccaggcgcgcacccacgagcgcgaacgcatcctgcgcgacatgcacgacggcgtgggttcgcacatcagctcggcgatccggcagctgcagtcgggccaggcgagttccgatgaactgctgcgcacgctgcgcgattcgctcgacaagctcaagctgtcgatcgattcgatccatttgccgcccggcgacgtcggcgccctgctggcggcattgcgctaccggctggagccgcggctggcggccgccggcatcgcattcgagtgggcggtggacgaggtgcccgcggtaaagcggctcgacgcgcagggcatgcggcaattgcagttcctgctgttcgaggccatttccaacgtgctgcaacacgcccacgccaagacgctccggatcgaggccgaaaacctggccggtgccgtgcagctgcgcgtggtcgacgacggacagggcttcgacacatcgcgcgtgcccagggcgctttcggagcgcgccgtcacggtcggcgcccggctggcgctcgaaagccgaccggggcgcacggtcgttcggctcgatttcggctgaggtacctcgcggggcgcggataatccgcccccatgtccgccgtgttcaatcagccctccctggcgcgccgagtcgcgcccatcttccagggcttcgacggctttctggcctttgcagtcctgctgctggcctttgccggactgctcaccatgtattcgtcgggctatgaccacggctcgcgcttttccgaccatggccgcaacatgctgctggccggcttcatcatgttcgtggtggcccaggtgccgccgcagcggttgatgatcttcgcggtgccgctctatgccaccggggtggcgctgctggtggcggtggcgctattcggcatcaccaagaagggcgccacccgctggatcaacatcggcgtggtgatccagcccagcgagatcctcaagatcgcgatgccgctgatgctggcctggtggttccagcgccgggaaggccagttgcggccgctcgatttcgtggtggccacggtgctgctggcggtgccggtggggctcatcatgaagcagcccgacctgggcacctcgctcctggtgctcgcggccggcatggcggtcatctttttcgccgggctgtcgtggaagctgatcgttccgccggtggtgatcggcgccattgccgtgacgctgatcgtgggcttcgagtcgcagctgtgcgccgacggcgtcgactggcgcgtgctgcacgactaccagaagcagcgcgtctgcacgctgctcgatccgagcaaggacccgctgggcaagggctttcacatcatccaggggatgatcgccatcggctccggcggcgtgggcggcaaaggcttcatgcagggcacgcagacgcacctcgaattcatccccgagcgcaccaccgacttcatctttgcggcctactccgaggaattcggcctcgtgggcaacctggcgctgatcgcggccttcattctgctgatcttccgcgggctggccatcgcggccaacgccacgacgctgttctcgcggctcctggcgggggcggtgacgatgattttcttcacctatgccttcgtcaacatgggcatggtgagcggcatcctgcccgtggtgggcgtgccgctgccgttcatcagctacggcggcaccgccatggtcacgctggggctggggctgggcattctgatgtccatcgccagggcccgcaagctcgcccagaactagggccgtacgcaaagcgtgggagcgagcaataatcccttcatgatctctcgcgaacccaccatcgagcgccttgccacggcgcaacagcttcttctcacgccgttcggcctcgacgaatcgcacctgggcaaggccctggccgagatcaccgcgcacaaggtggacgacgccgacctgtacttccagtacacgcgcagcgaaggctggagcctcgaagagggcatcgtcaa
